European Patent Application EP 4 635 975 A1 - sequence listing, part 2

SEQ ID NO: 201 - DNA, 4641652 bp, Escherichia coli (residues 2,320,827-4,641,652 of 4,641,652)
  source 1..4641652: mol_type = genomic DNA; note = U00096.3, strain K-12, substrain MG1655, complete genome
cacttaacgatctgattattgaaaacgctgccgatggcgtcattgccattgaccgccagggtgatgtaaccaccatgaacccagcagcagaagttatcactggctatcaacgccatgaactggtagggcagccttactccatgttgttcgacaatactcagttctacagtccagtactggatacgctggaacatggcaccgaacatgtggcgctggagatcagttttccaggtcgtgaccgcaccattgaactcagtgtcactaccagtcgtattcataacacgcacggtgaaatgataggtgctttggtgattttctctgatttaactgcccgcaaagaaacccagcgccgcatggcgcaagcagaacgcctcgccacactgggtgagctgatggctggcgtcgcgcatgaagtacgtaatccgttaacggctattcgtggttatgtacagatcttgcgccaacaaaccagtgacccaatacatcaggaatatctgtccgtagtactcaaagaaatcgattcaattaacaaagttattcagcaattgctcgaattttcacgtccacgccacagtcaatggcaacaagtcagcctcaatgcattggttgaagaaactctggtactggtacaaaccgccggcgtacaagcgcgggtcgacttcataagcgaactggataatgaattaagcccgattaacgccgatcgtgaactgctcaaacaggtactactgaatatcctgatcaatgccgtccaggctatcagcgcacgagggaaaattcgcattcaaacctggcaatacagcgactcacaacaggccatttcgatagaggacaacggctgtggcattgatctctcgctgcaaaaaaagatcttcgatccctttttcaccaccaaagcctcaggaaccgggcttggtctggcgttaagtcaacgcatcattaatgcccatcagggtgatattcgcgtcgccagtttgccgggctacggcgcaaccttcacgcttattttaccgatcaacccgcagggaaatcagactgtatgactgctattaatcgcatccttattgtggatgatgaagataatgttcgccgtatgctgagcaccgcttttgcactacaaggattcgaaacacattgtgcgaacaacggacgcacagcattacacctgtttgccgatattcaccctgatgtggtgttgatggatatccgcatgccagagatggacggcatcaaggcactaaaggagatgcgcagccatgagacccggacacccgttattctgatgacggcctatgcggaagtggaaaccgccgtcgaagcgctacgctgcggagccttcgactatgttattaaaccgtttgatctcgatgagttgaatttaatcgttcagcgcgctttacaactccagtcaatgaaaaaagagatccgtcatctgcaccaggcactgagcaccagctggcaatgggggcacattctcaccaacagcccggcgatgatggacatctgcaaagacaccgccaaaattgccctttctcaggccagcgtcttgattagcggtgaaagcggcaccgggaaagagttgattgccagagcgattcactacaattcgcggcgggcaaaggggccgttcattaaagtcaactgcgcggcgctgccggaatcgttgctcgaaagtgaactgtttggtcatgaaaaaggtgcatttactggtgcacaaaccttgcgtcagggattatttgaacgagccaacgaaggtactctgctcctcgacgaaattggcgaaatgccgctggtactacaagccaaattactacgcattctacaggaacgggaatttgaacggattggcggccatcagaccataaaagttgatatccgcatcattgctgccaccaaccgcgacttgcaggcaatggtaaaagaaggcaccttccgtgaagatctcttttatcgccttaacgttattcatttaatactgccgcctctgcgcgatcgccgggaagatatttccctgttagctaatcactttttgcaaaaattcagtagtgagaatcagcgcgatattatcgacatcgatccgatggcaatgtcactgcttaccgcctggtcatggccgggaaatattcgagagctttccaacgttattgaacgcgccgtcgtgatgaattcaggcccgatcattttttctgaggatcttccgccacagattcgtcagccagtctgtaatgctggcgaggtaaaaacagcccctgtcggtgagcgtaatttaaaagaggaaattaaacgcgtcgaaaaacgcatcattatggaagtgctggaacaacaagaaggaaaccgaacccgcactgctttaatgctgggcatcagtcgccgtgcattgatgtataaactccaggaatacggtatcgatccggcggatgtataacaccaaaacttgctatgcagaaatttgcacagtgcgcaattttctgcatagccgctcattctccttataaatccccatccaatttatcccttcatattcaattagttaaataactaaatccaataatctcattctggcactccccttgctattgcctgactgtacccacaacggtgtatgcaagagggataaaaaatgaaaacaaaattgatgacattacaagacgccaccggcttctttcgtgacggcatgaccatcatggtgggcggatttatggggattggcactccatcccgcctggttgaagcattactggaatctggtgttcgcgacctgacattgatagccaatgataccgcgtttgttgataccggcatcggtccgctcatcgtcaatggtcgagtccgcaaagtgattgcttcacatatcggcaccaacccggaaacaggtcggcgcatgatatctggtgagatggacgtcgttctggtgccgcaaggtacgctaatcgagcaaattcgctgtggtggagctggacttggtggttttctcaccccaacgggtgtcggcaccgtcgtagaggaaggcaaacagacactgacactcgacggtaaaacctggctgctcgaacgcccactgcgcgccgacctggcgctaattcgcgctcatcgttgcgacacacttggcaacctgacctatcaacttagcgcccgcaactttaaccccctgatagcccttgcggctgatatcacgctggtagagccagatgaactggtcgaaaccggcgagctgcaacctgaccatattgtcacccctggtgccgttatcgaccacatcatcgtttcacaggagagcaaataatggatgcgaaacaacgtattgcgcgccgtgtggcgcaagagcttcgtgatggtgacatcgttaacttagggatcggtttacccacaatggtcgccaattatttaccggagggtattcatatcactctgcaatcggaaaacggcttcctcggtttaggcccggtcacgacagcgcatccagatctggtgaacgctggcgggcaaccgtgcggtgttttacccggtgcagccatgtttgatagcgccatgtcatttgcgctaatccgtggcggtcatattgatgcctgcgtgctcggcggtttgcaagtagacgaagaagcaaacctcgcgaactgggtagtgcctgggaaaatggtgcccggtatgggtggcgcgatggatctggtgaccgggtcgcgcaaagtgatcatcgccatggaacattgcgccaaagatggttcagcaaaaattttgcgccgctgcaccatgccactcactgcgcaacatgcggtgcatatgctggttactgaactggctgtctttcgttttattgacggcaaaatgtggctcaccgaaattgccgacgggtgtgatttagccaccgtgcgtgccaaaacagaagctcggtttgaagtcgccgccgatctgaatacgcaacggggtgatttatgattggtcgcatatcgcgttttatgacgcgttttgtcagccggtggcttcccgatccactgatctttgccatgttgctgacattgctaacattcgtgatcgcgctttggttaacaccacaaacgccgatcagcatggtgaaaatgtggggtgacggtttctggaacttgctggcgtttggtatgcagatggcgcttatcatcgttaccggtcatgcccttgccagctctgctccggtgaaaagtttgctgcgtactgccgcctccgccgcaaagacgcccgtacagggcgtcatgctggtcactttcttcggttcagtcgcttgtgtcatcaactggggatttggtttggttgtcggcgcaatgtttgcccgtgaagtcgcccggcgagtccccggttctgattatccgttgctcattgcctgcgcctacattggttttctcacctggggtggcggcttctctggatcaatgcctctgttggctgcaacaccgggcaacccggttgagcatatcgccgggctgatcccggtgggcgatactctgttcagtggttttaacattttcatcactgtggcgttgattgtggtgatgccatttatcacccgcatgatgatgccaaaaccgtctgacgtggtgagtatcgatccaaaactactcatggaagaggctgattttcaaaagcagctaccgaaagatgccccaccatccgagcgactggaagaaagccgcattctgacgttgatcatcggcgcactcggtatcgcttaccttgcgatgtacttcagcgaacatggcttcaacatcaccatcaataccgtcaacctgatgtttatgattgcgggtctgctgctacataaaacgccaatggcttatatgcgtgctatcagcgcggcagcacgcagtactgccggtattctggtgcaattccccttctacgctgggatccaactgatgatggagcattccggtctgggcggactcattaccgaattcttcatcaatgttgcgaacaaagacaccttcccggtaatgaccttttttagttctgcactgattaacttcgccgttccgtctggcggcggtcactgggttattcagggacctttcgtgatacccgcagcccaggcgctgggcgctgatctcggtaaatcggtaatggcgatcgcctacggcgagcaatggatgaacatggcacaaccattctgggcgctgccagcactggcaatcgccggactcggtgtccgcgacatcatgggctactgcatcactgccctgctcttctccggtgtcattttcgtcattggtttaacgctgttctgacggcacccctacaaacagaaggaatataaaatgaaaaattgtgtcatcgtcagtgcggtacgtactgctatcggtagttttaacggttcactcgcttccaccagcgccatcgacctgggggcgacagtaattaaagccgccattgaacgtgcaaaaatcgattcacaacacgttgatgaagtgattatgggtaacgtgttacaagccgggctggggcaaaatccggcgcgtcaggcactgttaaaaagcgggctggcagaaacggtgtgcggattcacggtcaataaagtatgtggttcgggtcttaaaagtgtggcgcttgccgcccaggccattcaggcaggtcaggcgcagagcattgtggcggggggtatggaaaatatgagtttagccccctacttactcgatgcaaaagcacgctctggttatcgtcttggagacggacaggtttatgacgtaatcctgcgcgatggcctgatgtgcgccacccatggttatcatatggggattaccgccgaaaacgtggctaaagagtacggaattacccgtgaaatgcaggatgaactggcgctacattcacagcgtaaagcggcagccgcaattgagtccggtgcttttacagccgaaatcgtcccggtaaatgttgtcactcgaaagaaaaccttcgtcttcagtcaagacgaattcccgaaagcgaattcaacggctgaagcgttaggtgcattgcgcccggccttcgataaagcaggaacagtcaccgctgggaacgcgtctggtattaacgacggtgctgccgctctggtgattatggaagaatctgcggcgctggcagcaggccttacccccctggctcgcattaaaagttatgccagcggtggcgtgccccccgcattgatgggtatggggccagtacctgccacgcaaaaagcgttacaactggcggggctgcaactggcggatattgatctcattgaggctaatgaagcatttgctgcacagttccttgccgttgggaaaaacctgggctttgattctgagaaagtgaatgtcaacggcggggccatcgcgctcgggcatcctatcggtgccagtggtgctcgtattctggtcacactattacatgccatgcaggcacgcgataaaacgctggggctggcaacactgtgcattggcggcggtcagggaattgcgatggtgattgaacggttgaattaatcaataaaaacacccgatagcgaaagttatcgggtgttttcttgaacatcgacggcgaaggtaaccccattaatcaccagtcaaaacttttcaccagcgtcagctcgccagcattacgcatcggtacaataaatgtttcctgtttctcattgaccgatccttcatcggtgatcagcgtcagttgggcggtggttaattccgtttcgctgcgcccaccatagtagttgatatacacctgatagcgcccgtgaattggcgcgggcatggcgaaaatctcgggtccgtaccccgtcgtgacatccatatccagtgcaccactgtttttcagcacggtgttaccgtaccaggcgtgttcgccatcgggcgtaacaacgtgaaggtcgaggtcggtattgtccgtatcccacgagagaaccagccgtaaacgtgcacgaatcgttcctgtacccggcgttgagtaaaactgcattttttgtcggctttgcccatccgggctgatgacctgcacgctgttgctgccttcagtgaaaatataagggcgtgcaaatgaaccatcggattcaattctctgcggcatactggcaccgttgaccaccagccggccctgctgaactttacccgccgcagcataattctttattttgccgcggatctgcgctgagatattttgatcatctgccatgttgacggacgacgccgggtaattgatcgattgtgaaaaactggcatcttcgccctctgccggatgccagcctgagagcggtgcatcaatctcgacttcctgcacaccttcactgtgagcgacaggcgaaagcgccaccagtaacaacggaagaaaaatctttcgcatagcattagtccattaataattgtcgggtcagcgtttcgatatagttctcatcaagcccggtgggataaccatcaaaggccaggtgcagatactcatgggttaaatccagccgatcctgaagcgtaaagaagttacgaataaacagccgtttctgctgccgatcggtataggggaaacctgagactaaacggcaaaccgcaaacacgtctggttcgttgtaccccgtctcagcttgtaatatacgccgccactgcggcatttttttcgccagccaggctttcgctttgggtaataactggcaggttgagcgtggcgctccccagcggctaagactgttgtcgggataagcaaacgcgagtatctgatcgtaacgctctccctgccccgcctgggccgtggcttgccgccaggaaagtgtcccttcggtagcgcgactgccatgataatgaaccggatcgcctgcatagatgagatcctgcgtccaggcggtcatcgttcgcgcccccgtggtcgctggcgaagcagaaacacgctgcgtggcgctgctgtcggggatggtcaggcaatcgccttcccgattggcgttttgctgtaaaaaagtgcgaatcgccacggtcatggctttcgctgcctcagggggcgtacttttcgcctcgcgatccagaactctggcaacgtactcttcacgatcgagatgcgactgcaatttcagtttgcccttttcgctcagtaaggtcgtctcaccgtggctgacaaacgtaatgtggttaccattagtaaacgtcacacgatagcgcccattaagtacgccgggatttactgccgtcgtactcttttccgctgtgattttcttcagcggatagcgggcaaacagctccacctctacacattgcccactggcaacctgcgtcggcactggcaaaacccgattaagcaccgtcgcataacgggttagtaccgttttgctggtgccactgccagtaacccacagcggtgtaccatcggttaaccagccagcaaaaccaccctgacggatttcctgtttatcatcggcaaaccagctccaggttttcacccgtacccgactaccgagcatggatgcgacaccgattttcgcctcgtccagcaccacatccagtaagacttcctgagctttgttttgcgcgggtaacgtcgctaatgaatcaagcagcgatttaaccgttaccgaggtttctggcttcagcgtagtcagagacgctaaccacgcaggtgcctgacgctgttgccagtattgcccccacacatctgcgccaatatgcaaccgctgcggcgcaaaatagagcccacaggaacgtaccagcgcggtatcgcgcgttatgctctccccagcctgacaacaataaacctcttccggggagtttccgcgacactggtagggctgctccggttgatgggtatcctccagccaggcgtaaacatacagtttccacaaactccctaacggcgtggtgagcgagtcaggtaatgctgagactttggtcacgcctgatgacgacagctgatacagttgatcgtgctgcgcaccgcgcagcaccagttgtaacggcgtctcctccgcaagtgttggcagagtaaccaacgccaatagccagacgattctgcgccagttcacttatttcacctgcatcccggtccattcactccctgccgcaacactttgctgcgcaggtgcataggaacgcacataacgagcaggaggcagaacgaattgccctttttgcgagaagcgcagcaaatggcggaaagtgaccgttcccgtcagttctttcaccggcaccatataggccagttcgcccatttcatttcgcgctttttccagcaattgcccctgctgtttcgcggcgttgggtttattgaccgaaatgccccatgttgtgcgctcaacgtcggctcccggtggcagcggtacttccacctgaccgtagcgcagaactgcatcctgctcgctggtaagcgtgatttcatcgagatacagcgcatcgctgtcaatctcattgctggtcaccggttgcagaataaagctcatctcttcttcaccagggataagccgatacaactggcgttcaacggtcaccggaatgttactttgttgagccatttttgccggctcacgtcagcggacctgcacattttgcggcgataattcgtcaccaaaagagagaatgtccggcacgccctgaccaacccaacgccagtcttcgccccctccagttaacttatgtttagcccatgcgcccgcaggcgcaggcaaaacaactggaggcattgtcgccatatatttcgccagccagttcatggccagcgcgcgctcaatagtggattgctcagcggtcaaaccacttaaaatagcggccgtctgggtagcgtcgccaccgctattaagcagcacaaccgtgtgcgccagcggctgattgctgtttgccgctttatcccacgcatattgctgaacctgtggcatcaccgtggacttcaactgcgcttttttcagcaacgtcatggttaagacgtttgccaccgcatctgccagtggagactccggtgtatcgaggatcaggctatcattgatatcgcgggtgtcttcctcagagaaatcttcagttttagttccgcgccgggcgatagcttcatccaaccctttcaacaacgttttgcacggcaaattcatctcctgcgcccatgccagcaccagcgcccgatgcaataacggcatgttatctgcctgctccgcgtagctgtcgagcatatgctgccagtattccggttgttgcgttacgccgatcgcctggctggcctgccagtcggcgtaccatgcccatgccgtaaggaaggcgtcaccattgccatcttcaccccaccaggtaaagcgcgctccgggccccgccagttgcatcagccgcagacggttatcctgaatcatctgacgaatgtcgttagcggcggcactttgatgatcggcaagcgaacgccaggcgagactgagcgggatcagacggctaccggtgttgattacgccaccccacggttcatcgactaacgcatcaagattgttgcggaaaatctcctgcggcgtttcactactttgtagccggatattgctcgcctgctcgggcaacatcagcgcgttatcgccaccaccgagcatgacatttttctgctgttcaacgggccagctgttatccacaaaagacagttttgtgctaatgctgtcctgcacttgcccattttgttgcagttctgcacttaacaagccagattgctgaatattctgcgtcagcgaaatataattcgcccctttgtgcagcgtcagcgtctggcgcatctcagcgcctgcaaatttagtcaccagcgccaccggttcgttatcctgctgactgaagataaacagtcctgccgccggtttgtcgcccacgcgatacaccgttggcatactccacttcatgtagagatttttttccgaacgcagataagcacgcccctgcccgaccagcccgtcgccgttcatcccacgcgcggtgatacgccagcgggttaacgaatcaggcatcaggaacgtgaaatacgctttgccttgtttatcggttgtgagtgacggcatccatgccgcggtatccacctcttcacgccgtggacgttcaagcatttttactcgccgctcgctgcggttagttgcgccaggcgcaaccggctcgctggagagcgcctggtcgtagctgataaacgacagactggagctggtacgcacattgttacgccccagcggatagaaaaatttgccgatattcggcgcgatttctggttgcagcgcgtagatcatttcatcgaccacgcctaccgttagctgcgcagaaacaggtttacctttcagcgacgaggttaattcgacattgaccagttcaccaggctggtaatgggttttgtccgttttcacccggatatccagctggggaacggcaactttgatcccggcgttctgaaaactgtactgaccgttacgggtatacagcaccgaaaaagtgatgttaggcgcaaaggaattgctcactggaacccgggcttcatactgggtatcgtttaaacgttgtagcgttagccagtttgccggatgcgaaagcagcgactgctgttccacgcgatcgcgttccagcgtcaataatgcttcatcaattggctccggaaaggtaatcagcatcttcgcggtttcgcctggctggtacagcgttttatccgccacgatatctaccgtaccagtatgcgccgtgctgcccttaccgctgacggcatgacttaacccagcgagaattaagccgtctttatcgcgtaatgtcagattgtagttgccaggtttagcgaaattgacggtaaaggatttgccgcctgacggtagctctccgctatggctcgtgcggtcttcgagacgcaaccattcatacgtaacaggaacctgttttgaagattccagcgcggcataacggaacacaaccgactcgccgctattactgtattgtgcggcagtacttaatgagtaatgcgccagaccgcgttcaatgaggatctctttggtggtggtgacgcgatacgccgcgccgtcactggcggagacggttaacaaatagcggctcggtttatcggcggcggggagatttaacgccacatgaccgctggcgtcggacaccgtttcgctgccttccagcgacacggggaaacgtccggcataacgcaaatcgttaccgaccattgataattgctgagcgcgcaaacttaactgcacgcgggcattttttaccggctcgccatccgggtagagcagttgcagtttgccgctgaccgcttcgccagttttgaactcttttttggcgagagctaaaccaatctcgaaatgtggcttgatgtagtttgccacgcgaaaactgctgctatagacctgattgcggtaagcaagacgtaactcataacctccggctacggcattttctggcaggcggaaacttccctgcccgccattgcgcgcatccagcgtgacattgacggtttgcaacagactgccgttggcgtccagcaccgaaagcttcgccggggcgctgacgatgggggatgaatgcaacggatcgtggaactcgcggccgatcactttaacatcgacacgatcgcctgcgcgatatagcgggcgatcggtaaaaatatacaagcgggtgttgtagatttcgctttcgtagaagaagttctcggagacaaaaacgccgccttcagcatccttacccagaatgtatgaacgttctggcgatatatgttgtaactgcaaggtaccgctgtcatcggtcacaccgcgggtcatcacgccaagaccgtcagtccacaagatctctgagccgggcttcgcttcaccctgttttttacccgcggtccacaccagaagctctttgcctgacactttgctaagcgccacggtatcggaaacaaacaccaccgtcgtcgcccgatacccaccaaccatcgcctcgacgaggtacagtcccggctcttgttggccgagaggaatataaatgttacccggctgcggcgagatgaaattgctggatgcgccttccagttttaccccttgctgcggctcgaacggtttagcctgccatagtggataacggaactgtttcaccaggggatattttttcagcggggaaaactggttgttctgtacataacgggaaggtttaataatggcattgccgagctgtaattcgggtaacgcctgagtcacattctgccgtgactgagaagagaaagtacgctgcatcacgcggcgagatttgccgtaccagttatcccacagccaggttagcgtattgttcagcccgtcgcccagatattgcggttgcaccacaatgcgatgcaggtttttctgctggcgcaaaaatgccatcgggtcaggaatacgatacaggcgaacgtccacgccgccgtactcttccatctgatagcgccgataatcacgccccggcgcttccagtcgcactttcgcctcttcactgctgctaaaactgctgtcagcaagcaaaaagaatgttcccccggcaggcggcgcatagttgctggaaggaagcgaatcatcagcattagcaagccctgttcccacaagagacagggacaagcacgctgctatcgcgccagaaaatttaaacgataaatgccaatgaaattgggattggaatcgttgggtatccatcgggtgtccttccatgtcataagttgttgcagactgactgcgcgcattccgttgtcagttttcgtggcgcttccggtgtggtagatgacgtaacgccccatccagaccattaagtgctgggcatcgccctgatcgaaaaaaatcatatcgccaggcagcgcctggtttatgtcctggccaataaactggctgttgtactgaatcaaattaatcgcggtcacataggggccggttttcccgttcccctgattccagttttgcgccagttgacgctgttcaggtgttagcgtcatctctggcggcaaatactggctagataaaccgttactttttagccatttactgtcgtgaactttcagcgtctcgttcgccgcaaatcgcaccaggcccgcacaatcctgctgataccagcgtggacttggcccctggcggagctgttcttgtgcaatgcgtacaaaccaggcgcgaaacagcccggattgttcgacattcagcatttcgctatgggcaacaacacaacacagccagcaaatcagcgccagcagcccgtgcctcatagcggctgccaggttatgggtagccactgccaggcggcaccgggttccatctgggccagcttcatgacataacgcggttgttgagataaagcgtccagcttcggcattaataaagtttgtgcggcgttataaaaaaccggttcgagattcttcggcagactggtcaacgtttcgttacgcagcagtttcgctattccttgtggattgatatagagcggaacgatgccatcagtgggtattacatccaccattgccgggcgggttttattcagtgtttgcagcgcgttattaaccagcgtgtcatcgagggagaaaagcagcgttttgttttgcatcgccagcgacacacggaaaaaataatccgacattaattgatcgggttgcgccgcctgcgctttcggatactggccgtatcgggaactcacttcgcgacgccagatttgcgcttcgccctgctgagtctggcttaccggcaaaacaccttctggcgctttgctttcgtgcgcaccaatattttgcgtaaacagtttccctggcaattgcgcctgttcggcagtgccatcaaactgaccgacaaacagcggggtttgcaattttgagtcttcataccagcacagccccgcggcaccgtctaacgccccattcagcttgtcgttttcctggctgatgtgcgaaagcatctcttcggcaataccgtgtgaatacggcaccgccacacagaagctggctccggcaggcatactgttccataccggcgtaaaatcgaaactggcatctacgctggcggattcatcatttaacgccacaaaactgtgccagccgtcgttacccatttcgaagcgtacgccagcaaaagaaggcattaaccgctggtagccaaaccccagccacctggcgctgactacgatgcgctggcgtactggcgttttttcggcagtacgctcttccaggccaaagcttgcttgccagcgttttttgccgctcaacaaatcacctgcgatcgccgtggcttcggtatcctgctgatcatctttaaacaacatatccgtgctggaaaacaccagcatcttgtcctgataagtcgcgaacatcagggcgttattgccgttatagcgcaactgataaacaggaacagtttcactatttatcttgatgctactgatttccgttttgcttaactggctgtcgctggtagcggcaaacaacaatggctccagcagtttgcttaaaccactgcgctggatcagcaccatataatgtgaaagatggccttgtttatcgtgccacagcgctgcctgcgcgggctgatctaagagtgacgaaaagagcttatctttcagcgtgagatcgtgttcatagacaatacgacgaatgctgccttcaatgcccagacgatcggcatgattctgataatagaaaacgaaatcttcgctcagaacatcgtggagaaacggaatggtgaggagatctttgggaagctggctcagagagtcgctgtcgagaaagaggtccggctcattgagatcgatttgcagattgttgtgcaccaccagcggcgacaacgttttttctggcccactgccagcatattgcaacgcccagacgccagcggaaagcagtgctattgcgccaaaacctacaagaccatagaaccgccagcctttcgcctttttttcaccactcattgccacattccttgtgtatagccagccattttttacgggcacagccaaactttaccgtgccctaatacgacaaaagcccagactttgcagcctggacttttcaattcaaacaagggagatagctcccttttggcatgaagaagtaaaattattcttcttctggctcgtcgtcaacgtccacttccggagcgatttcatcgtccccttccgcggcactgccgtcgatggtatccagatcttcctcgtcaaccggttcagcaacacgttgcagacccactacgttttcatcttccgcagtacggatgaggatcacgccctgggtgttacggcccacgatgctgatttccgaaacgcgagtacgtaccagcgtaccggcatcggtgatcatcatgatctggtcgcagtcatctacctgtaccgcgccaacaactaaaccgttacgttcggtaaccttgatggagataacccctttcgtcgcacgcgacttggttgggtattccgccactgcggtacgtttaccgtaaccgttttgcgttgcggtgaggattgcgccatcgccacgaggcacgatcagagagacgactttatcgccttcacctaagcgaataccgcgaacaccggtggtgttgcagcccatcgcacggacagaagactctttaaagcgcaccactttaccttcagcggagaacagcattacttcgtcttcgccgctggtcaggtcaacgccgatcagctcatcgccgtcaaccagtttgatcgccactttaccggcggtacgcagacggttgaactcggtgaggacagttttcttcacggtaccgttagcggtcgccatgaagactttcacgccttcttcaaactcggtcactggcaggatcgcagtgatacgttcgtcctgctccagcggcagcaggttgacgatcggacgaccgcgcgcgccacgagtggcttccggcaactgataaactttcatcgaatagacgcgaccacggctggagaagcacagaatatggtcgtgagtgttcgccaccagcagtcggtcgataaagtcttcttctttaatacgtgcggcagatttacctttcccgccacgacgctgcgcttcgtattcagaaagcggctgatacttaacgtagccctggtgagagagcgtcacgaccacatcttcctgggtgatcagatcttccaggttgatgtctgcgctgttggcggtgatttcagtacgacgtttgtcaccgaactgttcacgaaccagctccagctcttcacggatcacttccatcagacgatcggcgctaccaagaatacgcaacagttccgcgatctgatccagcagctctttgtattcgtcgagcagtttttcgtgctcaagaccggtcagtttctgcaaacgcagatccagaatcgcctgagcttgctgttcggtcaggtagtacagaccatcacgcacgccgaactctggctccagccattccggacgcgcagcatcgtcgccagcacgttcgagcatcgcggcaacgttgcccagctgccacggattagcaaccagcgcagttttcgcttctgcaggcgtcggcgcatgacggatcagttcgatgatcgggtcgatgttcgccagcgccacggctaatgcttcaaggatatgagcacgatcgcgagctttacgcagttcgaaaatagtacgacgggtcaccacttcacggcggtgacgaacaaacgccgcgatgatgtctttcaggttcatgatcttcggctgaccatggtgcaatgccaccatgttgataccgaaagaaacctgcaactgggtctgggagtagaggttgttgagcacaacttcaccgaccgcatcgcgtttcacttcaatcacgatgcgcataccgtctttgtcagactcgtcacgcagcgcgctgatgccttccacgcgtttttcttttaccagttccgcaatcttctcgatcaggcgcgctttgtttacctgatacggaatttcgtggacgataatggtttcacgaccggttttggcgtcaacttccacttctgcgcgagcgcggatatacaccttgccgcgaccggtacggtaagcttcttcaataccgcgacgaccgttaatgattgccgccgtcgggaagtccggccccgggatgtgttccatcagcccttcaatgctgatgtcttcatcatcaatatacgccagacaaccgttgatgacttccgtcaggttgtgcggcgggatgttggttgccatacctacggcgataccggaagaaccgttcaccagcaggttaggaattttggttggcatgacgtccggaattttttccgtgccgtcatagttatcaacgaaatcgaccgtctctttttcgagatcggccatcagttcatgggcaattttcgccagacggatttccgtataacgcattgccgccgcagagtcgccgtcgatagaaccgaagttaccctgaccgtctaccagcatataacgcagcgagaatggctgcgccatgcggacgatcgtgtcatagaccgccgagtcaccatggggatggtatttaccgattacgtcaccaacgacacgggcagattttttataggctttgttccagtcattgcctagtacgttcatggcgtaaagtacgcgacggtgtaccggcttcaggccatctcggacatctggcagcgcacggccaacaatgaccgacatcgcataatccagataggagctcttcagctcttcctcaatgttgaccggtgtaatttctctcgcaaggtcgctcatctaaccgctatccctctactgtatcccggattcaaaggtcgcaaattataacacagccgcgcagtttgaggtaaacctatacgctttattcacatccaatgcctgatatactcgtttgtcttgccaattacggagtagaagtgccaatgaatgccgaaaaatcgccggtaaaccataacgtagaccacgaagagatcgctaaatttgaagccgtcgcctcccgctggtgggatctggaaggtgagttcaaaccgctgcaccgcattaacccgctgcgtctgggctatattgccgagcgtgctggcggtttatttggcaaaaaggtgctcgatgtcggttgtggcggcggcattctggccgagagtatggcgcgcgaaggcgcgacggtgaccggtctggatatgggctttgagccattgcaggtggcaaaactgcacgcactggaaagcggcattcaggtggattacgtgcaggaaaccgtggaagagcacgcggcaaaacatgccgggcagtatgatgtggtgacctgcatggagatgctggagcacgtccccgatccgcagtcagtggtcagagcctgtgcgcaactggtgaaaccaggcggcgatgtctttttctcgacacttaaccgcaacggcaagtcatggctgatggcggtggttggtgcggaatatattttgcgcatggtgcccaaaggcacgcatgatgtgaagaagtttattaaaccggcagaattgctgggctgggtggatcagaccagtttaaaagagcggcatatcactgggctgcattacaacccgatcactaatacttttaaactcggccccggcgtggatgtgaactatatgctgcacacgcagaataagtgaggttgatgtttggccgcgccaatgcctgatgcgacgcttgccgcgtcttatcaggcctacaaatgctccccgtaggccggataaggcgtttacgccgcatccggcaaccgtgccgactagacagtgattaccatttcaccgtcatcgacaaaaaccctgccgtctgggcaaaatcatcactccctttctgccacgccacgctgccgcgcagggacactcgctgactgatattgcccgtgactcccacttttatttcaccccgttgcttcaccgcatcgtcactgatagtgctgccatcctcttcaatttccgtcgaatggggatcgtgataataattcagatctaatgttggtatgacatgaacagcggtacgccattcgctgtgtaaacccagccgcgtctgaatatcatcaccctgcgattgtgacacgcgcgcacggttagcggcggtaaaatcatcctgctgcacgccctgataaatcacctgcgcctgcggttcaatcaccacaccacgccccggtaaccactgataccccgcctccagcgaggcgataatccccgacgagtggtaatgatctgtgccatcttcttgttcggaaacatcattgctaaaccacgcgtattgcagccagctatccagccaggccccttgcttctgattaccgtgctgaaaccagcttgatgtcagcccaacggcataaccgtggttctggttatcggcgcgagttccggtcatattcgagcggctgtcgccctggttatcgctgtagccaccaacaatcccaagcatccactcgccatccgtgccccagcgcccgctaaacagatcgccgctaagttgcaccgtagaagtgtcttcatgttgagccagttgccccgctgctgtgtaatgataatctccgccgataacacgtaaattcagcgtctgaccatcgccacctgcgtgatcgcgtcgctccatcataaacgcctgatttgccgcccgcaggttattaagataaccgccaactttggcattcaacaccggctggtaagcaggcgtaggttccgggtcgggtgttggatcaggatccggcgtgggatcaggatcgggagtcgggtctggatcaggtggcgatggcggcgttacttcttgcgatcgcagataccagtcgttgttatcttccaccagcgtgtagtcatacgctcccatattgacgtagccgctgcctgccagactgaactgcgcattgttttgaaactgcgtgggatcagctgcgaaatcaaccactttaatgcctgtcgatgtcggctcaccaatccctgtaatggagttaaccaccacagttgtgttgccagcagtattaccgttcatcaccaattgatcgcttaccgagtcatcgccgtttaattcgctatcgagcagtagcgtaccgccgccggtataatcaccgtttaccgtcagcgtatcgccagcgacgccattttgcaggctaaccgcaccggacgtattggtcagattgccattaaccgtcacgttggaaagataagtcaggctgtcagtttcaaggttggtattaagctcacctgtcaacgtcacaccatcggtggcattcaccagcgtcccatcgccgttaaatagtgaggcattaagggcgacggaagtatcctgcccggtcaggcgcaaaaccgtaccatcgctgatgtcgatagtgccgctggaaatagcatcaattgactgaatatcctgatccgcgccagtaacgaacgttgccccatcaccaacccacagtgacgaagcataaggaaggatatcagcaacatcacctttcagggtgccttcttcgacacgtaccgccgactgcgttgtaccgctggcggtcagctccagtgtaccagcccccgttttagtcaatgtgctaccctcatcctgatgctgcccgctgctgtcagccatcagtgcgccccactgcgtgtctacccccgcatcaactgccacttcaccgtcggcgcgcatttcaatatcacgtccgtggcctgccgcatctgaacgcgtgtcaacgtcggaggtaatctccatcacgctttcttgttgcttatcggtaaagataacctggcggttatagtgggtatctccaagctgcgagttgtcgctcaccatcagcgtaccggaggcgatttgtgttgtgcccaaataactattattgtttgccagacttacctgcccgtcgctcgcatcgaccaccacgtagacgccatctttcccgtcgccgccgatatgcaaattgtcgccacctgcaagatctaccacatcctgactgccgataaccgttccgctgctgccactgacttcaaggccatcgttgtatgatgtgccgctctgccaggtggagaaatcagagagatcgagcacaccgccgtttaacacgatcgactgcggatcgtcctggagagcggtaagatctgccgcgtcgccttccagcgaaagcaccgcaccatcatcaacgactatatcgccggttagcgccatcgactgcgcccctgccagcacgtagctgccgttttgcgcaatggtgagctgaccagcaccttcgatgatgccagcaaaactgccctgattaacagtaacgttgccaccagcatcgatatttaaagtgccattctgaaagcccgtcaatgcgtgcacaaaagtttgttgggtcgagccaacgtttagctcagcctgattctgatactgatcaatactccctatcgtcagaccgtagcagtcttgcggatcgtcctggcaatgcgtatcgccgacattcatcagggagttgctgcggcccagggtaacttcaccgttttcaatctgcatctcaccagtaaagtcattgttatctgcattaagtaccagatcgccggaacctgttttggtgattaacccggtaccagcaatagagtcaacagctccgtcattctctgtattgccaataaccagcgtttttccgtcggcaatatcaaaggtaacttcacttaagccgagatacataaagccacccgccgcagaggaaggaccatctccatagcctgctgcgctattgttctcatcgactaacacgcctccgttctggctgtagctgtcatcaacagaaatatcaataagatagggagccgtcacgctattggtatatatcgccccgccataaccttcggcagtgttatttgtaaaggcagtgttatttactatcgtataacctgaaggatgcttgctgtcgctattattatcggtaacatcgattgccccgccatcgccatcactgtaacttgttgatgtatatgcctggttgttatcaaaaataacatcacttaaataaacgtcattattaatggtataaattgcgccacctttgccatcattagcgatgttattgcgaaacatggcgttagtgacacgtaaatcgacggcaccagtatcgttagtaccagaagaatagattgcgccaccatagccgcctgcgacgttaccggaaaaaataacatcagtaagattcagcgttgagttttctttagcaaatatggccccgccgttattatattctcctgtaacggtgttattggcaaacagagtcattccagtttcattttctggtaatagtgaaaattccgctccttgttgcaaaaatacggccccaccgctggcgttattggtcatatccgaaaaaaccagccattgcccatcagcgatactccagtcctgcgtaatgcctgaaaggctttgcctgctggcctgacaactcgctttgacatcatatccctggcatgaatcagtgaccgccgcgacaccgttagcagagaaaagagatgcaatcattgacgggagtaaagataaatactccttgcgtagaaagataatccgcatattaatctaaccatcattttctataagacggcgtatttaatcgcattatacgatatggaatatctttcttttgtaaattgttcaacccggtgcaatggctattttgttattatttgatgaataatatcagtgcgtcataattcaagttaataaccttcagggatatcagttatatttaaactaaattaaagtcatgaataattttcttataatataaggtaaattaacaaaatggcttagcatttaacaataaccgaatagaaaacaaccatttcgccatcaacaatctcttacattcgcttatatattgaccacaactgatacatcagattatgtgatgactcgtgcttagatcaatttttgcaatcattagcaaaaagattaataagccatctatatcaatttatctaacctattatgccgttcaagaaatcgccgaacagttatttttaacaaatttttctcttcccattgactttcccggacaccttgtctgacctaaggtgcgcgaaagccactttttccttcctgagttatccacaaagttatgcacttgcaagagggtcattttcacactatcttgcagtgaatcccaaacataccccctatatatagtgttctaagcagcttcccgtactacaggtagtctgcatgaaactattgcggaaagaattccaaaaacaggtacgacatacatgaatcagaatctgctggtgacaaagcgcgacggtagcacagagcgcatcaatctcgacaaaatccatcgcgttctggattgggcggcagaaggactgcataacgtttcgatttcccaggtcgagctgcgctcccacattcagttttatgacggtatcaagacctctgacatccacgaaaccattatcaaggctgccgcagacctgatctcccgtgatgcgccggattatcagtatctcgccgcgcgcctggcgatcttccacctgcgtaaaaaagcctacggccagtttgagccgcctgcgctgtacgaccacgtggtgaaaatggtcgagatgggcaaatacgataatcatctgctggaagactacacggaagaagagttcaagcagatggacacctttatcgatcacgaccgtgatatgaccttctcttatgctgccgttaagcagctggaaggcaaatatctggtacagaaccgcgtgaccggcgaaatctatgagagcgcccagttcctttatattctagttgccgcgtgcttgttctcgaactacccgcgtgaaacgcgcctgcaatatgtgaagcgtttttacgacgcggtttccacatttaaaatttcgctgccgacgccaatcatgtccggcgtgcgtaccccgactcgtcagttcagctcctgcgtactgatcgagtgcggtgacagcctggattccatcaacgccacctccagcgcgattgttaaatacgtttcccagcgtgccgggatcggcatcaacgccgggcgtattcgtgcgctgggtagcccgattcgcggtggtgaagcgttccataccggctgcattccgttctacaaacatttccagacagcggtgaaatcctgctctcagggcggtgtgcgcggcggtgcggcaacgctgttctacccgatgtggcatctggaagtggaaagcctgctggtgttgaaaaacaaccgtggtgtggaaggcaaccgcgtgcgtcatatggactacggggtacaaatcaacaaactgatgtatacccgtctgctgaaaggtgaagatatcaccctgttcagcccgtccgacgtaccggggctgtacgacgcgttcttcgccgatcaggaagagtttgaacgtctgtataccaaatatgagaaagacgacagcatccgcaagcagcgtgtgaaagccgttgagctgttctcgctgatgatgcaggaacgtgcgtctaccggtcgtatctatattcagaacgttgaccactgcaatacccatagcccgtttgatccggccatcgcgccagtgcgtcagtctaacctgtgcctggagatagccctgccgaccaaaccgctgaacgacgtcaacgacgagaacggtgaaatcgcgctgtgtacgctgtctgctttcaacctgggcgcaattaataacctggatgaactggaagagctggcaattctggcggttcgtgcacttgacgcgctgctggattatcaggattacccgatcccggccgccaaacgtggagcgatgggtcgtcgtacgctgggtattggtgtgatcaacttcgcttactacctggcgaagcacggtaaacgctactccgacggcagcgccaacaacctgacgcataaaaccttcgaagccattcagtattacctgctgaaagcctctaatgagctggcgaaagagcaaggcgcgtgcccgtggtttaacgaaaccacttacgcgaaagggatcctgccgatcgatacctataagaaagatctggataccatcgctaatgagccgctgcattacgactgggaagctctgcgtgagtcaatcaaaacgcacggtctgcgtaactccacgctttctgctctgatgccgtccgagacttcttcgcagatctctaacgccactaacggtattgaaccgccgcgcggttacgtcagcatcaaagcgtcgaaagacggtattttgcgccaggtggtgccggactacgagcacctgcacgacgcctatgagctgctgtgggaaatgccgggtaacgatggttatctgcaactggtgggtatcatgcagaaatttatcgatcagtcgatctctgccaacaccaactacgatccgtcacgcttcccgtcaggaaaagtgccgatgcagcagttgctgaaagacctgctcaccgcctacaaattcggggtcaaaacactgtattatcagaacacccgtgacggcgctgaagacgcacaagacgatctggtgccgtcaatccaggacgatggctgcgaaagcggcgcatgtaagatctgatattgagatgccggatgcggcgtaaacgccttatccggcctacggctcggtttgtaggcctgataagacgcgccagcgtcgcatcaggctccgggtgccggatgcagcgtgaacgccttatccggcctacggctcggatttgtaggcctgataagacgcgccagcgtcgcatcaggcacaggatgcggcgtaaaatgccttatccggcattaaactcccaacaggacacactcatggcatataccaccttttcacagacgaaaaatgatcagctcaaagaaccgatgttctttggtcagccggtcaacgtggctcgctacgatcagcaaaaatatgacatcttcgaaaagctgatcgaaaagcagctctctttcttctggcgtccggaagaagttgacgtctcccgcgaccgtatagattaccaggcgctgccggagcacgaaaaacacatctttatcagcaacctgaaatatcagacgctgctggattccattcagggtcgtagcccgaacgtggcgctattgccgcttatttctattccggaactggaaacctgggtcgaaacctgggcgttctcagaaacgattcattcccgttcctatactcatatcattcgtaatatcgttaacgatccgtctgttgtgtttgacgatatcgtcaccaacgagcagatccagaaacgtgcggaagggatctccagctattacgatgagctgatcgaaatgaccagctactggcatctgctgggcgaaggtacccacaccgttaacggtaaaactgtgaccgttagcctgcgcgagctgaagaaaaaactgtatctctgcctgatgagcgttaacgcgctggaagcgattcgtttctacgtcagctttgcttgttccttcgcatttgcagaacgcgaattgatggaaggcaacgccaaaattattcgcctgattgcccgcgacgaagccctgcacctgaccggcacccagcatatgctgaatctgctgcgcagcggcgcggacgatcctgagatggcggaaattgccgaagagtgtaagcaggagtgctatgacctgtttgttcaggcagctcaacaggagaaagactgggcggattatctgttccgcgacggttcgatgattggtctgaataaagacattctctgccagtacgttgaatacatcaccaatatccgtatgcaggcagtcggtttggatctgccgttccagacgcgctccaacccgatcccgtggatcaacacttggctggtgtctgataacgtgcaggttgctccgcaggaagtggaagtcagttcttatctggtcgggcagattgactcggaagtggacaccgacgatttgagtaacttccagctctgatggcccgcgttaccctgcgcatcactggcacacaactgctgtgccaggatgaacacccttcccttctggcggcgctggaatcccacaatgtggcggttgagtaccagtgtcgcgaaggttactgcggctcctgtcgcacacgcctggttgcaggtcaagttgactggattgccgaaccgttagcctttattcagccgggggaaattttgccctgttgttgccgggcaaaaggcgatattgaaatcgagatgtgaattggttgtagtgccagatacaacgcttatgcgtcttatctggcctacaacgattacatggcgtagtaatacgctttcacctgctcccagtccgctttggggattggctccagatatttttccagctggcggaagtcatgattaatcgctttatcgcgacgcaagcggcgacgacttttctccaggtcaagaaaaccagcttctgcattaccttctgttttcacatagatatggcgaacataacaacagccatgctgacgattaatgctatgcattttcttaaacgccagcgccactgctttcaacatggcttgccgtacttcgtcagaataaggcgatactgcatgctgggcataccagtcagcaatgctgatgaaccccgccatatcttcagtcaccagcaacgctcgccattcaccctcaattttcaccgcttcaccaaaaacgatcttcggcacgatgacaccggcccgttccagttctttaattaccgcaacctcacggacaatcgttggtcggccgaacggataacgtacggaatgaaacagatgatgcgtcatgcgctttacatacagctttttgccgttgcgctcgacgcattgcaccccgctcataccattacggcgatagttaggctcttcaacccagtcgccctctgttgcccaccagtgattaaattcgtcgtactttgctgaaactgccataccctatcgcctgtcatttttattaacgacaatgactataggtggttacctgaggaaaatcttaatgaaacgtgtcgtattaatgaatttcttttgccactactagcttgacaccgcttttacccttcatttgcagcgcatagattccaccagccactaccactaatagtgcgcccagcagataaaatgtgaatttaatcaggcggatacagcgatgaattttattcgacagggattaggcatcgccttacaaccagagttaacgctgaaaagcattgcaggtgaattgtgttccgttcctctcgaaccaactttctatcgacagatttcgttgctggctaaagaaaagccggtagaaggcagtccactgtttttactacaaatgtgcatggaacaattagtggcgattggaaaaatttgatatgagacaggatggcgcatgaacgccatcctgcagtaacattactctttattaagaaattttactgccttatcagggaaatcagtaaacagcccatttacacccgctttgttatacagagcatcatataactgattcacatcaggagtgtattcaggcagtttatctgaccgcacggtataaggatgcactaccagtttattctgctgagcatcttgcaccatgccagtgagtttgatattacccggctgcgatgtctcctcaatcaacatatggtaatccggaccaataccatctgcatattccgccacctgtttcatggcacccggcttaaacatccagtcgtagttgtaattaacccagcttccatccggctgtttctgctgcgtttcattccagtcggtataggcaatcagctgtaccagattgagctccatgcccattttgggttccagctcattcttaatacgcttcagctcatcagcatcaaaacattgcaaataaactttatcgtctttaccggtgtaaccatatttcttcagcacttccagcgtttttgccgcaatatccttcccttcctgatgatggaaccacggcgctttgatttctggataaataccgatatttttcccggtagagtgatttaacccctgaacaaattcaatctcttcttcaaaggtgtgcacccggaagtcggacttacccattgggaaacgccccggataagtctgcacttttttaccgttttcaatatcgaaaccttcggtaaatttcaacgacttaatttcatccagcgtgaaatctatcgcgtagtaacgaccgtctttgcgcgcccgatccgggaaacgatcggcaacatcagtaacacgatcgaggtaatggtcatgcagaacaaccagattgtcgtctttggtcatcaccaaatcctgttccagataatccgctccctgcgcatacgccatcgcttttgctggcagcgtatgctccggcaaatatccactggcaccgcgatgggcgatgactattttttcgttgctgtccgccgccattgcactgcttcccatgactatagtgctcatcatgatcgccatgctaaggtttttcagcgtcaatttcatgccattagcctccgttgcgttcttgcagtaattgttcatggcgacgtttttcgccaatcatcacaacaatcaacaagataaccgccagaatgctgccgccaatcattaccataaagccgccatcccagccgaagaagtccacggtgtagccaacaatcgcgctcgccgccaccgaaccgcccaggtaaccaaacagcccggtaaagcccgctgccgtacctgccgcttttttcggtgccagttccagcgcatgcagaccgatcagcatcacaggaccgtagatcaggaagccgataacaatcatacaaatcatatcgacggttgggttacctgccgggttcatccagtaaacgatagtcgcgatggtcaccagtgtcataaagaaaacgccggttgccccacggttgccacggaagactttatccgacatccagccgcacagcagagtgcccggaatacctgcatattcataaaggaagtaggcccaggaggatttatctagcgcgaaatgcttaacctctttcagataagtcggtgaccagtcgaggatgccgtaacgcagcagataaacgaacacgttggcgatggcgatataccacagcagtttgttcggcagtacgtactgcatgaagatttgcttcgccgtcagctcctgttccgctttttcgttatagtcgtccggataatcatttttgtactcttcgatcggcggcaagccacaggattgcggggtatcgcgcatcatcgcaaaggcgaataatgccaccagaatggcgcagaaagcaggcatatagagcgccgcatgccagtcattgaaccaggccatccccagcaggaacagcagcggcggaataccaccaccgacgttgtgcgcacagttccacactgacacaatgccgccacgttctttctgcgaccaccagtgcaccatagtacgaccacacggcggccaccccatcccctggaaccaaccgcagaggaacaacagtacaaacatcaccgcaatgctcgacgtcgcccatggcacaaagcccataaacaacatcactgccgccgccagaatcaaacctgcgggcaggaaaacgcgcggattcgagcgatccgataccgaacccatgatgaatttcgaaaatccataagcaatcgagatccccgaaagggcaaaacctaaatcaccgcgtgagaatccctgctcaaccagataaggcatagcaagcgcaaagttcttacgaaccaaatagtaagccgcatagccaaagaatatccccaggaaaatttgccagcgcaatcgacgataagtcggatcgatctccgcggcaggtaagcgcgctttgtgtggcgctggtttaaaaatactcaacattgatagcctccgtggcccgtggtcttatttatgattaacagcctgattcagtgagagaacctgccgtttcttgagttgccgcgatgttaagaaaacattcataaattaaatgtgaattgccgcacacattattaaataagatttacaaaatgttcaaaatgacgcatgaaatcacgtttcactttcgaattatgagcgaatatgcgcgaaatcaaacaattcatgtttttactatggctaaatggtaaaaaacgaacttcagagggataacaatgaaaactcgcgactcgcaatcaagtgacgtgattatcattggcggcggcgcaacgggagccgggattgcccgcgactgtgccctgcgcgggctgcgcgtgattttggttgagcgccacgacatcgcaaccggtgccaccgggcgtaaccacggcctgctgcacagcggtgcgcgctatgcggtaaccgatgcggaatcggcccgcgaatgcattagtgaaaaccagatcctgaaacgcattgcacgtcactgcgttgaaccaaccaacggcctgtttatcaccctgccggaagatgacctctccttccaggccacttttattcgcgcctgcgaagaagcagggatcagcgcagaagctatagacccgcagcaagcgcgcattatcgaacctgccgttaacccggcactgattggcgcggtgaaagttccggatggcaccgttgatccatttcgtctgaccgcagcaaacatgctggatgccaaagaacacggtgccgttatccttaccgctcatgaagtcacggggctgattcgtgaaggcgcgacggtgtgcggtgttcgtgtacgtaaccatctcaccggcgaaactcaggcccttcatgcacctgtcgtggttaatgccgctgggatctgggggcaacacattgccgaatatgccgatctgcgcattcgcatgttcccggcgaaaggatcgctgctgatcatggatcaccgcattaaccagcatgtgatcaaccgctgccgtaaaccttccgacgccgatattctggtgcctggcgataccatttcgctgattggtaccacctctttacgtattgattacaacgagattgacgataatcgagtgacggcagaagaggttgatattctgctgcgtgaaggggaaaaactggcccccgtgatggcgaaaacgcgcattttgcgggcctattctggcgtgcgcccgctggttgccagcgatgacgacccgagcggacgtaacgtcagccgtggcatcgtgctgctcgaccatgctgaacgcgatggtctggacggatttatcaccatcaccggtggcaaactgatgacctatcggctgatggctgaatgggctaccgacgcggtatgccgcaaactgggcaacacgcgcccctgtacgactgccgatctggcactgcctggttcacaagaacccgctgaagttaccttgcgtaaagtcatctccctgcctgccccgctgcgcggttctgcggtttatcgtcatggcgatcgcacgcctgcctggctgagcgaaggccgtctgcaccgtagcctggtatgtgagtgcgaagcggtaactgcgggtgaagtgcagtacgcggtagaaaatttaaacgttaatagcctgctggatttacgccgtcgtacccgtgtggggatgggcacctgccagggcgaactctgcgcctgccgcgctgccggactgctgcaacgttttaacgtcacgacgtccgcgcaatctatcgagcaactttccaccttccttaacgaacgctggaaaggcgtgcaacccatcgcctggggagatgcactgcgcgaaagcgaatttacccgctgggtttatcagggattgtgtggtctggagaaggagcagaaagatgcgctttgatactgtcattatgggcggcggcctcgccggattactctgtggcctgcaactgcaaaaacacggcctgcgctgtgccattgtcactcgtggtcaaagcgcactgcatttctcatccggatcgctggatttgctgagccatctgccagatggtcaaccggtgacagacattcacagtggactggaatctttgcgtcagcaggcaccagcccatccttactcccttctcgagccacaacgcgtgctcgatctcgcttgccaggcgcaggcattaatcgctgaaagcggtgcgcaattgcagggcagcgtagaacttgctcaccagcgggttacgccgctcggcactctgcgctctacctggctaagttcgccagaagtccccgtctggccgctgcccgcgaagaaaatatgtgtagtgggaattagcggcctgatggattttcaggcgcaccttgcggcagcttcgttgcgtgaactcggccttgccgttgaaaccgcagaaatagagctgccggaactggatgtgctgcgcaataacgccaccgaatttcgcgcggtgaatatcgcccgtttccttgataatgaagaaaactggccgctgttacttgatgcgcttattcctgtcgccaatacctgcgaaatgatcctgatgcccgcctgcttcggtctggccgatgacaaactgtggcgttggttgaatgaaaaactaccttgttcactgatgcttttgccaacgctgccgccttccgtgctgggcattcgtctgcaaaaccagttacagcgccagtttgtgcgccagggtggcgtgtggatgccgggcgatgaagtgaaaaaagtgacctgtaaaaatggcgtagtgaacgaaatctggacccgcaatcacgccgatattccgctacgtccacgtttcgcggttctcgccagcggcagtttctttagtggcggactggtagcggaacgtaacggcattcgagagccgattctcggccttgatgtgctacaaaccgccacgcggggtgaatggtataagggagatttttttgcgccgcaaccgtggcagcagttcggtgtaaccactgatgagacgctacgcccgtcacaggcagggcaaaccattgaaaacctgtttgccatcggttcggtgctgggcggatttgatcccatcgcccagggatgcggcggcggtgtttgtgccgtcagtgctttacatgccgctcaacagattgcccaacgcgcaggaggccaacaatgaatgacaccagcttcgaaaactgcattaagtgcaccgtctgcaccaccgcctgcccggtgagccgggtgaatcccggttatccagggccaaaacaagccgggccggatggcgagcgtctgcgtttgaaagatggcgcactgtatgacgaggcgctgaaatattgcatcaactgcaaacgttgtgaagtcgcctgcccgtccgatgtgaagattggcgatattatccagcgcgcgcgggcgaaatatgacaccacgcgcccgtcgctgcgtaattttgtgttgagtcataccgacctgatgggtagcgtttccacgccgttcgcaccaatcgtcaacaccgctacctcgctgaaaccggtgcggcagctgcttgatgcggcgttaaaaatcgatcatcgccgcacgctaccgaaatactccttcggcacgttccgtcgctggtatcgcagcgtggcggctcagcaagcacaatataaagaccaggtcgctttctttcacggctgcttcgttaactacaaccatccgcagttaggtaaagatttaattaaagtgctcaacgcaatgggtaccggtgtacaactgctcagcaaagaaaaatgctgcggcgtaccgctaatcgccaacggctttaccgataaagcacgcaaacaggcaattacgaatgtagagtcgatccgcgaagctgtgggagtaaaaggcattccggtgattgccacctcctcaacctgtacatttgccctgcgcgacgaatacccggaagtgctgaatgtcgacaacaaaggcttgcgcgatcatatcgaactggcaacccgctggctgtggcgcaagctggacgaaggcaaaacgttaccgctgaaaccgctgccgctgaaagtggtttatcacactccgtgccatatggaaaaaatgggctggacgctctacaccctggagctgttgcgtaacatcccggggcttgagttaacggtgctggattcccagtgctgcggtattgcgggtacttacggtttcaaaaaagagaactaccccacctcacaagccatcggcgcaccactgttccgccagatagaagaaagcggcgcagatctggtggtcaccgactgcgaaacctgtaaatggcagattgagatgtccacaagtcttcgctgcgaacatccgattacgctactggcccaggcgctggcttaaactcctttctgatgcccggtaagcatgtggttaccgggcatttttgcgtacacgattccgtgcccaatgtatgcgttgcaacgcagtgaaaattcctctgaaaacgtctcgcaaaggctgaaactggcagatgtcaaaggcctgggataaccgtaatgtcgcgtcatcataaatatcaggtgacggacaaccatgaccgaatcaacaacctcctccccgcatgatgcggtatttaaaacctttatgttcacacccgaaaccgcacgggattttctcgaaatacatttaccagaaccactgcgcaagctttgcaacctgcaaaccttacgcctggaacccactagttttattgaaaaaagtttacgcgcttactactcggatgttttgtggtccgtggaaaccagcgacggtgacggctatatctactgcgtgattgaacatcaaagctctgcagaaaagaatatggcttttcggctaatgcgctatgccactgccgccatgcagcgtcaccaggacaaaggctatgacagagtcccgctggtggtgccgttgctgttttatcatggcgaaacctcgccttacccgtactcactcaactggctggatgagtttgacgatccgcaacttgcccggcagttgtacaccgaagcttttctgttggtggatatcaccatcgtacctgacgatgagatcatgcaacatcggcgtatagctctgctggaactgattcaaaagcatattcgcgaccgcgatttaatcggcatggtcgacaggatcaccacgcttttggttagaggcttcactaatgacagccagctacaaacactgtttaattatctgctgcaatgcggcgatacctcccgtttcacccgttttattgaggagattgccgaacgttcaccactacaaaaggagagattaatgactattgctgaacggctacggcaggaagggcatcaaattggctggcaggaaggtatgcatgaacaagccattaaaattgctttgcgcatgctggagcagggctttgaacgtgagattgtgctggcgacaacccaactcactgatgctgatattccgaactgtcattaaaaggagagattaatgactattgctgaacggctgcggcaggaaggacatcaaattggctggcaggaaggtaaattagaaggtttgcatgaacaagccattaaaattgctttgcgcatgctggaacagggctttgatcgtgaccaggtgctcgcggccacccagctaagcgaagccgatctggcagcgaataaccactaattaacacaggcccacagccgatccccatgggcctttgatatcaataactaccttttatgcgtggcccatttttgcctgatttaaacatcgccagtcgttgatccagggcatcgctgtagagcatcgtgtcaacgccaacagcgacaaagttcgctccccacgccaggcattgctgcgccatatcaggagccacagccagaaaaccagccgctttacccgcagcacggatccgccgaatactggtttcaataattcgctgcacttccgggtgcccggcgttatccgggtagcccaacgacgcagaaagatccgcaggtccaataaacacgccatcaatcccttcgacgtcgaggatttcgtccaggttatccagtgccgttttactttccacctgcaccaacagacaaagcgaatcgttaacttgcgccatgtaattctcaatgcgtccccagcgcgcagcccgtgccacactggccccgacaccacgctcaccgtagggaggatagcgcgtggcagacaccacctgacgtgcctgttcggcagtatcgaccatcgggatcagtagagtttgcgcgccaatatccaggacttgtttaatcagcggtttactgccttccaccggacggatcacgggttggctggcatagggcgctaccgcctgtagctgatgataaagatcctgaatggtgtttggcgcgtgctccccgtcaatcagcaaccagtcataaccagaagtggcggcaatttctgccatataggcagtcgttgagcttaaccacagaccaatttgcacttcgcccttgcgtaaacgttctttaaagggattgcttaataatgcgttcatcgtgttccttaacctatttaatgatgtgccacgtcggtctgcgcaacagtgcgatttacacgcagagtgaaaataatcagcgaaccgatgaccgccaccgctgccagcgtcagtaatcccgccgcatcgctggcaaataacgtttctgctttcacgcgcaggatcggggcaataaacccgcccactgcaccaaacaggtttacaaaaccaattcccgcagccagcgccgtaccggaaagcagttgtgtcggcatcgtccagaacactggctgcacggcaataaacccgatagctgcaacacacagcgctacgatcgccattactggagaaagcagcccggacagaccaataccaatgcccgccgccagtaatgtcagcgctgcgacattacgccgttcgccggttttatcggaatagcgcggaataagccaggtcccaaacaaggccgcaacccacggaatggcggtgaccaccgacgctgtaaagcccacttttgttcccagcaatgccgcaacctgggtcggcaggaagaaaattaatccgtaaaccgccacctgaatggtcaggtagataatcgctagttgccagactcggccattacgcagcgcatcgctcagccgagaagtcactttctgttgttcttcacttgccagttgattgataagcaacgttttttcttgtttactcagaaaacgtgcctgctccggtgtgtcatcaagccaaaagaatgtgaataccccagcaccgactgccaacaatccttcaatcacaaacatccagaaccagccgggatgccccataaatccatgcatctccaacagcgcgccggaaagcggtgatcccagtgttaacgccagcggtgcgcccatatagaacagccccataatgctggcgcgattacgctgcggaaaccattgcgaggtgagataaatcataccagggaaaaatccggcctccgcagcacgaagcagagtgcgaactatcagaaatttcgcttcagtatcggcccatgccatggctgccgaaagaaatccccacagcagtgttgtcgtaccaatccaggttctggcccccagtttgcgcatcaaaagattcgccggaacacccagaaacgcatataccacaaagaaaatgcctgctcccagcgcataagcttcattactcaacccggtatcaatctggtaggtctgtttggcaaaaccgatattcgaacggtcgagaaacgccagcacatacagcgccaacataaacggaattaaacgcacacggtttttcttcaccacggcgtcaagcaaagcggtgctcataaaaagctccttagaatatgtgggcgttaccgttgtcacagcaacgcccggagtgattagtggctgtaggggcgtttcaaattgcagtcacgattgagttcgacgccaaaaccgggtttatcaagcactgatttatgaatacgaccattcaccggaaccggctcattgagcagaatcgggtcaaactgcggacgcatcgttgaacaatccgggctggtcatcaggaattcgctgaatggcgtattggtgaaggtgatcaccgcatggtgagagtaaacagacgaaccgtgcggcaccaccagttgccccctggatttggcgattgcggcaatttccaccagcgtggttaaaccaccgcaccagccaacatccggctgcataatgtcgataccggtttctgaaagcgtacgaaaagattgcagtgtgccgtggtgctcaccgctggtgaccatcattccgactggcgcgttgcgtttcagttcgcgataactttcatactgctgtggcggcaggcactcttcgatccatttcaggttatagggcgcgcaagcgtgggccagtttggtcgcatagttcacgtcctgactcatccagcagtcgagcattaaccagaaatcctcaccgcatttttcacgcatatccgcgaccatagcggcatctttgcggatccccgcatcgccatcatgtggcccccagtgcgtcggcattttgccaccgataaagcccatctcttttgccagatccggacgcgcacctgtggcgtagaactgaatctcatcacgaacagcgccgcctaaaagtttataaaccggaagcccgaccactttgccgaacagatcccacagagccagatcgacacaagaaatcgtattcatcaccaggccaccagagccggagtaatacagggtggcactgagcatttgatcgtggatcagtttgatatcactgacacatttaccctcaatgaaacggttaagatgtttttcgacaataaaacagcccatttcaccggctgtcgaaacggcgaatccggtctggccgttttctgcttcgacttcaacaaccaacgtgccaagaacgttaatgccaaatgactggcgtgactgctcgtaatcgcggtatttactcatcggggtggcaatatgatcgtctatccagtgattcgccccctggtcgtgataatcaccgccgccagcgcctttttctgctgtcgcaccgccagtaaaccaggcgcgaacctgtttaatttttggtagggtcatgatgttctccattgttatgaggcttgtaagtcaaagggacttttccatcccaacagacgtgaaatatccctggcgcaggcaatggccttgcccgccagataatcacggtattcttcattgatttgtaagcgggtaccgaccaccgagatcgcagcggtaagctcgttattggcgttaaacaccggcgcagcgacacaacggacatcggcgtaatcttcgccgttgtcatagctccagccctgacggcgaatacgcgccagttcttcgtgaagttgctgtggatgagtaatcgttgtgggtgtcgcctgctcccagaccagcccttcgataatactttgctgtaccgctgcaggttgccaggcaagcaggcatttacctattccggagcgataaagcgaaaggctttttccttcatgggaacgcacgctgatagtggctgatgactccactttcaaaatgtaataagcgctgccgttatcaataatccccaggtgacataacagcccggtggtatccatcagttgcgtcaaacgcggtcgagccagttcccggagatccatcttgcttaacgcatgaccggaaagctccaccagcctggtccacaaacaaaaattttcctggtgatcaaggctaagaaaacgctgacgcctgagttcattaagcagcaaataggccgtgcttttagggattcccaatgtgtcaatgatcgtcgcagcactacaggggccaatgcgggcaatcaaattgagaatatcaatagcccgtgtcagggcgggaactttgcttgattccaacatactggactccagtcttagatactggaatcagtctcgttgctcagggggagtaaaattgtgaagcgcatcaaatcccgctcctcgtccagcagactggagaaattacgcacaaatttgtgaatcagcgcacggattttttcttattgagtacaacaggttggacaaattttgccggagggggaatgtgccggtgcagtaaaccggcacagagtggcggaatcagacagataaggtcatggactcaacaacctcaatccagccatgctcactggcgatatcctggccgtttaaccaacggcgcagcatattcagtgccatcattgcgcacacttcctgacggatagccaggctgtagcgcgtagtgctgaaacgcacacgcagagcgaaagtgccgtctggcgtggctagcgcaaagttgagatgctcgttctcgaaacccgaaacagccagtgccagcccggcaaaatggttggcccgccgttctgtaatccagtgcgcagtttgcgccagggtttcctcctgtgaaggaaccacttcacacgccagcaatggagcacctgcgcgagaaagttgcaaagccaataaaccaccggtgaattgctcgctcaacgtcaggctgaactggcggttttgcaattcgcgactgatctgcgcgggcagtccttcagtgccttcgaaaatcacgctctgtccggcaacacgtttaacatccagccacagtttttccatcgcctgttgctcgcttgccggtccggtgagtttcagttcgatgataggcattgaggagcgatagcccattgttacgcccggcggcagttgtagagtgtccaggctttgtgccagatcgctttccgaacgaccaaaagtagtcaaacgcagacaaaccggcggctgcggtaaagaaaaacgctcgcgcaggcgcggcaggatttcgtgctcgaccatcaccttaaattctgacggtacgccgggagtaaagaacatcaggcaacgattaagctgcacggcaaaaccacaggcggtgcctaccgggttattgataaattcagcactggcaggcagctccgcttgtttacggttgctcggtgccattactcgtccacgttcgtggaaatagcgttccatctctttgagccaggcttcatgcagcaccaggccttcaccttttgctgtcgcagcggcgagtgcgcttaaatcatcgctggtcggtcccagcccgccgttaacgatcagcacatcggcgtgctgactacgttcgcgaagaatggtgactaagtcatcaaggttatcccccaccgtattgcggcgagataatggcaacccctgatgaaagaaaaaatcggccagccaggcagcgttagtgtcaacgatttgcccgtgtaacacttcatccccggtggataacatttccacttttaacatggttatctcctgcttttgttatcgaatcactataacgcaaagggagataaggcgtagtaagaaactgaatggcgcgacagaatgccgcgccggaagggatcagaaactggcgttaaccccaacatacgggccgtcagccacggcgttgtcgcggttaccgtctttacccgacagattcaggtagcgataacccgcctcaatactgactggacgcataatggtgtaacgcgcgccagcattcgcttcttcataactttgaataccgctggagagcgaatccggagagtagtaatactcgccaaacaaacggaagctgttgccaattttccactgcaaaccacctcctaccgctgcggcataaccttcatcgccgtaattcgggttggtgtaaacgccttttccgccaacggtcgccattaacggcccgagaggcagattcaaccccagccccacgccagcgacatcaccgtcgtcgtcgttatgtgtccagttaccgcttaacgccaggcccgtcgtttcagtcccaaaaccgacaccaatattggtgtattctttacccgcctgaccgctgatgctcattgcattgaccgatgcagaaaccaacagcattccggccagacctgctagcgcaatttttttcattatcccctttcccacaagcaattaatcaaaattcccaaagctgcgggattgtactgcctggcacagaggattcaatgagcgaaaaaaaggatctagtcacttattgtaactaaatacttcttaaataattaaatgccgaaaaaataaacacactttatcgatacacacaaaaataataataagtacagttatcatcgcaaaagagattactgtcactttcacatatttgtgagttaccgtattctcatggtttctttttatttataaggaatatccctgtgcgacaacggactattgtatgccctttgattcaaaatgatggtgcttatttgctgtgtaaaatggccgacgatcgcggcgttttccccggtcaatgggcgatttcgggtggcggcgtggagcctggcgaacgaattgaagaggcactacgccgcgaaattcgcgaagaactgggagaacagctgcttttgacagaaatcacgccgtggaccttcagcgatgatattcgcaccaagacgtatgcagatggtcgcaaggaagagatttatatgatttacctgatttttgactgcgtttctgccaaccgagaagtgaaaataaacgaagagtttcaggactacgcgtgggtaaaacctgaagatctggtgcattatgatttgaatgtcgccacccgaaaaacgttacgtttgaaaggtcttctgtaacaatgatgacagccattactggctgtcagattgaaaatttagtggttaacgaattccccatccagataaactttgcctttttccacatgcatgactaaaccatccagataatcaggtttaaatgtcgcgtcacgcttatctttagcaatatatgtcaggcaatgattatgggtgaaaataacgatatttttatcaggcgctttgctttgtaagtccttaattgcactataaatctcattaccgcactgaagaagtcgtttatctaccgtcaattttttacccgctgaaaaccaggtagccgactgaatggtccggacggtattactggaataaagatcgaaatcagggatatcagcactaaaagcgttgcccagttcacgggcatcctgggtacctttaaccgtaatacctgttttatctgacaagcattgattggttgaacggtcgcaacgttcagcatgacgaaacaaaacgacaaccgggtgctgctgtgccagtctggccagtgttttattgtcgatacgtggcaaaccattgctactccaggcggcatgagtacccagtccggcaattgcagcgagcgccagtaaaatgatgatatatttttttgacttcaacgaagagcggcaaaaagctaacacgtaaactccacctatagacaagcgcaaccagacaattaccgtgaaattgagctacatttctggcgataattcgcagttggtgtaatattaaaaatcctacgatgtcggcaaaatgcctcaaaattttgccaaatgcaaagcctaaataagaaaaaatataaaaatttcaatatttacgtctaatattagtttcttaaggttaagttaatattctatccttaaaatttcgctccaaatggcaaaatatacacaacactctttatagcaaatataagtggacaggtattcaatggcggaaggaaaagcaatgtcagaatttttgcctttttcgcgaccagcaatgggcgtggaggaactcgctgcagttaaagaggttctcgaatccggttggatcacaaccggtccgaagaatcaggcgcttgagcaagctttttgccagttgacgggaaatcagcatgccatcgcggtcagttcagccaccgccggaatgcatatcacgctaatggcgttgaaaattggcaagggcgatgaagtgattacgccttccctgacctgggtttcaaccctcaatatgatttccttgttgggtgcaacgccggtaatggtggatgtcgaccgcgatacgctgatggtcacgcctgaagctatcgagtcagccattacgccacgcactaaagccatcattccggtgcattatgccggtgcgccagcagatattgacgccattcgcgccattggcgaacgttacggcatcgcagttatcgaagatgctgcccatgccgtcggtacgtattacaaagggcgacatattggcgcaaaaggtaccgctattttttcatttcatgccattaaaaatattacctgtgctgaaggtggcctgattgtaactgataatgaaaaccttgcccgccagctacggatgctgaaatttcacggtctgggtgtcgatgcctatgacagacaaacctggggccgtgcaccgcaggctgaagtcttaacaccgggctataagtacaatctgaccgatattaacgccgcgattgccctgacacagttagtcaaattagagcacctcaacacccgtcggcgcgaaattgcccagcaatatcagcaagcactggcagctctcccctttcagccattaagccttcccgcctggccgcacgttcacgcctggcatctgtttattattcgtgtcgatgaacaacgttgtggtatcagtcgcgatgcgttgatggaagcgttaaaagaaagaggcattggtaccgggttacatttccgcgccgctcacacacaaaaatattatcgcgagcgttttcccacgctgtcgttaccgaataccgaatggaatagcgaacgcatctgttctttgccgctgttcccggatatgactaccgccgatgccgaccatgtcatcacagcccttcagcaactcgcaggacaataagccatgtttgaaatccaccctgttaagaaagtctcggtggttattcccgtttataacgagcaggaaagcttaccggaattaatcaggcgcaccaccacagcctgtgaatcgttggggaaagagtatgagatcctgctgattgatgacggcagtagcgataattccgcgcatatgctggtcgaagcctcacaagcggagaacagccatattgtgtctattttgcttaaccgcaattacgggcaacattcagcgattatggcgggattcagtcacgttactggcgacttaattattacccttgatgccgatctccagaatccgccagaagaaatcccccgcctggtggcaaaagccgatgaaggttacgacgtggtagggactgtacgccagaaccgccaggacagctggtttcgtaaaaccgcttcgaagatgattaaccggcttattcagcgcaccactggcaaagcgatgggtgattacggttgtatgctgcgcgcctatcgccgtcatattgtcgatgcgatgttgcactgccatgaacgcagcacctttatcccgattctggcgaatatcttcgcccgccgtgccattgaaattccagtacatcatgccgagcgtgagtttggtgaatccaaatacagttttatgcgcctgattaatttgatgtacgacctggtgacctgccttaccacaacgccgctacgtatgctgagtctgctcggcagcattattgcgattggaggttttagcattgcggtgctgctggtgattttacgcctgaccttcggaccacaatgggcggcagaaggcgtctttatgctatttgccgtgctgtttacttttattggcgctcagtttatcggcatgggattactcggtgaatatatcggcaggatctacaccgatgtccgcgcccgcccccgctattttgttcagcaagttatccgtccatccagcaaggaaaatgaataatgaaaaccgtcgtttttgcctaccacgatatgggatgcctcggtattgaagccctgctggctgccggttacgaaattagcgccatttttacccatactgataatcccggtgaaaaagccttttatggttcggtggctcgtctggcggcggaaagaggcattccggtttatgcgccggataacgttaatcatccgctgtgggtggaacgcattgcccaactgtcgccagatgtgattttctctttttattatcgccatcttatttacgacgaaattttgcagctcgctcccgcaggtgcatttaatctgcatggttcgctgttaccaaaatatcgtggtcgcgcgccgctgaactgggtgctggtcaacggtgaaacggaaactggcgttacattgcaccgaatggtgaaacgtgccgatgccggggccattgtggcgcaactgcgcattgccattgcgccagacgatatcgctattacgctgcatcataaattgtgccatgccgcgcgccagctactggaacagacattacccgccattaaacacggtaatattctggaaatcgcccagcgcgaaaacgaagccacctgttttggtcgcagaacgccggatgacagtttccttgaatggcataaaccggcatccgtactgcacaacatggtacgtgccgttgccgatccgtggccgggtgccttcagctatgttggcaatcagaaattcaccgtctggtcgtcgcgtgttcatcctcatgccagcaaagcacagccggggagcgtgatttctgttgcgccactgctgattgcctgtggcgatggcgcgctggaaatcgtcaccggacaggcgggcgacggcattactatgcagggctcgcaattagcgcagacgctgggcctggtgcaaggttcacgcttgaatagccagcctgcctgcaccgcccgacgccgtacccgggtactcatcctcggggtgaatggctttattggcaaccatctgacagaacgcctgctgcgcgaagatcattatgaagtttacggtctggatattggcagcgatgcgataagccgttttctgaatcatccgcattttcactttgttgaaggcgatatcagtattcattccgaatggattgagtatcatgtcaaaaaatgtgatgtcgtcttgccgctggtggcgatagccacgccgattgaatatacccgcaacccgctgcgcgtatttgaactcgattttgaagagaatctgcgcattatccgctactgcgtgaagtaccgtaagcgaatcatcttcccgtcaacttcagaagtttatgggatgtgtagcgataaatacttcgatgaggaccattctaatttaatcgtcggcccggtgaataaaccacgctggatttattcggtatcaaaacaattacttgatcgggtgatctgggcctatggcgaaaaagagggtttacagttcaccctcttccgcccgtttaactggatgggaccacgactggataaccttaatgcagcgcgaattggcagctcccgcgctattacgcaactcattctcaatctggtagaaggttcaccgattaagctgattgatggcggaaaacaaaaacgctgctttactgatattcgcgatggtatcgaggcgttataccgcattatcgaaaatgcgggaaatcgctgcgacggtgaaattatcaacattggcaatcctgagaacgaagcgagcattgaggaactgggcgagatgctgctggcgagcttcgaaaaacatccgctgcgccatcatttcccaccgtttgcgggctttcgcgttgtcgaaagtagcagctactacggcaaaggatatcaggacgtagagcatcgtaaaccgagcatccgcaatgcccaccgctgcctggactgggagccgaaaattgatatgcaggaaaccatcgacgaaacgctggatttcttcctgcgcaccgttgatcttacggataaaccatcatgaccaaagtaggcttacgcattgatgtcgatacctttcgtggcacccgtgaaggcgtgccgcgtctgctggaaatcttgagtaagcataatattcaggccagcatttttttcagcgtcggcccggacaatatgggccgccatctctggcgactggtgaagccacagtttttgtggaagatgctgcgctcaaacgcggcatcgctttatggctgggatattttactggcaggtacggcctggccaggtaaagagattggtcatgccaatgccgatatcattcgtgaagcggctaaacatcacgaagtcggcctgcacgcctgggatcaccatgcctggcaagcccgtagcggtaactgggatcggcaaacaatgatcgacgatattgcacgcggtcttcgcactctggaagagattatcggtcaaccggtaacctgttctgccgctgcgggctggcgtgccgaccagaaggtgatcgaagcaaaagaagcgttccatttgcgctacaacagcgattgtcgtggggccatgccgttccgtccattgctcgaatcaggaaaccctggcactgcgcaaattccggtgaccttacccacctgggatgaagtgattggtcgggatgtgaaagcagaagattttaacggttggttactcaaccgcatcctgcgagataaaggcacgccggtttataccattcatgcagaagttgaaggctgcgcttatcagcataattttgtggatctcctcaaacgcgcagctcaggaaggcgtgacattttgccctttaagcgaactgttatcagagacgttgccgctcggacaagttgttcgcggaaatattgccggacgtgaaggctggctgggttgccaacaaattgcgggtagtcgctgatgaaatcggtacgttaccttatcggcctcttcgcgtttattgcctgctattacctgttaccgatcagcacgcgtctgctctggcaacccgatgaaacgcgttatgcggaaatcagtcgagaaatgctggcatccggcgactggattgtgccccatctgttagggctacgttatttcgaaaaacccattgccggatactggattaacagcattgggcaatggctatttggcgcgaataactttggtgtgcgggcaggcgttatctttgcgaccctgttaactgccgcgctggtgacctggtttactctgcgcttatggcgcgataaacgtctggctctactcgccacagtaatttatctctcattgtttattgtctatgccatcggcacttatgccgtgctcgatccgtttattgcattctggctggtggcgggaatgtgcagcttctggctggcaatgcaggcacagacgtggaaaggcaaaagcgcaggatttttactgctgggaatcacctgcggcatgggggtgatgaccaaaggttttctcgcccttgccgtgccggtattaagcgtgctgccatgggtagcgacgcaaaaacgctggaaagatctctttatttacggctggctggcggttatcagttgcgtactgacggttctcccttggggactggcgatagcgcagcgggagcctaacttctggcactattttttctgggttgagcatattcaacgctttgcactggatgatgcccaacatagagctccgttctggtactacgtgccggtcatcattgccggtagcctgccgtggctgggattactccccggtgcactgtacacaggctggaaaaaccgcaagcattccgcaaccgtctatttgttgagctggacgataatgccgctgctgtttttctccgtcgctaaaggtaaattgcccacctatattctttcctgctttgcatctctggcaatgctgatggcgcattacgctttgctggcagcaaaaaataatcctctggcgctgcggattaatggctggattaacatcgcttttggcgtcactggcattattgccacatttgtggtctccccgtggggaccaatgaacacgccggtgtggcaaaccttcgagagctataaagtcttttgtgcctggtcgattttttcgctatgggcatttttcggctggtacaccttaacaaacgtcgaaaagacctggccttttgccgcgctttgcccgctggggctggcgttgctggtaggattttcaattcctgacagagttatggaaggaaaacatccgcaattttttgtcgagatgacacaagaatcacttcagccaagccgctatattcttactgatagcgtcggtgttgccgcaggtctggcatggagcctgcaacgcgatgacatcatcatgtatcgccagacaggtgagttgaaatacggccttaattatccggatgcgaaagggagatttgtcagcggtgatgagttcgcaaactggcttaatcaacatcgtcaggaggggattattactctcgtgctttcggttgaccgcgatgaagatatcaacagtctcgccattccgcccgcagatgccatcgatcgtcaggagcgtctggtgctgattcagtatcgtcccaaatgatctggctaacattagtctttgccagcttgcttagcgttgccgggcagttgtgtcagaaacaggcaacctgctttgtggcgataaacaaacggcgcaaacatatcgtgctgtggctgggactggcgctggcttgtcttggtcttgccatggtgctctggctgctggtcttgcagaacgtaccggtaggcattgcttacccgatgttaagtctgaattttgtctgggtgacgctggctgcagtaaaactgtggcacgaaccggtatcgccgcgtcactggtgtggggtggcgttcattattggcggcattgtgatcctcgggagtacggtgtaatgggcctgatgtggggattattcagcgtcattattgcctcagttgcgcaattaagcctgggttttgcggcgagtcatctgccgccgatgacgcacttatgggattttatcgcggctctgttagcttttggcctggatgcccggatactgttactcgggctgctgggttatctgctttccgttttttgttggtataaaacgcttcataaacttgcgctaagcaaagcctatgccttgctcagtatgagttatgtgctggtatggattgcttcaatggtacttcccggctgggaagggactttttcgctgaaagcactactgggagtagcctgtattatgagcgggttgatgctgattttcctgcccacgacaaaacaacgttactgagttttccctgccactttacactgccgttcccactcatcggggctataactgcttgccgagaggactttcaccgtatgcagcttttcacgattaatacaataaagcgcattctgcaaaggcgagagtaaatcccccactttcacggcgaagtcactcttcacttcggcgatcatttttatcgcgccgccagcatcgcagagcataagtacatgtctgttatcttgtttattgcagcacgattttttgaccagccattccattgcattatcctgtttgctaagagttttcacatcaatttacagattaacagataaactctttatcaacggcaatggaatggcagaaatgagaagtgaaacggagggttaattattgctgacgttgcacccactcttttagcgcctgacgtgaaattttaataccgccgtttttcagctccggcggcagagttagccagcgcaccggttgttgaaaacgggccagcttatctttcacccattcactaagatcaacgctctcgtggtcatactccatcaccgccaccggtcgatgaccaaactccttgtcggcaacggggacgataaacacctgcaaaaccgcaggatgtgcagcaattacgcgctcgacttcttccggctgaataccctctccgccactgaagaatagattgtctaaacgtccgacaatggtcagcttgccattatgcatctcaccgcgatcgcgcgtagcgtaccagccttcgtcattaaccagtgaaaccagttgcccgttacgccagtaaccttctgccatactggcagcccgcagccacacttcattattaacgattttcacttcccgacccggcagcggcgaaccaacgtctgccaggccgtcggcttctttcgcacacaccgtggaggcaaactcggtcagaccatagccgcaaaagcaacgaatcccctgctcgcgcgcctgttccgtcaactcgaccgggatagccgcgccgccaagtaacaccgctttcagggaaacggaactacggttaaccagcaaacgccagagttgtgttggcaccagtgaagcgtgagtacagcctgccagcatttgctccaatggctgtttatcacgtaccgtcatccgcgcaccagcgtataaccagcgccacataattccctgaccggagacgtgaaacagcggtaaagagagcaaccaatcatcgtgatcgccaaacggaatcagcgataacacaccttgcgcactggcaagatgggcctgataagtatggacagcggctttcggcaaaccggtagaacccgaggtcaacgtcattgagcacagacgcgtcggctgccacgtagcggcatgtgcgccttcaaccagctgaatgtgcagcgacgttaatgccggaaacgtgttttccccatccggcaccagagcaaattgcagcgtcagattgggcagcaattcttcaagcaacggttgcggcagctgagggttcacgggcaacacccgcgccccgcattgcagtaacgccagccaggcgagcagcgtttgcggcgtattccacgcccgcaacatcacgccgctgccctcaaccaccccctgcaccgcaaatccggaggctaattcatcgacgcgagcacaaagctcgcgccagttgagttgctcgtcattaagacgtaaggcgatggtttctccccgcacttgccgccagtgacgccacggccagtcagagaagatcataacaaccgctccagtgcatcaacttccacgacaggcagcgtgctacccggccagcgacgtacctgctgcgcctgcatcagatccagcgtgtccagccctggaatggtgtccggcgttaaccaggcggcaatccgcgccagttgcgttaagcctaagctcgattcaatggaagaactgatcaccgccgtcagccccagcgcgtgcgccgcctgtacctgctcgcgtactttttccagactgcccgtgagcgtgggtttgataactaccgcgcgcacgccctcttcagccacaaaggcaaaatccggctcgcgcaggctttcatcccaggcaatggcaatgccggtttcacgggcaaacgctcgcgaatcatcgcgggttttgcacggctcttcgagaaacgcgatgcggtcgcgataatccgggttaacgtatttggcaaactgctgacctttcagcggtgtccaggcgcgatttgcgtcaagacgcaaatgcagatccggaattgcctccagcaacagattcaccaccatgccgtcgcgcaccgcttcgtacaatcccactttgaccttcgccactttctcgcctggcatatctgcaagtttgaggatcagatcgtccggatcgccattacacagcggtgccgcacggtagttggctgcttgcggcaacgtatctgtcagttctgccaatgcacagcttacgccaaaggccacggaaggcatctgcggtagctcgcaatcgcctgccagccagttatttacccaggcaagcagcacactttgcgcctcttcccaggtttcctgactgaagcccggcagtggggagatctccccccacccttcgcgctcgccttcacgcaggcaaacatacagcccgtcgcgggtttttaaccgcctgtcgcgcagaaccacccccgcgtccatggggatctgccagcggtatacctgcgcgctacgcattacggattccgtttgaatttgctgaagtcaggctgacgtttctggttgaaggcgttgcgaccttcctgaccttcttccgtcatgtagaacagcatggtggcgttgcccgccagctcctgcagccccgcctgcccgtcacagtcggcgttcagtgcagctttcaggcagcgcagcgccatcgggctgttttgcagcatttcgcggcaccaacggacggtttctttttccagatccgccagcggtaccacggtgttcacaaggcccatatccagcgcctgttttgcgtcgtactgacggcacaggaaccagatttcacgcgcttttttctgcccgacgatgcgagccatgtaggaagcgccccagccgccgtcgaaggaaccgactttcgggccagtctgaccgaagatggcattatctgccgcgatagtcaggtcgcacatcatgtgcagaacgtgaccgccgccgatggagtagccagccaccatcgcgacaaccggtttcggacaggtacggatctgacgctggaagtccagcacattcaggtgatgtacgccggaatcatctttatagccgccgtaatcaccacgcactttctggtcaccaccggagcagaacgctttatcgcctgcaccagtcagaatgatcacgccgatgttgtcgtcataacgcgcatctgccagcgcctggatcatctcttttaccgtcagaggacggaaggcattgcgcacctgcggacgattaatggtgatttttgcgataccgtcggtggatttttcataacgaatgtcctcgaaaccttcggagcagtcgtgccattcaaccggtgcgtaaagcattgcttcatcaggataaatcatattgtgtcctttagtcagaaacgcaagatctgcgccagacttgcgattacgccagcgggattttcccgatgcgcgttatgtccggcgcgaggaatgacatggcagtcggcagccagttccgccgccagggcgcggaatttgctgtcacgttcaccacataaataataaaacgcaaatgtgcgggcgctaaggttagcacgtaaatcaggctggacggcgagagaagtcgcctccagcatggcggcaagcgttgcgccattattgttgctgcgcagcgccaccagctcccggcgttgatcgtcattgagtgaggcaaaaacaggctgttgataccagtcggcaaataccgccgttaacggttctgtgagaaaacgctgcacccattggcgatcggaacgctgacgttccgcacgttgttcagcattttgcagccccggatgcccgccttcgacaataaccccacaaagccccgccagcccctggcaagccgccatcatcgccacccgtccaccaagcgagtaccccaccagccagaagtcaaggatgttgtaactaaccaaggttttacgcagtaagtcggtgacatcatcaaatccatcgacgctaatcgccgccgaaccaccgtgacctgggagatcaacatacaaccgtgagtagtcggcaaacgcctcgcccacttcttgccattcgtggcaatcgccggaaaaaccgtgcaaaaacaccagccagggtaaacctggttttccgtgttttgcctgcgcgtgcaggatcataaatggcttacctgcgccagaagttgctggagcgtttgcgcaccatcggtgtcgttaaccaccatttcaatcaccgtggtggttggcgtgcgccaggcgtcggcaaatgccgtttcaagttcctgccagttttgcggacgatgatatttcagctcgaacatcgcggcggcgtgctcaaaatggacgttttgcggcatcagatagaaacgctcacgctcgctttgcggcgttggcaacagcgagaaaatttgcccgccgttgttgttcaccacaattaataccagcggcgcagaaacctgacgcaataacgccagcgcgttgagatcgtaaagtgcggagagatcgcccacaatcgccagcgtcggtttgccgcttgcccgctgaacgccggcggcggtcgaaagcagcccgtcgataccgctggccccacggttgctgtacaccgggtaacctgccggaagttgcgaaagcgcatcaatcagacgtaccaccaggctgttaccaacaaacaattgcccctgttcaggcagatagtcgcagatgcgatgcgccagttgcgcttcgccaaacgcatcacggcgggcaataaccgcctgcattgcctgttccgccaggcgcgggatttcaacgcaccagggctggcgtttttctgccggatgcagctccagccagtcggcaatattggcaattaagcgacgtccgcgatggtgtgccggatcaagtcgcccttcaatgtcatcaacaatccagtactcttctggttcacagcttgcctgccattgcaggagccgtttccccgtcaggctgcttcccagttgcaccacaatttgcgcctgctgcagctcgctggtcgctttggcattgcctaaccaaagatcggcacacggcagcggctgcccggtttgtgacagcacatcgccaatcagcggccagccaagagtttgcgcccacagggcaacttttttgccctcttccgcactcatgcgcccggcaaccaccacgccgcgcttttgtcgccagaagaaccagtcgcgctgtttttcactttccagacgaggcgcttcacgcagccacggtttgtcgtcctgccaccagtcacccagacgctgttgccagctaagcccggtatcgtccatttcgccatacagcggttcagcaaacgggcagttgatatggactccccccgcatgaagcgtaccgagagcgtggtcgatggtagaaaccagccaacgtgcggggatatcctgggtcgggcgcggcaatgaaatactgtgcgtggggtgagaggcgaacattcccggctggcgaattgcctgattcgcgccgcagtcaattagctccggcgggcgatcggcggttaagagaatcagtttttctccggttaacccggcttcaatcagtgccggatagagatttgccaccgccgtgccggaggtcacaatcaccgccaccggctgcttgctgactttcgccagccccagcgccagatgccccaacccacgctcatcgaaatgggtgtggtgaatgaatgcggaattctccgccgccgctaacgttaacggtgtagaacgcgagcctggggcgatacagatgtgtctgacgccgtgacgcgttaatgcttccagaatgaccgccgcccagcgtcggttaaatgcgcttactgacatgagtttgtccggtatcaatattgcggctaagtataaggagctacaaaaatagattattgatatgaatcggtaatgatgcgactcattactattccatttgtaataaagtacgcagccctgccgctttgttgtcgatttcctgccactcttgctcggggtcggaaccacggacaatgcccgcgccagcatataatcgcacgacattgccgctaatttttgctgagcgcagggaaacgcagaattcgctttgttgtaatgagagatagcccgcagaaccggcgtaccattctcgggtgaacggttcgtgacgggcgataaactgtcgcgccagatcgcgcggtaagccagcaactgctgccgttggctgcaactgatgtaaacagatcacatcatccgctttgttgagtgaagtccagatacagcggcgaagatgctgcactttacgcagacgcagtacctgcggcggtaaaacatccagcgtctgggtatcggcctgtaatcgttgacagatatcttccaccaccagcatgttctcgcgctggtttttatcatccgccatcagccactctcctaactgctgcgcctgcttatcatcaggattatttgctactgttcccgccagcgcttcagtacgcagcgctttgtcacgccgccgccataaccgttccggtgaagagccaagaaaagcattttcgccatcaaaggccatgtaaaaatggtagcaattcagattcagtcgacgactggcagccatcatcgccgccgcgttgaccggacttgcgaaatgcaggtcagttgcccgagcgagcaccactttgtcgagctcaccttcggcgatggttttcgttgccagttcgattaattgcgtccagcccgttttgtccggccagtgttgttctcgcgtggtggttaaatgtaacccaggcaagggcttgatactcaccagtgtggcgataaattcttttgcctgaatcgcatcgtgctgaagggagctttcgctgaatagcgtcagccgcagcgtggctttaccgccacagcgtcgccattccaggcggggtaaaagtaaattgccctgcgacgggtcaaaagcattcagcccccaaatgcgtaagtcggcgtgttccgggtgctggcgaagaaaacgttgtgcctggtccaacgacgtaaaacgggtaatcgcgcccaggacgacagcttcttcatcaccattacgttgttgccagtagaattgcgggtatgtttgctgactggccagccagctcaaggcatcaaaagcgtctttgagagggaaaggaatatcgataacccgaatgccgggtgtcgccggaatctcttgcgacaaatggcgcagtagattttccagcgccgtagtaagtgattgcacgcggacctctccctgttaaaagcctcacattatacggggtactacaaaaaaaatgcagtaccccggtgtagggaggttttaacggcgtgccagcaacagtcctagtaccagcccaacggccgcgcccacaccaattccttgccagggtttttcgtggacgtagtcatcagcacgataaactgcctgcttcgcccgatagtaataactgtctgaagcctggctaacccgttttttcacatcatccagcgctttttctgcacgcgctttcagctcaacatatttctgatcggcgggatcgccagaggagcggagcacctcttccagtgtttcactaagcagcgtcaggtcgtcatcgatacgtgtatcaccaaactgattagacattctcgttctccatttgcgtaaaacctgtcactaactatagacaagggttgttgattacgcctgaattacctcgcgtgccatcccaatgtgtgggataccatcttcttcatagacctccgtcacagggataaaaccgaaactctggtagaagttttgcagatgcgcctgcgccccgaggtaaacaggcttatcaggccagtgatgcgtacatgtttcgagtgttttactcatcagctgctgccccactttttcgccacgcaacgcttcactgacaatcacccgacctataacgaccggctcaagatcatcatcacttttcagaatcctcgcatacgccaccagttcatcatttttccaaccgagaatatggcgattatcccccgtcaaatcatcaccatcgatatcctgataagggcaattctgctcgacaacaaacaccgcgcaacgcagttgtaataaggcataaagctgggaaaccgataattcagagtgatgcagatcttgccattcaatcataatgctctccttttagatgtatgccttatactagccggaatattttttgaaacgtgatgaactcatggaattaatttttttaggtacttcagccggtgtgccaacccgcacgcgcaatgtcacggcaatattgcttaacctgcaacatccgacccagagcggactttggttgtttgactgcggtgaaggcacccagcatcagctactgcataccgcctttaaccctggaaaactggacaagatttttatcagtcaccttcatggcgatcatctttttggtttacccggcttgctgtgcagtcgttctatgtcaggcattatccaacccttaacgatttatggtccgcaaggtatccgtgaatttgtggaaaccgcgctgcggattagcggctcatggaccgattatccgctggaaattgtcgaaattggcgctggcgaaattctcgatgatggcctgcgcaaagtaaccgcttatccgctggaacacccactggaatgttatggctatcgtattgaagaacatgataaaccgggtgcattaaatgcccaggcattaaaagctgctggcgtgccgcctggcccactgtttcaggaattaaaagcgggcaaaacaatcacgctggaagatggaaggcagattaacggcgcagattacttagctgctccagtgccaggtaaagcgctcgctattttcggcgataccggcccctgcgatgccgcacttgacctggctaaaggtgtcgatgtcatggtgcacgaagcgacgctggatataaccatggaagccaaagccaatagtcgcggccatagctctacacgccaggctgcgacactagcccgtgaggctggagtcggcaagctaatcattacccacgtcagctcgcgctatgatgacaaaggttgtcagcacctgttacgtgaatgcaggtcaattttcccggcgactgaactggcgaatgatttcaccgtgtttaacgtttaactctgcttattattaaaaacagggcgaaacttgccctgttatcgcaacccgcgctacatatatccacccacacaggcatattgagcgatttttgatatttattcatctccttacgcactatattcagagcaataagttgcctcttttcatcttgattcagcacaacctttgcaactaaaaggagcccatgatggttacagttgtcagcaattattgtcaattatctcaaacgcaactcagtcagacatttgcagaaaaatttactgtgaccgaggaattactgcagtctttaaaaaaaacagcgttatccggagatgaagaaagcattgagttactgcataatattgcgttaggttatgataaatttgggaaagaagctgaagatattctttaccatattgttagaaccccaacaaatgagaccctatcgattatccgacttatcaaaaatgcttgtttaaaattatataatctggcacatatcgcaaccaactcccccctcaaatcacatgattcagatgatctcctgttcaaaaaactattctccccttcgaaattaatgacaattatcggtgatgaaattcctcttatatctgaaaaacagtcgctttcaaaggtgcttttaaatgatgagaataatgaactgagtgatggtacaaacttctgggataaaaatcgtcaattaaccacagatgaaatagcttgctatcttcagaagatcgccgctaatgcaaaaaatactcaagtcaattatcctactggtctctacgtcccctactccaccagaactcacctggaagacgctctcaatgaaaatattaagagcgatccatcatggccgaatgaagtccagttattccccataaatactggcggacactggatattagtttcgctacagaaaatagtaaataaaaaaaataataaactacaaataaaatgcgtcatattcaactcattgcgtgcactaggctatgataaagaaaattcacttaagcgtgtcattaatagttttaattctgaactcatgggagaaatgtcgaataataatataaaagttcatttaaatgaaccagagataatatttttacatgccgatcttcagcaatacttaagccaaagttgcggtgcatttgtgtgcatggcagcccaggaagtgattgaacaaagggaaagcaattctgacagcgccccctatacgttattaaaaaaccatgctgacagatttaaaaaatattcagcagaagagcagtacgaaattgattttcaacatcgactggcaaacagaaattgttatttagataaatatggcgatgcaaatatcaatcattattatagaaacttagaaataaaacactcacaacccaaaaatagagcatccggcaaaagagtgagttaacatcattgttaattaattcgaccagtcagcaaatatgctgactggtcgaacatagtttgctaaacagtcatcactgactgatgtcagtcacaccatccgccagttcaatcaggcgaataaattccgccctgtaaccctgtggatcttccccttttgcctgctgagcccactgtttgatctgctgccaggaggtattgttcaggtattcagaaccgcgtaacttttgcccatatgcagctactgctgcgcgaaaacgcatatcttcagagggcgcgtttattgttggccccagcgggaattcaactaactgactttcttttccctgcgggtatttccagcgaatttttaaccaggccagttctttcgttttgtccgatttcgctaatttgttatccggggcatagcgtaacttatcaattgatgctttttgcccgttcagcgttaattcgaataacaacgttatatgtttgcctgcgcctatatcccctgcatcaacgttgtcgttattaaaatgttccacccgaagttggcgcttttcataaccaatctgacggtattccgttacccacgcggggttaaactcaatttgcgctttgacatcttttgctacggtaatcaacatctgccgcatttcactattcaatactttctgcgcttcagagagggtatcaatgtagctgtagttgccgttaccaacatcggcaattcgcaccatcattgcctcgttgtaattgctattccccacgccaaacgtcgacagagtaacaccagactcccgctgttttttgaccattgattcaatcgattttggatcgtcaatgccaacgttaaagtcaccgtcagtggctaataaaatgcgattgatgccgcccttaataaaccccttcgtcgcctgctgataagccagttccagcccggcaccgccattggtactgccttcggcatccagcgaatcaattgcggcattaatttccgccttatgactcccggagatagaaggcaatgcaatacgggagtcgccagcgtaggtcacgatggcaatgttatcctgctcacgaagttctttgaccaataatttcaacgaagactggataagtggcaaacgttcatcagaaatcattgaaccagaagtgtcgataagaaagaccagattagaagctggtaactcttcacttttgcgatctttcgccaggatatcaactttcagcaatgttcgctgttcattccatggtgcaggtgccaattcgtagcgcatagcgaaaggtattggcttagaggccggaatagattgtttgtctttgatatcccaatcagacgggaaataattgactatctcctccacccgcacagcgtctggcggaggtaacagcccttgattgaggaaacgccttacattcgcataactgccagtgtcaacgtcaagactaaacgtcgccaacggattttgcgctacctgcttaaccggattatcatcgaactgctggtagcgagcggttcctggatttgcgatatgtgtagcttttgctttagccgctcttgcaaatgttggcgcttcctgcaatcgcccctgtaaagcctgtttgtctgaatattgttgcacttcttgctgggccaaggctttcgcggcggcggcgctttgctcagcctcttttattgcagcttgctgcgcggcaagcacttgctgctctgtgggagtactgggttgttgttgctgactttccttattctcaggttgcggcccacatcctgacaaaatcaaactactcataagcaacatgattatatttttatttcgcatataaaatccttttaaataaactcaggcaccagacataaaatatactctttgtataatcctgctaatcttaataaaatacaatatcgaaacccatagcaaataatgattcaacaacgcaacccattaataatttgcatatgaaaaaaataatctttgcttttattatattatttgtgtttttactccctatgattattttttaccaaccctgggtcaatgcattaccgtcaacgccccgacacgcaagtcctgagcaattagaaaaaacagttcgttatcttacacaaactgtgcatccacgtagtgccgacaatattgataatctgaataggtccgcagaatatataaaagaggtctttgtcagtagcggtgccagagttacctcgcaggacgtccccattacgggtggcccctacaaaaacattgttgctgattatggtcctgccgatggaccgctgattattattggtgcgcattatgactctgccagcagttatgaaaacgatcaattgacctatacgccgggcgcggatgataacgccagcggtgtggcaggattactcgaactggcacgtttgttacatcagcaagtaccgaaaacaggcgtgcagctggtcgcctatgcgtcggaagaaccgcccttctttcgtagcgatgaaatggggagcgcggtgcatgcagcttcgcttgagcgtccagtgaaattaatgatagcactggagatgattggctattacgactctgcgcctggaagccagaattacccttacccggcaatgtcctggctttatcccgatcggggagactttattgccgtggtcggcagaatacaggatatcaacgccgttcgtcaggtaaaagcggcattgttgtcatctcaggatttatctgtttattctatgaataccccagggtttattcccggtattgatttctctgaccacctgaattattggcaacacgatattcccgccataatgattactgacaccgctttttatcgtaataaacaataccacttgcccggtgataccgcagacagattgaattatcagaaaatggctcaggtagtggatggtgttataactttgttatacaacagtaaataataaaaatttctcgaggcgggtccagaaaaagcgacatgcacattttattttccctcatctgttttaagatgcgaaacatgaaattcaacggaggaaaaataaatgggaatgattggctattttgcagaaattgactcagaaaagattaaccaactgcttgagtctactgaaaaacctttgatggataatatacatgacacgctttcaggattacgccgactggatattgataaacgctgggattttttacactttgggctgacaggcacctctgcttttgatcccgcgaagaatgatccgctgagtcgtgccgtgcttggtgaacacagcctcgaagatggcatagatggcttccttggattgacctggaatcaggagttagccgcgacaatcgaccgactggaatcactggatcgaaatgaactgcgtaaacagttttccattaagcgactcaatgaaatggagatttatccgggagtgaccttttcagaagagttagaggggcaactctttgcctcgatcatgcttgatatggaaaagctgattagcgcgtatcgacgtatgctgcgacaagggaatcatgcgctgacggttattgttgggtgatatagcttgatgcctgggggagaaagacccattagttaagatttacgccaggatcatcttgaaaaaatctttaaccatggtccggtttttatccccttgtataaatattactaaatgcttgcttagtcgcattgttaaatgcaataccgtatattcggtatgtaacagcgatatcctctgtgctggcaacgatctgtcatgcttgatgaaaacggaattgaacctgtcattaccaggtagataaaaagcctgttcaattttgggattattttttataactcgtgtctgttatggcgacacgggaaaacatcaatattgtccttcacaaattgcagtaatatagaatcaacctctcttgcaagttggtcacaatgtattataagcattttgaatatgtcatcctctgtaatctcgtgaaaattttcggccttgtcttttagctcatcatatcggattcttgcagtaaccattttttgggcgagttctaataaccccaaagcttgcaattgctggtgagtatgatcactttcaaaaaatatcccacactccattccttcccaaccaacatattcatgccattcataaaccagcataaatgtttgtaaaactggcggtaataattggatatctgcaaaaccaaaccaaaacttacgcttgagatcccactcatattcaatcgccaatgctatattgtttaaggcatctccggcatccttatttttacgcaaaatcaattccgtcagtgtatagcgttgttcatcaatacgccgaagagcttctgcaatatcatagtttgtagccaacaaaacattctctgcttcctgatgagtgacgtctgcttttgccgtcaatatattgatttggtcaatatgaaacaacttgatggcttcatcaacatcaccgccagtcctctctaacaaacgtctggcaacctggataccgacaggtacgttcttccgaagtttacgaatttcacttaaccattccatgtcaaacccctttaaatatttatgatattaaatataacaacgtctggataacgacccggcctgactgaatatctcacgttttcctgcttaacattcatgttatgatgctcttgaaactaataatacgtatggaattgtcactatttatctgctaatgaattcaaacaatgtcattcgtttgatgaatatattatttcagggaataattatgacacctttagaacgcattacccaacttgttaatatcaatggtgatgttaataatcctgatactcctcgtccattgttatctcttgaggatttttttattgacaataatatccatggttcaatatgttgcaatgtgattccagaacaatctccgcaagctatctatcaccattttctgaaaatacgtgagcgtaacaatgttagtgatgttttggtagaaattacgatgttcgatgacccagactggccctttagtgaaagtattttagttatcaccactgcttcaccagaagaagttcagagctggtttgtagaagaaattgcccctgatgagtgctgggaaggatggtcagaagatacggagcatggatgggttgaagtccctgtgggtatgcatccggttacttgttggtgggattaaaacatttatataaacagataagcggatgtttacataaatttttatgtgaaggaacatgatgaaacttattcctcgcagtagtgatatttcacctggcattgatggaatttgcccggggccttttcctccgaacggatttaccgtacttacagatgcagcatatggtaacggagactgtttcggtttgtactggcctattggtcaggagcataaactacctatagtgtgcgaaacgtaccatgacgaatggcgaatcgtacctgccttttccagcattaagaagttcgaagaatggctggaagtgaatgatgatgatccccatgaaaatggcatcagcatcgaagatcaagactttgcagcaaatctcttccgtgttgctcggaaatgtctttcaacgggaaggcttgatgacgcactgccactgttacagcgagcaacagaacaattgcctgaagtcagcgaatattggttagcactggcaatccagtatcgccgatgtaaaaaaacagaagctgcagcacaggctgcgcttaatgcttatcttggcaattgggcatttggtgttcctgacaataaagtcattcatttgctgtcacaggccgcagatgtcccgaatttccaggatgatcctgtgattcagtgcattaaagaacaaggattagatcttagctttggaggaacaaaggaaaataataattaccccttgatgcagatgtgtgttgatacttattttgcgcagagaaaaccgcttcaggcattaaccctgttacataattatgcctggataatgtccagtgaaacgactgcatttcaggaacgctatgattttaatatcgatgaatggcgggcaaaattcaggcagttatgtttagagtattttggcgatagtcgtacacagttcacttaacgctctgcgtctatctactatcccttctttttcagaaaaaccgccgagcatgtcggcggctttctgacttacaaagtaacagattacatcagcggcattgccaaacgcacaatgctaatcagcggttgtggccatacacccagcaccagtaccaacagtgcagagatcagcacaacgataccgcccgcgctgtactgccagtttgatggtgcatcgcgacccggttgttccggggcgtgaagatacaggctcaccgccacgcgcaggtagtagtagaggccgattgccgaaccgacaaccacggcacccaccagccaccacaagtgtgcctggacaccgaccgccagcacgtagaacttaccgataaagcccagcgtcatcgggataccggccagagacagcatcatcaccgtcatcactgccgcgaggatcggacgatgccagaacagaccgcggtaagagaacagggaatcagcatccgggccacgatacgggctggacatcaggctgaccacgccgaacgcgccgaggctgctgaacagataaccggccaggtaaacccctaccgcttccatcgacatctcgccggtttgcagcgcaatcagcgctaccagcagatagccgaggtgagagatagatgagtaaccgagcagacgtttgatattggtctggctcagcgccatcaggttaccgaagatgatggaggcaaaggcgataatcgccagcaccacgcgaatcgcttcgctgtcacccaccggtgcgtagaggaacagacgcatcaccacaccgaagatagcgattttgctcgccgtcgccaggaaagtggaaaccggcgcaggcgcgccctggtatacgtctggcgtccacaggtggaacggcaccagagagagtttgaagccgaggccaacaatcatcaggccgaaacctgccagcaacagcggctcgttgagcataccgtcgccaaggtttttacccaacgcgacaaacgacaggtcgccagactgcgcatacaccagcgccataccaaacagcaggaaagaagacgctgcggcagaaaggatggtgtatttgatactggcttccagtgaacgtttctggcggaaagcgtaaccgaccaggccaaacagcggcaaagagatcagttcgataccgaggaacagagacgccagatggttggcattcgccagcaggatcccgcccagcgcggcaattaacaccaacaggtagaactcatccttgttgtcgttatagccttcaagccacgggtaggcgaaagtacaggtggcgaggctcgccaacaataccagcccggtgtaaagcatggcgaaaccatcaacgcgcatcagcggcgtaacgtccatagcgcccgcctggccaacaaaccagagcgaaaccagcgccgcgttaagcccaataaccgagagcgtagcgttgaggaaatgattgcgtcgccacgcaatggagagcatcacaaccaccaccgtcaagccgacgatcagcaacggtagcagtgcgatcaggttttgtggagttattgtcatggcgatttacggccttgtagtagtaacggaattaacaaaccactgctggatattgccaatcgcggagtgcgaggtatccagaatcggctgcggatagaagcccagcagtaccagcagcaccaccagcaacaggatcataaacagctcacgcagcgacatccctggcagttcctggctggcaatctggcttttcgctttaccgaagtaagcgcgatgtaacatcgccagcgaataaacagatgcaaagaccagcccaaaggtagagataacggtaatcaccggtacaacctggaagctgccgaacagaatcataaattcgccgacgaagttaccggtgccaggcatcccaagcgttgccaccgcaaagaacagcgacagtgctggcagccatttcatcttgctccacagaccgcccatcatgcgcatgtcgcgggtatggatacgttcataaagctgaccacaaagaataaacagacccgccgccgacaaaccgtgcgcaatcatctggattaccgcgccctggtaggccaactggctgccggtgtagatagcaatcagcacgaagcccatgtgggaaaccgaggtgtaggcgatcagacgtttgatatcggtctgggcgaaggccatccacgcaccgtagaagatgccgataacacccagccacatagcaattggcgcgaactctgccgacgcgttcgggaacagcggcagggagaaacgcagcaaaccgtaagcggcagttttcagcaagatccccgcgaggtcaacggaaccggcggtcggagcctgggagtgcgcatccggcagccagccatgcagcggaaccaccggcattttgactgcgaaggcgatgaagaagcccagcattaacaggtattccacaccactggacattggcgtattcagcagctcttcatagttgaaggtccagacgccggtcgcattgtagtgaacaaaaaccagcgccaggatggcaatcaacatcaccaggccactcgcctgggtgtaaatgaagaacttggttgccgccgtgatacgcgttttaccgtcagaggctttatgcccccacagtgcgatcaggaagtacatcggcaccagcatcatttcccagaagaagaagaacaggaacatgtcgatggcaaggaacacgccgataacgccgcccaggatccacatcaggttgaggtggaagaagccctgatatttttcgatctctttccacgaacatagtaccgccagcacaccgagcagaccggtcagcacgaccatcagcagcgacagcccgtcaatggcgagatgaatagagataccaaaacgcgggatccacggcatgtcgaattcagactgccactgcggaattccggcggattgcgtcagtgaataaccgccctgcaaccacagttgcagcgacagcgccagcgtcaatcccatggtgatcagcgcgatccagcgtggcaccttgacgccaaagcgttcggtctgccagcacaggaagccgccaataaagggaattaatattagccagggtagtaacatggcgatctttattccttgtaaaagtcccgtcaggaccggattttcaacgaattctcacgacagaaaattctcttcggactgggggtagtgtcggatgcaccgcgaaggcggcttatccgacctacgttcttatatgcccaggggcaatcccacaatccttaactcaacgcagtaccatcaacagtgccagcaccacgaccgcaccgatgctcatggatgccacataccagcgcagatagccgttctcacttaacagcagacctttacctgcaaagcgggaaaggacagccgggatgttcatcattgagttcagcggatcgcgtttcagcaaccaggcaatacccaggaacggcttgacgaacactttgtcatacagccagtcaaatccccaggcgttgtaccaccaggtgcccagcagacggcccggcgcactgttggcgatggaggtcaccagagtacgtttacccagccacagccaggctgccagcagaatgccgaccaccgcgaccacgccagaggtaatttccagggtcaacatgctgccgtgcgccagttccgtcgtttgcggaagcacgccctgcagcggcggtacaatcagtgcgccaacgaaggtggaaaggatcagcagcacaatcagcggcaggctgtgagttacccctttcacggcgtgagcgtgaatttgttcttttccgtggaagacgatgaaaatcatacggaaggtgtagagcgaggtcataaacgcaccgaccagacctgccaccatcagattgatatgaccattcgccatcgcacccgcgaggatctcatccttactgaagaagcccgcagtgaccagcggtagtgccgacagtgctgcgccgcccaccaggaagcagagataaaccagcggaatagatttacgcagaccgcccatcttgaagatgttctgttcgtgatggcaggccagaatgacggaaccggatgccaggaacagcagcgctttaaagaacgcgtgggtcatcaagtggaaaatcgccgcatcccatgcctgcacgccaagcgcgaggaacatgtagccaatctggctcatggtagagtaagcgagaacacgtttgatgtcggtctgtaccagcgcggcaaaaccggccagcagcagcgtaaccgccccgacaatacccaccagatgcagaacttccggcgtcatcaggaacaggccgtgggtacgggcgatcaggtagacacccgcggttaccatggttgcggcgtggatcagcgcggagacaggcgtcgggcccgccatcgcgtcggcaagccatgtctgcaacggcaactgcgcagatttaccgaccgcaccgcccagcagcatcagcgtcgcccacatcagcatgttattgccgtcagcaaagtgcgctggtgccagttccaccatttcgcggaagttcagggtgcccagttcgttgtaaagaatgaacagtgcgaaagcgaggaacacgtcacccacacgggtcacgacgaacgctttcattgccgctgcgccattcttcggatcggtgtaatagaacccgatcagcagataggagcacaggcccacgccttcccagccgaggtacatcagcagcaggttgtcggcaagcaccagaaccaccatgctggcgatgaacaggttggtgtaagcgaagaagcgagagtagccctcttcaccgcgcatataccaggaggcgtacatgtgaataaggaaacccacaccagtgaccaccgagagcatggtcagcgacaggccgtccagcaccaggttaaaaccgatgttaaagtcgcctaccgacatccacgtccacagcggctggctgtatgtctgctcgccgttagcgaagaaatcaacgccgataaaggcggttaccagcgccgccaggcccacagagcctacgccgacgatcgccgagacgttttcagaccagcgcccacgggagaatgccagcaggacgaagccaatcaatggcaaaataatggttaaggcaagcatgttcatccgcgcatctcacttactgaatcgatgttcaggttctggcgacgacggtgaagttgcagcagcagcgcaaggccgatactcgcttctgccgccgcgaggctgatggcgagaatgtacatcacctgaccgtcggtctggccccagtagcttccggcgaccacgaaggccagcgcggaggcgttaatcatgatttccagaccaatcaacataaacagcagattgcgacggataaccagaccggttaagccaagaacgaataagattgccgcgaggatcagtccatgttgtaaggggatcatgcgtgctcctccgtttttcttttcgcgctgtcgtctttacgattgctcagcacttcacccgcacgctcttcacgaccgacgtggaaggccacaaccagacctgcgagcagcagcatagaagccagttccaccgccagtacgtaaggcccgaacagcgtaatacccactgctttagcactgattggcgtaccgtcgataccctgatcgttaacaccgaggatggcgtaaacaatcaccaccagcatgatggccgacaaaattgccggaccaatccacacctgcggtttcagccactggcgttcctgttcgatttctgaaccgcccaggttgagcatcatcaccacgaacacgaacagcaccataatggcacccgcgtagacgataatttccagcgcaccggcgaagtaagcgcccagtgagaagaacaccccggaaatcgccagcagcgaaataatcaggtacagcagtgcgtgtaccggattggtatgggtgatcactcgcaaggtcgcaagtatggctatcaggccacagatataaaaagcgaactccattgcccctctccttacggtaacaggctcttgacgtcgataggcttggcttcgttctctgcttcgcccttatctttgccgtcgattgccatacctgccatccggtagaagttatattccgggtatttgcccggaccggagatcagcagatcctctttctcgtaaaccagatcctggcgcttgtattcccccatttcgaaatccggggttaactgaatcgccgtggtcggacaggcttcttcgcacagaccacagaaaatgcagcgtgagaagttgatgcggaaaaattccgggtaccagcgaccgtctttggtttctgctttttgcagcgagatacagccgaccgggcaggctaccgcgcagaggttacaggctacgcaacgctcttcgccgtccgggtcgcgggtcagaacgatacgaccacgataacggggcggcagatagaccggctcttccgggtacattcgcgtttcgcgtttggcgaacgcgtgcaggccgatcatccagatactacgaacctgggtgccgaaacctactaacaattcttttaaggtcatggtcttattgccccttattgcgcctgccagagaatgacagccgccgttaccagcaagttgatcagcgtcagcggcaggcagattttccagccgaaggacattacctggtcataacgcggacgcggtaacgacgcacgaatcaaaatgaacatcatcataaagaacgcggttttcagcgcgaaccagatgaatggcggtaacaacgggccttgccagccaccgaagaacagcgtcaccatcaatgcagagatggtcacaatcccgatgtactcacccacgaagaacagaccgaacttcataccggaatattcaatgtggtaaccatccgccagttcctgctcggcttccggctggtcaaacgggtgacggtgacataccgccacgcccgcgatggcaaaggtaataaaaccaaagaattgcgggataacgttccacacatgcgcctggctgttgacgatgtcggtcatgttgaatgaaccggcctgcgccaccacgcccatcaaggaaagcccgaggaacacttcgtagctcagggtctgcgcagaagcacgcatcgcacccagcaacgagtatttgttgttacttgaccagcccgcaaacagcaccgcgtaaaccgccagacctgccatcatcaggaagaacaaaatcccgatgttcaggtcggcaaccacccaacccggactgactggcacaatcgcaaaggccagcagcagcgaggtaaaggcaatcatcggtgccagggtaaagatgacgcgatccgagaatttcgggatccagtcttctttaaagaacattttgatcatgtccgcaaccagctggagcgaaccgccccagccaacacggttaggtccgtaacggttctggaacagacccagcaggcgacgttcgccaaagctcatgaatgccccgcaggtgacaaccaccagcaggatcaccaccgctttgaggatggtcagcaggatctcaatcagttccggtgatatccaactcattgttgtgcctccttgagatcctcaagatgcgcgccagccagcaccggagcaatgccggacatacccatcggcaagcccacctgccctgccgtcagtccttcggcgatttcaaccggcagcgtgaccgtgttgccatcgtaactaaaggagacgcgtgtacctgcgttcacacccaacttcgcggcatccgctgggttgagtttgatgtacggctgcggcatacggctctggaagaccggagcacgctgtgacaattcatcgctgccaaacaggtggtaatacggcgcgatacgccatttcccgtcctgcggctggaagcgtgccggtacgctggtgaagtaatccagaccattttcgctggtttcaaacagacgcacgcccggatcgccaaagcgcagtttgccgcccacttcgtcctggaatttgttccacgcctgcggggagttccagcccggcgcccaggcaaacggcacttgcgaacggtgcgcagtcggctggttgttaccttccatcgagaaggtgaacatggtgtcaatatcctgcggctgacgcggctcatgaacgctgatattggcgcgcatggcggtacgaccgctgtaacggtgcggttcacgggccagtttctgcccacgaatacggaatgtcgcatccggcgcagcatctttgatacctgccagttccgggattttcgccacaacagcgtcaatcacatggtcgagctgcgtccagtccacttcacggctcagcagggtgctgtgcagcgagtgtaaccagcgccagctttccagcatgacagttttgctgtcgtaataagcaggatcgtaaacctggaagaaacgttgggcgcggccttcgttgttgatcaccgtaccgtcgctttcagcaaagctggcagcagaaagtaccagatgggcgttttccataatcgctgtgcgttgatgatcaaccaccatcaccagcggtgctttagccagcgcagcattcacgcggatagcagaagcgtgacgatgcagatcgttttccaacaccaccaccgcgtcggcgcgtccggtttccagttcggttaacgcttcttcaagcgaaccgccacccataatgcccagccccatgctgttgacggaacgggcaatcatggtgataccgacgtcagcgccgcgacctttcagggctttcgcgacgttagccgccgcctgaatcacctctaagctaccggcgttcgtcccggagataatcaacggtttcttcgcacctgccagtgcctgcacgatgacgtcgattttgctttgcagctcaggttcgataccgtcaaccgctggtgcagagttatccagcgcatgggcgatggcaaaacctaaacgcgcctgatcttcaaccggtgcgcggtaagtccacgccgcgatatcatccagacgggtgtcatcaacgttggtaacaaacagcggatgcttcgcacgttgaccgatgttgaggattgccgcaatctgccagtcagccactttctgtgctgccgccatttcgcgcgctttacctttcacagcctgacgcactgccagcgcgacgcgcgcgccggtctgggtaacgtcttcgcccagcaccagtaccgcatcgtaagattcgatttcgcgcagagccggagtataaatgccgccttcacgcagcactttcagcgccagttgcagacgttcctgctcaccgtgagcgataccggtgtagaagttttcttcgcccaccagttcacgcagcgcaaagttgctttccacgctggcacgcggagaaccaataccgatcactttcttcgactgacgcagaatatctgccgcgccctgcattgcctgttcggcgttgagggtaatgaaatcatcgccacgacgctgtactggctgacgcggacgatccttcaggttgacgtaaccgtaaccgaaacgaccacggtcgcagaggaagtagtggtttaccgtaccgttgtaacggttttcgatacgacgcagttcgccgtaacgttcaccggggctgatgttacagccgatggaacattgctggcagatgctcggcgcaaactgcatatcccatttacggttgtaacgctcggagtgcgttttgtcggtaaatacgccggtcgggcaaatttcgaccaggttaccggaaaattcgctttccagcgtgccgtcttccgggcgaccgaagtagacgttgtcgtgcgcaccgtaaacgcccagatctgtaccgtcagcgtaatctttgtagtaacgcacacagcggtagcaggcgatgcagcggttcatttcgtgagagatgaatggccccaaatcctgattacggtgggtacgtttggtgaaacggtagcgacggaagctgtgtccggtcatcacagtcatatcctgaagatggcagttaccgccctcttcacataccggacagtcgtgcgggtggttggtcatcaaccactcgaccacgctttcacggaactgtttcgcttcttcgtcgtcaatggaaataaaggtgccatcggaagccggtgtcatacaggacatcaccaggcgaccacgcgtgtcttccgcgttttggtattgcttcaccgcacactggcggcaagcaccgacacttcccagcgccggatgccagcaaaagtaaggaatatcaaggcccagagacagacaagcttccagcaggttgtccgctccgttgacctcgtattctttgccgtctacatgaattgtagccattagcatgcttccagttttctcagtcagagactgagcgttaatcgaaattcggttaccagcgctctttcagcaggttcggctgaatcccattaatcaaatgggtattgctgaacggctgtttgattcccgcctcaaattcttcgcggaaatatttgatggcgctctgtaacggctccactgcaccaggtgcgtgggcacagaaagttttacccgggcctaagaatcgacacagttgctcaagtgtttcgatatcgcccggctgaccttcaccacgctccagcgcacgcagaattttcacgctccacggcagaccgtcgcggcacggcgtacaccagccgcaggactcacgggcgaaaaactcttccaggttacgcaccagcgacaccatgttgatctcatggtcaaccgccatcgccagcgccgtacccagacggctgcccgctttaccgatactttcgaattccatcggcagatcaaggtgcgcttcggtcaggaagtcagtccccgcgccgcctggctgccaggctttaaatttcagaccatcacgcataccaccggcgtaatcttcgaggatctcgcgtgcggtggtgccgaacggcagttcccacagtcccggatttttcacccgaccggagaagcccatcagcttggtgccagcatctttacttttcgagatgttctgataccactccacgccgttagcgaggatcgccggaacgttacacagggtttcgacgttgttgacacaggtcggtttaccccatgcgccggaggttgccgggaagggtggcttcgagcgtgggttagcacgacgtccttccagggagttgattaacgctgtttcttccccgcagatgtagcgccctgccccggtatggacgaacagttcgaaatcgaaacctgttcccataatgtttttgccaagcagacccgcttcggtggcttcggcaatggcacggcgcagattaactgccgcttcgatatattcgccacgcaggaagatgtagccacggtaagctttcagcgcaaacgcggagatgagcataccttccaccagcaggtgcggcagttgctccatcaacaggcggtctttataggtgcccggctccatttcatcggcattacacagcaggtaacggatgttcatggattcgtctttcggcatcaggctccatttcaggccagtcgagaagcccgcgccgccgcgccctttcagaccagcgtcttttacctgattaacgatttcgtccggagacagcccggtcagcgccttacgcgcgccttcgtaaccgtttttgctgcggtattcgtccagccacactggctgtttgtcatcgcgcagacgccaggtcagcggatgcgtttcgggagtacggataatgtttttcatttataccgctccagcagttcagggatcgcttccggggtcagatgcgcgtgagtgtcctcatcgatcatcatgtttggccctttatcacagttccccaggcagcaagttggcagcagcgtaaagcggccatcaaatgtcgtttgccctggtttgatgttcagctttttctcgagcgccgcctgaataccctgataaccgttgatatgacagaccacgctgtcacaataacggatcacatggcgaccaaccggctggcggaagatctgactgtagaacgttgccacaccttcgacgtcgcttgccggaatacccagcacatcggcgatcgcgtggatcgcaccatccggcacccagccacgctgcttctgaacgattttcagcgcttcaatggacgccgcacgcgggtcttcgtagtggtgcatctcgtgctcgatcgcttcacgctctgccgcactcagctcaaaagcctcggtttgtggttgttgattctcgtgcataattagcggtccacatctgacataacaaaatcgatactgcccagataaacaatcaggtcagacaccaggctgccgcggatcgccgccggaatttgctgcaaatgcgcaaagctcggggtacgaacacgggtgcggtaactcatggtgctgccgtcgctggtcaggtagtaactgttgatccctttggtcgcctcaatcatctggaaagattcattggcaggcatcaccggaccccacgacacttgcaggaagtgggtgatcagggtttcgatatgttgcagcgtgcgctctttcggcggcggcgtggtcagcgggtgatccgctttgaacgggccttccggcatgttgttgaggcactgctcaagaatgcgcagactctggcgcagctcttccactttaagcattacgcgggtgtagcagtcagaaacgccaccacccaccgggatttcaaagtcgaagttttcatagccagaataaggacgcgccttacgcacgtcgaagtcgatcccggtagcacgcaggcccgcgccagtggtgccccactccagcgcctctttcgcgccataggcggcaacgccctgggaacgacctttcagaatggtgttttgcagcgccgctttctcgtaagacgccagacgtttcggcatccagtcgaggaactcacgcagcaggcgatcccagccgcgcggcaggtcgtgcgctacgccgccaatacggaaccacgccgggtgcatacggaaaccagtgattgcttccaccagatcgtaaattttctgacgatcggtaaaggcgaagaacactggcgtcattgcgccgacgtcctgaataaaggtcgagatatacagcaggtgactgttgatgcggaacagttcggagagcataacgcgaatgacgttaacgcgatccggcacggtgatcccggccagtttctctaccgccagcacgtaaggcatttcgttaacgcagccgccgaggtattcgatacggtcagtatacggaatgtagctgtgccaggactggcgttcgcccattttctccgcaccacggtggtggtaaccgatgtctggtacgcagtcgacaatctcttcgccatcgagttgcaaaacgatacggaaagccccgtgcgccgacgggtggttcggaccgaggttgaggaacatgaagtcctcgttttcggtgccgcgcttcatcccccactcttccggtttgaaggtcagggcttccatctccagatcctgtttggctttggtcagctcaaacggcgagaattcggtagcgcgcgccggataatctttacgcagcgggtgacctttccaggtttgcggcatcatgatgcgtcgcaggttcgggtgaccgtcgaaagtaatgccaaacagatcccaggtttcacgctcataccagttagcgttcgggaacagtttggtgaaggtcggtacgtgcaggtcgttttctgccagcgccaccttcagcatgatgtcgcggttacgatcgatagaaatcagatggtagaaaacggaaaaatccgcggcaggtaacccttcgcggtgtgtgcgcagacgttcgtccatgccgtgtaagtcaaacagcatgacgtaaggtttcggcagtttctttaagaaatcgccaacttccagtaattgttcacgcttgatccacacaacgggaaccccggtgcgagtcgcctgaacagtaaaggcatccggcccaaaacggttgcgcagttcgccaatcaccggatcatcaagatgatcgcgggtctgccaggcgggttcttgcgcggttaagtcggtcatattgttcaccattgcaaatggtccgtggtgactgtcggcgcagtaagcttcgcgaaatagatttaggaataagcgaagaaaaatccctttgccgacaggcgcaaattaaatctcgtcaggtgtacgcaggttagttacggcaatgcgttcaccgcgcttgcgttcgcgctctgattgcatattggcgcgataaacgccctgatcgccaaccacccaggagagcggacgacgttctttgccgatagattcctgcaacagcatcagtgcctgcatgtacgcttcaggacgcggcgggcagcccgggatatacacatcaaccgggatgaatttatcgacgccctgcacaacggaataaatatcgtacataccaccagagttggcacaggcacccattgagataacccattttggttccagcatctggtcatacagacgctgaataaccggtgccattttggtaaagcaggttcctgcaaccaccatcaggtcagcctgacgcggcgaagcacgcaatacttctgcgccaaaacgcgccacgtcatgcaccgcggtaaacgaagtcaccatctcaacgtaacagcaggaaagaccgaagttatacggccaaattgagtttttacgaccccagttaaccatgtcattgagcttgcccataaacacgtttttgttaacttcttgctccagagggtcggttacgatctcctgcttttgcagggggtaacggtcgttctcaccgttgggatctatgcgggtgagcgtataatccatcttaatgcctcgcggttagcgttgacgattagcgatactgttcgtttccgggttcatacgctcgcggcgtgaacgcgcgggcgtccagtccagcgcgccaatacgcaccagataaaccagacctgccagtaacacaaaaataaaaattgcagcttccacaaagcctacccagccgctttcgcggatagaggttgaccatgcgaacagatacagcgcttcaacgtcgaagataacgaagaacatggccaccagataaaacttggcggacaggcgtaagcgggcggagccgaccgagtcgataccggattcaaacggcacgtttttcgacctcgcgcgtgcgcgaccgcctaaaaaccaaccgcctaccagcatcaggcaacacaggccaatggcaacgataagaaagatagcgaatgcccagtgatgagcgatgacttcagtggatgttgacatactcattgcttactcatcaaaagtagcgccagattcactgctcttcacggcagatggacgccacatcgattcatggggaggaataaaaaaaaccttacaatcactgtagaaattcttttatacagctaattgatgtggttttttactcctttctataaccttttgtcaactttaacaaaagtttcttcacattagtttacataatatcaacaccattagcatttaatgccctttcaccccagatccttgacgactccaggataattagatgttgttgaatcgtgtccgttgtgaagcaatggaaaaaatacgggtctattttgacaggaatttgtgtcgattcctccccccaaaagagagtattttcttgatctgtgacacgcttttgtcattccataacaaaaacgcagcaacaaatttacgtattttttaacatcattgtagcaggtgatttttttcaggcgattatttgtgcgttcgggacgtgaatctctggtggttgaaaaatgaacagttttgtacgttctgcactatgcgatgaaggatttttactaaaaaaaagccgctggggtttaaaacacccccagcggctcgttttttacactattgtctcaggaattatctatcgtccgtcgattactcgatatccctttcaatcaacaatgaatcatccccttccggagcagacattgggctgtattgccacggattatggtagctctccatcgcctgatagatcacctgggccagctcattattactggacggatcatagcacagcaaatattcggtatcaggtagcggcggtaagccatctactccactcagcacacgcaggtccgggctcatcatctcaaccggccttgccgtcacgccaagaccggctttcactgccgcacgaacggccggaagcgtcgaggcgacataagccagtcgccatggaatatctgctttattaagcgtcgccagcaccatatcgcgaaacgggctaggatcatccagcaatacaagagggatcggctcgcctttttgcaatatgtattccgctgcgcagtaccagtgtgttggcgaggtacgcaggttcaatgccttaaacgctgaaggacgatgggtggttaccatcaaatccacttcctgggattccagcatttctgccatataggcattacgtttaacgcggacatccagcgctaatttcggataaaccgaactcacgcgatttaacaggaaaggtaagatcgtatcggcagattcatctgaagcaccgatagttaatacgccctgaagattactgaacattaatgatgagcaggcctcatcattaaaacgcaggattttcctggcgtaaccaagaagttgaatgccatgttcagttaacagtttgttgcgaccgtgacgagcgaacagttctttcccaacgagttgttccagacgctgcatttgctgacttacggcggactgagtacgacacacagcggcagctgcggcagcaaaagtgttcagatcggcaacagcaacaaatgttctcagcagatcgaggtcgaggttaattatcggacgatttgcacttatcatatattatcacttactggcggctcatactgagctggttaatgctgtgcacacacaaacaagcaattccatttgtaatgtgcctccctggcagtttcatccggaacccggacgaaagtaaaaatgcatatgagttgcactaaaaaagcgactcacattgttccgttataatgcctgaagtagatcacagaatatatcttcagggatcgcatatctattaagttactcactcttttctatttatgacatgcgcgtgtttgtataaatgtaaatgtgagtccttgttccactctcgtgcagcatcgctggtcatacgcgaacacgtaccaacagcaatggtgaggcggcatcaagagcagggatccgtcatttatccgagcattttaccccaaaaaccttttatttataagggtcattgcgaattatctgatgcaaagttatgttatgttaggcaaagtaatcttctattattaataagcacatcaaaacctttttgaatattaaataataattaattagcatcatcctcattcattaattccgcttaacaatagtttcacaccttgcccccattgcgacacctcggaaatcatcacgcagttaaactctccgtaatgaggaaatatcatcatcgcgtttcattagtgaattcttaaatgaggcattttcacacaattatcttacagataaaaaaaccagacttacaattaagaatcagaacaattcactatataacattgcatgtaaagcatatacacctcattattttgtcattattaagttattaacagcacaatcgagccttcccctctggcaaaatcttattctgcagaccttcaaaacaccgtcctgggggagtacattgttctaagctgacttccacggcagggagtggcgataacagcaaaaaaggtcaagattcatgtcccccattgaaaaatccagcaaattagagaatgtctgttatgacatccgtggtccggtgctgaaagaagcaaaacgcctggaagaagaaggtaacaaggtactgaaactgaacatcggcaacccagccccgttcggttttgacgcgccagatgaaatcctcgttgacgtgatacgcaacctgcctaccgctcaagggtattgcgattccaaaggtctttactccgcgcgtaaagccatcatgcagcactaccaggctcgtggcatgcgtgatgttaccgtggaagatatttacatcggcaatggtgtatcggagcttatcgttcaggcaatgcaggcattgctgaacagcggggacgaaatgttggttcctgcaccagattacccactctggaccgcggcggtttcgctttccagcggtaaagcggtgcattatctttgcgatgaatcctctgactggttcccggacctcgatgatattcgcgctaaaattacgcctcgtacgcgtgggatcgttattatcaacccaaataacccaaccggcgcggtatattccaaagagcttttaatggagattgtggagattgcacgtcagcataatctcattatcttcgccgatgaaatttatgacaaaattctctacgacgacgctgagcatcactcaattgcgccgctggcacctgacctgctgaccattacctttaacggactgtcgaaaacgtaccgcgttgcaggcttccgtcaggggtggatggtgttgaacgggccgaaaaaacacgccaaaggctacatcgaaggtctggaaatgctggcttcaatgcgcctgtgtgctaacgttcctgcgcaacacgccattcagaccgcgctaggtggttatcagagcatcagtgaatttattacccctggcggtcgtctttatgagcagcgtaaccgcgcgtgggaactgatcaacgatattccgggcgtttcctgcgtgaaacctcgtggtgcgctgtatatgttcccgaaaatcgacgccaaacgctttaacattcacgacgatcagaaaatggtgttggatttcctgttgcaggaaaaagttctgttggtgcaagggacggcattcaactggccgtggccggatcacttccgcattgtcacgctaccgcgtgtcgatgatatcgagctgtctttgagcaagttcgcgcgtttcctttctggttatcatcagctgtaatcttaatttcactgccggagattgcatccggcagcgttatcccgccacaatgacctgatgatgtcatcatacgtaaggtcactatgaaacagagccatttttttgcccatctctcccgcctgaaactcattaaccgctggccgctcatgcgcaacgtgcggacggaaaatgtgtccgaacacagtttgcaggtagcgatggtcgcccatgcgctggcagctatcaaaaatcgaaaatttggcggtaatgtcaacgccgaacgtatcgctttactggcgatgtaccacgatgcctcagaagtgctcaccggcgatctccctactccggtgaaatacttcaattcgcaaatcgctcaggagtacaaggctattgaaaaaatcgctcagcaaaaactggtcgatatggttccggaagagctgcgggatatctttgcgccgttaattgacgagcatgcatatagcgatgaagaaaaatcgctggtgaaacaggcagatgcactgtgtgcatatctgaaatgtctggaagaactcgcggccggaaataatgaattcttgctggcaaaaacgcgactggaagcgacgcttgaagcgcgtcgcagccaggagatggactacttcatggaaatatttgttcccagcttccatctttcgctcgatgagattagccaggattcaccgctgtaagcagccggagtctgcgtcgcatcaggcaataagcgccggatgcgacatcaggctcttgtcaaaacggaaacagcatcgggatcatcaccacacaaaccgccatcacgataatggtgaacggtacccccaacttcacaaagtcactgaagctgtaatttcccggacctaaaaccagtgtgttaacaggtgaagaaaccggtgtcataaaggcggcggatgctgccatcgccacgaccatcgcgaatggataaggcgacacccccatcgttttggcagcagccagcgcaatcggagccatcaacaccgccgtcgcggtattagagataaatagcccaataaccgccgacaagacaaacaaacaccccagcatcatatgtggcccgtaaccaccgccaatgtccatcagccctttcaccgccagcgcgacacctcccgttttctgtaatgccacagcaaacggcatcatcccaacgatcaaaataatgctcggccagtgaatggatttataggcgctttcagcatctatacagcggaatttccccatcagcaggcaggcgatgatagcggcaacaggattaggaatttcatctgtcagcattaacgccaccattagcaccagacagaaaatggcatggggtgcctggctgtgcgcgggtgatgcttcactcacctcttccggtaagttcagcgctacgaagtcgcggccctgtttggccagcataccgatcagtttccagttacccacaaccaggatgatatcgcccagcagcagaggctcatccgccagcgaaccttccagcgccacgccattgcgctttagccccaccacattcagtccgtagcgggtacgaaaaccaatttcgcgcaccgatttaccaatcagttctgactcaggaattaatgaaatctctgccatgcccacatcaagggcctggtcagaaaaatactcgccgcgcagtaccatcggctccagcaattgctcactacaaaattgccggagatcgacatcagccgcagacatatcaataagcaaaacgtcacgcgcgcgaaattcagaaaccccattaacgttcacgataacgcgacgaaaacgccgccagcgttcaacaccgatgacgttagcgccataacgctcacgtaatttgagatcatccagccgttgaccaatcattggcgatccggggcgaatagccagacgtcgcgcacgcccggtcagtcgatattcacggataagatcgcgaaaggttcgacgcgtccagccttcgcgctgcggggtctgggtatcccctttcagcatgaaacgcatcactaacatatacaaaatacccagcaccagcacgaccaggccaataggtgttacgctaaagaaactgaagccgtgatagccttcacgcagcaattcactgttgactaccaggttcggcggcgtcgccaccagcgtcatcatgccgctaatcagcccggcaaaacttaacggcatcatcagacgtgacggcgacgtttgcatacgcatggcaacgcttaacaccacgggaataaagatagcgacaacgccggttgaactcataaacgcgccaagccccgcgacggtcagcatcaacaaaaccaacattttgatttcactattgcccgcaactttgaccagccatgttcccattacggtggcaacaccggtacggaccaaaccatcgccaataataaacaaggcggcaatcaggacaacgttaggatcagaaaagccggaaaatacttctgggactgtcagcgttccgcttaatgcaaacgcgacaataacaaacaaagcgaccgcatccatacgcactctgcccgtcgcaaacaagacgatggcaacggccagtaatgaaagaacccaaatcaattcaccgttcacaacttatccttgttaattgagggggatgacttgattctgccataaaaaagccccgacgagacggggctaaatcatgatcaggtgtttcactgaataataacatcgccatttggctgtttggtcacagtaatttgctccagactgtggaggaccaaatcgacctcattcaggcgcggggtatctgccggagcgttaaccgcaatgacatgacaacccgccgccaggccagaaagcacgccagcgggagcatcttccaccaccacacactcctgcggcgcaagccccagcagctgcgcgcctaacagatacgcatcaggttctggttttccgcgcttcactcgctcagcggttacaaacacctctggtgcgggaagcccagctattttatggcgcgctcgcgctaccggcatggagccagaagtcacaatggcccacggaatacctgctttattcaaatgactgagtaaggcgattgcccccggaagcgcggtaataccttcggtttccgtggcctcgatgtgctccagacgcgtaaactcggcggcaatatcagcctcggatttgcccgccataaaatggcgcagagaggtgatcgcctgtttaccgtgaatgaaagccagcacctcttccggcgctaacccatgacgtctggcccagttgctccacgcccgttctaccgcaggcagggaatccaccagcgttccatcaagatcaaacagaaaacctttgcaccgcacgcgggcctcctcaggcattgataatttgattaatttcgttggcgctcaaatggtactgacgcgggcaggcatgccacacattaagcatgcgctgatatttttcccacattggcgtctgggcgttaaaaccgtgagttccggcgtcaaaatgggtatagcgcccttccacattaaccataaagcggacataaccgaggtaacgtgcttcagtggcggcgtcaaagccgaggaaggtgacacgacgttcatcgatggattgctggtcctgcaaattagaccaggaaacatgcaacgcatgatacatctccataatgtcgatgatagtgcggcaggtttcttctttcagctcgccaaactcgcgatccaattcacgcatctgtaatccgtaaccacgctcaataattgtttgcaggcgacggtaacgttcagcatttgccggatcgagcatagtcatcatcttgtactgattagacaaaataagacgttgcgcgttggtcatttccattgttgactcctgtatcactctactacggtgaaaaaaaagaaggctgagtatgccttcttttatatgcgtaatcaggggtcaattacaaatcatcaaggaaagttttatccagttgtttgaaggcgcgcttaagcgtgtcagctaatgcctggtaatcaggcttgccttcaacgggtgccaacacctgtccagactcctgcaatttaccgcgaacttcataaaaccagttaaggattgcagggggtaatggcgtgacagaacgcttgcccagccaccacaatccctgcatgggtaaacttaaggcgaacagggcagtggcaactgccggcccaagctgaccgcccagggcaatctgccagcagagagtaaatacggcgatcggcggcataaaacggatcgcataacgcgtcatcttgataacgcgattttcgacaaagaccggggcaaggcgtttttccagcggccacgtctttgagtaatgctgtccccggcgaaacaagctaaaaaaattaacagaacgattatccggcgttgacatgcttcacctcaacttcacatataaagattcaaaaatttgtgcaaattcacaactcagcgggacaacgttcaaaacattttgtcttccatacccactatcaggtatcctttagcagcctgaaggcctaagtagtacatattcattgagtcgtcaaattcatatacattatgccattggctgaaaattacgcaaaatggcatagactcaagatatttcttccatcatgcaaaaaaaatttgcagtgcatgatgttaatcataaatgtcggtgtcatcatgcgctacgctctatggctccctgacgtttttttagccacgtatcaattataggtacttccatgtcgagtaagttagtactggttctgaactgcggtagttcttcactgaaatttgccatcatcgatgcagtaaatggtgaagagtacctttctggtttagccgaatgtttccacctgcccgaagcacgtatcaaatggaaaatggacggcaataaacaggaagcggctttaggtgcaggcgccgctcacagcgaagcgctcaactttatcgttaatactattctggcacaaaaaccagaactgtctgcgcagctgactgctatcggtcaccgtatcgtacacggcggcgaaaagtataccagctccgtagtgatcgatgagtctgttattcagggtatcaaagatgcagcttcttttgcaccgctgcacaacccggctcacctgatcggtatcgaagaagctctgaaatctttcccacagctgaaagacaaaaacgttgctgtatttgacaccgcgttccaccagactatgccggaagagtcttacctctacgccctgccttacaacctgtacaaagagcacggcatccgtcgttacggcgcgcacggcaccagccacttctatgtaacccaggaagcggcaaaaatgctgaacaaaccggtagaagaactgaacatcatcacctgccacctgggcaacggtggttccgtttctgctatccgcaacggtaaatgcgttgacacctctatgggcctgaccccgctggaaggtctggtcatgggtacccgttctggtgatatcgatccggcgatcatcttccacctgcacgacaccctgggcatgagcgttgacgcaatcaacaaactgctgaccaaagagtctggcctgctgggtctgaccgaagtgaccagcgactgccgctatgttgaagacaactacgcgacgaaagaagacgcgaagcgcgcaatggacgtttactgccaccgcctggcgaaatacatcggtgcctacactgcgctgatggatggtcgtctggacgctgttgtattcactggtggtatcggtgaaaatgccgcaatggttcgtgaactgtctctgggcaaactgggcgtgctgggctttgaagttgatcatgaacgcaacctggctgcacgtttcggcaaatctggtttcatcaacaaagaaggtacccgtcctgcggtggttatcccaaccaacgaagaactggttatcgcgcaagacgcgagccgcctgactgcctgatttcacaccgccagctcagctggcggtgctgttttgtaacccgccaaatcggcggtaacgaaagaggataaaccgtgtcccgtattattatgctgatccctaccggaaccagcgtcggtctgaccagcgtcagccttggcgtgatccgtgcaatggaacgcaaaggcgttcgtctgagcgttttcaaacctatcgctcagccgcgtaccggtggcgatgcgcccgatcagactacgactatcgtgcgtgcgaactcttccaccacgacggccgctgaaccgctgaaaatgagctacgttgaaggtctgctttccagcaatcagaaagatgtgctgatggaagagatcgtcgcaaactaccacgctaacaccaaagacgctgaagtcgttctggttgaaggtctggtcccgacacgtaagcaccagtttgcccagtctctgaactacgaaatcgctaaaacgctgaatgcggaaatcgtcttcgttatgtctcagggcactgacaccccggaacagctgaaagagcgtatcgaactgacccgcaacagcttcggcggtgccaaaaacaccaacatcaccggcgttatcgttaacaaactgaacgcaccggttgatgaacagggtcgtactcgcccggatctgtccgagattttcgacgactcttccaaagctaaagtaaacaatgttgatccggcgaagctgcaagaatccagcccgctgccggttctcggcgctgtgccgtggagctttgacctgatcgcgactcgtgcgatcgatatggctcgccacctgaatgcgaccatcatcaacgaaggcgacatcaatactcgccgcgttaaatccgtcactttctgcgcacgcagcattccgcacatgctggagcacttccgtgccggttctctgctggtgacttccgcagaccgtcctgacgtgctggtggccgcttgcctggcagccatgaacggcgtagaaatcggtgccctgctgctgactggcggttacgaaatggacgcgcgcatttctaaactgtgcgaacgtgctttcgctaccggcctgccggtatttatggtgaacaccaacacctggcagacctctctgagcctgcagagcttcaacctggaagttccggttgacgatcacgaacgtatcgagaaagttcaggaatacgttgctaactacatcaacgctgactggatcgaatctctgactgccacttctgagcgcagccgtcgtctgtctccgcctgcgttccgttatcagctgactgaacttgcgcgcaaagcgggcaaacgtatcgtactgccggaaggtgacgaaccgcgtaccgttaaagcagccgctatctgtgctgaacgtggtatcgcaacttgcgtactgctgggtaatccggcagagatcaaccgtgttgcagcgtctcagggtgtagaactgggtgcagggattgaaatcgttgatccagaagtggttcgcgaaagctatgttggtcgtctggtcgaactgcgtaagaacaaaggcatgaccgaaaccgttgcccgcgaacagctggaagacaacgtggtgctcggtacgctgatgctggaacaggatgaagttgatggtctggtttccggtgctgttcacactaccgcaaacaccatccgtccgccgctgcagctgatcaaaactgcaccgggcagctccctggtatcttccgtgttcttcatgctgctgccggaacaggtttacgtttacggtgactgtgcgatcaacccggatccgaccgctgaacagctggcagaaatcgcgattcagtccgctgattccgctgcggccttcggtatcgaaccgcgcgttgctatgctctcctactccaccggtacttctggtgcaggtagcgacgtagaaaaagttcgcgaagcaactcgtctggcgcaggaaaaacgtcctgacctgatgatcgacggtccgctgcagtacgacgctgcggtaatggctgacgttgcgaaatccaaagcgccgaactctccggttgcaggtcgcgctaccgtgttcatcttcccggatctgaacaccggtaacaccacctacaaagcggtacagcgttctgccgacctgatctccatcgggccgatgctgcagggtatgcgcaagccggttaacgacctgtcccgtggcgcactggttgacgatatcgtctacaccatcgcgctgactgcgattcagtctgcacagcagcagtaatctcgtcatcatccgcagctttgcgctgcggatatctgaaccggaaataatcactatttccggttttttattctcttaatttgcattaatcctttctgattatcttgcttaactgcgctgcatcaatgaattgcgccatcccactttgcatacttaccactttgttttgtgcaagggaatatttgcgctatgtccgcaatcactgaatccaaaccaacaagaagatgggcaatgcccgatacgttggtgattatcttttttgttgctattttaaccagccttgccacctgggtagttccggtggggatgtttgacagtcaggaagtgcagtatcaggttgatggtcaaacaaaaacacgcaaagtcgtagatccacactcatttcgcattctgactaacgaagcaggcgaacctgagtatcaccgcgtacagctgttcacgacgggcgatgaacgcccgggcctgatgaacttcccgtttgaaggattaacctcaggatcgaaatacgggacagccgttggcatcatcatgtttatgctggtgattggcggcgcgtttggcattgtgatgcgtacaggaaccattgataacggtatcctggcgcttattcgccatacccgcgggaatgaaattctctttattcctgcgctgtttattctgttttcacttggcggcgcggtatttggtatgggagaagaggccgtcgcctttgccattatcatcgcaccgctaatggtccggctgggctatgacagtattaccaccgtcctggtgacctatattgccacgcaaatcggttttgccagttcgtggatgaacccgttttgtgtggtcgttgctcaggggattgccggcgttccggtgctttctggctccgggttgcgcatcgtggtgtgggttatcgccactctgattggcctgatctttaccatggtgtacgcctcacgagtgaaaaagaatcctcttctgtcacgcgtgcatgagtccgaccgcttctttcgtgaaaagcaggctgatgttgaacaacgtccgtttacctttggtgactggctggtattgattgtcctgaccgccgtaatggtctgggtgatttggggcgtgatcgttaatgcctggtttattccagaaattgccagccagttcttcaccatgggtctggtgattggcatcatcggcgttgttttccgccttaacggcatgacggttaataccatggcttcatcctttaccgaaggggcgcgaatgatgatcgcccctgccctgctggtgggtttcgccaaagggattttgctgctggtcggtaatggtgaagcgggtgatgccagcgtgttaaataccatcctcaacagcattgccaatgccattagcggtctggacaacgcggtcgcggcctggtttatgttgctcttccaggcggtatttaatttcttcgtgacgtccggttctggtcaggcggcgttaaccatgccgttactggcaccgcttggcgatctggtcggtgttaaccgtcaggttaccgtgctggcgttccagtttggtgatggcttcagtcacatcatttacccaacctcagcgtcgttaatggcaacgctcggtgtgtgcagggtggacttccgtaactggctgaaggtgggcgcgaccctacttggactgctgtttattatgtccagcgtcgtagtgatcggcgctcagttgatgggctaccactaaaaatgttaagagccgcaattgcggctcttttttcattctgccgtttcagtctctacggcttcatttttggcattgcgcttcatccacaacgctagcgctttcagcgagtctggagtgaactcatcgcagcgtgcggtgatttcttccggcgtcagccagcaaacttcactgacttcatcttcctgtagtgcgaagggaccgtgagagacgcagctgaacaatgcgccccagacacggcaatttttatcttcgaaatagaactgcccgtgctcggcaaaggggacaccggcaatgcccaactcttcttccgcttcgcgacgcgcggattccagcagttgctcatcggcctggactacaccgcctgcggtcgcatctaacatgccgggtaaaaagtcttttgtctcggtacgacgctggaccagaattttgcccatgccatcatgcacgacgatgtaagttgcacgatgacgcagacactgtgcccgcatttgttcccggctggcttgtgcaatgacttcgttctcttcattgacaatatccacccattcagtacttgccaaacgacgctgttccattatcaggaaaccttctttttctggcgctcttacggcgcattttgagttgtgggtaaattacggattaatcgcgacctgcgcaatgatactttgatcattgagtgcgattacactaagtacgtcattatccagcatgccataactcgccggattaccgcctttcggaatactcaccgagccggggttgaagtggaaaatctccccccgctgttctgccactggcagatgggtatgaccgtacaccagcacatcgttctggtttaaagcaggcagattttccgggccaaaaagatgaccatgcgtcaaaaacagacgttgtttttccagtaatacctgttgccacggcgcggttatcgggaaatgcagcagcatttgatccacttcgctgtcgcagttgccgcgcacagcgataaccttatgtgccacttcattaagccgttcagcgactttggctggcgcgtaaccctccggtaaagcattacgcgggccgtgattcaacacgtcgccaaggatcaccagccactgggcaccgctttgggcaaacaactccagaacacgttccgtcgccggtaacgacccatgaatgtccgatgcaaacatcagtttcatcactcactcctcgtcgaaaaaacgtaagctatgatactggattctgtcgttgctatcagccagattgcttcgccgaaagtgcaataaaacgctggacagacgctcgctgccactggaatgttgcataatccaccaggcgttctggcacctcatcgccatgtagtaccaggcggttaatcattagcgccagatcagtatcagcaatgcaccattcaccaaataaattcggctgacccagtactaacaaatgttctgccatcgcgaacagtttctctgcactggcttttccctcggccgttagtggcgcttttttcgcccccgcaaagacaacatccgtcggacgctcttcgcggatgggcatcagatcgctgcgcagccaggcctgaatctgtcgtgcacgcgcacgattttctaaatcaagcggataaatacgttcccaggtcggtggcgcaaatcgatcttccagatactccgcaatggcagaagattcactcaactcaaaatcatcgatttgtaataacggcacacggcgtgtctgaccgtaaccttgccacgtcggctgcaaatgttcaccgctgtcgaggtcgatggtcttgatatgaaacgacaggcctttttcctgcaacgccacccaggcggataacacataaggggagaaaaagtgggcatctgaccaaagcgtgatagcgggtttactcattatgtcctcggcaataaagggggctggctatcaaactatagagcctttttgtcactgtcacgtgacgaatactcacgtaagtcgccgcgctttctatacttgtggtgttcagatgattaaacaaccggagctgcaatgatcgatctctatttcgccccgacacccaatggtcacaaaattacgctgtttctcgaagaagcagagctggattatcgcttgattaaggtagacctggggaaaggcggtcagtttcgtccggaatttttgcgcatttcgcccaacaacaaaattccggcaattgttgatcattctcctgccgatggcggcgaaccgctaagcctctttgagtctggtgccattttgttgtatctggctgagaaaacaggactctttttgagtcatgaaacgcgtgagcgcgccgccacattacagtggttattctggcaggtaggcggactggggccgatgcttgggcaaaatcatcattttaatcacgcagccccccaaaccattccttacgctattgaacgttatcaggttgaaactcagcgtctttaccatgtactgaacaagcggctggaaaactcgccctggctgggaggcgagaactacagcattgcggatattgcctgctggccgtgggttaatgcctggactcgccagcgaattgacctagcaatgtatccggcagtcaagaactggcatgagcggatccgttcgcgccctgccaccgggcaggcactgctaaaagcacaactcggtgatgagcgttcggatagttaacagaaacaggttctcgtgtattatttcatcctaagtaaaacaacggagaacctgcaatggcacaacctgccgctattattcgtataaagaaccttcgtttgcgtacgtttatcggaattaaggaagaagaaattaacaaccgtcaggatattgttatcaatgtgacgatccactaccccgccgataaagcgcgcactagcgaagatatcaacgatgcgctgaattatcgcaccgtaacgaaaaacattattcagcatgtagagaataaccgtttctctttgctggaaaaattaactcaggatgtgctcgatatcgcacgtgaacatcactgggtgacgtatgctgaagtggagatcgataaactgcacgcgctgcgctacgccgattcggtatccatgaccttaagctggcagcgttaatcgccatatcgggaggctgcatgaacatagtgatcaccggagggacaggattaattggtcgccatttgattccgcgtttgctggagctgggccatcaaattacggtagtgacgcgtaacccgcagaaagccagttccgttctcggccctcgggtgacactatggcaagggcttgccgatcaaagcaacctcaacggcgttgatgcggtaatcaacctggccggagaaccgattgctgataaacgctggactcacgagcaaaaagagcgtctctgccaaagccgctggaatatcacgcaaaaactggtcgatttgattaatgccagcgacacgccaccgtcggtactcatttccggctcggcaacgggctattatggtgacttaggtgaagtggtggttaccgaagaggaaccgccgcataacgaatttacccataaactctgcgctcgctgggaagaaattgcctgccgggcgcaaagtgacaaaacgcgagtgtgcctgctgcgtaccggtgtagtgctggcaccggatggcggtattctcggtaaaatgctgccgccgtttcgtcttggcctgggcgggccgattggctctggtcggcagtatctggcctggattcatattgatgatatggtcaacggtattctctggctgctggataacgagctgcgcgggccatttaatatggtttcgccctacccggtacgcaatgaacaatttgcccatgcgctcggtcatgcgctgcatcgcccggccattttgcgcgtccccgcgaccgccattcgactgttaatgggcgaatcttcagtactggtattaggtggacaacgcgcgctgcctaaacggctggaagaagcgggttttgcgtttcgctggtacgatttagaagaggcgctggcggatgtcgttcgctgatgtggtttacagcaaacatccgccagttaactcccggtgttacaggattagtggctttgcgcgataagatcgtctggtgaaagtcgggtcaccatcataactaactctctgtctaaacctctatccagcatctcctgagcaatacgcagggcttcttcgtgtttgccctgcattgcgccttcttcacgtaatctgtcagcaatggtcatcagtttctccttttcttgtggtgcgcgttccgctatctcaccaataaatgcacgaaaacgctgggcatcccctgtttgtaatacgtaattaaacagggcttttagctgtctgtcattagtgttccctgtaactagcagcgaaacaatttggtcgactaatcccaacagatcgcgctgacgaatatgtttctgaattaactccaacagcgccattttgcggtgttgcataatctcgtcatccggcaccacggtaatatccaccaacggaaaagccgatgaatatattttgcgggctatagcaggctcggcaaattcatcaagccagcagagtgaataaggataaggacttctgcaaccatgataaaacagcatcgggagcaccaatggaagctctttatagcccgcatcaagatggttttgcattgccgcaatggaataacgcatcatgcgaaaagccattaattcttccggcttactttggtgctctatcactacataaatataacccactccctcctgcgttttcacagaccacaagaggtcggaataatattgccgcaggtcttcatcaataaaactgtttggttccagtttaagcgtcgttaaatcacacagtttgcgcagcggcgcgggaagatgaatatcaataaaatcccgcgcggtgtctggatggcgtaaaaaagatttaaataccgcatcatgcggcgtggaagttgtcgatattgtcatggcgttccgtcacccctcaaatttaagatgacgcgacaataaccacgattaacacccaatgcagcaggcagtttttatctttggacagcgaattcagaagtatttttagcggactgtaacttttacatttcagcggaagctgactcgcaaattccccatgaaaatactccggcagcgttagccaccggagaggaaattatttcagcgatcccttaaggaaccgttgcagacgagggctttgcgggttgccaaataactgctccggcgcgccctcttcttctattttcccctgatggaggaaaatgacatgagtagaaacatggcgagcaaagcccatttcgtgagtcactaccaccatggttttcccctcttctgccagttgctgcataatacgcaacacttcgcctaccagttcaggatcgagcgccgaggtaggttcatcaaacagtaaaacttccggttccatcgccagcgcccgcgcgatagaaacacgctgttgctgaccgccggaaagatgcaccggatatttcccctgcgcacgttcgtctatcccgacttttgccagatacttcaccgcccgctcgcgcgcttcctgcttgctcaggcccaacacctgaatcggcgcttccatgacgttttccagcaccgtcatatggctccagagattgaagtgctggaataccatcgtcaggcgtgtgcgcagtaagcgcagttgatttttatcggcgactttgagttgaccgtctttgtcgcgcaccagattgatcgtctggccattgaccacgatcgacccttcactcggtttttcgaggaagttaatgcagcgcagaaaggtacttttccccgatcccgacgatccgatgatgcttattacatctccggcattcgcttgcagtgatacccctttcagcacttcatgttcgccgtagcgtttgtgcaaatcgataacgtttaatttattctcggacatcgtattctcagtgcgttgaagaaggtttcacatgctgcaaccagcgtttttccgctctgcgaaagaggctgatcaggacataagagatgattaaatagagcaccgcggcaatgccgaaggcggtaaaaggttgatacgtggcggcgttaatatcgcgggctattttcagcagatccggcaccgtggcagtaaatgccaacgcagtagagtgcagcatcaggatcacttcgttgctgtatgccggtaacgcaatacgcagcgcagaaggcaaaataatgcagcgatacattttaaaagtcgagaagccataggctctggcggcttcaatttccccatgcggaaccgaacggattgccccagcaaaaatctcggtagtgtaagcgcaggtgttaagcgtcagcgccagcacggtacagttcaggccactgcggaagaaagcgttaaggaattcggttcccttaacaatctcaagcgtgtacatgccggaatagaacaccagcaactgaacatacagcggcgtaccgcgaaaaatataggtaaataaccagattggaaactggatgtatttattactggagacacgaccaatcgccagaaacagcgccaggactccgcctatcactaccgacaaaataagcagccacagagtgatcgccacaccagtaaagcgataaccgtcggtccacagcagcggtttccagtattcatgtaagatttcgatcacaggtcagccctcttcacacccacggagtagcggcgctcaaggaacagcagcacaccattggaaacagtggtgaaaaccaggtaaatcacgccacagacgatggcgaaatagaacggttcccaggtacttttgcctgccagttgggtggctttgaccacatcttccaggccgagtaacgaaaccagtgcggtagatttgaggatcacctgccagttgttgccaatgcctggcagggcgtaacgcatcatcgacggaaacatgatccgccgaaacacttgcccacgagtaaaaccgaacgccgtcgccgcctctatatgtcctttcggcactgccataaaagcaccacggaacgtttcggtaaaataagcaccgtagataaaaccgagagtgataataccagcgaccatcggatcgatatcaatctgcccgacgcccatcgcctccgtcaccgtgtttagcgcaatctgcaaaccgtagaaaatcagcagcatcaacactaagtccggcacgccacgaatcagcgtggtgtacccttcgaaaatcagccccgaaagccgattttgcgagagcttaccgccagcgccaattaaaccgatgattacagcgagcactacagagctgatagccagctccagcgtgacgagcgcaccctgtaaaataacacctgaaaacccatacaacatgctgcctgtcctgtcgtgtgtggtgaattaccgcctcttgtctccctccggttacccgaagggagcgggctttctttcaccgatggcgattagccaccataaacatcaaaatcgaagtactttttcgctaatttctcgtaagtaccgtcagcgcgcatttcggcaaaggctttgttcagtgcttcgcgcagttcgttatcttctttacgcaggcccatgccggtccctacgccaaacagtttttcatctttaacagacgggccaccgaatttgtaatctttaccgacaggttgtttgaggaaaccttcgctggcagcgacctcatcctggaacgcggcatcaatacgtccggcagtcaggtcagaataaatgttgtcctgcccctgatacgagacgatttcaatgccttttggtgcccaatgttcattaccgaacgtctcctgggtggtgccctgcaatacgcctacccgtttgcctttcagcgactcgactgtcggctgaatgtcagaatttttcgccaccaccaaacgagaatcggcagcgtacagtttgtcggtgaaggctatttcttgctgacgtttttccgtaatggaaagcgatgacatgatggcgtcaatcttcttcgcttttaaggacgggattaacgcatccagcggattttcgacaaacgtacattgcgtattgatgcgtttgcataattcctttgccagatcgatatcgaagccaaccagttcgccttgtgaattttttgattcaaatggcgcataggtcgggtcggtaccgatgcggatgttttgcggaatcgcagcaaacgccgcagttgcgctggagaaggccagaaccagagagagcgatagcaccagttttttcataatgtcctcaactgacagtctttttatagggaatatttacaggtttgttacacttatcgtgccataaaattgaccatcaaggcaaaatatcccgccccgttagacgtattatttttcattaaaaatgcttaagtatgcatttcaatgcaccacgatagtgcaacaaacctggcgtgcaccatgatgatcattccatcaggtacagcttcccagcgacgtatcagtcaccgtagacattaaagtcgaaatactttttcgccatcttgtcgtaggtgccgtcctgacgcagctcgccaagcgccttattgaaggcagccgtcagttcagcatcatctttacgtagccctacaccggtgccatcaccgaagtattttttgtcttttactgatgagccagcaaaggcgaaatctttaccagcaggttgcttgaggaatccttcgctggcagcaacttcatcttgtaacgcagcatccagacgtcctgcagccagatcggaatagaccaaatcctggttggcataggccaccacatccacgcctttactacgccaggtctcgttagcgtaagcttcctgggttgatccctgcagcacaccaacatgtttacctttcagtgaatccagcgttggctgaatcggtgaacctttggccgcaatcaaacgagaatctgcggcgtacagcttgtcggagaaggcaatctcctgctgacgtttatcggtaatggaaagcgacgaaataatagcgtcgatttttttcgctttcagtgaggggatcagcgcgtcaaagtcactggcaacccaggtacatttcacctgcatccgtttgcacatctcgttaccgagatcgatatcaaagccaacaaaatcacctttagcatctttcgatgagaacggtgcgtaggtggtatcggttccgatacgtaccgtctccggtagcgccgcatagctggaagccgctgtggagagaccgactaacaaagacagagcgagaatcgacttcttcatacataaccctcaagtgaaaatggcttttttatgttgtgtattgtgttgtgtgtttgcaggctctttcatgcaggtcttatgccatcttgacgacaacagtaacattcaacgttaaatatgttaataagacgttgcattattgtcctgaagttgaagatagcaggtatagcggttgaatcgcagcgtttcgattgaatggcagaaacaaaatgtcgaggatttgatcgcggttgcaaaattgccctgaaacagggcaacagcggagttatgcgccctgccagcgggcaaagagatcttcaggaagggttatcgcaaactggtcaagaacacgattaaccgtctgatttatcacatcatcaagggattgcgggcgatgataaaacgccggaacgggaggcataatcaccgcaccgatttctgccgcctgagtcattaaacgcagatggcctaagtgcaatggtgtttcacgcacgcagagcaccaacgggcgacgctctttcagcaccacatctgccgcacgggtcagtaagccatcagtatagctatggacaatgccggaaagggttttgattgaacagggtaaaatcaccatccccagcgtctggaaagaaccggaagagatgctggcggcaatatcgcgcgcatcgtgcgtgacatcggctaatgcctgcacttcgcgcagagaaaaatccgtttcgagggataaggtctggcgcgctgcctggctcatcaccagatgcgtttcgatatctgtgacatcgcgcagaacctgtaataagcgcacgccataaatcgcgccgctggcaccgctgatgcctacaatgagtcgtttcataaatagttgccctgtcagacttgcaggcagactttgcaggatttcggcgggagttgcaagtcagggtgccagaccggcaccctcagcgaaggcatcatccttcgttatgcatttcgagattttccacttcgttctgacgttgcactgctttggcgtcatcattacgtaacgtatcgaggaaatcgaggtagccctgatcaacatctttggtgacgtagacgccgttgaacaccgagcattcaaactgctggatatccggattttcagcgcgaacggcgtcgatcagatcgttcagatcctggaaaatcaacccgtcagcaccgatgatctggcgaatttcatcaacttcgcgaccgtgagcgatcagttccgtggcgctcggcatatcaataccataaacgttcgggaagcgaatttccggtgccgcagaagcgaggtacactttcttcgctccggcttcgcgtgccatctcgataatctgctcagaagtggtgccacggacgatggagtcgtcgaccagcaggacgtttttatcgcggaactcggcgcggttggcattcagtttacggcgcacggacttacgacgcagctgctggcccggcatgataaaggtgcggccaacatagcggtttttaacgaagccctggcggtacggtttgcccagaatacgagcaatttccagcgcgatatcacacgaggtttctgggatcgggatcaccacgtcgatatccagatcttcccattcgcgggcaattttctcgcccagtttcgtgcccatattcacacgcgcgctgtaaacggaaattttgtcgataaacgagtccgggcgggcaaagtatacatactcaaacaggcacggattgctgaccggattgtcagcacattgacgggtaaacaactgcccttcttcagtgatgtaaatcgcttcgcccggcgcgacgtcacgcaggaaatcaaagcccagcgtatcgagcgctacgctttcggaagcgaccatatattctgtacggttctcgtcaatatcacgttttcccagtaccagcggacgaatcccgtttggatcgcggaaagcaaccataccgtggccgataatcatcgccacacaggcatacgcgccgcggattaagcggtttgtggcagcaatggcagcgaaaatattgtcggcttccagcgggtagtggcggaagttgtccagctcgctggcgaagatattaagcagaatttccgagtcggaagtggtgttgatgtggcggcgtttttcttcaaacagttttttacgcaactcgtgagcgttggtcagattgccgttgtgggcaagcgtaatgccatacggggagttaacgtaaaacggctgcgcttcagaggcgctggagctgccagccgtggggtaacgcacatgaccaatgcccatattgccctgcaaacgctgcatatggcgagcttcaaatacatcgctcaccagcccgttcgctttacgcaaacggaagcagttattggcatctatggtgatgatgccggcggcatcctgaccgcgatgctgaagcaccgttaaggcatcataaatcgactggttaaccggcataacaccggcgataccgacaataccgcacatacgtctttttcctcgttaagccacatctcagagcacttacgctctgggcaagaaacttgacgagctttgcagataatcaaaaaaacatctgatgataaaactgaattgcgggatcagctgtgatttgctccagtcttcgcttttcgacaccccggtaaaggagtcgagaaagaagagaatggcagcaacaatcaacacaccgcgcaacgcaccgaaacagacgcccagcacccgatcggtgcctgacaaccccgttttctccaccaactggcctatcacgaagttcacgatagcaccaacgatcagggtagcgataaacagtaccgcgatggcaatcccatttcgaaccagttcgtcttcaaagcccgtaaaccagactgacaggtaagtgtagtaatgactggcaacaaagaaagcacaaccccatgtcaccagcgataacgcttcacgaacaaagccgcggatcaggctaaccagagaggaaaaagcaatcaccgcgattatggcgtaatcaatccagaccatatgtgtcccacgattttacgccctgtcatcctgttcggggcgcattctaacagaaaaagaaaacgtttgcgtagggatttccttcccgcgcatcaataaaaatggcgctgaaaaaatattcaacgccatcgactttttatgcctttgcggcatcgggcaatgcgtgtcggatgcggcgtaaacgccttatccgacctacggttctacccctgcgtaggcctgataagacgcgccagcgtcgcatcaggcaagaccgtattaattcggcgtatagcccattaccacgccacttaagccagaaagttgcttcaactcacccagcgaacctttcagcttatctttcgaggcatccggcccaaccagaatacgggtaattttaccctgcactggcgtggatggcgacgtataaacccgataaccggcaccgcgcagcttaccgacaatctcattcactttatcggcatttttcagcgcacccagttgcacaacataggctttacccgtcggtgcagctttttcttccacgaccggcttcggttctggcttcggcgcaggtggtgcttcaacctttggtttaggcggctccaccggtttcggcttcggtggggcgaccggtgcaggttccggttcaaactcggtgttattggctgcaatagtggccggatcgagcgacggtgctgcggcatcacctgcccgcacctcttccgctgcgccttccggcggctgcgtcggtaacgcctgggtggcggctggcatcatatcaggctcatcacgatcgcccgctttcggcaccagcgggatagccgcgaactcatcctgataatgttttttctgcccgtccagcagccctggaagtacaatcacccccagcgccaccagcacgatcgtgcccactaaccgattctgaaacttacttgccaccgcttctcctcgcgtcaatcacttccatgacatgtgcgaccgtgtggaaagaaccacacaccagcacggtgtcttccgctttagcgtccgccattgcggcatcccatgcctgcgcaacgctatcaaatgatttgccgttacccaaatgctcaagcagttgttctgccgtggcaccgcgcggcccttccagtggcgcacaataccagtcatcaaccacgcttttcaaccaggccagagttccggcaatatctttatcatgtagcataccgataaccgccagcacgcgcccgtttttcggtagcgctttcatacgcccggtgagatattccgccgcatgtggattatgcgcgacatcaaaaataacgcgtggcgactcgctcacaatctggaaacgtcccggcaaaattgcgctggcaatcccgtcgcgaatggcattttcactgacttccagcccgctggcacgcagtgccgccagcgctgttgcggcattcggttgcgggacaagcggcaacggcagattttccagcgtgccgtgagcatcgctaaacgcccagtcatgatcggtgacggaatagttccactcaacgccccgacgttgtaacagtgcacctttttcctgcgccacatcagcaatggtagaaggcatttccggctcaccgacaattgccggtttttcgctgcggaagatgcctgctttctcgcgaccaatactttcgcgatctggacccagccagtcggtatgatccagcgcaatactggttactaccgcgacatcggcgtcgacaatattggttgcgtccagacgaccgcccagccctacttccagaatcaccacgtcaagttgtgcctgcttgaacagccacaacgccgacagcgtaccgtactcgaaataggtcagggaaatatcaccgcgtgccgattcaatctccgcaaaagaggcggtgtgggccgattccggcaattcctggccctgcacacgtacgcgctcggtataacgcaccagatgaggcgaactgtagacgcccactttgtaccctgccgccatcagaatcgactccagcgtacggcaggtggtgcctttgccattcgtacccgcaacggtaaacacaaatggcgctggtttcaggacgccaagacgcgccgcgaccaggctcacgcgctcaaggccgagatcgatagttttactgtgcaggttttccagataagaaagccacgaagccagaggcgacgcggcttgaggagtgcgtttgataatcatggtatccgctgattcgttacggtgagaatagcaaaagggcagagccagtggccctgcccttatcagttatcaggcctcaggttcctgatccggtaccgggggtaccactacgccttcacgcggcgcttcaggattcggcgctggcagattcatcaacttcgccagaatgctcgccagtttcaggcgcatttccggacgacggacgatcatgtcgatcgcgcctttctcgatcaggaattcactgcgctggaatccaggcggcagtttttcgcgaacggtctgttcgataacacgcggaccggcaaagccgattaacgctttcggttcagcgatgttgagatcgcccagcatggcgaaacttgcagaaacaccgcccatcgtcgggtcggtcagcacggagatgtacggcaagccgcgctcctgcatttttgccagtgccgcagaggttttcgccatctgcatcagcgacatcagtgcttcctgcatacgtgcgccaccagaggcggagaagcagatcagcgggcagttatcttccagcgcctgctcaacggcacgcacgaaacgtgcacccacaacagaccccattgaaccgcccataaaggcgaactcgaatgccgcagcgacaaccggcattccatacagagtgcctttcatcaccaccagcgcatctttttcgccggtttctttctgcgcagatgccagacggtctttatacttcttggagtcacgaaacttcagcacatctttcggctcaagctcgctacccagctccacaaggcttccttcatctaacaggctatgcaggcgattacgcgctgtcatacgcatgtgatggtcacacttcggacagacctcaagattacgttccagctcagcgcggtataaaacctgaccgcagctatcacacttagtccacaccccttcaggaatgctcgccttgcgggtgggagtaatgttgcttttaattcgttcaatccagctcattagggacctttctgtctgaacctggttcgatgccagttttatctttggggacgcataatgccatttttgcccccaacagaccatgaatgttgcacattaaaacataacagcccgaaactttggataaaaaagtggtcgaaccgcggagttactttttattttgcggcgcgtgccgcagcgcgtttgtgacggattatttcgatgacgcccggcaaaatagaaaccacaataatcccgacgatcagcagcttaaggttatcctgaaccatcgggattgtaccgaagaaatagcctgcgtaggtaaaaagcagtacccacaacagtgcgccgatcacgttataagcggcgaaatgacggtacgacatgtggcccattcccgcaacaaacggggcgaacgttctgacgatcggcacaaaacgggcgagaataatcgttttgccgccatgtttctcataaaactgatgggttttgtcgagataactgcgacggaaaattttcgaattgggattactgaacaacttttcaccgaacaaccgcccgatagtgtaattgaccgcgtcacccacaatcgcggcgatcagcatcagcaccaccatcatatggacgttgagatcgttggtttccagtgatgccaacgctccggcaacaaacagcaatgaatcacccggtaaaaacggcgttaccaccagaccggtttcacagaacaaaattaagaacaaaatggcataaacccagacgccgtactccgcgaccagctctgccagatgcacgtcaatgtgcaggataaaatcgatgaggaaataaatcaggtccatatttgcctatgccttgtactcgtcatctttcaggctgtaactacgttggctacagcctgaaatgttccgagcattattctcgttagtccgccagaaatagcgggcccattggcggttttggaagatcataccggtcagggtaatccaccgcgaccagatacagcccttccgcttttgccgttgctgccgccagcgttctgtcctttgccgccagcaactctgctatccagctctccggctggttgtgggcaccgacttccatcaggctgccgacaatattcctgaccatatgatgtacaaaagcattcgctttaatatctaccaccacataaggaccgtgacgcgtgacattaatatgcataacgttgcgccacggggttcgggactggcactgcaccgcacggaacgaggtgaaatcattctcgcccagcaagcattgcgcagcccgatgcatccgttcagcgtccagcggttcgtaaaaatgggttacccctttactcagtaccgccgggcgcagccgatgattgtagatgatgtagcgataacggcgagccgtggcgctaaatcgggcatgaaaatcatcaggtacagttttaacccaacgcacagcgatgtcaccaggtaaattcgcatttacgcccaaggtccacgccgcgtctttgcgcagcgcggttgtttcgaaatgcacaacctgcccggtaccgtgtacccctgcgtcagtacgcccggcgcagaagacggtgatgggttcgttcgccacctgggagagcgccttttccagcttctcctgcacactgcggacttcgttctgccgttgccagccgtaatacttactgccgtcgtactcaatgcccagcgcaattttataaactggcggttgttgctggtcggacattagtacagatactcctgcaccagtttctcggcgatttttactgccatcagcgcgccgccaaagcgaacgttatcggccaccgaccagaactggacttgctccggcataccgtagtcattacgcacgcagccaacagaaagatgcggcgtacccgaagcatcacctacctgagttgggaattcgttctcttcagagagcacaatatcttcgccttgaacaaacgcatcacgcgcttcttctgctgccagtggacgcagagcttcaaagttgaccatctgggcatgaccgtagaataccggtgcctggacgacgctagccgaaatcatcagcccttcgtcctgcaggattttgcgtacttcgtcaacgatacgacgttcttcacgcacgctaccttcgctatccggcagtaacggcagcatgttgaacgccagctgacgcccgaagaaatcttcttcgtcaatcggaatgccgttgagcaatttcgcactctgccccgctaacgcatcgaccgcttttttgccctgggcggaggctgaaatcaggctggtaacgctgatacgtgataaaccgccctgatcgattaacggtttcagtgccgccagcagctggctggtcagactgtctggtacggcgatgacattccggttccggtaatctgtcagtacaaacgggtttacttccggcaccaccagcggtacgtcgggttcgagagcaaacaatccactgctgtcgatcaccaggcaacctgagttggtcgcttcttcaacccaggcagcggtagcttctttgcctgcgacaaaaaatgccagctgcgcctgcgtccagtcgaattcagcggcatcctgcacggtgattgtcttaccaccaaagcgcagttgttcgcctgcgctttcgttacgtgccagtgcataaatttccccaaccgggaactgacgttcagccagcgtttcaagcagggcttcgcccacagcgccagttgcgcccaggacggcaatgttccagccttcagacatggtggtttactccagaaatagcaaagctccctgccaatgttacagcagagagcatgaagaagagattaacgtgccggatgatgaacggcgttaaaacccagtttacacagcaatgatgccgcactggcgtcatcacaaattacatacagagatgaccattcacggcgctcaagatagtttttgcgcagtttatcgaactcacccggtatcccggcgactttacgcagcggtgcgtcatcgcggcgcacatcatacaccaaatgcaccagccttttcagcgtcggttgatcgagcgggccatgcagcgtaatgcgaccaaactctggcgcaggcagtaatgtatccagcgcaacgtgctgttcatgcccaataaacttgctataagcttcaaacacttgcgtagtaccgcgtgctttaccttccagggtatagcctgcgatatgcgacgtgccgatatccacttttttcagcagctcgacgttgagttccggttcgccttcccagacatccagcactacgcttaacttctggccttcattcaggcaggtcagcaacgcagtattatcgacgactgcgccacggcaggcgttaatcagaatcgctccgggcttcaggctacggatcagtttttcatccgccagatgtagcgttttgtacggaccatctttaaagagtggcgtatggaaagtcagaatatccgcgcgctggactaactcatccagcgagcggaaatcaccctcatccccacggtcggcgcgaggcggatcgcaaagtaaggttttaatccctaacgcttccagtcgcgcctgcaatcgacgtccaacgttaccaacgcccacgatccccaccgtacggtcgtacagtgaaaatccatcgcgttcggcaagcatcagcagggaggagaaaacatattccaccaccgcaatcgcattacagccaggtgcagcggaaaaaccaattcccgcctgcttcaaccatgcttcatcgacatggtcggtccccgcagtggcagtgccaacaaatttaatgggttttcctgccagcaaagattcattcactttcgtgaccgaacgcaccatcagcgcatccgcgtctgccagttgagcgacggggattggacgcccgggaaccgcggtcacctcacccaaacggctaaataagtcgcgggcataaggcatattttcatcaacaaggattttcacgtttgtgttacctgtatgagacgagagttaaccggacaagtgtgccataatctcgcggccaggcatacttgcgaagatttcaggtataaggatacgtaatgatacaacctatttccggccctcctcctgggcaaccaccaggtcagggagataatctgccgtctggcacgggcaatcagcctttatccagtcagcaacgtacttcgctggaaagcttaatgacgaaagtgacctcactgacgcaacagcaaagagcagaactgtgggcgggtatcaggcacgatattggtctgtcgggagattcaccgctgctttcgcgtcacttccctgccgctgagcataatctggcgcaacgtctgctggccgcgcaaaaaagccattctgcccgccagcttttagcgcaattaggggagtatttacgtctggggaataatcgtcaggcggtcacggattatatccgtcataactttggtcagacgccgctgaatcagctctcaccggagcaattaaaaaccattctcaccctgttgcaggaagggaagatggttattccgcaaccacagcagcgcgaggcgaccgaccgtcctttattaccggcggagcacaatgcgctaaaacagctggtgaccaaacttgcggcggcaacgggggaacccagcaaacagatctggcaatcgatgctggaactttccggggtgaaagatggcgagttaattccagcgaaactgtttaaccatctggtgacctggctacaggcgcgtcagacgctaagccagcaaaatacgccgacgctggaatcactacagatgacgctaaaacaacctttagatgccagtgaactggcggcgttatcggcatatatccagcaaaaatatggtctttctgcgcaatcatcgctttcttctgcccaggccgaggatattcttaatcagctttatcaacggcgggttaaagggattgatccgcgtgttatgcaaccgctgcttaatccttttccaccgatgatggacacgttgcaaaatatggcaacgcgtcccgcgctgtggatactgttagtcgcgattatcctgatgctggtctggctggttcgttaaccccgacgaaatgacagtatcgtgacaataatacccagcaccgcagagatcgccccggcaagaaataccgaagagtaaccaaacgtggtcgccagcattcccgccagcggcccggagacgccgagggcgatatcctgaaacgcggcgtaaccgcccagtgcggtgccgcgaacttgtgaggggacgcgtttaaccacctccacgcccagcgcaggaaagataagcgaacatccggctccggttaacgccgcgcccgctaatgcgacccatgcacctggggcttgccagagcagcaacaagcccaccgtttctacaagcagagagacaatcgccactttcacgccgccaaaacggtccggcatccagccaaacatgacgcgcatcacgacaaatgcgccgccaaacgcggtaagagtaaagcccgccatcgcccatcctttgctggcaaagtagagcgaaacgaaagtcccgataacagcaaaaccaacgccttgtagtgccagacctaaccctggtttccagataagcccgacaacgctccacagcgatggacgttctcccgccagggccggtactttgcgcactgtgccgttacaggcccacgccagtacgggtaataccattgtggtgatcgccagtgcggcaaaaccgtaatggctatgaatcaacaggccaagcggagcaccaacagcgagggcaccgtaaatcgccattccgttccatgacatcactttgccagagtgttttggccctacgatgcctagtccccaggtcagagcgcctgtcagtaactggctttcaccaaagccaagaatcaaacgcccgacgaccaacagagcaaatttgaacggtgcggagacaggcaaaatcgccgccagcagcaacgcgccgccagccagaccacaagctaacattccctgaagcgccgaacgttttgcaccatattgatcggccagtcgcccggcgtaaccacgcgtcagcaccgtagccagaaactgaatcccgacggcaatgccgaccatggtattgccatagcccagttcatgatgaacaaacagcgggataaccggcaacggcaaccctacggtcatgtaggtgagaaaaaccgcaaaagcgatgcggaagagcgaaaaattggcagaagatcgtgtttcggtttggcttacagcagtcatgcattactccagaatgcagcgcaaggcgaggagtatccccgtctcatctctctggtttcagggttacggtgcgttggcaggatttaacgcgtacgtcttttcagaaggaaatcgacaaagcgggaagtttgcctggaactggcggcgattgtcaatgatgtgaaaaagggaaccatcaggttcccttttgcgttagtgccggaggccgcattggcgcgtaacgtcggatgcgacgctggcgcgtctactccgacctactgcgaattaatctttcagcttgcgcattaccagcgtggcgttggtgccgccgaagccgaagctgttagacataacggtggtcagttcgcgatcggtcgtttcggtcacgatgttcagacccgcagcctgctcgtccagctcttcaatgttgatgctcggggcgataaagccgtgttccagcatcagcagagagtagatagcttcctgtacgccagcagcgcccagagagtgaccggtcatggctttggttgcagaaatcgccgggctcttatcgccgaacacttcacggatagctgccagctctttcacgtcgccaaccggagtcgaagtaccgtgggagttcaggtaatcgattggggtatcaacgccatgcatcgccatcttcatgcagcgtactgcgccttcgccagacggagcaaccatgtctgcaccatcagaggttgcgccgtagccaacgatttcagcatagatgtgagcaccacgcgccagcgcgtgttccagctcttcaaccactaccataccgccgccgccagcgataacgaaaccgtcacggtgagcgtcgtaagtacgggaggctttttccggggtgtcgttgtatttagtagacagcgcacccattgcgtcgaattcgcaagccatttcccagcacagctcttcgccgccgccagcaaacacgatgtcctgtttgcccagttggatctgctctactgcgttaccgatacagtgtgcggaagtcgcacacgcggagctgatggagtagttaacgccatgaattttaaacggggtggcgaggcaggcagaaacgccggatgccatcgctttggtgaccacatacgggccaaccgctttcaggccgcgcgggccgcgcattgcgtcagcgccgaacacctggaaacgcggggagccgccgccggaacctgcaatcaggccaacgcgcgggttattctggtaagcttccggagagaggcccgcatcagcgattgcctgctccatagaaaggaatgcataaatggatgcgtcgctcataaagcgcacaactttgcggtcaatgaggccagtggtatccagttttacgttgccccagacgtggctacgcatgccggaatccttcagctcctgagagaaagtgatccctgaacgtccttcacgcagagatgccaggacttcctgctggttattaccgatgctggaaacaatgcccaggccagtaatcactgcacgtttcattcaatacctctgtaagtcgcacatagagtaagtttcgaatgcacaatagcgtacacttgtacgccgaacaagtccgatcagccatttaatagagaaatttgcgcagccttacacacatcgctaagatcgagccaccgcctgtaagacgagtaacttacgtgaaacactactccatacaacctgccaacctcgaatttaatgctgagggtacacctgtttcccgagattttgacgatgtctatttttccaacgataacgggctggaagagacgcgttatgtttttctgggaggcaaccaattagaggtacgctttcctgagcatccacatcctctgtttgtggtagcagagagcggcttcggcaccggattaaacttcctgacgctatggcaggcatttgatcagtttcgcgaagcgcatccgcaagcgcaattacaacgcttacatttcattagttttgagaaatttcccctcacccgtgcggatttagccttagcgcatcaacactggccggaactggctccgtgggcagaacaacttcaggcgcagtggccaatgcccttgcccggttgccatcgtttattgctcgatgaaggccgcgtgacgctggatttatggtttggcgatattaacgaactgaccagccaactggacgattcgctaaatcaaaaagtagatgcctggtttctggacggctttgcgccagcgaaaaacccggatatgtggacgcaaaatctgtttaacgccatggcaaggttggcgcgtccgggcggcacgctggcgacatttacgtctgccggttttgtccgccgcggtttgcaggacgccggattcacgatgcaaaaacgtaagggctttgggcgcaaacgggaaatgctttgcggggtgatggaacagacattaccgctcccctgctccgcgccgtggtttaaccgcacgggcagcagcaaacgggaagcggcgattatcggcggtggtattgccagcgcgttgttgtcgctggcgctattacggcgcggctggcaggtaacgctttattgcgcggatgaggcccccgcactgggtgcttccggcaatcgccagggggcgctgtatccgttattaagcaaacacgatgaggcgctaaaccgctttttctctaatgcgtttacttttgctcgtcggttttacgaccaattacccgttaaatttgatcatgactggtgcggcgtcacgcagttaggctgggatgagaaaagccagcataaaatcgcacagatgttgtcaatggatttacccgcagaactggctgtagccgttgaggcaaatgcggttgaacaaattacgggcgttgcgacaaattgcagcggcattacttatccgcaaggtggttggctgtgcccagcagaactgacccgtaatgtgctggaactggcgcaacagcagggtttgcagatttattatcaatatcagttacagaatttatcccgtaaggatgactgttggttgttgaattttgcaggagatcagcaagcaacacacagcgtagtggtactggcgaacgggcatcaaatcagccgattcagccaaacgtcgactctcccggtgtattcggttgccgggcaggtcagccatattccgacaacgccggaattggcagagctgaagcaggtgctgtgctatgacggttatctcacgccacaaaatccggcgaatcaacatcattgtattggtgccagttatcatcgcggcagcgaagatacggcgtacagtgaggacgatcagcagcagaatcgccagcggttgattgattgtttcccgcaggcacagtgggcaaaagaggttgatgtcagtgataaagaggcgcgctgcggtgtgcgttgtgccacccgcgatcatctgccaatggtaggcaatgttcccgattatgaggcaacactcgtggaatatgcgtcgttggcggagcagaaagatgaggcggtaagcgcgccggtttttgacgatctctttatgtttgcggctttaggttctcgcggtttgtgttctgccccgctgtgtgccgagattctggcggcgcagatgagcgacgaaccgattccgatggatgccagtacgctggcggcgttaaacccgaatcggttatgggtgcggaaattgttgaagggtaaagcggttaaggcggggtaatctgctctcgcagtgtttgccggatgcggcgtgaacgccttatccgacctacgtgtgacgtgtaggcctgataagacgcgataagcgtcgcatcaggcatgctgctccagacgccgcaacttactgctgtgacgcctgctgaaacaggttttcccacatatcggtcaccagcgcctggtcacgcggcgacaattcaccagcaccaatggctttttccagactctggctaacggtcgtatgcaccgcctgagcggagtggtcatcaccactttccagttctgcgatggctaatgtcaggtggccacgcaaatacccactggcaaacaactcatcatcactggcatggtcaaccataccgtcgattaatgccagaatgcgtgattcaaactccgcgatcatcttctttcctcattgtaaaacgtggcgctggcttcagttgagcgcttccggccacgggaactgttccgccgtaagttccggcgtgtgataataattttgtagtgctttaatgaagcgtgccggacgttccggaatgccatttgtcagataatccatcacctgcgcatgtactcgccgttgaaacaccacacgatccggttcgaaatccccttccagattgtcgcaactgacgttaaacggatatcccgccgccacacagaacaaccagtcgagcgcctgcggcttcacttcaacatcttcaaactggctttgcgtttgggcatcgcgtccgtccgggcaataccagtagccgaaatcaaccagctcacggcgcgctttcccggcaatacaccagtgcgaaatctcatgaattgcgctggcataaaagccatgagcaaagacgattcggttatacggtacttccgcatcagcaggaagatagatcggttcgtcgtcgcctttaatcagacgggtattaaaatcatcggcaaagcagctattaaaaatttcaatcaactgctcgtagtggtgtgtactgttcattagttcatccccaaccagtggaggatctcctgtccgtggctgtcgtaaagtaatttggcactcatcaccgccgagacgataacaatcatcgggcggatcagcttttgtcctttgctcaacaccagtcgtgaacccatgcgcgcgccgaggaactgccccaccagcatgacaaagcccgtcgcccaaatcactttgccgccgagaataaacagcagtaaaccgccgatgtttgacgttgcgttgagtaatttggcgtgagccgtggctttggcgaggttaaatccgcacagcgtaacgaaggccagcgcgtaaaacgacccggcagccgggccaaagaatccatcataaaaaccgacgcagccaccggctattaacgcgaagggtaaaccgtacatccggcgctggcggtcttcttcacctagctttggcatcagcaagaaatagaggccgatacaaattaccagaatgggcaaaatctgccgtaagacatcagcctgaacgtattgcaccagcagtgcgccgctcattgagccgacaaaggtcatggcgatattgagtttctgatcgcttaaactaaccactttgcggcgaataaagtagatagtagcggaaatagagccgccgcaggcttgcagtttattggttgccagcgcattagcgggagacatccccgctgccatcaatgccggaatggtgagtaacccaccgccaccggcaatcgagtcgataaatcccgccagcatggcgacaaaaaagagaactcccagcaacagcggggaaaccataaacaggctattaaacgtttccattagatcacgtgctcatccagtagcgcctggcaggaaggcggcaacggaggcggtgtcttcttctcaggctttgttgttcccggttttggaggttcaaaccagctttgcagttctgccccgcaaccatcgcctgatggcggtaaaggttgatcttcacactccagactatcggcagggcaacgtaatcgtacatgcatatgcgcgcgatgctggaaccagggtcgcactttgcgcaaccagtcgcgatcggtgcccgcatcaaggcaaagttgttgtttaatcgccggattaacaaaaatgcgcgtgacgtctttgtcctgggcggcgagtttgatcaagctgaaaatttctggcttccacagcgtggagacaacgtgtttaccgtcgcgggaaactaagtccagtgcttgcgggcgcaagagctgcgcggaggtccagcgagttttcggcagttgcagaaagatatcgacatccagtccggtctggtggctggcatgaccgccgttgaaacgcccaccagcgggcatccccatatcgccaatcagcaccgtacccatgcccagattgctcacctggctactcagacgctggataaacatcaccagatccgggtgaccgaaatagcgacgctgatcggtacgcatgacctgataatgttcggactgtatcggcagcgtgtcagcgccgacaatacagccattagaaaaactgcctatcgattgtgcgctacccggcacaggttgggttattttttgccacggcgtcgctgccaggctggcgctactggcaagcagagccagcagcgcaatcgcggttttattcattttttaccagcgtggaatatcagtcttcacatcggcattttgcgcccgttgccgtaacaggtgatccattaaaacgatcgccagcatcgcttctgcgatcggcactgcgcggatcccgacacagggatcgtgacggcctttggtgatcatctcaacttcttcgccaaagcggttaatggtacgacccggcacggtaatgctggaggtcggtttcagcgccatatgggcaatgatttgctgcccgctgctgataccgccgagaatgccgcccgcatggttgctctggaaaccgtctttggtgatttcatcgcggttctggctgccgcgcagcgccaccacgtcaaagccgtcgccaatttccacgcctttcaccgcgttgatgctcatcagcgcatgggcgatgtcagcatccaggcggtcaaagaccggctcgccaagtccggcaggaacgccactggcaacaacggtgactttagcgccgatggagtcgccctcttttttcagcgcacgcatcaactcgtctaacgcgtcgattttgtcggggtccgggcaaaaaaacggattttgctcgacctgcgaccagtctttgatatccagcggaatgtcgcccatctgggtcaggcagccacggatttcaataccaaatttctcggcgagatattttttggcaatagctcctgccgccacgcgcatggcggtttcgcgggcggaagaacgtccaccgccgcgataatcgcgcagaccgtatttttgttcgtaggtgtaatcggcatggcctggacggaaaacgtccttaatcgcactgtaatcctgagagcgctggtcagtgttttcgatcaacaagccaatgctggtgccggtagtaacgccttcaaaaacaccggagagaattttgacctgatccggctcgcggcgctgggtggtatagcgcgatgtcccagggcgacgacggtcgaggtcatgttgcaggtccgcttccgtcagcggaatgcctggcggaacaccatcgacgatgcagccgagcgccagcccgtgcgattcgccgaaggtggttacgcgaaagagttgtccaattgtgtttccagccatcacggctccgttattgttgtgtttgcgtgtttacttaatctttataaatcgcgaaatgttctcgtgcggcaataagctgctctttggtgagcataaacacaccatcgccgccgttatcaaactccagccaggtgaacggaacatccggatattgttccataagatgtaccatgctgttgccgacttcacaaatcaacacgccatcatcagcaaggtaatctgccgcgttaccgagaatgcgacgcgtcagtttcaggccgtcagtgccagatgccaggcccagttccggctcgtggcggtattcgtttggcaggtcggacatatcttccgcatcgacatacggcgggttagtgacaatcaggtcgtactgcactttcggcaagtcgcggaacagatcggaacgaatcggaatgacgttgtggatcagaccgtgttcttcgatgttctgttcagcaaccgccagcgcgtctggagagatatccaccgcgtcgacttctgcatccgggaaggcataagcacaggcaatggcgatgcagccgctaccagtacacatatctaaaatatgctgcggttgcttgctgataagtccggcaaatttattgttgatcagttcaccaatcggcgagcgcggcaccagcacgcgttcatcgacgtaaaattcatggccgcagaaccacgctttgttggtcaggtaagccaccggaatgcgttcattgacgcggcggatcacgcgttcaacaatacggtgtttttcgctggaggtcagacgcgcggtgcgcatatcttccggaatatccagcggcaggtagagcgaaggcaacaccagctgtacggcttcatcccacgggttatcggtaccgtgaccgtaccagatatttgccgcgctgaagcggctcaccgaccagcgcaacatgtcctgaatggtttgcagctcatttactgcttcatcaacgaaaattttatccacgtattcctccagggcatgatcgcaataatttcggcggctagtttgccatgaagatgacgataaatcagcattcacgcgcggtgagtgaggaaaaatacgtttaaaacgatcgattgcgctacgagtcgggtaaactgtaggaaaattagaaatagagacagataaatgaaaaagaaaacaacacttagcgaggaggaccaggctctgtttcgccagttgatggcggggactcgcaagattaagcaggacacgattgtccaccgaccgcagcgtaaaaaaatcagcgaagtgccggtgaaacgcttgatccaggagcaggctgatgccagccattatttctccgatgagtttcagccgttattaaataccgaaggtccggtgaaatatgttcgcccggatgtcagccattttgaggcgaagaaactgcgccgtggcgattattcgccggagttgtttttggatttacacggtctgacgcagctgcaggccaagcaggaactgggggcgttgattgccgcctgccgccgtgaacatgtgttttgcgcctgcgtgatgcatgggcacgggaagcatattttgaagcaacaaacaccgctgtggctggcacaacatccgcatgtgatggcctttcatcaggcaccaaaagagtatggcggtgatgcggcgttgttggtgttgattgaagtcgaagagtggctgccgccggagttgccctgaggagttgagcgcgttgcgccaggtacgggtaatggcaggggcgaatgcccctgcctggtgtatctaagggctacaactcattcagtatgtactggaaccggcaagtagaatcgattggctgcatactgctggtatcaacacgcacgaccatatcgtgtaactgtttgtccgttatagggtgtcgatttggcgtgaccgagacttccgccttgtcacatcccgacgcggtaaaagttatcatctgtgcaacccagcggcagtaaccacctgtttcattcatctgcgtactgtcgcacaacttcccatctttcatcaaatacgttgaaagcgttttctcaaccacaccgcccgtcgactgcagggtgagcagttttgacttactgacataattctcattccatgaaacgtcataaggttgaacagaaacggatggacaaatcgtgtcgtgactatcaggcccctgatacgtcacgccccctggagaggcttcagagtcattcataataaccaaccatggacaagaaaagtaagattcaatctctgcagagacaataacctcaaatgtataatacccgcagttccacccagacggtaatccaggacaacttgctttgttgatattttgatggtagccaatcagcttaaccgaaggggcaggaggaggaccactccagctcacattttgcaatatttccccagtcatgagccattgactacttttatattcaccaacgtacactgcggatggcatcattatttttaaattaaaagtcgcaatattacgcgaatcaccgttgtaaccgtagtaaacgtcaacgctatgcccggcagccatagcttctgtagtagcaataagcatgaccagagcgaacaaccatcgtagtattttcattttaaatatactcaaatgtcgcagttaaagaggcggtaaattcaccgatcgtcacatcacggccgcttttcgcctgtagccaggctctgaaattgatatcgttattgccattggttagcgcaaaggtcgccccatttgtattgttgatggcaacctgcattccgtcggttttttccatgccaattcccactccctgagcggttgatgacgtatccagtgccagaaaaccgggttgttcgctgtcttctacccccgtgagcgtgacttttacgttgtatcccgccggccctttgcaatctttcagcttaaagactacgggtacacgagcggactggcctgcaacgttcaaatcctgacgactgaccgtgggaaagcgcacctctgccagatattggccatccaccaccagcgcacaggatttacttaataaattaccggagaaatgcagattattatctgccgcgaataacgtgctactcattgccaatatcagccccgctaacaggacgtaaccaccggactgaatcattgatttattcattgataatccacccgtaatgttgcgtaagccgaaaaattcgtatcgcttaacacagcatcactcgcttttaccggtacggcctccagcttcggcttttgcgtaaaatcagtggcgttgatagcaagcggagtattgagtttaaaacgctgaccatcgtgctgaagctcgataccaaaaccgggtacatcagtttcaattgctgcatcattaaaactggtttgtgtaccagtccaggtgagggtcatctcccaatctggatgacgggtcgtcgagtcacaagtgagttcatatggcacctctttacgaccatagttgccgttgatgtcgtcgataatgagatcgcgaaattcgacttcaatggttttaccaccgctgatgctacaggttggcggtgacaataatgtcccgtgaaaggtgatgtcttcatcagcagcatgagctatggcgctactgacacaaagcagggttaagaaagtctttctcattgatagtccaccaccatggtcaaactggcgttaaactcgcccgcagcaagttgcgccccgcttgccttcacaggtacagccttcaactgtggctggttattgatattaaatggcgtccagctattttcaccgacggcaaacaatgagttatcggcgctattttctatccgaatgcccagcccggtgatattggtactgagtaccgtttcgccgttaatcgttgaggtattgcccttaagttgcatccgcaagtcgttagcaagactgtttgtgcagttcaacgtgtatttcgcatcttgccgataattggtgccatcaacgttatcagcaatcatattgccgaactctacctggctgcccttgattgaacagggtggcggagcatcgaccaacacgcgcagaattaaatccacgggtttactaccagccatagcagataaactacagacactgcataccagcagccctgcgcccactacaaacttttgactcataactccccccgtcatcagcctttgcggctctgctcttcatccacctggcagctgttgccattgcactggaagaacagcggcatccgtgcgccaaagtcgttgacgtaagtcagcaccggtacgctatccattttcacattcagcggtaccgtggttttcggctcaatgaccagaggcgagaaccctgcagctggattaccgtttttctgcgcactggcgttgctgataatcacgtagtacggcgttgggttattgacggtaaatgcctgaccgctgcgggtgagcgtcaccttgtgctgccacggacttttcatactgaccttttccagcgcctttggtcgccagaacaacttgatacgcgtttgcagcgcgatttgcagggtattgggtttgtttgattttggcgggatctcgcgcacgttaaagtagaacatgctttcacgatcggctggcaatttgttgatatccggcattccctgcacttttacctgcccgttcatcattgaatcgatgcgttgcactggcggcagcacagttaacggcgaggtgatcttgttacccttttcatcttcaatccagctttgagccagataagggagtttcggatcgttattacgcagcgtcacgctgattgatttgtcgctttcattaaatatcaaacgggtacgatctggcgttacagacgccagggcagacaaactggtagcgctaagcagtaacgccagcgtcatagcacccaatttggcagagcaaagtaaatcagacatggatcattccttaatcacgttattggttagctgaaacagaaacagggggatcggtgggtgtcacctgttgcgtctgctcctgaatgacaggctttatgtcatcaggaacaaccggcgcgacgttgcctttatgctggcatggcagtaacaagccgttaaacagatcggcaggcagcgggtccggcaggttgatatcgcaatgcgcaacaccactccagaacacactcatatgttcgccaggtttcaccccagccagatagacactaccgtcatcatcgacaaggcccactgtctgctcgttatcattttttacttctgcgccaaacggtggatggctgccatcttgtaaacgcagcaccgccatcgctttttgaccactgatgacggcaaatttgcggtagccaatggctccttcagttagcgtggcttgcaccaccgactgggttgcttcggcgttttccggcaatttgttgaggtcgatatacgcctgattgcgataataattgttaacgtcagaaacgacggctttaccaaacatattggtataaacagcagccccgttaccttccaccggaacatcggcaacgccatcggcatcaatcagcaggcgtgtcccgcccatattctgggtacggtgaagtgcgccgccgtgggtagtaagcgttgcgccgccctgtaacgacaagcccgcagaggtgtattgcccttcatggtagttcgcactgaggtcaacctgcgccagcgaaccatcatggctgtagtagccatcaacgctggtgtgtttgtcactggtgccgatgttcaactgatagtgagtcgcgtcatcgacacggctaaaataaccgacctggctgctgtccgtcccactgccatagttgccgttatagctaacggtactgttgtcgccccacggcatactgagcgaaatctacatgcccttatccgcccggttgtcatactcgtagcggtagccagtcagggaaacgctcatattacgaatgctgcccatattgaaatagtgggagagcatgatgttgtagtttgtctgctcctcacgatcccagtaggtatggcgggtatagttgagataaaccgaaacacccgcatcgcggaagttctggttataagtggcggtgtacatctctttgtcgttgcccgtacggaccatttcgctgtcactggcatccagatactcgctcatggtcataaagttctcttccgagaagcgatatccagcgaaagtgacgcggctgttgagctggtcaaagtctttggaataactcacacggaaggagttaccgtccagcgaacctttgccataagcggtgtctttatccagtttggtatgcgaatgagtaacatcaaacgcgaccgcgccgaaggtagacaaatcgcgaccgacgcccagcgccgcagactgatagttttcatcacccagcgcaccgccatataacgaccagccgttagcgatgccccaggaggcttcagcaccagagaaaaatcccccctcgacatggtggccccactcttgcggacgtcccatcatgatcttatagcgaacctggcctgggcgagtgaggtatggcatcgaggcggtgctgatgtcatattcctgcacctggccgttctgttcttcaatgcgaatatgcaacgtaccggagacggaatcaccaagatcctgaatacgaaacggtccagccggaacctgcgtttcgtaaatcacacgccccatctggctgacggtcacttttgctgtggtgtgtgccacgccggaaatgtctggcgcgtagccgcgcagattgggaggcaacatttgatcgtcagtgctgacactgccaccaacataattaaaaccgtcgaaaatatcggaattgaggtaatcttcgcccagcgccagtttggcttttaatgacggtaacgcccgccaggcataatagcgactccactcccattttttttgtgtgtcatcgccgccaaattcatcgtcatcatcattactgcgcgtatgttgatagttggtctgccagtcagcgcgcatacgccatggccccaggttaaccccgaccgtcccgttgccgctgatctcgttactgtcatcgccgccattttcttcgtgtcgtgtttgcgcagtgatgctgtagtccgcaatgatcccggagatgccatcatcccaacgagaaggtggatcccagtcgggccaggtatattcgaggtaagcctgcggtagtgaaatgactaatgcggactggcttaaatcagccttaatttccacgccttccagttgaccgggcttcaggcatttaccatcgtggctccattgcagatttttcgccacgtcttcttttaaaccaaactgcgccaccagttccggtgtcagacaagcatagcttttgctaacgtcatcttcaccagcataccagtaaatatcgtactcttccgccaatggctgtttatttagttgaacctgtaaattgtattttccgggctcaacatacccctggctggaaaaacgcttcagatcaatttttgtgtcgccttttaattccagaaaacgggaatcaaactgaatgtcgtcttcagcccagacactgctataactccctgacattgccagcgcaatgcaccacggaagaatccgtaatcgaaaaagagaatggtcaggcatacacgtttttatccgtttttattcttgttcggtcaaaatccatttaaataccccatagcagtgtcgctatgggggtatgccttacaggtaagtaatctggaaggtggtatttgcttcgaaattacccagatctggcgcatcagctgcgccgaccagccaggctttaaagttcagagtctgcttcgctttgcctttattagtggcagtatctttcacgattttctggtcaatacccatgccgcttttgtaagaggtacccagagagtcaccgatcgccaggctaacattgttaaatgccgcaccggtatcggtattgaaaatggtgtaataattgccgctatttgcagaagaaacggtaccagtaaaggtagtggtcattgtttcctgagtatcaaatacgcaatcttgcaggcgaatctggaaatttttcggcgtggtggtgccgttatttttcagtttttcggcaccgatatcacccatatcaacttccagtttgtgatcgtccggaacgatagaacacactgagtcttcaatggtgccgtaaaaacgtgcagtaccgttgttacccgcagcgattgttgccgtagaggtgaacgcgcccatcaccattgccgcagcaatagctgttttaacaaacttactcattatttgtccttaaactataaataattaaaatataaacattgcaatacattgattcagtcaatagccaatgtttatacccagccattgaatacggcatgcgatccaaaaaaacaggtcgtaaaaaatgtattcgttggtgtggggtcgaatagtgatgttttcactcccctgattcaatttaattttactaatgagtaaatgtagatttaattaatatattgataggggaaagattatcttaaggatcttctaaaaaaacacgaaatatatatttagaaaaaacaggaagcatatcaacaatgaatgccaatagcttaaaaaacaaacaatgaacatataatgcgattggcattaacccgcttttgtcgatataatatataaacactatagccagaatttaatcaagtttcaattacgtcctgcctgattattcaactctattttctccattatctgtattaataaatgataatgagtgtcaaacagacattattcatttcaacatgtaactttgggcaaaatcaagatacgcgcagaagaatactttccgaatgaaagttaaaggtgttttatttatagatggggagagtcttcgatagtagtgaggttgacagatatccgctgcctgatgagcaattatgcccaatgaatctacctcattgggcataatttggaactcatcagatagcttttgccatcttcagattacacgggctcatctgccagttgaatgtgccgtttccgctttcatcaagcgttacgctggcaatggccgaggtggtaaacataggcggcgtttcgcccggacataactcggcaaccagatacccgactaacggtaagtgagagatcaccagtaccgaagcaacaccttcattggtcaacgcctgcaaataggcactgaccagaccaacatcgccgcagggcgttaactccggcagaacttctgcactggaaggcaggttcagacaatcccctacttcttccagtgtttgctcggctcgcaggaacgggctcaccagaacgcgttcgatttccactttttgacctttcagccagttcgccatcaggcgagattcgtcacaaccattagtggtcagaggacgaacggaatcactggcggcatcgagggctgcgtcgccgtgacgcatgataaaaacttgcatattgcaccgcttttgttaaccagattcgcccgttttctttcatctgaaaccagagaaagaaaacggtggccggcattgtgccttatccattcaccgaatgaaacgctgttttttacctcaatggcgtaagtatagtcaatatgcgtttacattttgaccaacactccgccattcagcgcggattcatatagctttgaccttcttattgcaggtcagttgcagttgttttccaaaaactttccccacgcgcgcccatctcgaccaaacgctcgcaaggggtaaaacgggaaccatactgcgtggcaagtcgttgcattattgcaaccacttcgcccgcgccgagagaatcgatatagcggaacggtccaccgagaaatggcggaaaaccaatgccaaataccgcgccaatatccccgtcacgcacgctacggataacctgctcatcaacacaacgtactgcttcattcagcatcaacatcacacaccgttcagcaacctgcggtgcggagattcgcccctgcccttgtgtgccaatcagcgggtaaatggcgggatcgacctgttttttgcttttacgccctttctgaccataaagatagaaaccccggccattttttctgcctttgcgatcgtcgttcaaaattgaagaaacaacatttgcaggcgcgctaaaacgttctccataagcggcttccagtacaggaataattttagtcccggtgtcgattcctacctcatccaaaagttggattgggcctaccggaaaaccaaatttcactagcgcggcatcaatgtgctctacccgttcaccttgggtcaacatgcggatagcttcattaatgtaaggcgctaagatgcgattgacgtaaaaaccggctttgtcacgcacgacaattggcgttttaccctgttttttcgccagttttactgtggtagcgatggtttgcgccgatgtccccgcatgaggaataatctccaccagcggcattttttccaccggactgaagaaatgcaggccgataacttgctcaggtcgcgtggcgtgagcggcgatatcaccaatcggtaaagatgacgtattcgaagcaaagatggtatgagcggcgcaattttgctcaacttccgccaccatctgttgtttcaattcgagattttcaaacaccgcttcaataatcagatcgcgatgggcaaagccgcgatagtccgtcgttccggagattaatgccagctgtttgtcacgttcgctggctttgagatgacgacggcgaactttgccctccagctgatcccaactgtacttcagcgcatgatttatgccctgcgggttgatatctttaattctgaccggaatccccgctttacaagcagtgacataagcaataccgccgcccatcaagccaccacctaaaatccccacgctgtttaatggcgcaggcggcgcatcactgccgggatctttcttcacgtccgtactggcaaaaaagatactacgcagcgcctgcgattgtggcgtcatcgccagttcgccaaacgcccgagcttcggcgtcataaccgctgctggtgccctgcgctaatcccgtttcaacaacctccaggatgcgttctgtcgccggataattgccttgagttttgtgttctgttttcttgccgaccattttgaacagcagcgcacgacctaacggccccgccagaatacgctcgcgtacaggtagagggcgggaagatgggcgctccttctttgccagctcaacagcggcttccagcagaatggagtgcggaacaacgtcatccaccagccccagctttaatgcctgtttcgcccgaagttgttttccggtgaggatcatctctaatgctgtgctgacgcctatcagacgcggtaaacgctgggtgccgcctgaaccgggtaacaatccaagttgtacttcaggcaaaccgagcaccgttttaggatcgtcagtacaaacgcgaccgtggcacgccagcgccaactccagcccaccacccaggcaagcgccatgaatagccgcgataacctgaatgggcaaagcatgaatctccgccatcaactgttggccctgccgcgccagagcttccgcttcttgcgccgttttgcagttgccgatcatgttgatgtctgcgccagcaatgaagttgtccggtttagcggagacaaacaccacgcctcgcaactctttgttttcacggagttgcttaataatggcgcgcacctgcgaggcaaactccgccttcagggtattcattttctcacccggtacgtcgatggtgataacggcaatgttgtccagacgaacattaagggtaaacgctgatgtcatttccattattccgcctccagaaccattgccgcgccaagcccaccggcagcacaggcggtaactaaaccaaatccaccgccgcgacggcgaagttcatgcaatgtctgggtaatcatccgcgcgccggtcgccgcgaagggatgcccgtaagcaatcgaaccgccaagcacgttaaatttgctatcgtccacttcgccagtggcatgtgcacgccccagtgcttcacgagcaaaacgttcactacccagcaactgaatattcgccagcgtctgagctgcaaaggcttcgtgcatatcgatcaatgtcagatcgctcatcgtcaaaccggcacgctccagcgccagcggtgttgaccaggctggaccgagcaacatgtcctgccagacatcaatcgcagtaaatgcgtagctgcgcagataccccagcggcaccagccctaattctttcgcccgggattcagtcatcaggatcaccgctgccgcgccatcggtcagcggcgtactgtttgccgccgttaccgttccgtgtttgcgatcaaacgccgggcgcagctttgcgtaatcggcaagcgaggaattaccgcgaatattgttgtcttcgacaagcggttgtttataaggagggataaaggcagtcatcacctcttctttgagttttccgtctgaccatgcctgagcggcacgctgatgcgaacggtgcgctaatgcatcttgctgttctcgggtgatgccgtaggttttcgccatttgctctgcggtgtcgcccatccgcaagccggtagaatattctgctaccgcaggtggtacgggcattaagtcgcgcaaacgcaggcgagagaagagtttcagtcgctggctcatggtacgagctttgttgacatcaaccagcacgcgcgccagttttttactgacgccaattggcaataccgaagaggaatctgccccaccggcaatccccgctcgaatagttcccgccatcaggctttctgcgacgtttgcaactgcctggaaactggtagcgcaagcgcggctgacgctgtaagcatcggtatgtacattcattcccgtaccgagaacaatttcacgcgcaatgttgggggcttcaggcatttgtacgacctgaccaaagaccagttgttcaatcacttcggcggggatctcgctgcgtgccagcagttcgcctaccaccatcttccctaaatcaaccgcgggaatgccatgaaaagccgtcgcctgacgggcaaaaggcgtacgtaaaccgctaacaatggcgatacgatcgccctggcgggtaaccagcggtaaaacctgacccataacactcccctgtaaaaaaataaataaagtggtctgacctgatcatagtcttaaccatttttttacatttagccaagtggagaaaagggaaagtgggagctatgacacagagagaaaagaagaagagaaaagaaaacgcccctgccagcaactgacaggggcgtacgtacccgagaggaattaacgcagacccagctggaaaatcagcatttcagcttcgcaggcaaaagtgaaatcgatatccaggcgcacaccgtcagactcttcagtgaaagtcggggtgattttgcaaggttcagattccacgctacgggctttttcagtcagcgccgccagcgtttgctctgcttctgcgcggtttgcaaacacgcggctgtaagacgcggtgcagtcggagttgtccataatggtgccaacatccatacagcagcaaaccggggtttcatcagcactacatttactcatcgttgatttcctctgtatgtgcacccaaggtgccagataaacgttgtggatattttacgcttccggaaagtgctgctccagttgttaattctgcaaaatcggataagtgaccgaaatcacacttaaaaatgatctaaaacaaaattcacccgaatccatgagtgcgccacctccaaattttgccagctggatcgcgtttcttagatcatatttgaaaaaagatagaaacatacttgcaacattccagctggtccgacctatactctcgccactggtctgatttctaagatgtacctcagaccctacacttcgcgctcctgttacagcacgtaacatagtttgtataaaaataaatcattgaggttatggtcatgagccagaaaaccctgtttacaaagtctgctctcgcagtcgcagtggcacttatctccacccaggcctggtcggcaggctttcagttaaacgaattttcttcctctggcctgggccgggcttattcaggggaaggcgcaattgccgatgatgcaggtaacgtcagccgtaaccccgcattgattactatgtttgaccgcccgacattttctgcgggtgcggtttatattgacccggatgtaaatatcagcggaacgtctccatctggtcgtagcctgaaagccgataacatcgcgcctacggcatgggttccgaacatgcactttgttgcaccgattaacgaccaatttggttggggcgcttctattacctctaactatggtctggctacagagtttaacgatacttatgcaggcggctctgtcgggggtacaaccgaccttgaaaccatgaacctgaacttaagcggtgcgtatcgcttaaataatgcatggagctttggtcttggtttcaacgccgtctacgctcgcgcgaaaattgaacgtttcgcaggcgatctggggcagttggttgctggccaaattatgcaatctcctgctggccaaactcagcaagggcaagcattggcagctaccgccaacggtattgacagtaataccaaaatcgctcatctgaacggtaaccagtggggctttggctggaacgccggaatcctgtatgaactggataaaaataaccgctatgcactgacctaccgttctgaagtgaaaattgacttcaaaggtaactacagcagcgatcttaatcgtgcgtttaataactacggtttgccaattcctaccgcgacaggtggcgcaacgcaatcgggttatctgacgctgaacctgcctgaaatgtgggaagtgtcaggttataaccgtgttgatccacagtgggcgattcactatagcctggcttacaccagctggagtcagttccagcagctgaaagcgacctcaaccagtggcgacacgctgttccagaaacatgaaggctttaaagatgcttaccgcatcgcgttgggtaccacttattactacgatgataactggaccttccgtaccggtatcgcctttgatgacagcccagttcctgcacagaatcgttctatctccattccggaccaggaccgtttctggctgagtgcaggtacgacttacgcatttaataaagatgcttcagtcgacgttggtgtttcttatatgcacggtcagagcgtgaaaattaacgaaggcccataccagttcgagtctgaaggtaaagcctggctgttcggtactaactttaactacgcgttctgataacgcgttcgcctggataaagtcacctgcatagcaggtgactttaactcccccacttcaccgaaagtagtgtcctcattgcttacctcctgagttttgcaaacagcctgttggcagcttgccctttcaaatcaataagcggtatccacagacaaacctgaagggaaaggcatattttcaggcgttctgctcgtccttctcaaagagtttacttttctgcatttccaggatactccccccccctggctattgtgcgctcatacactcaaattaaagataggttctaaataaatgagcgttttttgatagtctatttcattaggtaatatatatttgtaacaaatcaatcaaaatggaataaaatcatgctaccatctatttcaatcaacaataccagcgcagcttacccagaatccatcaatgaaaataacaatgatgaagttaatggattagtacaagagttcaaaaacctttttaatggtaaggaaggaataagcacctgtattaaacatctacttgagcttataaaaaacgccatacgagtaaacgacgatccttatagatttaatattaataattcctcagttacttatattgatattgactccaatgatacagaccatattactattggtatcgacaaccaagaaccaatagaattacctgcgaactataaagacaaagaactcgtccgtactatcattaatgacaacatagttgagaagactcatgatatcaataacaaggaaatgatcttcagcgcattaaaagaaatatatgatggagatcctggttttatcttcgataagatatcacacaaactcagacatacggtaacggaatttgatgagagcgggaaaagcgaaccaacggacttatttacctggtacggtaaagataaaaaaggcgactctctcgctattgtaattaaaaataaaaacggaaatgattacttatctctcggttactacgatcaggacgactaccacattcaaagaggaattcgtattaatggtgatagtctcacccaatattgtagtgaaaacgccaggagtgcttcagcgtggtttgaaagcagtaaagctatcatggcagaatcatttgcaactggttccgatcatcaggttgtaaacgagctcaacggggaaagactgagagaaccaaacgacgtttttaaacgttatggtcgagcaataagatatgattttcaagtggacgatgcaaaatataaatgcgaccatctaaaagaaatagtttctactttagtcggtaacaaaattaacgttggccattctcaaaaaatatataagcattttaaggatctcgaaggtaaaattgaagaaaggcttcaaaatcgccaggctgaatatcaaaatgaaattaatcaaccatctgcgccaggtgttaattttgatgatatttaaaattatttttccagttttttgatttttcaacagctgaatatcggaaatagtcagtgacgaacatcagtatttttacataattacgtctaggtcattgtcggtttatctccttttacttgtggtaattgagggataacaacaaaaaaggtgagttttgcgactcaccttttttatttgtttcttattcagaatcaatatcttttaaatcatcctgaatcgcttgtgcgttcggattttcctgcggtttgagttcgccgccattagcgatgaaatcatgacgctggaagtacgcttcgcgcaccataatataaggatcggacgactgacgcagcagaccatcggaatccagcagctgagcgcgggtttcgatcccttcaagcgtccatttacccacagacatcggccaggtcagccaggaaagaaccgggtaaaaaccatccgccatatcaccaccgtcatcacgcagcgtgaagctaccgtagaacggtaactgaacgtaaggcccataacccacgccataatgaccaagcgtactaccgaagcggtgaggttcagtccgttgcagtttcgggttcgccatccctgcaacatcaataaaaccgcccatccccaaaatggtgttcaggaaaaagcgggtaaagtggaccatcccctgataagggtcgccctgcaagaagtagttaaccatcaccgcaggttcttcaaggttgccagtaaagttgctcaaaccgttacgcgccggttgcggaacataatcacgccaggcgacagcgaccggtcgaacaatatacgggtctaatacattgaagttgaagttgtacatggtgcggttgaacccttctaacgggtcagaacgcccttgctgatctgtaccggaactcgcacaccccaccagaagcgtagttcccagagcaagcgccgacaggcgaagcttcataaatgtctccctgtttttttatggcttatgcagtttgccatccatgacggaacgataccgtatccgcctgtttaggtgtgggcgattgtaacagcacgtcaactgatgtccagacgccctgatttgctgatttgatcatagcctggtaatcgccgccctgtaggctacttgattctatagaaacagaaaaaggcaaacgcagccttttctacattttcagagtaactcccgtcagttgcgagcaaaaaagccgctacgctttagctatacgtgctaattcaagagaagagaccatggacaacgacaaaattgatcaacacagcgacgaaattgaagttgagagcgaagaaaaagagcgcggcaaaaaaatagaaatagatgaagaccgactcccctcccgggcgatggcaattcatgagcatatccgccaggatggtgaaaaagagctggaacgcgacgcaatggcgctactgtggtcagccattgcggcgggtctgtcgatgggcgcttcgttactggcaaaagggatatttcaagtcgaactggaaggtgtgccgggcagcttcttgctggagaatctcggttatacctttggttttattatcgtcattatggcccgccagcaattatttaccgaaaataccgtgactgcggtactacccgtcatgcaaaaaccgacaatgagcaacgtcggcttacttatacggttatggggcgtcgtgctgctgggtaatattctcgggacaggtattgcggcgtgggcatttgaatatatgcctatcttcaatgaagaaactcgcgatgcatttgtcaaaatcggcatggatgtgatgaagaacacccccagcgagatgtttgccaacgcgatcatttccggctggctgatcgccactatggtttggatgtttcctgcagcgggtgcggcaaagattgtggtgattatattgatgacctggcttattgccctgggtgacaccacccatatcgtggtcggttctgttgaaatcctctatctggtgtttaacggtacgctgcactggagcgatttcatctggcccttcgcactacctactttagcggggaacatctgcggcggcacctttatcttcgcgttaatgagtcatgcacagattcgtaacgacatgagcaataagcgtaaagcagaagcacgccaaaaagcagaacgtgcggaaaacattaagaaaaattataaaaacccggcataaatggcgagggtttaagcaatcgagcggcagcgtacttaccccgcactccattagcgggtatactcatgccgcattgtcctcttagttaaatggatataacgagcccctcctaagggctaattgcaggttcgattcctgcaggggacaccatttatcagttcgctcccatccgtaccagtccgcaaaatcccctgaatatcaagcattccgtagatttacagttcgtcatggttcgcttcagatcgttgacagccgcactccatgacgggtaaaaagtggataaaataattttacccaccggatttttacccatgctcaccgttaagcagattgaagcagcaaagccgaaagaaaaaccataccgccttctcgatggtaatggcctgtacctttatgtccctgtgtcagggaaaaaggtatggcagcttcgctacaagattgacggtaaggagaaaatcctgaccgtcggaaaatatccgcttatgactttgcaggaggcaagggataaagcatggactgcgaggaaagacatctcggttggcatcgatcctgtaaaggcgaaaaaggcttcgtctaacaacaattcctttagtgcgatttacaaggaatggtacgagcacaagaagcaagtatggtcagtagggtatgcaactgaacttgccaaaatgtttgacgacgacattttacctatcattggcggccttgaaattcaggatattgagccgatgcaactgctggaagtaatccgcaggtttgaagatcgcggtgcaatggaacgagccaacaaagcacgcagaagatgcggcgaggttttccgttacgctattgtcaccggaagggctaaatataacccggcacctgaccttgctgacgccatgaagggataccgcaagaagaacttcccgtttcttcctgcagaccagatcccggcattcaacaaagcactggcaacattttcaggaagtatcgtatcgctcattgcgaccaaagttttacgctacacagccctaagaacgaaagagcttcgttccatgctatggaagaacgtcgattttgaaaataggattatcaccatcgacgccagtgtgatgaaaggacgcaaaattcatgtggttcctatgtcagaccaggtagttgaacttctcactacgctaagctccatcaccaaaccagtctcagagtttgtttttgccgggcgcaacgataagaagaagccaatctgcgagaacgcggtactgcttgtgatcaaacaaatcggctatgagggtctggaaagcggtcacggattcaggcatgaattcagcacgattatgaacgagcacgaatggcctgctgacgctattgaagtgcaactggcacatgcaaacggcggatctgtgcgtgggatttacaaccatgctcagtatctcgataaacgcagagaaatgatgcaatggtgggcggactggcttgatgagaaggtggagtgagcgaccttaacaactatcgaatagcacaaagtcttgcaatccagtgcaaagctttgtgtgtataagttttgtctcatcaaccacagcaagtatcgatcgattaagacttggatgatagacttcattcctttgattattagctgatagaagaaatgttaaagctatttgcaaagtacacctctattggtgtgctgaacacccttatacactgggtggtttttggtgtttgtatctatgtcgcgcatacaaaccaagctcttgcaaacttcgcaggtttcgttgtggctgtgagctttagcttcttcgcgaatgcaaaattcacattcaaggcatcgactacaacgatgcgctacatgctatatgttgggttcatggggacactgagtgctactgttggatgggctgctgatagatgcgcacttcccccgatgataactcttgtcaccttctccgccatcagcctggtgtgcggtttcgtctattcaaagttcattgtctttagggatgcgaaatgaagatatctcttgtagttcctgtcttcaatgaagaagaagcgataccaattttttataaaacggtacgtgaattcgaagaattgaagtcatatgaagtggaaatcgttttcataaatgacggcagcaaagacgctacggagtcaatcattaatgctctggctgtttcagatcctctagttgttccgctgtcatttacacgcaactttggtaaagaaccagcattgtttgcagggttagaccatgcaaccggggatgcgataatcccaattgatgttgacctgcaagacccgattgaggttattcctcatcttattgaaaaatggcaagcaggtgctgatatggttcttgctaaaagatctgaccgctcaactgatggacgcctgaagcgaaaaacggctgagtggttctataagctccacaataaaataagcaatcctaaaattgaagagaatgttggtgatttcaggctgatgagccgtgatgttgtcgaaaatattaaacttatgccagaacgaaaccttttcatgaaaggtattctgagctgggtaggaggaaagacagatattgttgaatacgtgcgagcggaaagaattgctggagatacaaaatttaatggatggaaactttggaatttagcacttgagggtattacaagcttttccacattccctcttcgcatctggacatacatagggttagtggtagccagtgtagcatttatttatggggcgtggatgattttagatactatcatatttggaaatgctgttaggggatatccttcactacttgtttcaatactgtttttaggtggaattcagatgattggaataggagtattaggtgaatatattggacgcacatacattgaaaccaaaaaacgcccgaaatacatcatcaagagagtcaaaaaatgaataaagcaataaaagtatcattgtatatatcttttgttttgattatttgcgccttatctaaaaacataatgatgttaaatacatctgatttcggaagagccattaagccattaattgaagacataccagcatttacatatgacttacctttattgtataaattgaaaggtcatattgattcaattgatagctatgagtatataagttcatatagttatattttgtatacatacgtcctgtttattagcatttttactgaatatcttgatgctagggtgttatcgttatttctaaaagtaatatatatttattcattatatgcgatatttacttcatatataaaaacagaaaggtatgtaactttatttacattctttattttagcttttcttatgtgttcttcatcaacactgtcaatgtttgcatcattctatcaagagcaaatagttataattttccttccatttttggtgtattcattaacatgcaaaaacaataaatctatgcttttgctatttttttcgttgctaataatatctactgctaaaaatcaatttatattaaccccactaatagtgtattcatattatattttttttgatagacacaaactaattattaaatctgtaatatgcgtggtgtgcttgcttgcgtcaatatttgcaatatcttattcaaaaggtgttgttgaattaaataagtaccatgcaacatacttcggtagttatctttatatgaaaaacaacgggtataaaatgccatcgtatgttgatgataagtgtgttgggttagatgcctggggtaataaattcgacatatcatttggcgcaaccccaacagaagttggaacggaatgtttcgaatctcataaagatgaaacgttttcgaatgcactctttttattggttagcaaaccaagcaccatcttcaaacttccatttgatgatggtgtgatgtctcagtataaagaaaattatttccatgtatataaaaaactacacgtaatatatggagaatcaaacatactaacgactattactaacataaaagacaatatatttaaaaacattagatttatatcattgttattattttttattgcttctatttttattagaaataataaaataaaggcatctttatttgtagtatctctttttggaatatctcaattttatgtgtcatttttcggggaaggatatagagatttaagcaagcatttatttggaatgtatttttcgttcgacctttgcttatacataacagtcgtttttttaatttataaaataattcaaagaaatcaagacaatagcgatgtaaagcactaagtttaaattgcgcgccaatcatggcgcgcacaagctataataccaacctaatttctcctcctcttagagtgactatatctcctgatagaattgcggtattgactatcaaatgccctgattcgttgtttattgtaatatctcctctatctgcagacgataacttaaatgcatcattgcccacaacaaaccccctccagaaccaagtgctgatattatcatcaacagtgatagatacatatactaactgattatcgttataagtgattcctgtcttatacttaacataaggacttccactttgattctcgatagacacataacatccaggggttatgtttgtatgcgtcccgcgactatcgccccattaacgccatacgataaatgggatggtgagaaatgggtgacggataccgaggcacagcatagcgtcgcagtagatgcagcagaagcacagcgccagtcgctgattgatactgcaatggcttccattagtctgattcaactgaaattacaggctgggcggaagctgatgcaggcagagacctcccgacttaacactgtgctggattacattgacgcggtgacggcaacagataccagcaccgcgccggatgtcatctggcctgaactgccggaggagtaggccattcaatatctggcgcactggaagtatcgaccagctccagtgcgtccagataatccagccacaaattatattgcgccagttcctcacctttcagacgaccaatagccgctttaccagcccattgtttactgttcatataatcgttggcctgattaatcaattgctgctttttcagttcggctgcagcaatctgttcctcatgtgttggtggtggaatttcagaccatgcaggaaaaccattttctccagcgatacggatttttcctttcggcggtaatccggaaaactcaatatacacttgctcatcaacttcaacagcatcatctggccatgagccagcttgcgtgtaatcctctttcatctccaagggatagaaagagtttgtagtcgcggaatatatgtaattcatttttcactccataaagttaaaagaaattaacaccctaatgcgaaaaatgaagcaccgataccgggtacgcctgctctggaaataaatttcaccgggtcctggttataaccggcacaagctatatagccaacatttgcactgccgggagtgtaatcctgagtcgcaaatacccgcagacatctattcggaaatgcaatcggaaaataggttactgtgtcctgagacgtcagcggaacatcaattggcccccattgaataattaaaccggatggcaatttttgatatccaggaactgaagcagaaagcataaaactacccatatcaggtatctgattcgcccctgtccctacatttcttttagccgcttctcccaaaccaaggttttcgagagccttttgcaccgtgccgtccaatttgatatcgccaaacggattcttgcggcttaacagcagcgcacgaagcgcggtaagcagctggtcatgccgccccttctccaggctggcaccggaggcctccacaacgctgcaaagctcctcctgcaacatgtcaaagtagtcatcatccagatcggtggcaggcgtgccggtctgggggttaccacgggtacgggggattaccaaaggcagcacctttaagctccgcaagacgttctgaccagtcatgcgccagcgcgttgtcttccgcagtgtaatacgcggcacatttggcgttatcaccatcagtaaacagatccagaacaaacgggccaaacagggtgttaattccccagaaaatgttgtccggcgtgcgccactgatcgcccacttccttcagttcatgggctggtttgttccgcagctccaccagcgcctggcaatatttattactcattaagcccccacgtaattccctgagagataccactcttcacctgatgcagcccgcttactgcttttccgtaaacaccgttcacgacgcgccagaaaattgtttcgttctggctgggagtggctttcacggaatgccgccatccacaccgttgcagcacgacggtataagcccctggactccagttcttccgcctggcgggtcaggcacaaaatcacccgcgggtcgttagtgccgacatagaaattgcgcacaggtctggtttcacgaactggttgtggttccggatcctgcgctctctcagtcaggcgcgggaaatgtctgtgtgtatctccttcacaacggtgagccacacgcccactctgacgtaacttgcttgctgactgcagaacgcgctgccgtgagtaacctgcaaaagcatccgcaatgtctccggaagtacagcccggatgggcttcaatgaatttctgaacgtcattcaaaagactcatgctcaccccctgaatcctgccgggatctggctgtagtccacattgtcgtaactggctttgaagtacgggtcttcgcgtttttctgtgtacgtgctgacggacggcgataagcgcagggaaagctcatcccatttttcccgcagcttcgacgggctgagcacgttacggcaccagaacggatcgcggctgacgcggctgtacatctcgcagatttgtttgtgagtacgaccatcctgcacacacatcaggcgaatttcgtttgcccaggctgtccagttcggttctttgggacgaaccacctcgccgtcacattcggcggcctgctcgtacagggcgatgatttttttccagagccactgtgcgcaggtcaaatcatcctgcgttccccactggcgctttttagggctgaatacaaccgcatcaggatggcgagttaaaaaatcctgttcatccgtctgcgtgtccggttgcgaagcgtccggacgagaaggttttttatctgacggatcatgttttgattttactgacggatccccgccagattctgacgggtgaaaacccgattttttgccagatttcgacgcatcaaattttgacgggtcagattttgatgcgtcagattttgacgggtcagagtctgacagttgagaaaatgccgctgcctgaagcttcgcaacgttaagctgataaacattcgacgcattgcggttatgatgaggagcagcaaaatggctagcgaacgcagtactgatgtgcaggcatttatcggggagctggacggcggcgtatttgaaaccaaaatcggcgcagttctcagtgaagtcgcttccggtgtgatgaacacgaaaaccaaaggtaaggtctcactcaacctggaaatcgaaccatttgatgagaaccgtctgaaaatcaaacacaaactctcatatgttcgcccgactaaccgtgggaaaatttccgaagaagacaccaccgaaacgccgatgtatgtcaatcgcggtggtcgcctgactattctgcaggaagaccagggacaattactgactcttgccggtgagcctgacggaaaactccgcgcagcaggtcattaatatcattcttaattaactaattatttatctcatcactgaatatcttaatatagtgaggacttattatgtctcagaacttagacgcaaccgcaattaatcaaatccatgcccttatttctgctcagggtgttaatgaaattatcagtaagattggtgccgatgctgtggcattgcctgagaatttccgcattcatgatctggaaaaatttaatttaaatcgcttccgtttccgtggtgcgctttccactgccagcatcgatgactttacccgttattctaaagatcttgcagatgaaggcacccgctgctttatcgatgctgataatatgcgtgccgtcagtgtgcttaacctgggtactattgatgaaccaggtcacgcagataacaccgccactctcaaactgaaaaagacagcaccgttctctgccctgttgtctgttaacggcgagcgtaactcccagaaatcactggcagaatggattgaagactgggccgactaccttgtgggctttgatgctaatggtgacgccattcaggcaacaaaagcggctgcggcaatccgtaaaatcacgattgaagcaaaccagaccgctgattttgaagataatgacttcagcggcaaacgctccctgatggaatctgtcgaagcgaagaccaaagacattatgccagtggcatttgaatttaaatgcgttccgtttgaaggtctgaaagaacgtccgtttaaattacgcctcagcattatcactggcgatcgtcctgtactggttctgcgcattattcagctggaagcggtgcaggaagatatggctaacgaatttcgtgatctgcttgttgagaaattcaaagacagcaaagtagaaacctttattggtactttcaccgcctgatttcattactgcaaatgcccctgcgggggcatttatggaaacgtaattaactcaataatcaccggatggtgagggcttccttttacccaaactcagcgcggtgcagcgcatatacgtggagaacaaaatgtcatttattaaaactttttccgggaagcatttttattatgacaagataaataaagacgacatcgtgattaacgatatcgcggtttccctttcaaatatctgccgctttgccggtcatctttctcacttctacagtgtcgcccaacatgcggtgctttgcagccagctggtgccgcaggaatttgcttttgaagcattaatgcatgatgcaacagaagcgtattgccaggacatccccgcaccactgaaacgccttcttcctgactataaacggatggaagaaaaaatagatgcagtaatccgtgagaaatacgggttacctcctgttatgagcacgccagtgaaatatgccgatctcattatgctggcaaccgaacgccgtgatctcgggcttgatgatggctctttctggcctgtactggaaggcatcccggcaacagagatgttcaacgtgattccactggcaccgggtcatgcctacgggatgtttatggaacgttttaacgatttatcggagttacgcaaatgcgcatgaatgttttcgaaatggaagggtttcttcgcgggaaatgtgtaccgcgagatctgaaagtgaacgaaacaaatgctgagtacctggtacgtaaattcgacgcgcttgaagctaaatgtgcggcactggaaaacaaaataataccagtgtcagctgaactgccaccagcaaatgaaagtgttctgttatttgatgctaacggagaaggctggctgattggctggcgttctctctggtacacctggggacaaaaagaaaccggagaatggcagtggacatttcaggttggggaccttgaaaacgtcaatatcactcactgggcagtaatgccaaaagcaccggaggctggagcataatgaccacatttaccaataaagaactgattaaagaaatcaaagaacgaatcagcagcctagaggttcgagacgatattgagcgccgtgcttatgaaatcgcactcgtatctctggaagtagagccagatgaacgcgaagcctatgaattattcatggaaaagcgtttcggtgacttagtagatcgtcggagagcaaaaaacggcgataacgaatacatggcatgggatatgactctcggttggatcatctggcagcaacgagctggtatccatttttcaacaatgtcacaacaagaggtgaaataatagagccatacagcctcacactcgatgaggcctgtcagtttcttaaaatatcctgatctaccatcgccgtcatagagcgtatttttattacctgatttgcaggttcgattccctattcggagatagcactcatgcaacacgaactacagcctgattcactggttgatttgaaattcatcatggctgatactggctttggtaaaaccttcatctatgaccggattaagtcaggcgacctgccaaaagccaaagttatccacgggcgagcaagatggttatatcgtgaccattgtgaattcaaaaataagctcttaagccgcgccaatgggtaaaatagcgggtaaaatatttctcacatctaaaaaacaccattccaatcaatcccctgctgcttcaagtagatgtctgcaggggacaccatccttgtgtttatccctaaaaccacataaaaaccgtaaattaaattcgaactagcaggccgaataaggcacaccaggaactcgtggttttattcattatgaagtggtttttacctgttctcttagccagataataaacgcttcaatttttggccactgcctgcccggtaatgtggtgatgtaataatgctgatggcatttcaccgtcatatcgccaaacggcgcgacgagctcaccactggcaagccttttttgtaccaggcgttttcttcccatcgccaccccaatatgattcatcgcggcaataacagctaaatcagaacgatcaaagccaattccagaagatgtcggcaaattaaccgcataatgttgcgcccaactatgccattcatccgtaccggagtcgttgctccatgcctgtctgtcatggagcaacgtacagtgacacaggttaattaccgtgttggttaaagcatgtctttgagcgtattccgggctacatactggcaggatttcttcatccatcagaaagtgatgagtgagttgcgctgacggcgcatcatcaaagtagatcgccaaatcgattccggcacgttgcagattgacgttgtcattaccagtgagcacggtgagcgaaatagacggataccggcgtgtaaagtcacctaatgcgggcaccaaccagcattgggcgatagagggccgggaatacagagttaacgttcccgataactcctgatttttgatatcaagaatttcctggttcagggtatccagcgacgattttagcgcccaataaacacgtttcccctcgtgcgttaattccactttgcgatgggaacgaacaaacaactgaatgcccaattcttcttccagctgattgatacggtgacttaccgcactggggctcagcgacaattcctctgccgccagggcgaaggactgatgcctggcagccacttcaaaagtatgcatttttgataattgccagccgttaagcagccgatttcttatttcacgaaggggttccataatcacctcatttttcgcttaagtgtaaaaaaatagcggcaaaatttcagctatgagatgagctaaagtgaaccatatctcaattcaccttcatttttagatgtaaatcactccattgatgcaatttacctcatgtgaaaggcaaattttatcgtttgtcagcctgcgttgtttttttgtccaatatcatcaggttaatcacaggggaaggtgagatatgcactctcaaatctgggttgtgagcacgctgcttatcagcatcgtgttaattgtactgaccatcgtgaagttcaaattccacccgtttctggcgctgttgctggccagcttcttcgtgggaacgatgatgggcatggggccactggatatggtaaatgctattgaaagtggaattggcggaacgctggggttcctcgcagcggttatcggccttggcacgatactgggaaaaatgatggaagtatccggggccgcagaaagaattggtctgacacttcaacgctgccgctggctttcagttgatgtcattatggtgctggttggcctgatttgtggcatcacgctgtttgttgaagtgggcgtcgtgctattgattcctctggctttttcaattgccaaaaaaaccaatacctcattattaaagcttgccattccgctatgtaccgcattgatggcagtgcactgcgtggttcctccacatccggctgctttatatgttgccaataagctgggcgcagatatcggttcggtgatcgtctacggtttgctggttgggctgatggcatcactgatcggtggcccacttttccttaaatttctgggtcaacgactgccctttaaacctgtacccacagagtttgcagatctcaaagttcgcgatgaaaaaacactaccgtcattaggcgcaacgttattcaccatactgctacccattgcgctgatgttggttaaaacgattgccgaattgaatatggcgcgtgagagtggtttgtatatcttggttgagtttattggcaaccctatcactgccatgtttatcgccgtgtttgtcgcctattatgtgttgggtatacgccagcatatgagcatggggacgatgctcacacatacggaaaatggcttcggttctattgctaatattttgctgattatcggggccggaggcgcattcaacgccattttaaaaagcagcagtctcgctgatacgctggcagttattctctccaatatgcatatgcacccgattcttctggcctggttagtggctcttattctgcatgcggcagtgggctccgctaccgtggcaatgatgggggcaacggcaattgttgcacccatgctgccgctgtatcccgacatcagcccggaaattattgcgattgctatcggttcaggtgcaattggctgcactatcgttacggactcgcttttctggctagtgaagcaatattgcggcgctacgctcaatgaaacatttaaatactatacgacagcgacatttatcgcttcagtcgtcgctctggcgggcacattcctgctgtcatttatcatctaagcgcaaagagacgtactatggaaaacgctaaaatgaactcgctcatcgcccagtatccgttggtaaaggatctggttgctcttaaagaaaccacctggtttaatcctggcacgacctcattggctgaaggtttaccttatgttggcctgaccgaacaggatgttcaggacgcccatgcgcgcttatcccgttttgcaccctatctggcaaaagcatttcctgaaactgctgccactggggggattattgaatcagaactggttgccattccagctatgcaaaaacggctggaaaaagaatatcagcaaccgatcagcgggcaactgttactgaaaaaagatagccatttgcccatttccggctccataaaagcacgcggcgggatttatgaagtcctggcacacgcagaaaaactggctctggaagcggggttgctgacgcttgatgatgactacagcaaactgctttctccggagtttaaacagttctttagccaatacagcattgctgtgggctcaaccggaaatctggggttatcaatcggcattatgagcgcccgcattggctttaaggtgacagttcatatgtctgctgatgcccgggcatggaaaaaagcgaaactgcgcagccatggcgttacggtcgtggaatatgagcaagattatggtgttgccgtcgaggaaggacgtaaagcagcgcagtctgacccgaactgtttctttattgatgacgaaaattcccgcacgttgttccttgggtattccgtcgctggccagcgtcttaaagcgcaatttgcccagcaaggccgtatcgtcgatgctgataaccctctgtttgtctatctgccgtgtggtgttggcggtggtcctggtggcgtcgcattcgggcttaaactggcgtttggcgatcatgttcactgcttttttgccgaaccaacgcactccccttgtatgttgttaggcgtccatacaggattacacgatcagatttctgttcaggatattggtatcgacaaccttaccgcagcggatggccttgcagttggtcgcgcatcaggctttgtcgggcgggcaatggagcgtctgctggatggcttctatacccttagcgatcaaaccatgtatgacatgcttggctggctggcgcaggaagaaggtattcgtcttgaaccttcggcactggcgggtatggccggacctcagcgcgtgtgtgcatcagtaagttaccaacagatgcacggtttcagcgcagaacaactgcgtaataccactcatctggtgtgggcgacgggaggtggaatggtgccggaagaagagatgaatcaatatctggcaaaaggccgttaataacgtttcaacgcagcatcgcaatcctttccctgggtgagcgatgctgccgatggcgcagacttaagatccccggtcttacccgctataaccccctccttttatcatcacccaacgcctttcgctgtaaacggcggtttcgcaaaccaaaccaaaaccgtaagtaagataaaagcaatagccgccatacggaaaatctcatttgcagaaatagaaagtgactgctgggttatttcattattaatttcattaagaactcctgaaagcgaaccataatatttatccataatttgtgacgatgaattaaacacggggttaaattgatcgatggttgctgtcaactgactatggtgtaacgattcgcgtcgtccccacagcgtcattgtcaacgacgtaccaactgatcctgacaaggtacgaaaaaaattactcatactcgaggcattggcaaatttattatctggcaagcctgaaaacgaaatcgttgttaagggtaaaaagaaacaggcaacggcgaatccctgaaaaaactgcggcaaaatgatgcctgtaaaatcaatcgttggcataaatgtcacagaacgccagtaatagcaaaccgcatacatcaaaaaactaaatgtcactaacaaccgcatgtctattttgttgccataacgtcctatcaaaggtgaaattaatagtggcatgatgccgatgggcgcataagcaagtccggcccatatcgcattataccccatcgtttcctggagtaactgcggcataaggacgatcgctccagagtaaaataaatacgcgcatgtgatactcacaataccaatggtgaagttacgggacttaaacaaactgagatcaagaatcgggttctctgaggtcgactcccaaatgactaaagagatcagagaaataactgatactactgttaatattattattgtactcgagttgaaccaatccagatcgcgccctttatcaagcataatttgcaagccaccaacaccgagcactaacagggtcagtcctggtagattcattttgaccggtgaagtctcagtttctcttcctttaagtaaggttaagcataatgtcaggacgataatccccatagggacattgattaaaaatatccaaccccagctaaagttatcacaaatataaccgcccaatatcggcccacatatcggagcgataatcacggtcattgaccataatgccagagcaaatgttcttttttctggcggataattccttaataataaactctgtgacagtggaattaacggccccgccattaacccctgaacgactctaaaaaatatcagcacatcaagattggtcgataggctacacattaatgaagacagcgaaaaaaaagtgactgaaagtaaaaataatcttaattcgcctattctttgtgccaacctgccagtaacagggatcgcaatggcatttgctacaccaaacgaggtgataacccaggtgccttcgtctgttgatgctcccagaaagccagatattgtcggtattgcgacgttagaaatagtggaatccaacatttgcataaatgtcgctaatgacaatgcaatagtgacgcaccataacgtcccaccggttaatggtgccggagttgatttagtgattgccattaaagttgtccattatgcgaaataatgttgctaatttctttttctatcggactggtatcgataactaaagccttactggtataagccggcatggaggtcacggttgaagccagctcaggcatctcggcaatgtcttcgttcttcgtatcaatagttgctgtcatcgataaaccaatacgcaaggggtgttccatgagttcttttggatcaagagaaacttcaaccggtacacgctgaacgattttgatccagttccctgtcgcattttgtgcaggtaataaggagaacgcattgccggttcccatattgatccctgtcacccgaccatgaaacacaacattttcaccataaagatcgctgataatattgaccgattgaccaatccgtacatccgtgagttgtgtttctttaaagttggcattaacccacatttgacgtgccggtacgacagccattaacgattgtccggggctcactgtttcgccgacctgaacacttctctgggcaatatagccggtaaccggactcttaatatccgtacgtttaagcgccaaccaggcttctttagttgcatccgccgcttcaacgacttgtggctgacggtttaatggtgtgttcattactaaagctttattcgctttataagcctggatagcggcattcaatgccgctttgctacttattaacgtatctttggtatgctccagcgtttcttttgaaataaccccctgcttcgctaacggcactcgacggttataatcttctaaagattgttgatactgaatacgtgctgaagcgacttcggcactgtattgtttatcctgtaagtatagtttattcgtttgccgaacaatatttgccagattatttttagctttattgagtgcgatagtggcatcagttttatccagtgaaactaaaatgtcaccttgtcgaacgtagttcgtatctttatgattaacgacagtgacactacctgagacttgtgcagaaattggatctgcattccccgtgacataggcgtcatctgtactaatcatgtcttctaattccattgaccaataggcataggcacctgaaaacgcaataaataaaactaccgccaataaagaaaagtattttcttctgttagaatgttttttatttgaattaatctgttccactattatctctcatttctcatagatgaaatttatgaattgaatgaaaagagcattcattcttcatatcaaacacagtgcatgtgttgcacattatcccaggaacgttggaggcctaatttaaatgaggtgcaaaaaaaacaacagaggactaaaccgtggcttttgcaatacaattcttacgcctgtaggattagtaagaagacttatagtgccaacttgaaactataaatcatcggtacaatccctgattttattgttgacatttcatttatgccgactatttatatggtatacttgtcgaattatcttaaaggaagctcagattttcttatttttattgagaaaatgagatgacgccttatgtctgtattactacagggagaagggagatgcttcattgcaaagggaataatctatgaacgcaataattattgatgaccatcctcttgctatcgcagcaattcgtaatttattgatcaaaaacgatattgaaatcttagcagagttgactgaaggcggaagtgccgttcagcgggtggaaacacttaagcctgatatcgtcatcattgatgtcgatatccccggagttaacggtatccaggtgttagaaacgctgaggaagcgccaatatagcggaattattattatcgtctccgctaaaaatgaccatttttacgggaaacattgtgctgatgctggcgctaatggtttcgtgagtaaaaaagaaggcatgaacaatatcattgcggctattgaagctgcaaaaaatggctactgctatttccccttctctctcaaccggtttgttggaagtttaacgtccgaccagcaaaaactcgactccttatcgaaacaagaaattagtgtcatgcggtatattcttgatggcaaggataataatgacattgctgaaaaaatgttcatcagcaacaaaactgtcagcacttataaaagtcgcctgatggaaaaattagaatgtaaatcactgatggatctttacacattcgcacaacgtaacaaaatcggctaaccacatgaagtttttaccctatatttttcttctctgttgtggtctttggtcgaccataagtttcgcagacgaagattacatcgaatatcgtggcatcagtagtaacaaccgtgtcacacttgatccactacgtctgagcaacaaggaattacgttggttagcgagcaaaaaaaatcttgtgattgcagtacataagtcccaaacggctacgttgttgcataccgattcgcagcaacgggttcgtggtattaatgctgattatttaaatcttttaaaaagagcgttaaatatcaaattaacactccgggaatacgcagatcatcaaaaagcaatggacgcgcttgcagaaggtgaagtcgatatagtgttatcacatttagttacttcgccgcctcttaataatgacattgctgcaaccaaaccattgataattacctttccggcgctggtaaccacccttcacgactcaatgcgaccgcttacctcaccaaaaccagtaaatattgctcgggtagcaaattaccccccagacgaggtaattcatcaatcatttccaaaagcaacaattatctcttttacaaatttatatcaggcattagcatccgtctcagctgggcacaatgattactttattggtagtaacatcattaccagcagtatgatttcccgctatttcactcactccttaaatgtagtgaaatattataactcgccgcgtcaatataattttttcttgaccagaaaagaatctgtcattcttaatgaagtactcaatagatttgttgatgctttaacaaatgaagttcgctatgaagtatcacaaaattggcttgatacaggaaacctggcctttctgaacaaaccattagaactcactgaacatgaaaaacagtggattaagcagcatcccaatttaaaggtgctggaaaatccttactcgcccccctattctatgacggatgaaaatggctcggttcggggcgttatgggggacattcttaatattattaccttgcaaacaggtttaaatttttctccgatcaccgtttcacacaatatccatgctggaacacagcttagccccggaggatgggatataatacctggcgctatttatagtgaagatcgagaaaataatgttttatttgctgaagccttcataacaacgccttacgtttttgtcatgcaaaaagcgcctgacagtgaacaaacattaaaaaaaggaatgaaagttgccattccatattattatgagctgcattcgcaattaaaagagatgtatccggaggttgaatggatacaggtcgataatgccagcgctgcatttcacaaggttaaggaaggtgaacttgatgctctggtcgcgacacagctaaattcgcgttacatgatcgatcattactatcctaatgaactttatcattttcttattcctggcgttccgaatgcatcgctttcgttcgcttttcctcgcggagaaccggaacttaaggatattattaataaagcactgaatgcaattcccccaagcgaagttctgcgcctgacggaaaaatggattaaaatgcccaatgtgaccattgacacatgggacctatatagcgagcaattttatattgttacgacattatccgttttattagttggcagtagccttttatggggattctacctgttacgctcagttcgtcgtcgtaaagtcattcagggtgatttagaaaaccaaatatcattccgaaaagcactctcggattccttaccgaatccaacttatgttgtaaactggcaaggtaatgtcattagtcataatagtgcttttgaacattatttcactgcggattactacaaaaatgcaatgttaccattagaaaacagtgactcaccctttaaagatgttttttctaatgcgcatgaagtcacagcagaaacgaaagaaaatcgaacaatatacacacaggtatttgaaattgataatggcatcgagaaaagatgcattaatcactggcatacattatgcaatcttcctgcaagtgacaatgcagtatatatttgtggttggcaagatattactgaaacgcgtgatctaattaatgcactcgaggtagaaaaaaataaagcgataaaggctaccgtagcaaaaagtcagtttctggcaacgatgagtcacgaaataagaacaccaataagctctattatgggcttcctggaacttctgtcgggttctggtcttagcaaggagcaacgggtggaggcgatttcacttgcctacgccaccggacaatcactcctcggcttaattggtgaaatccttgatgtcgacaaaattgaatcgggtaactatcaacttcaaccacaatgggtcgatatccctactttagtccagaacacttgtcactctttcggtgcgattgctgcaagcaaatcgatcgcattaagttgcagcagtacgtttcctgaacattacctggttaagatcgaccctcaggcgtttaagcaggtcttatcaaatttactgagtaatgctctcaaatttaccaccgagggggcagtaaaaattacgacctccctgggtcacattgatgacaaccacgctgttatcaaaatgacgattatggattctggaagtggattatcgcaggaagaacaacaacaactgtttaaacgctacagccaaacaagtgcaggtcgtcagcaaacaggttctggtttaggcttaatgatctgcaaagaattaattaaaaatatgcagggcgatttgtcattagaaagtcatccaggcataggaacaacatttacgatcacaatcccggtagaaattagccagcaagtggcgactgtcgaggcaaaagcagaacaacccatcacactacctgaaaagttgagcatattaatcgcggatgatcatccgaccaacaggctattactcaaacgccagctaaatctattaggatatgatgttgatgaagccactgatggtgtgcaagcgctacacaaagtcagtatgcaacattatgatctgcttattactgacgttaatatgccgaatatggatggttttgagttgactcgcaaactccgtgagcaaaattcttccttacccatctgggggcttacagccaacgcacaggctaacgaacgtgaaaaagggttaagttgcggcatgaacttatgtttgttcaaaccgttgaccctggatgtactgaaaacacatttaagtcagttacaccaagttgcgcatattgcacctcagtatcgccaccttgatatcgaagccctgaaaaataatacggcgaacgatctacaactgatgcaggagattctcatgactttccagcatgaaacgcataaagatctacccgctgcgtttcaagcactagaagctggcgataacagaactttccatcagtgtattcatcgcatccacggtgcggctaacatcctgaatttgcaaaagttgattaatattagccatcagttagaaataacacctgtttcagatgacagtaagcctgaaattcttcagttgctgaactctgtaaaagaacacattgcagagctggaccaggagattgctgttttctgtcagaaaaatgactaaatagcggctcccacaatgttcaaatgtgggagctatttaccagcacatcttacatttatgatgagaactcctggcgaatttgttccccatgctggtcgagcgttgccgctcccggcataacatgcgggtccgcgcagccgctgatttttatcggattacccggcatcattattcccccggcttcaatcaacatatttctcgcctgagtttgtggcaatttaatggcctcagccacacttaataacggcgcgacgggtacaccaacttcatgtattctggctaaccaaacttcagctgcctgcgtttttaacgtccgctcaatatattgtttaagaatagcctggttttgtacgcgtaaaatattgctgctaaatcggggatcattaaccagttccgtaagctccagtgcctggcataacgcagaaaaaagcttgtcattaccacaacaaatcgtaatcggcttatcctgagtattgaaaacatcaaaaggtgccatgtagggatggcgatttcccagacgttgtggtgacttcccagttgcgatatatgccatcagaccatgctccagaaaactcagcgtggcatcaaacatcgctatatcgacatgcgcccctctctggctcttttcgcggccataaagtgcactcactattccgctgaataaatagacaccgccgcatagatccgcaagagatgtaccaacgcgcactggcggagcatcaggatatcctgtttccatcattatcccgctcattgcctgaatgatggtatcgtaggcaggagcatcttttagcggaccggtatgtccgaaacctgacgatgaagcatatatgaggcgcgggttgatttcttgaagcgtttcccatgaaaaccccagtttttccattgtacctgggcgaaaattctcagctaatacatcagcttgtttgagcatatttataaatatacttttatcgtgatcattctttaaatcaagaaccacactctctttgccatgattaataaaactgtaatagagtgactgtccatccacatagggaccaaatgtgcgggtatcatcaccatgacccggcggctcaactttaattacccttgcgcccatattacaaagaagttgagttccgaaaggtccattaaggacatgtgtcatatcgataactaataagccttcaaacggccctttgctttcattatttgtcatttgcttatgccttgaaaaaagccgaaggtgaaaagacacttcggcatttatgtaaaatcaataacatgattaattatgaaaccagtcgactgacataaatccacaagggagccgtgacgacaaagcccagtacgctcacagccaatgacgctgtaccagtacgggtgtagacattaaaccggctggcaataatgattccggagaatgccggcggtaatgcgcctgccagtaccatcatctgcagatgttcgctgttcaaatgacatgccataccaacgagaagcagtgccagtggcatcagaatcagcttcaggaaggtgttataagcaatttcggcactgaactcgaatttatgtgcagccagagtcaaccccgcagcgaataccgctacccctgagttagccttcgcaatcagattaaaggttgggtcccatgctgccggaatttttaccccaaccaacaccaggatcgttgccagaacaggtgcccatactactggctcctttgccgcagaaattaatgcgctcagattactattcttcttaccatccgctcctgaagaaggattcagcaaatacagaccaataggaatagtaattgcgttaacaataatagaaataattgctaccactaaacctgttgatacggaatcaccataaataggatcgagaactgcaaaccccaggaatccaatggtaggtgaacctgcaattaatgcacatacagctgcttctgcatgggtacgtttaaaaaatttgtagcaaccgaaccaggagaaaaagaaacatccgacaataaccacaagtgatacaagggtcagacgagtgtccgcaaaaatcatttccctgtttgcccgagtaatagatacaaatagagccgcaggaagcgcgtagtttaataccagtttattaaatgcccgagcttgatcttctgaaaatgtttctcgtctgccgctaaaataacccaacagcatgattacgataataggcaataaatcgccaataaaaaatgttagcataatagtatttccgataagggtcccctcaccatcgcataatgagttggcaagaggagacgatgtcagtatttaattaccagcgacttgttttgggttaagtttggtaatatggccactttcagttcctgctgcagggtcgatgaccacattaataatggtcggtttgcgcgactgaataccggtggttaaagcatgacgaagttcatctgtcgtggtgacgttatagccaacgccacgaaacgcatccattaatttgtcataccttgcatggtgcaacagatccgttggtgatggtgcaccagcgccactgagatcaacaccgtctcctctgtagatgccgccattattaaaaataacgatcgtcaccggcaggttatatcgacaaatcgtttcaatttccatcccactgaaaccaaaagcactatcaccttcaatggcgacaaccggagaaccagaagtcacgctagcaccgatggcatagcccataccgatgcccatgacaccccaggtaccacaatccagacgacgacgtggtttatacatatcaataatatttcgtgcattatccagggtatttgcaccttcattaactaaataaatatcctggttctcgcgcaatacgtcgcgcacagcacttaatgcattaaagtaatttaatggttgagtatctgtacttaatttttcatgcattttttgtgcattttgctgcttgtggatatttaaaatatcgcgccataccagtggagtcgtaaatgtgttttgtttcagttctgccagcataccttgcatactggatgcaatatcaccaacgactggcacagcaatggggcggttgctgtcaatttcctgcggttcaatatccagttgaataaactgtgtatctgccgcccatccttttttaccgtgtgccaataaccaattcagtcgtgcaccaacaagcatgacaacgtcagcatttgccagggcaaacgaacgcgcagctgccgcagaaagtggatgcgtatcttcaaggatccctttcgccatagacattggcaggaatggaatctgagcactttcaataaattcacgaagctgttcatcagcttgtgaatacgccgcgcctttgccaaggataattaatggccgttcagcttttgctaaaagcgaaattgcgctagtgactgacttcgggcatggcaataatgctggcgacggattttcaactttaacaatcgtggttaacgcttcgtctttttccatcgtcgcggccaggacatttgctggcaaatcaagataaactccgccagggcgacccgatacagagacccggatagcgcgtgccaatgcaatgccaagatcctgcggctgattaacgcgaaatgctgctttggcatacggttttgccgcattcatttggtccagctcttcataatcaccttgctgtaggtcgacgatcgcgcggtcgctggagccgctaatcatgatcatcggaaaaccatttaccgttgcgttggccaatgcggtcaaaccattgaggaatcctggcgcagaaactgtcaggcagatccccggtttttgggtaagaaaaccgcttgccgcagcggcatagcctgccgactgctcatgacgaaaaccaatataacgaatgccttccgcctgggcatggcgtgccatatccgtcacaggaatacctacaacaccataaatagtgtcaatattattctgttttaatgcttcaacgatgatatgcataccatctgtcatttgaagttgatctgacatgattaataacctcgaaatttttataaattgggagccagaagcccccgttaatatcagatggcgtggttttgcttcattgcagcaatttcatcgtcgctataacccagctcctgcaatacagcagcggtatgttcacctaatagcggcgcagctttaatatccggcgtaaaggcagagaatttcattggacaaccaacggtcagatattttccacgcaacggttgttccacttcaacaacactgccactttggcgcaaagagggatcaagtgaaatttctttcatacttaaaaccggtgcacaaggaatatcaaactgagtcaaataggccaccgcttcatgtttatcaatagtgacagtgtatttttcgatttcagcaaaaatatcgaaaatatgtggctgtcgtgcatgggctgtactgtatgccggatcggtaatccattctggtttgccgatggctttacaggtgttttcccagttttgctcctgaatagtgaaataaatataggcgttaggatcggtttcccagcctttacatttcaggatccagccaggctgaccgccaccacctgcattaccaccgcggggaactgcatcaccaaatgtaccattcggatactgcgggtattcttccagataacccaatttatcgagacgctgctggtcacgtaatttcacgcggcaaaggttcaatacggcatcctgcattgacatggtgactcgttgcccacgccccgttttttcgcgatgcagcaaagcagcaagtaaaccgatcagcaaatgcattccggtgttgctgtcacccaacgctgcagcgcttaccagcggcggaccatcccaaaaacccgtagtggatgccgcgccacccgctgcctgagcaacgttttcataggcttttacattcacataaggcgaacactcatcaaaccctttgatcgaaccaaaaatcagacgtggattgatttcttgaatatgctcccaggtgaagcccatgtgatcaatggcccctggatgaaagttctcgactaagatatcagcttcgcggatcagcttttccattacctctttgccttccgctgttttggtatttaactcaatagaacgtttgttactgttaagcatggtgaagtaaagcgcatcgatatcaggaatatctcgcagctggtgacgcgttacgtcaccaacgccgggacgttcaattttaataacgtcagcgccaaaccaggccagcatttgagtacaagatgggccagattgcacaccggtgaaatcgagaactttaattccttgaagtggagttgacatagcaatacctattagttaattaaatatgtgttaatttagcgtttatttaaggcgtaatatcttctataaataacccgcaaaatatcgtcgtagctgcactcgatatttttaaaatcctgtatcaagtgctgaaaatcatttcatcgccacttccaattcctttctgcatggtaagtagtgaggacgaaaagaagaatatgataaatattgattcgtggtaatcagagagagtcgcgacatttgtgatgttattcttacaactgtaagaagcgccggtgatttacaagcaagggtatgattacgctttttaaagcgtaccataaaacataacataataaatgatttgtgatgacacgggattattgcggtttactttgaggaatataaaatgcgagtttatagcaccgcgagcgccaaataattttatgaccacaacctgtcgtattgtggtcataaaaaattgtcggctggagggagttaaatcctttacctcaatatactgcctgtcagcattagttcacaaacagtgcttcgctatcgacgatgattccatcttccgcacctttaagcgccaggtttgcctcgtagtattgctttttatcaagcagtttctgcgcatcagcaagtgcattacgagtctgtttaagtggcatcagatattggttttccattacgccaacaccggccaggcgaagctcttccattgcgccctttttatcccctttcgccattttttcattggcaatttttatcgcggcttctttttcgggagttgctacataactctcagaaattccgacagatgcattaatgacaatatattggtcatcattgagattggtctttttacctggcttagcgaactttgcccattcggtactgtcatctgacagcaaagcggaagcttcattggtcagttcttttgccttttctggatcgccatgaaacagagccaggcgcgctacctgcacgtcacgcatcgcatataaaccttgttcagagatacgctctgctgccgctgccgttttctgggtttgctgaacttgctgagtttgctgttgtgccgctaccggagcattatcagcagcccatacagttgaagatgccagaattgctgtgaccatcgtggccataattaaacgtttcatacttacctcattctttaacagttttagaaaacgccgccatcatattgggtgagcatgaaatgagaaatcagagagcaacggtcattttgaaagggttatcttacagttgtagttattatcgcaagaagtattttagtcttacaattgtaggaatatgcttcctgtcgcagagaactattcttatataccacaaagagatgtcatttattatatcgatgtaaatactgattaattaaatgtaaatacagccataacatcgtaggttctcagtgaaccattttcaggataactttctatgaaagtaaacttaatacttttcagcttatttttattggtctctattatggcatgcaatgtttttgcattttccatttcgggtggtggaagtgagaggagctataaagagactgaaaaaacatcagcgatgacgaccacacactctacaaaacttcagccatcacaggcgattttgtttaagatgagagaagatgcgccaccattaaacctcacagaagaaatgccgcccccttttccgacaaaggcgaattatcttattcatcctgtgcgatagcgtctttcacatggcaggtgaacaatcatgtctgatgctgatgtgaacacctgcccaaatgagccatcctgacccactaccgcctgccataccccaccataaagcgaatcatcaagccacaagccggggcaagaaacataaatatccccgtcactagttcattaccgccagttaaccacatggtgaagtaataaatgagtgcagcgaggatcaccatgccgaagaaagaagagaccgccgataccacgttcagtacctgaccgatgtagccgcttacgcagacaatacacagggcgagaaacatccataaattaatcatagctcaacctcctgccgcgctaaaaaacctgtaacttcagtcactttaatagtaagacaatccttaacctctggcaatttttgctaagcatcaatgaaaacagcatgttaaatgcaagactgttgtgtacggaaaaatatttactttgcacgattaataatcagtagctgaaagcagtcagcgagtgataaagtacagataccgcattcatgctcctcgtggttatgtcctgactagtctttacactctttacaggaaccattgtcgtacatgatggcccaaccaattgagtgtaccgctgtcgacatggaatcttctgcgatacaacaattcgtatctacagaaggtaactatgtttccacaatgcaaattttcccgcgagtttctacatcctcgctactggctcacatggtttgggcttggtgtactctggctttgggtacagcttccttatcctgttctctgctttctcggcacgcgtattggcgcaatggcgcgaccattcctgaaacgtcgtgaatctatcgcccgtaaaaacctggaactttgtttcccgcagcattctgcggaagaacgcgagaagatgattgccgaaaactttcgttcactcggcatggcgctggtagaaaccggcatggcatggttctggcccgacagtcgcgtacgtaaatggtttgatgttgaagggttggataaccttaaacgcgcacaaatgcaaaatcgcggcgtaatggttgtcggcgtccattttatgtcgctggaactgggcggccgcgtgatgggactgtgccaaccaatgatggctacctatcgtccacataataatcagctgatggaatgggtgcagacccgtgggcgcatgcgctctaacaaagcgatgatcggcagaaataatctgcgcggcattgtcggtgcactgaagaaaggtgaagcggtatggtttgctcccgatcaggattatggtcgtaaaggcagctccttcgcgccgttctttgcggtggaaaatgtcgccacaaccaatggcacctatgttctctcccgtctctctggcgcagccatgttgaccgtaacgatggtaagaaaagcggattacagcggatatcgtttgttcatcaccccagagatggaaggctacccgacagatgaaaatcaagccgctgcctatatgaacaagattatcgagaaagagatcatgcgcgcaccggagcagtacctctggatccaccgtcgctttaaaacgcgcccggtgggagaatcgtcgttgtacatttaacaaactgctcttactctttccctcctcaaatcggccataataacctcatggtttttatggcttttttcttaaggttttttccttcgctgaatatctaattattaccgtcagaaattaaactgtcgccgatatgagacacttgtaagttactaaaagtaaataagaaaatgcctcttgtctcgtttcagttttaggcgtacattagcgccgtctcgagcagtttagctcagaattctggggtgatgcccacggtaaaatacagggcttttaaggtcgctttgcccggtgtcaactcactgtatcaggtgtaatgaagtcattcaggcgtaacagtaattacgcggagagatgtaaagtgaaatatttctttatgggcatttcttttatggtcatcgtttgggccggtacttttgccctgatgatctaaaagcaaactgtgcaatgaaaaacaggagccatcaggctcctgtttgcatttctgacgacggtgtttattccgcgttttcgtgaatatgtttgctgctggcgggtagtaaaccgtcggcacggaacatcgctttaatccctctgatggcctgacgaatacggtcgcggttttcaatcagtgcaaagcgaacatgcgtatcaccatagtcgccaaagccaatccccggcgagacacaaaccttcgcttcgttaaggagcttcttggcaaattccagcgatcccatggccgcatatggttccgggattttcgcccagacatacatcgaagccttcggcatttcaaccatccagcccgcttcatgcagccctttaaccaatacatcacggcggcgtttgtactgttcggcaatgtcgcgcacgcactgttgatcgccctccagcgccgcaatcgccgccacctgcaacggcgtaaaggtgccgtaatcgtgatagcttttaatacgagccagggcgctgaccagcgttttgttgccaaccataaagccgatacgccagcccgccatgttgtagcttttcgacagcgtaaagaactcgactgccacatcgcgtgcacccggtacctgcataattgacggcgctttccagccatcgtagacgatatcggcataggccaggtcatggaccaccagcacatcgtagcgtttcgccagcgccactactttttcgaagaactccagttccacgcattgcgcggttgggtttgacgggaagccgaggatcatcatcttcggtttcggataactttcacgaatggctcgctccagttcgttgaagaaatcgacaccttccaccagcggcactgagcgtacctgcgccccggcaatcaccgcgccataaatatggatcgggtaacttggattcggcaccagcaccgtgtcaccatgatccagcgtcgccagcatcagatgcgccaggccctctttcgaaccaatagtgacgatggcttctgattccgggtcgatttcaacgtcgtagcgatcctgataccagcgggaaatggcgcgacgtaaccgcggaatgccgcgtgaagtggagtaaccatgcgtgtccgggcgctgggccacagtacataatttttcgacgatatgcggcggagtcgcaccgtccgggttacccatgctgaaatcgataatatcttcgccgcgccgacgcgcagccattttcagttcagcggtgatgttaaaaacgtagggcgggagacgatcaatgcgcgtaaagcgacgttcagggcgagtgtcagccataatttcctcagattaacgttagcgcccggaccgtccgagcgacgctgccacgatggtggctgttttgaaaatagcctgattaatttctgtctgtccagcgttttagaacattttattaatgacgttaaatgaggaactctgctttaaaaacaggaaatttatctgcgctaacaagaaaattaccactcattttattaacataataatttcaataaatttactaaccagaagtgcattatcaagagatgcattgctaatacaccatttatctatcaatccccttttaaaattgtggtttttcctcaaaaacggcctgctggtcatcagccttcaggttacctatcatagaggtttaatccttattcagagtcacccgtgcacgaaatattcaacatgctgctggcggtcttcgatcgggcagcgttaatgcttatctgcctgttctttctcatccgtatccgcctgtttcgcgaactgttgcacaagtcggcgcactccccaaaagaattgctcgccgttaccgccattttctcgctgttcgccctgttcagcacctggtccggcgttcccgtagaaggctcgctggtgaacgtacgtattatcgcggtgatgtccggcgggattctgtttggcccgtgggtaggcatcattaccggcgtgattgcgggtattcaccggtatttaattgatatcggcggcgtgacggcgatcccctgctttatcaccagcattctggcgggttgtatatcgggctggatcaacctgaaaatccccaaagcacagcgctggcgcgtcggtattctcggcggcatgttgtgtgagacgttgaccatgattctggtaattgtctgggcaccaactaccgcgttggggatcgatatcgtctctaaaatcggcattccaatgatcctcggtagcgtctgtatcggctttattgtgcttctggtgcaaagcgttgagggcgaaaaagaggccagcgccgcgcggcaggccaagctggcgctggatatcgccaacaaaacgctaccgctgtttcgccatgtcaatagcgagtcattacgcaaggtctgcgaaattatccgcgatgacattcacgccgatgcggtggcgattactaataccgatcatgtgctggcctatgttggcgtgggtgaacataactatcagaatggcgatgacttcattagcccgactacccgtcaggcgatgaattacggaaaaatcatcattaaaaacaatgatgaagcccaccgcacaccagagattcattccatgctggtgatcccattgtgggagaaaggggtcgtgaccggaacgctgaaaatttactactgccacgcgcatcagatcacctcgtcattacaggaaatggcggtcggtctgtcgcaaatcatctccacgcaactggaggtttcacgcgccgagcagctacgtgaaatggcaaataaggcagagcttcgcgccctgcaaagcaaaattaatccccattttctgtttaacgctctgaacgctatttcatcgtcaatccgtctgaatccggataccgctcgccagttgatctttaatctgtcgcgttatctgcgctataacattgaattaaaagacgatgagcaaatcgatatcaaaaaagagctgtatcaaattaaagactatattgccattgagcaggcccgctttggtgacaagctgacggttatctatgatattgatgaagaggtgaattgctgcattcccagcctgctgatccagccgttggtggagaacgccattgtccacggtattcagccttgcaaaggtaaaggcgttgtcaccatcagcgttgcagagtgcggaaatcgggtacgcattgcggtgcgagataccgggcacggcatcgatccaaaggtgattgagcgggtcgaagcgaatgaaatgccgggcaataaaattggcctgctgaatgtccatcatcgcgtgaagttattgtatggcgaggggctgcatatccgccgcctggagccggggacggaaattgcgttttacattcctaaccaacgcaccccagtcgcctcacaggctacgttattgctttgagccggagtgatattgtgaaagtcatcattgttgaagacgaattcctggcacaacaggaactgagctggctaattaaagagcacagccagatggagattgtcggcacctttgacgacggtctggacgtgttgaagtttttgcagcataaccgcgtcgacgccatttttctggatatcaatattccgtcgctggatggcgtgttgctggcgcaaaacatcagccagttcgcccataaaccgtttattgtgttcatcaccgcgtggaaagaacatgcggtagaagcgtttgaactggaggcgtttgactacattctcaaaccgtatcaggagtcacgtattaccgggatgctgcaaaaactggaagcggcctggcaacaacagcagaccagcagtacgcctgccgcgacggtaacgcgtgagaatgacaccattaatctggtgaaagatgagcgaataatcgtcacgccaattaacgatatctattacgccgaagcgcacgagaaaatgacctttgtctatacgcggcgtgaatcctacgtaatgccgatgaacattaccgaattttgcagcaaactgccgccgtcgcattttttccgctgccatcgctcattttgtgtcaatctgaacaaaatacgcgaaatcgaaccgtggtttaataacacctacattctgcgactgaaagatctggattttgaagtgccggtcagccgcagcaaagtgaaagaatttcgccagttaatgcatctttaatcgggaactttcatgaaagcaccaggcttgcccgccgatcaacaatttttcgccgatctgttcagcggcctggtgcttaacccgcaactactggggcgcgtctggtttgccagccagcctgcctcgttgccggtgggcagtttatgtattgattttccccgtctggatatcgtgctgcgcggcgaatacggcaatctgctggaagcaaagcagcaacgtttggtggaaggagaaatgctgtttattccggcgcgcgcggctaatttaccggtcaacaacaaaccggtgatgctgttaagcctggtgttcgctccgacctggcttgggttatcgttttacgatagccgcaccacgtcgttgttgcatcctgctcgccagatccagcttcccagcctgcaacgcggtgaaggtgaagcgatgcttaccgccctcacccatcttagccgttcgccgctggagcaaaatatcattcagccgctggtgttaagtttgctgcatctttgccgtagcgtggtgaatatgccgccgggcaattcgcagccgcgcggcgattttctctatcacagcatttgtaactgggttcaggataattatgcccagccgctcacccgcgagagcgtggcgcagttttttaatatcacgcccaatcatctgtcaaaactgtttgctcagcatggaacgatgcgttttatcgagtatgtgcgttgggtgcgaatggcgaaggcgaggatgattttgcagaaatatcatctgtcaattcatgaagtggcacagcgttgcggttttccggatagcgactatttttgtcgcgttttccggcgtcagtttggtctgacgccgggagagtacagcgcccgttttcagggctaacgtcagaaggttaattctgtttccagcagcgtcaggatactttgtgcatcttgcgcggcaaacaacgactggcggaagtttttattcaccagtttacgcgccagctgcgagaagactttcacatgattcatcccttcgttagcacccagcgtcagcatgatcaccagttcgacttcgcccatttctgactgccagccaatcggtttcgccagccgggcaatgctgatactggaatgacggatccactgagatttggtgtgcgggatcgctacgccaaaaccaacgccggtggtaacaatctcttcccgctgccagacatcttcttccagctcaaacggatgttcagtgcgcccgttaacgccgaggttgccgcacaggaactggatcgcctgctctttattgctaaaatcctgatcaacaaagatattctccagcgccagcagtgggcgaacgtcttcttccggcgtaaaggcggtgagtaacgcttcaatttcctgcgcactgcggcattcacatgcctgacgcgccagttcccgacacgcctcgctatccagttgacgaagctggcttttcaccgccggaatacgcgggctactcatactcagctcatccaggcccagcccaagcagtagcggcagataacggctttcaccgcccagttcaccgcaaatgcctacccatttgccccgctgatgcgcagtggtaactatttgctgcaacatgcgcaggaacgatggcgtaatcgggttatatagcggcgatacgcgcgggttattacgatcgaccgcatacagatactgggtcatatcgttggagccgatactgaagaaatcgacctcatcgcagaagtggtcgatgatgtagcacaccgacggaacttccaccatgatcccaagcgtaatcgtctctgcatgacgcaggccatcgcgcttaagctcaacgatcgctttttggatctcgcctttcacccataagatctgatcgaggctgtgaaccatcgggatcatcaactgggcgttgccgaaactggcggcgcgcaaaatggcccgcagttgagtgcggaacaggccagcaaattccgggtaaatacgtaccgcgcgatagccgaggaacgggttctcttcctggggaatattcagataaggaatgcttttatcgccgccgatgtccatcgtgcggaagataatcggcttgtcgcccgccgccagtagcacctgctggtaggcttcaaattgctcctgctcgtccggcgcgctgtcgcgatccatatagagcatttcggtacggaacagcccgacaccttccgcgccgttggcaaacgcgcctggcgcttccagagcggtgccgatattcgccgcaatatcaatacgcttgttatcacgggaataggccagctgcgcggcagcctgcgcctgttgtttttggcgtttatccgccagcgtctgcgcgacctgataataaccgctcaccgcgtcattcgggttaatcgccagcacgccgcactgggcgtcaagcactgcaggttgcccggcataacgggcaatcgcatccagcggcaagccactcagtaccgggatcgccgaggcacgggccagaatcagtgtatgcgaggtgcgcccggttttctccagaatcatgcccgcaagatttttcaaatcaaggctcaaaaactggcttggggttaaatcttcagccaccagaatggtcggtttttcaagcaccagcttgttgcgcggcttcagttccggccaggtgatatgcagcaactgttcgctgatatcgcgaatgtcgctaacacgttcgcgcagataatcgctggcagaggcagaaagtttggcgcaaacctgctccatattgctgatgatcgccgcccccagcccctgatgctgttctgtcatcaggcgacggatattgcctgcaaattcatcatcctgaatcagcgacaaatgggcgctgaggatagttttgctttcgccgtcacgctcacgcaattgctggttcagttgctcggcaagcgttgccaggctgtgctccagccgggtggaatcttgcgcactggcggggattgcccgataactgtcgaggctgtcgctttgtaacagggtcagcgtacccacgccgacgccgcttgccagcacattgccgtacagtaaatccgggttaaggcggcttaatgaacgcggcagcggatgcgccgtcagttctgcctgcgtaggctgaacgctgtcgctgtcgataaagcgcacctggatgtactcttccagcacgcgccgcgcctgctcttcatcgctgccgctaatgttcaggctgcaactgtcattaaatagggtgccggtgccaatcagcgccagcgagcttttcgcatctgcctttgcgttctggcgatggttaataaaagtgatttcgctttgccactggctgcactgttctttaagttcccacgccggacgagcatgtagaccgttaggcaaaggacagagaaattgaatcgttaacataaccgctccgggttaatcaggagatcatctgaaatccgtcagttgaacaaccgtctcacgcgtaagacgttgaataagggcagataaaagttgctgcatctgcaaaatgtcgcggcaatcggcaatcgatgcggcgcaatgtccatggcgggttgctggccccatcaccactgtgggcacgccggtgccggttaagtgcaccgccccgccgtccgtgccgccgttgctgaacatatctgcctgcaacggcacgccaatttctgccgccacggtttcgacccaggcggtaagttttggcggcgcaatcagcgacttgtcgcttaacaccagcatcggcccgttaccaatctggcgatggttagccgcgccataatcaaagtttttcgcccagcaggcggtatcaagcacaatggcgacgtccggcgacaccgcgcgggtggcagtttgcccgccgcgtaatcccacctcttcgctggaacttgccaccagccacacttccgcaggtagttcggcgtcgtgcagttcgcgcagtaacgtcaccagcagatagcaaccgaggcggtcatcaaaggctttccccatcactcgctggtgagggagaacctgaaaagtggtatcaaacgtgacgcgatcgccgggacgaattcccgcctgcatcacttcgtcataggagcgcgcaccaatgtccacgcgcatggcgctgacgtcattcccctgccggtcgccgtcaagcaggcctggaattttgcactcttcacgggtggtgatgcgcaccggctgcagctggcgggcagccatgcgtacgttgccaaccggcagcacatcaatcgccccttcgcgggagatgctgcgcaccataaatcccacttcgtccatatgcgcacagatcatcaccttcggacctgtcgattcattcaggcggatcagcaccgatcccagaccatcaaatcgcacttctttttgcaggcgatccgcttcttccagcaggatctgccgcacttcctgttccgaggaggcgatcgcatctgcctcgctcaacgcttttaatagcgataaatccattatgcctctcccgtgagcaacactgttttcggcatggcgtagagcacttctgcgccttgcggggtaaccagcacaacatcttcgatgcgcacgcccccttgccctggcaaataaatccccggctccacggtcagtaacatgcctggctgtagcgtcgtggtgtcccgcggtgaaaaacgcggatcttcatgaacttcaatgccgatagcgtgaccggtgttatgaccgaaatagtcgccataacctgcttctgtaatgacccggcgcgcggcatcgtcaacctgctggcagcgcacgccggggcgaatcgcggagattgctgcgagctgtgcctgcaggacaatttgatagacgttaaacagcaggtgagattcggcgctcaccccttcgccattcaccagcaaggtgcgcgtcatatcagagcagtagccctgatacagcgcaccgaaatcgagagtgacaaactcgcccgctgcaacaatcttgtcgctggctttgccgtgcggcagcgccccacgccagccactggcgacaatggtgtcaaaagaggctttttctgcgccctgctggcgcataaaccactccagttcagcggctatctcgcgctcgctcatccccgcctgaataaagcggcgaatatgctctgcaccgcgatcagcaatcccacaggcgaggcggattttctccacctcctctggcgttttgatttgccgcagcacatccggcgtggcgctaaccagtttcgcattgagttcagactgccagcggtgcgcggtttcccaactcacctgctggccctcaaaaccgagcgtttgcaactgttcatcggcaatgatttgattgacgatagtggtaagcgtgttcgtcgcgtcaagcaaatgcagctggtagccttgcgcacgggcttccacctcaacgtaatagcgcgaatccaccagaatgtgcgcactttcacggctaatcaccacataacctgatccggtggagatccccagatgcggctgtttgttctgccgtgaggagagaagcactgcatccagttgttgcgccttaagccagtcgcgcagcgaagcgagtaatgtcatctggattttccttcttacaggctatcgattaacaatttgcctttacggaacatcatcagacgcaggaacaccaccatcagcgcagttatgactgcccccagcgcgatccccgccatatagacgcccaggttagtgaccagcggccatgcccagatagcggactccgggaaccattgcactgcgcccagccagacagcggcggttgagccgacaatagcgccgaccatatacgacggaatggcggtgatggggctttccagcgcaaacggaatcgcaccctcactgatccccataaacgccaggaacatggcggtcttaccctgcggataaagttgagcgttgaacaggcgtttgccggttaaacgacggtcgataatggtcgccagccccagaccaatcggcggaataacgatagcgatagaacgagcggtgaccggtaatacgtggtcagtggtaaagctgaaggcaacaaaacctgcggctttgttgatcgggccaccaaggtcgattgctgtcgccgcggcgatccccattgcgtacatcagcgcgcccttctcacctgcggcagtcagcacagtacggataccgccgttgatccagccaccaaagggggtgatgacgtagtacatcgccagcatgacaaaaatggcggaaagaatcgggagcaaaaatgtggttttgaacgctaacaggaaatccggtaactggattttctggttcatccacttcacaaggtaaccggcaacgatagaaataatcagcgcaccaatgaaggtggacggcaccggcgaagaggtcgcccattgcatagtgctgggatcgaagttcagcagttgcgtcggctgggtagacatcaacccgccgataaaaccagccgggaacgccagtttgccaccgatagagttcgccacaaaagcagcaaacatcggaatggcaaaaccaaacaacacgccgccgaaggactgcgacagccaggcaaatttaagtaaggagaggtcgaaaccggagaatttcccgctattaagagcatccatgatgccgatctcagcaggaattttaagccagctataagcaatcagctggctgaaagcgaggatcacaccgcccataattaaggtcggcaccatgcgtgaaatccctgacatcacatgctgcgggagttcaccccagaagctggttttagaggcctgcggattcttaactgccgctgccgcaccggatgcgccaggcacaacggttgcactgcgttttttaatggccataacaattatccctgtcgaatattactgttgttcagaggcaatcatctcttcgatttctttgatgatgcccgcagcgtttttaattgcgtcctgcaaagtgatttcataaacgtcgcgtgattcgaaacgttcgttatcttccggggtaactgccacggagtggatgatgatggtcgcttcggcgatatcctgcgccgtcaggcgattctggataccgtccgcgccctgggtttcaattttcacttcataaccggcttctaccgccgcttcttccagcgcctgagcggccataaaggtgtgagccaggcccatcgggcaggcacataaggcaatcagtttcttactcatcgttaattcctcgttcagtgatagttgacgagtgaaattatgaacgtgcaaaacaaatcgccgttaccagacaaataatgcatttactggagaattaatcccgctgtacggaagtgtgacgcaggtcgaccttgtgaggggacacaaagaaaaattgaataaactgtatgatttaaaagattatcgggagagttacctcccgatataaaaggaaggatttacagaatgtgacctaaggtctggcgtaaatgtgcaccggaaccgagaaggcccggattgtcatggacgatgagatacaccggaatatcatggacatattctttaaagcgccctttatcttcaaatgcggcacggaaaccggaggctttgaagaactcaaggaagcgcggcacgataccgcccgcaataaacacgccgccaaatgtcccgagattgagcgccagattgccgccaaaacggcccataatgacgcaaaacagcgacaatgcgcggcggcaatcggtgcagctgtcagccagcgcgcgttcggtaatatcttttggcttgagattttctggcaggcggttgtcagctttcacaattgcgcgatacaaattcaccagcccagggccagaaagcacgcgctccgccgaaacatgaccaatttccgcacgcaatatttcgaggataatggcctcttcttcactattcggcgcaaaatcaacgtgaccgccttcgcctggcaagcttacccaacgcttatcgacatggaccagatgcgcaaccccaagccccgttccggcaccgtaaaccgcaataggcttaccttcgaccggttctgcgccaccaaactgaatcagatgctcttttttcagcatcgggatcgccatcgatacagcggtaaaatcgttaataatttccagatggctaaaaccgagattctttttcatttcggcaattgagaacgcccaggtatggttggtcatcgccacccagtcaccggtaattgggcaagcgatggcaatacagccgtctttcacctcgaccttatgttcttcaagataaacgcgaatgaccgcttcgaggctggggtaatcaagccctgaataggtcttagcctgcgagatttcaccactggcaatatcacacagagcaagacgtgcgttggtgccgcccacatcaccgactaatgcatactttgtcattcttcaactgctccgctaaagtcaaaataattctttctcacactgtaaatacctgggggcataacaacaacgccggaaaggcaggctccctgtaaatatcgatctgggtcacacaattactttatcgtttcagcaccaattgcagcgatgcctttttgcaagctgggcaaactaagtatctgaccccgcataaggaatagaacatgctccatccgcgagccagaaccatgttgttattatcgctccccgccgtggcaattgggattgcgtccagtcttattctgattgtggtgatgaaaatcgcctcggtattacagaatttgctctggcaacgactgccgggaactctggggatagcccaggattcacccctctggatcatcggtgtattaacgctaacgggtattgcggtggggttggttatccgtttcagccagggtcatgccggaccagaccccgcctgtgaaccgctgatcggcgcaccggttccgccctctgcgctacctggacttatcgtagcattaattctcggtcttgctggcggcgtcagcctggggccggaacatccgatcatgaccgtcaatatcgcccttgcggttgccattggcgctcgtctgttaccgcgcgtcaaccgaatggagtggactattttagcctctgccggaaccatcggcgcactgtttggcactcctgttgcggcggcgttgatattttcgcaaaccttaaatggcagtagtgaagttccgctatgggatcgtctctttgcgccgttaatggcggcagcagctggtgcacttactaccggattatttttccatcctcatttttcactgcccattgctcattacggacagatggaaatgaccgatattctcagcggtgcaattgtcgcggcgattgccatcgcagcagggatggtcgccgtatggtgcttaccacggttgcacgcgatgatgcatcaaatgaaaaatccggtgctcgtgctgggtattggcggatttattctcggtattctgggggttattggtggaccagtttcgctgtttaaagggctggatgagatgcagcagatggtggcaaatcaggctttcagcaccagcgattactttttgctggcggtaattaaacttgccgccctggtcgttgctgccgccagtggctttcgcggtgggcgaatcttcccggcagtgtttgtcggcgtggcattagggttgatgctgcatgagcacgttcccgccgtaccagcggcaataaccgtttcttgcgctattctcggcatcgtgctggtggtaacacgcgatggctggttaagtctttttatggcggcagtcgttgtacccaataccacattgctaccgctgctctgtatcgtcatgcttccggcatggctgttattagcaggtaagccgatgatgatggtcaatcgtccgaagcaacagccaccccacgataacgtttagcaaaaaatgctctcctttatgatttaagagttatggcgatgatacggggctttacctccccgtaatattgcgttaacaggccgctgacggcttcgagcgtgaaggagaataacaatgttcaggtcactgtttctggcggccgccctgatggcatttaccccgcttgcagcaaacgcaggtgaaatcaccctactgccatcaatcaaattacaaattggcgatcgcgatcattacggtaattactgggacggtggtcactggcgcgaccgtgactactggcatcgcaattatgagtggcgcaaaaaccgttggtggcgtcatgataatggctaccaccgtggctgggataagcgtaaagcgtatgagcgtggctatcgtgaaggctggcgcgatcgtgacgatcatcgcggaaaaggccggggtcatgggcaccgccattaaacgcgtccgccaatggagcacaatgcctgatgcgacgctagtgcgtcttatcaggcctacaaaccggctctttaacgcgtagggcggataaggcgtttacgccgcatccgccaatagtgccagatgcgacgctcattcaactacaatcccagcgccgtccccaccaacaaccagatattcagcgccacgaccagcaccacaatcacccagcctgtctgttttacgcgtttgctgttcaccagatcgcccatcaacttgctgtcactggtgaaaatcagcagtggaaccagcgccagagcgataccaaaacttaacagtacctgactcataaccagaatccgtgtcggatctaatcccatcagaatgacaataaatgacggcaacatggtgactgtacgacgcacccacagcgggatatgaaagcgaatgaagccctgcatcaccacctgccccgccagtgtccccaccaccgttgaagacagccccgcagcaaccaggcttaatccaaagaccgttgccgcagcgtggcttaacagcggttgcagcgtcagataagcctcatcaagatcggcaacaccagtatgaccggaaaagtggaacgccgccgcagctgtagccatcatcgccagattgacaaaaccggcaatagtcatggcgatagccacatcccatttggtggcggaataacgttgttgacgcgaaccgccatgtaaatgctgagtgagcgaggagtgcaaataaatcacatgcggcataatcgtcgcccctaacacgcctgctgccaggaagaccgcttccgaagtaggtaaactcgggatcaccattcctttacccagctgcgccaggttaggctgggagaaaatcaactcgacaatgtaagccgcggcaacaaacaacagtaacccgccaatcactttctccagcggtttttgcccgcgacgttgcagcattaaaatcaggaaagtcgcgatccccgtcagcaccgcgccctgcaacaacgaaacaccaagaatgagtttaaaaccgatcgccgcaccaataaattccgccaggtcggttgccatcgcaataatttctgcctgaacccaatagaaccacactacgggacgcggatagtgatcgcgaatctgctccgccagatttttaccggtggcaatccctagtttggcagagaggatctgaatcagcatcgccatcaggttggcccaaacgacaacccacagtagctgatagccgaagctagcacccgcctgaatattggtcgcaaagttaccgggatcgatataaccaatcgccgcaatgaacgcaggtcccattaatgcgagcctcatcttgcgcgccgcccgtccgctgctactctcaacgcgatagttcgtcatcttgtgcctctaaaacatagcctttgctatgtttcatgctatgccaaacgagaatgattatcaaattcatttaaatggattgtggtgatttctctgatagaccaggattatgactacgaaaagattgatgacttgaatgttatggttatgtttaatgttagcacatttacataactttcagcttccatacacaacatagcagaaatgtatgacagatcactatttttgaagcctgtcacaggacgtcattatagtgtgtgtcagatctcgttttccttaaccatgttacatagaatgtgcacggaaatttaacctgcctcatatttggagcaaatatggaccgcgtccttcattttgtactggcacttgccgttgttgcgattctcgcactgctggtaagcagcgaccgcaaaaaaattcgtatccgttatgttattcaactgcttgttatcgaagtgttactggcgtggttcttcctgaactccgacgttggtttaggcttcgtgaaaggcttctccgaaatgttcgaaaaactgctcggatttgccaacgaagggactaacttcgtctttggtagcatgaatgatcaaggcctggcattcttcttcctgaaagtgctgtgcccaatcgtctttatctctgcactgatcggtattctccagcacattcgcgtgttgccggtgatcatccgcgcaattggtttcctgctctccaaagtcaacggcatgggcaaactggaatcctttaacgccgtcagctccctgattctgggtcagtctgaaaactttattgcctataaagatatcctcggcaaaatctcccgtaatcgtatgtacaccatggctgccacggcaatgtccaccgtgtcgatgtccatcgttggtgcatacatgaccatgctggaaccgaaatacgtcgttgctgcgctggtactgaacatgttcagcacctttatcgtgctgtcgctgatcaatccttaccgtgttgatgccagtgaagaaaacatccagatgtccaacctgcacgaaggtcagagcttcttcgaaatgctgggtgaatacattctggcaggtttcaaagttgccattatcgttgccgcgatgctgattggctttatcgccctgatcgccgcgctgaacgcactgtttgccaccgttactggctggtttggctacagcatctccttccagggcatcctgggctacatcttctatccgattgcatgggtgatgggtgttccttccagtgaagcactgcaagtgggcagtatcatggcgaccaaactggtttccaacgagttcgttgcgatgatggatctgcagaaaattgcttccacgctctctccgcgtgctgaaggcatcatctctgtgttcctggtttccttcgctaacttctcttcaatcgggattatcgcaggtgcagttaaaggcctgaatgaagagcaaggtaacgtggtttctcgcttcggtctgaagctggtttacggctctaccctggtgagtgtgctgtctgcgtcaatcgcagcactggtgctgtaagaccatacataaaaaagccggggataattcccataagcgctaacttaagggttgtggtattacgcctgatatgatttaacgtgccgatgaattactctcacgataactggtcagcaattctggcccatattggtaagcccgaagaactggatacttcggcacgtaatgccggggctctaacccgccgccgcgaaattcgtgatgctgcaactctgctacgtctggggctggcttacggccccggggggatgtcattacgtgaagtcactgcatgggctcagctccatgacgttgcaacattatctgacgtggctctcctgaagcggctgcggaatgccgccgactggtttggcatacttgccgcacaaacacttgctgtacgcgccgcagttacgggttgtacaagcggaaagagattgcgtcttgtcgatggaacagcaatcagtgcgcccgggggcggcagcgctgaatggcgactacatatgggatatgatcctcatacctgtcagttcactgattttgagctaaccgacagcagagacgctgaacggctggaccgatttgcgcaaacggcagacgagatacgcattgctgaccggggattcggttcgcgtcccgaatgtatccgctcacttgcttttggagaagctgattatatcgtccgggttcactggcgaggattgcgctggttaactgcagaaggaatgcgctttgacatgatgggttttctgcgcgggctggattgcggtaagaacggtgaaaccactgtaatgataggcaattcaggtaataaaaaagccggagctccctttccggcacgtctcattgccgtatcacttcctcccgaaaaagcattaatcagtaaaacccgactgctcagcgagaatcgtcgaaaaggacgagtagttcaggcggaaacgctggaagcagcgggccatgtgctattgctaacatcattaccggaagatgaatattcagcagagcaagtggctgattgttaccgtctgcgatggcaaattgaactggcttttaagcggctcaaaagtttgctgcacctggatgctttgcgtgcaaaggaacctgaactcgcgaaagcgtggatatttgctaatctactcgccgcatttttaattgacgacataatccagccatcgctggatttcccccccagaagtgccggatccgaaaagaagaactaactcgttgtggagaataacaaaaatggtcatctggagcttacaggtggccattcgtgggacagtatccctgacagcctacaaaacgcaattgaagaacgcgaggcatcgtcttaacgaggcaccgaggcgtcgcattcttcagatggttcaacccttaagttagcgcttatgggataattccccggtttttttacgcctgttaatcagctaatggctgcgggcgaccaatcaaatacccttgcagatattgcaccccgagcttatgcaatagcgcctgctgctgttgcgtctcgacaaactccgcgaccacactcaatgacttcgctttcgccagatcggtaattgatctcacaatcatcgcatccagcgtgttcgtgacaatatctttcacaaagacgccatcaattttgatgatatcagcctgcaaacgctttaaccgttcgtagttggcatatccggtgccaaagtcatcaatcgcaatccggaaaccaaacttatgcagctgctcgatgttgtacatgctgctttctgcgttagaaaacgcctgctcctcggtgatctcaagaatgaccgcctgcggggagatgtgataacgcttaaacagacgaataatccgcccggcaatattcttttgcagcagcgtgagcggcattaaattgactgaaaagcgcggtccttttttgtcgcaagggtgtgttgccagccacttcaacaaggattccagcacttgcaaatcaaaacgcgcgctaaggttaaactgagcaataaggggcagaaacttatccggggtcataatgccgccgtcatatttcagtcgcgcgaggatctcatcataaccttcaccctctttgttgcgaattggctgggcgtagagcagcaaatcaccctgatctaacgccgtgcgaatggtattcagcaatagcacctgtttagtggtctgcccggaaaccatctcctctctgctatccagcgccagcacatgatgatgtgcgcaggattgctccgccagccagcttaactgccccaacaagggttgcagggtttcctgatttccatcaaaacgcccccaggcagcaccatagcccatatccagcccggtattgttccagtgaatttgccgactattcaggatgttaaccatatgctggagtcgcccttccgtttccggcccgctcagcactaacagcagttcactacccggcaattgatacaacttttcgttttcctgcatcaacggcagcagcgtacggcaaattgagcggatacagtgaacgcgcatcattaagccgtaatgacgactcataaactcaagattatcaatgcgcaggcagcaaaaactcttgcccgcctcttgctccggcgcttgttccaacgcacgaaagttgggtaggagcgttaacggatctgtcagcgcctgcaaatgccagcggcgattaagccattcactgcgatgataaatgcgcaccatatagagcaggcaaacgctaaaggaaatcagcaccgcaagaataaatgccagcgaatattcggtttccaccccttgcaaaaagttctggttgtaattcagaaggcaaagcgttgaaacagcccaggtgagatttaaaaacggatagcgaagcttaccgaccccgagggtaaagatgatgaagaaaacgggtaccaggtaaccggcaataaagtcgttttcataaggtgtgcacaacagaagtagcagcacgcttaacgctgccagccagcttaaggtaaatgcgcgtttctctttgcccaacgacggagcgatatccctgcgccacaatatctgcgcaaagtggggacttacaatcatgcgagtgagatagtagaaaagcatgttgtaaatcagcacagcggtgaaaaggcttagcaaatcaacgaccgtgaaaatggcatccgcatcgccgaaaaaggtggatatctttagcgggaaatcaaagaagctccccacaagatacatgctgcatttgatgccgatcggcgtcaccaaaccaagccagaacagacgttgccagacatatcggctggtcaatccataacgccaacgcgtccccagctgccagcgtaatattgcgcaggcacacaacacgacaaacgtctggctaccgagcatgaccgcagtctgtaaaaaagagagatgaaagttccacagattggtgcaaaacatcccgcataaaacgggaacgacaccgcgccagccaaagataaacaagattgacagcattacgcacagtggcatccacgccagaaagatataactggaatggataatggcaagtggcgaaataaaacgggatagctgaataagtaccacggtgagcgtaaacgctagtgtgaatatcttgatattttttatcaggttatgctccacaaacatgagtacactactctcactgatcggggttttcaggcacacaaataataagtttattcgcatcgcgaagcaaacagggggccagcctgttgccgatttttcatccaatgatgctttcaccaggcggcactaacccggacgtagactgtattacaaaagcggcaaaaagcagagacaaaaaacccccgctttgcagcgagggttggaaatttggtggagctaagcgggatcgaaccgctgacctcttgcatgccatgcaagcgctctcccagctgagctatagccccacgatgcgtttacgtaccaagtttgctgggtgcaaaatttggtggagctaagcgggatcgaaccgctgacctcttgcatgccatgcaagcgctctcccagctgagctatagccccgtcacgtaaagcttgtcgagttgacgggcggcatcatatgaattccgcccgaatgtgtcaacggcaaattgcaacgtgtagtttcaatcgctgaaaaatcaggcaaatgaacaattttggaaaaccgctcgcattcagtagttattcatgtcacggtttcctgtaaagtggtgttataaaatgaactactaatagacccacatacattcagggaattgttatgttcaaggagaggatgacaccagatgaacttgccagactgaccggctatagccgccagaccattaataaatgggtacgcaaggaaggctggacaacgtcaccaaaacctggcgtccagggtggcaaagcccgactggttcacgtcaatgaacaggttcgtgaatatattcgcaatgctgaacgtccagaaggtcagggagaagcgcctgccctttctggtgatgcgccgcttgaagtattgctggtgacactggcgaaagagatgacgccagttgaacaaaaacagtttacatccttgcttctgcgggaagggattatcggattgttacaacgcttagggattcgcgatagcaaataatatgaaaagattacgcaataaaatgaccaccgaagaactggctgaatgcctcggtgtggctaaacaaactgttaaccgttggatcagagaaaaaggctggaaaacggaaaaatttcccggcgtgaaaggcggtcgtgccagacttattctggtcgatacgcaagtttgcgagtttattcagaacacgccagccttccataacacaccaatgttgatggaagctgaagagagaattgctgaatacgctcctggagcacgcgccccggcgtatcgacaaatcatcaacgcgatagataatatgacagacattgagcaggaaaaagtcgcgcaatttttgtcacgtgaaggaattcgcaatttcctcgcccgtctcgatattgacgaatcagcataaataaaaaacggcaggatattatctcctgccgtttatctttttacacgctaattactgctgattttcgcgttcagcaataaaatccagcgctttgttgatacgctcgatactgcgggtcttaccaattgcgtgaacggtaacatccagtgctggagactgccccgcaccggttacggcgacacgcagcggcataccaactttacccatacccacttccagctcatccgccgtcgcctgaatagcgtgatgaacgttttcagcggtccagtcagtaatcgcggccagtttgtcacgaaccacttccagcggctgacgcgctaccggacgcagatgttttttcgcggcgtcggcatcgaactcagcaaaatcttcgtagaaataacggcagctctgtgccatctctttcagcgtcttgcagcgttcgcccagcagtttcaccagatcagccagctgcgggccgttacgggtatcgatattttcctgctcaatgtgccactgtaagtgagtagcaacatactccggcggcagcgcgttaatgtagtgatggttcagccacagcagcttgtcggtgttgaacgcactggcagatttgctgacggcattcaaagtgaagtatttgatcatctcttcacgagtgaagatttcctgatcgccgtgggaccagcccagacgcaccagatagttcagcagtgcttctggcaaataaccgtcatcacgatactgcattacgctgactgccccgtgacgtttggacagttttttaccgtcatcgccattgatcatagaaacgtgcgcgtaaaccggcaccggcgctttcagggccttaagaatgttgatctggcgtggcgtgttgttgatatggtcttcgccacggataacgtgggtgatttccatatcccagtcatcgacaaccacacagaagttataggttggggaaccatcggtacggcggataataagatcgtccagttcctggttgctgaactcgatcggaccacggatctgatcgtcaaaaacaacagaaccttcctgcgggttagcaaaacgtacaacacacggttcatcatcagcatgatgctcatggctgtggcggcagcgaccgtcataacgcggcttctcacctttcgccatttgctcttcgcgcagcgcttccaggcgctctttagagcaatagcatttataagcagtgccctcttccagcatctgatcgatcaccgcgttgtagcgatcaaaacgtttggtctggtagtacggaccttcatcccactccaggctcagccagttcatgccatccataatggcttcgatagcttccggcgtggaacgctcaagatcggtgtcttcaatacgcagcacgaactcaccgccgtggttacgtgcaaaaagccaggagtaaagagcagtacgcgcgccgccaacgtgcagatagcctgttgggcttggcgcgaagcgagttttgattttcatgaaatggccttacgtttagaaagatgccgacaaccggcaaatcctggaaaaattaagtgggcgatattctatcactcccgcctgattcctcaatgtagttcgggtttctaccttacgcattattgttttcgttgacaaattgcgcaacacggtctgttttgcgatcatcttgcttaaatttacgacgaacgaacaatttctttagaaaatgcgttgactcattttgaactctccctataatgcgactccacacagcgggggtgattagctcagctgggagagcacctcccttacaaggagggggtcggcggttcgatcccgtcatcacccaccaactactttatgtagtctccgccgtgtagcaagaaattgagaagtgggtgattagctcagctgggagagcacctcccttacaaggagggggtcggcggttcgatcccgtcatcacccaccactttctcgccagctaaatttcttgtaaaaatgtgaagtaccgaagtgggtgattagctcagctgggagagcacctcccttacaaggagggggtcggcggttcgatcccgtcatcacccaccacttcgggtcgttagctcagttggtagagcagttgacttttaatcaattggtcgcaggttcgaatcctgcacgacccaccaatgtaaaaaagcgccctaaaggcgcttttttactatctgcgatactcaaagattcgaacctgcagcaggtttgagttgagcgcagcgaaacaacggagccgctcgcggcgacggcccgaagggcgagcgaagcgagtcatcctgcacgacccaccaatgtaaaaaagcgccctaaaggcgcttttttgctatctgcgatttgcgaaattgcctgatgcgcttcacttagcagactactatttccggcaattcctgtctcctcacctactgtgtcaatgcagccaacagcttaaccatcgcgggcgtcacctgctgtgtttcataaacaatatataaatctgcagggatgcgctgtttgagcggacggaaaatgacacctggccagttcatttgtgcgtagctgtccgctatcaatgtgataccaatgcccatactgaccatagcgagtaccgtttgcggttcattaacttcgcgaataacaaccggtgaaaatcccacctgctggcaaactcgctgcaaaaaatcccagtcagtgtaaacgggcggcattgtaacaaaatactcgtcacgtagcgcttccagcgggacggtggaaaatgatgagagatgatgctcttcaggcatcgccaccagaaacgccgattcatgcaaccgtaagctggtaaaaccagtcggtggttctgtcgccattcgccagatcccggcatcaagttcgcggcgttccagcaaggccatttgcatcgcgggcatcttttcgcgaaaaagaacgtcaacgttaggattttccctgaggaatcgccgcataaccgggcgcatccgtccccacattgccgttcccactacgccgagttcaatccgccctgcttctccccgacctatttgttcaatccgagccaatacattattagcattcaccagcaatcgacgcgattcttccatcaagattttgcccgcgtgtgtcagtacgacgctgcgcgaatggcgaataaaaagctgcgtgccgagttgattttccagctctttaatatgaatgctgagcggaggctgagacatatttaaacgcgctgctgcgcggccaaaatgcaactcttccgctacggcaagaaaataacggagcaacttaagatctgttctgtatacgcgttccataattaagtgctccatataataaatacatcgtattaaattatcatggcataaagtatttcaccaccagatatccgacatacataaacacaatggataatatacccggtaatacatttggtacaggaataggcaagcgcacgattgtaaacaaagcaccaataccaaaaccaacgccggaagaaaataaaatatctttcactaattaacctttatcataaaagcagctctgaagagcagagccgcgaatccttttaatgagtcaccgctcgatgctttatcttttcagggtcatgattatatttaaacccaaagaaaaatatcactgcgagaaaaagagcatatcctgcaaacaccagccagatagtttgccagtcttttacgccatccaccgaaaagtaatctactgccatgccactcagaatcgagccaacccatgcgccgacaccatttaccatggtcataaagagcccctgcgcgctggcacgaatgctggaatcaacttcctgttcgacaaataccgaaccagaaatattgaagaaatcgaatgcacagccataaacaatcatcgacagcagcagcaaaataaatccggttgttgacggatcgccataggcgaagaagccaaagcgcagcgtccaggccaccatactcatcagcatgacggttttaatgccaaatcgctttaaaaagaatgggatagtcagtataaagcccacttctgccatctgtgaaactgacagtaaaatggagggatatttcaccacaaaactgtcagcaaactccgggttacgggcgaaatcatgtaggaacggattaccaaaaacgttggtaatttgcagtaccgcacccagcatcatggcaaagaggaaaaagatggccatgcgtggatttttaaacagcacgaaggcatccagacccagcttgctggcaagcgatgtggtcgcttttttctccgcaaccggaatcttcggcaaagtcagcgcataagccgacagcagcaatgacgcaccggacgcgatatacagctgcagactactcaattccagatgcagcaggcttactgcccacatcgcgacaatgaaccccaccgtaccaaaaacgcgaatgggcgggaaagcggtcaccgggtcaagccctgcctgggcaagacaggaataagagacgctgttcgataacgcaatagtcggcataaacgccatcgcattgactaacatcacccaaaacatcatatccggatcagttacggatgccgcataaaaaagtacgcccgcacacaccaggtgacacagcatgtatgcacgttctgcgcgcagccatttgtctgcgatgatccccattataccaggcataataatcgcggcgatccctttggaactgtaaaccatgccaacattagcgccggtgaaatgaagagtattaatcatgtaagagccgagggtaaccagccagctcccccagataaaatattgcaaaaaggacattacctttaagcgcatcgcgatgctcataatcgtttccttgtcgcatcatttggcctcacccgcgaggccgtttcttattgtttttctcaggcaattttgcgcagaaagccacaaataaggttgatgaagttctgcttagagagctccgcagccgccagcgtttgcgcatgtgacaatttcacatcgcttaaaccttccgccatattggtaatcgcagagaccgcaacgactttaaggtcgcaatggcgagctgaaataacctcaggcaccacagacataccaacaacatccccaccaataatttgcatcatgcgaatttccgccgcagtctcgaaattcggccccggatacgagacgaacacgccctccgtcagagggaaaccctcttctttcgccactttttgtaacagtgcgcggtattccgcatcgtaggcatttgccagtgagaagaagcgctctccaaaacgatcatcgttaagacccaccatcggcgtaccgggcatggtgttgatatgatctttcaatgcgaccaggctgcctgcccccacttccggacgcagcgagcctgccgcattggtgcagaacagtagctcgcagcccagcagcttaaaggtacgaattgcgtcagtcataatggtcattccacgaccttcgtagaaatgtccgcgacctttcatacataccaccggtacgccctggagatggcccagcactaactcccccgcatgaccatgtaccgtacttaccgggaagcccggcagcttttcgtaggaaattgcgacagcgttctcaatctgatcggccagcgcgccgagcccggaacctaaaataaaggccactcgtggcgtgaaatcaggtttataagtcttgataatatctatgcaaaacagcgggttatgagaaaattgaacctgagacatacatatcctttttctgtagggtggaatctaacgcctttttatagcgaggttgtcccggctcttaccaatacacttttctcacgcattcaatagcgattcgatatcgatggatttatatcttttctctattaatccacggtaaaaactgtattggcgatattaattcctttgcattaacaatatgtcgtttttagcaaaccactttattaagcaatctactaataacgatcggcatagggaattatgctatgaaaaaacatcttttaactctgacactttcctctatattagcgatacctgttgtatctcatgcagaatttaaaggcggttttgcagatatcggcgtgcattatctggactggaccagccggactaccgaaaaatcgtcgaccaaatcacacaaagatgattttggttatcttgaatttgaaggtggcgctaactttagttggggagaaatgtacgggttcttcgactgggaaaacttctataacggtcgccataataaaccaggtagcgagcagcgttatacctttaaaaataccaaccgtatttacctgggtgacaccggatttaatctctacttgcatgcgtatggcacctacggttctgcgaatcgcgtgaatttccacgacgatatgttcctgtacggtatcggctacaatttcaccggcagcggttggtggttcaaaccgttctttgctaagcgttatacagatcaaacctattacactggcgacaacggctatgtcgccggctgggttgcaggttacaactttatgctgggcagcgagaaattcactcttaccaactggaacgagtacgagtttgaccgtgacgctacctatgcagcgggtaatggcggtaaagaagggctgaatggcgcagttgcactgtggtggaatgcaacatcacacattactacggggattcagtatcgatatgcggatgacaaactgggcgaagatttttaccaggatgcgataatctactccatcaaatttaacttctgattgattactgccggggctcccggcagtatgaattcactctatatctgatacaacggatccccttcccgcccagccattagcgcattgccctggtctcgtaccacgtcccataaagcttcagcggcggtggaaagtgaacggttcttcctgcgcaccagcatcaactggcgttcaacaaccggcgtaatgcgctttaccaccagtgggctaccttcaggcaatggtagcgccagtgcgggaagaatactgatgccgatgcctgcggctaccatcgggaacagcgtcgccggatgtccaatctcctgcacaatattcgcctgaataccattgcgcgccagcgctgcgtcaatcagcggtcggctgcctgacgcgtaatcctgcaacaccaatttcgctccctgtaatgcctgccagggtacataatcttccacggccaaagcgctatcgcgatggcaaagcagaaagaaaggctcggaaagaatcgcttcacattgcagatcgcccactgggcctggatcgatgacgatgccaaaatcgacatctccctggcgaatactttccattacccactgctgcggacgatcgtgcaggacaaactgaatatctggatagcggcgatggctttcagcaatgcattgcggaataagatgcgcggaaatggtctggctggcagcgacccgaacttttccgctcagttgttgccccatacgcccggtatcgcgcaacgtgctgttcagttcatccagcagtcgctcaagacgcaaagccagctgctgccctgcatctgtaagcaccacttcacgcgtggttctgtccagcaggcgaacaccagtatgattttccagttccttcacactgtgactcactgccgactggctcaggccgatacgctctcctgcacgactaaaacttttctcctgcgctactgtgacgaaaacctttaattgttttaaagaataattcatctgttttcttcatgaatggatgcaataaatcaattttatttctcaaactggaagaagcacaatagaaccatcgatcatctggagtctttatgaaactttttcgtatcctcgatcctttcaccttaaccctgatcacggtggtgttgctggcctctttctttccggccagaggcgatttcgtccccttctttgaaaatctgaccaccgcagctattgccctgctgttctttatgcacggcgcgaagttgtcgcgtgaggcgattattgctggcggtggtcactggcgactgcatttgtgggtaatgtgcagcaccttcgtgctgtttccgattctgggtgtactgtttgcctggtggaaaccggtaaatgtcgacccgatgctctactccggttttctctacttgtgcattctcccggctaccgtgcagtctgcaatcgccttcacgtcaatggcgggcggtaacgtcgcggcagcggtttgttctgcgtcggcatccagcctgctggggattttcctttcaccattgctggttggtctggtgatgaatgttcacggtgcagggggcagccttgagcaggtcggtaaaattatgctgcaactgctgctgccgtttgtgttggggcatctttcccggccgtggattggtgactgggtgtcgcgcaataaaaaatggattgcgaaaactgaccagacgtccattctgttggtggtttatacagcgttcagcgaagccgtcgttaatggtatctggcataaagttggctggggatcattgctgtttatcgtggtggtcagctgcgttcttctggctatcgtgattgtagttaacgtctttatggcacgccgactgagcttcaataaggcagatgaaattactatcgtcttttgtggttcgaaaaagagtctggcaaatggcatcccgatggcaaacattctgttccccacatcggtgatcggtatgatggtgctgcccctgatgattttccatcagatccaattgatggtctgtgcggtgctggcgcgtcgatacaaacgccagaccgaacagttacaggcgcagcaggaaagcagcgccgataaagcttaaagcggacgcttcaggggctggaccagttgcgtcagcccctcggttttaatcagcagcgtgatttgcattagctcaccgagcttccctgccgggaactcatctttgcgggcaaaccacagcagatactcctccggcaggtcgattaagcgacgccctttgtatttgccaaacggcattatcgtattggctatttcaatcagctgctctttttccatctcagctacccagcaaacgcagcatttccgcttcgtcgatgacttcaatgcccagttcctgcgccttcgccagtttagatcctgcagcttcacccgctatcaccagatcggttttcttcgacacgctgcccgcgactttcgcgcccagttcgaccagtcgagctttagcgtcatcacgcgacatctggcttaagctgcccgtaagcaccacggttttaccagcaaacgggctgtcaatctcttccgcgttgataacgatcggcgcaggccagtgaacaccttccgccaacagctcgctgatgacattgcggttgctttcttcggcaaagaagttgtgaacgtgggatgcaacgacaatgccaacatcaggcaccttttgcagctcttcaatcgaagcggcttccagcgcttccagcgtgccgaaatatgccgccagacctgctgcggtggcctcgccgacttcacggatgccaagtgcatagaggaagcgagcaaaggtggtttctttcgctttttccagcgcgttaaccacgttttgtgccgattttggccccatacgctccagtccggtcagtttgcctgcggtgagtttgaacagatctgccggagtatggacatattctttttcaaccagctgatcgatgattttgtcgcccattccgtcaacatccatcgcacggcgggaaacaaagtgtttcagcgactctttacgctgcgcaccgcaaatcaggccaccggtacagcgggcaaccgcttcaccttccacacgctcaacgtcagaaccacataccggacaatgcgtcgggaatacaacctcacgggtatcttccgggcgttcagaaagcacgacgttaaccacctgcgggatcacgtcgccagcgcggcgaatcaccactttatcgccaatgcgtaaaccaagacgttcgatttcatccgcattgtgtaaggttgcgttactcaccagcacgcctgcaacatggacaggttccagacgcgcaacaggcgtaatcgcgccagtacgcccaacctgaaactcgacgtcacgcacaaaggtcatctgctcctgcgccgggaatttaaacgctaccgcccagcgcggggcacgcgcgacaaagccaagctgctcctgctgtgccagtgagttgaccttaatcaccacgccgtcgatatcaaagcccagcgtcgggcggtcttcttccactttgtgatagaacgccagcacttcttccgccgattcacaaagcgttacccgatcgctgaccggcaacccccactttttaaattgcagtaaacggccaagatgagtatccggcagctcgccaccttccagaacaccaacgccatagcagaaaaaagtgagcggtcgcttcgctgtaatacgcggatcaagctgacgcagtgaaccagctgccgcattacgtgggttagcaaacactttcccgcccgtgcgtcgcgcatcttcgttaatcttttcgaaccccgcctgcggcaggaacacttcaccacgcacttccagacgcgccgggatattctctccgtgcagcttcagcggaatggcgcgaatagtacgcacattagacgtgatatcttccccggtggtgccatcgccacgggtcgcggcactgactaaaacgccattttcatacagaatactgacggcaagaccatccagcttcagctcacagcaccaggtgactttctcgttgtttttcagacggtcctgcacacgtttgttgaaagcaagaaagctttcttcatcaaaaacgttatccagtgacagcattggtacttcatggcgtatctggctgaaagccgccagcggcgcagcgcctacacgttgagtaggcgaatcaggcgtaatcagttctggatgtttggtttccagctcgcgcagttcgcgcatcagcctgtcgtattcagcgtcgggaatttccggcgcatccatcacatgataaagatattcatgatggcgaagcgtcgttcgcagttctgtcagttgttgttcgattgattccatatcgcaccatcaatgctaaaaacccccgacaagcgggggttcgaagaggagttaatttgccttaagtgtatcaggcgttggcgtctttgacttcgcggatgatgtcctggtactcgcgcaatttctgcggagtcatcatacggcgctgatcgtcaagcacgacaccgcccacttcatcggcaatatgctgcgcagattgcagcatcagcttgaagttctgcagctcgtcaccgtaagacggtacctgcataaagatagtgacacccggagtagtgaaatccttcatttcaggatcaaaggttcccggtttcaccatattcgccaggctgaataacgccgggccgctgccatccgggctaagatgacgatggtaaatattcatatcgccaaaaatgaagcccgcttgttgaatgctgttaagaagcagttcaccgtttagctcgctaccgtgatgcgccgcgacgttcatgataatcaccgcttctttgcgcttcggtttatccataactggagcaggttccgctacaggctcaggctgtggtgccgctacgggttctgcaggctggaaagcctgttgtgccggttgcggtgctgaatgcacaggctgcggcgctggcgcgacctgtggcgaaactggctgctgcaacggctgttcaggctgcggctgataggcaggctgctgcaccggctgcgctggatgcggagcatgttgcggcggtacctgcgcttcaggcggctgctggaccggttgacgcggctgcgcagacgcataaggcggttggtactggtgttgcggcgacggacgagcagcctcatgctcctgagcgttagccggggcatgattcacgcggtgaacacgaacctcaccaacgccctcatcatcttcgacatcctcgtcataagaatcgtcgtcacgttttgacttcattcgttttaatggccgatcgcggaacatagaagatcgttctttacggctggtccagaaaccatgtaccagtaaagcgattatggcgatcgcgccaacaatgattaatatcagacgcaaatcctgcatcattatattctctgttgttctaacaccttgccaccacggcaaacatttactcactaagagtatttgccgattacctcaagtgcaagtgcactattaactttcacagcacaaagatagatgaaatcgtgctttttgctgttttttcgaacatatcctaactgtccattgcgcaattacccggtaaaatacgcagaattttcctgggattggtcaaaaggagctcatcctgattatggtttcatcattcacatctgccccacgcagcggtttttactattttgcgcaaggctggaagctcgtctcgcaacctgggattcggcgtttcgttattttaccgctgctggtcaatattttgttgatggggggcgcattctggtggctctttacacagctcgatgtctggatcccgactctcatgagttacgttccggactggctacaatggctgagttatctgttgtggcctctggctgtcatctctgtgctgttagtgtttggctatttcttctccacgattgctaactggattgccgctccgtttaacggtttattggctgaacaactggaagcacgattgactggcgctacaccgccagataccgggattttcggtatcatgaaagatgtgccgcgaatcatgaaacgcgaatggcaaaaatttgcctggtatctgccgcgcgcaattgtattactaattctttacttcatccctggtattgggcaaaccgtcgcgccggtactgtggttcctgtttagcgcctggatgttagccatccagtattgcgattaccccttcgataaccacaaagtgccgtttaaagagatgcgcaccgccctgcgcacacgcaaaatcaccaatatgcagtttggtgctttaaccagcctgtttacgatgatcccgctgcttaatctgttcatcatgcccgttgccgtttgtggcgcgacggcgatgtgggtcgattgctatcgcgataaacacgcgatgtggcggtaacaatctaccggttattttgtaaaccgtttgtgtgaaacaggggtggcttatgccgccccttattccatcttgcatgtcattatttcccttctgtatatagatatgctaaatccttacttccgcatattctctgagcgggtatgctacctgttgtatcccaatttcatacagttaaggacaggccatgagtaagatttttgaagataactcgctgactatcggtcacacgccgctggttcgcctgaatcgcatcggtaacggacgcattctggcgaaggtggaatctcgtaaccccagcttcagcgttaagtgccgtatcggtgccaacatgatttgggatgccgaaaagcgcggcgtgctgaaaccaggcgttgaactggttgaaccgaccagcggtaataccgggattgcactggcctatgtagctgccgctcgcggttacaaactcaccctgaccatgccagaaaccatgagtattgaacgccgcaagctgctgaaagcgttaggtgcaaacctggtgctgacggaaggtgctaaaggcatgaaaggcgcaatccaaaaagcagaagaaattgtcgccagcaatccagagaaatacctgctgctgcaacaattcagcaatccggcaaaccctgaaattcacgaaaagaccaccggtccggagatatgggaagataccgacggtcaggttgatgtatttattgctggcgttgggactggcggtacgctgactggcgtcagccgctacattaaaggcaccaaaggcaagaccgatcttatctctgtcgccgttgagccaaccgattctccagttatcgcccaggcgctggcaggtgaagagattaaacctggcccgcataaaattcagggtattggcgctggttttatcccggctaacctcgatctcaagctggtcgataaagtcattggcatcaccaatgaagaagcgatttctaccgcgcgtcgtctgatggaagaagaaggtattcttgcaggtatctcttctggagcagctgttgccgcggcgttgaaactacaagaagatgaaagctttaccaacaagaatattgtggttattctaccatcatcgggtgagcgttatttaagcaccgcattgtttgccgatctcttcactgagaaagaattgcaacagtaatgccagcttgttaaaaatgcgtaaaaaagcacctttttaggtgcttttttgtggcctgcttcaaactttcgcccctcctggcattgattcagcctgtcggaactggtatttaaccagactaattattttgatgcgcgaaattaatcgttacaggaaaagccaaagctgaatcgattttatgatttggttcaattcttcctttagcggcataatgtttaatgacgtacgaaacgtcagcggtcaacacccgccagcaatggactgtattgcgctcttcgtgcgtcgcgtctgttaaaaactggcgctaacaatacaggctaaagtcgaaccgccaggctagactttagttccacaacactaaacctataagttggggaaatacaatgttccagcaagaagttaccattaccgctccgaacggtctgcacacccgccctgctgcccagtttgtaaaagaagctaagggcttcacttctgaaattactgtgacttccaacggcaaaagcgccagcgcgaaaagcctgtttaaactgcagactctgggcctgactcaaggtaccgttgtgactatctccgcagaaggcgaagacgagcagaaagcggttgaacatctggttaaactgatggcggaactcgagtaatttcccgggttcttttaaaaatcagtcacaagtaaggtagggttatgatttcaggcattttagcatccccgggtatcgctttcggtaaagctctgcttctgaaagaagacgaaattgtcattgaccggaaaaaaatttctgccgaccaggttgatcaggaagttgaacgttttctgagcggtcgtgccaaggcatcagcccagctggaaacgatcaaaacgaaagctggtgaaacgttcggtgaagaaaaagaagccatctttgaagggcatattatgctgctcgaagatgaggagctggagcaggaaatcatagccctgattaaagataagcacatgacagctgacgcagctgctcatgaagttatcgaaggtcaggcttctgccctggaagagctggatgatgaatacctgaaagaacgtgcggctgacgtacgtgatatcggtaagcgcctgctgcgcaacatcctgggcctgaagattatcgacctgagcgccattcaggatgaagtcattctggttgccgctgacctgacgccgtccgaaaccgcacagctgaacctgaagaaggtgctgggtttcatcaccgacgcgggtggccgtacttcccacacctctatcatggcgcgttctctggaactacctgctatcgtgggtaccggtagcgtcacctctcaggtgaaaaatgacgactatctgattctggatgccgtaaataatcaggtttacgtcaatccaaccaacgaagttattgataaaatgcgcgctgttcaggagcaagtggcttctgaaaaagcagagcttgctaaactgaaagatctgccagctattacgctggacggtcaccaggtagaagtatgcgctaacattggtacggttcgtgacgttgaaggtgcagagcgtaacggcgctgaaggcgttggtctgtatcgtactgagttcctgttcatggaccgcgacgcactgcccactgaagaagaacagtttgctgcttacaaagcagtggctgaagcgtgtggctcgcaagcggttatcgttcgtaccatggacatcggcggcgacaaagagctgccatacatgaacttcccgaaagaagagaacccgttcctcggctggcgcgctatccgtatcgcgatggatcgtagagagatcctgcgcgatcagctccgcgctatcctgcgtgcctcggctttcggtaaattgcgcattatgttcccgatgatcatctctgttgaagaagtgcgtgcactgcgcaaagagatcgaaatctacaaacaggaactgcgcgacgaaggtaaagcgtttgacgagtcaattgaaatcggcgtaatggtggaaacaccggctgccgcaacaattgcacgtcatttagccaaagaagttgatttctttagtatcggcaccaatgatttaacgcagtacactctggcagttgaccgtggtaatgatatgatttcacacctttaccagccaatgtcaccgtccgtgctgaacttgatcaagcaagttattgatgcttctcatgctgaaggcaaatggactggcatgtgtggtgagcttgctggcgatgaacgtgctacacttctgttgctggggatgggtctggacgaattctctatgagcgccatttctatcccgcgcattaagaagattatccgtaacacgaacttcgaagatgcgaaggtgttagcagagcaggctcttgctcaaccgacaacggacgagttaatgacgctggttaacaagttcattgaagaaaaaacaatctgctaatccacgagatgcggcccaatttactgcttaggagaagatcatgggtttgttcgataaactgaaatctctggtttccgacgacaagaaggataccggaactattgagatcattgctccgctctctggcgagatcgtcaatatcgaagacgtgccggatgtcgtttttgcggaaaaaatcgttggtgatggtattgctatcaaaccaacgggtaacaaaatggtcgcgccagtagacggcaccattggtaaaatctttgaaaccaaccacgcattctctatcgaatctgatagcggcgttgaactgttcgtccacttcggtatcgacaccgttgaactgaaaggcgaaggcttcaagcgtattgctgaagaaggtcagcgcgtgaaagttggcgatactgtcattgaatttgatctgccgctgctggaagagaaagccaagtctaccctgactccggttgttatctccaacatggacgaaatcaaagaactgatcaaactgtccggtagcgtaaccgtgggtgaaaccccggttatccgcatcaagaagtaattcttgccgcagtgaaaaatggcgcccatcggcgccatttttttatgcttccgccagcggcggcaaaatcaattcatcgctctcatgctgctgggtgtagcgcatcacttccagtacgcgcaaccccgctcggtgcactgcatcggttaacgccttccctttcagcaagccactgatgagctgagcacaaaacaggtcgccagtccctttcaggtcggtttttacccgtgaatgggaaatgacattcacgctgtcggcagtgaccaccacaacctgcatctcctgattttcttcattaccggaggcgctggtaaccaccacccattttaatgtgtctgaaagcagactttttgcggcagcaatggcactgtcgagatcgcggcaatttttaccggtcaggatttccaactcaaagatattgggggtaattccctgcgccagcggcagtaaatattgtcgatacgcttcgggaaggtcaggtttgacataaattccgctatcaatatcgccaatcaccggatcgaccatgatcaataggtcaggatggtctttgcgtagcgcagtcagccactcggcaaggattttgatttgcgatgccgttcccatatagcccgtggttacagcacgaagttggcgcagcgcatcacgctcctgaagcgcacgcaaatagccgctaaaccattcgtccggaatcgcaccaccgtagaaagtgtcataatgcggcgtattgctcagcaataccgtcggcacggcaaagacattcaggccgttctgtttgatagcaggcacggcaatgctgttgcccacgctgccgtaaaccacctgcgactgcacggcgacgatatccgcctgcagtgccctactcttatcgttaaacaacaacaaactactcatttaattttttctccttgccgatgatcctcatcgtaatccaaccgaaactttacctgattctggcagtcaaatcggctatcacaaaacaaggataaggtaattcaatgaagaaaatcatttgtctggtcattacactactaatgacactccccgtttacgcgaagttaactgcccatgaagaagcccgcatcaacgccatgctggagggattagcacagaaaaaggatttgatatttgtgcgcaacggtgatgaacatacctgctatgaagcggtttctcatctgcgtctgaagctcggcaatacccgtaaccgcattgacactgccgagcagtttattgataaggttgcttcgtcgtcatcgattactgggaagccgtatattgtgaagatccccggtaagagcgatgagaacgcacagccttttttacatgcgttaattgcgcagacggataaaacggtgcctgcggaaggaaattaatccgctttgggaaggcatttacaggaggtaacatgaaaaaacgctttatttatcacgatgaaaaatcgaataaattttggtggatagattacgaaggggatagtttagctgtcaactatggcaaggtaggtagtattggtaaattccagacaaaagagttcgataatgaagaacagtgtctgaaagaagccagtaaattgattgccgcaaaaatgaagaaaggctatcaagaagatccaaagtttaacttcatggatcgctactattttgatgatgaagaaattgggttacatgttaaaacgtcacacccaaacttccagtgccattttactgatccactttatatgtgttgctgggatgaagaatctccttttggcagcgatgaaggtgctgatgctctaaacgttcttgaaaatagcctccgtaaagagccggatctggactgtgctgatttccctcaaatgttaattgaaactatgtggggtatgaaatacatcgctatggacagtattcttgaagaggatgttcgtgcgcaattactagtcgatgaaatgagcactatccagagcaatatgattacctacgcaactgcattcggtcagattaaagtcatgggtaaaatctcccataaacttaaaaagatgggactcaatgcactagcgcgtcatcagcttaccgcaaaaattcttcaatggggtgacggtcaggactcaccaatacttcaaaaaatgattgatgaccttacggcgtttcctcacgaaaattaaatactgcatttgtcggcagcaacaactgttaaaaaagtgcgctttgtttatgccggatgcggcgtaaacgccttatccggcctacaaaatcgtgctaattcaatatattgcagaaaccttgtaggcctgataagcgtagcgcatcaggcagttttgcgtttgtcatcagtctccgatgctattaatccttaaatccccgccccctggctaaaatgctcttccccaaacaccccggtagaaaggtagcgatcgccacgatcgcagatgatcgccaccaccaccgcgtcagggttagcttttgccacccgcagtgctccggcaaccgcgccgccggagctgacgccacagaatattccttcccgcaccgccagttcgcgcatggtgttttccgcatcgcgctgatgaatatccagcacctcatccaccagagaagcgttgaaaatccccggcagatattccgtaggccagcggcgaatgccgggaatgctgctgccctcttccggttgcaggccgacaatggtcaccggtttggattgttcgcgcataaagcgtgagacgccggtgatagtgccggtcgtccccatgctggagacaaaatgagtgatgcgcccgccggtttgctgccagatttccggcccagtggtggtgtaatgcgcataagggttatcgggattattgaactgatcgagcagctttccttcgccacgattcgccatctccagcgccagatcgcgcgcaccttccatgccctgctctttggtgacaagaatcagttccgcaccataagcacgcatcgccgcacggcgttcctggctcatgttgtcgggcatcagcaatttcatgcgatagcctttcagcgcggcaatcattgccagcgcaatgccggtgttaccactggtggcttcgattaagacatcacccggtttaatttccccgcgcttttccgcctcgacgatcatcgaaagtgccgcacgatctttcaccgaacctgccgggttattgccttccagttttaaccacacttcactgccgttatccggccccattcgctgcaacttcaccagaggcgtattgcctattgtttgttctaatgtactcacgatctctatccatacgtggtgttgcctgatgcgacgcttgcgcgtcttatcaggtctacaggttacaaaccttgccattaaaaagcccggatcgcgggaagcgcctccgggcgtttaacattcactcaacctatcaggcgctttgtgcgagagcaagttcctcatcgcgggtttcgatacgctcgtcgccgttatacagccgcgcatgttgcagaccaacgaataaacgctcgccacgctgcggggcatcgtcgccatgcatcacgaccgtcagcggttcgttgtaccaccccagcggctgcaccactaattgggtgtagtgacctttcgggctggcttccagtacctgtaccggcagcggcgaatcgaggctggtacggcggctgatatccacttcccaagggcgcaggaagagatccaccggcccctgatacgcaggtgtgtagcccagcggccagcgatgcgcgccaacatggaactgcccgccgcgaatggttccctgcaggcggttcacttcgcccataaattcgagcacaaaacgggtcgccggttcgcgccatacctgatccggcgcgtcagcctgttcaatattgccctggctcatcacaactacacgatcagctacttcggtcgcttcttcctgatcgtgggtcacaaaaacgctggtgaattttagttcttcatggagttgacgcagccagcgacgcagctctttacgcacctgcgcatccagcgcgccaaacggttcatcaagcagcagaatttgcggttccacagccagcgcgcgcgccagcgccacgcgctgtttctggccgccggaaagctgcgccggataacgatccgccagatgggcaagctggaccatttccagcaattttgtcactttcgctttgatggctgcggcattcgggcgctcgcgacgcggcagcaccgtcaggccaaaagcgatattgtcgaacaccgtcatatggcggaacagcgcgtaatgctggaacacgaaaccgactttacgatcacgtgcgtgcaggcggctcacgtcggtgccgtggaagcgaatatgcccgctggtttgatgctccagcccggcgataatgcgcagcagcgtggttttcccggaaccggacggccccagcaacgcgaccatctgacctgaaggaatatccagtgagatatcgttcagcacctgggtgcgaccaaacgacttcttaatattggcaatctcaatgctcatgatgttcctcctgctgtgcgcgtttttcctgattctccaggcgccactgcaacatactttttaaaaacagggtgataatcgccatcagcgttaacagcgccgcagcggtaaaggagccgacggtgttgtagtcctgctccagcaattcaatctgtaacggcagcgacagggtttcgccgcgaatcgagccggaaaccaccgacaccgcgccaaactcgccaattgcgcgggcgttggtcaacaccacgccataaagcagcgcccagcggatgttcggtaatgtgacgcgacggaacatctgccagccggacgcgccaagcaaaatcgccgcttcgtcttcctggctgccctggcttaacatcaccggcaccagttcgcgcaccacaaacggacacgtcacgaagatggtgaccagcaccattcccggccaggagaacataatttgcaggttatgctcgtcgagccaaccgccgagcgggccgttagagccgtagaacagcaaatacaccagaccggcaaccaccggcgatacggcaaacggaatgtccagtagcgtcagcagtaactggcgtccagggaagttaaagcgcgtcaccagccaggccagcagaatgccgaacaccaggtttaccggtacggcaatcagcgcgatcatcaccgtcagccagatggcgtgcagcatgtccggatcggccagattctgtaaaaccggcatcagccccttgctgaatgcctgcacgaagatgtaaatcatcggcaccagcaggatgaacgccgaaaccagcatcccgatgccaatcagaaaccatttgccccagttaatcgggcgcgcgtcataacgcttcaattgggtaacttccgccattaatgacctaccacacgccgaccaaagcgactttgcagagtgttaattgagaacagcagcagcagagatgccgcgaggatcaccgaagcaatcgcgctcgctgccgggtaatcaaactcctgtaagcgcacaaaaatcatcagcgacgtcacttccgtcttccacgcgatatttccggcgataaaaatcaccgcgccaaattcaccaagactacgggtaaacgacagcgccacgcccgccaccagcgccggagaaagctccggcagcaccactttgcagaaactctgccagcgcgttgcaccaagcgtttccgccgcttcttcatattccgggcctaactcttccagcaccggctgcacggtacgcaccacaaacggaatgctggtaaaggccatagccaccgcaatccccagccatgtataggtgactttgatatcaaacttcgccagccattcaccgtaaaaaccgtttacggaaaagagcgaggccagcgttaaaccggcgacagccgttggcagcgcaaagggtaaatccatcagcgcatcaagcagcgtgcggcctgggaagcgatagcgggttaggatccacgccatcagcagaccgaaaacgccgttaaaaatcgatgccacaaacgccgacagcagcgttactttgtaggccgcgaccacctgcgggttggtgatcacctcccagtactgcgcccagctcatctgggccagttgcatcaccagcgcggagagcggcagcagcaaaatcaggcacacaaacagcagactggtgccgaggcttaaggtaaagcccggcagcacgcgtctggaggagacagcaaacatcagttacgccccgccgctaacagcttgtctaactcgccgccgctggtgaagtgggttttcatcacttccggccaggagccaaatttgtcttccacgcggaacagctcggtctgcgggaatttgtctttcagtttgtccatcacctccgggttattcacgcggtagtaatagtcggtgatgatggtttgcgcctgcgggctatagagccagttcagataggctttggcggctttttccgtaccgttggcctgcacgtttttatcaacccacgccaccgggaattccgccagaatgttggttttcggaatcaccacttcaaagccctgcgcttcatactgtttacggatgttgttcacttccgattcgaagctaatcagcacatcgcccaggccgcgctcggcaaaagtggtggtcgcgccacgaccgccagtatcgaacacttcaacgtttttcaggaactgggtcataaactgttcggttttgcctttgtcaccaccgtcagctttatccgctgcgccccatgccgccagataggtataacgcgcgttacccgacgttttcgggttcgggaaaatcagcttcacgtcggagcgcaccaggtcgttccaatcgtggatattcttcgggttacccttacgcaccaggaagcccatggtggagtagaacggcgagctattattcggcaggcgcgactgccagtcggccgggatcagcttgcctttatcgtgcaggatttgtacgtcggtcacctggttataagtgacaacgtcggcttttaagccctgtaaaatcgccagcgcctgttttgatgacccggcatgagattgttttatcgtcagtttgtcgccgccgttatcttttgcccattgttgctcaaacggcggattcagggcggcaaacagctcgcgggagacgtcataagaactgttcagcagttccgttgcctgtacatggcccgccagcagcagagaagcgaccagcgcgagtgagttctttttcagtaagttaacggccattgcgcacccttataaatttaatgactttctaatagccatcatatttataacggacgtgaaaggagtaacggttttatataccgtttggtgatttggaagttgaaaagggaataagaacttggttcaacaggcgtaattgttgcagtcagtttggacacgaacagcgcggagaaaccggagcgtacacatagtacgtgaggatttcgagcactgcccggggccaaaatgacaaataaaatagcctggtgaacttagttcaagacgaaatcctccccacaaatgcagggaggaaacagaggtgaatcagataccgacgctaaccgtctccggcagtgtgctgccgccatcaatcacattctgtgtaccggttaaatagctggattcatccgatgcgaggaaggccgccagttcgccgacttccagcggatcggcgaggcgacgcatcgggattgctttcgccatttcagtcagcaccgactctggatcttccgggttcgactggcgggcaatgctttccgccattggtgtgcgcacgtatcccgggcaaatggcgttaacgcgaataccagactgcgcgtactccaccgccagcgattttgtcaggccaacaatcgccgctttcgttaaggcgtacgccgtttcgccaggatcggccaccatatcaccagtgactgaagacatcatcacaatgcgaccatctttgcgggcaatcatctccggcagcaccgccttcgtgacgttccatacgcctttaatattgatgtcaatatggaaatcgcgatcgtcatcgctcatatcgaggaaactgcccagacgacaaacgcctgcgttattcaccaggatatcaatgcgcccttctttttccttcgcgcgtttgatagctgcggctaccgacgccgggtcacgcacatcggcgacaaccgccgtacagcgatgaccacgaccacacagttcgtccgccagcttttcgatctcaggggagatatccagcaagattaggttcgcgccatgacgtgcaaaagttctggcaattccttcgccaattccctgcaatgcgcccgtaatcagtgctgtcttgcccgtgagtttacccattttaatgctctccttgttaatacagagcgttacactccattccctctgaaaatacaggataaacaaaatattgctgcggatcagctcactaattcaggaaaatctcaatccagtcgctgctttatgcatcatttcaggcgttgtgttagctcactgctgcgctgaatcattttcaatgactccacatcattgagttgcacaaggccaacaaacagtaaatcggtaacagaattttgcgccgtgcgggtagacatcgacgagctacgccattcggtttctccggaaacggtatcgagggtgaaatgcgccagccgccgcagcggagagtcagtcagagaagtaatggcaatcaccgttgccccctgctttcgtgccgcttctgcgcacaagacaatctcttttttactgccgctgtaagagatagcgatttgtacatcgccttttttcaacgcctgagaaacggtggcttgtacgtgcgtgtcggcttcgcaggccacgcgatagccaattttcatcagtttgaacgacagatcgcgccccaccagcgccgatccgcccaggcccgttatctggataaacggtgctttactgatgacctcaatgattttttgcagccgcgcgtaatcgagcaacgcgcaggtttgctccagcgccagctctttttcgcgattcagtttgcgcgcgatcacttccagcgaatcatcactggtaatcgaactgtgcaggtgcagtgccgtggcattcgttttctcccggctggcactgtattcgcctattaacgccatacgcaattcagtaaatccttgcgcgccgagtttttgggcaaatttcactatgctcgactggctaatgccgagctgtttcgccatctgccgtgaagaaacggattgcagctcactcacgttggcctgcagaaagtcagcgattttttgctcgttttcggtgaattcactccccgcattgcttattttcgtcaggtacaacatcttccactctcctgggctggcagcataaattccgcttaagttcttatgacgctcttcacactctgcgagtgtagactcaatgattcctttaagcctgtcaattcgggatatatgattccatacatctgcaattatttgatcgtaaatagtaaggtcaccaccgatgcaatttgaaaagatgattactgaaggctcgaacaccgcctcggctgaaattgaccgcgtatcgacgctggaaatgtgccggattatcaacgatgaagataaaaccgtaccgcttgccgttgagcgcgtactgccggatatcgccgcggcgatcgatgttatccacgcccaggtaagcggcggcgggcgtctgatttacctcggtgcgggaacatccggtcgtctggggattctggatgccagcgaatgtccgcccacctacggcgtgaaaccgggtctggtggttggtttgattgctggcggcgaatatgccattcagcacgcggtggaaggcgcggaagatagccgggaaggcggtgttaatgatctgaaaaatattaatttaacggcacaggatgtggtggttggcattgctgccagcggtcgcacgccgtatgtgattgccggactggaatacgcacgccagctcggctgccgcacagtgggaatttcctgtaatccggggagcgccgtttcaaccaccgctgagtttgccattacaccgattgtaggtgccgaagttgttaccggttcttcgcggatgaaagcaggtacagcgcagaaactggtgctcaatatgctttccaccgggctgatgattaaatccggcaaagtgttcggcaacctgatggtcgatgtggtcgccaccaacgaaaaactgcatgtgcgacaggtcaatattgttaaaaacgccaccggatgtagcgcagagcaagcggaagcggcgttaattgcttgcgagcgcaactgtaaaacggccattgtgatggtgctgaaaaatctcgatgccgcagaagctaaaaaacgcctggatcaacacggcggctttattcgtcaggttttagacaaggaataacccatggccaaagagatcagcagtgaacttctgaacaccattcttacccgtgtcggcggaccgggaaatatcgccagttgtggtaactgtatgacgcgcctgcgtctgggtgtacatgacagttcactggttgatcccaatatcaaaacgctggaaggcgtgaagggcgtcattttgaccagcgaccaggtgcaggtcgtttttgggcctggtaaagcgcatcgtgccgcaaaagcgatgagcgagctgctgggagaagcaccggtacaggatgccgcagaaatcgccgcccagaacaaacgtcagttaaaagccaaacaaacctccggcgtgcaacaatttctcgccaaattcgccaccatcttcacgccgctgatccccggttttattgccgccggtctgctgctggggatagcgacgttaattgccacggtgatgcacgttccggcagatgctcagggaacactacccgatgcgctgaattttatgaaggtgttcagcaaaggtttgttcactttcctggtgattctggtgggctataacgccgcccaggcatttggcggcacgggcgtaaatggcgcaattatcgccgcgctctttttgctcggttataaccccgcagcgaccaccggttactacgccggttttcacgatttctttggtctgcccatcgatccgcgcggcaatattatcggcgtgctgattgccgcgtgggcctgcgcccgcattgaaggcatggtgcgccgctttatgccggacgatctcgacatgctgctgacctcgttaatcaccctgctgatcaccgctacgcttgcgtacctgatcattatgccgctgggtggctggttattcgaaggtatgtcatggctgtttatgcacctgaacagtaatccgttcggttgtgcggttttagccgggctgttcctgatcgccgtggtatttggcgtgcatcagggctttattcctgtttacctcgcgttaatggacagccagggattcaacagcttatttcccatcctttcaatggcaggcgcgggccaggtgggcgcggcgctggcactctactggcgggcgcaaccgcacagtgcgctacgcagtcaggtacgcggggcgattattcccggcctgctgggcgttggtgaaccgctgatttacggtgtcaccctgccccgcatgaagccgtttgttaccgcctgtttaggcggcgcggcgggcggtttgtttatcggcctgatagcctggtggggtctgccgatgggcttaaacagcgcctttgggccgtctggtctggtagcgctgccgctgatgacttccgcacaaggcatccttccggccatggcggtttatgctggcgggattctggtggcatgggtttgcgggtttattttcaccacgctctttggctgccgtaacgtcaatctggactgatatcatgaaacggacaatgctctatctttctctgctggctgttagttgtagcgtcagcgccgcaaaataccctgttctgacagaaagctcgccagagaaagcagggtttaacgtcgaacggcttaaccagatggatcgctggattagccagcaagttgatgtcggttatcccagcgtaaacctgctgatcattaaagataatcagattgtgtatcgcaaagcctggggagcggcgaaaaagtacgatggcagcgtgttgatggaacagcctgtcaaagccaccaccgggacgctgtatgacctggcctcaaacaccaaaatgtacgccacgaacttcgccctgcaaaagctgatgagcgaaggcaaactgcatcctgacgatcggattgcgaaatatattccggggtttgccgatagtccaaatgacaccattaaaggcaaaaacaccctgcggatttctgacctgctgcatcacagcggcggtttcccggcagatccgcaatacccgaataaagcggtcgcgggcgcgttatattcccaggataaaggccagacgctggagatgatcaagcgcacgccgctggaatatcagcccggcagcaaacatatctacagcgatgtcgattatatgctgcttggatttatcgtcgagtcggttaccggtcagccgcttgaccgctatgttgaagagtcgatttatcgcccgctcggcctgacacatacggtatttaacccgctgctgaaaggctttaaaccgcaacaaattgccgccacggaattgaacggcaatacccgcgatggcgtgatccatttcccgaatatccgcacctccactctctggggtcaggtgcacgatgaaaaagccttttattcgatgggcggcgtttccgggcacgcaggtttgttttccaataccggcgatattgcggtgttaatgcaaacgatgctgaacggcgggggctatggtgatgtgcagctgttcaatgcggaaacggtgaagatgttcaccaccagctctaaggaagatgccacttttggcctcggctggcgcgtgaatggtaatgccaccatgacgccgacgtttggcacgctggcaagcccgcaaacctacggtcacactggctggaccggaacggtgaccgttatcgatccggtgaatcatatgacgattgtgatgttaagcaacaagccacattcgccggttgccgatccgcaaaagaatcccaatatgttcgaaagcggtcagttgccgattgcaacttatggttgggtagttgatcaggtgtatgcggcgttaaagcagaagtaataaaaaggccagtcagtaatgttactggctggtctgagagtgctgacaaacgcaaaactgcctgatgcgctacgcttatcaggcctacgtggagcccacaatatattgaattagcacgatttcgtaggccggataaggcgttcacgccgcatccggcgtgtacaacgcgcacttggtcaacaatctgaggccagtcagtaatgttactgcctggcctttaatcaatgaatcagaaacgcttacagcgccatcaacttgtccagcgacggtgcgaaataatagccgccggttaccggtttggtgaaacgcaacatcgcatcacgcttaccatcggtatcgccaaacatgctcagcagttgctgctcaatgttatgcagacgcgcgcagtaggcgcagaagtacagaccgtgagtgccactggcagtgccgtacggcaggctctggcgaacaatcttcagccctttgccatcttctttcagatcaacgcgggtgaggtgagaggtttccggacgttcgtcgccgtcgatctcttcgttggcctctttggtgcgcccgatcaccatctcctgatcgtgaacgctcatccggttgagctgcttcaggttgtgttcccaacgctggacaaacacatagctgccgcccgcatccacgccgtctttgataaccgccacttcgcgacgcgtctcttcacccgccgggttttccgtaccgtcaacaaagccgctcaggtcacgctcttcaacccaacggaagccgtggatctcttctttcacttcaatgcagtcaccaaaggcttccatcgccgcctgggcgacagagaagtttacgtcgtgacgcagagaaagaatgtggatcaacacatcgaactgggtcgtcggcgcaaggcctttaccgtagcccggaaaatctttcagctcttctgccccaacgccgccgctcagagcgcgccaggtgttgttaccaaaggcaaccaccgcaccaagatgcgcgtccgggaatttcgcttcaaaagttgccagtttgtcggcaaatgttttactggccgcacgcagggcgtcaacttcccctttcacgttggcttcgatccaaatcgccgcgcggcaatgttctggcaaaatgccactctgaacctgagacattgttcctcctgaaaataataatgccacgcaatccgtggcattgttgagcgctattttacgtgttttttcgcggcggcggtttgttcagacgcaaattaacgccgccagataattttactgactttccagtttttcagggtatcgtccgaaggcattaacccttcaggaccacgccattccccgctgaactggtagctaatatgttgactgccttcggctttacattcgacggcacgattatcatcaccatcagctttttggcaattgccaaatgctttgctgtaaaggtcgctaaacggtgtaccgattttaacaccggtgtcagcaggaatatcgctatccagcacgtcaatgcgactgatcgtgccttgatcgccgttaatcaccatcgccacgttgtcgcccttcatcacttcaaaaaagcgcaccacgttgccgttcgcggttttcattccgctgcgcaggcgataatcgccatcaagcgcatcggcaatggcttgttcttgcagtggtgtggacgccgttaattcacccacgccctgctcgctcactttggtggacgacccaaaccagttccacgggttagcggcagaccagttaactgacgacatcgtggaacagccggtcagcatcaatggcatagcgcataacattaaacgcagcgatttcatgtcacttcctttggttattcaataacgttgcttggagtgcaaattcaccaaaaagtgccgttattcttttacttcataaaaacaagcgcgtaaacgtcgattggtcagcagccagattaacgccacaatatccgccactaccagcgccagaccgataccgctaacggattcaccgttcagccacagccacggttgccagcaaagtaaaaccacctgcgccaacagcaacagaaaatagagtacacgccaggtgcgaggaaacgtagcccgccgaccgctcaacaaaaacgccagcaccgccggaatgccaggaatcagccccagccagaaattatcgtgatcgggataaaacagatttagcagcgcagtaccctgctcgcgcgacgcaccggcaatgacaaacagcacccaggttcgcgcctgaagcaatagcacaagccagaagagcaagggtaaacgcaggcgaccgtgcgcatcataatggacaggatgaaactcagtactcttcatcttcaatcaaacgcttacccagactcagcacgtcggcgtgttcatatcccaggcgttcatacattccgagcaccatgtcgttatcttccggcacattgatctgaattttcgggcagccacgagcaatcagctttttctccagccgattaagcaacgcattggcaatcccacgcccacgaaactctggatgcacgccaagataataagcagacccgcgatgcccgtcataaccgcccatcaccgttccgaccacgtcaccgtttacctcagcgaccaaaaacaaactgacgtcatggttcatcttacgctcgatgtccatttccggatcgttccacggacgcagcaagtcgcaacgctcccaaagggtgatgacctcttcgaaatcttcctggcgaaatacgcgtatctccatggtattcgttacctttttgcgggttaaaaggctgattatggcgtgaacggtcgaattagccaatatctgacgaaaatcggttgaaaaagtggcataatggggagttgtcaactattgaaatgaaaagtaaaacaattctcaacagcaaaccgtcgtaacggattacgcgatacgatataacatctggaactttattattacaactcaggccgtatgagcacttttaaaccactaaaaacactcacttcgcgccgccaggtgctgaaagccggtttggctgccctgacgttgtcaggaatgtcgcaagccatcgccaaagacgaacttttaaaaaccagcaacggacacagcaagccgaaagccaaaaaatctggcggcaaacgtgtcgttgttctcgatccaggtcacggcggaattgataccggagcgatcggacgcaacggttcgaaagaaaaacatgtggtgctggcgattgctaaaaacgtccgttccattttgcgtaatcatgggattgatgcgcgtttaacgcgttctggcgatacgtttatcccactttacgatcgcgttgaaatcgcccataaacatggcgcagatctgtttatgtcaattcatgccgatggctttaccaacccgaaagctgccggtgcttcggtatttgccctctctaaccgtggggcaagtagcgcaatggcgaaatacctgtctgaacgcgaaaaccgcgccgatgaagttgccggtaaaaaggcgactgacaaggatcacctattgcaacaagtgctgtttgatctggtgcaaacagataccattaaaaatagtctgacgctcggctcgcatattctgaagaagattaagccggtgcataaactgcacagccgcaacaccgaacaagcggcatttgtggtgttgaaatcaccgtcggttccttcggtgctggtggaaacctcgtttatcaccaacccggaagaagaacggctgttaggcacggcggcgtttcgtcagaaaatcgccacagcgattgctgaaggcgtgatcagttatttccactggttcgacaaccagaaagcacattcgaaaaagcgataagttatgaaacccgacgcacaccaggttaaacagtttctgctcaaccttcaggatacgatttgtcagcagctgaccgccgtcgatggcgcagaatttgtcgaagatagttggcagcgcgaagctggcggcggcgggcgtagtcgggtgttgcgtaatggtggtgttttcgaacaggcaggcgtcaacttttcgcatgtccacggtgaggcgatgcctgcttccgccaccgctcatcgcccggaacttgccgggcgcagtttcgaggcgatgggcgtttcactggtagtgcatccgcataacccgtatgttcccaccagccacgcgaatgtgcggttttttattgccgaaaaaccgggtgccgatcccgtctggtggtttggcggtggcttcgacttaaccccattctatggttttgaagaagatgctattcactggcatcgcaccgcccgtgacctgtgcctgccatttggcgaagacgtttatccccgttacaaaaagtggtgcgacgaatacttctacctcaaacatcgcaacgaacagcgcggtattggcgggctgttctttgatgacctgaacacgccagatttcgaccgctgttttgcctttatgcaggcggtaggcaaaggctacaccgacgcttatttaccaattgtcgagcgacggaaagcgatggcctacggcgagcgcgagcgcaatttccagttatatcgtcgcggtcgttatgtcgagttcaatctggtctgggatcgcggcacgctgtttggcctgcaaactggcgggcgcaccgagtctatcctgatgtcaatgccgccactggtacgctgggaatatgattatcagccaaaagatggcagcccagaagcggcgttaagtgagtttattaaggtcagggattgggtgtaactccctcacccccactcccgcatccgctgatgcagcgtcagtgacggcttctcggaaaacagctgctggtaatccgtggcaaattgccccagatgccagaatccccactgcatggcggcgtcttttaccgtcatactttgcgaccacggacttatcagttcgcggcgtacggcgttcaggcgaatgcgtttcagccacgcgttcgggccaatgcctaaaatagcgtgaaacgcgttttgtagcgtgcggcggctgacatgcagttgattacacaaatccagcaccgtcaccggttcggacatgttttccagcacatattcacgggcgcgggaaagcaatcgacggtaactctgatgactgatgctttccgccgtcaccattggttgcgcttcttccagcatggcccccatcgccattagcaaattatcccccagcacttttcgcactgcaggctgatggagattttccggattctcgcaaaacgtcgccagcgcctgttggacaaagccccacagcgcggctttatgctgctctttcacttccagcgccgactggttacgcaacatatgtaatacccgatccgggttatgcaaaaagttagcctgccgggtgatgacatcttcagaaagcaccacgcccaggatcgtgtaatcatccggcgtgctcagttcaaattcagtgccaccagggcgggtggcgatttccgcgcttcccagacattgcgaaccgataaatccctgctcaccgcgcgtcgccggaatgccaaaccagaacgagttcggccagaccaggcacgactgacgcagcgccagaccggtgtattcacgaaaaacctgaatatcatcgagtagaatttccgtaaattcaccatgaaacttgcccggatgcagctgatcgtaaatctgctgccaggcggtaatcgttaaagcatgttcatagacatccgttgtctgtcgttgatgaacattatccacttcgaccttcggcgtgagcttcaggttttcgggtaagggttcatgataaagatggtgcaaattggctgtacgggtctttttcatgatgttaatgccgggtgttgtaggacacccggcacctccgacaggttaatggggcttgagacgataacgactactgcgtttacgtaacgtcccggcagaaaagagctgttcgagcgcatttctggctttttccagcggccagccaaagtgggcagccacttctcctgccgtcattccctgacgtactgatgttaacagcgccaacaactcgtcagcagattccgcgacgataactggcgcgtcgggttcccttacgggttgcttcggctggcggttaaagccagtaaccagccactgggtgtcatcgtctggccgaccgatctccttgcggctgatgacacgcccggtacgcatcgcggcagcacaacctgcgtccagcgccgcacgacacgccgccagatcgccttccaccaccagcgttaagcgaccagggtcaagcacttcgtgactgagcagacgaacgttagctgctttgagcatggcatccgctgcatctatcgcggcgaccatgccgtccacttccagcaatcccagtgcattgatcatcggcaacctccgttacgcacgctggattggattacgcgcgatttccagcactgcatcggtaaaggcgttacaggctgctttacacgctgcctggctaccggttaaaaatgctgccgagtagttggtttcagacggtggcgggacataggtcgccagctgtacgtcggcagacttcagggctgcatcaatgccataggtcgcttccagcggcggtgccaccagatacgccatcggatcgccaagcgtgatcccggcggttgatgagagataagaaccggtacgcgaaactacatgtgccaggaatgccgtatcttgcgcgtcattagcccactggaaagctgcgccattttcaatatgcgcaatcatcgcatccagacctgcacgcacttccgccgggtttggcccaccaagcataatcagcacttcaccggcagtcggtgacgggccgtgtgcagcgcccgcatatagcgagcggccatacaccacttccaccatcgcctgcttggtcgcttcatcagcggcaatgtaggtgacgtcatcggagtcggcagaaatcagaccgaggctacgaatatgcggcggcaatttcagttcacgcgcaaaatcggcgttaacggaggcaatcacccgcatagcggtgacagacggtcgaatcaaatctaaagctggcatgatgcctccttatcgggtcatgttgatgccggatgctttctgctccagcatacgtttcgccaaatccacaatgacggctgcggcttcaaccggcggcgtgccgccctggtgaatgttagagatacaggtgcgatcggcctcaacggtggtcgccatacgcggcgagtaaacggcgtagcaggagaggctttctgactgacccaaccccggacgttcgcccaccagcaggatcactactttcgcgccgaggatctcaccgatctgatcttcaatcttcacgcgaccataacgaacaaagaatggtgtaccgactttcagcccggcctgtttcaggcccgccatcagcggtggcaggatctcttcgtagttcacggtgatcgcatcagttgacaggccatcagaaataacgacctgtacgtccggattggcaacacactgcgctttcagcgcttcaacagcttctgcacacaggcggcggcccatatccgggcgagtcaggtagagatttttgtcgctaatttcagagcgtacttccagcaagccctgcgctttcacccactcttccggcacttctttcagtacggtatctttcgaacgagagtgatcggccaggaaacgcagcagcgcctgcgtacgtggacgcggaccggcacgaccggtacaaacgcgggccacggtgctgcggcgcagttctgttaatacgtctgcgcgatgcggattttcaacaccaatccacgcttttgcttcagcggaacctaaatccagcgcacagctttccgaggtcaccggtgccgcacagttggtggtggcgcactttgcttctgacggcgcgggggccgcttgtcccattgacgccatcacgctgcgtacaatttcttcaatctgtttttgatccatgatatgttatctccgcgtcatcagaagaacagtgacggatcgcccgcccgtttggtcaggcgaccgtttgccataatgcccatgctttccagccagcgttcaaactccggtgacgggcgcaggttgagtaactgacgcacagtggcggtatcgtggaatgcggtggtctggtagttgagcatgatgtcatcacccagcggcatccccatgatgtagttgcagcctgcggtggcgagcaggatcatcaggttttcgttgaggttctggtcagcgtcagcgtggttggtataacagcagtcacagcccatagagatgccgctcagcttgcccataaagtgatcttctaagccagcacggataatctggcggtcgttgtagagatactccggcccaataaagccgaccacggtgttgacgataaacggatcgtaatgacgcgccagcccgtagttacgtgcttccatcgttacctggtctgcgccgaagttagcgccagcggatagcgcagagccttgtccggtttcgaagtagaggcagttttccccggcgatacggttgaactccgcgcccactgcgcgcgcttcgtcgagcatcgccagctccacgccaaactctttcagccctttttcgctgccacagatactctggaaaatcagcccgcccggtgcgccacgacggatcgcttcgatctgggtggtgacgtgcgccagtacacagccctgagttgggatgttgaatttgtcgatcacgccatagatggtatccaacacgcggcttaagttttccacgtcgtcagtcaccgggttaacgccgatcaccgcatcgcccaccccgaaggaaagcccttcgtagatttgcgcggcgatactttgcacgtcgtcacgggtgtcatttggctgcaaacgggcgctaaaggtgcccggaataccgatggtggtattggcctttttgattaccggcattttcttcgcgccgtagatcaggtccgcgttggagcaaatcttcgctaccgccgcgaccacttccgaggtcagccctttgcgggtaaaggcaatgtcgtccacgctggtttcatcgctcagcacatactcacgcagttcgctgatgctccagtttttaatctggttgtaggccgtttcgttaacatcgtcctgaatcagccgcgtcacgcagtcatcttcataggcaatcaccggattattgcggatgtccgctacggtcatttccgacaacacctgctttgccgccacgcgctcctgtgagcttgccgctgcgacgcccgccagcacatcccccgaacgcagttcgttggctttagccagcacctcttttacatccttaaactgatatacattgccgaacaatgtggtctttagtttcataagtcgttccctcaggaagaatcgatgattggcatttttcacagcattctaacaatcacgtttcatcgtcagcccttgtcgtgtaaggtggttgcctaaacacgcccgttattcatcacgccgaacgcgccggatacatgatcggggttatccagtcgttaaatcaaggtatccggttttgagcaagacaccactcacagcaaaggccatagacgccgcacagccgcaggacaagccctataaactcaccgattcactgacgccggggctgtttttgctggtgcatcccaacggttcgaaatactggcgattcaggtattggctgaataaacgagagtttttgcaggccattggagtttacccgctaatcacactcaaagaagcacgcaggcgcgccacggagagcagatcccttattgccaatggaattaacccagtggaacaagcccgcaaggaaaaagccattgatgcgctcaacatggcggcaggatttaagaaggtggcggaagactggtttgctaccagggttggagggtggtcggaatcctatgcaaaacaggtcagatcggcactagaaaaagacgtctatccggtacttggcaagcggtcgattgtcgatataaccgcccgtgacgtgctggcattactccagaagaaagaacgtaccgcaccggagcaggcccgcaagctacgccggcgcatcggtgagatcttcaagtttgccgttatcaccgaactggtaacgaggaatccggttgcagatcttgatacggcactgaaggcccgccgacctggtcacaacgcgtggataccgattagtgaaattccggccttctacaaagcccttgagagggccgggagcgtccagattcagacggcaatacgtttgcttatattaacggcattaaggaccgcagaactgcgtttgtgccgttgggaatggataaacctggaggacgcaacaatcacattgcccgctgaagtcatgaaggcccgccgcccgcatgtggtcccgctatcacggcaggcggtcgagctattgcaggaccagttcacacgcagcggatacagtgctttcgtctttccaggccgattcatggataaacccttgtcagccagcgcgatacttaaagcgcttgagcgtatcgggtacaagtcgatagccacaggccacggctggcgcacaacgttcagcaccgcacttaacgaatcaggcagatactcgccggattggattgagatccaactagcccacgtcccgaagggaataaggggcgtttataaccaggctgcctacctgaagcaacggcgagcaatgatgcaggattacgccgacgctattgattcaatattggcaggtaacggcaatcctctagaaccggaatgaataattaagcggcttttttgcaaagcgcaattttgcattttgtataagtatttgttttgtgtggtttaactatcacctgataagaaacctgtattcaatttgccggattcgtccggcttttctttttcgctaattattccattattccaattaagtggaataaattattcaatatcaagaacttaaatccatgtttgcaacgaaagatccagagttcgaaaataggatcaacacaaataaaagcccccggaatgctgcaacatgccgggggcggtatgagaaacaagctaaaggagaatttctcatgtctgatatgctagcagtagaacaagaaacaaacaatgatgttcgtcaatttttaaacaaaattaacgagttacggaataaagcacccaaaaacgaagagactaaacacgaagaacacacgccagataatcacgaggaaacagatcatcacgaggcaaaacagcaggagcaagcctggcgtggcaacctgcgctacctggacacattaaaccgacttgatgaagtattgccccgcaaactgtacgaaagatgggagaaagaacatacagtcaacgacgaggctgtgctacgtgctctttgttacttcgctggtactggcaaaaactcacagttgggatggtgcagggttggtaggggaacaatcgacaaacgagccaggctatcaaaaaacacggttaaaaaatgcctcgatcgtctggtcaaccacttcaaacttgttgagcgtactgaaggctatataccaggatcggcagaaagggagtgcaacgaataccagttattattcaagccgtacaacatgaaataacggaatcaggcgggcaatgttcccgccttttctttgccttaattccatgaattcaggtgggtcaaaagttgccgttagtggtgggtcaaaagttgccgttaaggtgggtcaaaagttgccgttaaggtgggtcaaaagttgccgagtaagaattctactattaagaattctaggcgacgggagttttttagcctcccggtcggtcatagagagtcgcctagagttaaacagaagaattatttcgccgcctgataggtcggctggttgcgagcattaaccatgctgattagcgcaatcatttccagcaagctggaaacgcccattcactcacgcacaacctgaacagcagaccaacaaaccatcatggcattcgttcatggggagcgcggtatatctcaaagggtgatttcttattggtgggccttcggaaggcttcgagcaattgccagcttaaaagacgggcttagcagtgatggttatccgccacgaatgtccgtcatattgcattgcgcagaaacgcgtggcactgagggagttttccgaattagttttggggaccctttccctgcttctggagcaaaagacgaacggcaaatgcagtgcttccttgtacgactgcagcgaagaagaaaagctgtttgttaagcgcctgaagttaatcaaagcggatatccacgcccagctgaaggcctgtgattgcgatatttctgaatgacaggtggaatcatgaaacacgtttttaaatatcttgattttgcagaagaccgcgaacacgcagaatcagtggcgaccaaagagttaaaactggaccacgtagaaaaattcgctatccgcgatctagccaatgatatcaaagagcgtgggtgtgttgagcttgtccagcctggtggattcgatgagctggttcagatctatgaggccggaggcgatggaatagagccactcaattgtggaatcgaatcaaggaaggtggcaattgctgccctgcttcgcgtcatgcgtgaaccagactttcaatgcctggaaatggttcacgaaatcataagaattgctagagatttggaagcgccagttgacgctccgttagattgctaacgccaaaattagcgctgaattaatgggtaattattgcggtttttgtcaattttcaacctcaattcttgcgaaaaatggcaaaaataacggtatttttcatcatttattgggggttttatggaaggcgaactgatagaaaacaatgggttagacatttatgacaccagcgaaacaccgaaaaagcgcggtcggccagctaaatataatgaaaaaatagcaacgcaaatcgtcctattggtaagcgaaggttatagtttgcgcaagatcagcatgatgccagggatgccgagccaccgtcagatgatgcgctggcaactggagcatatggacttcagggaagggatagcctggatgtcgtggctatggtgcgctgaagctggccgacgtgccgtcgagataatcgacgaggttgatataaacgcagaggatgggccgaagcagttgcgcaaagcagaagcaaaggcaaaggcactactggcagcagccaagctgaatagtttgaaacattcaccatttggagatgacaaacaatgagcctgatccgcactgaaaccagagacacaaaacgcgcagctgacccactgcacgacctgcgtagcaagccgttttctgagtggggcgaagatgaaatcaggcgttttaatctgatagacgcgcttcttgagtttgtctacacagacacatccagcccgttcggtatcggcatgaccttcgattacacggagtgctgggaaattggtgttcgtgacgactgcctggtaatgacacgcgttaagccggtgcatccagaatatgcgaagcactggaacatgaaaggcgtcatgaatgacaaaacccgcttccacgccgacaagtgggtagggtacagcaaggtgcttgcctgggtgagcttatcgcacaaagacaccttcacgggtgcgaaacggtttcaatacttccaaacgatgtacgacatggaacggcaaatcaacgcaaacctgccggttggcggccttcccaacgttgacacagagcgaactggcaaactgttccaacgcgatgacttttctgaggatagccatgccaacgatccgaagttggttggtgatgattacgtcccccaggcaccggagcaaatcaactgaattttcggacaaacgcgcgcgtagccgacgtcagcggcaagactggcggtcatttccccgctcctacgcgaaaaatccctcacaactaccctgcaaattttccagatttcacgtacacgcgccaaaaataaaggcccaggcagttagcaacctacccgggcctttctcacaatccccgctgacattatatcacccatctttccgttttcaggtgggagactgatggccgccgacgttgcacaattgattaatttctgaacattcaaatcaactcccaccaaagccaacaagatgggaggtgaattttgtgatgcagatcgctttttcccttcaggcatttttgtttaattcaatcaacgaaaggcagttcccaacaacaaaataaagatgggaggtaaaaatgaaacggtgggaagtggctttactggtgatggtaatgttggtttgctgtattgaactgtgaaggaggacgccatgaaacttttaatcgcaatcatcctgatggtgctgactggtgtttgctttgcagatgttggtgattacaggctgaacggggaggataacgcaagaattgaatcagtcgttactgataactgtgaaaaaacagccgtattggtaggcggtgacaggcttgcgagggttgagatcgaatatatagcgacattgtgcaagccggtggctttggtgattatttacgacagatttgacgatatagcggcaatccctcttaaggtgacgttgaaaaaggtattgaaagagaatagcgatgaaaagattaacctattgaacaagatgggggatctggctggtcgtatcgttgcagagcagtatttaggcatgagttttgagtaaggaggcaatcatgaaagtgttaggtaatattttatggtgggcttttgttggtttcatggcttacgccactttgattaagccggacaacactgatccagctgttgtgaactatgaagagcctttgcctatggagcttgccaactatggcgaaccaggtgaaggggcgaaaatcatgaatgccgcaaaaataatgggtcgcgactacgcatggaaacatgtaaaagaagacaggttgccatgtctgtttgccgccggggttgttgctgataacatcctggtaaaataccatttcagcaatgaaactgagttcaaacttaaagcggcagcggtcagagaatgcgccaacgtagcagaaaacaacggctttgttttggtaggtagagtatttgaaaaacgtaattgattgcgaatagcaacaactaaacaaccaatacacccggcccctcgccgggttttttgtgatctgcgtcaatattcccttccgttacgcttaccctccaccaatacgcgtgttaacctcccaatggattctatgagatgggagataaaaatcatgagttacgaaatcaaaatttgcgacatcctcaaaggcgctgcgatggaaggacaatataagggcgctcaacgtggggccaaatgcgaggagatcgcaaacgagttaactcgccggggagttaaaaacaacaagggagaggttattactaagggcggcgttagccattggctggaaggtagacgggagccaaatttcgacactctggctgaactgtgcgacatgttcggcgtttatgccctgatgccgatgcgtggcggtaaatggattcgagttcacccggaagaccgtggagaaatggaattacgcgaggctgtagctgaacgagatgctattatcgacgacctgaaggcccgtatcgctgagcttgaggcggcactagcaaataaacaagtcccagcagaagcggaagagatgggaggtgaaaaagtggaagaagtggcagcagagcaagcgcccaacgatgaaaaagagatgggagctaaggagtgggttaacccgaacccgaaaaaatacagcgtcggcatgttgtgtcaggtactggctgcaatgggcggcgaatacctgggcaacaacgcagggttacagcagaagatcactgtgttggataacgacggcaaccggaagccaatcagtaacggcgcgttttatcgactgattgagcaggccaaagggagaggattgattagcgttgaacaggaaatcaaacacaagaaagacgaaaacggcaaccagatcggcaaaggcaagaaaggtgacaagctgataactttgcttcccaactggattgataagctgggagacgaataaaccagccttcaaccccatctcatcaatcaacgcccggccccgctgccgggtttttgctatgcaccacaattaccccaaccggatacacagccggatacaattccaccagcacccagccacccagcgccaccgctggcgaataccgcattcaggaaggaaatgcgagtgatttcaccgtcaccggcacaaccgatccgccaaaaagaggcgtaccaatgtcgatatagtcccccgcgcggacaatcacttcgtcaatgactgccaacgggagttgttgtagctgtgggcgcaacaacatgcccagagctttaccaaagtcctgcccggccaccaccagcaggggatgcggattcggaaaacgcgcgacgaaatcgaccaacgcgttgatgaccgtcagtaccgcggcgtaacgcacaggcagcgaggcgggaagcgccagcacgtacgcgtcagttttgggatcaagatccagctgaatcagcgcctgttgccaggcccccaccagatccgtttcatcaatcgggatcgccaccggcaaattgcgcagcggcagttgtacgccctcaagccagattgtgctgccagagagcgaaagggtatgcgcgcccgcgccaatcaccgtggcgcgcacggtttgcgccggaaactgtacgttcatctcacgcaggcgcggatggtcatgcagcgcagttgccagcagcgggccaatatcggcaaaacagaacgggtcggcgggctggtggcgataacattcgcccacgccgccagaaagcgtaatgatttcgggcgtaacacctgcgggcagcaaaccggtttgcatcaatgcctgcgcgagcggtgagagcgttccgtcaatcacttcgacaatcagttctgccatccgccgggtcacctgcaccagctgcgcgccggtcagcgaacgggcgtcggtgcctgcaccgaagcactcatccacaatcatctgccccggtttatgagcgtaaaccacgcgcccgtggctgtcggtttccagcaggcgaccaccgacgttgaggcaggcagtgccgctgatttttccggcatcgaacagggcgtagttcgcggtgccaccgccgatgtcgatattcagtacccgacacagccgttgttcagaaagggtttgtgccccggctccgtgaccggcgatcacggattcgaggtgcggcccggcgctggcaacgacaaaatcgcccagcgactgagagagcgccatcaccgccgggcgagcattgcgggttttcgcgctttcaccggtgatgatgatggcaccagaatcaacgctttccggctcaatacccgcagcatgatattgctcgagtattaaggttttcagttccgcttcttttaaaccgccctgtttatcgacaggggtaaagaacaccggactttgccagctaatttcgcgtttaatgaattcgtagcgcggcacctgcgacaccgccgcacggttaaccagctccagccgggagaaaatcacctgggtggtggtggtgccgatatcgataccgacgctcaatagctggcgagtgttcacgattgtgcctccgcttcggttttagtcgcggtcgcgtcttcttttggcaccagcatcatcgccacgccaatcgccgttacgccgccgatcaacttgccgacaatcatcgggaagatcatggcgttcatgttggcagcggcgaagcctaagtggtcgcccagggcgaaagcagcggaaacggcgaaggcgcagttgatgactttgccgcgggtatccatctgcttcatcatgccgaacatcgggatgttgttggcaagcgttgccaccatgccggctgccgcgatgttgttcatattcagtactttaccgacgctcatcagcggtttttcaaaccagcgagtcagcagcagcaccatcggatacgcccctaacagaacgcaggagatagaaccgataacttcaatggcgcgcatcacctcaccgggtttatcgccaggggccataaagataggatccagaccggggatcagttcccagccaagcaggaatttcactaccgcagcggcaagaccgagggtgatcaatgcaacgaggaatttggcgaagatctggaagccgttgatcattttttccgggatgaatttcagccccagcgccaccagaatcgcaacaatgatcaccgggatcatgttcatcaggatcagggcgaaagtgaattccaccggctggccgttgatctgcacaccggagtacatagcaaccagaccaccagcgatacaaccaatcggaatggtcacaatgcccgccagcacgccgagcgccagataacgacggtcagaaggttcgataatgccgagcgccaccggaatggaaaacacaatcgttggccccatcatcgacccgagaattaacccagagtatagccacgcggctacgtcgccgcccgccagctctttggcgaggaagaagccgcccatatcgcacgccagcagtgttccggcgaacatcgatgggttagcgccgagcatttcgtaaaccggaataattaccggcccgagaacgtgagccagtaccggtgccagcgcggtcataccgaccatcgccaggcccagtgcgcccattgccataaagccttcttcgaactgaccgcctgatccttcgatacttttaccgaacttaccgaggaaacgagcagaaccgccgaactgcgacaggatcctgtctacggcagctatcagcataaagaacatcatgatgtacatgatgatttcgttaattcccatcgcctttactccctgttagttgttatttattggcggatgcggcgtaaacgccttatccgccctacatgtgcaatcccgtaggctggataagacgcggcaagcgtcgcatccggcaattgcaccgcgccactggcggatgcggcgtgaacgccttatccgccctacatgtgcaatcccgtaggctggataagatgcggcaagcgtcgcatccggcatttattgcgccgctgcgtacaggccgacaatctgctccaggctggcggtacgcgggttactgcgcagacaaatatcttccagcgcggcctgcgcccatgcgccgtaatgcgcagatgtcgcaccaacatcgcccagtcgtttaccaatcccaacttccgcaatcagctcacttaccgcgttaatagcgtcacgatcgtcggattttttagttcgcagtgcccgaccaatctgactaaagcgttcacgacaaaccatccggttaaattccatcaccgttggcagcaacatggcgttcgcgagaccgtgcggaatatgcagcgccgcgcccggctgatgcgccatcgcgtggcacaacccaagacccgcactggaaaacgccattcccgccatacatgaagccagcaacatgctctcgcgcgcggcaaggtcgtgaccgtagcccaccgctttcggcagcgatttgccaatcatcgcaatggcaccaatcgccagactgtcggtaaacggtgtagcgttcagggcgctgtatgcttcaatggcatgggttaacgcatcaatgccggtcatcgccgtgacatgcgacggcacaccttcggtcaatgcggcgtcgaggatcgccacatccggcatcagcgaggcatgggctaacacctgcttgcgcccgctcaccgcgtcgataatcaccgttacattggtggtttcagagccggttccggcggtagttggaatggcaatcagcggcaagcgcggttgcagaacgctggtttctgacatctctgccagcgtgctatccgggttcgtcaccagcaacgtcacggctttcgccgcatccagcaccgagccgccgccaaacgcgatcaccccatcacagcctgactcacgcaactgcgccacggctgcacacacgtcggtaatgcacggttcgcccaccggacatggccagagcgtcatggcgatacctttaacggtcaggctacgcgtcagcccggcggtcatccctgcctgatgcaaaaagctgtctgccatcacgaacagatgtttcagcccacgcgtttgcgcttgctgtccgcaactgctcaccgagcccggaccgcaaagcgtcaccggtggaacgctaaatgtttttacccgttgcagattcagggtatcgaacgcctgaaagagcgcggtctgcaattcattttgcatatagcccctccgctttctctcgcccactactggcgatcgccagcggggtcataaacaaactgtgctgcggtaaatgcacctgtaacgccgggaattgtttgcgaaacagttccgccacgcccggttgcatacaagagccgcccgccagccataaatcagtaatgccctgcccttcaatatgccgggcgacaatgtccgccattttttcgtacaccggtttcaccgcaggccaaatctcttcaccgtgaccgcgcttgtactgctccgcctcttccagcgaaatacggcgatttccggcgagagtcagagagatgtgatgtccgccggtggcttcatccgccgagtacgtcaccttgccctttttcacgatggcaatgccggtagtgccgccgccgatatccactacaccggcgttgtccagttgcagcagatccgcaactgcggttggctcatccagcacatggctcacttccagtccggcagattccagcacgttgatggaaatacgcgggtccgtacctggaggaaatgaagtcgccgcatggctaaaacgacgaccgaattgctgctcgagcgtgtcgagatggcgacgaacaatggtgacagcgccgaagaaatcccagacgatgccgtcgcgaaccacatcggcccagtcgaggcataccgccactggctgaccgtcgcggtcgacaaccatcgacaccacatcgcaggtgcccagatccacccccagccacagcggagattccgtcgcggcgggcgtctggttacacagcgttgccgccgtttgcagacgtggggtgagccattgttcgtcgtgcgccatctgttactccttaaacaatgcgaaacgcatcgactaatacacagcgacgcagacggacaaacgtacgcgcgctggttaccccttcaccggttggcgtggtgatggtcatggtggtccagccttccccgcccagccccagcccggcaatgcacggtccgttcttaacgaaaatgctggtatcaatagcattcgccatctggttcatgttttcgatgttgcgcgagtgcattgccgccgtgtggtggcaaccgccttccagtttcaccgctagcgcaatggcatccgccacgttggcgacgcgcacgacgggcaacaccggcatcatcagttcagtcacggcaaacggatgttctgcggtggtttccacaaacagcaggcgcgtttcttgcggaactttaaggccgattgccgccgcgattttgcctgcgtcgcgaccaacccagtcacggctgacggtgccttttccgcgctcgtcgatatttttcagcaacaccggttgcagctgctgcgcctgttctgcggtcagtttcaccgcgtgctggccttccatcagacgcatcagttcatcggctacgctatcaacaacaatcagtaccttttcgtcggcacaaatgatgttgttatcgaaagaagcgcctttgacgatggactgagcggcacgggcgaggtcggcggtttcatccaccactaccggcgggttgccagcgcctgcggcaatcagacgtttattggtgtgtttacgcgccgcttctactaccgcttcgccgccggttaccaccagcaggccgatacccggaaacttgaacaagcgttgcgcggtttcgatatccggatttgccacagtaaccagtaagttttccggcccacctgcggcaacaatcgcctggttgagcagcgtaatcgcccgctgggagacttttttcgccgccggatgcggggcaaaaatgacgctgttgcccgcggcaatcaggctgatggcgttgttaattacggttgccgccgggttagtggaaggcgtcaccgaagccaccacgccccagggtgcgttttcaattagggtcaggccgttgtcgccagtcagcacttgcggagagaggcactcaacgcctggtgtgccgcgcgcctgagcgacgttttttgcaaatttatcttcaacgcgccccatgccggtttcactgacggcaagttccgctaaatctctggcgtgtttttcgcctgcttcacgaatggcagcaatggctaactggcgcattgccacgctttttaacccttgctgggcgactttggctgccgcaacggcgtcatccagggacgcgaaaacgcccatctcatgaacggcggcggacggcgtgtcactgctttgcattttcagcagtaccgctttcaccacctgttcaatatcctgttgattcatgatgttctgccttatttgtggaaaattacctgaccgccagacaccacctcatcgacaatgccaatcacgcacagatcgaccggtgacgtttcgcttttatgcgcctggcgggcggaactgccactcaccagtaacacccactccccggttcccgcgccaatattgtcgatggcgacggcgcattgcccgtcaggattaccttgtggatcaatcatttccaccatcagcaatttgtcatgcgccagtccgtgatggcgtacggtacaaacaatttgtccagtgacgactgccagtttcatacccgcctccgtggcgtatttcaggtaaaagctccccctaccctccgcagaaggtaaaatgaaaaaggagagagcgtgacgcccgaatcgacgtcacacagggtgattacaggttgctgctatcgcctttcaggccgatcgggaagacttcttccaggtcgccgtgcggacgcgggataacgtgtacagataccagctcgccgatacgctgtgccgctgcggcacctgcatcggtcgcggctttacaggctgcaacatcaccacgaaccatggcagtacacaggccgccgccaatctgcttaacaccaaccagcttgacgcgcgcagctttcaccatcgcgtcagaagcctcaatcagtgcaaccaggccccgggtttcgatcattcctaatgcttccattgtgctttcctctttatcagggtccagaacgggaccgttcattcaaccagtgtttgtaaactgctttcgcggttcacttctgtctgacgcggcacagctgccaccagcgccagctcgataatttcctgcacgctacaaccacgagagagatcgtgcatcggcgcggcaagtccttgtatcagtggcccgacggcacgatatccgccgagtcgttgtgcgattttgtaaccaatatttccggcttccagcgacggaaaaaccatcacattggccttgccctgtagcgggctggcaggcgctttttgcgccgccacttccggcacgaaggcggcgtcaaactgtaactcgccatccaccaccagctttggtgcgcgctcacggacgatttctgtcgcctgctggacgttagcaacacaggggtgacgggcgctaccattgctggaaaacgacagcatcgccacgcgcggctcttctccggtgatggcgcgccaggtttcggcactggcaagcgcgatatccgccagctgcgccgccgtcggctgtggcaccacgctgcaatcggcaaagcccaacgccgggccgctgtactgtggcaacatcaggaaaatggaagagagcgttttacagcctggctgcaagccgataatgcgtaatccggcacgcagcacatttgccgtggaagagaggttgcccgcgatacagacatccgctttaccggcgctgaccattgctgcggcgaacatcagagggtcggtaagtttttccagcgcatccggcggcgttttttcgcccgcgcgggccagccagcgatgagcaaattcttcccgcattgcgaggttgccatgcggatcaatcacctgtagcccgtccatcgccacgccgtgactgagcgcaaactgacgaagttcaaacggattggcgaccagaatgggcgttgccagaccttgttgatgtaaatattgcgcggctttcagcacacgttggtctaacgcatccggaaaaaccactctggcgggcgctcgcaacgccagttcacgacaacgttcaataatcattgcgtttcccccagtcgttgttggatctgcttcaccgttagcggctgcttcgttacgctcaggatcatcatcacgtagaccgtgctcgaaaggcggttcagcgcctgcaaaatgtccgggcgtaatacttcaaagctgcgggtgataaagacctgcgccgctacggtttcggtttcccgcactttggtgcgtagcagattgagcaacgcagcatcgcgcccgtggctggcttccggcaccagatgatcgtggtcgagatagcgcagcggctgatgagaaagccgatgcagatcttcgtcagaaagcccgacaatcgcctggcagcccagcggttcccccagcgcatcggcgcgcataatgttgccaagacgcgaacggatatccgccagccacggctgccacggttccgccagttcaatttgcagccacactgccagcgcaatggtgctgtcgagaaccgcgcgaaaacccagacgcggatcgcttttggcgaccattttttccgccgacaggtgagtcagcgtatccggcttttttgccaccggctggcgacacagttcgcagcacgcctgcggatgttcatcgctactggtcagcccatgaacgggctgcggctgctgctgttcatcgtcaacaaacaggcggccctgctcgtcaataaacttgatgcgcagatggcggctttccagcaactcccgggcagagggcgtcaggcgactgtccgcagggagatggatctctgcgccttcgctgagcgtatggttcgctcttagccatgcttcggtgatgaaatctttcatagggattgccagttagccggccaggcgacatacaggaatttcacgctggatgtcgtaccaaattcgatgctggagcctttcgggataaacatcacgtcgcctgctttggcgatcatggtttggccttcgtggcgaacatgcagctccccttccagcaccatgtcgatttcgtcgtagttcagggtccacgggaagaatgcgttctcccactgcataaaaccggcggccatgctgctgccgtcgtctccggtcacaagatcagtcaagcccacgcaatgcggctctgcgccgtcgaaacgaccaaacttgacgctactgccatcaatcactttgatgccgcctttgccggtcaccgatttgaagctcggctgcattgcgccctgctccagcgactgtttttccttcatcactttttccatcagctgtgcgaccaggctttcggtaaactggccttccggcagctgggcaatgatggtttcgcggatgcgctggctttcggttttgtcggctggcacgctggcgggcacggacgccgttaccgggatcgattcatcacattcggtgatggtaaaacccagtagatccgccacttcacgggcttccggggtaataatgctggcgcgcagaaccacggacattgcctgttcgccgcgcgcgtgtgcttcacgaatatcattcgctgtgatgagttttttcacctgcttcctcctgtttggtgagagatgccagataatccaccagttgctgcacgctttgcgggtcgtggctgtttagctcgaacatcggctcttcgaaacccgtctcaagcaataactttcgcgttgcggcgacgtcagcatctggcatgtccgttttactgatgacggcgatttgccgtttgctgacgccaatatccagcaacccggcaggcaaccgactttccgggtcatttgcgccatggacatagatcagcatgtctacatcctgtagcgtggtaattaaggcgtgataccagcggggatggttaaaatattcacccggcgtatcaatatcgcccttatcattaaattccacggcctgtgtttttctggcgagggtataattcccctgcaacgcattaaataacgttgtttttcctgccccgacgctacccacaaacgcaattcgtttcatgaatgcctcgtattaacttttggtcatttcacaaagcgtataatttaataagcgacctaaaccgctgacggtttgtgataacgcttcttctactgcgcccaccgagccataaatcaccaatgcaccgctgaatcggtcgagaaaaccgatatgcacatcagcggctttcagcgctaaatcaccggcgatcatcgccgtttcgccgggagttagcgtcataatgccaattgcgcccgcatccggaacgccgattttcttcgccagttcctcaccgggatgcgcgatgagatgcgccagtgtgacctgtttgccgggcacaaattcctgaatgatgcgttctttatccatgagtcgccgcctgtgaaaaactttcgtgtatcgtgacaatttttcgtcagagtaaataacaaaattcggcaagcgcgtttaaaaggtgaggtagatcactaagaatggagagatattcgctgtggtgcataaactttcatatgcaacgcatgaatataaataaaataatatcgagatattatatagactgcttttttttattattcgcaaactcagtaataagctttactaatatattgcagctaaactgcttaccctgaatattcagggtaagcgtgagagttaaaaaaaattacagcggttgggtttgcgcttctaccacggccagcgccaccatgttgacgatacgacgcaccgatgcgatcggcgttaacacgtgaaccggtttcgccacacccatcagcaccgggccgacagtcacaccttccgagctggaaacacgcagtaagttgtaactaatgcgggcagcttccatgttcggcatcaccagaatattggcggaacctttcaaagagctgtccggcatacggtcgttgcgaatcgcttccaccagcgctgcatcgccgtgcatttcaccatcaatcatcagttctggtgcacgttccctgaccagttccagcgcctgacgcattttgctcgacgacgggcagtcagaagaaccaaagttggagtgcgacaacaaagcaacgcgcggctcaataccaaaacgacggacagtttctgccgccatcaaggtgatctccgccagctcttctgcatccggttcatcattaacatatgtatcggcaataaaggtgttaccactcggcagcagcagcgcgttcatggcacctgcggtgtgaacgccatcgcgataaccaaagacatttttcaccacgctaaaatgttcatgataatcacccaccgtaccgcaaatcattgcatcggcttccccacgctgaaccatgatcgcgccgatcactgtcgggttactgatcagcgcccgctgcgcctgttcctgagtgacgccgcgacgcttcatgatctggaagtattcggtccagtactctttaaagcgcggatcggattcgttattgacgatctcaaaatcaacgcccgctttgatctgcaagcccagtttctgaatgcgcatttcgatcacgttcggacgaccgataaggatcggtttcgccagtcccagcgttaccagttcctgagtggcatgcagaacgcgcgcctcttccccttccggcagaacaacgcgcttcggcgctttgcgagcctgggagaaaatcggcttcataaacaggttggttttgtaaacgaactcagtcagcttgtcgatgtagacgtcgaaatcagcaatcggacgagtcgccacgcccgactccatcgcggctttagcgaccgcaggagcgatcttaacgatcaagcgcggatcaaacggttttggaatgatgtattccggaccaaagctcagatcctgatcgccatacgctgaagccaccacttcgctctgttccgcatgggcgagttctgcaatcgcacgtaccgccgccagtttcatctcttcgttgatggcggttgcgccaacgtccagcgcgccacggaagatgaacgggaagcacaggacgttgttcacctggttcggatagtcagaacgaccggtgcaaatgatggcatccggacgcacttctttcgccagcggcggcagaatttccggttccgggttcgccagcgccaggatcattggcgcacgagccattttcttcaccatttcctgggtcagcactttcgggccggaacagcccaggaaaatatccgcgccttcaatcacatcatcgagggtacgtttgccgtcatccaccaccgcatatgcggctttggtttccgccatgtttggctcacggccctgatagataacgccttttgaatcgcaaaccacgatgttatgtttttgcagacccagcgctaccagcaggttcatacaggcgattgctgcggcacccgcgccggaaaccaccatccgcacgtcggagatgtttttctccaccacgcgcaagccgttgaggatggcggcagtgctgataattgccgtgccgtgctgatcgtcgtggaataccggaatattcatccgctcgcgcagtttctgttcaatatagaaacattctggcgctttaatgtcttcgaggttgatgccgccgaaggttggttcgagcgcggcgacaacttcaataaatttgtccgggtcgagttcgtcaacttcaatgtcaaatacatcaatcccggcgaatttcttaaacagaacgcccttgccttccatcaccggtttgcctgccagcgcgccaatgttgcctaaccccagcaccgccgtaccgttagagatcaccgccaccaggttacctcgggcggtatatttgtaggcttttaacgggtctttttcgatttcaagacaaggtgcggcaacgcctggtgagtaggccagcgccagatcgcgctgtgttgccagaggcttggttggagaaacctggattttccctggaactggaaattcatggaaatcaagtgcactttgttttaactggtcatccatttggttgttcctttcacgtaacgttcacaaataaagtgtgtgggcaacagcccctgcccacaacgtggcgcacattattaccctgccggagtctacagactttgagcaagtccaaactctcaccattaatataatgttttggtaataatcctataacactgatgttacctgcttaatccagcaataccatgcctgtctgctatgcttttttgatgcgtttagcgaaatttctcagaagtgtgaattaacgcactcatctaacactttacttttcaaggagtatttcctatgaacgagttagacggcatcaaacagttcaccactgtcgtggcagacagcggcgatattgagtccattcgccattatcatccccaggatgccaccaccaatccttcgctgttactcaaagctgccggattatcacaatatgagcatttaatagacgatgctatcgcctggggtaaaaaaaatggcaagacccaggaacaacaggtggtcgcagcgtgtgacaaactggcggtcaatttcggtgctgaaatcctcaaaatcgtacccggtcgcgtgtcaacagaagttgatgcacgcctctcttttgataaagaaaagagtattgagaaggcgcgccatctggtggacttgtatcagcaacaaggcgttgagaaatcacgcattctgatcaagctggcttcgacctgggaaggaattcgcgcggcagaagagctggaaaaagaaggtattaactgcaacctgacgctgctgttttcttttgcacaggcacgggcctgtgcggaagcaggcgtttttctgatttcgccgtttgtcgggcgtatttatgactggtatcaggcacgcaagccgatggacccgtatgtggtggaagaagatccgggcgttaaatcggtgcgcaatatctacgactactataagcaacaccactatgaaaccattgtgatgggcgcgagcttccgtcgcaccgaacaaatcctcgccttaaccggctgcgatcgactgactatcgcaccgaatttactgaaggagctgcaggaaaaagtttcgccagtggtacgtaaattaatcccaccttctcagacgttcccacgcccagctcccatgagcgaagcggagttccgttgggagcacaatcaggatgcgatggcggtagaaaaactgtctgaaggcattcgtctgttcgccgttgatcaacgcaaactggaagatcttcttgccgccaaactataaaccagccacggagtgttatatgtcccgaaaagaccttgccaatgcgattcgcgcactcagtatggatgcggtacaaaaagccaactctggtcatcccggcgcgccgatgggcatggctgatattgccgaagtgctgtggaacgattttcttaaacataaccctaccgacccaacctggtatgatcgcgaccgctttattctttccaacggtcacgcgtcgatgctgctctacagtttgctacatctgaccggttacgacctgccgctggaagaactgaagaacttccgtcagttgcattcgaaaaccccaggccacccggagattggctatacgccaggcgttgaaaccaccaccggcccgcttggacaaggtttggcgaacgccgtcgggctggcgatagcagagcgtacactggcggcgcagtttaaccagccagaccatgagatcgtcgatcacttcacctatgtgtttatgggcgacggctgcctgatggaaggtatttcccacgaagtctgttcgctggcaggcacgctgggactgggcaagctgattggtttttacgatcacaacggtatttccatcgacggtgaaacagaaggctggtttaccgacgatacggcaaaacgttttgaagcctatcactggcatgtgatccatgaaatcgacggtcacgatccgcaggcggtgaaggaagcgatccttgaagcgcaaagcgtgaaagataagccgtcgctgattatctgccgtacggtgattggctttggttcgccgaataaagcaggtaaggaagaggcgcacggcgcaccactgggggaagaagaagtggcgctggcacggcaaaaactgggctggcaccatccgccatttgagatccctaaagagatttatcacgcctgggatgcccgtgaaaaaggcgaaaaagcgcagcagagctggaatgagaagtttgccgcctataaaaaggctcatccgcaactggcagaagagtttacccgacggatgagcggtggtttaccgaaggactgggagaaaacgactcagaaatatatcaatgagttacaggcaaatccggcgaaaatcgctacccgtaaggcttcgcaaaatacgcttaacgcttacgggccgatgctgcctgagttgctcggcggttcggcggatctggctcccagcaacctgaccatctggaaaggttctgtttcgctgaaggaagatccagcgggcaactacattcactacggggtgcgtgaatttggcatgaccgctatcgccaacggcatcgcgcaccacggcggctttgtgccgtataccgcgacgttcctgatgtttgttgaatacgcccgtaacgccgcgcggatggcggcactgatgaaagcgcggcagattatggtttatacccacgactcaattggcctgggcgaagatggtccgacgcaccaggctgttgagcaactggccagcctgcgcttaacgccaaatttcagcacctggcgaccgtgcgatcaggtggaagcggcggtgggctggaagctggcggttgagcgccacaacggaccgacggcactgatcctctcaaggcagaatctggcccaggtggaacgtacgccggatcaggttaaagagattgctcgtggcggttatgtgctgaaagacagcggcggtaagccagatattattctgattgccaccggttcagagatggaaattaccctgcaagcggcagagaaattagcaggagaaggtcgcaatgtacgcgtagtttccctgccctcgaccgatattttcgacgcccaggatgaggaatatcgggagtcggtgttgccttctaacgttgcggctcgcgtggcggtggaagcaggtattgccgattactggtacaagtatgttggtctgaaaggggcaattgtcgggatgacgggttacggggaatctgctccggcggataagctgttcccgttctttggctttaccgccgagaatattgtggcaaaagcgcataaggtgctgggagtgaaaggtgcctgatggtgattgccggatgctgattgccggatgcgacgctgacgcgtcttatccggcctacagcgtcttatccggcctacatgtcccgccattttgtttaacgggtgatccacaacgtgggccaggcgtctggcccatgccagttatcgcaggtgggttctgcggcgtaacgcaccaggcgaaaacgctgaccgtcaaagcgccagcgcgcctgaatgccacaatcgcttaatccgcgccctttcgctaaggtcaccagttcacgcgatttctcatcaaatgttgcgttcatcagttccagttcattcgtctcctgaccgttgttgaacggcaaacgcaaccgaaccgggcgcgaagctagtggctttttacgcgacacaatccatgccaaatcaatggtgttataggcccctgcctcacagctaatcatcatcagcgctttatcatcagtcagcgcagtgacattcacctcacgacgcaatggatcaagcgagcagcgcagaccattcatccgccagtttccataatccagcaaatcgttgcgttcttcgagtgagagtggcgtcggcgttgggttaaccaccgcgacctctttcagcgcaggcgcgggcggtacgctgagcggcggttcgtcccctttcttgatccacgcggtttcactgccaacgcgcttttgctgagcatcaataaacaacaacgctgcttttaagccactcagagaaatggtctgatcgccatcgcgtaaggtgattgccttcccttcctgaatcatctgcaaaaacgcggtgatggttgccgtatcatcggttactaataaccatggtgaaatccgccacttgtcaccacttaacgccaacggctcgccatctaacagcagccgtggcgctatctccccttctgacgcctccggcgacttcaatccgccgcgctcaatacgtaaaacggcatcggtatgcgccccggcgctgcggctcagggtcatcaccagtccattatgatcgcccgtattacgcgccacgcagaaattttggttattacaggtgacctgccagtcggaaaacgcccgttgcgctggtgccgcccacaccaaagacgtcggcaacaaagcgaaaaaaaagagaaggaaaatgcgatagcgcatggacggtacgaccccagaagttcaaacaaacagcacaagtcgtatcttcgttgcgcaggtagcgcggctcaatcggatttgtcggattgagccaataataaacaacgaaatattattgttatttttcagtccattaaatgtgacgtttgcaaatagttaagcaataacaccgtcttaccgtcacgtatctcgccggttttgatcatctccagcgcctggctgaacggcagctcgagcacttcaatatcttcatcttcgacaccgccaccggcgttagcgcgctgattgtcactgtattcggcgataaaaaagtggattagctcagtcacaccgcctggcgacatatacagttcaaataatttgcgcacttcacccacttcatagcccgtctcttcaatcgcttctttgcgaatacacacttccggttcgtcgttatccagcagcccggcgcagctttcaatcagctgcccgctttcattgccattaacccaggtagcgacacggaactgacgaatcagaaccacggtctttttcttcgtgttgtacaggaggatcgtcgcaccattgccgcgatcgtacacttcacgtttatggcggataacttcgccgtctttgcgcgtgagatcgtaagtaatgttgtgcagggtgaaatagttatcggagagaattttgtctttaatgagggtgatttgttgcgtcataccgactccacagcgcgaaatgaacaattatcttacgctgtgaagtcgggtttgtctgcgcaggctatcagtgagatttgactgattttacccccagccagtcaataatcccctgtgccgcatgacgtccttctgccattgcggtaaccaccagatccgcaccacgcacggcgtcaccaccagcgaagattttcggattggtggtctggtaacggtactggctttccacatccgcgatgatgcggccccatttgtctaccgttacaccgtgcgactccagccacggcatcccgtgcggattgaagccaaacgccataatcaccgcgtcggctggcatgacaaattcactgccttccaccggcactggacgccgacgcccctgggcatccggctctccaagacgcgtgcgcaggaaacgaatcccgcagacgtgaccttgttcattcagctcaagcgccaccggctggacgttaaattcgaagttggccccctcttcgcgggcgttcttcacttctttcttcgagcctggcatgttagcttcatcacgacgataagcgcaggtgacgttactcgcgccgtggcgcagtgcggtacgcacacagtccatcgcggtgtcgccgccgcccagtaccacgacgttaagtccggcggtattgataaacggctcttccggtagctcttcgagccccatcacctgtttagtgttggcaatgaggaacggcagcgcgtcataaacgcccggcgcatcttcattgggtaaacccgctttcatggaacggtaagtgcctacgccaacgaagaccgcgtcgtattgttccaaaagcgaatccaaagagacatctttacccacttcacaattgagttcgaagtgaatccccatcgcgctgaagatttcccgacggcgtgccagcagggatttatccagtttgaaagaaggaatgccgaaagtgagcaagccaccgatttctggatggcgatcgtacaccgtcacccccacgccattgcgggtcagaacatccgcacaggccagccctgccggacctgcaccgataatcgccacccgcttgtccactttggtgacatggcttaagtcaggacgccaacctttcgccaacgcctgatctgaaatgtagcgttcaatgttgccgatagttaccgcgccgtgctcatcgcgaatagtacaggcaccttcacacaaacggtcttgcggacaaacgcgtccggtaatttccggcagggtgttggtctggtgagaaagctcgacggcggcgtcgatgtttccggctttcaccagttcaatccactgcggtatatggttatgcagcgggcaggtccattcacaaacgctgtgctcgccgcacttaaggcagcgcgaggcttcccgttgtgcctggtcggcgcgaaatggcagataaatttcatcaaaaccggttttgcgcgcttcaatcgccagtttatccggctcgccacgcgcgggcgttgcctgcatttgttcgactttactcattaccggcatttcttgcgccgcggtactggcatgccacggttgatgttcctgacgcgcggtgcgcaagcggcgggatttcgccatgccggagagtgcgacgtcagtgaccagttgcagcgcgtccgccgggcaattctcaacacaggcaggaccgttttcgcgccccgcacaaaggtcgcatttatgcgccgtggcttttacttttcctgccgcgacgggtgtcaggacgatttgcatcgtaccaaaaggacaggccaccacgcaggatttacagccaatacacttttgctgattgacctgaatgctgtcatcaacgtggctgattgcgccattagggcagctacgggcgcagggcgcatcttcacaatggtgacaggtcactgcactacgttgctgttgatgtttgataaccgtaattcggggatgaaaatggtgttggctcaggacatgttgctcatcattgtgagccatgacacaggcgatttcacaagcatgacaacccagacattgctgactgttggccataataaaacgattcataacgaccttcttttttggttgtaaaaaccttattctttatatgagtgttgttattacccgacttacaggggaatcggcaatgttcatgtgcccagaataagtaactatttcgctataaactgtggcagatcaaataatcccatcactgactaaattgcgtttcagcgaactggaacattaatgattttttgtggagaagacgcgtgtgattgttaaacgacccgtctcggccagtctggcccgggcctttttttacattgtgctgctgtcgattctttccacgggtatcgctctgctaactctggcgagcagtttgcgcgacgctgaggctatcaatattgccggatcgctgcgtatgcagagttaccgcctgggctacgacttgcaaagtggcagtccacaactcaatgcacatcgccagttatttcagcaggcactgcattcaccggtattaaccaacctcaacgtctggtatgtgccagaagcagtaaaaactcgctatgcgcatctgaatgccaactggctggagatgaataatcggctcagcaagggcgatttgccgtggtatcaggccaatattaataattatgttaatcagatagacctgttcgtactggctttacagcactacgctgaacgcaaaatgctgctggtggtggcgatttccctggctggcggcatcggtattttcacgctggtcttttttactttgcgccgcatacgccatcaggtggttgccccgctgaatcagctggttaccgccagtcagcgtattgaacacgggcagttcgactcgccgccgctggataccaacctgccgaatgagcttggtctgcttgcaaaaacctttaaccagatgtcgagcgagctgcataaattgtaccgttcgctggaagcgtcagtagaagaaaagacccgcgatctccacgaggccaagcgtcgtctggaggtgttgtatcagtgttcgcaggcgctgaacactagccagattgatgtgcattgtttccgccatattttgcagattgttcgcgacaatgaagcggctgaatatctggagttaaatgtcggtgaaaactggcggattagcgaagggcaaccaaacccggaattgccgatgcagattttaccggtgacaatgcaagagacggtttacggcgaactgcactggcaaaatagtcacgtttcatcatcagaaccgctgcttaacagcgtttcgtcgatgctgggacgcggtttgtactttaatcaggcgcagaagcattttcagcaattattgttgatggaagaacgtgcgaccatcgcccgcgaattgcacgactcgctggctcaggtactttcttacttacgtatccagttgacgttactgaagcgttcgataccggaagataacgccaccgcacaaagtatcatggccgatttttcccaggcgttgaatgatgcttatcggcagttacgcgagctgttgactactttccgcctgacgctgcagcaggcggatctcccctccgcattgagggaaatgctggatacgttacaaaatcaaaccagcgccaaactgaccctcgactgccgtctgccaaccctggcactggatgcgcaaatgcaggtgcatttgttgcaaattattcgcgaagcggtgctgaatgcgatgaagcacgccaacgccagcgaaatcgccgtcagttgcgtcaccgcgccggacggcaatcacacggtttatatccgtgataacgggattggtatcggtgaaccgaaagaacccgaaggtcattatggtctgaatatcatgcgcgaacgcgcggaacggctaggtgggacgctgactttttcacaaccttccggcggcggcacgttagtgagtattagctttcgctctgcggagggtgaggaaagtcagttaatgtaatgcctcctactgaccaaagaatacttgcacttaaggttcagtataaaagggcatgataatttacattaactcctttttttctccacgattggctcgtaccttgccgctacagtgaagcaagtcaagcctacaacgatacgcagaaacacgaggtcctcttttaatggcgaatttctttattgatcgccccatttttgcctgggtgctggcaatcctgttgtgtctgacaggtaccctggcgattttttcattgcccgttgaacaataccccgatctcgcgccaccgaatgtgcgagtgaccgctaactatcccggcgcatcggcccagacgctggaaaacaccgtgacccaggttatcgagcaaaatatgaccggcctcgataatctcatgtatatgtcatctcagagcagtggcaccggtcaggcatctgtcactttaagttttaaagcaggcaccgatccggacgaagccgtgcagcaagtacaaaaccagctgcaatcagccatgcgaaagttaccgcaggcggtgcaaaatcagggcgtgacggtgcgtaaaaccggcgataccaacattctgaccattgccttcgtctctaccgatggttcgatggataaacaggatattgctgattatgttgccagtaatattcaggacccgttaagccgcgtgaatggcgtcggggatatcgatgcctatggttcgcaatattccatgcgtatctggctggacccggcgaaactcaacagtttccagatgacggctaaagatgtcactgatgccattgagtcacagaacgcgcagattgcggttgggcaacttggtggtacaccttccgtcgataagcaggcgctcaacgccaccattaacgcccagtcactgctgcaaacaccagaacagttccgcgatatcaccttgcgggtcaatcaggacggctcagaggtaaggctgggcgatgtcgccaccgtcgaaatgggggcggagaaatacgattatcttagccgcttcaatggtaagccagcctccgggctgggggtaaaactggcctccggcgctaacgaaatggcgacagcggagctggtgctcaatcgtctcgacgagctggcgcagtatttcccgcatggactggaatacaaggtggcgtatgaaaccacctcgtttgttaaagcctccattgaagacgtggtgaaaacgctgctggaagctatcgctctggttttcctcgttatgtatctgttcctgcaaaacttccgcgccacgctgatacccactatcgccgtgccggtggtgttgatgggaaccttctccgtactttacgccttcggttacagcgtcaacaccttaaccatgttcgcgatggtgctggcgatcggtctgctggtggatgacgccatcgtggtggtggaaaacgtcgaacgtattatgagtgaggaaggactcactcctcgcgaagccacacgtaaatcgatggggcagatccagggggcactggtcgggattgcgatggttctttcggcggtatttgtaccaatggccttcttcggcggcaccaccggtgccatctatcgccagttctctattaccattgttgcggcgatggtgctgtcagtactggtagcgatgatcctcactccggctctgtgtgccacactacttaagccactgaaaaaaggtgagcatcatgggcaaaaaggcttttttgcctggtttaaccagatgtttaaccgcaacgccgaacgctacgaaaaaggggtggcgaaaattctccaccgtagcctgcgctggattgtgatttatgtcctgctgcttggcggcatggtgttcctgttcctgcgtttgccgacgtcgttcttaccgctggaagaccgtggcatgtttactacctcggtacagttgcccagcggttcaacgcaacaacagaccctgaaagtcgttgagcaaatcgagaaatactacttcacccatgaaaaagacaacatcatgtcggtgtttgccaccgttggttctggccctgggggtaacgggcaaaacgtggcgcgaatgtttatccgcctgaaagactggagcgaacgcgacagtaagaccggcacctcgtttgccattatcgagcgtgcaacgaaggcgtttaaccaaattaaagaagctcgcgttatcgccagcagcccgccagcaattagcggtcttggtagttctgcaggttttgatatggagttgcaggaccacgctggagcgggtcacgatgcgctgatggcagcacgtaatcagttgctggcgctggcggcggaaaacccggagctaacccgtgtgcgccataacggcctcgacgacagtccgcagttgcagattgatatcgaccagcgtaaagctcaggcgctgggcgttgctatcgacgatattaacgacacactgcaaaccgcctggggttcgagctatgtgaatgactttatggatcgcggtcgcgtgaagaaagtctatgtgcaggcagctgcgccgtatcgcatgctgccagatgacatcaatctctggtatgtccgaaataaagatggcggcatggtgcccttctctgctttcgcgacctcacgctgggaaacaggctcgccgcgtctggaacgctataacggttattctgcggttgagattgttggggaagccgcaccgggggtcagtaccggtacggcgatggatattatggaatcgttagtgaagcagctgccaaacggctttggtctggagtggacggcgatgtcgtatcaggagcggctttccggcgcgcaggctccggcgctgtacgccatttccttgctggtggtattcctgtgtctggctgcgttgtatgaaagctggtcggtgccgttctcggtaatgctggtcgtgccgctgggggtaatcggcgcgctgctggcaacctggatgcgcgggctggaaaacgacgtttacttccaggtgggcctgttaacggtcattggtttatcggcgaaaaacgccatcctgatcgtcgagtttgctaacgagatgaaccaaaaaggccacgacctgtttgaagcgacgctccacgcctgccgtcagcgtttacgcccgattctgatgacctcgctggcatttatcttcggcgtattgccaatggcaaccagcacgggtgccggttccggtggtcagcatgcggtgggtactggcgtaatgggcgggatgatttcggccactattctggctatttacttcgtgccgctgttctttgtgctggtgcgccgccgcttcccgctgaagccgcgcccggaataagcaataaaaaaggcgacatgccaatgtgtcgcctttttcaactttccgattaagaacctgctcagcgggttcttgctgtttgtactttgtctcaggaattacttacgaagcataacttcgataaagtctttccagttccccagttcacgttcaatcataacaacctctcttataattatgggtattctacggaaacaatataccgtggtgaagctaatttactcgattgctgcgatgactacctccgggggacaaatcttatgtaaatactatggtcctgcggtgatgatttgtatgtgatacacagcaacatttcgagatattcatacggcatctaatactgatttaattctggttaaaatacagacagataacaagatgaatattcttaatgtttacgttaaaaatgtttaatattatttaatagttgttaatttgaatacttcgataatgttatatttcctgataatcatttgcaggcaaaatgttttcacccttaaatgagtatttattctcataaatcgaaaaaggattcattatggttacactttacggtatcaaaaattgtgacaccattaaaaaggctcgccgttggctggaagccaataacatcgactatcgttttcatgattaccgcgtcgatgggctggacagcgaattattgaacgattttatcaacgaattaggctgggaagcgttactcaacacccgtggtacaacctggcgtaaactggacgaaaccacccgcaataaaatcaccgatgcggcctctgcggcggcattaatgactgaaatgcctgcaattatcaaacgtccattgctctgcgtgcccggtaagcctatgctgctgggtttcagtgattccagttatcagcaatttttccatgaggtgtagtctatgtcgtgcccggttattgagctgacacaacagcttattcgccgcccttccctgagtcctgatgatgcaggatgccaggctttgttgattgaacgtttgcaggcgatcggttttaccgttgaacgcatggactttgccgatacgcagaatttttgggcatggcgtgggcagggtgaaacgttagcctttgccgggcataccgacgtggtgccgcctggcgacgccgatcgttggatcaatcccccgtttgaacccaccattcgtgacggcatgttattcgggcgcggtgcggcagatatgaaaggctcgctggcggcgatggtggtggcggcagaacgttttgtcgcacaacatcccaaccatacggggcgactggcatttctgatcacctctgatgaagaagccagtgcccacaacggtacggtaaaagtcgtcgaagcgttaatggcacgtaatgagcgtctcgattactgcctggttggcgaaccgtcgagtatcgaagtggtaggtgatgtggtgaaaaatggtcgtcgcggatcattaacctgcaaccttaccattcatggcgttcaggggcatgttgcctacccacatctggctgacaatccggtacatcgcgcagcacctttccttaatgaattagtggctattgagtgggatcagggcaatgaattcttcccggcgaccagtatgcagattgccaatattcaggcgggaacgggcagtaacaacgttattccgggtgaactgtttgtgcagtttaacttccgcttcagcaccgaactgactgatgagatgatcaaagcgcaggtgcttgccctgcttgaaaaacatcaactgcgctatacggtggattggtggctttccgggcagccatttttgaccgcgcgcggtaaactggtggatgcggtcgttaacgcggttgagcactataatgaaattaaaccgcagctactgaccacaggcggaacgtccgacgggcgctttattgcccgcatgggggcgcaggtggtggaactcgggccggtcaatgccactattcataaaattaatgaatgtgtgaacgctgccgacctgcagctacttgcccgtatgtatcaacgtatcatggaacagctcgtcgcctgatgagtggttctgcaagaggaaataagcatggactggctggctaaatattggtggattctggtgattgtctttttggtaggcgtcctgctgaacgtgattaaagatctcaagcgcgtcgaccataagaaatttctcgccaacaagccggagcttcccccgcatcgtgatttcaacgataagtgggacgatgacgacgactggccgaaaaaggatcaaccgaagaagtaagctgagtgctcaaccgtaggccggataaggcgttaacgccgcatccggcaatggtgaacgatgcctgatgcgacgctcacgcgtcttatcaggccaggtaatctgtcttttacatcatttcaatcacatcatcatcgccaggcttaccgccacttagcgcttcgtcgaaataatgtttcggaatggtataacgcaagtgatccagggcaaattgcatactgcgattgtcgatcgcatggcctaaatcctccacgatatccagcgtcacgtcaccaccggcactgattaacgcttcctgcgccgcaaccgcatgcgccagatcgataaccggatcttcaccgccatgaatcaggtgaattgtcgtggctgtagacgcagtttccggcaggctcgcatagcgtccgttaaaagcaatgacgcgtgaagcaaggcccggttcggctttaatgctctccagcaccataatcgcgccttgagagaaaccgatgagcgccgtggcgttagcccctactccgctctgtttctgccagtagcgcaccgtttcaataaacgtcggcatgatcgcatccacacgcgcctggcgattatcttccgtaataccctgcaccgaaaaccactgacgccccgccggattaccgctcggctccgcgccaccgacactcaccaccagcgcatcaggaaacagcggtgcaaaccagttgcctatttcccccattgccaccgggttatccccgacaccgtggaaaagcagtaacaactgttgcgcaggtttatccgggctttgaacaacaaaatggtcatgtttcatggcgaactccttaactgatgtcattaattttacgccgctgactcacaatgaccatgagataaaattgaaggagtcagtgaaataattgccattgcgttatgcgatcgcgcagacgctcagtgcgaacatcattaagtgcgaacagcgcctgcgcggcctcttcccgctgacggaccagtaacatcttgcggcctgaaagtttaagtgtggtacataactgcgcatcactggcgtttttctgtaaacgcccacgcagcgccggtaatgccagttcactggtttgtaacagacgcaataagcaacctaacgacgttaatagcggacgatgagcgaaagcaaaaccggccagttcaagccagtcgtcgtcagaaaggacggcatcgtttagtggatcaacaggaagcgtttcgccattccactgcgcgagagcttgcgcatcgcgacgtaaacggtaatgctcacgttcagccagctgtttacccgcatcactcatcggtaacagcgccatcgccgtatagcaaccgctgctggcttcccgatgattacccatccgcaccagcacaaaaccgcagcgttgccagaaacgccataactccccggtgtaaccaaaactcaccgaaagatagtcgaggtcttgcgtatattgcaaagcaccagcaataagttgccgccctgtgccttcccgctgacgagccggatgaactgctatccggctgacccgccgtccacgcaatgtcgccgccagtggattgttgccgtgcgccgccagcgactgggccaccagattaccccgcgggcgacgaaaacctgcccataccgcctgactgagttgttgagataatccaccctcatccaccagccacagcgccccggcaatctcgttttcgccagccgcctgtaaaaaatgttgccctggtgcatccatcatccggcgtaaatccagcggcgaagtccgatagtgcgcaccagacaagagctgataaacctttaacggcgtttctggatcgctttgccataacgtctgttcaaatgcggaaatgacaatattgccttgtggtgtatgggtgaagttttcatcgtcaaaaaccagtgcctcgctgaccattttttccagcgggcatccctgcgcccagcggatcggctgttgcagttcaaaacggtgtaaatgcggaaagcgagcgcaaaatttcagcaaaaaaccacgtccggtgccttcgtagccctgcaccgtagtggttaacaacgttcgaggaaaacgcgataccagttgatgcaacaatggcgcaggtatggctgcggcttcatcgaccaccagccagtcggcttgctcatcgctggctaacaaggcatccggcgcaataaagcgaaacttctcgcccgcaaattgtgccagtacatccgttgacgcttttgcgggcgcggtgacaatcgctctgcccgcaatacgagaaatgagttgccctgccaacgccgacttaccgcgcccacgcgcagccgttaccgctgccacgcccggcggcatggtcattagctgctttaagagttgctgttgttctggttgtggtgcgccagtcgcggggtaccagtcagtacggggagtaaaatgcgccaacgagaatggctggttttgccgccagaggatagcctcgttatccgccgtaagtacgcgtttgagatgctggacaaaatgcggcgtcgcaatagggtcagggcaatcactccagcgcagcgagtcggcatcaggttggttttcccactcttcccatacagggagtaacaaaaccagccagcttcccgctttcaacgttccgctaagtgcggcaaaggcagcggcatcaaagccgtggcgggcgtcgaataccgcatgccggaactcgcgcccaagtaaagtttgtagtgccgagggagaacagtggttttcagcatctggccgcggcgaaatccacagccagtcgccaggtaaggcatcacgcaacttaagagtatgctcaaaacaccaaccctcttccccgctcaacaccagcaagcggcggatcccttcacgtttcatttgcgctgttaatgtgtgaagcgcagtcagttcagccatccctgccccggaagttaaatgcttttaccaaaagtattgcattgtgccggatcgccgctgtcgaaaccacgtttaaaccagctgtagcgttgctgagaagtgccatgagtgaaactgtctggtactactcgcccctgactttgctgttgtaaacggtcatcgccgatggcctgcgccgcgttcagcgcctcttccagatcgccggtttccagaacgccttgctgctgcatactatgcccccagacaccggcaaaacagtcggcctggagttccatacgcacagataagcggtttacttccgcctgcgtcgcgttttgttgcagttgacgaactttcggctcgatgcctaacagtttctgcacatgatgaccgacttcatgggcgataacgtacccctgggcaaaatcgccatccgcgccaagtttgtctttcatgtcatcatagaaggagagatcgatataaaccgtgccatccgccgggcaatagaacggccccattatggactggcccgccccgcagccggtacgcgtcattccacggtacatgaccagcttcggttgctgataggtcttacccatcttctcgaactgttgtccccaggtgtcttccgtggttgccagaatcaccgaggtgaattttgcggcttcgtcttcatttgggctaattgaccgcgttgattgttgttgggaaaccggctgcccggtcatcaacccggttaaatcaacaccatagtagcctgcaaccagcacgactatcagtaaaatcagcccgcctttaccgcttggcaggcgaaaaccgggaccgcccatagatggaccaccagagctgttgcgcctgtcttcaacattgtcactttcacgtcgcccttgccaacgcatagatacctcaacaatatattcattatagaaatgatcgtaggtggttcagaggaagattaccacaggaaagcgggatgaaatggcggaggaatgagcgttcaatgcatatattccgagagcggttgtcttgccgtgccagctgcacggcaagatgatgaacagaaaaatcagtccagctgtacacccaggcggcgggcgacggcttcataggcttcgatcaggccaccgaggctctggcggaaacggtctttgtccattttctccagcgtttctttgtcccacaggcggctaccgtccggggagaactcatcacccagtaccacttcgcctttgtacagaccaaattccagcttgaagtcgaccagaatcagaccagcatcatcgaacagttttttcagcacgtcgttcgctttgtaggtcagctctttcatacgcgccaggttctctttgctcacccagccaaaggtttcgcagtaagattcgttgaccatcggatcgtgcatggcgtcgtttttcaggaacagatcgaacagcggcgggttcagctcaataccttcttcgattccaagacgtttcaccagagagccagcagcacggttacgcacgacacactcaaccggcaccatatccagctttttcaccagacattcggtatcggagagcagacgctccatttgagtcgggatacccgcttcagccagtttgctcataatgaagtagttgaacttgttgttcaccatacctttgcgatcaaactgctcaatgcgcgcgccatcccctgctgacgtatcattgcggaattcgagcaccaacaggtccgggttttccgtgctgtatacggttttcgctttaccacgatacaactcagcttgcttttgcatctttatcactcctgggtgtgaattaacgttttaaaatcttttgctgtctggtgtgccggatgttttgtcggatgcggcgtgaacgccttatccgaactacgtccgacaaacaaatttcgtgcgaattaccgctaaaatcgcgttttcctgcagacgcacacgtttgcgtatcatatcagaaaaaagggccggatgattccagccctgtatttttacttgctaaacgcagcctggaagacagctaccagcgcgtcgttctgactctgagtcagagtatgacctttcggatcgatgaactgtaggctgctgcggttatctaaatcgccaacctgcagtttatagtcaccggatgccaggcctggatcgctcgcgcccagttcctgccagtcgctgtcagacagcggcttataagttacggccatgttgccctgcgaacgggtgctgtcggtcactttcatgcccactttttccagcgccgctggcagacgttgccaaaccacattgaacggcccgcgtacgaccagcattggtaaaccggtgtcatcagctgcactttgtacgtccatagtggtggaggcacgattttgcgcagcgttcgcggcgtcagtggcagatttatccagaccggcggaaataacgttcatcatctccgtgctgtaacgctgcatggaagccgcgtctgcaaccggtttgcccgcctgttccaggttcagcagtttaaccgtaaccgcctgctgataaccctgcggcttaacagagatttgataacgaccacgatactgctcgtcttcgtccagacggttccattgtacccaatcggtggtcagtgtctgaccagcatcatcacgttgggtgatggtgtagtttttcgcctgcagcacgctaaccacctgcggccacagagtattgccacgaccattttccaccagcaatgaagcggtatcgcccgtgaactgggtacgcgcgccagaaaccagtgccagcggctgggctggtggacgaatgtccagcgccttaccgacagcaccactaccgttggtcaccgggattgcataatcaccggaggtcaccggcaaaatcattccagccggggcatgaagctccgcaagcggtgccgcttccaggtaggcttcatcaccactgacctgacgcttatagcgtgagtcagaactacaggcagcgagtaataaaacaagcgaaacacccgcaacctttgccaggcgcgacttttgaacagagtaagccatcaaatctccctaaactttacagcaaaccggcatgcttaagcgccgctctgaccgtctcacgaccactgtcggtgattggtgtcattggcaggcgcagcgtatcggtcgccacaagacccagttccttacatgcccatttcaccgggattggattgggttcgacaaatagtttgttgtgtaatggcatcagacgctgattaataacgcgtgcctcggcaaaatgcccttctgctgccagtttgcacatctgggccatatcacgcgctgcgacgttagccgtaacggaaataaccccatgaccgcccaattgcatgaagtccagcgcgctcgcatcatcgccgctcagcagaacaaaatcatctgaaaccagctctttgatctggtttacacgcgttaagttccctgttgcctctttgattccgataatattttttactttcgccagacggcccaccgtttccgggagcagatcgcagccagtacgggacggcacattatacagaatttgcggcaggtcagtatgctcagcgatggctttgaaatgctgatacaaaccttcttgcgacggacgattgtagtaaggggttaccgtcaggcagccgacgataccactgtcattgaagcgctgcgtcaggctaatggcttccgcagtagcgttagcgccggtcccggcaattaccggaatgcgcccatcagccagatccagcgtcatcatcaccacatcagcatgttcgtcatgatttaaggtagcggactcgccagtggtgccaacagaaacgatcgccgaagtaccgctggcgacatgataatcaatcagttttttcaagctagcccgacagacattacctttttcatccatcggagtaacaatcgcgacaatacttcccgtgaacatgggccatcctctgtgcaaacaagtgtctcaatggtacgtttggtatggcattaaaagcaagcagacagaaccgttctgattgttgtatgcatgttttttttatgctttccttaagaacaactcaccccttaaaggaataaccagtttgacactgtcatcgcaacattatctggtgatcactgcgttgggtgccgatcgccctggaattgtgaacaccatcacccgtcatgtcagtagttgcggctgtaatattgaagacagtcgcctggcgatgctgggagaagagttcacgtttattatgctgctttccggttcatggaatgccattactctgattgaatcaacgttaccgttgaaaggtgccgaactggatcttttaatcgtgatgaagcgcacgacggcgcgtccgcgtccgccaatgccagcatctgtctgggttcaggtcgatgtggcagactccccgcatttaattgaacgcttcacagcacttttcgacgcgcatcatatgaacattgcggagctggtgtcgcgcacgcaacctgctgaaaatgaacgggctgcgcagttgcatattcagataaccgcccacagccccgcatctgcggacgcagcaaatattgagcaagcgttcaaagccctatgtacagaactcaatgcacaaggcagtattaacgtcgtcaattattcccaacatgatgaacaggatggagttaagtaatgaatccactgaaagccggtgatatcgcaccgaaatttagcttgccggatcaagacggagaacaagttaatttgaccgacttccagggacagcgtgttctggtttatttctacccgaaagccatgacccccggctgtaccgtacaggcctgcggcttacgcgataacatggatgagttgaaaaaagcgggcgttgatgtgctgggtatcagcaccgataaacccgaaaaactctcccgttttgcggaaaaagagctgcttaactttacgctcctgtctgatgaggaccaccaggtgtgcgaacaattcggcgtctggggtgaaaagtccttcatgggcaaaacctacgatggcattcatcgcatcagcttcctgattgacgctgatggcaaaatcgaacatgtctttgacgatttcaaaaccagcaatcaccacgacgttgtgctgaactggctgaaagaacacgcctgattactttgctccattccgtgctggctgcgcttgcggccagcatacctcacttctcgtgatcaagatcacattctcgctttcccctgcgacacgggtgtcgaatccattttttgctgaacgttaatgaccatcatttttgtaccgttcagaatccagttaatacataacttattgaatatattgagttaatcagaatggcatcctttatgcaatatgaaatgcaatgtttcatatcattttcaaggagccgacatgaaccgctttgtggtggccgaaccactgtggtgtacaggatgtaatacctgtctcgctgcctgttcggacgtgcataaaacgcaaggtttacagcaacacccgcgcctggccctggcgaagacgtcaacaatcactgcccctgtcgtgtgtcatcactgtgaggaagccccttgcctgcaggtctgcccggtcaatgccatctctcagagggatgatgcgatccaactcaacgaaagcctctgtattggctgcaagctttgcgccgtggtctgcccatttggcgcaatcagcgcttcaggaagccgtccggtgaatgcccatgcgcaatatgtttttcaggctgaaggctcactcaaagacggcgaagaaaacgcgccaacacaacatgctttgctgcgctgggaacctggtgtccagaccgtcgcggtgaaatgcgacctgtgtgatttcttgccagaaggtccggcctgcgttcgcgcttgcccgaatcaggcgttacggctgatcaccggtgatagcctgcaacgtcagatgaaagaaaaacagcgccttgccgcaagctggtttgccaatggcggggaggatcccctttccctcactcaggagcaacgctaatggatgccctgcaattattaacctggtcgctgattctctatctgtttgctagtctggcttcgctgtttttactcggtctggacagactggctattaagctttccggcatcacatcgctggtgggcggcgtgattggcatcatcagcggaattacgcaattacatgctggtgtaactttagtcgcccgttttgcccccccttttgaatttgccgatttaaccctgcgaatggatagcctctcggcatttatggtgctggttatctccttgctggtggtggtttgttctctctattcattgacttatatgcgcgaatacgagggcaaaggcgcggcggcgatgggcttctttatgaatattttcatcgcatcgatggttgccctgctggtgatggacaacgctttttggttcatcgtgctgtttgaaatgatgtcgctgtcttcctggtttctggtcattgccaggcaggataaaacgtcgatcaacgctggcatgctctacttttttatcgcccacgccggatcggtgctgataatgatcgccttcttgctgatggggcgcgaaagcggcagcctcgattttgccagtttccgcacgctttcactttctccggggctggcgtcggcggtgttcctgctggcctttttcggttttggcgcgaaagccgggatgatgccgttgcacagctggttgccgcgcgctcaccctgccgcaccatcgcacgcttcggcgttgatgtctggcgtaatggtcaaaataggtattttcggcatcctgaaagtagcgatggatctgctggcgcaaacgggtttgcctctgtggtggggcattctggtgatggcgatcggcgcaatctccgcgctcctgggcgtgctatatgcgctggcggaacaggatatcaaacggctgctggcctggagtaccgtcgaaaacgtcggcattattttgctggcagtcggtgtggcgatggtcggtctgtcactgcacgacccgctgctcaccgtggttggactgctcggcgcactgtttcatctgctcaaccatgcgctgttcaaagggctgctatttctcggcgcgggagcgattatttcgcgtttgcatacccacgacatggaaaaaatgggggcactagcgaaacggatgccgtggacagccgcagcatgcctgattggttgcctcgcgatatcagccattcctccgctgaatggttttatcagcgaatggtacacctggcagtcgctgttctcactaagtcgtgtggaagccgtagcgctacaacttgcgggtcctattgctatggtaatgctggcagtcactggtgggctggcagtaatgtgcttcgtaaaaatgtacggtattactttctgtggtgcgccgcgcagtacacacgctgaagaggcacaggaagtgccaaatacgatgatcgtcgccatgctactgctcgcggcactctgcgtattaattgcgcttagtgccagttggctggcaccgaagataatgcatattgcccatgcgtttaccaatacccctcccgccactgtcgccagcggaatagcacttgtacccggcacgtttcatacacaggtcaccccctcattactgttgctgttactactggcgatgcctttgctgcctggcctttactggctgtggtgtcgttcgcgccgcgcagcgtttcgtcgcacaggagatgcctgggcatgcggctacggctgggaaaatgcgatggccccgtcaggcaatggcgtgatgcagccgctgcgtgtggtcttttctgcgctatttcgtctacgacaacagctcgaccctacgctgaggctaaataaaggtcttgcgcacgtcaccgccagggctcagagcacagaacccttctgggatgagcgggtgatccgccccatcgtgagcgccacccaacggctggccaaagaaatacagcatctgcaaagcggcgactttcgtctctattgcctgtatgtggtcgccgcactggttgtgctgctaatcgctattgccgtctaaggaaatcaccatgagacaaactctttgcgacggatatctggtcatttttgcgttagcacaggccgtgattctgctgatgctaaccccactttttacgggtatttcccggcagatacgcgcgcgtatgcactcccgccgcgggccggggatctggcaggattatcgcgatatccacaaactgtttaaacgccaggaagttgcgccgacatcttcaggtctgatgttccgcctgatgccgtgggtattaatcagcagcatgctggtgctggcgatggccttaccactgtttattaccgtttccccttttgcgggcggcggcgatctgatcacccttatctatcttcttgccctgtttcgttttttctttgctctttccgggctggataccggaagtccgtttgcgggagtcggtgccagtcgcgagttgacgctcggcattctggtcgaaccaatgcttattctctcactgctggtattggcgctgatagcaggttccacgcatatcgagatgatcagcaatacgctggcgatgggctggaactcgccgctaaccaccgtactggcgttactggcctgtggttttgcctgcttcattgagatgggaaaaattccctttgatgttgctgaagcagaacaggaattacaggaaggcccgctgaccgaatattccggtgccgggctggcgctagcgaaatgggggctggggctgaaacaggtcgtgatggcatcactgtttgtggccctgtttctgccctttgggcgcgcgcaagaactttctctcgcctgcctgctgacttcacttgtcgttacgctgctcaaggttttgctgatttttgtactggcctcaatcgcagaaaacacgctggcacgcgggcgttttttactcattcaccatgtgacctggcttggcttcagccttgctgcgcttgcatgggtcttctggttaaccggtctgtaaggagcactgacggaatatggaaaatcttgctctgacgacgttattgctgccttttatcggcgcactggtcgtttcgttttcgccacaacgtcgggccgccgaatggggggttttgttcgccgcgctgaccacgctgtgcatgttgtcactgatctccgcgttttatcaggccgataaagttgccgtcacgttgacgttggtcaacgtgggggatgtggcgttgtttggcctggtcattgatcgcgtgagtacgctgattctgtttgtggtggtgtttctcggtttgctggtcacgatctactccacgggttatctgacggataaaaatcgcgaacacccgcataacggcacgaatcgttattacgcatttttactggtgtttatcggcgcgatggcgggactggtactctcctcgacgctgctcggtcagttgttgttttttgaaattacaggcggctgctcctgggcgttgatcagttattaccagagcgataaagcgcagcgttcagcactaaaagcgttacttatcactcatatcggctcgttggggttgtatcttgccgccgccacgctgtttttgcagaccggaacgtttgcgcttagcgcgatgagcgagttacacggcgacgcacgttatctggtttatggcggcatcctgtttgccgcgtgggggaaatcggcccagctaccgatgcaagcgtggctaccggacgcaatggaagcgccaacaccgatcagcgcctatctccacgccgcatcgatggtgaaagtgggcgtttacatttttgcccgcgctattatcgacggcggcaatatcccgcatgtgattggcggcgttggcatggtcatggcactggtcaccattctttatggctttctgatgtatttgccacagcaggatatgaagcggttgctagcctggtcgaccatcactcaacttggctggatgttcttcggcttgtcgctctccatcttcggctcgcggctggcgctggagggcagcatcgcctacatcgtcaaccacgcgttcgctaaaagcctgtttttccttgtagcaggtgcgctgagttacagctgcggcacgcgcttgttgccgcgtctgcgtggcgtattgcacaccctgccgttgccaggcgtgggtttctgcgtggcagcgctggcgattaccggcgtgccgccgttcaacggcttcttcagtaaattcccgctgtttgctgccggttttgcgttgtcagtggagtactggatcctgctgcccgccatgattcttctgatgattgaatcggtcgccagtttcgcctggtttattcgctggtttggtcgcgttgtgcctggcaaaccgagcgaggccgtcgccgatgccgcaccgctgccaggatcaatgcgcctggtgttgattgtactgattgtgatgtcgctgatttccagcgtaatcgccgcgacctggttgcagtaaggagatgatgaatgaccggttctatgatcgtaaataatctggcgggactgatgatgctgacatcgctgtttgtgattagcgtcaaaagctatcgcctgtcatgcggattttacgcctgccagtcactggtgctggtgtctattttcgccactctctcgtgcctgttcgccgcagagcaactgctgatctggtccgccagcgcctttatcaccaaagtgctgctggtaccgttaatcatgacttacgctgcacgaaatattccccagaacatcccggaaaaagcgttattcggtccggcaatgatggcactgctcgcggcgttaattgtcctgctttgcgcatttgtcgttcagcccgtgaagctaccgatggctaccgggctgaaaccggcgctggcggtagcgttaggtcattttctgcttggcctgctgtgcattgtcagccagcgcaatatcctgcggcaaatttttggttactgcctgatggaaaacggctcccatctggtgctggcgcttcttgcctggcgagcaccggaactggtggaaataggtatcgctaccgacgccatcttcgccgtcattgtgatggtgttactggcaagaaaaatatggcgtacccacggcacgctggacgtgaacaacttgaccgcgctgaagggataatgagatgagttattctgtgatgttcgctttactcctgctcacgccgctgcttttttcgctgctctgttttgcctgccggaaacggagactttctgcgactcgcacggtgaccgtattacatagcttagggatcacactgctgctgattctggcactctgggtggtccaaactgccgctgatgcaggagaaatattcgctgcgggactgtggcttcatattgatggtctgggcggtttgttcctcgccattcttggtgtgattggctttctcaccggtatttactcgattggctacatgcgtcatgaagtggcacacggcgagctttcacccgttacgctgtgcgattactacggtttcttccatctgtttttgttcaccatgctgctggttgttaccagcaataacctgattgtgatgtgggcggcgatcgaagccaccaccttaagctcggcgtttctggtaggcatttacggtcagcgttcatcgctggaagctgcatggaagtacatcattatttgtactgttggtgtcgcttttggtctgttcggtaccgtgctggtatacgccaacgccgccagcgttatgccgcaggcagaaatggcgatattctggagcgaggttcttaagcaatcgtccttgcttgacccaacattaatgctgttggcctttgtgtttttgctaattggctttggtaccaaaaccgggctatttcccatgcacgcctggctgccggatgctcacagtgaagcgccgagtccggtcagcgccctgctctccgccgtattgctgaactgcgcgctgttggtgctgattcgctattacatcattatttgccaagccatcggcagcgatttccccaaccggttgttgctcatcttcggcatgttgtcggttgccgtggcggcatttttcattctggtacagcgggacattaagcgtctgctggcgtactccagcgtggagaacatggggctggtcgcggtggagctaggcattggcgggccgctgggaatttttgccgcgctgctgcacatcttaaaccacagtctggcaaaaacgctgctgttctgcggttccggcaatgtactgctcaagtacggcacgcgcgatctcaacgtcgtctgtgggatgctcaaaatcatgccatttaccgccgtgctgtttggcggcggtgcgctggcgctggcagggatgccgcccttcaacatttttcttagcgaatttatgaccattaccgccggactggcacgtaatcacctgctgattatcgtcctgctgttattgctgttaacgctggtgctggcgggcctggtacggatggctgcgcgggtgttaatggcgaaaccgccgcaggccgttaaccggggtgatctcggctggttgaccacctcgccaatggtgattctgctggtcatgatgctggcgatgggaacgcatattccacaacctgtcatcaggatcctggcgggcgcttccactatagtcctctcagggacgcacgatctgcctgcacaacgtagcacctggcatgattttttgccttcaggcaccgcatctgtttcggagaaacacagtgaacgttaattcatcgtcaaatcgtggcgaagcgattctcgccgccctgaaaacgcagttccccggcgcggtgctggatgaagagcgacaaacgcctgaacaggtcaccattacggtgaaaatcaatctgctgcctgacgttgtacagtatctttattatcaacatgatggctggcttccggtcctgtttggcaacgacgagcggacacttaacggtcattacgcggtttattatgccctttcaatggaaggggccgaaaaatgctggattgtggtgaaggcgctggtcgatgccgacagtcgggagtttccgtcagtcacaccgcgcgtccctgccgcggtctggggcgagcgagaaattcgcgatatgtacgggctgattccggttggcctgccggatcagcgtcgcctggtgttgcccgatgactggccggaagatatgcatccgctgcgcaaagatgcgatggattatcgactgcgccctgaaccgacgactgattccgaaacgtatccgtttatcaatgagggcaacagcgatgcgcgggtgatccctgtcggcccgctgcatatcacctccgatgaaccgggtcacttccgcttgtttgtggatggcgagcaaattgtcgatgctgattaccgcctgttttatgtccatcgcggcatggagaaactggcagaaacgcggatgggctacaacgaagtgaccttcttatcggaccgcgtgtgtgggatttgcggttttgcccacagtgtggcctataccaattcggttgaaaatgcactggggattgaggtgccgcaacgagcacatactattcgctcgattctgctggaagtcgaacggctacacagtcatttgcttaaccttggcctctcctgccatttcgttggttttgataccggctttatgcaatttttccgcgtgcgggaaaagtcgatgacgatggcggaattgctgatcgggtcgcgtaaaacctacggtctgaatctgattggtggtgttcgccgcgatattctcaaagagcaacgtctgcaaacgctgaaactggtgcgcgagatgcgcgccgacgtgtcggagctggtagagatgctgcttgctacgccgaatatggaacaacgcactcagggcattggcattctcgaccgacaaatcgcccgtgatttgcgctttgatcacccctacgccgactacggcaatattccaaaaacactgtttacctttaccggcggcgatgttttctcccgcgtgatggtccgtgtcaaagagacgtttgattcgctggcaatgctggaatttgccctcgacaacatgccggataccccactgctgaccgaaggctttagctataaacctcacgcattcgcgctgggctttgttgaagcgccacgcggtgaagacgtgcactggagcatgctcggtgataaccaaaaattgttccgctggcgctgccgtgccgccacctacgccaactggccggtgttgcgttacatgctgcgcggcaataccgtttctgacgcaccgctgattatcggtagccttgatccctgctactcctgtaccgaccgtgtgacgctggtagatgtgcgcaagcgccagtcaaaaaccgtgccgtataaagagatcgaacgctacggcattgatcgtaaccgttcgccgctgaagtaaggacagaagatgctgaagttactgaaaactattatgcgcgccggaaccgcgacggtgaaatatcccttcgcgccactggaggtcagccctggctttcgcggaaaaccggacctgatgcccagccaatgtattgcctgcggtgcctgcgcctgtgcttgtccggcaaatgcgctgactatccagaccgacgaccagcaaaattcgcgcacctggcagctctatctggggcgttgtatttactgcggacgttgtgaagaagtgtgcccgaccagagccatccagcttaccaataactttgaactgaccgtcaccaataaagccgatctctatacccgcgcgacgttccatctacaacgttgcagccgttgcgaacgcccgtttgccccgcaaaaaaccatcgcactggctgctgaattgttagcacagcaacaaaatgcgccacaaaaccgcgaaatgttgtgggcgcaagcgagcgtctgcccggaatgcaaacaacgcgcgacgctgatcaacgacgatacagatgtactgctggtggctaaggagcagctatgagtccagtgcttacacaacatgtcagccagcccatcacgctggacgagcaaacgcaaaagatgaagcggcatttgctacaggatatccgtcgctcggcttacgtttatcgcgtcgattgcggcggctgcaacgcctgtgaaatcgaaatttttgctgccattacaccagtattcgacgcagaacgttttggcattaaggttgtttcatcaccgcgtcacgccgatattttgttatttactggcgcagtcacccgggcgatgcgtatgcctgcacttcgggcgtatgagtctgcccccgatcataaaatttgtgtttcctacggcgcgtgcggtgtcggcggcggtattttccacgatctctacagcgtctggggcggtagcgacaccattgtccccattgatgtttggatccccggctgcccgccaacaccggccgccaccattcacggtttcgccgtggcgctcggtttgctgcaacagaagattcacgctgtggattatcgcgatcccaccggggtgactatgcaaccgttgtggccgcagatcccgccatcacagcgtatcgccattgagcgagaagcgcggcggctggcgggctatcgtcaggggcgagaaatttgcgatcggctcctgcgccatttaagcgacgatcctacaggaaatcgggttaacacctggttgcgcgatgccgacgatccacgtctcaatagtatcgttcagcaactctttcgcgtactccgggggttacatgactgaagagtgcggggaaattgttttctggacgctgcgaaaaaagtttgtcgccagtagcgacgagatgccggaacacagctctcaggtaatgtattactcgctagctatcggccatcacgttggcgtgattgattgtctgaatgtcgccttccgctgcccactgacggaatacgaagattggcttgcactggtcgaagaggagcaagcccgacgtaagatgctgggggtgatgacttttggtgagattgttattgacgccagccacaccgccctgttgacccgggcattcgcgccactggcggatgacgcgacgtctgtgtggcaggcgcgtagcattcaattcattcatctgttggatgaaattgtgcaggaaccggccatctatctgatggccagaaaaattgcgtgagaaggatttctcattaataaggactgttgatggctatgtcagacgaggcgatgtttgccccgccacaaggaataacaattgaagcggtaaacggaatgctcgcggagcggttagcacagaaacacggcaaggcgtctttattacgcgccttcatcccgctgccgccgccgttcagcccggtacaacttattgaactgcatgttctcaaaagcaacttctattaccgctaccatgatgatggcagcgatgtgacggcaacaacagagtatcagggcgagatggtcgattattcgcgtcacgccgtccttctcggcagtagtggaatggcggagctacgctttattcgcacccacggcagtcgttttacttcccaggattgcacactgtttaactggctggcgcggataatcaccccggttctgcaatcatggctcaatgatgaagaacagcaggtggcgctgcgtttgctggagaaagatcgcgatcatcatcgggtactggttgatattactaatgcagtgctgtcacatcttgatctcgacgatctgatcgctgacgtcgctcgtgagatccatcattttttcggtctggcttcagtcagtatggtactgggcgatcatcgaaagaacgagaagttcagcctgtggtgcagcgatctttctgcctcacattgtgcgtgtctgccacgctgtatgcctggcgaaagtgtattgctgacacaaacgctacaaacccgacaaccgaccttgacgcaccgtgcagatgatctgtttctctggcaacgcgacccgttattactcttacttgcatctaacggctgcgaatctgcgctccttataccgcttacctttggcaaccatacaccgggtgcattgttgctggcgcatacctcttccactctctttagtgaggaaaactgccagctactacaacacatagccgatcgcatcgctattgccgttggcaatgccgatgcctggcgtagcatgaccgatttgcaggaaagtttgcagcaagaaaaccaccagcttagcgagcagctcctttcgaatctgggcatcggtgacattatctatcaaagccaggcaatggaagacctgctccagcaggtagatattgtggcgaagagcgacagtacggtgttgatttgtggtgaaaccggaactggcaaagaggtgatcgccagagcgatccatcaacttagcccgcgacgcgacaagccgctggtcaaaatcaactgcgctgccatccccgccagtcttctggaaagtgagttattcggtcatgacaaaggggcgtttactggtgcgattaatacccatcgtggtcgttttgaaattgccgatggcggcacgttgtttctcgatgaaattggcgatctgccgttagaacttcagcctaaactgctgcgcgtattgcaggagcgggagattgagcgtctcggcgggagtagaacgatcccggtgaatgtcagagtcattgccgccaccaaccgtgatttgtggcaaatggttgaagatcgccagtttcgcagcgatctcttttatcgcctgaatgtcttcccactggaattgccgccgctacgcgaccgtccggaagatatccctcttttagcaaaacatttcacgcaaaaaatggcgcgccatatgaatcgcgcaattgacgccatcccgaccgaggcactacgccagttgatgtcgtgggattggccgggcaacgtgcgcgagctggaaaacgtgattgagcgggcggtactgttgactcgtggtaacagtctgaatttacatctaaatgtccgacaaagccgtttactgccgacgctaaatgaagattcagcgcttcgcagttcaatggcgcagttactgcacccgacgacgccagagaatgacgaagaagaacgtcagcgcattgttcaggtattgcgagaaaccaatggcattgttgccgggccccgtggcgcagcgacgcgattagggatgaagcgcaccacgctgctgtcacgaatgcagcggctggggatctcggttcgcgaggtgttgtaatctgcttttgcaggagtatgcatgagaaacaaactctctttcgacttgcagttgagcgccagaaaagcggcaatcgctgaacggattgccgcccataaaattgcccgcagtaaagtgtcggtctttttaatggcgatgtccgctggcgtgtttatggcgatcggatttactttttacctttccgttatcgccgatgccccgtcttcacaggcattaacccatctggtgggcggcctttgctttacactcggctttattttgctggcggtttgcggcaccagcctgttcacctcgtcggtaatgacggtgatggcaaaaagtcggggcgttattagttggcgaacttggctgattaacgcacttctggtggcctgcggtaatctggcaggtattgcctgtttcagtttgttaatctggttttccgggctggtgatgagtgaaaacgcgatgtggggagtcgcggttttacactgcgccgagggcaaaatgcatcatacatttactgaatctgtcagcctcggcattatgtgcaatctgatggtttgcctggcgctgtggatgagttattgcgggcgttcgttatgcgacaaaatcgtcgccatgattttgcccatcaccctgtttgtcgccagtggctttgagcactgtatcgccaatttgtttgtgattccgttcgccattgccattcgccatttcgcccctccccccttctggcagctggcgcacagtagcgcagacaattttccggcactgacggtcagccattttattaccgccaatctgctcccggtgatgctgggtaatattatcggcggtgcggtgctggtgagtatgtgttatcgggctatttatttacgtcaggaaccctgaaaaatcagcccggcgaaacagttcgtcgggctgaagattattcttgcgcgatttgcccatcgggccaggcatgaatcacggctttgatcagcgtcgccaacggaatggcgaagaatacgccccagaatccccacaaaccaccgaagatcaccaccgataaaataatcaccagcggatgcaggttaaccgcttcggagaacaacaccggcactaacaggttgccgtccagcgcctgaataatcagatacaccgcgaagcagctccagaattcagtacctgcgccaaactggaatagcgccacgccaaccaccggaatggtcaccacaaatgcgccaatgtacggaataagaaccgagaagccgaccagcactgccagcagcagcgaatagttcagcccgaagagcaagaaccccagccaggtggcgatccccaccacgatcatctccagcactttgccgcggatatagttggtgatttgttgattcatctccttccacacctgtcctgccagcccacggttacgcggcagcacccggcgaacggcgttcagcatctgctctttgtctttcagcaggaagaagaccatcaatggcaccagcaccagatagacggctatggtcagcaaaccgaccagcgaggcgagggaaattttcaccaccgaatcgcccatggtcagcatccgactgcgcatattttcggccattgcatcaataatgcccgcgtccattaacgccggatagcggcgcggcaacgtggcggcaaagtcagaaagcttattgagcatccccggcatatcgcggattaagtagatgccctgttgccaggcgataggcagtaccacgaacgccatcagtagcaatataccgacgaaaaccaccaatacaatcgacgtcgcccagcggcgggagcagccaatagattgcagacgcacggttggccattccagcaaataggccagcacaatagccaccagcaacggagcaagcaggccactaaagaaaaagataatgccaaatccggcaactaaaataaccagcaaggcaatcgcttccgggtcgctaaaacggcggcgataccattgcatcaacatttcgagcataaagaccttccctgaacctcaagagcgggattgcgatccgcaattgtatcgaaatgtcacaaaaaagacttcgctttttatgacggattcaggaaactgaaaagtcatttgagtgggctaatcttcgccgttacactcaaaggcggcgcggtgggaacgatatttcacagtatcggtcaaatgactatctccagaaatacaggatagaggttatgttcaggcagttgaaaaaaaacctggttgcaaccctcattgctgctatgaccattggtcaggtagccccggcgtttgccgacagcgcagacaccttgccggatatgggaacctccgcaggaagcacgctttccattggtcaggaaatgcagatgggcgactattatgtccgccagctacgcggcagcgcgccgttaattaatgacccgctgttaacgcaatatattaattcgctggggatgcgtctggtttcgcatgccaattcggttaagacaccgtttcatttttttctgatcaacaacgacgaaattaacgcctttgctttctttggcggcaacgtggtgctgcactctgccctgttccgttattccgataacgaaagtcaactggcttcagttatggcgcacgaaatctcccacgtcacccaacgtcacctggcgcgagcgatggaagatcagcagcgcagcgcgccgctgacctgggtcggcgcgttaggttctattttactggcgatggccagtccgcaggcggggatggcggcgctgaccggtacactggcgggaacgcgtcaggggatgatcagtttcacccagcaaaatgaacaggaagcggaccgcattggtattcaggtgctgcaacgctcgggattcgatccgcaggcgatgccaaccttcctcgaaaaattactcgatcaggcgcgttactcctcgcgcccgccggaaattttattgactcacccgttgccggaaagtcgtctggcagatgcccgcaaccgtgctaatcagatgcgcccgatggtggtgcagtcgtcggaagatttctatctggcgaaagcgcgcacactggggatgtataattccggacgtaaccagctcaccagtgatttgctggatgaatgggcgaaaggaaacgttcgtcagcaacgagcagcacaatatggtcgtgctttacaggcgatggaagccaataaatacgacgaggcgcgtaaaacgctgcaaccgttactggcggcagaacctggcaacgcatggtatctcgatctggctactgatatcgatcttgggcaaaacaaagccaatgaggcgatcaatcgtctgaaaaatgcccgcgatttacgcaccaatccggtgttgcagctcaacctggcgaacgcttatttgcaaggcggtcaaccacaagaagcggccaatattctgaatcgctacacctttaataataaagatgacagcaacggctgggatttgctggcacaggcggaagccgcgctaaataaccgcgatcaggagctggctgcgcgagcagaaggttatgcgctcgccggacgactcgatcaggccatttcgctgttgagtagcgccagttcgcaggtgaaattaggcagcctgcaacaagcgcgttacgatgcgcgcatcgaccagttgcgccagctgcaggaacgctttaagccttataccaagatgtaattcgcattaaaggaagaacaatgaccaaacaggtaaaaatctaccataacccacgctgttcaaagagccgggaaacgctgaacctgctgaaagaaaacggcgtggagccagaagtggtgctctaccttgagacacccgccgatgcggcaacgctgcgcgatttgctgaaaatactggggatgaatagcgcccgtgaattgatgcgccagaaagaggatctttataaagaactgaacctggctgacagttcgcttagcgaagaggcgctgattcaggcaatggtggataatccgaagctgatggagcgcccgattgtggtcgcgaatggcaaagcgcggattggtcgtccaccggagcaggtactggaaatcgtgggttaagatgtgctccatcgctagttgaagcacattgccggatgcgacgcttgccacgtcttatccggcctacgaatactatggattaacttcgcgtagttcggataaggcgttcgcgccgcatccgacaataaacaccttatctacaacttcagaatttctttcacaaacggaatggtcagcttacgttgcgcggtaatcgacgcacgatccaactgatccaacgtcataaatagcgtgcgcatttctctgtcgagccgcttcagcaagaaacgccccacatcttccggcagttcaaaaccacgcaaacgcgcgcgtaactgtagcgcctgcaacttatcttcatcagaaagtggctgcaatttgtagatctgcccccagtcgagtcgcgacgcgagatccggtaatcccagattcaactgccgcggtggacgatcgccggtgatcaacaaccgtgttttgcccgattccagaattcgattgtagagatcgaaaatcgccatctcccacaactcatcgcctgcaatacactcaatgttgtcgatacagaccagcgacaaatgctccataccgtcgagcacttccggaacaaaccaggtgcgtttatccagcgggacatagcccaccgcatcgccacgctgcgacaattccgcgcaagccgcgtgcagcagatggctgcgccccgcgccttcgcgtgcccagagatagatgtaaccgctatgttcctgacgcagcacgttttgcagcgcggccagtaaagaggagttatcccccggccagaaacttgcaaaggtttcgtcgtcaggaagataaagtggcaaagagagctgtgccggtgtgttcagagatacctcaaccaggatttcacaaaatcgcgagaagtttaccacagaatcccatgatgtttgaaccgggcagcaacactgcccggtcggtacattatttgtctgttatatccgcgtcttctgcgtccagcaccacttcttcagggcgcagcacactgatcagtttgaagatcaaacttaagccgataccgacgatggtcgccagcgccataccttttaactccgccgcgccgatgtttaccttcgcgccactgacgccgatgatcaaaatcacggaagtcaggatcaggttctgtgctttgttgtaatccactttcgattcgatcaaaacacgaataccggaagcaccgatgacaccataaagcagcagcgaaacgccgcccatcaccggcaatgggatcatctggatagcggcagccagtttaccgacgcaggaaagcaggatagcgaaaatcgccgccccgccgataacccaggtactgtaaacacgggtgatcgccatcacgccaatgttttctccgtaagtagtatttggcgtagagccaaagaagccggaaatcacggtcgacaagccattagcaaacatcgaacggtgcagacctggatcgcgcagcagatcttttttgacgatattagccgttactaccaggtgccctacgtgttcggcaataaccactaacgccgctggcagaatagtcagaatggcaaaccactcgaagcgcggcgtatagagggttggcagcgcaaaccagtgagcattaataatcggcgtggtatcgacaattcccattgcgaaagagagcgcgtaccccaccagcacgccaattaaaatcgggataattgccaggaaaccacgaaacagcacggaacctaaaaccgtgaccgccagggtggtaatagagatgatgatggttttggagtctggcgtttgcccttcagccgggagtaaacccgccataccggcagctacgcccgccagctccagaccgatgacggcaacgattgcgcccattgccgcaggtggaaacagcacgtccagccagccggtccccgctttcttcacgataaaagaaaccaggcagaacagcacgccgcacataataaagccgcccagcgcgacttcataccctaacggcaacagtaacaataccggtgaaataaaggcaaagctggaaccaagataagccggaattttccctttacagatgaagagatacagcagcgttccaataccgttaaataacagtacagtcgccgggttaatatgaaataagacgggcaccaggacggttgcaccaaacatggcgaacaaatgttgcaaactaagcgggattgtctgtaaaagtggcggtctttcactcaccccgatagcacggcgcgtcatagtattatcctctgtattatgtgttataggcgctttactcaaaaaaaagccgactcttaaagtcggctttaattatttttattctttatttcgtaccaaagattttgtcaccggcatcgccgaggcccggaataatgtatccgtgctcgttcagtccctgatcaatcgatgcggtatacagttcgacgtccgggtgcgctttttccagcgcagcgataccttctggcgcagctaccagcaccagaactttgatgctgctgcagcccgcttttttcagcaggtcgatggtcgcgataacggaaccaccggttgccagcattgggtcaacgatcagcgccatacgctcatcgatgttagaaaccagtttctggaagtacggtaccggctccagcgtttcttcattacggtacataccgacaacgctgatgcgcgcgctcggaacgttttccagcacaccgtccatcataccaagacccgcacgcagaattggcacaacggtaattttcttacctttgatctggtcgatttctaccgggccgttccagccttcgatagttactttttccgtttcgaggtcggcggtcgcttcgtaagtcagcaggctacccacttcggaagcgagttcgcgaaagcgcttggtgctgatatcttgctcacgcatcagtcccagcttgtgtttgacgagtgggtgtttgacttccacgatcttcatactctttctcctttgaggggcagccacaaaaaaaatcgacggattatacctcctttcttcaaggcggcaatattcttttcgttgactttagtcaaaatgataacggtttgagataaagttattttatattcagatggttatgaaagaagattattccatccgaaaactaacctttaccctggcacaagtcttctttcgccgcgcgcctggggaaaagacgtgcaaaaaggttgtgtaaagcagtctcgcaaacgtttgctttccctgttagaattgcgccgaattttatttttctaccgcaagtaacgcgtggggacccaagcagtgaccgataaaacctctcttagctacaaagatgccggtgttgatattgacgcgggtaatgctctggttggaagaatcaaaggcgtagtgaagaaaacgcgtcgtccggaagtgatgggcggtctgggcggcttcggtgcgctgtgtgcattgccgcaaaaatatcgtgaacccgtgctggtttctggcactgacggcgtaggtaccaagctgcgtctggcaatggacttaaaacgtcacgacaccattggtattgatctggtcgccatgtgcgttaatgacctggtggtgcaaggtgcagagccgctgtttttcctcgactattacgcaaccggaaaactggatgttgataccgcttcagcggtgatcagcggcattgcggaaggttgtctgcaatcaggctgttcactggtgggtggcgaaacggcagaaatgccggggatgtatcacggtgaggattacgatgtcgcgggtttctgcgttggcgtggtagaaaaatcagaaatcatcgacggctctaaagtcagcgacggcgatgtgctgattgcactcggttccagcggtccacactcgaacggctattcgctggtgcgcaaaattcttgaagtcagcggttgtgatccgcaaaccaccgaacttgatggtaagccattagccgatcatctgctggcaccgacccgcatttacgtgaagtcagtgctggagttgattgaaaaggtcgatgtgcatgccattgcgcacctgaccggcggcggcttctgggaaaacattccgcgcgtattgccagataatactcaggcagtgattgatgaatcttcctggcagtggccggaagtgttcaactggctgcaaacggcaggtaacgttgagcaccatgaaatgtatcgcaccttcaactgcggcgtcgggatgattattgccctgcctgctccggaagtggacaaagccctcgccctgctcaatgccaacggtgaaaacgcgtggaaaatcggtatcatcaaagcctctgattccgaacaacgcgtggttatcgaataatgaatattgtggtgcttatttccggcaacggaagtaatttacaggcaattattgacgcctgtaaaaccaacaaaattaaaggcaccgtacgggcagttttcagcaataaggccgacgcgttcggccttgaacgcgcccgccaggcgggtattgcaacgcatacgctcatcgccagcgcgtttgacagtcgtgaagcctatgaccgggagttgattcatgaaatcgacatgtacgcacccgatgtggtcgtgctggctggttttatgcgcattctcagcccggcgtttgtctcccactatgccgggcgtttgctgaacattcacccttctctgctgccgaaatatcccggattacacacccatcgtcaggcgctggaaaatggcgatgaagagcacggtacatcggtgcatttcgtcaccgatgaactggacggtggcccggttattttacaggcgaaagtcccggtatttgctggtgattcggaagatgacatcaccgcccgcgtgcaaacccaggaacacgccatttatccactggtgattagctggtttgccgatggtcgtctgaaaatgcacgaaaacgccgcgtggctggatggtcaacgtctgccgccgcagggctacgctgccgacgagtaatacccccgtaattaaagcgccagctctgccgctggcgtttttcaattcacctgtaaatcgcaagctccagcagtttttttcccccttttctggcatagttggacatctgccaatattgctcgccataatatccaggcagtgtcccgtgaataaaacggagtaaaagtggtaatgggtcaggaaaagctatacatcgaaaaagagctcagttggttatcgttcaatgaacgcgtgcttcaggaagcggcggacaaatctaacccgctgattgaaaggatgcgtttcctggggatctattccaataaccttgatgagttctataaagtccgcttcgctgaactgaagcgacgcatcattattagcgaagaacaaggctccaactctcattcccgccatttactgggcaaaattcagtcccgggtgctgaaagccgatcaggaattcgacggcctctacaacgagctattgctggagatggcgcgcaaccagatcttcctgattaatgaacgccagctctccgtcaatcaacaaaactggctgcgtcattattttaagcagtatctgcgtcagcacattacgccgattttaatcaatcctgacactgacttagtgcagttcctgaaagatgattacacctatctggcggtggaaattatccgtggcgataccatccgttacgcgctgctggagatcccatcagataaagtgccgcgctttgtgaatttaccgccagaagcgccgcgtcgacgcaagccgatgattcttctggataacattctgcgttactgccttgatgatattttcaaaggcttctttgattatgacgcgctgaatgcctattcaatgaagatgacccgcgatgccgaatacgatttagtgcatgagatggaagccagcctgatggagttgatgtcttccagtctcaagcagcgtttaactgctgagccggtgcgttttgtttatcagcgcgatatgcccaatgcgctggttgaagtgttacgcgaaaaactgactatttcccgctacgactccatcgtccccggcggtcgttatcataattttaaagactttattaatttccccaatgtcggcaaagccaatctggtgaacaaaccactgccgcgtttacgccatatttggtttgataaagcccagttccgcaatggttttgatgccattcgcgaacgcgatgtgttgctctattatccttatcacacctttgagcatgtgctggaactgctgcgtcaggcttcgttcgacccgagcgtactggcgattaaaattaacatttaccgcgtggcgaaagattcacgcatcatcgactcgatgatccacgccgcacataacggtaagaaagtcaccgtggtggttgagttacaggcgcgtttcgacgaagaagccaacattcactgggcgaagcgcctgaccgaagcaggcgtgcacgttatcttctctgcgccggggctgaaaattcacgccaaactgttcctgatttcacgtaaagaaaacggtgaagtggtgcgttatgcacacatcgggaccgggaactttaacgaaaaaaccgcgcgtctttatactgactattcgttgctgaccgccgatgcgcgcatcaccaacgaagtacggcgggtatttaactttattgaaaacccataccgtccggtgacatttgattatttaatggtatcgccgcaaaactcccgccgcctattgtatgaaatggtggaccgcgagatcgccaacgcgcagcaagggctgcccagtggtatcaccctgaagctaaataaccttgtcgataaaggcctggttgatcgtctgtatgcggcctccagctccggcgtaccggttaatctgctggttcgcggaatgtgttcgctgatccccaatctggaaggcattagcgacaacattcgtgccatcagtattgttgaccgttaccttgaacatgaccgggtttatatttttgaaaatggcggcgataaaaaggtctacctttcttccgccgactggatgacgcgcaatattgattatcgtattgaagtggcgacgccgctgctcgatccgcgcctgaagcagcgggtactggacatcatcgacatattgttcagcgatacggtcaaagcacgttatatcgataaagaactcagtaatcgctacgttccccgcggcaatcgccgcaaagtacgggcgcagttggcgatttatgactacatcaaatcactcgaacaacctgaataaccctatgccaatacacgataaatcccctcgtccgcaggagtttgctgcggtcgatcttggttcaaacagttttcacatggtcatagcccgtgtggtagatggtgccatgcagattattggccgcctgaaacagcgggtgcatctggcggacggcctggggccagataatatgttgagtgaagaggcaatgacgcgcggtttaaactgtctgtcgctgtttgccgaacggctacaagggttttctcctgccagcgtctgtatagttggtacccatacgctgcgtcaggcgctgaacgccactgactttctgaaacgcgcggaaaaggtcattccctacccgattgaaattatttccggtaatgaagaagcccgtctgatttttatgggcgtggaacatacccaaccggaaaaaggtcgcaaactggttattgatattggcggcggatctacggaactggtgattggtgaaaatttcgaacctattctcgttgaaagccgccggatgggttgtgtcagctttgcccagctttattttcctggcggggtcatcaataaagagaattttcagcgcgctcgcatggcggcagcacaaaaactggaaactttaacctggcaattccgtattcagggctggaacgttgcaatgggcgcttccggtaccataaaagccgcccatgaagtgttaatggaaatgggcgagaaagacgggataattaccccggaacgtctggaaaaactggtaaaagaagttttacgtcaccgtaatttcgcatcgctgagtttaccgggtctttccgaagagcggaaaacagtcttcgttccgggactggcgattttatgcggtgtgtttgatgctttagccatccgtgaactgcgcctttctgacggggcgttacgcgaaggcgtactgtatgaaatggaaggacgtttccgtcatcaggatgtgcgtagtcgcaccgccagcagcctcgccaaccagtatcacatcgacagcgaacaggcccgacgggtgctggataccactatgcaaatgtacgaacagtggcgggaacagcaaccgaagctggcgcatccgcaactggaggcgctactgcgatgggccgccatgctgcatgaggtcgggttgaatatcaaccacagcggtttgcatcgccactccgcttatattctgcaaaacagtgacttgccgggttttaatcaggaacagcagctgatgatggcgacactggtgcgctatcaccgtaaagcgattaagctcgacgatctaccgcgctttaccttgtttaagaagaaacagttcctgccactgatacagctattgcgccttggcgtattactcaacaatcaacgtcaggcaaccaccacaccgccaacattgacgctgattactgatgacagtcactggacactgcgtttcccgcatgactggtttagtcagaatgcgctggtactgcttgatctggaaaaggagcaagaatactgggaaggcgtggctggctggcggttgaaaattgaagaagaaagtacaccagaaatcgccgcttaatactttgcgggccgacgagaaatgtcggcccgcattattcaggcactttcgcgaatgggttcgatttcattcagcgtatcaattaacggctgcggcttaccaataagataaccctgcatataatcgatccccaaagagagcaccgcctcgcggatctcttcgttttcaacgtactctgccactaccagcattttcttcattcgcgccaggtggcaaatcgatgccactatctgataatccagactatttgacacaatattgcggataaaactgccgtcaattttaagcagatcggcattcacatttttaagccgcgcatagctggcgtagccggtgccgaaatcatcaatcgcaatctggcagcctaattcctgaagatgctgcaaggtgatttgcgcctgcttaacattggtcagagcattactttcggtgacttcaaaaataagttgccacgcttcaatctgatatttagccagcaactgactgacttcaacaggaaaacgagcctgacataccgaggttggagacagattaatagcaaaacggtgagcgggcatcttcgctctgttttcagccataaattgcagcgtatgctcaatgacccacatgtcgatactcgacgataaaccaaattcgtgcgcgaccggcaagaagctatcggggctgatcagttcatcattctcacctttcatgcgcagaagaatttcatggtaaacatcaccacgcataccggtaatcggctgggccatcaggaaaaaatggttgtgttccagcgcctgctgtagtcgattcatcatcgcgactttatctttcaattcgcgttgcaaatacattgccccgcgacgctgcatattttccggggcgttggtcacgatggaaagttcggcgaccgtatttagctctcccagcagcaggtagatatgattcactggcgagcgcacatagcagtaactgacgccaatctgcggttgcatcggcatgccatcccaaaagaaacgaaattgcttgagatggctatccagtgcggtaatgcgctcctggtgcgattctgtattcagtcgcagcgcgagatcgttacccgaaagctgataaacatcttcacccggttccagcaagggtgacagccagtgagaaagtttttgcttgtattgaatccgcagcatgatgccatagttcttaaccagcatttccatgccagggatgcgtaaataacaaagcgcagaccagggggcatcacgcaacgcgcgattcagggcgcgaacatttggcagatgaaccaccgggtccacatacgcaagccgctgaatgcgtctgactaccgctctctgacgggttgccagtacagccatataattgacaataaaagagaataccagataactggaggaggttatggtcagctgcgtggtatagccaggataaatgggaatgtaattttgatagctgtggatgctgatcatcaacacgaccgcccagagcagcgaaatcagcttataaccatagcgcatcgctccccacatcatcaggggcagcaataatgacaaggtataattggtgctaaaaattgtgcttttttcatttaacggcatgcataacagcaacaataaagcacctaatgccagtagccagagcgcgaactcttttttggtgactttggcatcaacctgctgttttaattgcgaataatagctacgtaaataaaatggatttcgcactacccgaatgatgaagtagcacagcgggacaccgatcagattacccaccagtaaggcctgataattgattaaagtcccgaggttaaaaggcatgacaccgaccagattttctctgctcgccagtaatcctacaaatgcagcaaactggaaaagtatcagaaacagcgttgcaggaaacacaatctgccagaatatacgctgggaaattaaacgggtatcaccatgtgaaacgttgttacgccggggagtaaagaccctgtaaccgccccaacagagaatgataatgataataaaattagccgttaatgatagcgtttcgtaaaaacccagctctgcatatttgcggacaaaaatccctaaggcgatccctggcaatgccgcccagctgaaaaacatcatcatgctgatcatcagtgccagaggcagataaaagagaaaaacctcaccggaagaaatatgcgcgaaagtattaatgtgggcgaaaatgggcaagattaaagaaggcaggaacagcggaagcccccaccatttatcacgtatttttatataagttgcattcagtttcatagatgctcagcagaatcccccacatcctgaaggaggtgtattcagacaggcatcccacctgacttcgaatgatgattattcatcactatagagagcattgattctaagtgtcatatgaaagtaccaattgatatatatcaaacaaaataaccctgattaatgaattattacgtttatcatgttaattcatcattattacatcatcattgtaaataattaaattaacttccataacattaaaatatgtatccactgacgcttttttacataacgaagaattgaccattttgtcctgttgtgccttaatgtaagtaccgtccacagcgtgggacatacttcaaggaaccttttgtgagtcaggcaaccagtatgcgaaaacgacaccgatttaacagtcgcatgacccgtatcgtactgctcatcagctttatcttcttctttggccgttttatctactcgtccgtcggtgcctggcagcaccatcagagcaaaaaagaagctcagcaatccacactctccgtcgaatcaccggtacaacgttagcggttaccttctccactttcacagaacataacggcacttcgctgtcggatgcttttgctgtttgggattatcaaagcggcagatattctttcatcttaaattttacgtctttatcctgactgatgtttatcctgtttggctgcgaaataaatataaaattaatatatatgttgtaatgatatatttttataaattattccctgcgtgaattttaataaatttaatctatccctttatacgcaatacatttactttcctcttttgatgatcttaaatgtcttatttttcgtaatgtgtataacaaggaatagtgatgaaatttaaaaaatgtcttctgcctgtggcaatgttagcgtcattcactctggcaggatgccagtcaaatgctgacgatcatgctgccgatgtttatcaaaccgatcaactgaataccaaacaagaaactaaaaccgttaatattatttccattcttcccgcaaaagttgccgtagacaactcccaaaataaacggaacgcacaagccttcggcgcgcttattggcgcagtcgctggcggtgttatcggccacaacgtcgggtctggcagcaattccggaacgacggcaggtgcagttggcggcggagctgtaggcgcggcagcgggttctatggtgaatgataaaaccttagtggaaggtgtttctttaacctataaggaaggcaccaaagtgtatacctctacccaggtgggtaaagagtgccagtttacgacaggtttagccgttgttattaccacgacgtataacgaaacgcgtattcagccaaataccaaatgtcctgaaaagagctaataatcaggaggagtcatgaagaaagtttttctttgcgccatcttagcctccttaagctatccggctatcgcctcatcattgcaggatcaactctctgctgtcgcagaagcggaacagcaaggtaaaaatgaagagcaaaggcagcatgacgaatgggtcgcggagcgcaacagggaaatccagcaagagaagcaacgtcgcgcaaatgcccaggccgccgctaacaaaagagcggcaacggcagcggcaaataagaaagctcgtcaggataaactggacgccgaagcctctgcggacaaaaaacgcgatcaaagttatgaagatgagctacgcagcttagagattcagaaacaaaaactggcgctggcgaaagaagaagcccgcgttaagcgagaaaacgaatttatcgatcaggaactgaagcacaaagctgcgcaaaccgatgtggtgcaatctgaagctgacgccaacagaaatatgactgaaggcggtcgcgatctgatgaaaagcgtgggcaaagcagaagagaacaaatcggacagctggtttaattaatcgatgttagtaacttcaatcctataattcttgaagataaaaaaccctctgtagtaacagagggttttgttcattcatagtgcagggtcaaatcattcccactcaatggtagctggcggcttgccgctgatgtcatacaccacgcgggaaataccgttcacttcattgataatgcggttggaaacgcgaccgaggaaatcgtacggcagatgcgcccagtgtgcggtcataaagtcgatggtttcgacagcacgcagagagacaacccagtcatacttacgaccatcgcccattacgccaacggaacgtaccggcaggaacacagtgaacgcctggctgactttgtcgtacaggtccgctttacgcagttcttcaatgaagatggcgtcagcacggcgcagcaggtcacagtactctttcttcacttcacccagaacacgaacgccaaggcctggtcccgggaacgggtgacggtacagcatgtcgtacggcaggcccagctccagaccaatcttacgcacttcgtctttgaacagctctttcagcggttcaaccaggcccatcttcatctctttcggcaggccgcccacgttgtggtgagatttgatgacgtgtgctttaccggttgcagacgccgcagattcgataacgtcagggtagatggtgccctgcgccagccacttcacgtcttccagtttcagcgcttcttcatcgaatacttcaacgaaaacgcgaccgatgattttacgttttgcttccggatcgttttcgccagccagcgctgacaggaagcgatcttctgccggtacgtgaacaatgttaagaccaaagtgatcgccaaacatatccagaacctgctctgcttcgttgaggcgcagcaggccgttgtcgacgaatacgcaagtcaggtttttaccgatagcgcggtgcagcagcattgcggttacggaggaatccacaccaccagagaggccgaggatgactttatcgtcgcctacctgctcgcggatgcgagctacagcatcgtcgataattttcgctggcgtccacagggcttcacactggcagatatcacgcacaaaacgctccagcatgcgcataccctggcgggtatgagtcacttccgggtggaactgtacgccatagaagcgtttttcttcgttagccataatggcaaacgggcagctttcggtgctggctacggtgatgaagtcggacggaatagcggtaactttatcgccgtggctcatccagacatcgagcagcggtttaccgtctgcggtcagcgcatcttcgataccgcgaaccagtgcgctgtcgtttacgacttcaacctgcgcgtagccaaattcacgttcgttagaggcttcaacgtgaccgcccaactgcattgccatggtctgcatgccatagcaaacgccgaataccggtacgcctgcttcaaagacatactgcggcgcacgcggactgttttcttcagtagtactttccgggccgccggaaagaataatgccgcttggattgaagtcacgaatttgtgcttctgtcacatcccacgcccacagttcgcagtaaacacccagctcacgcacgcggcgcgcaaccagttgagtgtactgagaaccgaagtccagaatgaggatgcgatgcttatgaatgttttccgtcattgacgcttattccgaggcaagtgaaacagataatataaatcgcccgacatgaagtcgggcgaagagaatcaggagcccagacggtagttcggggactctttagtaatggtcacgtcgtgaacgtggctttcctgaatgcccgcaccgctgatacgtacaaactccgctttagtacgcagttcgtcgatagtaccacagccggtcagacccatacaggagcgcaggccgcccatctgctggtgaatgatctctttcaggcgacctttataggctacgcgaccttcgataccttccggcaccagtttgtcggcagcgttatcgctctggaaataacggtcagaggaacctttggacatcgcgcccagggaacccataccacggtaagatttgtaagaacggccctggtagagttcgatttcacccggagattcttcagtacccgccagcatggaacctaccatcaccgcgcttgcgccagcggcgatagctttggcgatgtcgccggagaagcgaataccgccatcagcgataaccggaataccggtgccttccagggcttctactgcgtcagcaacagcggtaatctgcggaacaccgacgccagtcacgatacgagttgtacagatagagccagggccaatgccgactttaaccgcactgcaaccagcttctgccagagcgcgtgcacctgcagctgttgccacgttgccgccgataatttgcagatccggatatttagcacgggtttcacggatacgttgcagtacaccttctgagtgaccgtgggaggagtcgatcagcagaacgtcaacgcctgcggcaaccagcgcgtcaacacgctcttcgttacccgcacctgcgccaaccgctgcaccaacacgcagacggccttgctcgtctttacaggcgttcggtttacgttccgctttctggaagtctttcacggtgatcatgccgatcaggtggaattcgtcatcaaccaccagcgctttttcaacgcgtttttcgtgcatttttgccagcaccacttcacgggcttcaccttcacgcacggtgaccagacgctctttcggcgtcatgtaaacgctaaccggctggttcaggtcggtaacaaaacgcacgtcacgaccggtgataatacccaccagttcgttttcttcggtaacgaccggatagcccgcaaaaccgttacgctcggtcagttctttcacttcgcgcagcgtcgtggttggcagaacagtctgcggatcagtcaccacaccagattcgtgttttttcacacggcgaacttcttctgcctggcgttcaatggacatgtttttgtggataaagccgataccgccttcctgagccagagcaatagccaggcgcgcttccgttacggtatccattgctgcggaaagcatagggatattcagacgaatagttttcgtcagctgggtgctgaggtcagcagtattcggcagaacggtagagtgagcaggaacgaggagaacgtcgtcaaacgtcagagcttctttagcgatacgtagcatgggcaatatctcgaccagagtggttaataaatattgccgcggcattatacagagcgtaaccgattgcatctacccctttttgcaaaaaatgcttgctatccccgaagggcgggttactatcgactgaataacctgctgatttagaatttgatctcgctcacatgttaccttctcaatcccctgcaatttttaccgttagtcgcctgaatcaaacggttcgtctgctgcttgagcatgagatgggacaggtttggatcagcggcgaaatttctaatttcacgcaaccagcttccggtcactggtactttacactcaaagacgacaccgcccaggtacgctgcgcgatgttccgcaacagcaaccgccgggtgaccttccgcccacagcatgggcaacaagttttagttcgcgccaatattacgctctacgagccgcgcggcgactaccagataatcgttgagagtatgcagccggccggtgaagggctgctgcaacagaagtacgaacagctcaaagcgaagttgcaggctgaaggtttgttcgatcagcaatacaaaaaaccacttccctcccctgcgcattgcgttggtgtgatcacctcaaaaaccggtgctgcgctacatgatattttgcatgtgttaaaacgtcgcgatccttctctgccggtgatcatctaccctgccgccgttcagggcgatgacgcgccggggcaaattgttcgcgccattgaactggcgaatcagcgcaatgagtgcgacgtattgatcgtcgggcgcggcggcggttcgctggaagatttatggagttttaacgacgaacgcgtagcgcgggcgatttttaccagccgcattccggttgtcagcgccgtcgggcatgagacggatgtgaccattgccgattttgttgccgatctgcgtgcgccaacgccgtctgccgccgctgaagtagtgagccgtaatcagcaagagttactgcgccaggtgcaatcgacccgtcaacggctggagatggcgatggattattatctcgccaaccgcacacgtcgctttacgcaaattcatcaccgattacagcaacagcatccgcagctccggctggcacgccagcaaaccatgcttgagcgcctgcaaaagcgaatgagctttgcgctggaaaatcaacttaagcgtaccgggcaacagcagcagcggttaacacagcggctgaatcagcaaaatccacagccgaagattcatcgcgcgcaaacgcgcattcagcaactggaatatcgtttagcagaaaccctgcgcgcacagcttagcgccacgcgtgaacgtttcggtaatgcagtaacgcacctcgaagccgtaagcccactgtcaacgctggcgcgtggatacagcgttactactgctactgacggcaatgtactgaaaaaagtgaagcaagttaaagcgggtgaaatgctaaccacacgtctggaagacggctggatagaaagtgaagtaaaaaacatccagccagtaaaaaaatcgcgtaaaaaggtgcattaagccagcacgaattcaacgcgttttttcgatatcaagccatgcccgtgctgacagaagtaatctactgcaccacaggcttttaacacctgcaacggttgatggcagtctggacaaagagctttcatttcaataaattccccgcaggatcggcaacgcgcatggccgttatcctgatcaagcacatgctgacattgtggacaatgcagttccatatgaattcctccggtagccattccctctacattcatagagggaatggcagataaaatacttacggataattatttatttttcttgatgtgcttcatcagacgcttacgtttacgcatctgggttggcgtcagggtgttacgcttattcgcatacgggttttccccttctttgaactgaatacgaatcggcgatcccattacgtccagcgatttgcggaagtagttcatcaagtagcgcttgtaggaatcaggcaggtctttcacctgattaccgtgaatcaccacaatcggcgggttataaccaccggcgtgggcatatttcagcttcacacgacgaccgcgtaccagcggcggttggtgatcttcaacagccatcgtcatgatgcgcgtcagcatagaggtccccacacgacgggtggagctgtcatacgcttcacgtactgattcaaacaagttaccaacaccactgccgtgcaaggcagagataaagtgcacacgagcaaaatcgataaagcccagacggaagtccagcgtttctttcacctgctctttcacttcctgactcaggccatcccacttattcaccacaatgacaagtgagcgcccactattgagaataaagcccagcagcgagagatcctgatcggaaataccttcgcgcgcatcaatcactaacatcaccacgttggcgtcttcaatggcctgcaacgttttgattacggagaatttctctacagcatcggtgattttgccgcgtttacgtacgccagcggtgtcaatgagcacatactcacgtccatcgcgttccattgggatgtagatgctgtcacgcgtcgtgccaggcatgtcgtaaacaacaacgcgctcttcaccaagaatacggttagtgagtgtagacttacctacgttcggacgacccacaatcgccagtttgatcggcagactttgcgggtcgaagtcgtcttcctcttcttcttcgccgttctcttccgcttcaaattgcgcccagtattcagcgtcttcgtcgacttcctcttgcggtgcgagatcttccatccacggcagcagcacatgctccagcagacttaatacgccacgaccgtgagacgcggcgatcgggtagatttcacctaaaccaagcgagtagaaatcaaccactgcctgatcgggatccagaccgtcagttttgtttgccaccaggaaggtcggtttttcacgggagcgcagatgtttggcaatcgcttcatctgccggcatcaggcccgcgcgcgcatccaccataaacagtacgacgtccgcttcttcaatcgccagcagcgactgttccgccatgcgggtttctacaccgtcttctgtgccatcaatcccgccggtatcaatacagataaactcacggccttcaatttccgcacgaccgtacttacggtcacgagtcagacccgggaaatccgcaaccagcgcatctcgggtgcgagttagacggttaaataacgtggattttcctacgttagggcgcccgacaagcgcgaccacaggtaccatgtttaaagcctcatttttataaatcatcagacaacgcacgctatattcgcgtcgttgttaaaaacaggaaaacggcccctgtccaggagccgttttcaaagtgaacgacagagacgattaacgtgtaatagagtacacggttccgtcttttgcctggatcagcagtttgccgtcagcggcaaccggttcagtctggaaaccggaactatcaactttttgctgggcaacgaaacgaccatcttcgacgttaatccagtgcagataaccttcactgtcaccgaccaccaggttgccattatacagcaccggagaagtcagcaggcgatgcagcagatcgctttgtgtccacagcgtaacgccgccatcaatggtcaacgccatcacccggtcattttgatcgaccagatagatgcgattgccgtcgacgatgaaatcattcaccgaacccagttcgcgtttccacataatctgaccactgcgcagatcaagcgccgtcaggttaccattataggccagcgcgaaaacaacgccgttaacaacgacgggagtcgtgtcaacatcgctcagacggtcaatttcggtagaaccggtcgcctgggaaatacgctgctgccaaatcatctggccctgttccatcagcactgcgctgacgcgaccattatcgccccccacgacggccgcaccaaaagccgttgtcggcgcagactcgccacgcaaagagagcgaaggcatatcgaggttaactgtccatttgacagcgccgtcagcttcgttcagcgcttgtaactgaccgttactggtgtggattaacaccagaccgtcgctgaccaccgggcgcgaaagtgcttcacccgcgactttagtttgccatgccacagtaccatcgctggtattcagcgcgtaaacctgcgccttttcgctgccaatgtagacatgcccaccagacacggtcacaccgccagaaagtaatgcaggctctttagagaaccagccatctttctcggccaggctgacagaccagatttctttgccatcatccgcattcagcgcttttactaaaccagcgcggtccgctgcatagacaacgttgtccgccagtgccggatgaagattggaatagaagttgccaatgccgctaccaacggaagtgctccacgccgtggtcggcgtaaactggttttcaacggttggcaatggggacatctttaccacatcttcttcgctgttaaacagcgaacagccgcttaaaagggtaacggaaagcagtcctggcagcagtaatttacgcaattgcatcgggtccctctcagatggacaaattattaattttcatctgcatcatttcgctcagtgccggagtaacatcgcttttcacgcctgcttcccatgcactacgcgcaccttgcttatcacctttgctcagcaatgcttcaccacgcaggtcggcaacaatggcagcccacccttcacctttgatggtatcaagggttttcagcgcggcatcagcctgcttgagctgtacctgaacgcgagcaagacgcagatttatcacggctttgagattttcatcgctcgtgtctgccagcccctgttgtaactgggcggcagctttctctagttcatttttgtcaacaaattgctgcgcaagttccaaagaagccagcgcaccataagtatttttattttcagcagcaaatttttccgccgccgggatgctatccggtttgccttcgctcactgcggtaaccgcattttgataggcaagagaagcggagcgtgcagaatcaacctgatggctgttccagtagcgccagccaatcagtgcgccaacgcccaaaatcaccccaacagccagtgctttgccattttcagcaaaaaagcgtttaaccgcttctacctggtcgttttcgttctcgtaaatttccacgctgtccttctccttccttaacccagtaacgtgcgcaaatgcgcggctacgctatcctgcgcaactgccgtttgctcaccagagcgcaaatccttcactactgctgtgccgttagccacttcagactcacccagcaccacagcaacgcgggcaccccatttatcagcacgggcaaactgtttcttaaagttgccgccgccgtggttggtcatcaatttcacgcccggtaattcatcacgcagacgctcagctaatgccatagccgcagattgtgtatcagcacctgaagccaccaggtatatatcgacaacaggatcggctttaaattccggattaacggcctgtactaacaatacaagacgttcgaggcccatagcaaaaccgacagccggtgttgcacgaccgcccagttgttccacaagaccgtcataacgaccgcctgcacacacggtgccctgggagccgagactgttagtcacccactcgaaaacggtacggttgtagtaatccagaccacgcaccagacgctggtttacggtgtaagcgatccccgcgctctccagcagtttgcacagaccggcaaaatgctcacgagattcctcgtccagatagtcacctaatgccggagcgtcgttgagaagcgcctgcacttccggattttttgaatccagcacgcgcagcgggttagtgtacatgcggcgtttgcagtcttcgtccagcttttctttatgctgctcaaggaatgccaccagcgcatcgcggtaattggcgcgtgcttccagcgaaccgatagagttcagctcaagagttacgtgctcggaaatacccagcgcgcgccaccagcgggcagtgagcataatcagttcagcgtcgatatccggaccttgcagaccgaaaacttcgcagcccaactgatggaactgacgataacgccctttctgcggacgctcgtgacggaacatcggcccgatataccacagacgctgttcctgattgtacagaagaccatgctcgatgccggcgcgtacacagcccgccgtcccttcagggcgcagagtcaggctgtcgccattgcgatcctcaaaggtgtacatctctttttcaaccacgtcggtgacttcaccaatcgcacgtttgaatagcggggtctgctctacaatcggcaagcggatttcactgtaaccgtagctgccgagcacgtttttcagtgtgccttcaatgcgctgccagatggccgtttcgccaggcaggtaatcgttcatgccgcgaatggcttgaatgttttttgccacgtttattctctttctgaatataaaaatgaaccctcaacgcttccctcaatgtttcgggagccatgcgggttcaatcatacacgggaagcgaggcgcttcccatcacgttattatttttcaacctgctgaacgtcaattcgacgcgcttcgtccagctgactggctttcgcacgaatgcgtgcttccagctggtcgatcatatcgttgttgtccagacggtctttgcgcacgccatcttcatagaggccgcttttcttgttgccgccggtgacgccgagtgtagaaaccagcgcctcacctgggccattcaccacgcagccgataatcgaaacgtccatcggagtgatgatatcttccaggcgttgctccagcgcgttaaccgtaccgataacatcaaattcctgacgcgaacaggtcgggcaggcgatgaagttgatccctcgcgaacggatacgcagcgatttcaaaatatcgaaaccgactttgatctcttcgaccggatcggccgccagcgatacgcgcagcgtgtcgccgatgccttcagacagcagcagacctaaaccaatggcggattttactgccccgctgcgcgcaccaccggcttcggtgatccccagatgcaacggctgatcgatctgttttgccagcaaacgataagactcaacagcgaggaagacgtcagacgctttcacgctgactttgaactgatcgaagttcaggcgatcgagatgatcaacatgacgcatggcagattccagcaacgcctgcggcgtcggttcgccatacttttcttgcagatctttttccagcgatccggcgttaacgccaatacggatcggaatgtttttatcgcgcgcacagtcaaccaccatgcgaatacgctcttcattaccgatattgccagggttaatacgcagacaatcgacgccgtattccgctactttcagcgcaatgcgatagtcgaagtggatgtcagccaccagcggcacgttaacctgctgtttgatgagtttgaacgcttctgccgcgtccatcgtcggtacggatacacggacgatatcagcgccaacgcgttccagcgccttgatttgattgaccgttgcttcgacgtctgtcgtacgcgtattggtcatggactgtacggcgatgggagcaccatcgccaatcggcacattcccaacgtaaatacgtgttgattttctacgttgaattggagcctggttatgcatgaaaaatctcccgcgttacccgtctgttactgcgccggtgattgttcggcattgagggtcagacgcgcaacctggttagttctgataaaacgactcagatcgacaggtttcccttgatactggatctgtactgcggctggcgcaccaattttcagtttgtacggtgcctggccggttaagttcaaattaccgtctttacgctgcataccgctaaacaattttttaccggtagcatcagtgacctccagccagcaatcggcagtaaagttcatcaccagcgcattcggatcagccaccggcgtggtcacgccagcctgatcggttggcaacggcgcagcaccatctggcgttgttgctgccgttggtgccggggtcgcggcggtatcaacatttgcctgcgaaggcgaaacaaccgcattctgttgcggatcaacagctggtgctggcgcagttacggcaggtgtttgcgtgttggttgcggtagtatccacagacgctggcggcgtggacgttgtagccgggtctgtagttgtcgacgtatttaatggaacactctgcccctgctcgctattactgctcagttccgccgaagattgatcggccatagtggtgatctcttcctgctgagctttgcggtcttgccaccaccaggcaccgctcaggccgataaccacaaacaacaccagccaagtgaaggtcatcagccagccgtcgcgttttttgcggcgtttaccgagggaaaaactctgcatcggcgcaacttttgcagcccgaagtggagcctgcttttccagccctggcagcagttcttcttctggaatatgtaccagacgcgcataagagcggatatatccgcgcaggaatgttgaagcaagatcggcgggtgccttatcttcttcaatgtcgcgtaccgtggaaaccttcaggcaaagtcgctcggcaacggcctgctgactaagtcctagttgttcgcgagcattacgcaggcgagcgccggtagtaagtgcttcattttggtcgtgcgtggcttcagtattcattcgctgcaggtacgtttaaatgagaattgagatgccggtgaaccatcatgctcacccacaccgcgaaacatccgttaagttaaccgttatcatacagtataagaccgtctgtgtgctcgtgacaaagcccacattcactaaggctaacttactgttgcatcgttacatactgccttaaagtcagcaaaaacgcaccgttaatattgaccagacaattgcaacttaatacttcattcataaaacattacgccacggtacataaagtaaccgtggcgtaatggctatcagaccgctttaatgtcgatggcttcaccctgcatccgtttacgcagggtacgtttcgtacggtcgataacatcgcccgccaactgaccacaggcagcatcgatatcatcaccacgagttttacgcacaatagtggtgaaaccgtagctcatcagcacttttgagaaacggtcgatacggctgttcgagctgcgtccatacggcgcacccgggaacgggttccacgggatcaggttgatcttacacggcgtatctttcagcagttccgccagttggtgcgcgtgttcagtgccgtcgttaacgtggtcaagcatcacgtattcaatagtgactcggccctgattggcgttggatttctccagataacggcgcaccgcagcaaggaacgtttcgatattgtactttttgttgatcggcacaatttcgtcacgaatttcgtcgttcggcgcgtgcagggaaattgccagtgcaacgtcgatcatatcgcccagtttatccagcgccggaactacaccggaagtggaaagcgtgacgcgacgtttagacaggccaaaaccgaaatcatcaagcatgatttccatcgccggaacgacgttgttcaggttgagcagcggctcgcccatgcccatcatcactacgttagtgatcggacgctgaccggtgacttttgctgcgccgacgattttcgccgcacgccacacctggccgataatttccgacacccgcaggttgcggttaaagccctgctgggcggtggaacagaatttacactccagcgcacaccccacctgcgaagagacgcagagcgtggcacggtcgtcttccgggatatacaccgtttcgacgcgctgatcgccaacggcgatcgcccatttaatggtgccgtcagatgaacgctgttcttcaaccacttccggtgcgcggatttccgccacctctttcagtttgccgcgcaacactttgttgatgtcggtcatctcatcaaagttgtcgcagcaatagtgatacatccacttcatcacctgatcggcgcggaagggtttttcacctaaatctttaaaaaactcccgcatctgctgacggttgagatccagcaggttgatttttccatctttcgtggtgacgttttcaggtgtgactaattgttcagacatatgctattccggcctcgttattacacgttatggcccctggagggttgaaaaaagaaacgccccggtgagcggctgctcgtccgggggcgctgcattgtacaaattctggcgcacggatgccacgtttgcacgcggcatttacgaaattattaacgggtgcgcgggcacacttcgccttcgccaaagaaataagcgatttcgcgagcggcagattcgacggaatcagaaccgtgggtaccgttttcggtcaggctgtcagcgtaatcagcgcgcagagtaccagccagtgcgtttgccggattggtcgcgcccagcagatcgcggtgacgctgaacggcgttttcaccttccagcacggaaaccacgatcgggccagaggtcatgaattcaaccagaccatcaaagaacggttttccatcgtgttcagcataaaagccacgtgcctgttcaacggtcaggtgcagcattttggtgccaacaattttgaaccctgcagcttcaaagcgcgcaaagatattaccaatgacgttttttgctaccgcgttcggtttgatgatggaaaaagtacgttcaatagccatttttacctctgtaaattgttctgttgttgtctgtaccagcgtacgagatggcgcggattataatgagcaacagggccgttgactattgatgaaggtaacatttttttaaaataaaatgagttttagcaacaatcagggacaaaacagactattgcatgacaaatttcactgtcgcgatttgccccacgtcatccatcaccagcaattgataatcacctttatccgtcaaatgcagggtcacgttgcgcccgcgttcagttaacggttcgccattcagaaaccaccagcgttcacctgcccctccacttgattgcaacggcaaagtcgcttccgctgcgcccggtaaacgtttaataatcgcgccatcgcgaacgcctgtcagctgcagcgggagctgggcatcgtgaccgtatggcgggcaacttgtcgaggccggtggtaagcgcacagcgcgacgttctgatgcgggcagccagggttccagcggtagcggccagacatttatcatttcttgtcgcgcttgcgggcaatcagcggcaacacgtttgccattttcatccagccagatggggaaacgaatgccattaatgccttcctgctccggcagtaatagagttggcggctgactcccgtccagcagccaggttgccaggcggcggcgacagttaccgtcaccttccggcaaagactgtccgcccggccagcagataacgccacgagtgactgagttcgggcgcgggtcttccggcagattcgcactgcgcgacagtaagatattattgacctgattcaacaatggtacggcactggcaaagccaaactgaccaacaacgggcgtgccgtccggtctgccagtccagatcccaatgacatagcgagcgttaaccccaatcgcccaggcgtcacgatagccatagctggtgcccgttttccatgccagtggggcgacgcgcggcaaggcactatccggcaagggttgcgcttcatcagccataatccggcgaatgatccacgccgcccccgacgacattaaaggccgttcaagcagcggatcgtcaggctgtaagcgcaatttgcctgccttgccgtggcgagcaaacgcggtatacgctgccgccatatcttccagttttgcaccagcgccgccgagaatgagtgaaagattcggcgcagcaccgttgggcaaatataacggcaatccaacattgcgtaactttgccgcaaaccgtttcggtccataggcttccagcacctgcacagcaggtaagttcagcgagcgcaccagcgcctcgctcatgctgatcgggccatgaaaaccgctatcaaagttacctggtcgataatcaccggtgcgccgggggacgtcttgcagcagtgatgccgggtggatcaagccttcatccagcgccagaccataaacaaacggtttgagcactgatcctggcgatcggatcgaattgaccatatcaacatgaccaaagcgtgaatcatcgttgagatcaaccgatcccacccagccgcgaacacgcatatcggtatgatcaaccacgatcatcgccagtgagctgcgcggtggcaaccgccctttccagttttgcgccagttcttccagacgtcgttgaagaccggcatccaacgtagtagtgattttgtcgcttttgcttttaccgagcatcatgcgcgaaaacagcggtgccagttgcggcatttgtcggggggccagccagatgggttcttcccttgactcttttacctgctcacgggaccacacaccttgcacggccatccgttcgagcactttattacgcgcggcttcggcacgctccggccaacgatccgggcgaagacggctgggcgcttgcggcaaaaccgccagcattgccgcctcggaatagcttaaattcgcaggcgattttccgagataagcccaacttgccgcaccgatcccctgcaacgtaccgccaaacggagcgcggttaagatacaaggtcagaatttcacgcttagacagatgccattccagttgcaacgcgcgccagagctggcgaattttgccgccaaatgttttggggtgaggatcaagcagacgagcaacctgcatagtgagcgtgctgccaccggaaataacccgtcccgaagtgagatcttgccatgctgcgcgcgccaccgagaatggattcacccccggatgcttccagaaccagcgatcttcataattgatcagcgcttcaaggtaacgtggagaaacatcttcgattgttaccggataacgccagatgccgtcagcatcggcgaagcgccagagcggcgtaccatcctgcgccacgaccactcgtgcgggattgacttcatgcagcggtagaggccagagtttatctgctccccacgctgcaagaaaaaggagaaagggcgcggctgccaacgttatccagcagccgcgtttggttaacaagcgaggcatttacggtctgacaatcagcagatcttcagccgcgccggtcgcccgccattggggaacatacattgattccaccatcggttgcggtacctgatacgttcccggcgtcaccgcccgcgccagatacaccagcgttaccggttggtattcatcaacggcaaccgccgccacaaagcgatcgtcacggaactcaatgtgcttaatgctcgcctgctgcatctggttcagtaagttctgcacttcgccaccactttgctccaggctggcgctaccgttcgccagattctggttttccagttccagacccgcaggcagcagatccacgactaacgcatccggcacgctgttactggcttttacctgcaaccacaccagcaccagatcgccgctacgtaacgagtccagcgatttgctcttaccatcagtaccaagaatatgacgctcgatttgcagcacattgttcgccggtaaaggtgcggattgcggataaccgctggcatccatacgcaaccataacggctgatcgccactgttgctcacctgcaaggtgacaagttgatcgctattcagattgctgttttgcgctttctcgcctgtcagctgctcagctgagaaagaggtttgcgcctgccatttaccgggtaaatcctgaatcgtacgggcagccaggaacaacgcgttactttcctgcgtcgatagccagcgttcaccaaacgcctgctgcgaaagtgtgttcagcaaagtgtactgctcatcgggtagcagtttattttcttccagcaaggagagcattaacgcgttgtcgcgcagtgaactaccgtaatcacccagccatatccgctcatcactattacgcggcgttttcagcgccagcgcaatcgcttcttcaccacgcgtcgcatcacccatggttttcagcgcaacgccaagttgcagcagcggtaaaccagaagcggcatctgcacgatgctcccagatttcacgcagcgcacccagcggagccttttgctgacgggccaacaccagcgcagcgtaagactgtacggcgaatttactggctttgagattatccgcgtacgggatcgacatcatgcccggatcttgtaaatagcgcagcagacgctcattaccccggttaatggcgtctgtcggcacgctgtaaccctgttcgcctgcgcggaccaggaaatccatcacgtaagccgtcagccagtactcttcgtcaccgtttttatcccacagcgcaaagccgccgttatcacgttgcatttgcagcaaacgggaaatgccgatatcgaccgatgcacggcgtttctcatcactgtcgcctttgatgcccaacgcctgcagttgggctgcgttggtataaagtgacggaaacaggccgctggcggtttgctcaagacagccgtacggatacgcttttaactctttgatataacgtgcgatgttcagcggtggtttgccgctcaacaacaattgcccttccagcgtaacaggcgagaagttttgcaatccatccgccggaatcgcccatgtctcaccaggctgtaacgccgtaccgtaattaaccgtttgtgccgggaacgccggacggacgccgattttccactgcttatgctgatcggcaacggtttcacccggtaacgctaacccgctaatggtggcctgaatttctccatcgccataacccggcaatgctcgcaccgggataaacagcgtagtacgcacacctggcgctaattcaacggctgcgggtgaatcgctgaccagttcaagcaaaccactggcggtcagggcaacgttcagtttttgcggtttatcggtaagattagtgatatccagcgtcagacgcgaggtatcgccactcgccataaagcgcggcatgttcagttcagcaatcaccggtgcggcaactatcactttactttcgttgctaccgaagtcatctgccgtccaggcttgcgccatgacgcgcaattcaccgttaaaatcgccaatcggcagtgtaaccgagccttcgccctgttcgttgagcgttaccggcagcgcctgctgcacgacaatattgacgtgattgaccggcggtttaccaccacgtttcagctcatcaccatcgccaccgaaacgcagagctgccagacgcccctgaccttcaataacctgaccgtaaatatcgtaaatgtctgcgccatagcgtttctgaccaaagaacgcctgccacggatctggcgtgacgtagtcagtaatattcagcacaccactatcaacggcagacaccagcacattcacctgtttaggcttctcgccatttttagtgctggctttaattttcacggttaatggttgattgggacgcatttttgctggtgtttccagcgccagatcgaggcgacggttttcatcgccaagcggcagatgcaacacaccaaccgcgcgttttggcgtcgcggagcgagatttatcgccaggacgtaccaccagcgtacttaaatacagatcatgacgattccaggttttatcgaccggaatcgtcagatccagcccttgagcccgaacatcaatctcttgccaccacagcggcccttcactggactcgaccatcgcataacctttacccgccgttggcgcggcgatatgcaacttaatggtgtcgccagggcgataactggctttatccagtttcagcgtgacacggtcgggtcgcactgcgccgctaccgtcgctgttgtcctgccagctatagccagcccagaaacgaacactactgaccgcttcattcggcgctttgacttccagacgataagcgccccactctaccggaaaactgaccttgccggtttcgtccgctttcagatccagagtttgttcattttcgatcagatctttttgatcaaactgtgactgccagccttcatcttctgaccagttccagtagtaatcgcggcgttcgcgaatcaggcgcacctgcaagcccgacacggcttttttcacgccttgcgcatcgctataaacgatgtcaaaagcggcgttactgccttcatcaacaatgggctgtttcaccgtgctgtcagtacgataatcgtaaaccgatttcgaggcgaactgcggacggatccccggcaatgcatcggcaggccagatagcctgctcagcgcggcgcgtcaccgggcgaccgcccgattccagcaaactaccctggaaaataacctgtaatggggaatgcgtttccttccactggctttctgtagaaacttcgccgcgccctttatcatccagcgtcaactgaacttcatccagcgtgcgggaaagattttcggcagctatatcgccgaattcaaaaccaggtaaggctgacacagcttcacgcagtgggcgcaggaaaagttgcccttgcaaagtattaccattagcaggtgcaccatacaggtagtaccccaccacggagaatttcacttcatctttcggcgttagcggggttttctcaccggtcagattcagcgccatgcgctctggcataaaatcttcgacgtggaaatcccacatccgatactgattatcgcccgtgttagcgcgaatatgccacataccggttgccgcattgctatcgagtggccaggtaaagtggtagaggccattctccggctgactaacgacgctcctgagtacctgcccatcgggtttaatcacgtctaacttgatgggttgattgggcaacgctttaccgtctgcatcacgcagcaaaccattgaggattaccgtttcacctgggcgataaagatcgcgtgggccaaacatgaaaaactgtttgctatagcctggcgcgccagcaatgttaaattctgctaagtccagcgccggaagttttaaatcgagtagcgttgtctgaccgtctttacgcgccaacagtaatgccgcgtttttatcattttccagctgcacatgcccctgagcgtcactggttgcctgagtcagagtctgccctttctcatttaataaagagacttcaattccttgctgggccgcgccgttttccagactttgggtaaagatatccagacgattgtgataacggtgagctgaaacgccgatatcacttaacgtaaacagcgtcgcgggattactgtaatcgtaacgtccagcctgattcatcacagccagatacacgcccgcctgctgaagcggtttgatatcgcccagcggcagcaataatttttcacgggtgttacgcgcaggattgagatcaaaccgtccggtgtagaccagatccgccatctgcagcagtttgtctgactgccagttcgccagcgaattgcggtattcccattggctaatgaatgctggcagagattctggcttaacgcggaagaagttaacatcgacattattaacgttgagcgccattaccggcagcccttcaacgactttgccaggcagcagcgaaccacggctggcaaaaccgacgctgggttggatgtcgcgggtagttatagttttttcgtaatctttactgaaggttgcgttgttgagtgctttgacctccttgccaatagtaacgatcaaatcacgtttcggttcgaggtggcgtaaacgtaactctttaagattatctgacagctcccaggcaccatccactttgccgctttttttatcgacgacatgaataacgcgtgagaaatcctgatccgggtcgagagggatggagaacgtcagcaccagcgtggctgcaccatcaagttggacttcagagagatccagcaatgtcagcaccttaccggcactctgttgggccagtttttgtctctccggcacggagagttttgctgaactcgcgttttctgaagaggccgctttagtaacttcagaaggcgcatcttttttcaccgctgttggcgcgttatcgttgttgtcgcaccctgccagcgccagcattagcatgcaggcggctacgcgtaactttttcatttttcatccctgccacaatggcccgttagcaacgtcgaataattattatgcgtgagaatttacgttatgtaattcagtatcacgcccatacaatccgaattttagtgagaattgtggctcagacagccaaatcagcctcttttgcttgtcgcttttcactaaacatccgacaatttagcctaaccccggcaaaaatggagatgcctatgtccacgacatggtttgtaggagccgactggctcgccgaacatattgatgacccggaaattcagattatcgatgcccgcatggcgtcgcctggacaggaggatcgtaacgttgctcaggagtatctgaatggacatattcccggcgcagtgttttttgatatcgaagcgctttctgatcacacttccccgcttccgcacatgctgccgcgcccggaaacgttcgccgtggcgatgcgtgaattaggcgttaaccaggataagcacctgattgtctatgacgaaggtaatcttttctcagccccacgagcatggtggatgctgcgcacctttggtgtagagaaagtgtcgattctggggggtggacttgcaggctggcagcgcgatgatctgctgttagaagaaggtgcagtagagctgccggaaggagagtttaacgccgcgtttaatcctgaagccgtggtgaaagtaaccgatgtattattggcaagccatgaaaatacggcgcaaattattgatgcccgcccggctgcacgttttaacgcagaagttgatgaacctcgcccaggtttacgtcgcggacatattcccggagcactgaatgttccgtggacggaactggtgcgcgaaggcgaactaaaaacgaccgatgaactggatgcgatattttttggtcgcggcgtcagctacgacaaaccaattatcgtcagctgcggctctggtgtaacggcagccgtggttttgttagcactcgcgacgctggatgtgccaaacgtgaaactgtacgacggcgcatggagtgaatggggcgcgcgggcagatttaccggttgagccagtgaaataagtattttacaggcaataaaaaaccgccgaatttggcggttttttattgctagtctggttcgcggcctttccagcaggttgacttgtgttacatgagcaacgcaggtgcttcacagcaaaacaatactcaccagtaactctctttttgtcaagcaaaagagagtaattattgtttatttagcgtattatcgacaccggccctttccgccgtgttcggtaataaaataacctggcttattagtccgaattcagacaaatataaataaatcctgctcaaaattaaaaattctaaccggtaaaagatattacttaaacatgtaaattcactttcctttaaaaaacaaaaaaccgccaaaatcaggcggttttttgttgctggtccggttcgcggcctttccagcaggttgtattaccgtagtaatgcaagcgcgtctcagcggagacaatactcgccagtaactctctttttgtcaagcaaaagagagttattattgttctgttagtgtattatccactgcggccctttccgccgtctcgcaaacgggcgctggctttaggaaaggatgttccgtggccgtaaatgcaggtgtttcacagcgcttgctatcgcggcaatatcgccagtggtgctgtcgtgatgcggtcttcgcatggaccgcacaatgaagatacggtgcttttgtatcgtacttattgtttctggtgcgctgttaaccgaggtaaataataaccggagtctctccggcgacaatttactggtggttaacaaccttcagagcagcaagtaagcccgaatgccgccctttgggcggcatattttagattatccgattctgtttaaagtcacgcaaaaaaccaccccagcgacgttcatagaatggcgcaatatgttcggtaataaagtggctaattcctttttccccttttttcacctgacaaatatcgattggttcatcgccaggtaatgtatcggtcgctacacttcccgtcgcctgaataatttcttcgatatcaccatcggcttcaatgccaataagtaaattaggctgtgcctcttcgttctctttaattgaacaaataaaagcacgcttcaccggcttaatggttttaaataaggtggtgagtgaatcaatcatttgtgctggcggctctgcgacttccgataatatcagcgattcaccgccttccaggatttcctggctgctcagcggatttccctcttcaccaatcaacaaactgatttcacgcggcataaattctttaccggttggcagtttggcattaaggaagagcgtttcgccaagtgtcatctcaaacagcgtgcgaacgggcattacgacaaatgcctgttcgtcttcaaccgcctgttgaagtgcttctaacgaggtgaaaaaaggaatgacgctggtgccgtcttctttttcccagtgctgtaaatcaagcgcgctatcttcaaccacagcctcgccctgcgccgccgtaccaggcacccagacggtggattccagtagagtacggaaaaaggccgggcggtgcgccggttcagttgctgctttttccagcaggtcttcaagttcgttttttgtttcggacataagaaccacaattcattcaacgttcggggcgcaaatgcctgatgcgctacgcttatcaggcctacaagggattcgcaatttgttgaatttgcagaatttgtaggccggataaggcgtttacgccgcatccggcatattagtttacgccgttaacagattagctatcgtgcgcacaccaagtcccgtagcgcccgcagaccactgttcaaccggcgctttacggtaagtcgccgagcagtcgatatgcagccagccttgctgatagttctcaacaaagtgcgacaggaagcccgccgccgtgctcgcgcctgccggatacgccgcgcttccggtattgttcagttcggcaaagttagacggcagctggctgcggtggaactccgccagcggcagacgccagaacggttcgttctcctgcgcggcactcgccagcaagcgaccggccagcgcatcgtcaaaactgaacagcgcgtgataatcattacccagcgcagttttcgccgccccggtgagggtcgccgcatcaatgatcatttccggtttctgcgcactggcatcaatcagaccatcggcaagcaccagacgcccttcggcatcagtgttcatcacttcaacttttttaccgttgcgataggtgatgatatcgcccagcttgaacgcattgccgctaatcaggttatccgcacagcagaggaacagcttcacgcgcttgttcagtccgcgcgtaatggcaaatgccagcgccccggtaaccgttgccgcgccgcccatgtccgacttcatcgagtccataaacgcagtctgtttgatgctgtagccgccggagtcaaaagtgatacctttacctaccaggcacgcgtacactggcgcttctttatcgccagttgggttgtaatccagcgccagcaataccggagaacgttctgaaccgcgtccgactgtgtgcagccccatataaccttgctcacgcagatcttcgcctttggtgatccgataagtcacacgatcgcccgcgacgttgctgatcagatcaacagcacgctgtgccagttgcgatggtcccaattcttctgccggtgcgttgatggtgtcacgcacccagtcgatgatcatcaggcggttatccagttcctggcgctgggcatcgtccagatccggccacaccactttacgcgtgcctttcggggctttgtaaccttgccagaatgcccagcagcgatccgcatcccagccttcaccgcttaactgaacatgcttgatgcccagaccgtcaatcttgcgcgccgcacgctggatcagccccagatcgtctgccccgttcaaatgcagggtaatgccgtcattattaatgctgtaagttgctttttctccccagcgcgcgtcggcaggttgggtagagagggtaatcttcatcgcttctgtcattttagttatccttctttgtaaaagggccgccagttggcagccccaggatttttccgctaaatgattcgcgttgcaggaaggcggcaagtgagtgaagccccaggagcatagataactatgtgactggggtgaacgagcgcagccaacgcatctgcggcgtgaagcatgacgcggaaattattcggcctcgtccagccagactaacaaaatcgcttcgaggattttctcgttggatgcctgcgggtcgtcgtcgaaatcttccagatcgcaaatccactgatgcatatcggtgaatcgaaccgttttcggatcaagatcgggatacgcatcgtacagtgcttcgccaatttcgcggctatcggtccacttaagtcccatactaacctctgttaatgctcacgcgcatggttgatagtgtaacgcgggatttcgactactaaatcttcgtcggtaacgcgcgcctggcagcttaaacggctttccggctccagtccccaggctttgtccagcatgtcgtcttcctgctctgagctttccggcagtgagtcaaaaccttcacgaacgatgcagtggcaggtggtgcaagcacaggatttttcacaggcgtgttcaatctcgataccgttacgcagagctgcgtcgagaatggtttcaccgctattagcttccagaacagcgccatcagggcagagatcctgatgaggcaaaataacaatctttggcatattaaacctcgtccacggaatggcctttcagcgcacgacgaaccgactggtccatgcggcgagcggcgaaatcctgggtttgtttgtctacgtttttaatcgcttgttcgatggcgtcaacatcatcgccctgcgccacttcactcaggtgagcggcagcatcgtcaatgacctgacgttctgcggcgcttaacagcgcggcatcagcagccagcgcgccgtgcagactttccagcacacgcgccgcttctactttttgttctgccagcattcgggcttttacgtcctgctcggcatagctcattgagtctttgatcatcgaagcgatttcgctatcggtcagaccgtaagacggtttgacctgaatagacgcctcaacgccggtggatttctccatcgccgtcacgctcaaaagaccgtcggcatcgacctggaacgtcacgcgaatatgcgcaccgccagccggtagcgccggaataccacgcagcgcaaaacgcgccagtgagcggcagtcctgcaccagttcgcgctcaccctgcattacatggatagacatcgccgtctgaccatctttaaaggtggtgaaatcctgagcgcgggccaccggaatagtggtattacgcggaatcactttctccaccaggccgcccatcgtttcgaggcccagcgacagtgggatcacatcaagcaacagcatttcgctgtctggcttgttacccaccagaatatccgcctgaatcgccgcgccaatagcgacgactttatccgggtcgatggaagtcagcggtggacgaccgaaaaattcgcctacccgttcacgcaccagcggcacgcgagtagaaccgcccaccatcaccacttccagcacttcatcagcttctacacccgcgtctttcagcgcgcgacgacaagccagtaaggttcgttttaccagtggcgcgatcagttcattgaattgttcacggctgatttcgccctgccagcccgcaacgttaacggtcacggagtccgcatcgctcagcgcgattttggctgcaatggcggcatccagcagttcacgctgaacgcggttatcgctacgatcaggaatgcccgcctgctcgcgaatgtaatccgccagcagatggtcgaaatcatcgccgccgagcgcggaatcaccgccggttgccagcacttcaaacacgccgcgacttaagcgcagaatggaaatatcaaacgtcccgccaccgaggtcataaacggcgatcacgccttcctgaccggaatccagcccgtaggcgatagccgcagcggtcggttcgttaagtaagcgcaggacgtgaaggcccgccagacgcgccgcgtctttggtgccctgacgctgggcatcgtcaaagtacgccggaacggtgataactacaccatccagctcgcctgccagggcttcagttgcccgcgccgccagtgctttgaggatgtccgcagaaacgcgcaccgggttcagcagccccgccgccgtttcaatcatcggcaggccgttttcgctggcctggaattgataaggcagatgcggatagcgttgctggatatcagccagcgagcgtcccatcaggcgtttaacagaactaattgtgttggcggtatcgagcgctgcattagtacgcgcgtcataacccaccgaatgcccttgctgttgatagtgaacaacagatggcagcaggtgacggccttcatgatcggctaacgtttcggcctgaccgctgcgcactgtcgccaccagcgagttggttgtgcccaggtcaataccggccgccagacgacgctgatgcggcgcagcactcaaaccaggttcactaatttgtaataaggccatgtttagcttccagaaattaaaaatcgagcagtttttcttcgagttgttcggcactgcttcgcagtttatcgagaaaacgcagcttacgcacggtatccgccgccgcgtcccacgtctcgttgtctaactgttcaaccatcaactgatggcgggtatcaaacatctttttcacacgtttgataaagctttccagccgcgcttcatctttcgcctgttcgatctcgtccagctcttcgcgcagctccaactgttccatcaggaacgcggtgtcgcgcacagtatgctgctcgctggcgagatcaaagccgtgcaaagaaagcaaatattccgcgcgcattaacggatgacgcagcgtttgccaggcctggttaatggttgcagattgctgtacggcggcgagttgttccgcctggcttccgctggcgaatttatcaggatgatactgacgttgtagatcctgaaaacgcaggctcagcgcctgggtatcgagttgatagcgggcaggcaagccaaagagggtgaagtaatccataacattctcagggctgcgatccgccgcgataacggcgaatcaggtaaaacaaaccccacgcgcaggcgaccacggtggggttatcggtatgcgcatcaaacgtggaagctttcgccgcaaccacactcatctttgacgttcgggttggtgaatttaaacccttcgttcaggccttcttttacgaagtccagctgcgtaccgtccagaaattgcaggctcttgccatcgaccacgactttcacgcctttgtcttcaaacacgatgtcttccggcgtcggttcgtcaacaaattccagtacataagccatacctgaacacccggaggttctcacgcccagacgcaggccaaaccctttaccgcggttagccagaaaggtatttactcgcgctgctgcactgtcgctcagtgtaatcgacataaccaaacctcaactcttattttgcttcacgtttgcttttatagtccgcaatggcggctttgatcgcgtcttctgccagaatagaacagtgaattttcaccggcggcagttcaagttcttcagcaatatcggtgtttttgatcgcctgcgcttcgtcgagagacttccctttcacccattcggtgaccagggagctggaagcgatagcggaaccgcagccgtaagttttaaaacgcgcgtcttcaatgataccttcatcgttgactttaatctgcaacttcatcacgtcgccacaggccggtgcccccaccatgccgctgccgacgttctcgtcgttgttgtcaaaggaacccacgttacgcggattctcgtaatggtcgataactttttcgctgtaagccattataaattctcctgattccgataccgattaatgatgagcccattcgatgctgttcagatccacgccctgcttgtacatttcccacagcggagaaaggtcacgcagacgaccgatggatttacgaactaactcgatggtgtagtcgatctcttcttcagtagtaaaacgacctaaagagaaacggatagagctatgtgccagctcgtcgttcagccccagcgcgcgcagcacgtaggacggttcgaggcttgctgacgtacaggcggaacctgaagaaactgcgaggtctttcagcgccataatcagcgactcaccttcaacgtagttgaagctgacgttgagaatgttcggcgcaccgtgttccaggtcaccgttcaggtaaacttcttcgatatctttgatgccgttccacagacggttacgcaggccgcgcagacgttccatctcggtcgccatctcttcttttgcgatgcgataggcctcgcccattccgacgatctggtgaacaggcagagtgccggaacgcataccgcgctcgtgaccgccgccgtgcatttgcgcttcgatgcgtacgcgcggtttacgacgtacatacagcgcaccgatacctttcgggccatagattttgtgaccggagaaagacatcaggtcaactttcaactggctcaggtcgataggcagtttacccacgctctgggttgcatcaacgtgatagataatgccacgagcacggcacatttcgccgatagccgcgatatcctgcaccacgccgatttcgttatttacgtgcatgatggacacgaggatggtgtcgtcacgcatcgctgcttcaagttctttcaggtcgataatgccgttacgctgcggtgccaggtaggtgacttcaaaaccttcgcgctccagctgacggcaggtatccagtaccgctttgtgttcggttttgctggtgatgatgtgcttgccttttttctgataaaagttggctgcacctttgatcgccaggttgtcagattcggttgcaccagaggtaaagacgatttcacgcggatcagcgccgaccagatcggcaatctgattacgggcgatatctaccgcttcttcagcctgccagccgaaacggtgagaacgggaggccgggttaccaaaggttccgtccatcgtcataaactgcatcattttctcggcaacacgcgggtccaccggcgtggttgcggagtagtcgagataaatcggtaatttcattgctctataaactccgtacatcactcaatgcaaggaatcaggctaccggctggatgtacgaccgtgtttacggagtatttagcactccggcctgattctgaattctttttattaagcgcgtaacttaacgtcgatcgcgtcttgtgtgcgggtgcgtggcgcgtcgtgagtatgctgacgaccagacacatccagcacttcctggttattaaccagttcgcctaaagtaatgttgttgagaaaaccggtgagacggtcgctcaaatcacgccacagcgcgtgggtcaggcatttatcgccgccctggcagccgcctttaccctgacaacgggtggcatctacagattcgtcaacggcgctaattacttcgccaacggcgatgctgctggcatctttgcctaacagataaccaccgcctggtccacgtacgctggaaaccagaccatttttacgcagacgggaaaacagttgttccagataagaaagggaaattccctgacgttcggaaatatcagccaacggtaccgggcccgcttcagagttgagcgcaacgtcaagcattgcggtcacggcatagcgccctttagatgtcagtctcatgtcttacttcacctcaaactcgcccctgcccggggttttttattgtaaaagtgggggtattgcatagcagggtcaagtctgacattcccgagtaaattggtcaactatttacttgactgatttagtcgggtatttaaccttcagtgccatttttttatcgtggcgtttgtacctgttgtcggatgcggcgtgaacgccatatccgccctggggttctgtacactgtaggcctgataagacgcattacgcgtcgcatcaggcaacggctgtcggatgcggcgtgaacgccttatccgacctacggttctgttcactgtaggcctgataagacgcattacgcgtcgcatcaggcaacggctgtcggatgcggcgtgaacgccttatccgacctacggttctgttcactgtaggcctgataagacgcattacgcgtcgcatcaggcaacggctgttattcggccttgttacctttattctgctgctcaatagaagccagaatcccgcgcaggatattcaactcctggctttccgggcgcgcacgggtaaacagacggcgcaatttattcatcacctgccccggatggttttcacggataaaaccggttgccagcagcgtttgttccagatgaccataaaaacgctccagatcatcgaccagcggatacggcgtctcttcatgctcgacctgctcgccgttttcctgagttgccagccaggccatgcgcacttcataggcaataacctgaaccgccatcgccaggttcagcgagctgtattccgggttagccgcaatcgcgacatgataatggcatttctgcaactcttcattggtcaagccgacgcgctcgcgaccaaacaccagcgccaccggggtatttgccgcttcagcgacgcttttcaggccgcattcgcgcgggtcgagcatcggccatggcagcgtgcgggaacgtgcgctggtgcccaccaccaggctacaaccggctaacgcttcgtcgagcgtatcgacgatgtgagcattaccaatcacatcgctggcccctgctgccagggcaatcgcctgggagtcgggtttcaccagtggattaaccagccacagattggttaatcccattgttttcatggcacgggcaacagaacccatattgccggtgtgtgacgtctccaccagcacaattcgaatattttgcagcattgtctttcttcatctaaagattattcacgcatcttatcataaaacgaagacagatgccgatctcgctgctatactctgcgccgttttcccgttctttaacatccagtgagagagaccgatgcatccgatgctgaacatcgccgtgcgcgcagcgcgcaaggcgggtaatttaattgccaaaaactatgaaaccccggacgctgtagaagcgagccagaaaggcagtaacgatttcgtgaccaacgtagataaagctgccgaagcggtgattatcgacacgattcgtaaatcttacccacagcacaccatcatcaccgaagaaagcggtgaacttgaaggtactgatcaggatgttcaatgggttatcgatccactggatggcactaccaactttatcaaacgtctgccgcacttcgcggtatctatcgctgttcgtatcaaaggccgcaccgaagttgctgtggtatacgatcctatgcgtaacgaactgttcaccgccactcgcggtcagggcgcacagctgaacggctaccgactgcgcggcagcaccgctcgcgatctcgacggtactattctggcgaccggcttcccgttcaaagcaaaacagtacgccactacctacatcaacatcgtcggcaaactgttcaacgaatgtgcagacttccgtcgtaccggttctgcggcgctggatctggcttacgtcgctgcgggtcgtgttgacggtttctttgaaatcggtctgcgcccgtgggacttcgccgcaggcgagctgctggttcgtgaagcgggcggcatcgtcagcgacttcaccggtggtcataactacatgctgaccggtaacatcgttgctggtaacccgcgcgttgttaaagccatgctggcgaacatgcgtgacgagttaagcgacgctctgaagcgttaatgactcaggcgggtgatatcactcacccgccctcgcctttcaggcgctattccgaaatacttcctcactgctttactttctttcgtcactctcccaccatctttccccgattaatggatgataaagaagtcgcaaggaaaggttatggcactgccagtgaacaaacgcgttcccaaaattctgtttattctctttgttgttgccttctgcgtttatttagtgccgcgcgttgccatcaacttcttctattatcccgacgataaaatttacggtcccgatccctggtcggcggaatccgtcgaatttacggctaaggacggtactcgtctgcaaggctggtttatcccttcttcgacgggccctgctgacaacgccatcgcaaccatcattcatgctcacggcaatgccggaaatatgtccgcccactggccgctggtcagttggttacccgagcgtaatttcaacgtttttatgtttgattatcgcgggtttggtaaatcaaaaggcacgccgtcccaggccggattgctggacgatacgcaaagtgccatcaatgtggtgcgccatcgcagtgatgtaaacccacaacgtctggtgctgttcgggcagagtattggcggggcgaatattctggatgttattggtcggggtgatcgtgaaggcatacgtgcggtgatcctcgactccacatttgcctcttatgcaaccatcgccaaccaaatgatccccggcagtggctacttacttgatgagagttacagcggcgaaaattatatcgccagcgtcagcccgatcccgcttttactcattcacggtaaagctgatcacgttatcccatggcagcacagcgaaaagttgtatagcctggcaaaagagccaaaacggttgatcctaatcccggatggcgaacacattgatgctttttccgatcgtcacggcgatgtttatcgcgaacagatggtggactttatccttagcgcgttgaatccgcagaactaacccatgatcgctagcacgataatcattcacaaaaccaccttaagacatgctaatccactggtcagaacagtttaagatgagaaaaattctgtgacgcttgccaacatttctgatgattagcattcccttcgccatttccttgagcaaactttagctattcttatcaattatgcttatgggagatctacagatgatgcctacgcttgctccaccatctgtcctttcggctccccagcgccgctgccagatcttgctgacgctctttcagccggggttgaccgccaccatggcaaccttcagcgagcttaatggtgtggatgatgatattgccagtcttgatatcagcgaaacaggacgggagatcctgcgctatcatcaactcacactgacgactggttatgacggtagctaccgggttgaaggtacagtgcttaaccaacgtttgtgtttatttcactggctacgacgtggtttccgtctgtgtccgtcatttattaccagccaattcacccccgccctgaagagtgaactgaagcggcgcggaattgcgcgtaacttttacgacgataccaatctacaagcgttagtgaatctctgctcccgacggctgcaaaaacgctttgaatcgcgcgatattcatttcctgtgtctgtatctgcaatattgtttgctgcagcaccacgctggaattacgcctcagtttaatccgctccaacgtcgctgggcggaatcctgccttgaatttcaggtagcgcaggaaattggacgccactggcagcgtcgggcgctccagcctgtaccacctgatgagccactgtttatggcactacttttttccatgttgcgggttcccgatccattgcgggatgcgcatcagcgggacagacaattgcgtcagtctatcaaacgtctggtaaaccattttcgtgagctgggaaatgttcgtttttatgatgaacaggggttatgtgatcagctttatacccacctcgcccaggcgttaaatcgcagtttgtttgccatcggtattgataataccctgccggaagagttcgccagactgtacccacgcctggtgcgcaccacccgcgcggcgctggccggatttgaaagtgaatacggcgtccatctttctgatgaggaaagtggtctggtcgcggtgattttcggtgcctggctaatgcaggaaaacgatctgcatgaaaaacagattattcttcttaccgggaatgatagcgagcgagaagcgcagattgagcagcagttacgcgaactaacgttactgccgctcaacattaagcatatgtcggtaaaggcatttttgcagacaggcgctccgcgtggcgcggcactgattattgcgccttataccatgccattaccgctcttttcaccaccgctgatctatacggacctgacgctgacaacacatcaacaggagcagatccgcaaaatgctcgaatcagcatgagggaacaactttcgggcgcaaaaacattgccggaagcgccaccagcgccattacccagaacacgccgtggcccagatattgatacaggaaaccggcgaaaacggtcatgatagcgatactgccgcccatcgcgacggcagagtaaaccgcctgtaaacggatgacttcgctaccctggcgagcagcaatataacgcatggcggccaggtggcagaccgtgaaggtgccgcaatgcagaatttgcaccactatcaaccacggcaacgccgtagttgctcccataatgccccagcgcactacgccgcaaatcgccgagatcaacagcatatcgcgtgcactacaacggcggaaaagtttattactcagcgcaaagataatgacttccgccaccacgcccagcgaccacaaataccccaccgccgaggccgagtagccagctgcctgccagtaaatggcgctaaaaccgtaataggccgcatgtgccccctgcaataaacaaacgcaggccagaaagcgccagttctggcgaaccagcgccaaccacgcagaccaaccggtgctctcctgctggcgacttgccccttgtggctgaatcgtcggacggatgagaaagccgagcagcatggatgccacgcccaacgtcaacagcgcgaggatcacccgataatcaaacatagtgaccagtttgcccgtcagcgccgagccaatgacaaacgccaccgagccccacagtcgcactttgccgtaatcaagcgggaactgcttttgccacgtattcgccagtgcatcggtcaacggtaccagtggtgagaaaaagaggttaaagccaatcatcaccagcatcagccacgctacgtgcgcccccgcccagaaggcgacagcaaagagaagtgtcagcagtgccagcacgcgcaaggcggaaatcaggcgggaaggatcgctgacgcggggcgcgatgagcaaactcccgaggaaacgggcaaccagacctgcccccaataacaggccgatggtttctggcgttaaaccaatccctttaagccagacgctccagaaaggtagaaaaatgccgtaactaaaaaagtatgtgaaatagccgagcgccaaccagcgcgtggattgcaaaaccatgagtccctcccgtcaggaggcgttagtctggggttaatcgaatgttggtgcaagttgaaaaataagaatattcgagcctgcttcccgatgtctgtaacgccagttcacaagcactaaaaaactgagatccgcgacgcatgttgcaaaaataatgcgtaattatgccgttacgcttgccaaacgttcctgcacaatggcgatgaaatcgcgtaatgccggcttcatctcccctttcttccacgccatcagtaaagcaatggaaggcacatttccggcaatgggacgaaaaacaacctgtccggtattaaaattattcatataaccgggtatcaaagtgacgcccagccccatgcccaccagattcatggtcaccagaatattcgttgccacctggacgatatttggctggctgttttcttgcgcaaaccacgctttaacgatcggcgcaagcgaaccggaatacaccggatcggtactgacgaaattcacgccatccagttgcgcggcggtgatctctttttcatgtgctaaagggtgatcaaccggtaacacaaccactaatggttcgtcaaaaagctccagataatcaatctccgggctataaacaggatggcgcattaagccgacgtcgagttcaccacggcgaattttttcctcctgttgcgtggtgattaaactcaccagctcaatcaaggtgtctggctgtctgagacgaaacatcggtaatacttttggcagtaaattcacttccgccgatggcacaaagccaatggttaattgtctgtcttcctgaacaattttccgcgcccgtaatttggcattttccgcttgttcgaggattgccagcgcgtcctggagaaaacattctcccgccgccgtcaacgcgactttgcgcttatccctcaccagtaacggaacaccgacacagttttcaagatcgcggatctggctgcttaacgaaggctgtgaggtatgcagtttttccgccgcacgggtaaagttcagtgcctgcgccactgcgacgaaatagcgtaaatgccgtagttccatcaccttccccttgttatcgaaaaaacgtctcagctggtagaaattaactatttcacatattagcaaccaaccagcaacatccttatggcacaaaaatagaaggtcaatacatcttatctttcaggattaaaaaatatgaccacaccctcagatttgaacatttaccaactgattgacacccaaaatggtcgggtcactccgcgtatttataccgacccggatatttaccaactggagcttgagcgtattttcggtcgttgctggctatttctcgcccacgaaagccagatcccaaaacccggtgatttctttaacacctacatgggagaagatgcggttgtcgtagtgcgtcagaaagacggcagcatcaaggcgtttctcaaccaatgccgccaccgggccatgcgtgtgagttatgcagattgcggcaacactcgcgcctttacctgcccgtatcacggctggtcttatggcattaacggcgagttgatcgatgtaccgctggaacctcgcgcctacccacaagggttgtgtaaatcccactggggactaaacgaagttccttgtgtggagagttataaagggctaatttttggcaactgggataccagcgcaccgggcctgcgtgattacctgggtgacattgcctggtatctggatggcatgctggatcgtcgcgaaggcggcaccgaaattgtcggcggcgtacaaaagtgggtgatcaactgtaactggaaattcccggcagagcagttcgccagtgaccagtatcatgctctgttcagccatgcttctgccgttcaggtattaggggcgaaagatgatggcagcgataagcgcctcggtgatggacaaaccgcccgcccggtgtgggaaaccgccaaagatgcgctgcaatttggtcaggacggtcacggtagcggtttcttctttactgaaaaaccggatgctaatgtctgggtcgatggcgcagtttcaagctattaccgcgaaacctatgccgaagcagaacaacgtttaggtgaagttcgcgccctgcgcctggcgggtcataacaatattttccccacgctttcatggctaaacggcactgccacactccgcgtctggcatccgcgcggccctgatcaagttgaagtgtgggcgttctgtattactgacaaagccgcctccgatgaagttaaagccgcttttgaaaacagcgccactcgtgcttttggtcctgctggttttctcgagcaggatgactcggagaactggtgtgaaatccagaaattgcttaaaggccaccgcgcccgcaacagcaaactgtgtctggaaatggggcttggtcaggaaaagcgccgcgacgacggcattcctggcattactaactatatcttttcagaaactgccgctcgtggaatgtaccaacgctgggccgatcttctgagtagcgaaagctggcaggaagtgctcgataaaaccgccgcttaccagcaggaggtgatgaaatgagtgcgcaagtttcactagagttacatcaccgcattagccagtttctctttcacgaagccagcttactggacgactggaaatttcgtgactggctggcgcagctcgacgaagagattcgttacaccatgcgcaccacagttaacgcgcaaacacgcgaccgccgcaaaggcgtccagccaccgacaacctggatttttaatgacaccaaagaccagctggagcggcgaatcgcccgtctggaaacgggcatggcctgggcagaagagccgccgtcacgcacccgtcacttaatcagcaactgccagataagcgaaaccgacatcccaaacgtatttgctgtgcgggtaaattatctgctttatcgggcacaaaaagagcgcgatgaaacattctatgttggaacgcgtttcgacaaagttcgccgtctggaagatgacaactggcgcttgctggaacgggatatcgtcctggatcaagcggtaatcacttcccataacctgagtgtactgttctgatgaatcgaatttatgcgtgtcccgttgcggatgtgccggagggtgaggctctccggatcgatacctcgcccgtcatcgccctgttcaacgttggcggcgagttttatgccattaacgatcgttgcagccatggtaatgcgtcaatgtcagaagggtatctggaagatgacgccacggtggagtgcccgctacacgccgccagtttttgcctgaaaacggggaaagcgttatgcctgcccgccaccgatccgctcaccacttatccagtacacgttgaaggtggtgacattttcatcgacttaccggaggcgcagccatgagcgatctgcataacgagtccatttttattaccggcggcggatcgggattagggctggcgctggtcgagcgatttatcgaagaaggcgcgcaggttgccacgctggaactgtcggcggcaaaagtcgccagtctgcgtcagcgatttggcgaacatattctggcggtggaaggtaacgtgacctgttatgccgattatcaacgcgcggtcgatcagatcctgactcgttccggcaagctggattgttttatcggcaatgcaggcatctgggatcacaatgcctcactggttaatactcccgcagagacgctcgaaaccggcttccacgagctgtttaacgtcaatgttctcggttacctgctgggcgcaaaagcctgcgctccggcgttaatcgccagtgaaggcagcatgattttcacactgtcaaatgccgcctggtatcctggcggcggtggcccgctgtacaccgccagtaaacatgccgcaaccggacttattcgccaactggcttatgaactggcaccgaaagtgcgggtgaatggcgtcggcccgtgtggtatggccagcgacctgcgcggcccacaggcgctcgggcaaagtgaaacctcgataatgcagtctctgacgccggagaaaattgccgccattttaccgctgcaatttttcccgcaaccggcggattttacggggccgtatgtgatgttgacatcgcggcgcaataatcgcgcattaagcggtgtgatgatcaacgctgatgcgggtttagcgattcgcggcattcgccacgtagcggctgggctggatctttaaggaagcacgatgaaagaaaaaacgatcattattgtcggtggcgggcaagcggcggcaatggctgcggcctcgctacgccagcaagggttcaccggtgagctgcatctgttttccgatgagcgacatcttccttatgaacgacctccactctcgaaatccatgttgctggaagattccccgcagttacagcaggtgttacccgctaactggtggcaggaaaacaatgttcatctgcattccggtgtaaccatcaaaacgctgggtcgcgacacacgagagttagtgttaaccaacggcgaaagctggcactgggatcagctttttatagcaaccggcgcggcagctcgaccgctgccgttgcttgatgcactgggagaacgctgctttaccctacgccatgccggtgatgccgccagactgcgagaagttctgcagcccgaacggtcagtcgtgattatcggtgccggaactattggtctggaactggctgccagcgccacgcagcgcagatgtaaggtgacagtgattgaactggcggcaaccgtcatgggccgtaatgcaccaccgcccgtgcaacgctatcttttacagcgccaccagcaggctggtgtgcgcattctgctcaataatgccattgaacatgtggtcgatggtgaaaaagtagaactgacgctgcaaagtggggaaacgcttcaggctgatgtggtgatttacggtattggtatcagcgccaacgagcaactggctcgcgaggccaaccttgatactgccaatggcattgtcattgatgaggcttgccgcacctgcgatcccgcgatctttgccggtggcgatgtggcaatcactcgtcttgataatggtgcactacaccgctgcgaaagctgggaaaacgccaataaccaggcgcaaattgccgctgccgcaatgttagggctaccgctaccgctactgccgccgccgtggttctggagcgatcagtacagtgataacttacagtttattggcgatatgcgtggcgatgactggctttgtcgtggcaacccggaaactcagaaggcgatttggtttaatctgcaaaacggcgtgcttatcggtgcggtcacgctgaatcaggggcgtgagattcgcccaattcgcaaatggatccagagcggcaaaacgtttgatgcgaaactgctgatagatgagaacatcgcgcttaaatcactgtaaccaggataattagcgaatatctcaatgcctggggcgtggcgaggtgcaagagtgtgtattacgtttaaatcacattatcttgcaaagggattggttatgaacacactacgttattttgattttggagctgcccgccccgttttgttattaattgcccgtatcgccgtggtcttaattttcattatttttggttttcccaaaatgatgggctttgacggtacggtccaatatatggcctcgttgggcgcgccaatgccgatgctggcagcgattattgcggtagttatggaagtgcccgccgcgatattaatcgtgcttggctttttcacccgtccgctggcggtgctgtttattttctacacgctgggtacggcggtgattggtcaccattactgggatatgaccggcgatgcggttgggccaaatatgattaatttctggaagaatgtcagtatcgctggcgcgttcttgctattggcaattaccgggccgggggcaatttctctcgatcggcgttaggaaagatgccggatgcggcgtgaacgccttatccggcatttaataaattacagccactctacccgcaacgacatctctgaagttgttgattcccctggtgctagcgcaatgagatcacccccttccgggcgatgatgatcatccggcgcatggctcatcggttccagacagaagaaatcaaacgcatatcctttatcaaacgcagggtcggaaacaaagatgaaataacacggtgcaggtggcgtcgtttccatgatgatggcataaccttcctgcggctgctcgatgcgggcctgaccattccatccggcaaaaccattgttcacccactggcgcggcaacggcgcgggctggttaaaatccagttcctgcggtagctgctcgcaaaactcacccgccagccactgctcccgctccagccagtaaccgctcgcctgtgcctgaatccgcgtttgcggcgacaacggaaaataaggatgccagccggtaccaaatggcagcgtctctgccccttgattggtgacagagagcgtcaccgtcagcgtatccgccgttaaatgaaacgcctgacttacccgatagtgatagacaccgctgcgatgttcatacaccagacacaaactatcatcgctgtgcgagacacattgccactcgcccagccagccatcgccgtgtagatagtgcgcatcccactcaacattcggttgcagttgatactcacgcccctgccagacaaaacgattgccgctcacccggtttgcaaatggcaccagcggaaaacatgaggcatcggttgccacaccgctttttttaccaggacgtaagagcggcgtcgtatcgcgccagaagccttcgattacgccgccctggtcagaaacgtccagctttagcgacccgtgggataaggtatagatggtcatccgctaactccttaatccgggaagttaatcacaactttcccgcatttgccgctcgccatcagcgcataggcatcacctgcctgttccagcgagaagcgatgggtaatggcgttacgcggccacagcttccagtccgtcagatcatgggcgcatttttccatatggaacagactggtcacccaggagccgataatccgccgttgatggtgcatcagatcggcgctgacctcgaattccacttttccggtttcaccaatgtaaaccacccgtccccagtcagcggtggattgcagtgccagcaagcgacctgcggcattaccggaacaatcgagcgcaacatccgcgccaccgtgggtgagttcggcgataatctgcggcagaccttcggtggttgctaaatagccgtgatccatcacccctaactgttttgccatcgccagacgttccggcagcatatcaacgccgatgatccgttttgcaccgcgacctttcgccagcatcatcgccatcatgccgactggccccagaccgaccaccagcacgttatcactgccggaaacttcgccgcgcaaaattccttcatacgctgtaccaacgccgcaactgataaacgcaccatcttcgtagctcagcgcatccggcaggaggatcagatctttttcttccgccagcaagtattcggcatgaccgccgtcacgctgccagccgtaagccgcttttccttcgccagtacaagaaataggaaaaccgcgacggcagttcgggcaaaaaccacagccagaaatgtgatacaccagcacgcggtcgccctctttaaaatggcggcagccttgccccatcgccacaatctgcccgcacggttcatgaccgttgataaagccctggtataacggtttatcgggtgccgccgctgtggcacggtgttgatgatagatatagtggacatcgcttccgcaaatcccggaggatttcattttgatcagtacctggttaatccccggcgtcggcaccgcaacttcccgcagatcgacggtcgaatttcctggtaaataagctgccagcatcgttttcataaatccctcattaacaatacgattaattttcatccctgccgcacccgcgccaggggcgttaaggtttagcgtttcgctttactgcttcgctgggtcagcaagatattcgccagcaccgccaccacgatgatgacgccgcgtaccacctgctggaaaaaggagttaataccgagcagcaccagaccgttaccgattagcgtaatcaccagcacaccaagcaatgtaccgaacagggaaccgcgaccgccggaaagtgccgtaccgccgaccacgaccgcggcgatgacgtcaaactccagaccgtttgcggcacctgcgttaccagaaccgaggcgcgccgccaacaaaatgccggtcaccgccgctaataatcccgaaagggtaaagataagaatgcgcacccgacgaacgttgatgccgcacaactgcgccgccgtagcattaccgccaacggcaaaaaccgagcgcccgaaggcggttttgcggctgatgaacacaaacagcgcaaacaacacaatcatgatcagcgcggataccggcacaccgagaaattgtccgcccagccagtccagcacctcgttttcatcaatcggcactggcagtgcgttcgtcataaacagccccattccgcgcagggcgctccacagccccagtgtggcaacgaaacttggtacattaaacacgccgcgcagcaccccggccagcgttcccatcagcgcgcctaacagcaacaccagcaggcacgccaccgccagcggaacttcaaattgcagcaaaaatgccaggcacaccgagacaaaagccaccatcggcccaacgctgacatcaatttcaccggagataataatcagcgtcatcgcccaggcggcaatcccaatggtggcggcatcgcgcagcacgttcatctggttattcaatgagataaagccaggcgcgttcagggagaagaccagataaagaatggcaatcaccaccagcaaaccgatctcattaatatggcgactgacaaattgtttgagcgagacgctcttgccctgcggcaatggtaatgacgaagcagacatcttcaggttcctcggtaaaattcatcagtgcacagacagaatggcggacatcagctcatccacattgaccggagcgtgaaactcctgcgagaacgtgccgtgctgtaataacaggatgcggtcacacaccagcggcaactcctccacttcactggagataaacaccacgctttttccttcggcagccagctcacggacaatacggtaaatctgctgtttggcttcgatatcgacgccgcgcgttggctcgtcgagcaacaaaatctggctggcagcatagacccaacgaccgatcaccactttttgctgattgccaccagaaagcgtgccgatgggtgtttcgctactggcggccttgaccgtcatccgctgcatcacctcttcggtcaggcggcggatggtggaccattgcagcacaccgttggcgctgattttttgccgattggtcagcactgtattttcgtcaacgcccaaccagggaatgatccccgcttctttgcggttttctggcgtatagccaatgccgcgtttcagcatgtcgccgtaatcggggcgcgtgattttctcgccgttgataacaatttcgccctgttcatactcctccagcccaacaatcgccttcagcaattcactgcgccctgcccccagcagaccagcaatgccgagcacttcgccacgacgtagcgtaaaactgatatcctccagcttgggcttatggcgtaacgcacggacttccagcacggcctgatccacaatttcctgaggggctaccggcgcaatatcaacgtgatcgcgcccgagcatcagcgacacaatatgatgcgtggaggtgttttcgagcatcacatcgcccgccacctgaccatcgcgcataacggtggcacaggaggcaatgcggcgaatttcttccatccggtggctgacataaatcaccgccacgcccagtgccgacatctttttcaccgcgctgatcaccagttcaacttccgcactcgcaagcgaactggtaggttcatcaagaatgaccacgcgcggctcgcccttcatcacccgcgcaatttccaccagctgcttttgcgccgggcttagcgttgaaacaagttgttcaggactaacgtcaacgcccagcgcctgtaagcaacgttgggcatcctgcgccatttgcaggtaatcaatcatgccgttgcggcggggccactgaccgaggcagaggttttccgccactgtcagcccttccaccagacttaactcctgataaaccgcgcgcacccccagttcagcggcacggcgagtcagcgtagcttcgtcaccttccagtcgcgtctcgccaatccagatatcaccgctatccgggcgttcgctgccggtaagcattcgaatgagagtcgatttgcccgcgccgtttttacctaacagcgcacgaacttcgcctttattgagcgtgaagttaacgttatccagcgcaacgacgccgggataacgcttatttcctgccaccacttttgctaccgggactgcctctgttgccgtgaacatagggacctctgcgaatcagcgattagggcagaccatcaacgtgcgttgccagccactgtttaccgtcttccgttttggtatagagatcgataggcacctgaatcactttttcaccgtcggcttgtttattgataaccttcaatgtttgcgcgaaaacagcattgcccattttcttaccggaaatatccactaccgctttcagcacctgattgttttccagctcctgagcaatttcggttgtcatatccgaaccgaaaacagcaatttttccggcctgattttgattacgtaccgcttttaccgcgccgagtgtcgcaccgcccgattcccccataatggcgttgagatccggcgtggagataattagtttttcaccaacggaaatcgctttatctaaaacagtcccttcctgattagcgacaatttgcgcgccgggaacgcgggattttaaaacttcttcaaatcctttacgtcgctgcacacaaacttcaaaggcttcgcaattgatgacggcaattttcggctggtcaattttattggcaataaaataatcagcggcagcgttacccagttttttaccaaattccagcggatcgccgaccagatacgccgagacatatttatcgacccccttttgattaatacaggtgttgtagcaaatcaccggaatgcccgcttcactggcgcgacgaacggtacggctactgccattttcagacactgccgataaaataatggcatcgacattacgcgccacgagggtatcaacaaaggtactttctttcgaaatatcaccctgggcgttagtttctattaactgaacttgtactgaggaatcttttgccgcatcctgaacgccctgacgcactccagcgtagtatccctgagtatcaaggtatattgcgccaatggtcatttctttttccgcagccctggcaaatagtgcgctacctaatagcgtagccattaataatagattacgggttgttctcatttttgtaggcatagagcctcctgtagggtttttattaacaacggcttattctaattattttgtgatgagcggcagcgcgtgccgctcaaatattacagttaatagggtttagtgaacgcggttaaaaataaaaggcatcacggtggtgaataatgccgctttcggccaagccggattaatcgccgtcaattcagcgcgagcagactcatattgcgcaacctccccgagtcccgcggacgccagcatcgccaccatcaggcatttttctttatgctgctgttgtaaatcgccatacagcgacaacaagtcaggttgcgagacggcaaagaaatccgcttcgatactggttttcgccatctcttgcgcccactgtttcatttcactaaacagttgctgtgcggtttgttgttcgcccagcagtcgcagcgccatcccttgccagaagagataatcaaccggctgatcgttgtaataactgtgaatgttaatagtgcgatcgccggtcgccgccagacgtaaacaacgcgtcgcttcagtttcatcgccctgcgcgttggcgcatatcgcctgccagaaccagatgtcgttatcagtttgccccggtaaacggccttcgcttaaattctccggataatgcagcgcggcatgaagcagttcgcaggcctgctgcggctgtctggcatcaagatgctgccaggcgcgtaataactggttgaggataaactgactggtgaccttcccttccccgccttcccacgggtggaatttgcgcgtggcgagaatgtccgccgctttgtctgcctgacccgtgagatgccacaaattgagcagttctgcggtcatgtcgtcgcgtttcagcgcaatttccagattattttccagacgcgccagtcgtttctccggtgtggctccacttaacttatccagcaaatcccgttcgaaaagcagacgtgcatcctgcggcgcaagctgataagcattatcaagataacgcgcggccagctcataatcgtgttgcttattccacgcatggatcgctaacccgcgccagccgtcggcaaactccggcgacatctctacgcaacgttgccaaaaggcaatggctttgttgtagctacgtttgttgtagtagaagcaagctagtaaatggcgagcaaaccagcactcttcaatactctccagcgccgccacttcttccagcgtattcgggaaacggacaaactgcgggaagacatcaatggcttttgcgaccagttcgccacgttcggctttcggcagcaagctggcttgcaggtaaagcggcagcgtgcgctggcagtccagtgcgttcagcatctctgccgccagggtgggcattccccagttaatcagttgcccggcggtcatcagggcgttaacgtcgcgtccctgacacagaccgcgccactgcgcgagagctgattcgctacgaccatcgaaccagttcagccaccacagagtggcgttcagcggataatcgcgcagcagtttctcgcgctgcacacgcgcgttgtcctgacgaccacttaacaccagcagcagattatgcaggcaaagcacttcctgattggttgggcaggcgcgaagactttgttggcaaaaatccagaccagcgtcgaagttaccattacgcgccgccagtcgtgccaggccataatagccaccggctttgctgttgccgctccagaccgcacgccagaaatcctcttcggcttgttgatattgtccctgacgttcgtaagcactggcgcgaatcaaactcgcctgtccgcactgcggatttttgttcagcgcatgtgcgcgtttcagagcctgagtggcatacgccaccgcttgcgggaaatctgcgcggttatattccagcatcgccagcgccaggttacagcgataatccagcgggtccagcgccacgccgcgcaggtagtaatcgaacggtgaacggctggcgtgatgatattgctccagatgctgaccgataaaccaggcttcatctgtactggtaatgtcttgtgctgccagtggcgctttggcgacgtccggtaacggcaacgcttgcggctgatgttcctgataactcagtacaatattgccgtcggcatcggagagctcaatggtcagcctttcaggattgataccgtgcaacacgccctggatggcggtcgcaggcatcagtgccacggcatcatcaagtaacgcgttgcatttaccgatttcgcggatcgccaggcggtatccgttcaacggagagatggcatacagcccccactcaatcccccgcttactacgctggagttttatcaccgcatcgcgggaggcattttgcaccatgcccaaagaatgataaggcaggaaatactgctcaaaacgcttctcttcgtaagcatcaagccaggtaaaatcgggctggttatcggcaaaaataccggtcatcagttcgatatacgggccgttattgtcggtcagactcttatcccacgcctggccaaattcactgtgtccccaactccactgttttttacctggcgcaatatggtggttggcaacgtgcagcaaaccgccatcttcatcgtgacaccacgcgccgacaaaatcgtactgcgatttttcggccatatatgaggttggaacaggcacatttttatagcgagaaatgtccactccagcggagtagtccactttgtagtaagtgccggtagcgatggggaaagcggagacggcccgtttgccgtgatcaaacaccgccgttacatccggcgggaagacgctctgatgcccttccccccctttcactgccgggttggcccaccacaagaaatgacgcggcgtggcgttcccgttatagacgcggctggcgatttccagcgccgcccggtcagggcgcagggtgaaacctgtcatcacctgtaaaccatgcatcggctccgtttcgcctacccacaccgtctgtgcaccgtcttcatgggcttcgagggtgaaatcaacgggcataaaggtggtcgggcgatgatgttgcggccagttaaactcaatcccaccggaaatccacggccccagcagccccaccagcgcaggtttaatgacttcattgtgataaacaaaatcgcgctgtttcactttatcccacgcgcgatgcacccgaccgcccagttccggcaggatcatcactttgatgtagtcgttttccagccacaccgcctgccaggatttcagggttttctgctcgctcagcgtatcggtcacgccgtagggataaaccgcgccggacgatccctgataaacgcgattttccaggaacatgggatgtatatcctgcggcccggtttcataggtcgggatctcaacgcgctcttgccacacttttactggagtcatggtgccctcaatattaacaagacatactgaattaaaagatttgtggcagtgtattgaacaatctggcaatgttttcgcggaataatcacgcaattaactaaacaaggtttagtgaagatgagagcctgcattaataatcaacagattcgccaccataacaaatgcgtgattctggaactgctgtaccggcaaaagcgcgccaataaatcaacgctggcccggctggcgcaaatttcgattccggcagtcagtaatattttgcaggaactggaaagcgaaaaacgggtggtgaatattgacgatgaaagccagacgcgcgggcatagtagcggtacatggctgattgcgccggaaggtgactggacgctgtgcctgaacgtgacgcccaccagtattgagtgtcaggttgctaatgcttgtttaagtccgaaaggtgaatttgagtatttacagattgatgcaccgacgccgcaggcgctgctgtccgaaatcgaaaaatgctggcatcgccaccgtaaattgtggccggaccataccatcaacctggcgttggcaatccacggtcaggttgatcctgtgaccggcgtgtcgcaaaccatgccgcaagcgccgtggacaacgccggtggaggtgaaatatctgctggaagagaagctcggcattcgggtgatggtcgataatgactgcgtgatgctggcgctggcggagaaatggcaaaataattcgcaggaacgggatttctgcgtgatcaacgttgattacggcattggctcgtcgttcgtgattaacgagcaaatttatcgcggcagtttgtatggtagcggacagattggtcacaccatcgttaatccggatggcgtcgtctgcgactgtggacgttatggctgcctggaaactgtcgcctcgttaagcgcattaaaaaaacaggcgcgggtatggctaaaatcacaaccggttagtactcaacttgatcctgaaaaactgactacagcgcagttaatcgctgcctggcaaagtggagaaccgtggatcaccagctgggttgatcgctctgccaatgccattggtttgagtctgtataacttcctcaacatcctcaatattaatcagatttggttgtacggtcgcagttgtgcctttggtgagaactggcttaatactattattcgccagacaggatttaacccgttcgaccgcgacgaaggaccgagcgtgaaagcgacgcaaattggctttgggcaattaagccgcgcacaacaggtgctgggaattggctatttgtatgttgaggcgcagttacgacagatttgatggcgcgataacgtagaaaggcttcccgaaggaagccttgatgatcataaacgaaaaattgcctgatgcgctacgcttatcaggcctacacggagattgcaatatattgaatttgcaaagttttgtaggccggataaggcgttcacgccgcatccggcatgaacaacgagcacattgacagcaaatcaccgtttcgcttatgcgtaaaccgggtaacgtgcgcagatgtcgagaactttacctttgatgcgctcgataacggcttcatcattgatgctgtccagcacgtcacacatccagccagccagttctttcgcttcggcttctttaaagccgcgacgggtaatcgccggagtacctacacgaataccggaggtcacaaacgggctcttcggatcgttcggtacgctgtttttgttgacggtgatgttagcacggcccagagcggcgtctgcttctttaccggtcaggtttttatcaaccagatcaaccaggaacaggtggttatcagtgccgccggaaaccactttgtagccgcgctcgaggaacacttctaccatcgctttagcgtttttagcgacctgctgctggtaagttttgaactcaggctccatcgcttctttcagagcaaccgctttaccggcgattacgtgcatcaacggaccgccctgaccaccagggaaaacggcagagttcagttttttgtacagctcttcgctaccacctttcgccaggatcaggccgccgcgcggacccgccagggttttgtgagtggtggtagtaacaacgtgagcatgaggaaccgggttcgggtagacgccagcagcaaccaggcccgcaacgtgcgccatatcaacgaacaggtaagcaccgatgctgtcagcgatttcacgcattttcgcccagtccaccacgccggaatatgcagagaaaccaccgataatcattttcggcttgtgttctttggcttgtttttccagatcggcgtagtcgatatgaccggtagcatcgataccgtaaggaacgatgttgtacagtttaccggagaagttaaccggagaaccgtgagtcaggtgaccgccatgcgccaggttcatacccagaacggtatcacctggttccagcagcgcggtgtagaccgcaaagttagcctgggagccggagtgcggctggacgttagcgtagtcagcgccgaacagttctttcgcacgatcgatcgccagttgttcaacgatatcaacatactcgcaaccgccgtagtagcgtttgcccggataaccttcagcatatttgttggtcagctgagaaccctgcgcctgcattacgcgcgggctggtgtagttttcggaggcgatcagttcgatgtgctcttcctgacgtactttttcctgctccatagcctgccacagttcggcatcataatcggcaatgttcatttcacgctttaacatccgcatctcctgactcagctaacaataaaatttttggcctttataggcggtcctgttggacaacggcgaacagtataaccgaatcattgtgcgataacaggtcttgacaaaggaatttacgcaaacgattaccttcaggctacgcaaggctttggagaataaagagcttgcaaccggaaacggatttcttttcaggtttgtgatgcaaatttttcacttcatcacattctttctgaaaaacaccaaagaaccatttacattgcagggctattttttataagatgcatttgagatacatcaattaagatgcaaaaaaaggaagaccatatgcttgacgctcaaaccatcgctacagtaaaagccaccatccctttactggtggaaacggggccaaagttaaccgcccatttctacgaccgtatgtttactcataacccagaactcaaagaaatttttaacatgagtaaccagcgtaatggcgatcaacgtgaagccctgtttaacgctattgccgcctacgccagtaatattgaaaacctgcctgcgctgctgccagcggtagaaaaaatcgcgcagaagcacaccagcttccagatcaaaccggaacagtacaacatcgtcggtgaacacctgttggcaacgctggacgaaatgttcagcccggggcaggaagtgctggacgcgtggggtaaagcctatggtgtactggctaatgtatttatcaatcgcgaggcggaaatctataacgaaaacgccagcaaagccggtggttgggaaggtactcgcgatttccgcattgtggctaaaacaccgcgcagcgcgcttatcaccagcttcgaactggagccggtcgacggtggcgcagtggcagaataccgtccggggcaatatctcggcgtctggctgaagccggaaggtttcccacatcaggaaattcgtcagtactctttgactcgcaaaccggatggcaaaggctatcgtattgcggtgaaacgcgaagagggtgggcaggtatccaactggttgcacaatcacgccaatgttggcgatgtcgtgaaactggtcgctccggcaggtgatttctttatggctgtcgcagatgacacaccagtgacgttaatctctgccggtgttggtcaaacgccaatgctggcaatgctcgacacgctggcaaaagcaggccacacagcacaagtgaactggttccatgcggcagaaaatggcgatgttcacgcctttgccgatgaagttaaggaactggggcagtcactgccgcgctttaccgcgcacacctggtatcgtcagccgagcgaagccgatcgcgctaaaggtcagtttgatagcgaaggtctgatggatttgagcaaactggaaggtgcgttcagcgatccgacaatgcagttctatctctgcggcccggttggcttcatgcagtttaccgcgaaacagttagtggatctgggcgtgaagcaggaaaacattcattacgaatgctttggcccgcataaggtgctgtaatttgatgttgccggatggaaacatccggcaacccttgacgcggtttaaattgccgcgtcgtcctcttcaccggtacggatgcgaatgacccgtgccacgtcaaagacgaagattttaccgtcaccgattttgccggtttgcgccgtgcgaataatggtatcgacacaggtatcgacaatgtcgtccggtacgacaatctcaattttcactttcggcagaaaatccaccatatactccgcgccgcggtacagctcggtatggcctttctggcgaccaaagcctttcacttcggtcaccgtcatgccggtaataccgacttcggccagtgcttcgcggacatcgtccagcttgaagggttttataatcgcatcaatctttttcatgctattccttgaaaaggtcgcctgtcttttgatctgctaaacgtaacacataacgccaattcattccttgaaatcgtttgcatccagctcgtgtcgggaaagcagtttataaaattctgtccggttgcgccccgccattctcgccgcgtgggtgacgttgcctttggtgatttgcagcagcttacgcaaatagttgagttcaaactgattacgtgcctcaacaaaggttggcagcgccgtattttcaccctccagcgcctgctccaccagcgcatcactaatcaccggagatgaggtcagcgccacgcactgttcaatcacgttgaccaactggcgcacattacccggccagctcgcggtcatcaggcgtttcatcgcatcggtagagaacgcgcggacaaacggtttatgtcgctctgccgcctggcgcaacaggtgatttgccagtagcggaatgtcttctgtgcgctccgccagtgccggaattttcaggctgacaacgttgaggcggtaatagagatcttcgcggaattccccgcgcgccatcgcttttggcagatcacggtgagtggcagaaataatccgcacattgatatcaatatcgcggttactgcccagcgggcgcactttacgctcctgcaacacgcgcagcagtttgacctgtaacggcgcaggcatatcgccaatttcatcgagaaatagcgttccgccttccgccgcctggaataaaccttcgcgattgctgacagcgccagtaaacgcgccacgcgcatgaccaaacagctccgactccagcaattgctcgggcaatgcgccacagttaatagcaataaatggtttgctgttgcgcgggctggcgttgtggatagcctgggcgaaaatctctttcccggtgccgctctgaccgttaatcaaaacgctgacgtctgattgcgccaccagccgcgcctgttccagcaaacgcagcatcagcgggctgcgggtgacaattgcctcgcgccagcgttcatcggtggctggcgcggattgctccagcgcatcgtcaattgcctgatatagcgcgtctttgtcgacaggcttggtgaggaaactaaaaacgccctgctgtgttgcagcaacggcatcgggaatagaaccatgcgcggtaagaataattaccggcattcccggctgcactttctggatttcagcaaacagctgcataccgtccatttcatccatccgcaggtcgctgatgactaaatctactttttcgcgattcagtacccgtaatccttcagcgccactttccgccgtgaccacactgtagccttcgctggtcaggcgcaggccaagcagtttcagcaatcccggatcgtcatcgaccaataataaatgcgcaggtttatggctcatcaggagtgacctcatgggtggatggcgcgggcttttcactctcgtgcggcgtatccggcgagaaatttccagccggtttgcgggtcgagagctggcgttcaatatcggtcaggttttccagcttgcgggtggtgagttccagttgctgctgtagaacgtgatgttgctggcgcaatgtatccagctcgctgtcgctggactgctggagtttactgtaacgttggcgctcttccgccagttgcagttgcagcgcctgaccatcgcgccagagttgatacagtgggcgaacctgtgccgggatctcggtacttaacgcttcaatacgcgcgaccagctggcggcgctcatacggcgtaattttggcgtcggcgagcaaaatcccttgtttaaaggtattttgccagctgccgtcgtcatattggcgagcttgctgacgcgactgcgcaggcattaaacgatcagcacaatccatcgcccgcagccagtaaagcggattggtttcggttgatttaccttgcagcgcccagatgtcgctacattcagtagaaagatagtcagccagttgataaaccggaattttttcttctgctggcgtatcaatggctggcttattgtgattctgcacgcaacccagcaatgccagacatggcagccctgccagccacagccgtcggggcaataatcgttgaaaaatgtgtcgcatattcaccagacttaaagcctatcccagtgggcgtaattgttgcagacagtctggacatggacagcgcggagaaaccggagcgtacatatcgtacgtgaagatttcgagcactgcccggggccgaactgacaaataaaatagcctgataggataggctgttagcattatttcgtgtttttcgacgacggtaattcaatgcggaaacaaacgtcttgcccgctctcgtcgaccagatacagttccccttgcatacggcgaatacaatccctggcaatgcttaatcccagaccgctgcccttcaccgccccttttcgctggtggcttccctgaaaaaagggttcgaagatcatggcgcgttcctcttgcggaatgggcgtgcctgtattgatgacatcaatataaacccgcgcaccatgtaaactgctgcgaaggcaaatgttaccggattcagccccgtagtgcaccgcattggagtaaagattatccagtacgctcatcagcagcattggctccgccaggcaagctgttgctttgagatcgacgtcggtatgcatcattttagcccgtgcgggcaggctatgagcagaaaccactgtctccaccagcggtgctaactcaacattctccagttccaccgcactgtccgcctgtttacggttgtaatcaagcagttgttcgatcagtttttgcaaattgcggctgctgctatcaagaatgctcaccacctctttttgctctggcgtaagcggcccgacaacctggtcagccagtaattcagtgccctcgcgcatactcgccagtggcgtttttaattcatgagataaatgtcttaaaaattgatggcgttgggattccagccatgacaggcgctcacttaaccaaagaatacgttgcccaaccgagcgtaactcgctcggtccactgaacgagacgctattgcccagagaacgcccttcccccagacggttgatcatgcgctcgatatttttcaccggcccgataatcatccgcgtgaaaagcagtaccattaccagactcaccagaaatagcaccagcgattgccaaccaaaatattgcccacgttcggcgatttcacgctgaagctgctgcccacgagagaacaccactgtgcgcgtggcctgtaccatttcggtattggcactggcaaaggcttcaagacgtgcggcggcggcagcatcgggaccgctgttgttacactgaagttgagccagattgtgcaaatcctgacgtaatgcctggtagagtttatcgtccggcagcacgcctgcgtgggcatcgagcatttcgctgtaacgcttgcgctggctttgataaaccttcgccagggttgggtcgtccagcacgcaatactgacggtaactacgctccatctccagcgccgcgttggtcatcgcttcactgcgccgggcatcaataagcgtagtgcggttaaccagcgccgcctgatcgctaagcgcattcaggctttgccaggcttgccatgccagcaccaacaggggcagcagaatcagcaaaaatgccagcattaccagttgtcgtaatgagcggggaaaaacgggccagcgtttcaaggtgttactctcgtcagacgcgaatagcctgatgctaaccgaggggaagttcagatacaacaaagccgggaattacccggctttgttatggaataaggcggtgcctaactcgacgtttcgcccgatggttgatatagctacgctgatatcagaagttggacggcaggcaccttgttgtgcgtcattcgtattttatgtagcacgtcccgaaggggctgacataagtcggtgaatgagccactggttactattatgcagtaactgtgccaataaagaaaatagtttggtaacgtactgattatacgttgctttgaggggtttatgtctcctccgctgtttgaatgtaaatcagccactgtgtcgctaaaaagagacaacttaagataaacttattagataatattaaaatcaatgagttaagtgtcgccagaaagcgacacggcaaaccacccattgtcgtgatttacagacacaaaaaagctcccggagttgggagcttatgatagtggttggtgcttaatgccgcatccgggctgcaaaaccaatgggctgacgacttaccccaactgcttacgcgcattgcggaaaatgcgcatccatgggccatcctcgccccagttttccggatgccaggagttgctgacagtacggaaaacacgttccgggtgcggcatcataatggtgactcgaccactttcagtcgtgactgccgtaataccgttcggtgaaccgttcgggttagccgggtaggtttcagtgactttgccgaagttatcgacatagcgcagtgccaccagccctttgctttccagtgccgccagatgcgccgcatcacgcacttccacgcgcccttcaccatgagagacagcaatcggcatttgcgagcccaccatcccctgcaacagcagagacgggctttgggttacttcaaccaggctgaaacgcgcttcaaagcgatcggaggtattgcgcacaaaacgtggccacaactcactacctgggatcagttcacgcagattagacatcatctggcaaccgttacatacccccagcgccagcgtttgcggacggtggaagaaggttgcaaactcatcgcgtacacggtcattgaacaggattgacttcgcccaaccttcaccggcacccagcacatcaccgtaggagaaaccaccgcacgcgaccagggcgtggaaatcttccaggcccgtgcgtccggtcagcaggtcactcatatgcacgtcgatagcatcaaagcctgcacggtggaaagctgccgccatttcaacatgcgagttcacgccctgctcacgcagtacggcaactttcggacgtgcgccagtggcaatatacggtgctgccacatcttcgttgatatcgaacgacagttttacattcaggcccggatcggcgtcgttagatttcgcctgatgctcctgatcggcacactccgggttgtcacgcaggcgctgcatctgccaggtagtttctgcccaccagacacgcaacgtggtgcggctttcgctgaatacagtctgcccgttggcggtaatcacaaaacggtcaccggaaaccgcctgccctacataatggacacaatcagcaagcccatgctgtgccagtacggactcgaccgcttcacggtcagcggcacgaacctgaatcaccgcacccagttcttcgttaaacaacgccgccaggcgatcgtcacccagagtggcgatatccgcgtcaatgccacaatgaccagcaaaggccatttccgccagcgttaccagcaggccgccatcagagcggtcgtgatacgccagcagcttacgctgtgcaaccagcgcctgaatcgcgtcatagaagcctttcagttgcgcgacatcgcgtacatctgccggtttgtcgccaagctgacgataaacctgcgccagcgccgttgcgcccagcgcgttattgcctttgcccaaatcaatcagcagcagtgcgttatcttcggtagaaagctgcggcgtgatggtgtgacgtacatcttccacgcgggcaaatgcagaaatcaccagcgacagcggcgacgtcatttcgcgctcttcgttaccttcctgccagcgggttttcatcgacatggagtctttacccaccgggatcgtcaggcccagcgccggacaaagctcttcgcccacggctttaacggcttcatacaggcccgcatcttcaccagggtggcctgccgccgccatccagttggcggaaagtttgatgcgtttgatatcgccaatttgtgttgcggcgatgttggttaacgcttcaccgaccgccagacgggcagaggcggcgaaatccagcagcgcaaccggcgcacgctcgccaatcgccatcgcttcaccgtagtagctgtcgaggctggcggtagtgaccgcgcagttagcgaccggcacctgccacggccccaccatctgatcgcgcgctaccatgccggttacgctgcggtcgccaatggtcaccaggaaggttttttccgccacagtcggcagatgcagcacacgtttcaccgcgtctgcaatggtgatcccttcacgggccagcgcgtcgcctttcgctttcagcgtttgtacatcgcgggtcatcttcggcgttttaccaagcaggacgtccagcggcagatcgatcggctgattatcaaaatgacgatcgtgcagagaaagatgcagttcttcggtcgcttcaccaatcaccgcgtagggtgcgcgctcacgcttacacagttcgtcaaacagcggtaattgatcggcagcaaccgccagcacgtagcgttcctgggattcgttacaccagatttccagcgggctcatgcccggttcgtcgcttagaatctcgcgcagttcaaatttaccgccgcgcccgccgtcgctcaccagttccggcatggcgttagaaagaccgccagcgccaacgtcgtggataaacaggattgggttggcatcaccaagctgccagcaacggtcgatcacttcctggcagcgacgctccatctccgggttgtcgcgctgtacggaagcaaagtcgaggtcggcatcagactgaccagacgccatagaagacgctgcaccaccgccaagaccgatgttcattgccgggccgccgagaacgaccagcttcgcaccgacgttgatctcgcctttttgtacgtgatcggcgcgaatgttgccgatcccgcccgccagcatgatcggtttgtgataaccgcgcagctcttcgccgttgtggctgttcactttttcttcataagtacggaagtagccgttcagtgccggacgaccaaattcgttgttaaacgccgcgccgcccagcgggccttcggtcatgatgtccagcgcggtgacaatgcgctcaggcttaccgaaatcttcttcccacggctgttcgaagccaggaattcgcaggttggaaacggagaaaccaaccagacccgctttcggctttgcgccgcgcccggtggcaccttcatcgcggatttcaccgccggaaccggtcgccgcgcccggccacggagaaatcgccgtcgggtggttgtgagtttcgactttcatcagaatatgcgccggttcctgatggaaatcgtagcggcccgtttcgtggtcagcaaagtagcggcccacttcagaaccttccattacggcggcgttatctttataagcagagagaacgtgatctggcgtggtttcgaaagtatttttgatcatcttgaacagcgatttcggctgctgttcaccatcgataacccagtcggcgttaaaaattttgtggcggcagtgctcggagttcgcctgggcaaacatatacagttcgatgtcgttcgggttacgaccaagctttgtgaaagcatcctgcagatagtcaatttcatcttccgccagagccaagccaagacgcaggttagcgtcgatcagcgcctgacggccctgccccagcaaatcaacgctggtaaccggagtcggttgatggtgggcaaacaactgctctgcatcatctaaagcaaaaaagaccgtttccatcatgcggtcgtgcagttcagcggtaacctgctgccattgttcattggtcagcgtaccggcttctatatagtaagcaacgccgcgctcaaggcggtttacctgttgtagcccgcagttatgggcaatatcggtcgctttcgaagaccagggagagatggtgccaggacgcggggtcaccagcaggagtttgccttgcggggcgtggctggcgagtgccgggccatatttcagcaggcgttcaagttgtgcgtgctcatcatcgtttaacggcgcattgaggtcagcaaaatggacatactcggcgtaaatattgtgaaccgggagcctggcagcctgaaaacgtgccagcagtttgttgattcggaatgccgacagtgcaggcgaaccacgcagaatttccatcataagtctctcgtcttctaagctttcggtgtacccaagggggggaaacgggcgtcattataaagaatctgatgcgctgacgaaaccgtttgcgtggaaataaaatcaccatcgtgaattagcaacgcgtgccgccaatggctgtaataagttgccatctggcgcaggtttacgcaaaatgccgctcatttatgagtaaacctttcactattattacgttttttcaagctgggacgcgcacgacacagagaattaactaattgaaaaaattaaagattaattatctgttcatcggcattctggcactgctgctcgcggtcgctctctggccatccattccctggtttggtaaagccgacaaccgtatcgccgccattcaagcgcggggagagttgcgtgtgagcaccattcatactcccctgacttataacgaaatcaacgggaaaccttttggcctggattacgaactggcgaaacagtttgccgattacctcggcgtaaaactgaaagtgaccgtgcggcagaatatcagccagctgtttgacgaccttgataatggtaacgccgacctgctggcggcaggacttgtctataacagtgagcgggtaaaaaattatcagcctggccctacctattattccgtgtcacaacaactggtttataaagtgggtcagtatcgcccacgtacgctgggcaacctgacggcggagcaactcaccgttgcaccgggtcatgtggtggttaacgatctccagaccctgaaagaaacaaaattcccggaattaagctggaaggtagacgacaaaaaaggctctgcggaattaatggaagatgtcatcgaaggaaaactcgattacaccattgctgattctgtcgccatcagcctgtttcagcgcgttcacccggagctcgccgtagcgctcgatatcaccgatgaacaaccggtgacttggtttagcccgttagatggcgataataccctttccgccgccctgctcgacttcttcaacgaaatgaatgaagacggtacgctggcacgcattgaagagaaatacctggggcatggcgatgattttgattacgtcgatacgcgcacatttttacgcgccgtcgatgcggtactgccgcagttaaagcccctgtttgagaaatacgccgaagaaattgactggcgtttgctggccgctattgcttatcaggaatcgcactgggatgcacaggccacttcaccgacgggtgtgcgcggcatgatgatgttaaccaaaaataccgcgcaaagcctcggcattacggatcgtaccgatgccgaacagagcatcagcggtggcgtgcgttatttgcaggatatgatgagtaaagtgccggaaagtgtgccggagaacgagcggatctggtttgccctcgctgcgtacaatatgggctatgcgcatatgctggatgcccgcgccctgacggcaaaaaccaaagggaatcctgacagttgggctgacgtaaaacagcgtctgcctttacttagccagaaaccctattacagcaagctgacttacggctacgctcgtggacatgaagcctacgcttatgtcgaaaatattcgtaagtatcagattagcctggtgggttatctgcaagagaaagagaagcaggctacagaagcggcgatgcaactggcgcaggattatccggcggtatcgcctacggagttgggcaaagagaaatttccttttctctcgtttctttcccagtcgtcatcaaactatttgacccattctccctctctgctgttttccaggaaagggagtgaagagaaacaaaattaatccgtcgaggattgcgcttttttctgcgctttaatttcctggcggcgcatgcgaaagaagtcactgagcaacgccgcgcactcatccgccagtattccttccgtaatttccactcggtgattcatacccggatgatgcagcacatccattaaagatcccgcagcgccagttttcgcgtcacgcgcaccaaagaccacgcgaccaatgcgactgtggatcatcgctccggcacacattacacatggttcaagcgtgacatacaacgtggcgtcgatcagacgataattttgcatcaccagaccaccctgccgcagggccatgatttctgcatgtgcggtgggatcatggcgaccaatcgggcggttccagccttcgccgattacccgattgttatgcactaataccgcgccgaccggcacttcccgctcatcccaggcacgtttcgccagcgtcagcgcgtgacgcatccagtattcgtggctaaattcgacttcagacaaaaagaaaactccggttataaaagcgcggcgcattatacacggacgctatgctttactctattccagttgctggagttcaccgcgcggggttactcgccaacgatgctgacagaaataaagcagcggattgtcctgattactgtcgctatagccactgtacagccgcagcggagtgccgattttgcgctccagttgtgcgaccttttcatgtcccagacaacgcatcgtcaatacccaaccaccatagccacgctgaatttggctggcgataagattaacccgcggcagccagggcgtatcgaaataaaccgcttcaaccagcggctgcggagagccggtaatcaaccagatatcagcatcggaacttaacaggtaggtggttaatcgctcctgaaccagcggaaaggcggtaacattgtcgcgaaaccagcgcacgaaatcggcctgcaacgtctgtaaacgtgcttcgctgtgaccaaaagtgcacccccacagaagcagactcatcggccagcgtgccgcacgaccttttatcaataacgcaatggctataatcggtaacaacggcaggacaagtaacgcattcagcggttggcgacgtagtaaatagcgcagaaaactgccgaacatatcctgctgatgcaatgttccatctaagtcaaaaaacaccacacgacgctcgtgagttgccaaaccatactcctctggactgaaacatcctgattaattttcgctactacatagcctaacagatagatcatcacttttccggcaacaatcgaccgcatcatggctaactggaatttttaattcatggcaattagcggcaatggaatataaaattcactcgcgtgtgtctcatattgcctgttgtcgccactatttcatcgcgaggaaagatatgaacggcttacttcgtatccgtcagcgttaccaggggcttgcccagagtgataaaaaactggcggattatctgctgctacaacctgatacggcgcgccatttaagctctcagcaactggccaacgaagccggagtcagtcagtccagcgtcgtgaagttcgcgcaaaaactcggctataaaggttttccggcgcttaagttggcgttgagtgaagcgctggcaagccagccggaatcaccctccgtgcccattcataaccaaatccgcggtgatgatccgttacggctggtcggcgaaaaactgattaaagaaaatactgccgctatgtacgcaacgctaaacgttaatagtgaagagaaactgcatgaatgcgtaacaatgttgcgctctgcgcggcggataattctgaccggtattggcgcttcgggtctggtggcgcaaaactttgcctggaagctgatgaagattggcttcaatgctgccgcagtgcgcgatatgcatgcgctactcgcaacagtacaggcgtcgtcccctgacgatctgttattagccatttcctacaccggtgtacgacgcgagttaaacctggcggcagatgagatgctgcgagtgggcggaaaagtgctggcgattaccggctttactccgaatgccctgcaacagcgtgcttctcattgcctgtataccattgccgaagaacaagcgacaaacagtgcttcaatctctgcttgtcacgctcagggaatgttaacggatttgctgttcattgcgctgattcagcaggatctggaactggcaccagaacgtattcgtcatagtgaagcgctggtgaaaaaactggtctgagtaaagaatgcgcgtataatgcccgcccggtttgtgttgttttgagagtttccttatggcgttgttaatcactaaaaaatgcatcaattgtgatatgtgtgaacccgaatgcccgaatgaggcgatttcaatgggagatcatatctacgagattaacagcgataagtgtaccgaatgcgtagggcactacgagacaccaacctgccagaaggtgtgcccgatccccaatactattgtgaaagatccggcgcatgtcgagacagaagaacagttgtgggataaatttgtgctgatgcaccacgcggataaaatttaatattctactctggaagtagagtattaattatattactgggaagccttaacgccattatatttatttaattgatgacattagcataatcattcactaagttaatttatatagtatctgcccagacacttatttatagttattaaaggtgcgtccgactggttcaccggacgcaccttaagtacgtttccttgtgttataagaacagaaggatcagctgtaaaacagcaatgatgattttgatgacccgtttaatcaggtatcggcaatcagtcattcgtttttccttaaacaaggaatgcagccattcagattagcccttacatctccccaaaactgaacgtgcgagttattgagggtgcatgctgcactccacaccagagctttgacgacaccactcgtttcaatgggggaattctgtggcatggtgtaaagcacagcaaaatcttcaataacgaagccaattttaatgtacttacgaattggcggtcacgttaatctttccatcaatattgctttcttcgtaaaggctcgagtttttatgctaaagattgcaagttgcttgtaaaagataagtacactgatccataatcgctgttgttgagggtgcatgctgcacaaaattaaagttaaaaagtaaaacccccgttccttaccagttcgggggttttactttttaaagagaacggtattatttttaactttcaataattaccgtggcacaagcatagtgccgctcatctgccagcgttacatgcatatttgcaacgcccagcttttccgccagttttaatgcctcgccccatagccgtagccgtggtttgccgagctcatcattgaatacttcaaattgattaaacgccagaccattgcggatcccggtgccaaacgcttttgctgcggcttctttcacagcaaaacgcttcgccagaaaacgcaccggctggtggtgcgttttccagatagcccattcgttatcgcttaatacgcggcgtgccaggcgatcaccggatcgggcgatcaccgcttcgatgcgagcgatctccacaatatccgtgcctaaacctaatattgccattagccacgcgcttccagcatcagacgcttcatttctgccaccgcatctttcagtccggtcatcactgcacgaccaataatggcatgaccgatattcagttcatgcatctcagggatggcggcaatggctttcacgttgtgataggtcagaccgtgtccggcgttaactttcagaccgaggcttgcggcaaaggtcgcggctttggcgatacgcgccagctcttgcgcctgttcggcgtcagttttggcatcagcatagcaaccggtgtggatctcgataaacggtgcgccaacctctgccgcagctttgatctgctcttcatcggcgtcaataaacagagaaacctgaatcccggcatctgccagacgtttgcaggcatcgcgcattttgtcacgctgccctgcgacatccaggccgccttcggttgttacttcctgacgcttttccggtaccaggcagcaaaaatgtggcttcgtctcaacggcgatcgccagcatctcttcggtcaccgccatctccagattcatgcgggtatccagcgtctgacgcaggatgcgcacgtcgcggtcagtaatgtgacggcgatcttcacgtaaatgcacggtaatgccgtccgctcccgcctgctcggcaataaacgcggcctgcaccggatccgggtaagcggtaccgcgcgcgttgcgcagcgtagcgatatggtcaatgttgacgcctaacagtaattcagccatgacaatcctcatcattcataatgtgttttcaccgttcgcttaggcataaactgccggaacagttccctgctctttaaaggtttaccgccaagatacggcttaagcgccatgcgggtaaagcgtttcgcggcgcgcagtgtgtctgcgtcaggaaattcccgtgcgtttaacgcttttaactgccttccggtgaacgttttattgtcgataacgacgcttgcgataaaccctttttcttcgcgataacgatacgtcatggtgtcatctaccggctcgccgctacccgcacaatgggtaaaattgacgccataacccagatgcccgagcagtgccagttcaaagcggcgcagcgcgggttctggcgtaccagtgacccctgcaagagactgaatgcagtgcaagtaatcgaaaaaaagttcagagaagcgcgtctcgtattccagtacgcgggagagaagttcgttgatgtacagaccgctgtaaagcgtgataccgcttaatggcagcgccagcgagacggcttcagcactgcgcagcgttttgacttcgccacgcccgccaaaacgtagcaagagaggggtgaaaggctgtaatgcacctttcagggtagagcgtttagagcgtgcgcctttggcaaccagacgcacgcgccccgattcctccgtgaagacgtccagcatcaggctggtttcgctccacgggcgactatgcaggacaaatgcgcgctgccagccttccatcggagttactcttaaagatcgtcaacgtaaccgagactgcgcagtgcgcgttcgtcgtcggcccaaccggatttcacttttacccacagttcaaggtgaacaggcgcttcgaacatttcctgcatgtctttacgcgcttcaatcccgatggttttgatcttggcccctttgttgccaatgaccatcttcttctgcccttcacgctcaacgagaatcaaaccgttgatgtcataaccaccgcgttcgttagagacgaaacgttcgatctccacggtcacggagtacggcagttcagcgccgaggaaacgcatcagtttttcgcggatgatttcagacgccataaaacgctgtgagcgatcggtgatgtaatcttccgggaagtgatgagtcgcttcaggtagatgcttacgcacgattgccgcaatagtgtcaacattcagcccggtttcggcagagattggcacgatatcgaggaagttcatctggcttgccaggaactgcaggtgcggcagcagatcggctttctcctgcacgttgtccactttgttcaccgcgaggattaccggcgctttgccttcgcgcagtttgttgagcaccatttcgtcgtccggcgtccagcgggtgccttcaacgacaaaaatcaccagctcaacatcgccaatagagctgctcgccgctttgttcatcaggcggttaatggcgcgtttttcttccatatgcaggcccggtgtatcgacgtagatcgcctgatacgcgccttcagtatggatccccacaatgcggtgacgagttgtctgcgccttgcgggaagtgatggagattttctgccccagcagtttgttcaacaatgtggatttgccaacgttcggacgtccgacgatggcaataaatccgcagtaacttttatcgatgctcattccagctccagttttttcaacgcctgttcggcggcagcctgctcagccttacgacggcttgaacctgtgccaaccaccggttcactcaggccgctgacctggcagtggatagtaaattcctgatcgtgcgcttcgccacgtacctggactaccagataagtcggcagcggcagatggcgaccctgcaaatattcttgcaagcgcgttttcggatctttttgtttatcgcctgggctaatttcgtccaaacgagtttgataccagttgaggattaatttctcgacggtttgaatatcactgtcgaggaatacgccaccaattaatgcttcgacggtgtcggcgagaattgactcacgacgaaatccaccgcttttaagttcacctggccctaaacgtaagcactcgcctaactcaaattcgcgcgccagttccgccagcgtattgccacggaccagcgtggcgcgcatccggctcatatcgccttcatccacacgagggaaacggtgataaagcgcattggcgataacgtagctcagaatagagtcgcctaaaaattctaaacgctcgttatgtttactgctggcactacgatgagttaatgcctgctgcaacagttcctgatgattaaaagtgtagcccagcttccgttgaagccgattaattacgatggggttcatgcgataccaataaataaatgcgtcaacaattcagcacacgaaacagacctgatatacatggttctgctaactgcttcgctgcagtttcagtttaccggtatatggggaccaacgctgtttcgtgtgccgtggcaacctggaggtgccaaccttaaacttcgggggaatattctatacacaacgacgggggatgtcgttagccacgggagatttatctcataaataattcacgttgtcgccataacggcgacaacgtgaacgaagatggctattaatggatgccgccaatgcgacttaagcgcagaccagtcggccattcgccttcttgcttatcgaagctcatccagatagccgttgcccgaccgaccagattcgcttccggcacaaagccccagtaacggctgtccgcgctgttgtcgcggttgtcgcccatcatgaagtattgtcccggaggaacaatccaggttgccagttgttgccctggctgctggtaatacatccccacctgatcctgcgcaatcggcactgtcagaatgcggtgcgtcacatcacccagtgtctctttacgctcggaaagacgaattccattttctttggtttcgtttttcggcacttcaaagaatccgctggtcgcttccccaccattacggcgtgagaaggtctgaacgaaatcgctcggttccacgtttgagtaggtgaccggcagcgcgttttcacacgcctggccggaactgcatcccggttgaatcgtcagctcttttgagaccggatcgtaagtgactttatcgcccggtaaacccaccgcgcgcttgatgtaatcaagctttggatcttccggatatttaaagaccacgatatcgccgcgtttcggatgaccggtttcgatcagcgttttctggtagataggatctttaatgccataagcaaacttctctaccagaataaaatcaccaattaacagagtcggcatcatcgaacctgacgggatctggaacggttcataaataaacgaacgcacaatcaatacgatagccagtaccggaaaaacagaagcaccggtttccagccagccaggcttcggcgcaacctttttcaacgttgctttatccagtgagtccccggcagccgcctgcgccgctgcctgacgttcccgccgtttaggtgcgaaaaagaatttatccacgcaccataaaatgcccgtcaccagtgtggcaatcaccagaatcagggcaaacatattcgccatgccaactcctaagggttatttgttgtctttgccgacgtgcagaatggcgaggaacgcttcctgcggcagctcgacgttaccgatctgcttcatgcgtttcttaccttctttctgcttctgcagcagctttttcttacggctgatatcgccgccataacatttagccagtacgtttttacgcagctgtttcacggtggatcgcgcaatgatgtgcgtaccaatcgctgcctgaatggcgatatcaaactgctggcgtgggatcagatctttcatcttctccaccaactcgcgaccgcggttttgcgaattatcacggtgggtgatcaacgccagcgcatcaacacgttcaccgttgattaatacgtctacacgtaccatgtcggacgcctggaagcgcttgaagttgtaatccagagacgcataaccacgcgaggtagatttcaggcgatcgaagaagtcgagcaccacttccgccatcgggatctcgtacgtcagcgccacctgattaccgtggtaaaccatattggtctgcacgccgcgtttttctacgcacaacgtaataacgttgccgagatatgcctgcggcagcagcatgtgacactctgcaatcggctcgcgcagttcgtagatgttatttaccgcaggcagcttggatgggctgtcgacgtagataacttctcttgacgtggtttcaacttcatacactacggtcggcgcagtggtgatcagatccagatcgtattcacgttccagacgttcctggatgatctccatgtgcagcaggccgaggaagccgcagcggaaaccaaagcccagcgcgctggagctttccggctcatagaacagtgaggcatcgttcaggctgagtttacccagcgcgtcacggaaggcttcatagtcgtcggaacttaccgggaacagaccggcgtatacctgcggtttgactttcttaaagccaggcagcgccttttctgccggattacgcgccagcgttaaggtatcgccgactggagcgccgtggatatctttaatcgcacatacgagccagcctacttcgccacatttcagttcagtgcggtcaacctgtttcggcgtgaagatgcccagacggtcggcgttataggtctgcccggtactcatgactttcactttgtcgcccttacgcagggtgccgtttttaatacggataagtgaaacaacgcccaggtagttgtcgaaccatgagtcgataattagtgcctgcaacgggccttccggatcgccttccggcggcggaatgtcgcgcaccagacgttcgagaacgtcctgcacaccaacgccggttttcgctgaacagcgcaccgcgtcggtggcgtcgatgccgacgatatcttcaatttcttccgccacgcgttcaggatcggctgccggcaggtcaatcttgttcagtaccggcacaacttcgagatccatttccatggcggtgtagcagtttgccagggtttgcgcttctacgccctgcccggcgtcgaccaccagcaatgcaccttcacaggcagccagcgaacgggaaacttcataggagaagtctacgtggcccggggtgtcgataaagttaagctgataggtttcgccgtcagacgctttgtagtccagcgtcacgctttgcgctttgatggtaatgccacgctcacgctcaagatccatggaatcgagaacctgcgcctccatttcacggtcagacaggccaccgcagatctggataatacggtcagacagcgtcgatttaccgtggtcaatgtgagctatgatcgaaaagttacgtatattcttcataaagtatgattattgtgccttaatgcccggttaaccaggcttttagaagtcgctgttctgagcttaacgtctgtattaatagaaacgccgcattctacactacaacattgaggcgaggaaatgttcataccgtatggattgtggtatctggaaacgtcctcgcatttgttatgcaaaatgcaacaaagccagtgaaatcactggctcgcgtcttccgaagatgtttcaaatcgcacaaggccaggcggcaatgccacgcttaagatgatcggttgccattctgcccgggcagcaaacttacgcgagtagccgcgcgcaatcaggaacccgccaataccaccgaggatcgcaccacataatgctgcgacgtcagaagcaaagagtagctgaaatagcgaagcgataaggaataatcccaccagcggcgacatataaaccagtaatgcggagctaagcaggctgccttcggcgatccccaattccactttttgccccggcactaacggctcatcacagggtacgacaatggtatgcgtggtttgcgggccaagtttatttaacacgcggctaccgcaaccggcgcgtgaagcgcagctgctgcatgaagctttaacatcacaactgaccagcgcctgcccgttttgccaggagacgacggtagcccactctttgatcattgcgctgccccgaacttaatattctcggcaatgcgtttcgccgtttgcggcggcagttcaccgacaatggtgatttcggcgttatcacgtacgcttgtactgacggttctgcgtccggtgcgcaacatctgatcggtgctcgatggcgtagcgcggttaacgtttaccgagaagctgaataatccgtcggaatagagacgtgattcgataggcatgttgtccatcgtcggtagcggacgtcgactactggaaacttcgctaaaaccctgtggcaaccaggttggcgtccagctgaatttagctttttcacctacaggaacagaaagcaacggcggcaaatttgccttcgccagcgtctgcatactgctgctgatatcctgattgacgttaaaagcaatcacgcgaaattgttccagcgtttcaccatcgcgatcaaggagatcaacccgcatcggtaatttcgattcggtgtccatccacacgatgtagctgtagcgtgtaccatctcgggcaaccacgcgaatgacttcgcaaagacgatcagcaatacgcgtgcgcccgacggagataaagtcgtagtaaggagaaaggcgtttgaaatcggtatagataagcgatggcagagaatcaacaatgtaatcgccattaagcgtgaacggttcaagtcccggttcaaaatagctgatttcattgccgcgctgtaccacttcccggcgcgggccatccatttgcaacaattgtgcaagaggacggttatcgaggcgtgcatgtcgataacgcagagactcaacaccctgtttattgatgctgatgaatgacagctcgtaattcagtgactgactggccaggttcatctgctgtaataacgccccggacgcgggagtggccgaggcgttagcagagaataacaggctacctgtcactaatgacatggcaaaccaaagttgcttcattactgcgattgcgttcctaaagtttgaattcctggcacctgtacagcggcttgctgggtttgcgcctgctcaaactgaagctgttcagagtggagtcggcgttgcagttcgtaatcctgcaacattgcattaatgcgacgacgctgctcctgtacctgctgctgttgaccattgtttgcggtcgcttcagaaggtactcccaggcttaccgggctggctttacccatcatcggcagtgtattaaataccggcgtttcgggctgctgggacgtttcagattgtccattatagtgctggacgccaacgataactgcaagcgatacgcatgcggctacgcccatttgggtaagctgtgccgcccacggacgtactttctgccagaatggcattttctgccattgatgcggcgcaggctgggcttccgggatcaatgtcgccggttgacgtactggctcttcttcaatggcggccatcacgcgtgaagagatatcgaaatggagcacctcgggagtatcaccccgcattgagtcacggattaagtgatagctttcccaggttttctgcatttctgggttatgagccagttcgttaagcagctcactatccagcgtttcgccatccattaaagcggaaagttgttctttctgcatgcctaatacccttatccagtatcccgctatcgtcaacgcctgataagcggttgaactttgttatcaatagcttccctcgctcggaagatacgtgaacgcaccgtacctaccggacaatccatgatagcggctatctcttcatagctcaggccatccagctcccgcaaggttattgccatgcgtaaatcttccgggagggactcaatagttcggaaaactatctgtctcagttcttctgacaacattaagttctcagggttcgaaatttctttcaacgcgccgccactttcgaagttttcagcttcaatggcatccacatcactggaaggtggacgacgcccctgagcaaccaggtaatttttcgctgtatttacagcaatccgatacagccatgtataaaaagcgctatctccccggaacgaatccagcgcacgataggctttaataaaagcttcttgtaccacatcgggaacatcacccgacggcacatagcgggaaaccagactcgccactttatgctgatagcgcactaccagtaagttaaaggctttctgatctcccttctggacccgttcaaccaggacctggtccgttaactgctcgctcatccgaggtaaagtctccccaaaccaaatttccacgcgctatcgaaacgccactccattagctgcaatttgagcaagcaaagggttagagtgtctcgtttttgtaaagttccgtaacgcatctgtttttgtttgtcatgctgtagacggatcattatctatcattataagtctacagaatctgaacatcgcattatctgtgtagaaatgcccatttaactgcctgaagagtaacccaacggcctttttatttcaccacctaatcctccaccagccagtaacttctctttttctcgccgccctgcgtcagcgtgtttagcaactgtaacaaatattaaaatagcaggtgtttatccgcacaacatgatgctatgctgaccaaaccatgtttagtaaattaaacaaagaaaatgaatactctccctgaacattcatgtgacgtgttgattatcggtagcggcgcagccggactttcactggcgctacgcctggctgaccagcatcaggtcatcgttctaagtaaaggcccggtaacggaaggttcaacattttatgcccagggcggtattgccgccgtgtttgatgaaactgacagcattgactcgcatgtggaagacacattgattgccggggctggtatttgcgatcgccatgcagttgaatttgtcgccagcaatgcacgatcctgtgtgcaatggctaatcgaccagggggtgttgtttgatacccacattcaaccgaatggcgaagaaagttaccatctgacccgtgaaggtggacatagtcaccgtcgtattcttcatgccgccgacgccaccggtagagaagtagaaaccacgctggtgagcaaggcgctgaaccatccgaatattcgcgtgctggagcgcagcaacgcggttgatctgattgtttctgacaaaattggcctgccgggcacgcgacgggttgttggcgcgtgggtatggaaccgtaataaagaaacggtggaaacctgccacgcaaaagcggtggtgctggcaaccggcggtgcgtcgaaggtttatcagtacaccaccaatccggatatttcttctggcgatggcattgctatggcgtggcgcgcaggctgccgggttgccaatctcgaatttaatcagttccaccctaccgcgctatatcacccacaggcacgcaatttcctgttaacagaagcactgcgcggcgaaggcgcttatctcaagcgcccggatggtacgcgttttatgcccgattttgatgagcgcggcgaactggccccgcgcgatattgtcgcccgcgccattgaccatgaaatgaaacgcctcggcgcagattgtatgttccttgatatcagccataagcccgccgattttattcgccagcatttcccgatgatttatgaaaagctgctcgggctggggattgatctcacacaagaaccggtaccgattgtgcctgctgcacattatacctgcggtggtgtaatggttgatgatcatgggcgtacggacgtcgagggcttgtatgccattggcgaggtgagttataccggcttacacggcgctaaccgcatggcctcgaattcattgctggagtgtctggtctatggctggtcggcggcggaagatatcaccagacgtatgccttatgcccacgacatcagtacgttaccgccgtgggatgaaagccgcgttgagaaccctgacgaacgggtagtaattcagcataactggcacgagctacgtctgtttatgtgggattacgttggcattgtgcgcacaacgaagcgcctggaacgcgccctgcggcggataaccatgctccaacaagaaatagacgaatattacgcccatttccgcgtctcaaataatttgctggagctgcgtaatctggtacaggttgccgagttgattgttcgctgtgcaatgatgcgtaaagagagtcgggggttgcatttcacgctggattatccggaactgctcacccattccggtccgtcgatcctttcccccggcaatcattacataaacagataaaaagcctgggtcagcgccgtatacgcttcggaatagttctggtctggcccacgaatgactaagcgatcgctaaagcattctcccgcctgcggggagaatgccagcagcacccgatgcggcagtcgcgcttcgttttccgccacatccgtccgcaaacgtaaatgccagcccatgcttaatgccagctccgtaaaaccattaccaatctgctctggcagcactacgcagaaaaatccctcttcggtaatgcactccgccgcacaggtcagcaacgatgggtgatcaagcgtagtggtatagcgagcctgttcccgttgaggtgtcgagcactctactccctgctgatagtaaggtgggttactgatgattaaatcgaagcgtactgtctgctgtgtgatccactgctgaatatccgccgtatggacgttaatccgctctgcccacggggactggttgatattttcctgcgcctgcgcggcagcttcactttccagttcaactgcatcaatcatcacgctgtcatcggttcgctgcgccagcattaatgccagcaacccgctacccgcgccgatatcaaggcaacgttttaccccagccaccggtgcccatgcgcccaataaaataccatccgttcccactttcatcgcacagcgatcgtgagcaacaaaaaactgtttaaaagtaaatccattacgacgaagcacggatgtagactgtgacatgaaaataaaaccttgcaggaaaaacggcgatagcaccgggtgagaacaatacccgagaagcgatatccatacaaacagatgaagattgcagccgtaacgtctataatcagcgccccacacagaggtagaacatgactgtaacgactttttccgaacttgaactcgacgaaagcctgctggaagccctccaggataaaggtttcactcgcccgaccgccattcaggctgccgccattccgcctgcgctcgatggccgtgatgtactcggttctgcgccgacaggcaccggtaaaacggcggcgtatctgctgccagcgttgcagcacctgctcgatttcccgcgtaagaaatccggtccgccgcgtattttgatcctcaccccaactcgcgagctggcgatgcaggtgtccgatcatgcccgcgaactggcgaaacatacgcatctggatatcgccaccatcaccggcggcgtagcctatatgaaccacgcggaagtgttcagcgaaaatcaggacatcgtggtcgccacgaccggacgtctgctgcaatacataaaagaagagaacttcgattgccgcgcggttgaaacgctgatcctcgacgaagcagaccgtatgctggatatgggcttcgctcaggatatcgaacatattgctggcgaaacgcgctggcgtaaacagaccctgctcttttcggcaacgctggaaggcgatgcgattcaggactttgccgagcgtctgctggaagatccggtggaagtttctgccaatccctccacccgtgagcgcaaaaaaattcatcagtggtattaccgcgccgatgatcttgagcataaaaccgcgttgctggtgcatctgttaaaacagccggaagcgacccgctcaattgtgtttgtgcgtaagcgtgagcgtgtgcatgagctggcaaactggctgcgcgaagcgggcatcaacaactgctatctcgaaggtgagatggtacagggcaagcgtaacgaagcgatcaagcgtttgaccgaaggtcgcgtaaacgtactggtcgcaaccgatgttgccgcgcgcggtatcgacattcctgacgtcagccacgtctttaacttcgatatgccgcgcagtggcgatacttatttgcaccgtatcggacgtaccgcgcgcgccggtcgtaaaggcaccgcaatttcgctggtggaagcccatgaccatctgctgctgggtaaagtaggccgctatattgaagagccaattaaagctcgcgttattgatgagttacgcccgaaaacgcgtgcgccaagcgaaaagcagaccggcaagccatcgaagaaagtactggctaaacgtgctgagaagaaaaaagctaaagagaaagagaagccgcgggtgaaaaaacgccatcgcgacaccaaaaatattggtaagcgccgtaaaccaagcggaacgggcgtgccaccgcaaacgacagaagagtaatctcaatgccaggtttaagcctggtattaaaagtgctggcaaacgcaaaactgcctgatgcgctacgcttatcaggcctacgtggctcatgcaatatattgaatttgcacgatcttgtaggccggataaggcgttcacgccgcatccggcatgaataaagcgcactttgtcgacaagttaaatgccgggtttaatcccgacattatttttatccagccacaaaactctcttcaacacactgaataaaagtgtgcatcgccgggctaaccgcttttccagcatgatgtgcgcacatggccgtaatggtctgcgactgttcgccaaaaggcaattcaattaattctccgcactccaactcttttgccaccgcaaagcgcggtaggtagctgaccccgatattcgccgcgacacaacgcttgatgctttcgatacttataagctcaatggtgttttccaccgtgatccgccgctgacgcagcgtgctctcaaatatctgccggaagacacattgcggttcgttgataataaagctacaggcgttatgtcttcccggctcagtaaaatcgacatctgcaatttgcggtgaagccaccagcaccagtgattgttcacccaactctcgtcgattcagagcatcatcattccctacacgataaaagacgccaacatcggcctcatcattcagtagcgcatcacggatcacgtaacagttcagcgactgcaacgataaacgcacttttggggcgcgttgccgaaaacgctgcaacacctgcggcattcggtaagagagcaacgtttcgcccgaaacaacgcgtagttccccgtccggatctgactcctttttggcagcctcacgaagcgtatccatcactcgggtaagttcataaatgtgcggcagcaacttttttccttcgcgggtaaggcacatccgtcggccaattttctcaaataactggactgaaaactcctgctcaagctgctgaatatgaaaagtcaccgtcgattgtgtacagcacaatttttgcgaagctcgcaaaaaggaaccctcttccaccacggttttaagcgtaataaaacggcgcagatccataaccccaaacctatcgaaaatatcgaatctagaatataaaaacattcatttttttaaatgttccgtgtcgggtactgtctaccaaaacagaggagataacaagtgacaccgacccttttaagtgctttttggacttacaccctgattaccgctatgacgccaggaccgaacaatattctcgcccttagctctgctacgtcgcatggatttcgtcaaagtacccgcgtgctggcagggatgagtctgggatttttgattgtgatgttactgtgtgcgggcatttcattttcactggcagtgattgacccggcagcggtacaccttttgagttgggcgggggcggcatatattgtctggctggcgtggaaaatcgccaccagcccaacaaaggaagacggacttcaggcaaaaccaatcagcttttgggccagctttgctttgcagtttgtgaacgtcaaaatcattttgtacggtgttacggcactgtcgacgtttgttctgccgcaaacacaggcgttaagctgggtagttggcgtcagcgttttgctggcgatgattgggacgtttggcaatgtgtgctgggcgctggcggggcatctgtttcagcgattgtttcgccagtatggtcgccagttaaatatcgtgcttgccctgttgctggtctattgcgcggtacgcattttctattaacgaaaaaaagcggaagaggtcgccctcttccgcttagtaacttgctacttaagccttacaggctttcagtaaaggtacgagcgataacgtcgcgctgctgttccggagtcagagagttaaagcgaactgcataaccggatacacggatggtcagctgcggatatttttccggatgcttaactgcatcttccagagtttcgcgacgcagaacgttaacgttcaggtgttgaccaccttcaacgcgaacttctggtttcacttctactggaacttcacggtattcaatgtcacccagtttgcttactgcaaccacttcatcttctgcataacctgcttttgcaacgatgcaacgcgcttcgcctttttcgctgtccagcagccagaaagagttcagcagatcgtcgttagcggctttagtaatctggatacctgtaatcatgtgatgcctccccggcaaaattatttgatttgttcagcctgtcgcggccaattggtaaaaccattgttgcttgagtgtatatatactcctcaaacacccttgaatctttgatttaaatcaataaaaaccacacatcaagtatggtcgcaaatggattttattgttttacatcaacttatgcgggtgtgaaattttaccaatttacatttttttgcactcgtttaagtctaaaaaatgagcatgattttgttctgtagaaagaagcagttaagctaggcggattgaagattcgcaggagagcgagatggctaacgaattaacctggcatgacgtgctggctgaagagaagcagcaaccctattttcttaatacccttcagaccgtcgccagcgagcggcagtccggcgtcactatctacccaccacaaaaagatgtctttaacgcgttccgctttacagagttgggtgacgttaaagtggtgattctcggccaggatccttatcacggaccgggacaggcgcatggtctggcattttccgttcgtcccggcattgccattcctccgtcattattgaatatgtataaagagctggaaaatactattccgggcttcacccgccctaatcatggttatcttgaaagctgggcgcgtcagggcgttctgctactcaatactgtgttgacggtacgcgcaggtcaggcgcattcccacgccagcctcggctgggaaaccttcaccgataaagtgatcagcctgattaaccagcatcgcgaaggcgtggtgtttttgttgtggggatcgcatgcgcaaaagaaaggggcgattatagataagcaacgccatcatgtactgaaagcaccgcatccgtcgccgctttcggcgcatcgtggattctttggctgcaaccattttgtgctggcaaatcagtggctggaacaacgtggcgagacgccgattgactggatgccagtattaccggcagagagtgagtaaatttgcggggaaatgccggatggcagagttgccacccggctgatttatcaggctttattctgacgccaccattcaccaagcaaaacgccggttgcgacagagatattcagcccggcaacgttgcccgtaccgtcaatcttcacgcgcagatcgttcggatcgcgtgcggcatccggtaacccttcatattcctgacccagcaccagtaccattttcgctggcagactagttttgaacagcggtttaccctgctcgctggaagtggtcactacggtgtaacctgcctgacggaaatcatccagcacgttaacaatgttgtcgccagtaatcggctgaacgtgctctgcgccgccttctgcggtacggatagccgcccccgactccagcagtgccgcatcctgcaccacgacacctttcacgccgaagtgcgcgcagctgcgcatcatgccacccaggttatgcgggttagattcgttttccagtgccagaacgcaatcctgcgcgcctgcctggcttacccactgctgcacggttgtaccgttacgctttttgatcaagaagcaaacgccgccgtgatgttccgtgcctgacgcttttgtcaattccgcttcatccaccacatggtacgctttgcggtttgctgccatccagcgcaaagcttctttaaaacgcggcgttacactctggataaaccaggcgcgaacaatcgcttccggacggctctggaaaagtgcctgacatgcattttcgccgtagacgcgggtttcttccgcacgctgacgacgcaacacttccggatcaataaaacttttaccactgatgccaccgtgatcggccttttccggcgtctcatcacccggcgcgcgggaaaccgtgcgccacggcgaatcttcccacttgcggtcacggggctgactctgtttgtcatcgcgggcggggcgacggccaccgtcagcacgagattttcctggacgcccgccccctttcccggtacgcgggttgtgggtacgtttatcagaatcatcatcactgcggacatacatcactttgaccttgccgcttttacctttcatttcatcgttcatgcttttctccaccagcgctgcgcgaagcgcgcagattacccgaagtccgcgcggttcgccatgatttcgtaccaaagcctgcgactatcatacctattgaataaaacagattgttgtctggaacaatgtccccgataatatgtaacatattagaaacataccggcgtcgttgccgataagtctccttactcatcccgaggttagttatgaataccgtttgtacccattgtcaggccatcaatcgcattcccgacgatcggatcgaagatgcggcaaaatgcggacgctgcggtcacgacttgtttgacggagaggtgattaatgcgaccggtgaaacactcgacaaattgctgaaggatgatctacctgtggtgatcgacttctgggcaccgtggtgcggcccctgccgtaatttcgcaccaatttttgaagatgtcgcgcaagagcgtagcggtaaagtgcgctttgtgaaagtgaataccgaagctgaacgtgaattgagcagtcgctttggaattcgtagtataccgacgatcatgattttcaaaaacggtcaggttgtcgacatgcttaatggcgcagtaccgaaagcgccgttcgatagctggctgaacgaatctctttaatcttaccggggcgcatcttgtgccccgttttctcctctgcgacaatggcgttttttcgacgctctcttatgaccgaaaacgctgttctccagttacgcgccgagcgtattgcgcgcgcaacacgtccttttcttgcccgcggtaatcgcgttcgtcgctgccaacgctgtcttttgccagagaaattatgtctctgttcgacaattaccccagcacaagcaaaaagtcgcttctgtttgctgatgttcgacaccgagccaatgaagcccagtaataccgggcgtctcattgctgatattttgcctgataccgttgcgtttcaatggtcgcgtaccgaaccctcgcaggatttgctggagttggtgcaaaacccggactatcagccaatggtggtctttcccgcttcgtatgctgatgagcaacgggaagtgatcttcacaccacctgccggtaagccaccgctgtttatcatgctcgatggtacctggccggaagctcgcaagatgtttcgtaaaagtccgtatctggataatcttcccgtcatttccgtcgatctttcccggctttctgcctatcgcctgcgtgaagcccaggctgaaggccaatattgtactgccgaggtagccatcgcactgttagatatggccggcgataccggggcggcggcagggttaggcgagcattttacccgctttaaaacacgctatctggcaggaaaaacgcaacatctgggtagcatcacagcagaacagttagaaagcgtttaaaatcattcggtcacttctgcgggagaccggtatgagtcagcgaggactggaagcactactgcgaccaaaatcgatagcggtaattggcgcgtcgatgaaacccaatcgcgcaggttacctgatgatgcgtaacctgctggcgggaggctttaacggaccggtactcccggtgacgccagcctggaaagcggtgttgggtgtgttggcctggccggatattgccagcttgccctttacacccgaccttgcggttttatgtaccaatgccagccgtaatcttgctcttctggaagagctcggcgagaaaggctgtaaaacctgcattattctttccgccccggcatcgcaacacgaagatctccgcgcctgcgccctgcgccataacatgcgcctgcttggaccaaacagtctgggtttactggctccctggcaaggtctgaatgccagcttttcgcctgtgccgattaaacgcggcaagctggcgtttatttcgcaatcggctgccgtctccaacaccatcctcgactgggcgcaacagcgtaagatgggcttttcctactttattgcgctcggcgacagcctggatatcgacgttgatgaattgcttgactatctggcacgcgacagtaaaaccagcgccatcctgctctatctcgaacagttaagcgacgcgcgacgctttgtttcggcggcccgtagtgcctcgcgtaataaaccgattctggtgattaaaagcggacgtagcccggcggcacagcgactgctcaacacgacggcaggaatggacccggcatgggatgcggctattcagcgtgccggtttgttgcgggtacaggacacccacgagctgttttcggcggtggaaacccttagccatatgcgcccgctacgtggcgaccggctgatgattatcagcaacggtgctgcgcctgccgcgctggcgctggatgccttatggtcacgcaatggcaagctggcaacgctaagcgaagaaacctgccagaaactgcgcgatgcactgccagaacatgtggcaatatctaacccgctcgatctacgcgatgacgccagcagtgagcactatattaaaacgctggatattctgctccacagccaggattttgacgcgctgatggttattcattcgcccagcgccgctgctcccgcaacagaaagcgcgcaagtattaattgaagcggtaaagcatcatccccgcagcaaatatgtctctttgctgacgaactggtgcggcgagcactcctcgcaagaggcacgacgtttattcagcgaagccgggctgccgacctaccgtaccccggaaggaaccatcactgcttttatgcatatggtggagtaccggcgtaatcagaagcaactacgcgaaacgccggcgttgcccagcaatctgacttccaataccgcagaagcgcatcttctgttgcaacaggcgattgccgaaggggctacgtcgctcgatacccatgaagttcagcccatcctgcaagcgtatggcatgaacacgctccctacctggattgccagcgatagcaccgaagcggtgcatattgccgaacagattggttatccggtggcgctgaaattgcgttcgccggatattccacataaatcggaagttcagggcgtcatgctttacctgcgtacagccaatgaagtccagcaagcggcgaacgctattttcgatcgcgtaaaaatggcctggccacaggcgcgggtccacggcctgttggtgcaaagtatggctaaccgtgctggcgctcaggagttgcgggttgtggttgagcacgatccggttttcgggccgttgatcatgctgggtgaaggcggtgtggagtggcgtcctgaagatcaagccgtcgtcgcactgccgccgctgaacatgaacctggcccgctatctggttattcaggggatcaaaagtaaaaagattcgtgcgcgcagtgcgctacgcccattggatgttgcaggcttgagccagcttctggtgcaggtttccaacttgattgtcgattgcccggaaattcagcgtctggatattcatcctttgctggcttctggcagtgaatttaccgcgctggatgtcacgctggatatctcgccgtttgaaggcgataacgagagtcggctggcagtgcgcccttatccgcatcagctggaagaatgggtagaattgaaaaacggtgaacgctgcttgttccgcccgattttgccagaagatgagccacaacttcagcaattcatttcgcgagtcaccaaagaagatctttattaccgctactttagcgagatcaacgaatttacccatgaagatttagccaacatgacacagatcgactacgatcgggaaatggcgtttgtagcggtacgacgtattgatcaaacggaagagatcctcggcgtcacgcgtgcgatttccgatcctgataacatcgatgccgaatttgctgtactggttcgctcggatctcaaagggttaggcttaggtcgacgcttaatggaaaagttgattacctatacgcgagatcacggactacaacgtctgaatggtattacgatgccaaacaatcgtggcatggtggcgctagcccgcaagctcgggtttaacgttgatatccagctcgaagaggggatcgttgggcttacgctaaatcttgcccagcgcgaggaatcatgagtaaggtactggaaatgttgaccacttaatcgggactggtgttattattgcccgcttatgtcgtctgcattgcacagaggacccttcaatgaacagagaagaaatgcactgtgatgttgtcaaaatttaagcgtaataaacatcaacaacaccttgcccaactacccaagatttctcaatcagttgatgatgtcgatttcttttacgctcccgccgacttccgggagacgctgctggaaaaaatagccagcgcgaagcagcgcatttgcattgtcgccctgtatctcgaacaggatgacggtggcaaaggcattctgaacgcgttgtatgaggctaaaaggcagcgtccggaactggatgtgcgggtgctggtcgactggcatcgtgcacaacgtggacgcattggcgctgcggcatctaacactaacgctgactggtactgccgcatggcgcaggaaaatccgggcgtagatgttccggtttatggcgttccaatcaatactcgtgaagcccttggtgttctgcactttaaaggctttatcatcgacgatagcgtactttatagcggtgccagcctgaacgatgtttacctgcatcagcacgataaatatcgctacgaccgttatcatctgatccgtaaccgtaagatgtcagacattatgtttgaatgggttacacagaatattatgaatggccgcggcgttaatcgtctggatgatgttaatcggccaaaaagcccggaaatcaagaacgatattcgtctgttccgccaggagctgcgtgatgccgcttatcatttccagggcgatgccgacaacgatcagctttctgtaacgccgctagtggggctggggaaatcgagtctgttgaacaagaccattttccatcttatgccttgtgccgagcagaaactaaccatctgtacgccatacttcaacctgccagcaatccttgtgcgcaatattatccagttgctgcgcgaagggaaaaaggtcgaaattattgttggtgataaaaccgcgaatgacttctacattccggaagatgaacctttcaagataattggcgcattgccttatctctatgagatcaatctgcgtcgtttcctgagccgtttgcagtattacgtcaatactgaccagctagtggttcggttatggaaagatgacgacaacacctatcacctgaaagggatgtgggttgatgataagtggatgttgatcaccggtaataacctgaacccgcgcgcctggcgtctggatctggaaaacgccattttgatccacgatccgcaacttgagctggcgccacagcgagagaaagaactggagctgatccgcgagcataccaccatcgttaagcactatcgcgatctgcaaagtattgccgattatccggtgaaggttcgtaaactcatccgccgtttgcgccgtatccgcatcgaccgattaattagccgcatcctgtaatcacaaccccgtcctgtacggggtttgttttttggaggccacgttttgcgtattctttttgtctgttcgctattgttactttctggatgcagccatatggctaacgatagctggagcgggcaggataaagctcaacactttatcgcctcggcgatgctttccgccgccggaaatgaatattcacagcatcaggggatgagccgggatcgcagtgccatgtttggattgatgttctctgtcagtttgggggcgtcaaaagagctttgggatagccgccccgaagggagcggctggagctggaaggatttggcctgggatgtcgccggtgcaagcaccggctataccgtctggcaactgacccgtcactaaagacgcatccccttccctttgcgatgtagcatcaaagaaaccagaaacgccaccacggccatcaaggtcacataccagaagaaggctgtttccattcctattgatttcagcgacaacgctacgtactccgccgaaccaccaaatatagcattagcgaccgcatatgacagaccaacgcctaatgcgcgaacctgtgccgggaacatctcagccttcagtattccactgattgatgtataaaaactcactatcagcagggcacacatcaccagaccaaaagcggcataaggcgaggaaacgttttgcaatgctgagagaataggaacggtaaaaatggctgccagcgaaccgaaacataacattgaggtacggcgaccaatcttatccgacagcgcgccaatgagtggttgaataagcatgaatacaaacaatgcggcagtcataatgccactcgccacgttggcatgcattcccgcagtatttaccagatacttctgcatataagtagtgaaggtatagaaacaaagggagcccgcagcggtaaaaccgagaaccatgatgaatgcacggcgattgcgccataatcctttcagagatccagcttcttttaaagcgcgcgtttcttgttgcgaagtttcatctaactgacgacgtaaccacaacgccacaacagctaacacagctcctaacgcgaaaggaatacgccatccccactctctgagtgcagcgtcttccatggtgtgttgtaaaaccacgacaaccagtagggctagcagttgtccgccgatcaacgtcacatactgaaatgatgcgtaaaaacctttgcgcccttcaacggcaacttcactcatataggtggcgctggtgccatattctccgccaacagataatccctgaaataaacgagcgagaagcaataatgccggagcccacgtacctatagtttcataacctgggaggcaggcgataaccagcgatccgaaacacatcatacacaccgataacagcatcgattttttgcgaccatgtttatcggctatgcggccaaatagccaaccgcctattgggcgcatcaggaatcccgcagcaaaaacacctgctgtttgtagtagttgagtcgtcgtgttcccggaagggaagaagatgtgggcaaagtagagtgaacagaacgagtagacatagaaatcgaaccactcgaccagattacctgaagaggcccccacaatcgcccaaatgcggcgacgagtatcactacttgtcagtttgctgtctgccgttacagtactttcagccatgccattatgtctcctgccgtaatccgatgcttttgtcggtcgcttttgtttattttttttgtaaaggaaatattatacatttgttgcatatcattatgcaaccttaaccatgaatttagttagcaggaaaatggttattgaggagcttaaggataaatttctggtaaggaggacacgtatggaagtgggcaagttggggaagccgtatccgttgctgaatctggcatatgtgggagtataagacgcgcagcgtcgcatcaggcatttttttctgcgccaatgcaaaaaggccatccgtcaggatggcctttcgcataatttgatgcctggcagttccctactctcgcatggggagaccccacactaccatcggcgctacggcgtttcacttctgagttcggcatggggtcaggtgggaccaccgcgctacggccgccaggcaaattctgttttatcagaccgcttctgcgttctgatttaatctgtatcaggctgaaaatcttctctcatccgccaaaacagcttcggcgttgtaaggttaagcctcacggttcattagtaccggttagctcaacgcatcgctgcgcttacacacccggcctatcaacgtcgtcgtcttcaacgttccttcaggacccttaaagggtcagggagaactcatctcggggcaagtttcgtgcttagatgctttcagcacttatctcttccgcatttagctaccgggcagtgccattggcatgacaacccgaacaccagtgatgcgtccactccggtcctctcgtactaggagcagcccccctcagttctccagcgcccacggcagatagggaccgaactgtctcacgacgttctaaacccagctcgcgtaccactttaaatggcgaacagccatacccttgggacctacttcagccccaggatgtgatgagccgacatcgaggtgccaaacaccgccgtcgatatgaactcttgggcggtatcagcctgttatccccggagtaccttttatccgttgagcgatggcccttccattcagaaccaccggatcactatgacctgctttcgcacctgctcgcgccgtcacgctcgcagtcaagctggcttatgccattgcactaacctcctgatgtccgaccaggattagccaaccttcgtgctcctccgttactctttaggaggagaccgccccagtcaaactacccaccagacactgtccgcaacccggattacgggtcaacgttagaacatcaaacattaaagggtggtatttcaaggtcggctccatgcagactggcgtccacacttcaaagcctcccacctatcctacacatcaaggctcaatgttcagtgtcaagctatagtaaaggttcacggggtctttccgtcttgccgcgggtacactgcatcttcacagcgagttcaatttcactgagtctcgggtggagacagcctggccatcattacgccattcgtgcaggtcggaacttacccgacaaggaatttcgctaccttaggaccgttatagttacggccgccgtttaccggggcttcgatcaagagcttcgcttgcgctaaccccatcaattaaccttccggcaccgggcaggcgtcacaccgtatacgtccactttcgtgtttgcacagtgctgtgtttttaataaacagttgcagccagctggtatcttcgactgatttcagctccatccgcgagggacctcacctacatatcagcgtgccttctcccgaagttacggcaccattttgcctagttccttcacccgagttctctcaagcgccttggtattctctacctgaccacctgtgtcggtttggggtacgatttgatgttacctgatgcttagaggcttttcctggaagcagggcatttgttgcttcagcaccgtagtgcctcgtcatcacgcctcagccttgattttccggatttgcctggaaaaccagcctacacgcttaaaccgggacaaccgtcgcccggccaacatagccttctccgtccccccttcgcagtaacaccaagtacaggaatattaacctgtttcccatcgactacgcctttcggcctcgccttaggggtcgactcaccctgccccgattaacgttggacaggaacccttggtcttccggcgagcgggcttttcacccgctttatcgttacttatgtcagcattcgcacttctgatacctccagcatgcctcacagcacaccttcgcaggcttacagaacgctcccctacccaacaacgcataagcgtcgctgccgcagcttcggtgcatggtttagccccgttacatcttccgcgcaggccgactcgaccagtgagctattacgctttctttaaatgatggctgcttctaagccaacatcctggctgtctgggccttcccacatcgtttcccacttaaccatgactttgggaccttagctggcggtctgggttgtttccctcttcacgacggacgttagcacccgccgtgtgtctcccgtgataacattctccggtattcgcagtttgcatcgggttggtaagtcgggatgacccccttgccgaaacagtgctctacccccggagatgaattcacgaggcgctacctaaatagctttcggggagaaccagctatctcccggtttgattggcctttcacccccagccacaagtcatccgctaatttttcaacattagtcggttcggtcctccagttagtgttacccaaccttcaacctgcccatggctagatcaccgggtttcgggtctataccctgcaacttaacgcccagttaagactcggtttcccttcggctcccctattcggttaaccttgctacagaatataagtcgctgacccattatacaaaaggtacgcagtcacacgcctaagcgtgctcccactgcttgtacgtacacggtttcaggttctttttcactcccctcgccggggttcttttcgcctttccctcacggtactggttcactatcggtcagtcaggagtatttagccttggaggatggtccccccatattcagacaggataccacgtgtcccgccctactcatcgagctcacagcatgtgcatttttgtgtacggggctgtcaccctgtatcgcgcgcctttccagacgcttccactaacacacacactgattcaggctctgggctgctccccgttcgctcgccgctactgggggaatctcggttgatttcttttcctcggggtacttagatgtttcagttcccccggttcgcctcattaacctatggattcagttaatgatagtgtgtcgaaacacactgggtttccccattcggaaatcgccggttataacggttcatatcaccttaccgacgcttatcgcagattagcacgtccttcatcgcctctgactgccagggcatccaccgtgtacgcttagtcgcttaacctcacaacccgaagatgtttcacttcagagttgcgaaaatttgagagactcacgaacaactttcattgttcagtgtttcaattttcagcttgatccagatttttaaagagcaaatatatcaaacaagacttaacagtctgttttgagatattgaggtcggcgactttcactcacaaaccagcaagtggcgtcccctaggggattcgaacccctgttaccgccgtgaaagggcggtgtcctgggcctctagacgaaggggacacgaaaattgcttatcacgcgttgcgtgatattttcgtgtagggtgagctttcattaatagaaagcgaacggccttattctcttcagcctcactcccaacgcgtaaacgccttgctattcacttttcatcagacaatctgtgtgagcactgcaaagtacgcttctttaaggtaaggaggtgatccaaccgcaggttcccctacggttaccttgttacgacttcaccccagtcatgaatcacaaagtggtaagcgccctcccgaaggttaagctacctacttcttttgcaacccactcccatggtgtgacgggcggtgtgtacaaggcccgggaacgtattcaccgtggcattctgatccacgattactagcgattccgacttcatggagtcgagttgcagactccaatccggactacgacgcactttatgaggtccgcttgctctcgcgaggtcgcttctctttgtatgcgccattgtagcacgtgtgtagccctggtcgtaagggccatgatgacttgacgtcatccccaccttcctccagtttatcactggcagtctcctttgagttcccggccggaccgctggcaacaaaggataagggttgcgctcgttgcgggacttaacccaacatttcacaacacgagctgacgacagccatgcagcacctgtctcacggttcccgaaggcacattctcatctctgaaaacttccgtggatgtcaagaccaggtaaggttcttcgcgttgcatcgaattaaaccacatgctccaccgcttgtgcgggcccccgtcaattcatttgagttttaaccttgcggccgtactccccaggcggtcgacttaacgcgttagctccggaagccacgcctcaagggcacaacctccaagtcgacatcgtttacggcgtggactaccagggtatctaatcctgtttgctccccacgctttcgcacctgagcgtcagtcttcgtccagggggccgccttcgccaccggtattcctccagatctctacgcatttcaccgctacacctggaattctacccccctctacgagactcaagcttgccagtatcagatgcagttcccaggttgagcccggggatttcacatctgacttaacaaaccgcctgcgtgcgctttacgcccagtaattccgattaacgcttgcaccctccgtattaccgcggctgctggcacggagttagccggtgcttcttctgcgggtaacgtcaatgagcaaaggtattaactttactcccttcctccccgctgaaagtactttacaacccgaaggccttcttcatacacgcggcatggctgcatcaggcttgcgcccattgtgcaatattccccactgctgcctcccgtaggagtctggaccgtgtctcagttccagtgtggctggtcatcctctcagaccagctagggatcgtcgccttggtgagccgttaccccaccaacaagctaatcccatctgggcacatccgatggcaagaggcccgaaggtccccctctttggtcttgcgacattatgcggtattagctaccgtttccagtagttatccccctccatcaggcagcttcccagacattactcacccgtccgccactcgtcagcgaagcagcaagctgcttcctgttaccgttcgacttgcatgtgttaggcctgccgccagcgttcaatctgagccatgatcaaactcttcaatttaaaagtttgatgctcaaagaattaaacttcgtaatgaattacgtgttcactcttgagacttggtattcatttttcgtcttgcgacgttaagaatccgtatcttcgagtgcccacacagattgtctgataaattgttaaagagcagtgccgcttcgctttttctcagcggcgcggggtgtgcataatacgccttcccgctacagagtcaagcatttctttgcttttctctgttgagattctcaggagaaccccgccgacccggcggcgtgtttgccgttgttccgtgtcagtggtggcgcattatagggagttattccggcctgacaagcgaaaaatataaaaactttatcgttcgctcacttttcaggcaaaacatcttaaatatagtcttttccgtctaacttatagacaaaaacgagccccgaagggctcgttttatcatttactggacggcgacaatccggtcttcattaacttccaggcgaatcactttacccggaaccaattcaccagacagtatttgctgtgccagcgggttttcgatctgctgctgaattgcacgtttcagaggacgtgcaccatagaccggatcgtaaccgttctcgctcagcagtttcagcgcctcgtcagaaatgtggatttcataaccacgttcttccagacgtttgtacagacgtttcaactgaatctgcgcaatcgaggcaatgtgctgttcacccagcggatggaagaccaccacttcatcgatacggttaatgaattccggacggaagttatggcttaccacaccgagcaccagctctttcatgtgcgcataatccagttcaccgaagcgttcctgaatcagatcggaaccgaggttagaggtcataatgacgaccgtattacggaagtcgaccgttctcccttgcccgtcagtcagacgcccatcatccagtacctgcaacagaatgttgaagacatccggatgcgctttttccacttcatccagcaggatgacggaatacggacgacgacgcaccgcttcggtcaggtagccaccttcttcataaccgacatatcccggaggcgcaccaaccaaacgagacaccgagtgtttctccataaactcggacatatcgatacggaccatcgcctcgtcgctatcaaacataaagttcgccagcgccttacaaagctctgttttccccacaccagttgggccgaggaacaggaatgaaccaatcgggcgatttggatccgccagccccgcacggctacgacgaatagcgttagataccgcatcaaccgcttcgttctgaccaattacgcgatggtgcagttcttgctccatacgcagcagtttttcgcgctcgctttccatcatgcgagaaaccggaatccccgtccaacgcgccagcacttcagcaatttcggcgtcggtcactttattacgcaacagacgcatagttttgccttcgagctgcgttgcggcttccagttgcttttccagttccgggattttgccgtattgcagttcagacatccgcgccaggtcccccacacggcgagcctgttcaatagcgattttcgcctgttccagttccgctttaatggtctgcgtaccagaaagcgatgccttctctgctttccactcttcttctaactcggagtactgacgttctttgtcgctcagttcttcgttgagcatatccagacgttttttactggcttcatcagactctttcattaacgcctgttgttccagtttgagctggatgatacgacgatcgagtcggtcgagttcttctggttttgagtcaatctgcatacgaatgctggatgctgcttcatcgatcaggtcgatggctttatccggcagctgacggtcagcaatgtagcgatgagacaacgtcgccgctgcaacaattgccgggtcagtaatttgcacatggtggtgcaattcgtaacgttctttcaggccacgcagaatcgcaatggtatcttcaacagaaggctcggcaacaaacactttctggaaacgacgttccagcgcagcatctttttcaatgtactggcgatattcgtcaagcgtcgtggcacctacgcagtgcaattcaccacgcgccagcgccggtttcagcatgtttccggcgtccattgcgccatcggctttacccgcgccgaccatggtatgtaattcgtcgataaataggatgacgttgccttcctgtttggcaagatcgttaagcacgccttttaaacgttcttcaaactcaccgcgatatttcgccccagccaccagcgcgcccatatccagcgccagtacccggcggcctttcaacccttccggcacttcgccgttgataatacgctgcgccagaccttcaacgatggcagttttaccgacgccgggttcaccaatcagtaccgggttatttttagtacgacgttgcagcacctgaatggtacggcgaatttcttcatcacgaccaatcaccggatcgagtttgccctgttcggctcgttcggtaaggtcgatggtatattttttcaaagcctgacgttggtcttcagcaccttgatcgttcacgctttcacctccacgcatttgttcaatcgcttgagtaatgttggcggtggtcgcccctgctgctttcaggatgtcggccagcgtgccgcgagactcaagtgccgccagaacgaacagttctgacgagataaagttatcaccacgtttttgcgccagcttgtcgcaaagattaagaacgcgcaccagatcctgtgatggctggacatcaccaccagtaccttcaacctgcggtaaacgatttaatgcctgattgatatctgtgcgcaactggccagcatttatgccagcggatgttaataaaggactaaccgaacccccttcctgattcagcagggcgctcattaaatgaagtggttcgataaattggttgtcgtgcccgagtgcaagtgattgggcatcggcaagagcaagctggaatttattagtaagacgatccagacgcataactcctcccataacggatcaaagttgctactggagattaaatgaggtcatccctcaattattcaaggttattgaccagattaatgtgaaaagaaaatcacgcgtaccggatcgtcttgattctttaggttatatcagccaaatgaaacttgccatacgaccggtggtcttgtcgcgacgataagagaagaaagtctcattttccgtatatgtacaacggtcgccgccgaaaatttgctcaacacccacgttcgccagacgctgccgggcaagctgataaatatccgccagatacttatcaccatgctgaatgaaagctgcacttgctttagcgtctactgccataaacgcctcgcgaacctccccccccacttcgaacgcgcgtggaccaattgccggccctaaccaggcgagaatattttccggattatcagcaaaacaggaaaccgtctcttccagcacgcctgcgcacagtccacgccagccagcatgagcggcggcgacttccgttcccgctcgattgcaaaacagcacagggaggcagtcggcagtcatcactgcgcaaaccgtgccgggcgtattgctataagaggcatccgcccgttttgaggcataaggttcgccagtgagcttaagcacatctttgccgtgtacctgctcaagccagaccggtttagaaggcaaattgcccgcagcaaaaagtcgcttgcgattctcctcaacgtgatccgggttatcgccacaatgggcaccgaggttgagtgagtcatacgggggcaagctcacgccgccgatacgagtggagctacaggccgcaacaccttttggctgcggccactgcgggacaatcagcttactcataaccagtccacttcatccttatgttcttcgaaatcggcgcgcatcacctcaatcagctccaccatatcttgtggaataggcgcatgccattccatttcgatgccggagatcgggtgataaagacgcagcatggttgcatgtagcgcctggcggtcaaacttacgcagcgtggagataaatgcttccgaagcaccttttggcggacgcggacggccaccataaaccggatcgcccaccagcggatgagtgatatgggccatatgcacgcggatctggtgcgtacgtccagtttccagacgcaaccgcagacgcgtgtgcacacggaagtgttccatgatgcgatagtgagtcaccgctggtttgcccatcggatgcaccgccatatgggtacgtttggtcgggtggcgactgattggctcgtccaccgtgccacctgcggtcatatgaccaatcgccaccgcttcatactcacgagtaatttcacgccgttgcaaagattcgactaaacgcgtctgagccggaacggtttttgccacaaccatcaggccagtggtgtctttatccagacgatggacgatgcccgcacgcggtacatcggcaatgggtggatagtaatgaagcaacgcattcagtaccgtgccatccgggttacccgcgccaggatgtaccaccaggtcgcgcggtttattaatgataataatgtcttcatcttcatagacgatatccagcgggatatcctgcggttcaaaacgcgcttcttcttcaatctcagcgttgatggcaacctgctcgccacccaatactttttctttcggcttatcacaaactttgccgttaaccagcactcgctggtcgaggatccattcttttattcgcgaacgtgaataatccgggaacatttcggccaaagcctgatctaagcgttgaccgagttggttttcggacaccgttgcagtgagctgtactcgttgtgccatatatactgcttcttcgtttatcgttggggttttacggctttgccgtttaatatagtgtgctattgtagctggtcttaaccgggagcaggaacagagaatctcccgtattacattttgaggaaagtcaaaacgtcatgacgcgcatgaaatatctggtggcagccgccacactaagcctgtttttggcgggttgctcggggtcaaaggaagaagtacctgataatccgccaaatgaaatttacgcgactgcacaacaaaagctgcaggacggtaactggagacaggcaataacgcaactggaagcgttagataatcgctatccgtttggtccgtattcgcagcaggtgcagctggatctcatctacgcctactataaaaacgccgatttgccgttagcacaggctgccatcgatcgttttattcgccttaacccgacccatccgaatatcgattatgtcatgtacatgcgtggcctgaccaatatggcgctggatgacagtgcgctgcaagggttctttggcgtcgatcgtagcgatcgcgatcctcaacatgcacgagctgcgtttagtgacttttccaaactggtgcgcggctatccgaacagtcagtacaccaccgatgccaccaaacgtctggtattcctgaaagatcgtctggcgaaatatgaatactccgtggccgagtactatacagaacgtggcgcatgggttgccgtcgttaaccgcgtagaaggcatgttgcgcgactacccggatacccaggctacgcgtgatgcgctgccgctgatggaaaatgcataccgtcagatgcagatgaatgcgcaagctgaaaaagtagcgaaaatcatcgccgcaaacagcagcaatacataacagaaacctgaaacacaaaacggcagcccttgagctgccgtttttttattctgtcagttgtgaaactgaagcgatttagtcgctatcgatctcatcaaatatggctcgctttgagatattcctcaagtaaaaaaacatctcttcctgcgatttctcacaaaaaagattcgttgacaaaaagtgacaaaattatgagattttcatcacacattttgacatcaggaacggtatgctgaattcaccaagacgggaagacaagaggtaaaatttatgacaatgaacattaccagcaaacaaatggaaattactccggccatccgccaacatgtcgcagaccgtctcgccaaactggaaaaatggcaaacacatctgattaatccacatatcattctgtccaaagagccacaagggtttgttgctgacgccacaatcaatacacctaacggcgttctggttgccagtggtaaacatgaagatatgtacaccgcaattaacgaattgatcaacaagctggaacggcagctcaataaactgcagcacaaaggcgaagcacgtcgtgccgcaacatcggtgaaagacgccaacttcgtcgaagaagttgaagaagagtagtcctttatattgagtgtatcgccaacgcgccttcgggcgcgttttttgttgacagcgtgaaaacagtacgggtactgtactaaagtcacttaaggaaacaaacatgaaacacataccgtttttcttcgcattcttttttaccttcccctgaatgggaggcgtttcgtcgtgtgaaacagaatgcgaagacgaacaataaggcctcccaaatcggggggccttttttattgataacaaaaaggcaacactatgacatcggaaaacccgttactggcgctgcgagagaaaatcagcgcgctggatgaaaaattattagcgttactggcagaacggcgcgaactggccgtcgaggtgggaaaagccaaactgctctcgcatcgcccggtacgtgatattgatcgtgaacgcgatttgctggaaagattaattacgctcggtaaagcgcaccatctggacgcccattacattactcgcctgttccagctcatcattgaagattccgtattaactcagcaggctttgctccaacaacatctcaataaaattaatccgcactcagcacgcatcgcttttctcggccccaaaggttcttattcccatcttgcggcgcgccagtatgctgcccgtcactttgagcaattcattgaaagtggctgcgccaaatttgccgatatttttaatcaggtggaaaccggccaggccgactatgccgtcgtaccgattgaaaataccagctccggtgccataaacgacgtttacgatctgctgcaacataccagcttgtcgattgttggcgagatgacgttaactatcgaccattgtttgttggtctccggcactactgatttatccaccatcaatacggtctacagccatccgcagccattccagcaatgcagcaaattccttaatcgttatccgcactggaagattgaatataccgaaagtacgtctgcggcaatggaaaaggttgcacaggcaaaatcaccgcatgttgctgcgttgggaagcgaagctggcggcactttgtacggtttgcaggtactggagcgtattgaagcaaatcagcgacaaaacttcacccgatttgtggtgttggcgcgtaaagccattaacgtgtctgatcaggttccggcgaaaaccacgttgttaatggcgaccgggcaacaagccggtgcgctggttgaagcgttgctggtactgcgcaaccacaatctgattatgacccgtctggaatcacgcccgattcacggtaatccatgggaagagatgttctatctggatattcaggccaatcttgaatcagcggaaatgcaaaaagcattgaaagagttaggggaaatcacccgttcaatgaaggtattgggctgttacccaagtgagaacgtagtgcctgttgatccaacctgatgaaaaggtgccggatgatgtgaatcatccggcactggattattactggcgattgtcattcgcctgacgcaataacacgcggctttcactctgaaaacgctgtgcgtaatcgccgaaccagtgctccaccttgcggaaactgtcaataaacgcctgcttatcgccctgctccagcaactcaatcgcctcgccgaaacgcttatagtaacgtttgattaacgccagattacgctctgacgacataatgatgtcggcataaagctgcggatcctgagcaaacagtcgcccgaccatcgccagctcaaggcggtaaatcggcgaagagagcgccagaagttgctcaagctgaacattttcttctgccaggtgcagcccgtaagcaaaagtagcaaagtggcgcagtgcctgaataaacgccatattctgatcgtgctcgacggcgctaatacgatgcagccgagcgccccagacctgaatttgctccagaaaccattggtatgcttccggtttacgtccatcacaccagaccacaacttgctttgccaggctaccgctgtccggaccgaacatcgggtgtagccccagcaccggaccatcatgcgccaccagcatggcctgtaatggcccatttttcactgatgccagatcgaccagaatacaatctttcggtaaaggcggtaatttgccaataacttgctcagtaacgtggattggcacactaacaatcaccattccggcatcggcaacaatatcagccgctcgatcccagtcatgttgctccagaatccgcacctgataacccgagagggtcagcatcttctcgaacaggcgtcccatctgaccgccaccgccgacgataaccaccggacgcagtgacggacaaagtgttttaaatcctttgtcgttttcactggagtaagattcacgcatcacccgacgcaaaacatcctcaatcagatctggcggtacacccagagcttccgcctctgcacgacgcgaggccaacatagatgcctcgcgctccggaacataaataggcagtccaaagcggcttttcacctcgcccacttcagcaaccagttccagacgcttcgctaataaattcagcagcgctttatcgacttcatcaatttgatcgcgtaatgcggtcaattcagcaaccataataaacctcttaagccacgcgagccgtcagctgcccgttcagatcctgatgaatttcacgcagcaaggcatcggtcatttcccagctaatgcaggcatcggttacggatacaccgtatttcatttcactgcgcggttgctcggaagactgattgccctcgtggatattactttcgatcatcagaccaataattgagcgattgccatctttgatttgagcaaccacggattctgccaccgcaggctgacggcgataatctttattggaattaccgtggctgcaatctaccatcagagacgggcgcagtcccgcctgttccatctctttttcacattgcgcaacatccgcagggctatagttcggcgctttaccaccgcgcaggatcacatggccgtccggattcccctgagtttgtagcaacgcaacctgccctgcctggttaatgccaacaaaacggtgcggctgggcggcggcgcgcatagcgttaattgctgttgccagactgccgtcggtgccgtttttaaaaccaaccggcatggaaagcccggaggccatttcacggtgagtttgcgattccgttgtacgagcaccaattgctgaccagctaaacagatcgcccaggtattgcgggctattcggatctaacgcttccgtcgccagtggcagtcccatattcaccagctcaagcagcaatttacgcgcgatctgcagcccggcttctacatcaaaagagccatccatatggggatcgttaattaaccctttccagccgacagtggtacggggtttttcaaaatagacgcgcattaccagatagaggctatcgctgacctctgcggcaagggctttaaatcgacgagcatattccagagcagtttccggatcatgaatggaacaaggaccacatactaccagcagacgaggatcgcgcccggcgataatatctgaaatgcttttacgcgagtcagcaatctgggcttcttgttgcaggctcaatggaaaagcggccttcagttgttccggagtcattaaaacctgttcgtcggtaatatgtacgttattcagcgcgtctttttgcatgatggcgatcctgtttatgctcgtttgcgatagttgatcctcagcgaggatgacgtaacgataacacataaagtaaagttttcaatccatatttcgtacatttttatttacacaggcaatttagtcgcgctttcaacccttacctctgtatagataaatttacactccctttgaaaacaatccgctatgctttgaaaaaggagaaagaaatgatgaaaaagtttatcgcccccttgttggctttactggttagcggatgtcagattgatccttatactcacgcgccaaccttgaccagcaccgactggtatgatgtcggtatggaagatgcgatatcgggcagcgccataaaagatgacgatgcatttagcgattcacaggcggatcgcggtctataccttaaaggatatgccgaaggacaaaagaaaacttgccagaccgattttacttatgcccgaggactttccggtaaaagctttcctgccagctgcaacaatgttgaaaatgccagccaactgcatgaagtatggcaaaaaggggctgatgaaaatgccagcacaatacgattaaattaattaaaaccccacaaataaattaaacataagattttactcattgtgttttatttctcacattgatgacggtcgcatgaaaaaatgatattttaatgagcattctgaaaaaatatcgatgcatttcgagcgaagatggtggggatccctgaatgcgtttttctcaccgactgttcttacttctgattctcctgctgacgggagcaccaatactcgctcaggagccttctgacgttgcgaaaaacgtgcgtatgatggtttccggtattgtcagttacacccgctggcctgcgctatcagggccaccaaagttatgtatcttttcatcttcacgttttagtaccgccctacaagagaatgccgcgacatctttgccttatctgcctgtcatcattcacactcaacaagaggcgatgatttcaggctgcaatggtttttattttggcaacgagtcaccgacattccagatggaattaaccgaacaatatccgtcaaaggcgttattattaattgccgaacaaaataccgagtgcattattggtagcgccttttgtctgatcatccacaataatgacgtcagatttgccgtaaacctggatgccttatcgcgtagcggtgtaaaggtcaacccggatgtcttaatgctcgcacggaagaaaaatgatggataacgataattctcttaataagcgccccacgtttaaaagagcattacgcaacatcagtatgaccagcatatttatcactatgatgctgatctggttgctgctttccgtgacctcggtgctgaccctgaaacagtacgcgcaaaaaaacctggcactgacagcagcaacaatgacttacagtctggaagcagctgtcgtttttgccgatggccctgcagcaactgaaacactggcagcgctgggccagcaagggcaattttcaactgcagaagtacgtgataagcagcaaaatattctggcatcctggcattacacccgtaaggatccaggcgatactttcagtaatttcataagccactggctcttccctgcccccatcattcagccgattcgtcacaatggtgaaaccattggcgaagtacgcttaaccgctcgcgacagttcaatcagccattttatctggttttcgctcgccgtactgaccggttgtattctgctggcatcaggcatcgcaattaccctcacccgccatttgcacaatggcctggtagaagcgctgaaaaatatcaccgatgtcgtacatgatgtgcgttccaaccgcaatttttcccgacgagtttcggaagaacgtatcgctgagtttcaccgcttcgctctcgacttcaacagtctgctggatgaaatggaagagtggcagcttcgtttacaggctaaaaatgcgcagcttctacgtaccgcgctacatgacccattaaccgggctggctaaccgcgcagcgtttcgtagcggcatcaacacgttgatgaacaattccgatgcccgaaaaacgtcggcgttactatttcttgatggcgataatttcaaatacatcaatgatacctggggtcatgcgacgggcgatagagtcttgattgaaatcgcaaaacggttagctgaatttggcgggctgcgacataaagcataccgcctgggcggcgatgaattcgctatggtgctctatgatgtacagtcggaatctgaagtgcagcagatatgttcagcactgacacaaatctttaatctcccgtttgatcttcataatggccatcagaccaccatgacattaagcattggttacgcgatgaccattgagcacgcctctgcggaaaaattacaagagcttgccgatcacaatatgtatcaggccaaacaccagcgtgccgaaaagctggtgagataacaaggatatatcgatatgataaagcacctggtagcacccctggttttcacctcactaatactgactggctgccagtcccctcagggaaagtttactcctgagcaagtcgccgctatgcaatcttatggatttactgaatccgccggcgactggtcgctgggcttatcagatgccattctgttcgcaaaaaatgactacaaattgctcccggaaagccagcaacagatccaaaccatggcagctaaattggcctcgacagggctaacacatgcccgtatggatggacacaccgataactatggtgaagacagttacaacgaaggcttatcattgaaacgggcgaatgtcgtggccgatgcatgggctatgggtggacaaattccacgcagcaatctcaccacacagggtttaggaaaaaaatatcccatagccagtaacaagaccgcccagggccgcgccgagaaccgccgcgtcgcagtggtgattactaccccttaaaacaccagcaaacagataaaaaagggccagccaattggccagcccttcttaacaggatgtcgcttaagcgaaatcttagttaagacgctctttgatacgagcagccttaccagtacgctcacgcaggtagtacagtttagctttacgaacagcaccacgacgtttgacagaaatgctgtcaactaccggagagtgagtctggaagacacgctcaacgccttcgccgttggaaattttacgaacagtgaatgcagagtgcagaccgcggttacgaatagcgataaccacgccctcgaatgcctgcagacgttttttggaaccttcaacaacccatactttcacttccacggtatcacccggacggaaggaaggtacgtcctgcttcatctgctcttgttcaagttgcttaataatgttgctcataatttaatctcttatcctgggtaaactgatatctcgggggcttacgccatcccatcatgtttatgttgctgttgtgcgtgttccgttttgaactccgccagcaaccttgcttgctcttcagtcagagccaggttttccagaagttcaggtcttctaagccaggtacggcccagcgactgtttcaaacgccagcgacgtatctcggcatggttgcccgacagtaacactggcggaacttccatcccttctaacacctcaggccgcgtatagtgcgggcaatccagcaatccttcagcaaaggaatcttccgttgccgaggcttcatgtcccagtactcccggaataaaccgggaaacggagtcaatcagcgtcattgctggtaactcaccaccactgagaacgtaatcgccgattgaccattcttcgtcaatttcggtttggatcacgcgctcatctataccttcgtagcgaccgcacaccagaatcaatttttgattcgttgccagttcgctgacgcccgcttgatcaagcttgcgtccctgtggtgacagataaatcacctttgcgccttcacccgccgcggcttttgctgcatgaatggcgtcccgcaagggttgcaccatcattaacatccccggtccgccgccgtaaggacgatcgtccacggtacggtgccggtcatgcgtgaagtcgcgaggactccagctctggatgctcagcaggccatttttaactgcccggccagttaccccgtaatcggtaattgcgcggaacatttcaggaaacaggctaattatgccaatccacatagcgccgtcttttaccgtttatccggtggtttaaaaaccaggatcccaatctacttcgattgaacgagtagtgagatcgactttcttgataacctgcccatcgaggaacggtacgagacgttccttgataccaaacgcatctttcaggtttgccttaatgacgagaacgtcattagatccggtttccatcatatcgacgactttaccgagatcgtagccttcagtggttactacctggcagcccatcaggtctttccagtagtagtccccctcttcaagctgaggcagctgcgatgaatccacgacaatttcacaattcgtcagcaggttcgccgcatcacgatcgtcaacgcctttcagcttgatgatcatgtcctgattgtggtgcttccagctttccagctggacttgctgccactgacccgccttctggataaaccagggctgatagtcaaaaatgctttcggcgtcttcggtggaagaaaacactctgagccacccacgaataccgtaagacgaacccatttttcccaaaacgatgggatcaacaggtgcttgcgcggtgagttgtttgctcatcatgaccaccgtgacagattaagctgctttgtttacttctttgatcagcgcagcaacgcgatcagaaatagttgcgccctggccaacccagtgagcgatgcgatccagatccaggcgagtgccttcttctttttcgctagcgattgggttgaagaaaccaacgcgctcgatgaagcgaccgttgcgtgcattacggctgtcagcgacaacaacctggtagaacggacgctttttagcgccgtgacgtgctaaacgaatagttaccataacatcctcttgtgtgaataaaacaaccggaccccatcgaggaacggagtccggtgtcatattaaaagcccgaaaattttactcatttttgcgggaattgcaatcaacagttgctaactctgctgtaaaaggccgtcggcggtgcagccagtttggtgccggagtgcgcgcagtcaccggagcgtacacgcagtacgtgaggatgacgagcacatcccggtgccaaaatggcaaacaagccaggccgattagcgaccagggaagcctgggggcatcatacccttcatgcttctcatcatcttcgccattccgcccttcttcattttcttcatcatgcgctgcatgtcgtcgaactgtttcagaagacggttaacgtcctgcacctgcataccgcaaccggcagcaatacggcgtttacgcgaacctttgatgatttctggcttagcgcgctctttcatcgtcatcgagttgatgatggcttccatacgcaccagcactttatcgtccatctgtgacttgacgttatccgggatctgccccatgcccggcagcttgcccatcagactagccatgccgcccatatttttcatctggcgcagctgctcaagaaagtcgttgagatcgaagccgtcaccttttttcagcttgctggctaatttctctgcctgcgcgcggtcaactttgctttcgatatcttcgatcagcgacagtacgtcgcccatgccgagaatacgcgacgcgatgcggtccggatggaacggctccagcgcctcagttttctcgccaacaccgaggaacttgatcggtttgccagtgatgtgacgaatagagagcgccgcaccgccgcgggcatcgccgtccactttggtcaacactacgccggtaagcggtaacgcttcattgaatgcttttgccgtattggccgcatcctgaccggtcatggcgtcaaccacaaacagggtttcaaccgggttaatcgacgcatggacttgtttgatctcgtccatcatcgcttcgtcaacgtgcagacgaccagcggtatccaccagcagcacgtcgtagaatttcagtttggcttctttcagcgccgcgttaacgatatctaccggcttctgaccaacatcagaagggaagaaatcaacgcccacctgctctgccagcgtctcaagctgtttgattgccgccgggcgataaacgtcggcagaaaccaccagcactttcttcttgtgcttctcgcgcaggaacttaccgagtttaccaacgctggttgttttaccggcaccttgcaggcccgccatcagtacgaccgcaggcggttgcgcagccaggttcagggtctggttctcttcgcccatcgccgcaaccagttcgttacggactattttgacgaactcctgccccggcgtcaggctcttattaacttcatgaccaaccgctttctcttttacgcgattgataaactcacgcactaccggcagagctacgtccgcctccagcagcgccatgcgcacttcgcgcagcgtatcttttacgttgtcttcagtgaggcgtccacggccactgatattgcgcagcgtgcgcgacaaacgatcggttaaattatcaaacattgtctctcgcctggggtggaaacggttggccgcaatcgcgacacatcatcagtattttgccgcagtataacatgaaggcgtctttgttgttatgcaacggttggagcagcgttcacctgacgctatactgcttctctttcttattgctcaaactgtcgacatcactatgcccgtttttgctctgctcgcgcttgtcgcctactccgtcagtcttgcgctgattgttcccggtctgctgcaaaaaaacggcggctggcggcgcatggctattatttctgcggtcattgcgctggtctgccacgcaatcgctctggaagcccgcatcctgcccgacggtgatagcggacaaaacctcagcctgctgaacgttggttcattggtcagtttgatgatctgtacggtaatgaccattgtggcttctcgcaatcgtggctggctgctgctacccattgtctatgcctttgcgcttatcaacctggcgctggcaaccttcatgcccaatgaatacatcacccatctggaagctacgcctgggatgctggtgcacattggcttatcgctcttttcctatgccacgctaattatcgccgccctgtacgcgctgcaactggcgtggattgattaccaactgaagaacaagaagctggcgtttaaccaggaaatgccgccattgatgagtatcgagcgtaaaatgttccacatcacgcagattggcgtggtgctgctaacgctcacgctttgcactggcctgttctacatgcacaacttatttagcatggaaaatatcgacaaggctgtgctctctatcgtggcgtggtttgtctatattgtgctgctgtggggacattatcatgaaggatggcgtggacgccgcgtcgtctggtttaacgttgcgggcgcggtaattctgacactggcctacttcggcagccgaattgtccagcagttaatcagctaaacccagaaaaggagtttcccctggaacacatttctactactacgttgatcattattctgatcatcatggtggtcatttcagcctatttttccgggtccgaaaccggaatgatgaccctcaaccgctatcgtctgcgacatatggcgaaacagggtaatcgctcggccaaacgcgtcgaaaaattgctgcgtaagccagaccgcctgataagcctggtgttaatcggcaataacctggtcaatattcttgcctccgcgctcggcactattgttgggatgcgtttgtacggcgatgcgggcgtggcaattgcgactggtgtgctgacttttgtcgtactggtatttgctgaggtattgccgaaaaccattgccgcgctgtacccggaaaaagtcgcttatccgagtagttttctgctggctccgctgcaaattttgatgatgccgctggtctggttgctgaatgctatcacccgtatgctgatgcgcatgatgggtatcaaaaccgatatcgtggttagcggctctttgagcaaagaagagttgcgcactatcgtgcacgaatcacgctcacaaatttcccgtcgcaatcaggatatgctgctgtcggtgctcgatctggaaaaaatgaccgttgatgacatcatggtgccgcgcagtgaaattatcggtattgatatcaacgatgactggaaatcgattctgcgccaactctcccactcacctcacgggcgcatcgtgctctaccgtgattcgctggacgacgccatcagtatgctgcgagtacgtgaagcctggcggttgatgtcggagaaaaaagagttcaccaaagaaaccatgctgcgcgccgcggacgagatctattttgtgccggaaggtacgccgctcagcacgcagttggtaaagtttcagcgcaacaaaaagaaagtcggcctggtcgtcaacgagtatggagacattcaggggctggtgacggttgaagatattctggaagagattgtcggcgatttcactacgtcgatgtcgccaacacttgccgaagaggtcacgccgcaaaacgacggttcggtgattatcgatggcaccgccaacgtgcgggaaatcaacaaagcctttaactggcatctaccggaagatgatgcccgcacggttaatggcgtcattcttgaggcactggaagagatccctgtcgcaggcacccgcgtgcgtattggcgagtacgatatcgatattctcgacgtacaggacaatatgattaagcaggtaaaagtttttcctgtgaaaccgctgcgcgagagtgtggcggagtaacgaaaacggcccggcattcgcatgcagggccgtgaattattacgaaagcagaaattaagcttttgctttcgctacagtaaccatcgccgcacgaatcgtacgaccattcagcgtataacccttctgcataatgcccagtacgttacctggcgcaacgtcatcagattccaccattgcgatggcctgatgcacattcgggtccagtgggacgttagtttcggcgatcacttcaacgccaaacttacgcacaacatccagcatcgacttcagcgtcagctcaatgccttcaaccatcgcagacatatccgggttagctttatcagccacttccagcgcacgatccaggctatcaatcaccggcagcaattcgttgatgaatttctccagcgcgaatttgtgggctttttcaatatccagttcagtacgacgacgcaggttttccatttcggcttttacacgcaaaatgccgtcacgttcacgggtctgggcttcagccagctgagcttcgagattcgcaactttttcatcgcgcggatccacctgctcagcagaagcttctggctcaactgcctcaatctcttcgtgctgatccatgataatttcttccggggcttgcccctcaggcgttttctgttctttactactcatgaatttctccgcgtttttttcgcattcatctcgctaacttcgcttattatggggatcagtttcagggtttcaagggaagcactcacattgtcatcaatcttcgcaacaaggacctcggaaaaatgaataatcatttcaagtgtattggcattgtgggacacccacggcaccccactgcactgacaacacatgaaatgctctaccgctggctgtgcacaaaaggttacgaggtcatcgttgagcaacaaatcgctcacgaactgcaactgaagaatgtgaaaactggcacgctcgcggagattgggcaactagctgatctcgcggtagtcgttggtggcgacggtaatatgctgggcgcggcacgcacactcgcccgttacgatattaaagttattggaatcaaccgtggcaacctgggtttcctgactgaccttgaccccgataacgcccagcaacagttagccgatgtgctggaaggccactacatcagcgagaaacgttttttgctggaagcgcaagtctgtcagcaagattgccagaaacgcatcagcaccgcgataaatgaagtggtgcttcatccaggcaaagtggcgcatatgattgagttcgaagtgtatatcgacgagatctttgcgttttctcagcgatctgatggactaattatttcgacgccaacaggctccaccgcctattccctctctgcaggcggtcctattctgaccccctctctggatgcgattaccctggtgcccatgttcccgcatacgttgtcagcacgaccactggtcataaacagcagcagcacgatccgtctgcgtttttcgcatcgccgtaacgacctggaaatcagttgcgacagccagatagcactgccgattcaggaaggtgaagatgtcctgattcgtcgctgtgattaccatctgaatctgattcatccgaaagattacagttatttcaacacattaagcaccaagctcggctggtcaaaaaaattattctaattttacgccagcctctttactgtatataaaaccagtttatactgtacacaataacagtaatggtttttcatacaggaaaacgactatgttggcacaactgaccatcagcaactttgctatcgttcgtgagcttgagattgattttcatagcggcatgaccgtaataactggcgagaccggcgcgggtaaatctattgcaatagatgccctcggtctttgtctcggtggtcgcgctgaagccgacatggtgcgtaccggcgctgctcgcgctgacctgtgcgcccgtttttctctgaaagatacgccagcggctctgcgctggctggaagaaaaccagcttgaagacgggcatgaatgtttgcttcgtcgcgtgatcagcagcgatggtcgctcccgtggtttcatcaacggtacagctgttcctctgtcacaactgcgcgaactgggtcagttgctgattcagatccatggtcagcacgctcatcaattactcaccaaacctgagcaccaaaaattcctgcttgatggctatgccaatgaaacctctctactgcaggaaatgaccgcacgttatcagttgtggcatcaaagctgccgtgacctcgcgcatcatcaacagttaagtcaggaacgcgccgcccgtgcggaactgctgcaataccaattaaaagaacttaacgaatttaatccgcagcccggagagtttgaacaaatcgacgaagagtacaaacgtctggcgaacagcggtcaattgctgaccaccagccagaatgcattggcattaatggccgacggtgaagacgcaaacctgcaaagtcagctttacacggctaaacaactggtgagcgaattgattggcatggacagcaaactgtccggcgtacttgatatgctggaagaagctaccatccagattgctgaagccagcgatgaactgcgccactactgcgatcgtctggatctcgatcccaaccgactatttgaacttgaacagcgcatctcaaaacagatttcgctggcacgtaaacatcacgtcagccctgaggcattgccacagtattaccagtcgctactggaagaacagcagcaactggacgatcaggccgactcacaagaaacgcttgcgctggcggtaacgaaacatcatcagcaggcactggaaatcgcgcgcgcattacaccaacaacgccagcaatatgcagaagaacttgcacagctgatcaccgacagtatgcatgcgctctcaatgccgcatgggcagtttacgatcgatgttaaatttgacgagcatcacctgggcgctgacggtgccgatcgtattgagtttcgggtaaccaccaacccaggtcagccaatgcagcctattgccaaagtcgcatccggtggtgaattgtcccgcatcgcactggcaatccaggtcatcacggcgcgtaaaatggaaaccccggcactgatttttgatgaagtggatgtagggattagcggtccaacagcggcagttgtcggcaaactgctgcgtcaactcggcgaatcaactcaggtgatgtgtgttacccacctgccacaagtcgcgggatgtggtcatcaacactattttgtcagcaaagaaaccgatggtgcgatgacagaaacgcatatgcaatccctgaataaaaaagcgcggttacaagagctggcgcgcctgcttggtggcagtgaagtcacacgtaatacactggcgaatgcgaaagaactgcttgcagcgtaaacttttttcctgcttcacggtcagagtaaacagcaaaacgccgtaagaccggaaagcaaaaggttttaaagtgatgaaaggtctattatcatcggcatattacagatgagccacgtactgctcgggcccgaaaaggaatcaaatcactatgcgctgtaaaacgctgactgctgcagcagcagtactattgatgttgaccgcaggctgttccactctggagcgagtggtttaccgtcctgacatcaaccaggggaactatctgaccgctaacgacgtatccaaaatacgtgttggcatgacgcaacaacaagttgcgtacgcattgggtacaccgctgatgtccgatccatttggtacgaatacctggttctatgtcttccgccagcaaccaggtcatgaaggtgtaactcagcaaacgctgacgctgacctttaacagtagcggtgtgttgaccaatattgataacaaacctgcgctgagtggtaactaataataaagttgctctcaaagacgttaaaaaaggtgctcaatgagcaccttttttctgtctgttatttattcgctgatttttctgctcgttgcctgcgaagctctttcggatcggcaatgagagggcgataaatctccacccgatcgccatcatgcacactatcgcttagttttgccggacggctgtaaatgccgactttgtttttagttaaatcgatatcggtacgcaattccagcaagccactggcgcgaatagcttcttcaaccgtcgcgccctcctgcagcgtcactcgctgcaggtactgcttctcaggtagcgcataagccacctcaacggcaattttacctggcactgtaaacctctttcgcacgaaccgtaaaagcctggaccatattagccgccagctctttaaacacgcgaccaaaggcgagttcaatcaacttattggtaaactcaaagtcgagatgaaactcgatacgacacgcctcctggctcagcggcgtaaacttccatccaccaatcaatttcttgaacggcccatccaccagattcataagaatactttggttactggtcaactggttgcgggtagtaaacgttttgctgatcccagccttagagacatctaccgccgcagtcatctgcccaggagtggactccagaatccgacttccggtacaacccggcaaaaactgaggataagactgaacgtcattcactaactgatacatttgctccgcgctgtagggtaccagtgcggtccggctaatctgaggcataacaatttccatcaacaaaaatccaacaaataatatcatttatcctgctgtaaaaaaaacgctatcccggcgctgggtaacatcgggttcatgctaagatagagccttgtcccccgcaggattgatatggggtgttttcgatttcagattaccgatgattcacgacgcttatgacgaagaaaaaagcacataaacctggttcagcgaccatcgcgcttaacaagcgcgcccgtcacgaatactttatcgaagaagagttcgaagcgggacttgccctgcaaggctgggaagttaaatccctgcgcgcaggaaaagccaatatcagcgacagctacgtccttctgcgtgacggagaggcatttctgtttggcgctaacatcacgccaatggccgtggcctccacgcatgtggtgtgcgatcctacccgtacccgcaagttacttctcaaccagcgcgaactggactcattgtacggtcgcgtcaatcgagaaggctataccgtagtggcgctctccctgtactggaaaaatgcctggtgcaaagtgaaaatcggcgtcgccaaaggtaagaaacagcacgataaacgttcagatatcaaagagcgcgaatggcaggtggataaagcacgtatcatgaaaaacgcccaccgttaaacctgcactccaattattgaccagttcctcaccgcgcctccctctccggcggcgcgaatgaacatcttattggctatcacatccgacacaaatgttgccatcccattgcttaatcgaataaaaatcaggctacatgggtgctaaatctttaacgataacgccattgaggctggtcatggcgctcataaatctggtatacttacctttacacattggggctgattctggattcgacgggatttgcgaaacccaaggtgcatgccgaggggcggttggcctcgtaaaaagccgcaaaaaatagtcgcaaacgacgaaaactacgctttagcagcttaataacctgcttagagccctctctccctagcctccgctcttaggacggggatcaagagaggtcaaacccaaaagagatcgcgtggaagccctgcctggggttgaagcgttaaaacttaatcaggctagtttgttagtggcgtgtccgtccgcagctggcaagcgaatgtaaagactgactaagcatgtagtaccgaggatgtaggaatttcggacgcgggttcaactcccgccagctccaccaaaattctccatcggtgattaccagagtcatccgatgaagtcctaagagcccgcacggcgcaagccctgcgggcttttttgtgccctcaatttgtcccgcgaagtccgaagagaactaattaaatccgaaccttttaggcccattgataggcccaacgaaaagctctattgtttacgttgggcctaaacgcagggagactccccatggcaagaaaaaccaagccgttaactgatacggaaatcaaagccgccaaacctaaagatgccgattaccagctttatgacggtgacgggcttactctgttaatcaagtccagtggcagtaagctttggcaattccgttactatcggcctttgaccaagcagcgaaccaaacagagcttcggtgcctatcctgccgtctcgctttctgatgcacgtaaactcagagccgaatctaaagttttattggcgaaagacattgatcctcaggaacatcagaaagaacaggtgaggaattctcaagaggccaaaaccaataccttcttgttagttgccgagcgttggtggaatgtgaagaaaaccagcgtaacagaggactatgccgacgatatctggcgctcgcttgagagagatattttcccggcaatcggtgatatcagtatcactgagattaaggctcatactctggttaaagcagttcagccggttcaggccagaggtgcattagagactgttcgccgcctttgtcagcgtattaacgaagtcatgatttatgcgcagaacacaggcctgattgatgctgttcctagtgtaaatatcggaaaagctttcgagaaaccgcaaaagaaaaacatgccaagcatccggccggatcaacttccgcagctaatgcacaccatgcgtacggcaagtatcagcatgtccacaagatgcctgttcatgtggcaacttctaaccatcacccgccctgccgaagctgctgaggctcgatgggatgagatcgatttcaatgctagcgaatggaaaattcctgcagctcgaatgaagatgaaccgggaccatacggttccactatctgatggggctcttgctattctggaaatgatgaagcctctcagtggtggccgagaatttatctttcctagccgtatcaagcccaaccaaccaatgaatagccaaacagtgaatgcagcactcaagcgtgctggcttaggaggtgtacttgtttcacacggcttgcgttctatcgccagtacggcactcaatgaggaaggatttccacctgatgtcattgaagcagcgcttgctcatgtagacaaaaatgaggtgcgtcgcgcttataaccgcagtgattatcttgagcaacgtcgtccgatgatgcaatggtgggctgatctcgtaaaagcagcagatagtggtagcatcgttttaactcatttgagcaaaattcgtcttgtcggataaaatatttatcagcccagctctctgggctgatatttctaaaagatcgcactaaatagctacgcggaatagtgctctactttcgtttagccctttcagaggtaagacattagggcaatttcactgtatgactgcgcagtcatcgagtctgtggggtgttgctccttttgcaacgtatcacttgtcaataaatagaaagtgtagatgtattaggcgcagctatttagtctatatggcaagtagtaattatttacttcttttttttctacgaacagcgctatcgaaagcttgttttacatcttcattttttaaagaccattgatttaaaatagtatcaaccaaagcatcttgactcattgttgctacacgatattttttattttgattatttatctcaaactctgacatttgaataaaatcccatagcggttcgataagttcattaactgctacaaccttatttttccacccatcattcggaacagagtcattaattagctcaaccaacttcagttgaatgatatggtacacttccgctttgcttttgccacccttctttcctgcactccgcctgacttctgataattttttttgattacaaacagagatgttaaaccaagtcatacctatgcacttatcaaataactccgcagcccgatgaaatgctttaaaggcaacgttttcattttcagacatgatagattttccccagaaaaaagagattgaggcgaacataaggtgtgccttgaaaatgtcattaatggaaaatggctcgataacaagaggtaaaaacgtttccttggtaaggtttgaacttagatttttccagcattcttgagctggatcatataattcagtgtattcttcctttatctccagttgcccattcactgtatggtgccttgtttcccatggtacatcgcaggaatataacctcacacgagtacctattttctcagagctccagaattgctctcgcattctgcctagctcaatccgtatttccggatgatcttcctctagaacatcagtatccaccgcccattcgcattcggacatgtgataggcgagatcacgtcgttttctacaaatttgttcataaaaatcattcagagaaatcataaaaccaccataaatcaatgtattagaggttgtaaaaattgtatttttggtacatgggttttttgccttaaagatacccattaatctctctgcaaccaaagtgaaccaatgagaggcaacaagaatgaacaatcgatcggccgttagaatactacggttaccagcggttatccaaaaaacaggtatggcacgggccaccatctatgactggttgaaccccaaatcaccacgatacgatgccacctttcccaaaaagcgaatgctcggcgtgaaatctgtcggatggattgaggccgagattgatgagtggttatcacaacgctgtaaacttatttgagggtgttacatgaattcatactcaattgctgtcatcggagtgtaaacatcctgctatttccgccattaatagcggaatagccatatttgctaaacaatttcttaatttaattaaataagaggcattgcatgttcaatggtcgtcctttccctgtagatgcatttcctaaaattatcaggaatgcaatttatgaagtggaacagcatacgcaggcccctcaaggtttgattgctgcttctgctcttggggtaatttctcttgcctgtcagaaccggattgatgtttgccgattgaataatctacgtggcccggtatcacttttcttaatgactctggctgaatcaggtgaacgtaagagtacggttgataaactgctgatgaagccattatatcaactggaagaggatttatttgaaaaatacacccacgatcttaccgcatggagaaatgatgaagcaatttttaatattgaaaaaaaagcactgatgtcaaaacttaaatcagatattcgacgtaacaaagatcacttggcaacaaatgaaagacttaaagaactacttacgacaaacccgaaagctccagtgagattcaaatttttatttaacgatgccacacctgcagctattaaagctcatctctgtgggcactggcgatcagtcggcatcatgtctgatgaagctgggatcatttttaatggttacacacttaacgagctgccgtttatcaataagatgtgggatggttcaatatttacggtggaaaggaaaaacgagcccgagaaattaattagagatgcaagaataacactgtcgctgatggtccagcctaatgtttttaagggttatatcgacaggaaaggagatatggcaaaggggattggattttttgcacggtgcctcatgtgccagcctgcttcaacacaaggtaacagaaaaatttccaacccaattttttcaaatgaacatttgccggtatttcaccaacgtcttatggaaattgttaatgagagcatcattaaaattaatgaaaataatcgcatctgcctccgattctctgcagaagcagaaagacattggatcgaattctacaaccaggtcgagtcagaaatgagaatgattggccttctttatgattttaaggattatgcttctaaaatggcggagaacatggcgaggcttgctgccttacttcattacttcagcggtgatggaggcgatatatctgttaccgcagtaaaagcagcagtggagatagtggcttggtatattgaagaatacatccgcttgttctctaaaaaagaagagttttctttagatgtttcagaagcagatgagctttattgttggataaaagattactgcacgcaaaaattttcttcctgcatcaagaaaaatattatcttacaatttgggccaaataaatttagaaatcgtgacaaggcaaatgaattaattagaatcttaatttcacaaaacaaaatatttatatcttcatggggtaaaacaaaaataataaacataactcattgtgttttttgattttaatgacaatctaaaaggacttaatttaagagtaaaaacaaactctaaacccagttcggataaaagcttgtcatcttgataggtaatatataggtacatagacacatcagaacgatcacttactccaatatcattggccaggatactatatgacatacgatagtgaattcggatcacatgtatccctatatcgggatagaatcaaacaggttattgatgactccctaaacgaacatcttaactcaatgattctacgtgttgatctgcatgacccaattgatacagaaaatatggataacccattctttcaacccagggttgactctggtgctatatctcgctttaccagtgcgttaaaagcaaagcttaaacatgataagcatattaaaactcaacggaaagactggcctgatagtcgacattccactttacgttacgcatgggtcagagaatataccaaaaatagaaagcggcattaccatttgatactgtgtttcaatcaggatgcttattatcatttaggtgattacgacttaaaccgtaacacgttacgtacaatgataacgacagcttggtacagtgcacttggcatccctatagatagctcggggaagttagttaattacccgccaaatggcaaataccttctcaatcgtaaaagggacaactttgagcagacttatagcgatttgatgaatagggtggattacatgaccaaagtaaggactaaaatagtcggtgacggagaccgtaatttcggctgcagtcgcgggtaatttattttttacaacaatggcctttcttatggctggaaaggcctgatttgtttgtattaagatatcggtaatcttttgatggttggaagcccgtcctggtagacgacctagcctaccgaagatgtgagttattcaaaaatgtcgctttcccgcgttccgtagacaaacgtacctaaatcaatgtcgtctaataccgagcgcgcgcctgataaacatctgatcaacgtacccaatcgatctactccaaatgtcctgagtatcccgaagatactggctcaactcatccacatcagcctcgtcggaaaattccagcaagtctaccagtcggtgtaacgtctgaatgggaatgccaatctcttctaaggcattgacacctggtggtagatggaaactttcgaacgccaatttgacatgtgtgtaatcgactttgctgcgtataccacgctttacagcgtggtgtttaactacatcctccatcaagctgagcaccttaggtagggtatagccgaaggtattggttatgagcttcaaatcattgttgagggcaatggaaagagtacgtttctccccttcagaaatccactgtcgtgcataatcgatctgatttttcagatattccgaataactttcagcacttaaatagccggcaagttttgcgatcatgacatccgtaggcttaacagggaccccattgcgactgaacgtatggggaaccagtctggcaatgatctttgcaaaggtcttgaggaagtttgtcgcgggagtccagtgaaacactaacgaggaaaattcgttatcgtccatcatctcgaacatgctttgcagcatttcgaactgctcgacacggaagtacgaatgcttcttcacaaggtcgatggaaacacggtcgtttatgaaaacctcatcaaagcgatcctgtgaaaactcggacaagtggtctggttgaacgctggctaacaggttgattggggtatcaatgccctgaataccgagcggaatatccacctcttgattgagattgtcttccgggatttcctccaggcaaaagattttgccgacgaagtgaacgcccatgcgcccggcgcgacctttgatgttcccatgggtgaatttgtcaatgctgcgagttccatcgcggttgtcgtagatcacaacgttcttagcgatagtgttgactccttcaatgatcgtggaggtgcagagcaaaaagcgcagttttccagcattgaattggtcggcagtgtattgctgcagtgccctcggtagcgcgccaaaatgcaagccaataccgtttctaagggcgactgtgtaatcccagtcggcatcgaactcttcgctgacccagtcgacatggggattctcagtcggagtgccatgcccaagcctgatcagctcgcgcgccaccaggcccgcaacagttggtgacttgcaataaatgatcgttgcgtcgacacatgcgtgcgcgatttcccccagcgctttgagcttggctttgtcgtcattcgctttgatgccgaacgtcttaacatctagcgcgactgtattgaagtcggtagaaacgaaagtatgcggatatccaagtttttcgagaccgcgaatgctgttaacgaacggtcccgtcaggtaaaactgcctggagaccttaagcagtttgcttaacgcaatgttgagctcgatgactcgttcgtcttgatgatcaatgtccccgcttttcagttgtcggaacgccaacttgtaaaactcgtcaatgacgaagaggtcaatgtcgacgatgtcgtcacgctcgttcactcgctcctgagttaacacataaacagcctgatcggaatggcacacttgggaactgtggtggatgatctgatatcggtcaccgaatcgctcttgcagtcggcgacgggtttcgtcggcaagagccacggttggaacaaccagaacaagccgtttcaaagttcccatgccgagcaatgaatcgacgattgcacttttgcccatgcttgtaggtgcactcagcaccacgttttgaccagacttgagcagatcgaatatgtggaactgcattgagtggaaaacataaccatccgagaatggcgtccggtatagctcaagcaccctcaggtcatccggtgtcaggctggtgaactcctttttgagatacgggaacaaacctgattttctcaccatatttttcaaaattgtggtgtgctcggaaaaccgctcgcgcgaatcgagagctcgcacgatcaagtcccgtcccaagtcatacgaaacagggttagacaacagcttgttaaccgcaaacagataattgaacgatgagaagtcctcaccctgcaggctatgtttcgcctgttcatagatctctgtcatacgacctctctcaccttctcatcaactaattgggttaaccgctcaagactcggggctggataaatgaatacgtggatgcaaagattcgcaaacggcgaatcctcgatgaggtcagccgcgaatttttcgaacagcaccgctgtttctttctccaggtcatcctcgaaccccggcgtttcaggctcggttagtagattagagtcgtagcccacgaacagaacaaacgtgaaacgatcgaggtgagcatcgaaaggttggctgccatcaagaatttcgtcaatgtcgtggcgaagcaggtagttatcgtctttaatgtcgaggatttttttgcgcgcggtatcgatgcaatccgaaatgtcctcgtacaactgatcccgtatctccggcaatctgacggcaatgttaatatcagtcaccaactcgctgaagccaatccaaagctgatcaccttctggatcgcggcgaacgatatgcacgttttcaagaattttttcggcccctgctttttccacgtatagcatgcaaggaataggctggctttcgtggtgctgccggatcgttgcgtgcaacagcactcgacccaaaaattcgctgacgtcatggagcgatttgaagacggaattctttagtcgttctcgcttttcaatgaatgtcagtttatgaatatcagacatttcttttggtcggagaaaaacctcatccaaccattgacagacgttatccgcgatgtgcttgtagcggtatttcttaagtgagtactgctgatgtagaacctggcctttacgcttagcgcagaccgaagccataggcgctctaaatggcgtaaggatgtggggtaagtcccgtttgacgtagattttgcggcctgaccgagattggtcatcttcgacacgctgcttgaaccactcaagtaggtctggtcgtaagtaggacttgtcatcagcactgtgaatgcgtcgagaatgctcgcccttgcgcgtcacagtatcaaggatgcggcaccaaatgtcttcggcgacggtttcggaactgagaatgaccccatgtagatcttgggaggccagccgtatgttcttgatccctagaagttccagttcgcgcagggatgaaaacacttcccatgtagccgcatcgatccaatctgaaacgcttatacctgagtctgttaaaaaattgtctgtgcgtttgttgaggtcatcgatgagttcctgtcgacctggcttatctagtcgggcgtttgggctgatcgtcaagtactcaagggttttgttgaccttttcctctgtgacgatggagtacctacgtccaagggacaggtcagactcacactgcattgatttgtgcaaaattgaactgcaggggatcgtctttttatcagcaccttttgaattctgaacgatgtccgaaatgttccaacgtgttttgccggtgctttttacctgaacgaagtcgatgtatccatcagatacaatgtcgatatcgtctgtgacctcgcagcgcacactgcggatagtcttgtcacgaagcattcgggtgacatggtaagcggctacgcagtcctgaaataagaaaccgtgcttggcggctactccgcctgaatcgttcgactccatttagacatccgtgacaattttgcgaaaattaaggagatgttatgacacagtccaatcggatcactgcatcatcaccagtgatctaaatacttcacagccattctcggtcgcaggtatcaagcttttcaggattccacaaatattgtaaccctgacgtctaatttggttatataacatactgccccaactaacgtaaggtaggcacagccttaatcaaggttttggttttcaaatagttcagagctgagaccgccaaccgcactatggcactatggcactatggcactatggcactatggcactatggcaccgccagcgattgtaatcacacttgatattataaaacacagttgcacgcattatttcctggttggtagggtcatatctcgatgctctttgagcaatgtcaacatcgcgtgttcatggctttctatattgttgatgccttgcccatccggaccccactccttatagctcatcatgatggcttgttttgggctctctgctcgttctgtttcgacgtagaattttttcttgtctgctggcgaataattactaagtatcgagttgctgcttggtgagatcaggaagaggttaccgaaacgatggacatcatcccccattttgtggactgcccccccggtagacgatcctgccctatagttggagtgccccctattcaggtggctaaatttagcaaatcaatacacttcaggggggtattattgtagagtttccccatatgtttctatgggatccaggaaatgacaatcaggagttacaaaaacttaaatctggtcagggcaaatatcgagactgaatccagacaattcattgaaaataaaaactattcaatccaatcaattggtcctatgccagggtcaagggctgggcttcgggtcgtatttaccagaccaggggttaacttggcaactgtggacattttttataacggggacggttcgactacaattcaatatctcactggagccaatcgttctctgggccaagagttagcggatcatctttttgaaaccatcaatcctgctgaatttgagcaggtaaatatggtactgcaaggatttgtagagacaagcgttctacctgtacttgagctatcagcagatgaatcgcatatagagttcagagaacactctcgtaacgctcataccgtagtgtggaaaattatttccaccagctatcaggacgaattgactgtgagcctgcatatcacaacaggtaagctccagattcagggccgaccgctgtcatgttacagagttttcacgtttaacttggcagccctgcttgatttacagggtttggagaaagtgctaatccgccaggaggatggtaaagctaatattgttcaacaggaggttgcccgcacttacttgcagactgtaatggccgatgcttacccgcatctccacgtgactgccgaaaaattgctcgtttcagggctatgtgttaaactcgccgcccctgatttgcctgactactgtatgttactttatcctgaactacgcaccattgaaggtgtcttaaaaagtaagatgagtgggttaggcatgccagtacagcagccggcaggttttggaacttactttgataaacctgctgctcattacattctgaaaccgcaatttgcagctactcttagaccggaacagattaacatcatcagcacagcctatactttttttaatgtggaacgtcattctctgttccacatggaaactgtggtcgatgccagccgtatgatttctgatatggcccggttgatgggtaaagccactagagcgtggggaataatcaaggacttatatattgtttgaaatcaccggaattaacgtctcaggggctctaaaagctgtcgttatggcgaccggcttcgagaaccctttgtcctcagttaatgaaattgagacgaaactttctgccctactgggtagtgagaccactggtgaaatcctttttgacctcttgtgcgctaacggtccagagtggaaccgcttcgttacgctggaaatgaaatatggccggatcatgctggatacggccaaaattattgatgagcaggacgttccgacacatatcctgagcaaactgacttttactttacgtaatcatcctgagtacctagaagcctctgttttgtctcccgatgatgtacgccaagtcctgtcaatggatttttgaaactcttctttctaaacgaaccagtatagaattcgcccttttggcatgatattaacttgtccaatatgatcaaatagcattaaccccccctcacaacgtcctgcatagggaacacgttttcccctgtgcacccacgactaaatttccccccctttaaacttctcaataatgtcaccaattttctggaaatcctatgatgcctttcccggtaaatggtgctgtgagttcagaaagattctgcaatctatgtgcattgaaaaaatcttcagatagatatcattctcctgaacaatccgatgaacggcagaacctcgcggttctgccgtttttgttttacttttcagaggagtggtgatgaaaaattttgaagttctgcagccactacagaactccctttccggtctaccgctatgggtatctgaacgtatattgcagcagataaatcagttaacccactacgagccagtgatcggcatcatgggtaaaactggggcgggaaagagtagcctttgcaatgccctgtttgccggtgaagtatcgccggtcagcgatgtagcggcctgtacacgtgatcctttacgctttcgcctgcagattggagaacactttatgaccatcgtggatctgcccggcgtgggcgaaagtggcgttcgcgataccgagtatgctgcgctgtaccgcgaacaacttccccggctcgacctgattctgtggctgattaaggctgatgatcgggcactggcgactgatgagcatttttaccgtcaggtgattggcgaagcataccggcataagatgctgtttgttatcagccagtcagacaaagctgaacccaccagcggtggaaatatcctttccacagagcagaaacaaaatatcagccgcaaaatctgcctgctgcatgagctattccagcccgtgcatccggtgtgtgccgtgtcggttcgcctgcagtggggactaagggtgatggcagagcggatgattaagtgtctgccgcgtgaggccagcagcccggtagtagcgctactgcaacatccctttcgaacaacggtagcccgggagcaggcacgtgacgatttcggtgaaaccgtaggtgccatactcgatacggtaagcacctttccccttattcccgccccggtgcggaccattattcaggccgtgcgttcctcggtggtgtcagtggcccgcgctgtctgggatttcttcttctgagtgtttaattctgccctattattctccgagccctgtcgcaagtgcggcagggctttctttatttgttttacccatactgaggagtctgcttatgacccgtctggcttcgcgctttggcgctgcaaatcttattcgccgtgaccgtccgttaacccgtgaagagttatttcgcgtggtgcccagcgtattcagtgaggataaacacgaatcccgcagtgaacgctacacgtatatacccacaatttccctgctggacagcctgcagcgggaaggcttccagccattctttgcctgtcagacacgggtacgtgacccccgtcgtcgtgagcatactaagcatatgctgcgcctacgtcgggaggggcaaattaccggtaaacaggttccggaaattatcctgcttaactctcacgatggcaccagttcgtaccagatgctgccgggcatgttcagggcggtgtgccagaacggtctggtctgcggcgagtcgtttggcgaggtgcgggtgccacacaagggggatgtggtgagtcaggttattgagggggcgtatgaagtgctggggatttttgagcgtgtggaagaaaagagggatgccatgcagtcgttgcttttaccgccacctgtgcagcaggcactggcaaaagcagcgcttacgtatcgctttggtgaggaccaccagccggttactgaatcgcagatactctccccacgccgctggcaggatgagagcaatgacctttggaccacctatcagcggattcaagaaaacctgattaagggcggactcagtgggcgtaatgctaaaggcggacgaactcatactcgtgccgtgcgtggcattgacggggatgtgaagcttaaccgtgcgctgtgggtgatggcagaaacactgctcacgcaactgcagtagacgtttcatgttgccacgttgttaatatcggacaccacctgtccgcatcgctatgtgctcgtgtgcctcaatcccccggttatagcttttaacccccgttacatctggcttttgcagaaataaaaaatagtttctgcgttgtccataccctgtccgcccccctctttaaagtaatcacatcattttcagtcagttaactttcctggagaatctctcatgacacaggcagaacgccgccatgaccggctggctgtcaggctgtcactgataatcagccgtctggttgcgggtgaaacgttgagcgtgcgcaaactggcggctgagtttggcgtgtcagtgcgcacgctgcggcgtgattttcgtgaacgactgatgtatctggacctggagtatcagtccggatactgccgcttacgcactgctggcagtgagatgcagatggtgcccgacgtgcttatctttgcccaccgcagcgggctggccgggctttttcccggccttgaccgccgtctggtgaatgcactgctgatgtgcgatgagtctccctgcgtgatagcaccagccaatccggttccttcgccttcaggagcattgtctttctggagactgattcaggccattaccgggcgcaggcgggtgacgctgattgcagaggggcgacgctgtgagcgcctagctccctgccggttactcatccaccagcagacctggtatctggtggctgaacacgaagggcatatcgccgtattcacacttgatgaaatccatctgattcagcctttgcaggagacttttcgccgcaatgacagtctgtgtcgcctggttgaagacccggtcttcattcaggccttaccccattttcgctttatccagcattcactgcttacgtttgttccggccgacagcccaccggaatagcgcaggcgttgttatcaacccggcaacatggaggagcccagtgcccgttattgccattatcgccattgttatcatcgtcatcattctgaacaaaaccggagtgtccgacagcctcacggccctgacacttgcaaccgttgccgcactactgacgggaggtggtgcagccggtgctgccagtgtcgcgctgacgccgttcgtcggcgtgccggtgggtatttttgtgggaatttatgtctttgccaaagtggttcgtctgatttcagggaaaaaataatgaaacgtaaaacactacctctgctggcgctggttgccacctctctgtttctgagcgcctgcgatgacaggagtgatgacctcaaagctatcagtaaatttaaggacctcacgcccccgcgcttcagcgatgtggtcagccgtcaggatgatgtcagcgaagaatggtcacaggttggcttctcatccggtctcaccctgcaggtcttacgtacccgtgagtcgcccgatggttgcgagggtggcagttactactatctggtagatatggaggagaaaaccgtccagccgctgatgaatgcgctttgtattgccgacaatatcaaactggaataccacgaagttacggacccgtatacgaaagaaaaatacttcgaatattcccatgacggcaaactgatgggacggctgctgataccgtcaaaccctgataaccgggaataaaaacaacgagaaaggagacataaatgaaaatacgttcactaagccggtttgtactggcaagtacaatgttcgccagctttacagcctctgcggtccccggactctggcaacaggggtacggtcagggcaatgcggaatacagtgtgacggatgccagcggaaagatgtttaccatcaactgcacgggaaatccggaccagaacggtatttaccagcactcggtttttctgatcctcgccggggataaaacggtcagctcgcatgatgacagtaccggcatcacagtggtgatggaccataagcaatatgccattccctcaacccttggctggcgtaacggagataatgcctggttcagcttcatcatggatatccgtaaggcccggcagttcgacgtctacgtcaatgaccagaaagttggatcgtttaaccctgatgttcggaatgcacaaaaggtcctgccaacattagcggactgcactaacgactgacggctgcgccttccctaccataacaaccctgattgcctccggcggtcgggggtttcttttttctccttaatctccagaggtaggccacgtactttcgaacgatgagcgcagtggtcagtttttttcagatatatttatctttttttggctgtaagctccgctgtgagcgcaggctgtgttaaaactcctgatcactttttggtctaagcgatggtttcatatgatcaaccattcttgataaacccatgagacggactaactttttcattaaaattaaaaagatatgaatgaatactgcggatatcaacatggccaatcacattcaaggacaaggcaggcatcaggtgacattgctccctgatgcactcgatgattttgtcactgaagatatctgaaataagtttaatcagttcatcacgggtcggtggcatatcgagataattaattattgtcggttcgttgccgttgttatgaagcatctccagcgtgttgcgtgaggtgccacaggccgggttgtgatagatggtaatgttgctcatatcagtatctaattacaaagtgacagagagccgccacgccagcgcggccagagtgacaaacagcaccggcacagtcatgacaatgccggtacggaagtaatatccccaagtgattgtcatatttttctgggcaagcacatgcagccacagcagagttgccagactgccaatcggggtgattttcgggcctaaatcacagccaatcacattggcataaatcattgcctctttgacgacgccagtcgccgtactcccgtcaatcgacagcgcaccaatcagcaccgtcggcatattgttcatcactgatgagagaaatgccgtcaagaagccggtgccgaacgtcgctgcccataaccccttgtctgccagcagattcagcacgccagacaggtactccgtgaaccctgcattgcgcaggccatagaccacgatgtacatgcccagtgagaaaataacgatctgccatggcgcaccgcgcaggacttttccggtgttgatcgaatgacctcttttcgccaccacaaacagcactgctgcgccagcggccgctatcgcactgaccaggattccctgcggctccagaaagaagaaaccgacaagcagcaataacaggacaatccagcccgccctgaaggttgccagatccttgatcgcactggcaggcgtcttcagcagcgaaacttaatacgttgccggaataactctgcgaaagaagagatacagcataatcagcgtggccgcaatcgctgccgcatccacggagatcataacggaggcgtactgcgcaaagctcagaccgaagaagtccgccgagacgatattcaccaggttagaaacaatgagcggcaggctggccgtatctgcaataaatcctgcagccatgacaaaggccagtgtcgtgccctggctgaacccagtgcgatcagcatcgcaatcacaatcggcgtcaggatcagcgcggcgccgtcattggcaaacaacgcatcaacagcggcaccgagcaagactttccaggtgaacagcgctctaggtaggaactttgtcgttgatagagtcttcagccatcaacactgtatcgagtaatgaaattggttgctagaaagtcgatgatttgttgcgtatgattaaaaatcaaccttaaaggctttatacatggatttgctatggcttttgtatcagaaagagaaattgtaagaaagatatttagcaaaaaaattgactttacgatcttggcatttttctatatttcctctattttttttcttctttgtagtggcgttctctttcaatattttaccgctgccttcacaaaaggtaattgttatgaatgctcaatgaaacttgattacataaaacaattttatttttcactggaaaccgcatggtacctcatatctgctgttgcagtatttattgcatctgtttttatacagcatagaattaaagcttatttaacattattagctattacatggattgtactaacaataacagatgtggcgttaatacacgccttagacaatatagccatgaataatattttgttaaatatactatataatctttttggggcgattttattgtcactgtttatgtgtttatcaaattccctccttttccaccttaataagataaaacatattccaatgattttatcggcaatgattccattagtttccgcaataataatagccatactcataaccgctgttatatatttattgtttgcccggcaggcggtagagattgagatggatatatctgaaggttcagacatcgcatatgtaggtgtaaaagataatgaggaatcatttgggtttttaaatgataaaaaaacagacacaccaacgtatctggatgtaatcaaaaatggtagtttgatatataatgatacacagggtttaagtggtgctgatatttatattgtctccggttgttatgcccttccagatttacttcgcaatgtaccgcttgatgctaaaaaatcttttctgaatgtaaaaaagctagaaatcacacagaaacttccaatgatggggttcatacaaggtgaatccgctgatgtgatgcctaaagcagcatccaggttaagtttgagcaagcaagatgataaatttatgctagcctcaagtgttactgactctcaaataaaatttaaatcaaacaatgcacaattgatggttgctttcgcatttatgccaataacaacgaatggtattttacatgattatacatacgatataataataaatgataaaaaatataaaattgaaaatcatgttgcacctctatctaggcttgataaaaataagaagatgaagtgtgaataccagcaaatatcggatttaacaaatacgtataacattaatgcaaattacttaacgggttttttacttgtcctaaaaccagatgatattattaattacaacaatagcccttccgtactactcaagactgattttgcgttctataaaaaaacataccagaagcttgataaaatatatgatgacataagcaatggaaaattatcttcactgagagcaacaggtatctcccagtttagtatcaacgggaaacatttgtcgttaaggccagaatcggagattattatttctgaagggagtttgtatggactagttaataaaagcaaaaaaatcaaaatatatggcacagcagatcttgtttttgttgataacaagataatgaaccttcgtaaaataacttatttgcaatctaagctagaaatttttggttcttctattatggatatattaaagtatatatttggtttaggtctgctagcaatttctataaaattcattcattcttactttaagaatgatgtgaatgaaaatttattcttgtaacgcatttggctccaattggagcctttttatgactatttattaaaatatcctaagttaagcctgtttttaaagcaggcttgagcgtgaagcggacactcatacctgctttaaagtggcgtttttgtcgttacccatacctatattttctgttgtttaactgccagaactgagcggttgaaaagccagaaatatgccgagccagcggcatggaagcgccagcagctgttgaatggagtactgtaggcaaatggtgccgtaaccggctttcgtactgaaaggttctgtctatcccatcccttctcttgtatctaacatttagttgtgaatagctactgtaaatgcccctacaaaatgaaccattatttttagagggcgtctggcactccaacttccgcttttggcacagaacggcctatcagcaatataaaagcattcagatatatatcatttctacaaacatacccgattaacggcagaatctcaggattctgccgcttttttattatttttcaggggagtagtaatgagcaactctgaaggttggtagtcattttagcaaacgctttctggtctgccgcagtgggcatcggctgattgcgtagcagggccactggtatctgccggtatcaccgacattaacattgaagacgaccagggcattcacgtccgcctgatagttcgtgatgccgaaggtcggatggttggcgggcatggaactttgaaccggacgccggtgaaggttttaaccgctatatccacaggtcaggcatccgcaccgacaccttcccccgctgactccgaatcatttaccagcaacatttcaccttcccaaacgcgctttattacctcatacgccagccatcgccgctggcgttttttattcacggagacatacccatgacaacacagacacagtacgacctcgtacccgctaacggatccgaatttgagttgagcgtaacgcaggtacccgatgaacagcatatccgcttctggccgcagcactttggcaccatcccgcagtggataacgctggaaccgcgcattttcgcctggatggaccgcttctgtgatgagtactgcgggggtatctggtccttttacacgctcagcaatggcggagcgtttatggctcctgatgctgacggtgacgataaatggcatttgctcaacggcatgaatggcaatggtgcggaaatgagcgcggaagccgcaggtatcgctgtctgcctgattgaatatagccatcacgcctgcctcaccgaatgcgatgccatgacggagcactattaccgcctgcgggattacgctctgcagcaccctgaatccagcgccattatgcgcattattgattaaggatactcatgatggaacagtcactcatcccacagacaccggtacttccactgaccgcacaacgcacggtaaaacgcgccttaacgctgcttgaccgacacctgcgcgaaacaggcgtggcattcacctccactcaggctgctcgtgactggctgaagctgaaaatggcggggctggagcgtgaagaatttatgatgctgtatctgaaccagcagaaccagttgattgcccacgaaaccctgtttgccggttctattagcagtaccgaggtacatccccgtgaggtggtcaaacgcgccctgtatttcaatgcagcagcagtgatactggcgcataaccacccctccggcgacactactcccagccaggcagataagactataacgcagcgtctggtgcaggcgcttcagctcgttgatatccgtgtccctgaccatctgattgttggtggcaggcaaatctattcgttcgcagaacacggtctgctttgaggtattacatgagaattatcagtaaacgccgggcaatgacgatataccgccagcatcctgagtcccgaatctttcgctactgcaccggaaaatatcagtggcacggtagcgtctgtcattacaccggcagggatgttccggatatcacaggagtcctggctgtgtacgccgaacgccgcaggaccgcagcggaccgtatgcttgactgatgagtatcaccctgaactgacaataaagaggttatgaatgagcaacaccacatggggcctgcagcgagatatcacgccgcgcctgggagcacgtctggtgcaggagggcaaccagctgcactatctggctgaccgggccagtatcaccggtaagtttagtgacgccgaatgtcctaagctggatgtggtatttccacattttatcagccagatagagtcgatgctgaccactggtgaactgaatccccgccatgcccaatgcgtcaccctgtaccacaacggttttacctgcgaagccgatactcttggtagttgcggctacgtatacatcgctgtttaccccactcaacgctaactaatttcacgagagcaagcatgaacactctacctgctacaatttcgcaggcggcgaagccctgcctgtcgccagtggctgtctggcaaatgctactgacacgcctgctggaacaacactatggcctgacactgaacgacacgccgttcagtgatgaaactgttattaaggaacatatcgatgctggtatcactctggccgatgcagtcaattttctggtggaaaagtacgaactggtacgtatcgatcacagaggattttcgtggcaacaacagtctccatatatttccgtagtagatattctgcgagcaaggcgctctaccggcttgctaaaaactaatgtgaaataaacgcttaaatacagagcagactgaaggaaagcaaaatgctaatctcatagacgaagagactcccgctgtaacctcccctcccccgaaaaaacctgacattttcttttaggaccaacaatgggaccaaaatgaaaattgaactgaagattacaatcaatttaacaacaagttacacaaccaattcagactccgccagcccaccaatcatgattggacggtgtaaggacaacaccaacaaaaacaggaagttagaagtctcagcaaaacaccgaccagacggtgaggagacataaaaggatacgcaaaggagccgcggctcctggtaacatgaaagcccacagatgtgggctttttcgttgatggtcagaacgaccagttcacaccagctaccgcgttccacggggattccacaccggcactatggctataccccaccccaagatgcccgcttaacgtactgctgaatgaggctttaatacctgcctggtatattccacgtctgcccgacaaataattgacgaaattaccgtcactattcactttcacccggttatcatcgacaaattctttgcgcacagccgccttcagccacggctcaacttccataccgttccccagacgcatgttgtaactcagcgttgcgcccagttcacgatatatactgcgggtatcgactgatttcgatttcatgccattggataaatgatattcggggttatcagcggtgaaccccgttaacgatgcatacggcgtcaggttccagttaccatcggtaaatcgcatcccggtttcaatgtgaccgcccagcccgttgctgtggtaactgccattggcggctccaccgctgctcattttacctgctacgttacttttaaaacggttcagcttcacgacaccgtccagatagaaaccactttcatgttcccaactggcatagccgcccagagaataactgcccacactgccatgtcctccgcgatcaaaaccgatatgtgaatgggaatagcccataaaagcgcctagcgtggtaattccttcaggaatatcattacggctgtcgatccccactgtcattccggtcagcgtctgctcaaacccggcacccgcatcggtggtgacattattacgggtgttatacgtcgccccccagacattattgttgtgtggactcgctttcattatgttcaaccgctcgcgaatactgtttagctcagcatcaaataccaacggtaatgttgctgccatattgagtacggctgccgtagaaggcgtaatgcgtttctccggaacgggtgtcggcgttggatcgggagtagggtctggttttggatttgggtctggctttggatcgggttttgggtctggctttggatttgggatggggtccgggttgggtttgacatcattggtcaggttccagttgctgttgccgtcacttttcaggacatactcataggtcccaagatcaacgaaaccgccggtattgcccagcgtaaacgaagcatcccctccccctgttttcaccagcgtcatcgcgtcgtcagactgtgggctgacgccggtatcctgaacaaagattttaaaattaccagtggcgttgttgttgacgaccagttgatcgccccgggagcctgcaacgttggtatgcaggtagaaattaccgctaccggaaagttcattggttgtcagcgtattgtagataccgttagttgtggcaggcgctgctgtttgtgctgacaaataaacatcaccgtcgttgagtagcaaactgtttactctatattcgcagttgctggtacctgcacaggaattattgctgttaagccagacactgccccggctggcagccgtcaggtcggcaagcgtggtatcgacgccatttcccagagtcaatgtcgcgctatcggtaatccggaccgccccttcgagtttaactggcgtaacattatcccgtggcgtcattaacgacaggcttcctgtcgcgccactgaccgatgcatccgccagcgtacctgcgtagacgattgccgtaccgccagcgacctggagatcttctgcccgggccagagcctgaaactcatcttttgaccgcccaagggtatattgcccgccagagttaacctttgtggcggagtcctgacccaggttttgcattgccccacccttgccaaccgtggagtcgcgagcttcggtacctgctaataccaataaattaccgccattttccagcaacatattggtcgctaaattgccggaaatggaaaaagtaccgtactggtgagtaccgctgatttcaataccgttagccgtgctcgtctggagagcggcaccgctgttctggacgatatctgtcgctttgccattatcgttgactgtcagcgtaccgccttcattgatctttgtttttattgcctctccgttagctgaaactgtttgtattccgccgtcgttaattgttgtctcattcgccacaccctcgacaatttgttcaccgccggtgagcgtcgtgcctgtcgcagtggcttttgttttgacgatctcccgtccgcccatattgacctgtgttttgtcagaagaggtgtctgactccacggttaacacgccgccatttgccagcaggatattgttcgccgcaccctgctcgatgctgaacgcgacgccatccgcgcgtgttcctgtgacccgcgtcgccctggtggttgcaaccaaagcgccctggctactctgctgtatccccgttgcgctgcctttctcccgcacatcgagtgtgccgccgtcattaagcaccgagttttcagccaggccgccctcattaactacctgtgaacccccattaataatggaaccttccgctgtcccgtttgccataatttgttgtaggccagagacgatatcggtattgattgccttaccataattctgaacggtttgcgtgccaccattgatgtgtgttttctctgttgacccaccatcaacaatttgttcaccactttcgatatttgcttcagtggctaaaccatataccgtttgcttgccacctttgatatttgctttatcagaagtggcactggcatatattgtttgggtgccagcactattgagtacagtgccaacatcttttccataaacatccattttgccgttggcattaataatcgtgtcaactgcgcgggaaccagtgacgactgttaatgagccagcgttttccagcactacatttttagcttctgaattcctgatgtagaaagcatcaccataactgttggttccttcgataagtgttccggaggtcgtggaagcaattaatgcgccgccggattgttgctcaacatgcttagcctcaccaccgtcctgaacctccagaacgccgccattattaagtctggtgctatctgttttagcctccttctggacaatcagcttaccgccagtatcaatggtagtatttttcgccgaggttttagccactaccgtcagttcgccggtattttccagcacaacataattagcctcccctccggtaatagtgaagtgagagagcttgttgtatccttcgatatcagtccctgcacccgtgttggcaactaaagcactgcccgtctcctggttaaccccatgtgcaataccgccggtatagacaatcagcgagcctccggcgctaatattgctgccaattgccgtaccatctttctcaacaacctgccggctcccggaggatataattgttgtgtcagctttcccgccgcttttgatattttgcgttccgctgttgatattggtgcctgtggctatgccataattattaatattctgtgtgccaccattaattatggtatttgtcgcgtttcctgcaacatccataaccccgccattatctattcgggtcgcatcagctttagcattggttaaaactgacattgttcctttatctttaataatcgtcttgtttgccgaaccatatgcgtttatgtctaaatgaccaccgttttccagcaacacattgtctgccacgtgattgtggatggagaatgcaccttcactattcgtaccgctcaccgtcgtaccgttagtgttagtttttaaaattgcaccatcgtgctgggtaacatttgttgccgtaccacccctaacatcaagcacgccaccagaataaacttcaataacatccgaggtgctggtgttatcaacaatttgcgtgccaccagaatagatatgcgtattttttgccgttgacttactattcagagactgagttccgccttcaatcgtcgtgtccagcgcacggctctcatatactctttgctcaccgccatttttaatggttgttgtttctactgtgctctgttcaacatactgtcgaccaccatttatggttgtgttcgttgccagacttccttgtactacgtcctgagagccagacttatttatcgttgtaccatcagcatgcccttgaacttttactatctggctaccaccatcaatgagtattccattcgcactccctccctctacgcgtgaagcaccgcccttaattgtcgttccattgctgataccccctttataaacgtcctgattgccactctcgattgtcgtacctgtggaaatacccccgtcatgaattgactgtctgccaccgttaatggttgtattattagcctgccccacaaaattgttatgacttcctatatcttgatatccaccagattcaataagacttccattagataccccgccatgaacattctgctggccatggttgataatatgagtgttatttgttgtacctcgttcatccactttttggttgccatctacagtctcatcgtttaccacaccaataacattagtagtgaaggcagccatcccgggcggggcatatatcaaggcagatatcaataaggaaagtactgagcggcgacaataatagggactggtcctgttcataaatttcatcctctgaaaagtgaatactgagtagcgtttaagcgaccttagctttgctgcaacatcagcccacaggcaccagaccaggggattcatcctgaagagacagcgcaagtgtattgtgttcaccgctcatcaaagacatcatgatgaaatgatgatattccgcataagaatgaggcattttttaaacgcagtgcgctgaagtgtggttggataaaaaagtcaatccattcaggaaatacgggcgtattcttttctttcgacaatgaggccgttggcaaaataaaatgatttacataatcgtttctgatgaatatcttctgctcacataaaaatcacacaataactttgagatcgcagattgttttacttttacagcattcgtccccccattgttgggcaaatatagattgggccagagcacgaaagttaataccacgttcgcacagctcctccaacagcacgacaagatgccacatactgcgccccagtcggttcagtttacagactagcagtgcgttccctgccgatgatgtcctgaccagttttttcagtccggacctcctgccacggttttacgttgaagtggtaaccctgagcacgcagttcttcagtcaggcgtggtgcaccgtaacgctgttattgctgggtaagatcaaaaaactttcaggcagctaaggaaagttgaaccagacattagatgaaatatttcaaccaattacagcaccaattcagtcactgccagcccaccaaataaatcaaggggttacatgaaaacgtagcccctttttctttggtagtgacactaaaatggatgtagtgtgaagaataatcccgtttactcaatcaataatacatattgtttcaatctacgttattatctctttgtaaaaattgccatttattaatcattgaaaactgcttttagaacttgatacaacgggactagtcacaacaggactattctcaacgggatcatcctcagaggaactatcatcaaagtcatcatccataaataaaatatcatcgaatggtgccacgcccgtgatgagttttattttattattacgatcagtcaatactccacttaaaccgttttcgctcacaggttttaatgatttttcattactcttgttgtaagcaggcgcattaaaaatacacggagtatcaacatcaaacaatgacgttccccagttcacatattgaatatcatagttactgaagttctgtccagaaaagaagcaccccttaaaatccaatccacgtaaattatataaaccaccctcttctttttggagagtaatgttaattttggctatctcccggacatcatcgccatttttgtatttgaataccgtttcaagatgttctccagacagcttgacttcaggaaataatttgaaatcaaagcctatattattatgtgtcaacgtagatgaacaaaaaatggaaaaagcttgcagtgctgaattatagctatcgattttatcttgaggctgagctcttggtaaaaacttatagcaacactcataaaaattaaacagaagctctgaagaccttgtatttttatcaaataatacccccttgaactcattcacaaacgcatcttttttttcttgaatatctatggggtgttcctttgactctgacaaagatgaaatctcatctattttgttttcatatgaattacgtgattccatacagacatttggcggcgtttctaaaataacactacgcgtactacttggcttaagtaaaccaacatgaaaatcactttttcttatattatcgaaaaggttctattcatttcttttagcgcattcaaaaaactgatcggcattatttttattcgataattttttagtttcagaaaacacattttcattgttttccagctttagtttaatgagaagattttcccagacctgcttgcttaaacatattacgtcaggctcaccagaactaactaactcgtgattattattaaagtgtacgttgaatacctttaagttattttcaccaacttcatatttaatacgttttaattgttctccagctcccataatgacaaaggcgttgccttcttgatatatacattcagacatcattttttgtaaagtttcaagagcaccgcgatacgtctctgatgcagcttccttacaaattaattttaaaatactatgagctagtagctccatgtgtttagaagatttattttcattataacttccactacccaaaactgcgctagcgttaaatccgttgcttttactaactaacattgtctattcctcaattaatgtctacatggctatttttaatgttattactgtttgtcactataaaaaaacgctcatttgagacaattactgacattaactgcttcacttgctacgcatggaacttttaattaaattagcacaggaatgttaaatttaataaacaaaaggttatttcgctgtatgataaaaaaaaccgttataatttattagtgaaaatcgtttttcaagtgttagaaatttatatctcaatagcgttggttaatgagcatagccacgctcctgtaacgctcacaaaactcatctgcctgcggcgggtgttctggtcagtagtagatgtttaaggcgtggcagagacatttcatccttactctacggcattgttctacatacattggttgtggtactcacttatcatcagtgagcgaacagagaatagttcagtgatttgagtaattaacctgattaaatgaaggggtataataaatgataatactctggctttatcgttaattacttaattccacatgtaagcaatttgcccgcttggcatagcaggcattttttccaggtacttttgaatgagtactgatggataaatacattgcagtggcgtgccacgtaccaaaacaccagccctcattcgaaaccacccaccgcacttcttccttgaaatggcgttagtcatgaaatatagaccgccatcgagtaccccttgtacccttaactcttcctgatacgtaaataatgatttggtggcccttgctggacttgaaccagcgaccaagcgattatgagtcgcctgctctaaccactgagctaaagggccttgagtgtgcaataacaatacttataaaccacgcaataaacatgatgatcatatgatgtaaataacagatttttatgcgttcccattcaccttgggtcgtgattacacgcgacataaaacccgacaccgcctccattcgcaaagtcgatactcgcagtcaacaagcaaatgttaataattagcactatctatagttatcatcgattcaatgatactttgtaatgattttgtatctaataatataactttattacattagctgaagagttttcgcatcattatgatatctgttacttttcactccataaaaataaacttcgtatagcaatatattctttcatagatcttattctgctaatcattagtttcgtatgagcgatttttgacagttgcctctccagaccacatcgataattaataaaacagatttaagcattatccttttccatataaatattggataaaagtaggacatctgtttgcaattactttcacaacaattaaacatttttatgtttccgtatacatcatattactctaccattagaggaactttattatgttttctataaaaccaggacccagaaatttacctatcgacaaccccacattgttatcatggaacattactgacggggatctaaattccaaattaaatacattagaatatctaaactgtataacaaatattattaattcttgtggagtttaccctcaaggattaaaagacagagaaattatatcaacttttcacgcagaaaaagttattaatgatctgttaaaaaacgattataaaatttccctttctccagatacaacttaccgagagttgaataaagcagcacagcgtagcattacagcgccagacaggataggagaaagaaaaacataggtttatcaacgagatacaatgattgaaagaggtgataacagcggtgtttatcagtatggtcgtgctgaacatttcacccacattatatctgacaaaccttccccaaaagataaatatgttgcatatgctattaacattcctgactatgagctggcagccgatgtatataatattaacgtgacgtcaccttccggacagcaagaaacatttaaaatattaatcaatctagaacatctacggcaaacacttgaacgtaaatctcttactgctgttcagaaatcacaatgtgaaatcatcacccccaaaaaacctggcgaagcgattcttcatgcttttaatgccacctaccagcagatcagagaaaatatgtctgaatttgcacgttgccattatgggtatatacaaatccctccagtgacaactttccgcgccgacggaccagaaactcccgaagaagaaaagggttactggtttcatgcttatcaacccgaagatctttgtaccatccataatccaatgggagatttgcaggattttattgcattggttaaagatgctaaaaaatttggtatcgatatcattcctgattatacctttaactttatgggaattgggggtagtggtaaaaatgacctggattatccctctgctgatatacgagcgaagatcagtaaagatatagaaggtggtatccctggctattagcaaggtcaggttttgattccattcattaaagatccagtaacaaaagaacgtaaacaaatccatccagaagatatacatctcactgcaaaagacttcgaagcaagtaaagataacatctctaaggatgaatgggaaaacctccatgcattaaaagaaaagcgtttaaatggaatgcctaaaacaacacccaaaagtgaccaggttattatgttgcaaaatcaatacgttcgtgaaatgcgaaaatatggcgtacgaggtttacgttatgatgcggcaaaacactcaaaacatgaacaaatagaaagatcaataaccccaccgcttaaaaattataatgagcggttacacaatactaacttatttaacccaaaatatcataaaaaagccgttatgaattacatggaatatctggtaacttgtcagttggatgaacaacaaatgtcatcactgctttatgaaagagatgatttaagcgccattgatttttcattgctcatgaaaacgataaaagccttttcatttggtggagatcttcaaacccttgcatcaaaaccgggttccacaatctcaagtatcccatcagaaagacggatattgattaacattaaccacgattttcctaacaatggtaatcttttcaatgactttctatttaaccatcaacaagatgaacaattagcaatggcatatatagccgctctgccgttcagcaggcctttagtttactgggatggccaagtattaaaatcaacgactgaaattaaaaattatgatgggtccacgcgtgtcggcggtgaggcgtagcttaataaaggttgctctacctatcagcagctctacaatgaattccacgcattatatatagataaagcaggaatatggagcgcatttgagggtgtatctgcaactaaaaacgttctggcctttagtcgtggggattctgtgaacattaatcactctcctcatgatggactagttataataaataaaggaaacgaagaagttgaaggtacctggcctaacaaattgcaacctggaatatacaaaaacatggggagtaatagcgttaacattattattaataatacccgaaaaattatcccccctggtaaagtatttacgcttagaggcggaactctaaatatcaatattcctgggcgtagcgctcttcttttagggaaaacaggagaaccgccgaactatctctatttataatttaatgttatatctgccccgataaaacggggcagataatatgtttagtttactaacggtcattttgcagtgaagccatttactgttttttatcgaccagataatctgttctctaatgttaactccccctaacctgttgctttagttattcatttcctgtctcactttgccttaataccctacgttaaatgttactaatttgttgcttttgatcacaataagaaaacaatatgtcgcttttgtgcgcatttttcagaaatgtagatatttttagattatggctacgaaatgagcatcgccatgtcaccctacatctcataagaggatcgcttctgatgaatgcactgaccgccgtacaaaataacgctgtcgattcaggccaggactatagcggattcaccctcaccccgtcggcgcaatccccgcgtctgctggaactcaccttcaccgaacagacgaccaaacagtttcttgagcaggttgccgagtggcccgtgcaggcgctggagtacaaatcgtttctgcgttttcgggtagccaaaattcttgacgatctatgtgcgaaccagctgcaaccattgctgttgaagacgttgctaaaccgcgctgaaggtgcgttgttgatcaatgcggtgggtgtcgatgatgtgaagcaagcggatgagatggtgaagctggcgacggcggtggcgcatctgattggccgttccaatttcgatgcgatgagcggtcagtattacgcgcgttttgtagtgaaaaatgtcgataactcagacagctatctgcgccagccgcaccgcgtgatggagctacacaacgacggcacgtatgtcgaagagataaccgattacgtgctgatgatgaaaatcgacgagcaaaacatgcagggcggaaattcgctgctgctgcatctcgatgactgggaacatctcgacaactatttccgccacccgctggcgcgtcgcccgatgcgctttgccgcgccgccgagtaaaaacgtcagcaaagatgtttttcatccggtgttcgacgtcgatcaacagggtcgcccggtgatgcgctatatcgaccagttcgtccagccgaaagacttcgaagaaggcgtgtggttgagcgagctttccgacgccattgaaaccagcaaaggcattctttctgtgcccgttcccgttggcaaattcctgttgattaacaacctgttctggctgcacggtcgcgaccgctttactccgcacccggatctgcgccgtgaactgatgcgccagcgtggctatttcgcttacgcctctaaccactaccagacgcatcagtaagcgcaaaggaattgagcggatgtatgattttgtgattattggcggcggcatcatcggcatgtcgaccgccatgcaactgattgatgtctatccggacgcccgcattgcgttgctggaaaaagagtccgccccggcctgtcaccagacgggccacaacagcggcgtgatccatgccggggtctattacacgcccggcagcctgaaggcgcagttttgcctggcgggaaaccgcgccaccaaagccttttgcgatcaaaacggcattcgctacgacaactgcggcaagatgctggttgccacgtccgatctcgaaatggaacggatgcgcgccttatgggaacgcacagcggcgaacggtatcgagcgcgaatggcttaacgccgacgaactgcgcgagcgcgaaccgaatatcaccgggctcggcggcatttttgtgccgtccagcggcattgtcagctaccgcgacgtgacggcggcgatggcaaaaatcttccagtccagaggcggtgaaattatctataacgccgaagtcagcgggcttaatgagcataaaaacggcgtggtgatacgtacccgtcagggcggcgaatatgaagcatcaacgctgattagctgttccgggctgatggctgaccggctggtgaaaatgctcggactcgaaccgggctttatcatctgcccgttccgtggcgagtatttccgccttgcgccggagcataaccagattgttaaccacctgatttaccccattcccgacccggcaatgccgtttttgggcgttcatctcacccgcatgatcgacggcagcgtgaccgtcgggccaaacgcggtgctggctttcaaacgcgaaggctatcgcaagcgcgacttctcatttagcgacacgctggagattttgggctcgtcggggattcgccgggtgctgcaaaaccatctacgctcaggactgggcgagatgaaaaactcgctgtgcaaaagcggctatctgcggctggtgcaaaagtattgtccccggctttcgttaagcgatctccagccctggcccgccggtgtgcgggcgcaggcggtatcgccggacggcaagctgattgacgattttctgtttgtcaccaccccgcgcacgatccacacctgcaatgcgccctccccggcagcgacatcagcaattcctattggtgcgcatattgtcagcaaggtacaaacgctgttggcaagccagagtaaccccggacgcacgctgcgagcggcacgtagtgtggatgccttacacgccgcatttaatcaataacctttgaaaacaggatgtagcgatgaaacttaacgacagtaacttattccgccagcaggcgttgattaacggggaatggctggacgccaacaatggtgaagccatcgacgtcaccaatccggcgaacggcgacaagctgggtagcgtgccgaaaatgggcgcggatgaaacccgcgccgctatcgacgccgccaaccgcgccctgcccgcctggcgcgcgctcaccgccaaagaacgcgccaccattctgcgcaactggttcaatttgatgatggagcatcaggacgatttagcgcgcctgatgaccctcgaacagggtaaaccactggccgaagcgaaaggcgaaatcagctacgccgcctcctttattgagtggtttgccgaagaaggcaaacgcatttatggcgacaccattcctggtcatcaggccgataaacgcctgattgttatcaagcagccgattggcgtcaccgcggctatcacgccgtggaacttcccggcggcgatgattacccgcaaagccggtccggcgctggcagcaggctgcaccatggtgctgaagcccgccagtcagacgccgttctctgcgctggcgctggcggagctggcgatccgcgcgggcgttccggctggggtatttaacgtggtcaccggttcggcgggcgcggtcggtaacgaactgaccagtaacccgctggtgcgcaaactgtcgtttaccggttcgaccgaaattggccgccagttaatggaacagtgcgcgaaagacatcaagaaagtgtcgctggagctgggcggtaacgcgccgtttatcgtctttgacgatgccgacctcgacaaagccgtggaaggcgcgctggcctcgaaattccgcaacgccgggcaaacctgcgtctgcgccaaccgcctgtatgtgcaggacggcgtgtatgaccgttttgccgaaaaattgcagcaggcagtgagcaaactgcacatcggcgacgggctggataacggcgtcaccatcgggccgctgatcgatgaaaaagcggtagcaaaagtggaagagcatattgccgatgcgctggagaaaggcgcgcgcgtggtttgcggcggtaaagcgcacgaacgcggcggcaacttcttccagccgaccattctggtggacgttccggccaacgccaaagtgtcgaaagaagagacgttcggccccctcgccccgctgttccgctttaaagatgaagctgatgtgattgcgcaagccaatgacaccgagtttggccttgccgcctatttctacgcccgtgatttaagccgcgtcttccgcgtgggcgaagcgctggagtacggcatcgtcggcatcaataccggcattatttccaatgaagtggccccgttcggcggcatcaaagcctcgggtctgggtcgtgaaggttcgaagtatggcatcgaagattacttagaaatcaaatatatgtgcatcggtctttaactggagaatgcgaatgaacagcaataaagagttaatgcagcgccgcagtcaggcgattccccgtggcgttgggcaaattcacccgattttcgctgaccgcgcggaaaactgccgggtgtgggacgttgaaggccgtgagtatcttgatttcgcgggcgggattgcggtgctcaataccgggcacctgcatccgaaggtggtggccgcggtggaagcgcagttgaaaaaactgtcgcacacctgcttccaggtgctggcttacgagccgtatctggagctgtgcgagattatgaatcagaaggtgccgggcgatttcgccaagaaaacgctgctggttacgaccggttccgaagcggtggaaaacgcggtaaaaatcgcccgcgccgccaccaaacgtagcggcaccatcgcttttagcggcgcgtatcacgggcgcacgcattacacgctggcgctgaccggcaaggtgaatccgtactctgcgggcatggggctgatgccgggtcatgtttatcgcgcgctttatccttgcccgctgcacggcataagcgaggatgacgctatcgccagcatccaccggatcttcaaaaatgatgccgcgccggaagatatcgccgccatcgtgattgagccggttcagggcgaaggcggtttctacgcctcgtcgccagcctttatgcagcgtttacgcgctctgtgtgacgagcacgggatcatgctgattgccgatgaagtgcagagcggcgcggggcgtaccggcacgctgtttgcgatggagcagatgggcgttgcgccggatcttaccacctttgcgaaatcgatcgcgggcggcttcccgctggcgggcgtcaccgggcgcgcggaagtaatggatgccgtcgctccaggcggtctgggcggcacctatgcgggtaacccgattgcctgcgtggctgcgctggaagtgttgaaggtgtttgagcaggaaaatctgctgcaaaaagccaacgatctggggcagaagttgaaagacggattgctggcgatagccgaaaaacacccggagatcggcgacgtacgcgggctgggggcgatgatcgccattgagctgtttgaagacggcgatcacaacaagccggacgccaaactcaccgccgagatcgtggctcgcgcccgcgataaaggcctgattcttctctcctgcggcccgtattacaacgtgctgcgcatccttgtaccgctcaccattgaagacgctcagatccgtcagggtctggagatcatcagccagtgttttgatgaggcgaagcagtagcgccgctcctatgccggaggcgacgctgcgcgtcttgtccggcctacggggatccaggtcggataaggcgtttacgccgcatccgacaatctgtacgtgaacaggaagaaatctatgttggccgggtaaggcggagccgctctccggcaaaaagaatcaataacaattatacgcgtgacccggcgcgggaaatgtcggggcgctctcccaagtgacacactttcgagaggattcaggatggggcaatcatcgcaaccacatgagttaggcggcgggctgaagtcacgccacgtcaccatgttgtctattgccggtgttatcggcgcaagtctgtttgtcggttccagcgtcgccatcgccgaagcgggcccggcggtattactggcctatctgttcgccgggctactggtggttatgattatgcggatgttggcggaaatggcggttgccacgcccgataccggttcgttttccacctatgccgataaagccattggtcgctgggcgggctataccatcggctggttgtactggtggttttgggtactggttatcccgctggaagccaacatcgccgccatgatcctgcactcatgggttccaggcattcccatctggttattttccctcgtcattaccctcgccttaactggcagtaacttattaagcgttaaaaactacggcgaatttgagttctggctggcgctgtgcaaagtcatcgctatcctggcctttattttccttggtgcagtcgcaattagcggtttttacccgtatgccgaagtgagcgggatctcaagattgtgggatagcggcggctttatgcccaacggtttcggtgcggtattaagcgcgatgttgatcaccatgttctcgtttatgggcgcagaaattgtcaccattgccgccgcggaatccgacacgccggaaaaacatattgtccgcgccaccaactcggttatctggcgtatttctatcttctatttatgttctatttttgtcgtcgtggcattaattccgtggaatatgcccggactaaaagccgtcggttcttatcgctcggtactggaattgctcaatattccccatgcgaaattaatcatggactgcgtgatattactttccgtaaccagttgcctgaactcggcgctgtataccgcgtcaaggatgctctactccttaagtcgtcgcggtgatgctcccgcggtaatgggtaaaatcaaccgcagtaaaaccccgtacgtggcggtgttactctccaccggcgcggcattcttaacggtggtggtgaactattacgcgcctgcgaaggtatttaaatttctgatcgacagctccggcgctatcgccctgctggtttatttagtcatcgccgtttcacagttgcggatgcgcaaaattctgcgagcagaaggaagcgaaattcgcttgcgaatgtggctttatccgtggctcacctggctagtcatcggctttattacctttgtgttggtagtgatgctattccgtccggcgcaacagttagaagtgatctccaccggcttattagcgatagggattatctgtaccgtgccaattatggctcgctggaaaaagctggtattgtggcaaaaaacacccgttcataatacgcgctgatcatgatcaggagtcacaccatgaccattacgtctctggatggctatcgctggctgaagaacgatattattcgcggtaattttcaaccggatgaaaaattacgaatgagtttgctgacatcgcgttatgcacttggcgttgggccgttacgggaagctctttcgcaactggtggcggaacggctggtcacggtggtgaatcaaaaagggtatcgggtggcgtctatgtcagagcaggagctgctcgatattttcgacgcccgcgccaatatggaagcgatgttagtgagtctggcgattgcccgcggtggcgatgagtgggaggcagacgttctcgcaaaagcgcatctgctgagtaagcttgaggcctgtgacgccagcgagaaaatgcttgatgagtgggatctgcgtcatcaggcgtttcatacggcaattgtggcgggctgtggttctcactatttgctgcaaatgcgtgaacggttgtttgatctggcggcgcgttatcgatttatctggctgcggcgaacggtgctttcggtggaaatgctggaggataaacacgatcagcaccagaccctgactgcggcggtactggcgcgagataccgcgcgcgccagtgagttaatgcgccagcatttactgacgccaattcccattatccagcaggcgatggctggcaattaactactcttccggaatacgcaacacttgccccggataaattttatccgggctttttagcatcggtttattcgcttcgaagattttattgtacagattagcgttaccgtagacctgtttggaaatggcactcagagtgtcgccagacttaacggtataaaactggctggcagtggctggtgtcgccgttttcacctgatcatcgacactggcaataccggaaatattccccaccgcaacaaggattttctccttcgcctcctgactcaggccgtcaccagtgaccgtcgctttgccgtcggcaatttgaatattcactttatcggcatccggtataccggttttgttcagatgctcctgcaccttcttcgcctgatcgtctttatcgtgctgacctgtaaccgcgtcccagagtttttctccggcatctttcacaaaattgaacagacccatagctacctcattcgttaacggaaacactcagaaagtgtagcagaggaacgcggcgcgttaacgccgcggggatgagcacaggtttaatcgcgggtttgcacccagaacgcgtgaatcaaaccggggatatacccaagcagtgtcaacagaatattaataatgaacgcccaaccgaaccctttaccgagcagcacgccgagcggcggcagaatgatggtgatgacgattctccagaaacccatatgtactccctataagaaaattactcattgtttaaaaagagattttatctcttaagcgtagtaattttagcggagcctgccagtttcagcttacgcttttactctcatttacgctgctgaggctggtatatgttgcatttttagtttagagtttacttaatttagaaaatacttaaataaatatgactgaactcgcgcaattacaggccagtgccgaacaggcagcggccttattgaaagcaatgagccaccctaaacgattgctgattctgtgcatgcttagcggttcccccggcaccagcgcgggagagctgacgcgcattaccggactgagtgcctctgcgacatcacagcatctcgctcgtatgcgggacgaagggcttatcgacagccaacgggatgcccaacgcattctatattccattaaaaatgaggcggtaaatgccattatcgccaccctgaaaaatgtctattgtccgtaaggagtcactatggctttgacaaccatttcgccgcatgatgcacaagaattaatcgcacgcggcgcaaagttaatcgatattcgtgatgctgatgaatatcttcgtgaacatattcctgaagcagatctggctccattatccgtgctggaacagtcaggtcttccggctaaattacgtcacgagcaaattatattccactgccaggcaggtaaacgcaccagtaataatgccgataaattagcagcgattgccgcccccgcagaaatctttttactcgaagatgggattgatggctggaaaaaagcaggattgccagtagcggtaaataaatctcaacccttgccgttaatgcgccaggtgcagatcgctgcgggtggtttaatattaatcggcgttgtactgggttataccgtaaatagcggtttcttcttattaagtggctttgttggtgccgggttactgtttgcaggaatcagcggtttttgtggaatggcaaggttgttagataagatgccgtggaaccaacgagcttgagaagcgacgccggacgcgccctagcagcgacatccggcctcagtaattagatcaggaaatcgtcgagagatttaccttctgccagcgcctgagcaattggcttcggtgtacggccctgaccggtccaggttttagtttcaccgttaacatcggtgaatttatatttcgccggacgcggctggcgttttttaccagcgcgtggtgcagcagcagagctattacccaataactcttccgggttaattccgtcagctttcatcagctccagccaggtgctaattttttcctggcgctctgccagttcacgctgctgctgttcttcttcttcacgtctttctttagtgacaaccctgaatttttcgagcatttcttcaagaacgtcaatggagaattcgcgagccatcgcacggagggtgcgaatgttatttaaactttgtaacattacggacataataaagaaaaccttttaacgccaaaacaaaaaaagtatttcgtcgcgtagtgtaagcgatcacttattatatttccacaaaatttaatctatttacagtcctgcgcgagattatttcagctgttattttctgaaactctcagaataatttcaagattatatattagccattttgatgagtaatttagattattggtgaacagagcggcgctctctgctcgctaattccgcaagcctgacaaaatcaaagtgaataaaaatgcaatataacagaataaaagaaaacatccatcactggtgctttctgctgttaatgtacattgtctggcataaaaaatgctgaaaatgacccagctactacatacaccgaattctctacgcttatagcgttacctcacccccaaactttcattagtgatattaaaggtaaggccatatctaattgatttaattaaaaataaatcatatcggcatgtaaaaatccacaatgtacaaaaaacgagccgttacggaatattttatctacaaaaactgactaaataaaaatttttcactaattgattagtcatagccagcgatatacgctatgcgaaaatgcagatggcaatgagatccactgctttcatctccattaacatcccattacgcttttattaaggagcattagcatgttctcaccgcagtcacgcttgcgtcatgcagttgcagatacgttcgcgatggttgtttactgttctgtcgtgaacatgtgtattgaagttttcctctccggaatgagcttcgaacagtctttttattccagattggtagcgattccggtgaacatcttaattgcatggccatacggtatgtaccgtgatctgtttatgcgcgcggcacgcaaagttagcccgtcgggctggataaaaaatctggcggatatcctggcttatgtgacgttccagtcaccggtgtatgtggcgatcttgttagtggtgggcgcagactggcatcagattatggcggcggtcagttcaaacatcgttgtttcgatgttgatgggggcggtttatggctacttcctcgattattgccgccgactgtttaaagtcagccgttaccagcaggtaaaagcctgactcttcttttcgcgactggcatcgccagtcgcgtctttaactggcttcgccaaataaaccattcaaataacgttcaagcgcaacacgcgaactaaagccatgcgggataccgtaatgctcgtgtcgctcgcctgctaaatagagcggaaattgctggtaatgatcgcaagttttaatatcggaagcgggttcagccagtgtcgaactgcgttcttttaatgttggatgaattaccagagcggtacgtcccattcgcgcttcgcgattaacatagacataattttccccacggcggtaaccatacgctttctgggttaccacatcgacagtaaaaccgactttttcaagtacgcgcgccacctcgtctggtcgtaaatacatatttgatcctcgttattatcaaccgcgggcctaccttacctgattgcgcattcacaacgctttcagaaaagtccataaagccgcgatgaacctcagttaagaaaattatggtctacactgaaaattacatcgaattctaatgggggatcatatgtttaaccgaccgaaccgcaacgacgttgatgatggcgtgcaggatatccagaatgatgtcaatcaattagctgacagcctcgaatctgtattgaagtcctggggcagcgacgccaaaggggaagctgaagccgcacgcagtaaagctcaggcattgctgaaagaaaccagggcgcgaatgcatggtcgtactcgcgtccagcaagccgcgcgcgatgccgttggctgcgcggattcttttgttcgtgaaagaccctggtgtagcgtgggtacagcagctgcggtaggtatttttatcggcgcactgttaagcatgcgcaaatcgtagtgcaaaaatgataataaatacgcgtctttgaccccgaagcctgtcttcggggtttctttttgcctggtgaatcacaaaaatccccctaccccgtcacgctcatatccagggtaatttcgaccactatttgctatatattgtgtggttgaatcttttttcaactacatctagtatctctgtatcaacagagagacaacccgacgcgtatcatcgcgccgtatcttcattttaaacggaaatacgaatcatgcgcattactatttacactcgtaacgattgcgttcagtgccacgccaccaaacgggcgatggaaaaccggggctttgattttgaaatgattaatgtcgatcgcgttcctgaagcggcagaagcgttgcgtgctcagggctttcgtcagttgccggtagtgattgctggcgatcttagctggtctggtttccgtccggacatgattaaccgtctgcatccagcgccacacgcggccagtgcatgagccagctcgtctacttctccagcagctccgaaaacacgcagcgttttatcgaacgtttaggtctgcccgcggtgcgcatcccgctcaatgagcgggaacggattcaggtagacgagccttacatcctgatcgtgccctcttacggcggcggcggtacggctggcgcggtgccacgacaggtaattcgctttttaaacgacgagcacaaccgggcgttgcttcgcggcgttattgcttctggtaatcgcaactttggtgaggcgtatggccgcgccggagatgtgattgcccggaaatgcggcgtgccgtggctgtaccgttttgaactcatgggtacgcaaagcgatatcgaaaacgttcgtaaaggagtaaccgaattttggcaacgacaaccgcagaatgcctgacgcaggaaacgatggattaccacgcgctgaatgcgatgcttaacctctacgatagcgcaggtcgcattcagttcgataaagaccgccaggccgttgacgcctttattgcgacgcatgtgcgtccgaacagtgtgaccttcagtagccagcagcagcgcctgaactggctggtcaacgaaggttactatgatgaaagcgttcttaatcgctactctcgcgactttgtcattacgctgtttacccacgcacacaccagcggttttcgtttccagacattcctcggggcatggaagttttacaccagctatacgttgaagacattcgacggtaaacgttatctggaagattttgccgatcgagtaacgatggtggcgctgacgctggcacaaggcgatgagacgctggcgttgcaactgaccgatgaaatgctgtcaggacgctttcagccagccacgccaacattcctcaactgcggtaagcagcagcgcggcgaactggtttcctgttttttgctgcgtattgaagacaatatggagtcgattggtcgggcggtaaattccgcactgcagctgtcgaaacgcggcggcggcgtagcatttttgctgtcgaatctgcgagaagcgggcgcgccaattaaacgtattgaaaatcaatcttctggcgtaattccggtgatgaaaatgctggaagacgcattttcctatgccaaccaactcggcgctcgtcagggggctggtgcagtctatttacatgctcatcatcccgatattctgcgttttctcgacacgaaacgggaaaatgccgacgaaaaaatccgcattaaaacactgtcgcttggcgtggtgatcccggatatcactttccatctggcaaaagagaatgcgcagatggcgctgttttcgccttatgacgtagagcgagtttatggcaagccgtttgccgatgtggccatcagccaacactatgacgaactggttgccgatgaacgcattcgcaaaaaatacctcaacgcccgtgatttcttccagcgactggcagaaatccagtttgagtccggctatccctacatcatgtatgaagacacggtaaaccgtgctaaccctatcgccgggcgcataaatatgagtaatctctgctcagaaattttgcaggttaacagcgcctcagagtatgacgagaatctcgactatacccgcacaggccatgatatttcctgcaatttaggttcgttgaatattgcgcacaccatggattcccccgattttgcccgcacggtagagactgccgtgcgcggtttaacggcagtatcagatatgagtcatatccgcagcgtgccgtccatcgaagccggaaatgccgcctcgcacgccatcggactggggcagatgaatttacacggctatctggcgcgagaaggcatcgcttatggttcgccggaagcactggatttcaccaatctctatttctatgccatcacctggcatgcactgcgtacctcgatgttgctggcacgcgaacgcggtgaaaccttcgccgggttcaaacagtcacgctatgccagtggtgaatattttagccaatatctgcaagggaactggcagccgaaaacggcgaaagttggcgaactgtttacccgtagcggtattacgttacctacccgtgagatgtgggcgcagctgcgcgacgacgtgatgcgctacggcatatacaaccagaatcttcaggcggtgccgccaaccggttctatctcttatatcaaccatgctacgtcgagtattcatccgattgtggcgaaagtagagatacgcaaagagggcaaaacaggacgcgtttactaccctgccccgtttatgactaacgagaatctggcgctgtatcaggacgcttacgaaattggcgcagaaaagatcatcgacacctacgcggaagcgactcgccatgtcgatcaggggctgtcgctgacgctttttttccccgataccgccaccactcgcgatatcaacaaagcgcagatttacgcctggcgcaagggtatcaaaacgctctattacatccgcctgcgtcagatggcgctggaaggcactgaaattgaaggctgcgtctcctgtgcactttaaggaatatctatgaaactctcacgtatcagcgccatcaactggaacaagatatctgacgataaagatctggaggtgtggaatcgcctgaccagcaatttctggctaccagaaaaggtgccgctgtcgaacgatattcctgcctggcagacattaactgtcgtagaacaacaactgacgatgcgcgtttttactggcctgacgctgctcgacacgctgcaaaatgttatcggcgcgccttctctgatgcccgatgcactcacgcctcatgaagaagcggtattatcgaatatcagctttatggaagcggttcatgcccgctcttacagttcgattttctcgacgctatgccagaccaaagatgtcgatgccgcctacgcctggagtgaagaaaacgcaccgttgcagcgaaaagctcagattattcagcaacattatcgcggtgatgatccgctgaaaaagaaaatcgccagtgtgtttcttgaatcttttttgttctattccggtttctggctgccgatgtatttttccagccgcggaaagctgaccaataccgcggacctgatccgtctgattatccgcgatgaagcagtccacggttactacataggctataaatatcagaaaaacatggaaaagatatctctgggacaacgtgaagagttgaagagtttcgccttcgatttgttgctggaactctacgacaacgagttgcaatacaccgatgagctgtacgccgaaaccccgtgggctgacgatgtgaaagcgtttctctgttacaacgccaataaggctttgatgaatctgggctacgaaccgttatttcccgcagaaatggcggaagtgaatccggcaatcctcgccgcgctttcgccgaatgccgatgaaaatcacgatttcttttccggttcaggctcctcttatgtgatggggaaagcggttgaaacagaagatgaagactggaatttctgagggtgttattttcaaaaatatcactacccgcagcagggaaataattcccgccaaatagctttttatcacgcaaataatttgtggtgatctacactgatactctgttgcattattcgcctgaaaccacaatattcaggcgttttttcgctatctttgacaaaaaatatcaactttctcgatttgctctcagcccttatatcacgggaaattccggcgatttgctcgcatcaatattcatgccacatttgccatcaggggttgcctcagattctcagtatgttagggtagaaaaaagtgactatttccattgggtaatatatcgacatagacaaataaaggaatctttctattgcatggcaattaaattagaaattaaaaatctttataaaatatttggcgagcatccacagcgagcgttcaaatatatcgaacaaggactttcaaaagaacaaattctggaaaaaactgggctatcgcttggcgtaaaagacgccagtctggccattgaagaaggcgagatatttgtcatcatgggattatccggctcgggtaaatccacaatggtacgccttctcaatcgcctgattgaacccacccgcgggcaagtgctgattgatggtgtggatattgccaaaatatccgacgccgaactccgtgaggtgcgcagaaaaaagattgcgatggtcttccagtcctttgccttaatgccgcatatgaccgtgctggacaatactgcgttcggtatggaattggccggaattaatgccgaagaacgccgggaaaaagcccttgatgcactgcgtcaggtcgggctggaaaattatgcccacagctacccggatgaactctctggcgggatgcgtcaacgtgtgggattagcccgcgcgttagcgattaatccggatatattattaatggacgaagccttctcggcgctcgatccattaattcgcaccgagatgcaggatgagctggtaaaattacaggcgaaacatcagcgcaccattgtctttatttcccacgatcttgatgaagccatgcgtattggcgaccgaattgccattatgcaaaatggtgaagtggtacaggtcggcacaccggatgaaattctcaataatccggcgaatgattatgtccgtaccttcttccgtggcgttgatattagtcaggtattcagtgcgaaagatattgcccgccggacaccgaatggcttaattcgtaaaacccctggcttcggcccacgttcggcactgaaattattgcaggatgaagatcgcgaatatggctacgttatcgaacgcggtaataagtttgtcggcgcagtctccatcgattcgcttaaaaccgcgttaacgcagcagcaaggtcttgatgcggcgctgattgatgcgccgttagcagtcgatgcacaaacgcctcttagcgagttgctctctcatgtcggacaggcaccctgtgcggtgcccgtggtcgacgaggaccaacagtatgtcggcatcatttcgaaaggaatgctgctgcgcgctttagatcgtgagggggtaaataatggctgatcaaaataatccgtgggataccacgccagcggcggacagtgccgcgcaatccgcagacgcctggggtacaccgacgactgcaccgactgacggcggtggtgctgactggctgaccagtacgcctgcgccaaacgtcgagcattttaatattctcgatccgttccataaaacgctgatcccgctcgacagttgggtcactgaagggatcgactgggtcgttacccatttccgtcccgtcttccagggcgtgcgcgttccggttgattatatcctcaacggtttccagcaattgctgctgggtatgcccgcaccggtggcgattatcgttttcgctctcatcgcctggcagatttccggggtcggaatgggtgtggcgacgctggtttcgctgattgccatcggcgcaatcggtgcctggtcgcaggcaatggtgactctggcgctggtgttaaccgccctgctgttctgtatcgtcatcggtttgccgttggggatatggctggcgagaagtccgcgagcggcgaaaattattcgtccactgcttgatgccatgcagaccacgccagcgtttgtttatctggtgccaatcgtcatgctatttggtatcggtaacgtgccgggcgtggtggtgacgatcatctttgctctgccgccgattatccgtctgaccattctggggattaaccaggttccggcggatctgattgaagcctcgcgctcattcggtgccagcccgcgccagatgctgttcaaagttcagttaccgctggcgatgccgaccattatggcgggcgttaaccagacgctgatgctggccctttctatggtggtcatcgcctcgatgattgccgtcggcgggttgggtcagatggtacttcgcggtatcggtcgtctggatatggggcttgccaccgttggcggcgtcgggattgtgatcctcgccattatcctcgatcgtctgacgcaggccgttgggcgcgactcacgcagtcgcggcaaccgtcgctggtacaccactggccctgttggtctgctgacccgcccattcattaagtaactctgcacttgcccggtgacgccgggcattatcaccctgccaaaaaaaggaataacaatgcgacatagcgtactttttgcgacagcgtttgccacgcttatctctacacaaacttttgctgccgatctgccgggcaaaggcattactgttaatccagttcagagcaccatcactgaagaaaccttccagacgctgctggtcagtcgtgcgctggagaaattaggttataccgtcaacaaacccagcgaagtagattacaacgttggctacacctcgcttgcttccggcgatgcaaccttcaccgccgtgaactggacgccactgcatgacaacatgtacgaagctgccggtggcgataagaaattttatcgtgaaggggtatttgttaacggcgcggcacagggttacctgatcgataagaaaaccgccgaccagtacaaaatcaccaacatcgcacaactgaaagatccgaagatcgccaaactgttcgataccaacggcgacggaaaagcggatttaaccggttgtaaccctggctggggctgcgaaggtgcgatcaaccaccagcttgccgcgtatgaactgaccaacaccgtgacgcataatcaggggaactacgcagcgatgatggccgacaccatcagtcgctacaaagagggcaaaccggtgttttattacacctggacgccgtactgggtgagtaacgaactgaagccgggcaaagatgtcgtctggttgcaggtgccgttctccgcactgccgggcgataaaaacgccgataccaaactgccgaatggtgcgaattatggcttcccggtcagcaccatgcatatcgttgccaacaaagcctgggccgagaaaaacccggcagcagcgaaactgtttgccattatgcagttgccagtggcagatattaacgcccagaacgccattatgcatgacggcaaagcctcagaaggcgatattcagggacacgttgatggttggatcaaagcccaccagcagcagttcgatggctgggtgaatgaggcgctggcagcgcagaagtaatttttattcgggcggataaggcgtttttgccgcatccgccgttctgtgcacaatgcctgatgcgacgctggcgcgtcttatcatgcctacaaaccacatcgcacatttcaacaatctatctttcatcccatattcatcaacatccgctattattgatttccagcttaatcatcacctgatgaacaaaaataatgactaaacctaatcatgagcttagcccggcgctgatcgtgctgatgtctatcgccaccggtctggcggtagccagtaactattacgcccagccattgctcgacaccatcgcgcgtaacttttccctttccgccagttcggcaggctttattgttaccgccgcgcagttgggctatgccgcaggtctactgtttcttgttcccctcggtgatatgtttgaacgccgccgcctgattgtctcgatgaccttactggcggcatgttgattaccgccagcagtcagtcgctggcgatgatgatcctcggtacggcattaaccggtttattctcagtcgtggcacaaattctggttccgctggcagcgacgctggcttcaccggataaacgcggcaaagtggttggcactattatgagcggtctgctgttggggatcttgctggcacggacagttgccggattgctggcgaatctcggcggctggcgcaccgtcttttgggttgcttcggtgttaatggcactgatggcgctggcattatggcgtggtctgccacaaatgaaatcagaaacccacctcaactacccacagttgttgggttccgttttcagtatgtttatcagcgataaaattctgcgtacccgcgcgttgctgggctgcctgacctttgccaatttcagcattctctggacctcaatggcctttttgcttgccgctccaccttttaactacagcgatggtgtcattggtctgtttggacttgcgggagctgccggagcgttgggcgctcgtccggcgggcggttttgccgataagggcaaatcgcaccacaccacaactttcggtctgctgctgctattactttcatggctggcgatctggtttggtcacacttccgtactggcgttgattatcggaatcctggtgctggatctcaccgtgcagggcgtgcatatcactaaccagacggtaatttatcggatacatcctgatgcgcgcaatcgcctgaccgcaggttacatgactagctactttattggcggtgccgccggttcgctaatttcagcctcagcctggcaacatggcggttgggctggcgtttgtctggctggcgcgacgattgccctggttaacttactggtctggtggcgaggttttcatcgtcaggaagccgcaaattaagcaatcagcaaccgttttcgtggctttacacttataagggtgttaagaagcccatcagtctgataaggttaagatattcattcagtctatttataatattaacaatcgttaagcgtacactctatggaaagccctactccacagcctgctcctggttcggcgaccttcatggaaggatgcaaagacagtttaccgattgttattagttatattccggtggcctttgcgttcggtctgaatgcgacccgtctgggattctctcctctcgaaagcgtttttttctcctgcatcatttatgcaggcgcgagccagttcgtcattaccgcgatgctggcagccgggagtagtttgtggattgctgcactgaccgtcatggcaatggatgttcgccatgtgttgtatggcccgtcactgcgtagccgtattattcagcgtctgcaaaaatcgaaaaccgccctgtgggcgtttggcctgacggatgaggtttttgccgccgcaaccgcaaaactggtacgcaataatcgccgctggagcgagaactggatgatcggcattgccttcagttcatggtcatcgtgggtatttggtacggtaataggggcattctccggcagcggcttgctgcaaggttatcccgccgttgaagctgcattaggttttatgcttccggcactctttatgagtttcctgctcgcctctttccagcgcaaacaatctctttgcgttaccgcagcgttagttggtgcccttgcaggcgtaacgctattttctattcccgtcgccattctggcaggcattgtctgtggctgcctcactgcgttaatccaggcattctggcaaggagcgcccgatgagctatgaggttctgctgcttgggttactagttggcgtggcgaattattgcttccgctatttgccgctgcgcctgcgtgtgggtaatgcccgcccaaccaaacgtggcgcggtaggtattttgctcgacaccattggcatcgcctcgatatgcgctctgctggttgtctctaccgcaccagaagtgatgcacgatacacgccgtttcgtgcccacgctggtcggcttcgcggtactgggtgccagtttctataaaacacgcagcattatcatcccaacactgcttagtgcgctggcctatgggctcgcctggaaagtgatggcgattatataacccacaagaatcatttttctaaaacaatacatttactttatttgtcactgtcgttactatatcggctgaaattaatgaggtcatacccaaatggatagttcgtttacgcccattgaacaaatgctaaaatttcgcgccagccgccacgaagattttccttatcaggagatccttctgactcgtctttgcatgcacatgcaaagcaagctgctggagaaccgcaataaaatgctgaaggctcaggggattaacgagacgttgtttatggcgttgattacgctggagtctcaggaaaaccacagtattcagccttctgaattaagttgtgctcttggatcatcccgtaccaacgcgacgcgtattgccgatgaactggaaaaacgcggttggatcgaacgtcgtgaaagcgataacgatcgccgctgcctgcatctgcaattaacggaaaaaggtcacgagtttttgcgcgaggttttaccaccgcagcataactgcctgcatcaactctggtccgcgctcagcacaacagaaaaagatcagctcgagcaaatcacccgcaaattgctctcccgtctcgaccagatggaacaagacggtgtggttctcgaagcgatgagctaacgcgtcatctcgctcaaaaatccagatttataaaagaaaaaatgactggccagcatcgcaacatgctggcctttttggcaagcaggtcggctcagccgatgagttaagaagatcgtggagaacaatatgagcgcaaatgcggagactcaaaccccgcagcaaccggtaaagaagagcggcaaacgtaagcgtctgctcctccttctcaccttgctctttataattattgccgtagcgatagggatttattggtttttggtactgcgtcacttcgaagaaaccgatgacgcatacgtggcagggaatcaaattcaaattatgtctcaggtgtctggcagcgtgacgaaagtctgggccgataacaccgattttgtaaaagaaggcgacgtgctggtcactctcgacccgacagatgctcgccaggcgtttgaaaaagccaaaactgcactggcttccagcgttcgccaaacccaccagctgatgattaacagcaagcagttgcaggcgaatattgaggtgcagaaaatcgccctcgcgaaagcacaaagcgactacaaccgccgtgtgccgctgggcaatgccaacctgattggtcgcgaagagctgcaacacgcccgcgacgccgtcaccagtgcccaggcgcaactggacgtcgcgattcaacaatacaatgccaatcaggcgatgattctggggactaaactggaagatcagccagccgtgcaacaggctgccaccgaagtacgtaacgcctggctggcgctggagcgtactcgtattatcagtccgatgaccggttatgtctcccgccgcgcggtacagcctggggcgcaaattagcccaacgacgccgctgatggcggtcgttccagccaccaatatgtgggtggatgccaactttaaagagacgcagattgccaatatgcgtatcggtcagccggtcactatcaccacggatatttacggcgatgatgtgaaatacaccggtaaagtggttggtctggatatgggcacaggtagcgcgttctcactgcttccagcgcaaaatgcgaccggtaactggatcaaagtcgttcagcgtctgcctgtgcgtatcgaactggaccagaaacagctggagcaatatccgctgcgtatcggtttgtccacgctggtgagcgtcaataccactaaccgtgacggtcaggtactggcaaataaagtacgttccactccggtagcggtaagcaccgcgcgtgaaatcagcctggcacctgtcaataaactgatcgacgatatcgtaaaagctaacgctggctaatccagaggtgcgtgtgatgcaacagcaaaaaccgctggaaggcgcgcaactggtcattatgacgattgcgctgtcactggcgacattcatgcaggtgctggactccaccattgctaacgtggcgatccccactatcgccgggaatctgggctcatcgctcagccagggaacgtgggtaatcacttctttcggggtggcgaatgccatctcgatcccgcttaccggctggctggcaaagcgcgtcggggaagtgaaactgttcctttggtccaccatcgcctttgctattgcgtcgtgggcgtgtggtgtctccagcagcctgaatatgctgatcttcttccgcgtgattcaggggattgtcgccgggccgttgatcccgctttcgcaaagtctattgctgaataactacccgccagccaaacgctcgatcgcgctggcgttgtggtcgatgacggtgattgtcgcgccaatttgcggcccgatcctcggcggttatatcagcgataattaccactggggctggatattcttcatcaacgtgccgattggcgtggcggtggtgttgatgacactgcaaactctgcgcggacgtgaaacccgcaccgaacggcggcggattgatgccgtggggctggcactgctggttattggtatcggcagcctgcagattatgctcgaccgcggtaaagagctggactggttttcatcacaggaaattatcatccttaccgtggtggcggtggtggctatctgcttcctgattgtctgggagctgaccgacgataacccgatagtcgatctgtcgttgtttaagtcgcgcaacttcaccatcggctgcttgtgtatcagcctcgcgtatatgctctacttcggcgctattgttctgctgccgcagttgttgcaggaggtctacggttacacggcgacctgggcaggtttggcctctgcgccggtagggattattccggtgatcctgtcgccgattatcggccgcttcgcgcataaactggatatgcggcggctggtaaccttcagctttattatgtatgccgtctgcttctactggcgtgcctatacctttgaaccaggtatggattttggcgcgtcggcctggccgcagtttatccaggggtttgcggtggcctgcttctttatgccgctgaccaccattacgctgtctggtttgccaccggaacgactggcggcggcatcgagcctctctaactttacgcgaacgctggcggggtctatcggcacgtcgataaccacgaccatgtggaccaaccgcgagtcgatgcaccatgcgcagttgactgagtcggtaaacccgttcaacccgaatgcccaggcgatgtacagtcaactggaagggcttgggatgacgcaacagcaggcatcaggctggattgcccagcagatcaccaatcaggggctgattatttccgccaatgagatcttctggatgtcagccgggatattcctcgtcctgctggggctggtgtggtttgctaaaccgccatttggcgcaggtggcggcggaggcggtgcgcactaagtacaactaagccagttcatttgaactggcttttttcaattaattgtgaagatagtttactgactagatgtgcagttcctgcaacttctctttcggcagtgccagttcttcgttgctgttgatgcgtacgtcacgttccagaatgctacgcgcaatatcctgcgcttcctgcaacgagtgcatctggtaagtgccacactggtagacgttcagttccgggatctgattctgatcctgcactttcagcacgtcttccattgccgctttccaggcatcagcaacacgctgctcatctggcgtaccaatcagactcatataaaaaccggtgcggcagcccattggcgagatatcgataatctctacaccattaccgttaagatggttacgcataaaaccagcaaacaggtgctccagggtatggatccctctttctggcatcacttctttgttcggcacgcagaagcgcagatcgaacacggtgattgcgtcgccatgcggggtgttcattgttttcgccacccgaactgcaggcgcttccatccgggtatgatcgactgtgaagctatctaacaacggcatttagccacctccggtaatttttttaaaaattttctgaactctttcttcccaggcgagtctgagtatatgaaagacgcgcatttgttatcatcatccctgaattcagagatgaaattttggccactcacgagtggcctttttcttttctgtcaggcgtgtttttccagccacaccgcaaacggttcggtatcagcggcttccatttcctgctgacggcgttcagacgcctcgcgctcggctacaaaatcctcttcgcgcagaatttccagcggctcttcacgcagcagattacggtaggcttctgcaaatgctttgcctgttccgccaataccagtatcaatcatagaccttaagatacgggcagagaaagtcagatcgggattatcgaagcaggcaaccagttcatcacacactttctgatacgcttcgccgccgttaatactatccagcgtttgcgcgacgcgtttcagatcgcggaacagatctttacccacctgcggtaacgggaactgtgcggtttcgcagccgatacccagcgtcagacccggtttgcgaccttcgaggatcacccggttccagttaacgcgtgtacaggcaagttcgctactgctcatttccggtgcatcagccagcgcacaccagaccataaacaggtcgaggaatcgcacctgctgttcatctacaccaatcggcgagaacgggttgatgtccagcgaacgcacttcaatatattcaatgccgccacgtaacagcgcatcagaaggcgactcgccgctgcgggtaacgcgttttggacgaatcggcgcgtacagttcgttttcaatctgcaacacgttgctgttgatttgcagcctcttaccgtctttctcaataccaatcttcgcgtactcttccgatggcgttttgattgcctgtttaaggcccgctacgtactcgtaaagatcgttgaaggtaataccaagattgctttgcgatttattggtatagccgagatcgctcaaacgaagagaggtcgcatacggcaggtaatacataccgcactcggttttctcaaacggcagcgacgttggttttccttgcaggaaagaagaacaaatcgccggagatgcaccaaacagataaggaatgacccaaccgaaacgatagtaattgcggataacgcggaaatagcccgcagaaattttctctttggcatcagcgcccgagatatcaccgcacttcgcttgccagaatgccattggcaaagagaaattgtagtgcacgccggaaatggtttgcatcagcgcgccgtagcgatttttcagcccttcacgatacagcgttttaaagcgtccggtgttagaagtgccgtactgtgccagttcgatgtcctgaccttctgcgatgtagcatggcatacttaacggccacatccgctcatcgcccatattgcgcgccgtataacgatgcagatcgcgcataaaggtcagcatatgttcaatatcaccatccactggtgtaatgaattccagcaatgcttccgcaaaatcggtagtaatccatttgtgcgtcagtgcggaacctaatgcttcaggatgacctgttgttgccagtgtgccatcagcattaacacgcaaagtttcgcgctccagcccacgctgtatcccctttaacgcctgaggatgtttttccagccaggccagcgcctgtgatacgtccgggatcaaattgacctcccgcctgtcaaaatcgttttaattagcataactgtaatggtgaccatatgtgcaggcctacaattagtgccaccacatcatgccctgaacggtcgctgctgcaactgcaacatagcgtaacgctttaccaaggcacaaaaaaaagattaccggtccccacgagatgcgcatccatcccgctaacagacacagtaaatcgccaaccacgggcatccagcttaataatagcgtgactgcaccatagcgtttcagccagccggtagctttctcttgccagcgcgatgttttacgcaatggaaagaaacgcccaaggataacgttagttaaccctccaaggctattacccattgttgctgttaaaactaaaacccagggatgactgatcccggaaagcaacattgccaccagcacgacttcggagttgccgggtaatagtgtagcgctgagaaaactactggcaaacaacgagaaaagcgataacgcttcactcacagcaagcgaacatccacggcgtccatgcctgctgcacgggccgcctgaataccgaaatcggcatcttcaaagaccacacactgcgtcggttgcacgcccatacgctgcgcgcacaacaaaaatgtgtctggcgcgggtttatggtgtttgacgtgatcggcagcgacgacggcgtcaaaataatggcgtaatcccaggtgcgccagcaatgcctcagcgatggcgctttcactccccgttcctacagccattgggcgacgaccatgccaacttttcaccacatcaacaagaggaagcggttcgacgctatccagcagcatacttcttactgcttctgttttttcacgcgctaacgcatgcgggtcgagatcggcctgattcagctcaataattgcctgagcaatacgccaggtgggcgatccattaagcgcaatcatcgcctgaatatcgtactgaagaccgtagtgccctaatacttcgcgccacgctttacggtgcgtaggctccgtatccaggattgtgccatccatatcaaaaattaaacctgcataacgctcgtacatggtcttctcgcaagtcgaaaaatatgacgctactttagcgtaattgcttgattttgtcgctgatggcgaaggagaagaaaattcaggaaatggataaaggagttatttagaaatgagatatttttgaaggaaattttttggagaagatggtgcatccgggaggatgactcactgacgttcgcccttcgggccgttgctggcgcaacgttatccttcctggtgcctgcggttaataccgctatctcttcgataccttcattgctgaaggttacggagaatatggtgcatccgggaggattcgaacctccgaccgctcggttcgtagccgagtactctatccagctgagctacggatgcatcgggaaaacttattctactgctgatattgataccgctactaaagccatatcaattaagagatggtgcatccgggaggattactcgccttgcggctcgcccttcgggccgttgctaaagcaacgttatcatccctagtgcctgcggttaattccgctacctcttcgataccttcattgctgaagatttcggagaatatggtgcatccgggaggattcgaacctccgaccgctcggttcgtagccgagtactctatccagctgagctacggatgcatcgggaaatttattttactgctgatattgataccgctactaaagccatatcaagtaagagatggtgcatccgggaggattcgaacctccgaccgctcggttcgtagccgagtactctatccagctgagctacggatgcatcgggaaacttactttactgcagattttttgataccgctactaaagccgtatcaagtaagagatggtgcatccgggaggattactcgccttgcggctcgcccttcgggccgttgctaaagcaacgttatcctccctggtgcctgcggttattaccgccacctcttccataccttcatcgctgaaagtacgtagaatatggtgcatccgggaggattcgaacctccgaccgctcggttcgtagccgagtactctatccagctgagctacggatgcaaatggcggtgaggcggggattcgaaccccggatgcagcttttgaccgcatactcccttagcaggggagcgccttcagcctctcggccacctcaccacacgcctcttacgagtgcttcgaagaacttgtttatcgctcatcgtcgctgcgtggcgcacatattactttctgagacttataagtcaaacaatttttcctacacttttatcgtttgcacacttcacgttcaattagtctgtaaaaacgtcaaaaagagtgttttatcaacagaagaatggaggtctgacagatagtagtaatgcaaaaaaatggagacttaagttgaatgaacgggagtaaagcgaaaagactatagagtgaaggagaaattttgagggtgcgtctcaccgataaagatgagacgcggaaagattagtaactggactgctgggatttttcagcctggatacgctggtagatctcttcacggtgaacagaaacttccttcggggcatttacgccaatacgtacctggttgccctttacccctaaaactgtcacggtgacctcatccccaatcatgagggtctcaccaactcgacgagtcagaatcagcattctttgctccttgaaagattaaaagagtcgggtctctctgtatcccggcattatccatcatataacgccaaaaagtaagcaatgacaaacacattacatctaagcagtcatggcattacattctgttaaacctaagtttagccgatatacacaacttcaacctgactttatcgttgtcgatagcgttaatgcgaatgccgtgaagcgagtccacggcattgcctgacgcttatattattgcaatttcgcgctgacccagcctttcacactggctaacgctgcaggtaaggccgcagcatccgtaccaccggcttgcgccatgtcaggacgtccaccacccttgccgcccacctgctgagcgaccataccaatcagttcccctgctttcacacgatctgtgacgtccttagatacgcctgcaatcagagaaaccttaccttcgactaccgttgccagcacgataattgtcgaccccagctgattttttaaatcgtcaaccatggtacgcaacattttcggctcaacaccgctaagctcgctaaccaacagcttaacaccattaacatcaattgccttactggaaagatttgcgctctcctgtgcggcagcttgttctttaagctgttgtaactctttttccagctgacgcgtacgttccagtactgagcgcactttatcagccagattattgctatcgcctttcagcagatgcgcgacttcgcttaagcgatcgctgtctgcatgaacggtggcgatagcaccttctccggttaccgcttcgatacgacgaacgcctgcagcagtacccgattcagagatgatgcggaacagaccaatatcaccagtgcggctggcgtgagtaccgccacacaactcggtagagaaatcgcccatgctcagcacgcgtacgcgctcatcatacttctcgccgaacagcgccatcgcacctttcgctttcgccgcttcgagatccatgatgttggtttcgatcggcaaattgcgacgaatctgtgtgttcaccaggtcttcgaccgcacgaatctcttctggtttcatcgcttcgttgtgtgagaagtcgaagcgcagcaccttgtcgttaaccagtgaacctttctgcgatacatgagtacccagaacctggcgcagcgcagcgtgcatcaggtgcgttgcggagtgattcagacgaatacgggcgcgacgagcctcatcaacatcagcctgcaccgcgtcgcccactttcagagaacccgcagcaagtttaccgatgtgaccaatcgcctggccgtatttctgcgtatcttccaccgcaaaggagaagttagcgcctttcagttcgcctttatcgccaacctgaccgccggattccgcatagaatggcgtttgatccagcacgaccacagcttcctggcctgcattgatggcatcaaccgctttaccatcaacaaacagcgcagtcactttgccgttcagttccagatggtcatagcctttaaattcagatgcactgtcaacacggatcattgcgttgtaatcggcaccaaagccgctggcttcgcgcgcgcgacgacgctgctcttccattgcagcttcaaaaccagcttcgtcaactttgatgttgcgctcacgacaaacatcagccgtcaggtcaaccgggaagccataggtgtcgtacagacggaaagcagtttcaccatccagcgtatcaccagaaagttttgccagctcttcatccagcaacgccagaccgcgctccagagtacgagcaaactgctcttcttcagtcttcagcacctgctcaacctgcgcctgctggcgtttcaggtcttcacccgcagagcccataacgtcgatcagcggaccaaccagtttgtagaagaaggtttctttcgcgccgagcatattaccgtgacgcactgcgcgacgaatgatacgacgcagtacataaccacggttttcattggacggcattacgccatccgcgatcaggaacgcacaagaacgaatgtggtcagcgattacgcgcagcgatttattgctcagatcggttgcgccagtgactttcgctaccgcctggatcagcgtgcggaacaggtcgatgtcatagttagagttaacgtgttgcagcaccgcagcaatacgctccagacccataccggtatctacagacggcttcggcagcggttccatcgtgccatcggcctggcggttgaactgcatgaagacgatgttccagatctcaatgtagcggtcgccgtcttcttccgggcttcccggagggcccccccaaatgtggtcgccgtgatcgtagaagatttcggtgcacgggccgcacggaccagtgtcacccatctgccagaagttgtcagatgcgtatggcgcacctttgttatcgccgatgcgaataatacgttcgcgcgggatccctacttctttttcccagatttcgtaggcttcgtcgtcgctttcatagacggtaacccacagacgctctttcggcagggcaaaccatttttcgctggtcagcagttcccatgcaaactgaatggcatcgtgtttgaaatagtcgccgaagctgaagttgcccagcatttcgaagaaggtatggtgacgcgcggtgtaaccgacgttttccaggtcgttgtgtttaccacccgcacgcacgcagcgttgggaagtggtagcgcgggaataattacgcttgtcgagcccaaggaacacatccttgaactggttcatcccggcgttggtaaacaacaaagttgggtcgttatggggtaccagggagctgctggcaactacctgatgtcccttactatggaaaaagtcgagaaacgcctgacggatctcagcggtgctcttgctcataattatcctgaaatcaagctaacgaaatatcgccaccagctccagcgtgtcttaaccgccgggctggtaactgaaaagtgggaataagataagttttcttgactgggaagtaaaataccgtatgcgttcagtcggcaaaatttcgccaaatctcctggatatcttccatcagatagccacgatagagcagaaaacgctggatcttaactttttctgaaaagacagttggcaaaggttcgccatattttcgcgtcgcctgatcgcgcgccagtgcgcaccagtcgatgtcacattcacgcatcgctttttctgtcgcttcgcgggaaatacctttctgattcagttcctggcgaatacgcgcaggtccataacctttgcggctacggctggcgataaagcgcgcaacaaatcggctgtcatcgagatagccatgttcatggcaccaggcaataacgcgctcgtaatcttctgccgtagcatcaatctcttctgggccatttttgcccataatcggtgccgcgagtttacgtcgcagttcttgctcactgtgatcgcgcaccgccagaatgcgtaccgcacgatccaacaggcgagcatatgccgggcgacgggatgttgattctgtcatggcatatccttacaacttaaaaaagcaaaagggccgcagatgcgacccttgtgtatcaaacaagacgattaaaaatcttcgttagtttctgctacgccttcgctatcatctacagagaaatccggcgttgagttcgggttgctcagcagcaactcacgtactttcttctcgatctctttcgcggtttccgggttatctttcagccaggcagtcgcattcgctttaccctgaccgatcttctcacctttgtagctgtaccacgcgcctgctttctcgatcagcttctcttttacgcccaggtcaaccagttcgccgtagaagttgataccttcgccgtagaggatctggaattcagcctgtttaaacggcgcagcgattttgttcttcaccactttcacgcgggtttcgctacccaccacgttttcgccctctttcaccgcgccgatacgacggatgtcgagacgaacagaggcgtagaatttcagcgcgttaccaccggtagtggtttccgggttaccgaacatcacaccaattttcatacggatctggttgatgaagatcagcagcgtgttggactgcttcaggttacccgccagcttacgcatcgcctggctcatcatacgtgccgcaaggcccatgtgagagtcgccgatttcgccttcgatttccgctttcggcgtcagtgccgccacggagtcaacgacgataacgtctactgcgccagaacgcgccagggcgtcacagatttccagtgcctgctcgccggtgtccggctgggagcacagcaggttgtcgatatcgacgcccagtttacgtgcgtagattgggtccagcgcgtgttcagcatcgataaacgcacaggttttaccttcacgctgcgctgcggcgatcacctgcagcgtcagcgtggttttaccggaagattccggtccgtagatttcgacgatacggcccatcggcagaccacctgccccaagcgcgatatccagtgaaagcgaaccggtagagatggtttccacatccatggaacggtcttcacccaggcgcatgatggagcctttaccaaattgtttctcaatctggcccagtgctgccgccaacgctttctgtttgttttcgtcgatagccatttttactcctgtcatgccgggtaataccggatagtcaatatgttctgttgaagcaattatactgtatgctcatacagtatcaagtgttttgtagaaattgttgccacaaggtctgcaatgcatacgcagtagcctgacgacgcaccgcatcacggtcgccgctgaagcattcccgccgggtaatgccttcaccgcgggcagtggcaaaagcaaaccagacggtgccgacaggcttctcttcactgccgccatccggcccggcgataccactaatagacacggcataatcagcacgagccgctttcagtgcgcctatcgccatttccaccacgacgggttcactcaccgcgccatgctgcgccagcgtctcttcgcgtacgccgatcatctgcgctttggcttcgttactgtaggtgacaaatccgcgttcaaaccaggcggagctaccggcaatatcggtaatcactttcgctacccaaccaccggtacaagactcggcagttgttacggttgcgccacgggctttcagcgcctgcccaacctgttcacttaactgcatcagttcactgtcagtcatcacaacctctgtcagtcaaaaatttatgccggacaagatagcactttcgtcaggaagatggtgttggcgttgcaattttacgaggaggattcagaaaaaagctgattagccagagggaagctcacgcccccctcttgtaaatagctactgtactcgcgccagcgccacggcttgtcctaactgccagaccgccattgcgtaatgggtgctgtggttgtaacgggtgatggtgtagaagttcggcagaccgtaccagtactggtagccggtgccaacatccagacgcagcaggctggcttgttgatggttgcccagcggctgctgtggcgttaaacctgcggcggcaagctgcgaaatgctgtacttagttttgaagccatttggcaagcctggagcctgaccgtttgccattaccgcgacctgatcgcctttcacccagccgtgcgctttgaaatagttcgccacgctaccgatcgcatcaaccggatcccacaggttgatatgcccgtcgccgctgaaatctaccgcatattgtttgtaagacgacggcataaactgtccgtagcccatcgccccggcaaaggaacctttcagattgagcggatcgtcctgctcgtcgcgcgccatcaacaggaaggtttccagctcgccagagaaatactccgcgcggcgtgggtagttaaatgacagcgttgccagcgcatcgaggatgcgagttttccccatcacgcgcccccagcgggtttcaacgccgataatcccgacgataatttccggcggtactccatacacctgccacgcgcgattcaacgcatcttcatactgattccagaaaaccacaccgttctgcacgttgtccggcgtaataaattttttgcgataacggagccatgcgccgttcggacctgatggcggtttcaccgatgtggttggtgcctggttatccatcagccgcagtaccgaatccagacgcttcgcctgggagagaatttcctgcaactgctgacgatcgaaaccgtgtttgttcaccattttgtcgatgaactgctgggcattcgggttattagcgaaatcgccgcccatctgcatcacattgtgctgcggctcaagcaggaagccgccagacggcgttccggtggtcgtatcagtctcagtaggttttggcttgctgctacaggcggcaagcaacacaaaaaggggaagcaatgttacataacgacgcttgaacatgaggggtccatttaacagattcaaccaggggcaagtatggtaaagcatcacgccccgcacaaggaagcggtagtcactgcccgatacggactttacataactcaactcattcccctcgctatccttttattcaaactttcaaattaaaatatttatctttcattttgcgatcaaaataacacttttaaatctttcaatctgattagattaggttgccgtttggtaataaaacaataaatcctgaaggagagaacaatgatagaaaccattactcatggtgcagagtggtttatcgggctgttccaaaagggcggagaggtgtttaccgggatggtgaccggcattcttccgctgttgattagcctgctggttatcatgaacgcactgattaattttatcggtcagcatcgtattgaacgttttgctcaacgttgcgccggtaaccctgtttcccgttacctactgttaccgtgcattggcacgtttgtcttttgcaatccgatgaccctaagcctgggtcgctttatgccggaaaagtacaaacccagctactacgcggcggcctcttatagctgccactcaatgaatggcctcttcccccatatcaaccctggcgaactgtttgtttatcttggcattgccagcggtctgacaacgctgaacctgccacttggcccactggcggtgagttatctgctggttggtctggtcaccaatttcttccgcggctgggtgaccgatctgaccaccgccatttttgagaaaaagatgggcattcaacttgaacaaaaagttcacctggcaggagcaacatcatgacgcatattcggatcgaaaaaggaacgggtggctggggcggcccgcttgagctgaaagccacgccgggaaaaaaaatcgtctatatcaccgccggtacccggcctgcgattgttgacaaactggcacagcttactggctggcaggctattgacggatttaaagaaggtgaacccgcggaggcggaaattggtgtcgcggtaatcgactgtggcggcacattacgctgcggcatctatccgaaacgacgtattcccaccattaatatccactcgacgggcaagtccggtccgctggcgcagtacattgtggaagatatttatgtctctggcgtaaaagaagaaaacatcactgtagtaggtgatgcgacaccacaaccctcttccgtgggccgtgactatgacaccagtaagaaaatcaccgaacaaagcgatggtttactggcgaaggtgggaatgggcatggggtccaccgttgcggtgctgtttcaatctggtcgtgacaccatcgacactgtattaaaaaccattctgccgtttatggcattcgtctcggcgctcattggcatcattatggcttctggccttggtgactggattgcccacggtcttgctccgctggcgagccatccactgggtctggtcatgctggcgctcatctgttccttcccactgctttcacctttcctcggcccaggcgcagttatcgcacaggttatcggcgtattgattggcgtgcagattggtctcggcaatattccgccgcatctggctttaccggcactgtttgccatcaacgcgcaggcggcctgcgacttcatcccggtcggtttgtcgctggcggaagcccgtcaggacacggttcgcgtcggtgtcccttctgtactggtgagccgctttttaaccggcgcgccgactgtactgatcgcctggtttgtctccggttttatctatcaatagaggctgaaacatgaccgttatttatcagaccaccatcacccgtatcggcgcgagtgccattgacgccctcagtgaccagatgctcatcacctttcgtgaaggcgcgcctgcggacctcgaagagtattgcttcattcattgccacggcgagttgaaaggtgcactccatcccggtttgcaattttcactcgggcagcatcgctatccggtgaccgctgttggcagcgtggcggaagacaaccttcgcgaactgggtcatgtcaccctgcgcttcgatggtttaaacgaagcggaatttccgggcactgtccatgtggcaggccctgtccccgacgatatcgcgccgggatcggttttgaagtttgaatctgttaaggagtaaaaaatgaatcaggttgccgttgtcatcggtggtgggcaaaccttaggcgcgttcctgtgccacggtctggctgccgaggggtatcgcgtcgcggttgtcgatattcagagcgacaaagccgcaaatgtggcacaagaaattaacgccgaatatggtgaaagtatggcgtacggttttggtgctgacgccactagcgagcaaagcgttctggcgctctctcgtggggtagatgaaatctttggtcgcgtggatttgctggtctacagcgccggaatagcaaaagcagcctttatcagcgacttccagctcggcgattttgaccgttcgctacaggtgaatctggtgggttatttcctgtgtgcgcgtgaattttcgcgtttgatgatccgcgacgggattcaggggcgcattattcagatcaactcgaaatccggcaaagtgggcagcaaacacaactctggctacagcgcagcgaaatttggtggcgtcgggctgactcaatcactggcgctggatctggcggagtacggcattacggtgcattcactgatgctcggtaacctgctgaaatcgccgatgttccagtcactgttgccacaatacgcgaccaagctgggtatcaaaccggatcaagtcgagcagtattacatcgacaaagtaccgctcaaacgcggctgcgattatcaagatgtgctgaatatgctgctgttctacgccagtcctaaggcgtcgtactgcaccggacagtcgatcaatgtcaccggcggtcaggtgatgttctgatcaacagcggagatccattaaggatctccgtgagactatagaatgcctgatgcgctacgctcatcaggcatacaggacttccgccactacattaaggaaaagttatggtatccgcactcatcaccgtcgccgttatcgcctggtgtgcgcaactggccttaggcggctggcaaatttctcgttttaaccgtgccttcgacacactatgccagcaagggcgggttggcgtgggccgttccagcgggcgctttaaaccgcgggtcgtggtcgccatcgcgctggacgatcagcagcgcatcgtcgacaccttgtttatgaaaggactgaccgtcttcgcccgaccgcaaaaaattcccgcaattaccggtatgcatgcgggtgatttacagcccgatgtgatctttccccatgatccactatcacagaatgctctatcattggcgcttaaactgaaacgtggataatttcgttgtgaatgttacttgcttgcgaagttatcattttgaaacctaaatcaggtaatcacgcccatgaaacctcgtcagcgtcaggccgccattctggagtatctgcaaaagcagggtaaatgctcggttgaagaattggcgcaatactttgacaccacaggcacaaccattcgcaaagatctggtcattctggaacatgccggaaccgtcattcgtacttatggcggagtggtgttgaataaagaggaatccgatccgcctatcgatcataaaacactcatcaacacccacaagaaagagctgattgcagaagctgccgttagttttatccatgatggcgattcgatcattcttgatgctggcagtaccgttttgcagatggttcccctgctctcgcgctttaataacatcacggtgatgaccaacagcctgcatatcgtcaatgcgctatccgaactggataacgaacaaactatcctgatgccaggcggaacgtttcgcaaaaaatcggcctcatttcacgggcaactggcagagaatgccttcgagcatttcaccttcgataaattgtttatgggcaccgacggcatcgatctcaatgcgggcgtaaccacctttaacgaggtttataccgtcagtaaggcaatgtgcaatgccgcgcgcgaagtgattttgatggcggactcatcaaagtttggccgtaaaagccccaacgtagtttgcagtcttgaaagcgtcgataagctgattaccgacgcaggtatcgatccggcgtttcgtcaggcgctggaagagaaagggatcgatgtgatcataaccggagagagcaatgagtgaagcactactgaacgcgggacgtcagacgttaatgctggagttgcaggaagcaagccgtttaccggaacgtctgggcgatgattttgttcgcgccgccaatatcatcctgcactgtgaaggcaaagtggtggtttcgggaattggcaaatcgggccacattggtaagaaaatcgccgcaacgcttgccagtaccggcactccggctttttttgtccatccggcagaagcgctgcacggcgatctggggatgatcgaaagccgcgatgtgatgctgtttatctcttactccggtggcgcgaaggaactggatctgattattccgcgtctggaagataaatctatcgcgctgctggcgatgaccggcaaaccgacgtcaccgctgggcctggcggcaaaagcggtgctggatatctccgtagaacgcgaagcctgcccgatgcaccttgcgccgacctccagcaccgtcaataccctgatgatgggtgacgcgctggcgatggcggtcatgcaggcgcgcggatttaatgaagaagattttgcccgctcccacccagccggggcactgggcgctcgcttgctgaataaagtgcatcatctgatgcgccgtgacgatgccatcccacaggtggcgttaaccgccagcgtgatggatgcgatgctggaactcagccgcaccggtctggggctggtggcggtatgtgacgctcaacaacaggtacaaggcgtctttaccgacggcgatttacgtcgctggctggttggcggcggcgcactcaccacgccagtcaatgaagcgatgacggtcggcggcaccacgttgcaatcgcaaagtcgcgccatcgacgccaaagagatcctgatgaagcgcaaaatcactgccgcaccggtggtggatgaaaacggcaaactcaccggcgcaataaacctgcaggatttctatcaggccgggattatttaatccttcaatcccagacgtttcgccagccgatgcaggttggcgacgtcggtttccagcatccgcgcgcaggcagcccagttgtgatgattttgtgccagtgcctgacgaatagtttcacgctggaacgcttctgtcgcttcacgcaggttttgcttaacaacgggcaccgccgccacttctggcgtcggcaacgtcacctcaggaaaagcaaaatgttgcgcctcaagaatcacttcatcgccgctgcgggtggctctcgccagaactaccgcccgatgaatagcatgttccagttcgcgcacgtttcccggaaaactgtagtgttgcagtaaatttcgcgctccggcacttaataccacgcgggagagcccctgccgcaaacgacactgctcgcagaaataccccgccagcagaatgacatcatcgccccgctcacgcagcggcggcaccgaaagtggaaacacgctcaggcgatgaaacaaatcggcgcggaatcgccctgccagcacctcttcgcgtaaatcgcggttagtcgccgccagcacgcgcacatcgacccgcaaacaacggtcatcgccaacgcgctgaatatcgccatactgcaacaccctcagcagcttggcctgcaatgccaacgacaactcgccgatctcatccagaaacagcgtgccgttatccgccatttcaaacttcccgctgcgattactgatagcgccagtaaacgctcctttcacatgcccgaacaactcactttccgccacactttccggcagtgcagcacagttgagatagaccagcggattcaccgcccgtggcgaggcttcatgaatcgctttcgccaccagctccttaccggttccagtctcaccgctgatcaggacgttgagatcggacgccgccacaatctcaatctcttttttcagttgcgtcatgccaggggacaagccaatcatctgcgtctgtttcaccgcttcaaacggcgtggcatcgcctggcagcatattctggctttccagttgttcaatcagcaacgcattgcttaacgctcccgccgccagcgcagcaatcagccgtagctcttcgtcgctgaaaacatcgaactgatcgggctgcatcccgtcgagcgtcagtgcgccgatcaggttttgcccggcaaacaatggcagaccaacgcaggcgtgaaccttcagactctcctgcccaggaatcaaaccgtcatagggatcgggcaattcgctgtctgcgggaaagcgcaccacatccccggcgcgggcaatcgcttccagccgtggatgcccttccagcgcaaagcgtctaccgagtacatcctttgccagaccgtcgatggcaagcggaataaactgccgcgaatcgtaacgtagcaacgcagacgcatcgcactccagcacctgacgtagcgtggtgatcaggcgctgaaaacgatcctggtgaccaatcccacgctgcaattcgatggcgatattcgccagcacatcaacggaaaaactcatctttgcctcactgtcaatttgactatagatattgtcatatcgaccatttgattgatagtcattttgactactcattaatgggcataattttatttatagagtaaaaacaatcagataaaaaactggcacgcaatctgcaattagcaagacatctttttagaacacgctgaataaattgaggttgctatgtctattgtggtgaaaaataacattcattgggttggtcaacgtgactgggaagtgcgtgattttcacggcacggaatataaaacgctgcgcggcagcagctacaatagctacctcatccgcgaagaaaaaaacgtgctgatcgacaccgtcgaccataaattcagccgcgaatttgtgcagaacctgcgtaatgaaatcgatctggcggatatcgattacatcgtgattaaccatgcagaagaggaccacgctggggcgctgaccgaactgatggcacaaattcccgatacgccgatctactgtacagccaacgctatcgactcgataaatggtcatcaccatcatccggagtggaattttaatgtggtgaaaactggcgacacgctggatatcggcaacggcaaacagctcatttttgtcgaaacaccaatgctgcactggccggacagcatgatgacttacctgacaggcgacgcggtgctgttcagtaacgatgctttcggtcaacactactgcgacgagcatctgttcaacgatgaagtggatcagacggagcttttcgagcagtgccagcgttactacgccaatatcctgacgccgttcagccgcctggtaacaccgaaaattaccgagatcctgggctttaacttaccagtcgatatgatagccacttcccacggcgtggtatggcgcgataacccgacgcaaattgtcgagctgtacctgaaatgggcggctgattatcaggaagacagaatcaccattttctacgacaccatgtcgaataacacccgcatgatggctgacgctatcgcccaggggattgcggaaaccgacccacgcgtggcggtgaaaattttcaacgtcgcccgaagcgataaaaacgaaatcctgactaatgtcttccgctcaaaaggcgtgctggtcggcacttcgacgatgaataacgtgatgatgccgaaaatcgccgggctggtggaggagatgactggtttacgcttccgtaacaaacgcgccagtgctttcggctctcacggctggagcggcggtgcggtggatcgtctttccacgcgcctgcaggatgcgggtttcgaaatgtcgcttagcctgaaagcgaaatggcgaccagaccaggacgctctgaagttatgccgtgaacacggtcgcgaaatcgcccgtcagtgggcgctcgcgccgctgccgcagagcacggtgaatacggtagttaaagaagaaacctctgccaccacgacggctgacctcggcccacggatgcagtgcagcgtctgccagtggatttacgatccggcaaaaggcgagccaatgcaggacgttgcgccaggaacgccgtggagtgaagtcccggataacttcctctgcccggaatgctccctcggcaaagacgtctttgaagaactggcatcggaggcaaaatgagtaacggcattgtgatcatcggttcgggcttcgccgcccgccaactggtgaaaaatattcgcaaacaggacgccactattccattaaccctgattgccgccgacagcatggatgagtacaacaaacctgacctcagccatgttatcagtcaggggcaacgtgccgatgaccttacccgccagacggcgggtgaatttgccgagcagtttaatctgcacctgtttccacaaacctgggtgacggatatcgatgccgaagcccgtgtggtgaaaagccagaataatcagtggcaatacgacaagctagtactggcaaccggtgccagtgcctttgtcccgcctgtgcctgggcgtgagttaatgctgacgttaaatagtcagcaagagtatcgcgcctgtgaaacgcaactgcgggatgcccgacgcgtgttgattgttggcggtggtttgattggtagcgaactggcgatggatttttgtcgtgcaggcaaagcggtcacgctaatcgacaacgctgccagtattctggcgtcgttaatgccaccggaagtaagcagccgcttgcagcatcggttgacggagatgggcgttcatctgctgttgaaatctcagttacaggggctggaaaaaacggattctggcattcaggcaacgctggaccgccagcgcaatatcgaagtggatgcggtaattgccgccaccggactgcgcccggaaaccgccctggcacgacgcgccgggctgacgattaatcgcggcgtttgcgtcgatagttatctgcaaaccagtaataccgatatttacgcgctgggcgattgcgcggaaattaacggtcaggtattgccgttcctccagccgattcaacttagcgcgatggtgctggcaaaaaatcttctcggcaataacacgccgctgaaactcccggcgatgctggtgaaaatcaaaacgccggaattaccgctgcatctggcaggcgaaacccagcgtcaggatttacgctggcaaattaataccgaacgccagggaatggtggcgcgcggcgttgacgatgctgaccagcttcgcgcctttgtggtcagtgaggatcggatgaaagaggcatttggattgttgaaaacattgccgatgtaggtgggctactgtgcctaaaatgtcggatgcgacgctggcgcgtcttatccgacctacggggacgcatgtgtaggccggataaggcgtttacgccgcatccggcaatggtgtccaaatgcaacacgttttatccgttctggacttcacccgctaaccaacgcgccgcagcaataaccccctgccccagagacaaaccgccatcacccgccggtaaactctgtggaaagagcaatgtgaaatcagcgagataatgcgccagacgtgcacgcagcaaacggttatgaataaccccgccgctaaataccagcgtagtgataccacgcatcgtggcctgctcacgcatcaacgcggcaaaaccctgcgccagcgcatcatgaaacgcccacgcgcgttgattaaccggtgcctgccagttcagccactgctgccagaaagtggcgagatccagttgattgtccacccgcggcattgtcaccggatgcgtcactccgtggcatgaggctgcgagcgcctccagagcacaagccgcttcaccttcataacttaacgtggctggcgcacagcccagtgccgccgccactgcatcgaaaaaacgcccacacgatgacgccagcggcgcgttaattccacgctcaatggcccgcgccagcacgctccagttttgctgttgcacacttgctgtttcagagtaattctgccactccggcacaaagcgcaggcactgcgccagcaggtttcgccacggctgcttcgctgccaaatcgccacccggaagcgccactgcaggcaagccgcccaggtgctcacattcgcgatagttcacccgcaggcactcgccgccccacaaagcgccgttctcccccataccgataccgtcgagcgtcaaagcaatgacatcaccgccatccagcggccactgatgctctgccagacacgccgctgcatgggcatgatgatgcagtaccgtttgcgtcggcagattcatttcacgcgcccactggctggagacatagcccggatgcgcgtcatgcacaacgtattgcggggtaaaatcgtagatgttttgcatcaggcgtaacgcttcgcgccactgcatctggatgccatcgtcacttaaatcgcccagatgctgactcaacaccgcttgttcaccgcgcaccaggcagaaggtatttttcagatccgcgccgagacacagcacaggcggaacatttttaaagcccggaggcaaagccagcgcatccggcacatacccccgcgaacggcgcagcatttcgccgctttcgcgcaccaccgaatcatccatccgctgcacgatgtcgcggttatgtatcaagaatccgtcggcaatgccctgcaaatccgccagcgcctgttcgttgctgatagctggtggtttaccgctcaggttgccggaggtcatcaccagcgggcattgcagttcctgtaacagcaaatgctggagcgggttcgcaggcaacattaccccgacttcgttaaggtcaggggcgatatcatcacaaagctcaggaacgtattttttatccaccagcacaatcggcgcggcgggcgtggtaagcaactggcgcgcagcgtctggtaaaccgtcagccactggcaacatgaccgccagcggtttcgccgggcgatgtttgcgcgcccgaagtgtcgccaccgcgttactgttacgtgcatcgcaggcaagatgaaatccgccaatccctttgatggcgacaattttgcccatttttaactgtgcgatagctgcctgtaatgccgcctcttgttccgcatgttcaccatgacttacccattcaagatgcgggccacactccgggcaggccaccggctgggcgtggaagcgacgatcgagcgggtcacggtactctttgtcacaggccggacatagcggaaacgccgccatcacggtaaacgggcggtcgtaaggcatggcgcgaataatggtgaaacgcgggccgcagtgggtacagttgataaacggataacgataacgccgttcgcctggggtattcatttcggcaaggcaagcagggcaagtagcggcatcgggaacaatttgcgtattcatggtgccgcctgtgctctggcgtatagtgaactcggtgggcagttgtgaccagataaacggctcacgctcgacgctatcaatacgcgccagcggcgggcagtgctgatacaattgaacaagaaacgtttccgggtcttcccgcagccggacttctacgccatcgccgtcattacagacatcgccgtgaagatttaattgctgtgccagctgccagacaaacggacgaaaaccgacgccctgcactttgccacgaatacgcagttggacaccgcaagatgtgttttttgccattgagttattcccgccatcatgaattgcgtaacccgccctgccggacacgacagcgtcgcatccggcagtcacaggtcggcgataccgcccgctccgtattctacgaatatttccgggaattcctttgatgccagaacagttctgtaagatttttagaacatcagcgccgtacggcggcgtttttctgcgctcagttgttcaagtttattacgatcgacacaaatcagcgcatgagtcgggcaagccgccatacacgccgggccgtcttcacgatggttgcacaggtcgcatttattggcttcggctttgtcagcccgtacattcagacccgcgccgctgttgcggatcaccggacgtaccaccacttccatcgcaccatacgggcaagccacaacgcaggttttgcaaccaatgcaacgttcctgcatcacatgaacaaaccctttatcacggctgatagcaccattcgggcagacgttagcgcacggtgcatcttcacactgacggcaaactgtcgccgtggaaatgttcacacctttaatgacatggatacgcggtaaaaaagtttccggggtcagcgatgcacagtcctgattttcctgatgagaaaccacgcacgctacttcacaggtacggcaaccaatacatttactcgcgtcagcaatgatgaaacggttcatcaaattctccagcaatgacagttaatgcgccgatacattcacaaatcatgccagtttttaatttactgttatttaaggaaattaatttctgtaatgcaggaaaaacgatgtcatcgacactagtgacgatgacatgtgatgacaatgtttatcgcgaaggagcaatgagtgagtcgcggcggatcagttttccgctgaaggttttcggcggtgagaaatccccgccatcgagcataaaaatcagccgtccaataatttcctgaatcatctcagtcaccggaatttttacgctggagagcgccggaacggtgtagggggcaatagcgatatcatcgaatccgataactgacacctgctctggcaccgctacgccgcgctcgtgtaacgctttcatcgcacctatcgccatatcgtcgttactggcaactaacgcgctaaatttagccccacgttcgagcaacatttctaccccttcggccccgctggcaggcgtccatttaccgttagcgataagtttttcattgagcgcaataccatgctgcgccagcgcgtctttatacccggcaagacgttcaatgctggtgggggaatccatcgagccggtaaggaaagcaatctcctgatgcccggcgtttatcaactctgccacggcgttaaaactggtctgtttatgatcgcaccagacgctatggctgctgtttttgcgcaggcggcgattaagcaccattatcggctgactgtgcgcgtcaatgatgtcatcgatctcatccacgcttaaaaaacgcgggtaaatcatgatcgcgtcgcagcgcagatccagcagatactgaatcgcctggcgctcttcttctgcgctgtgtttaccatctgccaatagcaactgccgccctttctcttccgccattcgcgcggcatgaaagagtaattcactaaaataaatgccgtggtaaagcgtgttggtcactaccagccccagcgtctgagtactcttcgccgacagattgcgcgccagcaagtttggacggtaaccgctctcttctaccgcctgaaacacgcgatctttagtctcctggctgacgtagccattacctgaaagcacgcgggaaacggtcgcttttgaaaccccggcgcgcttcgccacttccagcatcgtcgtcatcattttcatccctttacacgcaatcaacgcagtgtactgcaccgtttgccgattgtccttgcacaatcggcgggaaaaatattcaggtgaccggtttcacaaatataaaaaatgaacaattcactctcttgcttatttagtgacaactattcatgattttgtgaaaccggtttcttaattccgtttcagcatcggcatttttccgtcacgtcgactgataacaactacatctaccctactgataacaggataaaatccgatggccaaaaattatgcggcgctggcacgctcggtgatagcggcactgggcggcgttgataacatctcggcggtcacgcactgtatgacgcggttgcgctttgttatcaaagatgatgcacttatcgacagcccgacgttaaaaaccatccccggcgtgctcggcgtggtacgtagtgacaaccagtgtcaggtgattatcggcaataccgtttcacaagcctttcaggaagtcgtcagcctgctgccgggagatatgcagcccgcacagcccgtgggtaaacccaaactcacgctacgtcgcattggtgcggggatcctcgatgcgctgatcggcaccatgtcaccgctgatcccggcgattatcggcggatcgatggtcaaactgctggcaatgatcctcgagatgagcggcgtgctgacaaaaggatcgccgaccttaaccattctgaatgtgattggtgacggtgctttcttcttcctgccgctgatggtcgcggcatctgccgccatcaaatttaaaaccaatatgtcgctggcgattgccatcgcgggtgtgctggtacatccgagttttattgaactgatggcgaaagcggcccagggtgaacatgtcgaatttgccctgattccggtcaccgcggtgaaatacacctacacggtgatcccggcgctggtgatgacctggtgcctgtcatatatcgaacgctgggtggacagcattacaccggcggtgaccaaaaacttcctcaaaccaatgctgattgtgttgattgccgcaccgctggcaatcctgctgattggcccgattggtatctggatcggtagcgccatttcggcgctggtttacaccattcatggttatctgggctggctttcagtcgccattatgggcgcgctgtggcctctgctggtaatgaccgggatgcaccgcgtctttacgccaaccatcattcagaccattgccgaaaccggcaaagaagggatggtcatgccgtcagagatcggcgctaacctgtcgctgggcggttcatcactggcagtggcgtggaaaacgaaaaacccggaactgcgtcagacggcgctggctgcggcggcatcagccattatggcggggatttccgaaccggcgttatatggcgtggcgatccgcctgaaacgtccgcttatcgccagtcttatcagcggttttatttgcggcgcggttgccggtatggcggggcttgccagccactcaatggcagcgccggggctatttaccagcgtgcagttcttcgatccggcgaatccaatgagcatcgtctgggtgttcgcggtcatggcgctggcggtggtgctgtcgtttatcctcacactgttgctcggctttgaggatattcctgttgaggaagcggctgcccaggcgcgaaagtatcagagcgtacaaccgaccgtcgccaaagaagtaagtcttaattgaggatgaaaatgtcagtatttccagaaagttttttatggggcggcgcgcttgccgccaaccagtctgaaggtgcgttccgtgaaggtgacaaaggtctgaccactgtcgatatgatcccacacggcgagcatcgaatggcggtgaaactggggctggaaaaacgttttcagttgcgagatgacgagttttatcccagccatgaggcgacggatttttatcatcgttataaagaagatatcgccctgatggcagagatgggattcaaggttttccgtacctcaattgcctggagccgtctctttccgcagggcgatgaaatcacgcccaatcagcagggcattgctttttatcgttctgtctttgaagagtgtaaaaagtacggtatcgaaccgctggtcacgttgtgccacttcgatgtgccgatgcatctggtcaccgaatatggctcctggcgtaaccgcaagctggtggagtttttcagccgctacgccagaacctgctttgaagcatttgatggtctggtgaaatactggctaaccttcaatgaaatcaacattatgttgcatagcccgttctccggcgcgggtctggtgtttgaagaaggtgaaaatcaggatcaggtgaaatatcaggccgcgcatcaccagctggttgccagtgcgctagccaccaaaatcgcccatgaggttaacccgcaaaatcaggtgggctgtatgctggcgggcggtaacttctacccttacagttgcaagccggaagatgtctgggcggcgctggagaaagaccgggaaaacctgttttttatcgatgtgcaggcgcggggcacgtatccggcttactctgcccgcgtattccgcgaaaaaggggtaaccatcaacaaagcaccgggcgatgatgaaatcctgaaaaacaccgtcgattttgtctctttcagctattacgcctcgcgctgcgcctcggcggagatgaacgccaacaacagcagtgcggcgaacgtggtgaaatcgctgcgtaatccgtatctacaggtgagcgactggggctggggaattgatccactcggtctgcgtatcaccatgaatatgatgtacgatcgttatcagaagccgctgtttctggtggaaaacggcctgggcgcaaaagatgaatttgctgccaatggcgagattaacgacgactatcgcatcagctacttacgcgaacatatccgcgcaatgggcgaagcgattgcagacggcattccgctgatgggctacaccacatggggctgtattgatttagtttccgcctctacgggtgaaatgagcaaacgctacggctttgtctttgttgaccgtgacgacgcaggcaacggtacgctgacgcgcacgcgtaagaaatcattctggtggtataaaaaagtgattgccagtaatggggaagatttagagtaggtaacagtgccggatgcggcgtgaacgccttatccggcctacatgtcgcacgaaccatgaaggcccgataagcgcagcgcatcgggcaatttagcatttggcatcagagctggttcaccccatcaagaacatccctgtcctgattccttaatgaaaaactactcttcttccaccgctaactgcgcgaagccgccatttccttcccagccttccagtcgttgataaacggtttctaccgcatctttaatcggctgggtcatcgggtagtaaaagccgacgatatccggctgaatgccgaggaaaatcacttcgccaatatcttctttcaactggtcgataaggtaattcaacggcatgttatgggtagtcatcataaacatctcggcgatatcatccgggtcgatgatgcggatctcgccggggtttagccccatatccgtggcgtcgacaatcagcagtcgtgtcgggcgcagttcacggatagcgacgatgtcgttttccggtgcgctaccgccgtcaatcaccacccagttacctttcggcgcggcggcgcacttttccgccagcagcggacctgcgccatcatcgcccatcatgctattgccaacacagagtaaaacgtcagtcacgcagtctcctcaccatcaaatagatggcgttttcctgatgaatatcatgcagcatacttaacagcattgtactccattcctgctgctgcgaagtttgcgctgcccgggctttatcgaatgcgttggccagcatcggcacatggttaatgtcgatgacgatctcaccatatttcggcacgccttccattttgcggcgggcttcactgcctgcctccagagtggcaatccatgccagatattcatcccacgggcaggtgagcgccgcttccaggcaatcgataaccccaaggtggtgaccaatcgccaggctgtaatagaccacctgctgcgcctcggcgggcgtggcatcgttctcatcaataaatttacggctcagttgactgaacaccaccttttcactcatcggatacgcgcctcttcaacaacatgattcagatggctgacaatctcgttcagacgcggatcgttttccgcttccagccagcgtgcaacctgttcttcgccctgccctaactgtgtaaggtaatcatcggcaatctgacgaccgtaacgataacccgccaggcgacgtgcttcgcgatccactttcacgcgcagcggctgcaccatatcaccatgcaggatctccgccggttgttcatccagttcacccggcccacgggcgtgaattttctgctccagcaggccgagcgccattgcaaagccgtacagcgtggcggcaggcgttggcgggcagccagggatataaacatccacagggacaattttatccgtaccgccccacacgcagtagagatcgtggaagatcccgccactgttaccgcaggcaccgtaggagatacaaattttcgggtccggcgcggactgccacgcacgcagcgcaggggatcgcattgcacgggtgaccgcgccggtaaacagtaaaatatccgcatgacgcggtgaaggaacgactttaatgccgaagcgttctgcatcaaacagcggcgaaagcgtggcgaaaatttcgatttcgcaaccgttgcagccgccgcagtccacgcggtaaacataggcagaacgtttgatttttttcagtaacgacgccttcatgctggcgatggattcatccaccgtcatggggaccggaatgccgttggcgtcacgggggcctaataaattgctcatcagatggcctctttcatatggcgagtcagttcaatacggtcggacggcaccaggcatttctggcgcttacattccgggcaagtctcaaagctttcgcggtggttttccgcgcggctgtcgccgttgtgcttaagcagcgcaatggcgtagtcgatctctttctggacggcgaaaggacgattgcagacgcggcagttgcacagcgcgaagcgggactgttgcaggaagtcttctttcttccacaccgccagttcgtactcttgcgacagtttgatcgccgccgtcgggcagacttcttcgcagcgtccacagaagatgcagtgcccaagattaaactcccaggcaagctctcctgtggcgaggtcagtttcaaccgttaaggcgtttgacgggcaggcattgacgcaggccgcgcagccgatgcactgctgcgggttctgctctggcttaccacggaagtttttatcaaccgcaatcggctccagcggataagacgaggtcgccgtgccggttttgatgacttttttgataaaggtaaacatggcgattccttatttcagcggcgagtttttacgctcaatgctgtaacgctcgagttctttgtacggcaccactttgctcttcttcttacgcacatcgaccacggtcatgcggtcggtacaggagtagcaagggtcgaggctaccgataatcagcggcgcatcggaaacggtgttgccgcgcagcatgtagcgcagggtcggccagttcgcgtaggtcgcggcacggcagcgccagcggtacagcttctggttgtcgccggtcatgctccagtggatatcatcgccgcgcggcgcttcggcaaagcccagcgcaaagcggtgcggaatgtaggtaaagccttccaccatcagtgggccacccggcaggttatccagaccgtagtcgatcatgttcagcgcggtatagacttcgttgatacgcactttcagacgggaaataacgtcgcagccctgctcgctgtggacttccattggcagcaggccatagccgacaaacgggtgatcggcgcgggtatcacgggcgtgaccgctggcacggaccatcgggccgacgttactgaagtcgcgagcgatttccgggtccagacgaccaatgccgacagtgcgctgttccatgttcggagtgctcagcagcacatccaccagctcctgcacttcacgacgcatctgttgtgccagctggcgggtctggatcatgtcgtctttcagcagatcgcgacgaatcccgccgatcaagttcaggccgtaggttttacgcgcaccggtaaggatctctgccattttcatggaggtttcacgcacgcggaagaactgcataaagccggagtcgaagccggtaaagtgacaggccaggccaaggttgagcagatgcgagtgcaagcgttctacctccagcagaatggcgcggatcatctgcgcacgttctggcacctgaatacccatcgcgttttccaccgacgtggtgtaggcggtgctgtgggcaaagccgcagatcccgcacacacggtcagagaggaaggtcacttcgttataacccatacgggtttccgccagtttttccatgccgcgatggacgtagaacagacggtagtcggcgtcgataatgttttcgccatcgacgaacagacggaagtggcccggttcatcagaagtgacgtgcagcggaccaatcggcacgacgttgtttttcttgtcgcccagttcgttgatgaactcgtaggtttcagcatcggtggtcggtgccggacgctgacgataatccatgctgtctttacgcagcggataaagttcatccggccagtcatccggcagcaccagacgacgttcatccggcagaccaaccggaatcaaaccgtacatatcgcgcacttcacgctcgccccacaccgccgccggaacgcgcggcgtcacggacggatattccggtttgttggcgtcaacttcgacgcgaaccgtaatccaacacttagtgcccttctccatcgacagcacgtagtaaacggcgtaatgaccattcagtttgcgttcgtcgttaccaaacagcaccgacagccagccaccctgtttgtagtaaagaaactccaccacttccggcaggtagttcacctttacggtgacagtcagctgatctttggtctgccaggcgtggtccagcacgacgcccggaaatgcctcattcagcgcggcgagataatgttgacctaatttttcttcagacatgctcaaactctctttaatcacgccgccagcaaggagacgaacgctaaaaatgcaaagccaaacccagcccaggtaatgcgcggagtaatatcaagacgcagacgggccatgctgttttcgaacagcgcgataaccaggacgccgaccaccagttttacgatggcaatcaccagcgccagcagcagtccaccggcggtgaaggtttccatttgtccccacggaataaacaccccgacgaacatctgcaacaccaccagctgtttcaggctgataccccatttcatgacgccaaagccgctgccgctgtattcagagagcgggccttcctgcagctcctgctcggcttccgccaggtcgaacggcagtttgcccatttcgataaaggtggcgaacgcacaggcacaaagcgccagtaccagcgggatgctctggctcagcggccagtgataaacggtgtcggtgatgttgctgatgttggtggaaccggcaacctgtgcggcaacccacagaccaagcagcagcatcggttcgaccagcacgccaagcatcgcttcacggctcgcgccgatagcggtaaacgggctaccggtatccagaccagaaatggcaaagaagaaacgcgcgatggcaaagagatacagtaaggtgatcaaatcacccagttgcggcagcggagaaccgacggtcaccaccggcagcgcagtagcgatagtcagcatgacgcccaccatcacatacggcgtcaggcggaacacccagccggaggcatccgggccgacgctctgacgccccagcagtttgataatgtcgcgatactcctgcaacacgcccggcccgcgacggttatgcaagcgggcgcgcgccacgcgggttataccggagagcagcggcgcaacggcaaataacaccagcgcctgaattaacggatataaaacactcattctcaggctcctcgtgaaacaataatcaccaccagtaccgccagttcaaccagcgccatccggcggaacagcaacgcactcccctcgcactgccagcccggcaccagagacaccggattcagccatttgcgtagtttcagcaccggcgcaaacgcctgtttcaccggcatggcaaaaccgtgagcggtaatcaccattgatttttcgtggtcgtaaccgcacacccaggccgcaccgcgggaacgcgatggcaaacgatcgcctttgcaaatcgccataatgatgaatggcagcagcgggcaggcaatcagcagcaacgtgatcatcggttgagaaacggtggtgttagcaggctccagcggcagaggtacagcagcagagagcatcggcagtagccacggcgcagcaacaccgccaattacgcagcaaatcgccagtgccactacgcttacgctcatcaggagcggcgcacaggtggcgttttcggcttctttggtgcgcggcgcgccgaggaacgtgacgccatagactttcgccatacacatcaccgccagcgcaccggtaattgccagccccacagcgagcagcggccccagcagacgggcaacaaacgcgccactattgctcagtttgaaaaatgattgatagataacccattccccggcaaaaccattcagcggcggcagcgcagccattgccatcagcccgactaacatggcgatggagataaccggcattttcttgccaataccaccgagtttttcgatatcgcgatgaccggtacggaaccagacgctccccgccccgaggaacagtacgcttttgaacaggctatggttaagcagatggtacagaccaccgaccaggccaagagcaatcagcgccggttgttcgagcgcgatacccgttacgccagcgcccagccccagcaggatgatgccgatattttccagggtgtggtaagccagcaggcgctggatgttgtgctccaccagcgcatacagaccaccgacaaacgcggtgatcatgccgagcaccagcagcgcgatcccccaccacagcggtgcattaccgcccagcagtgacagggttaaaatgcccagcaggccaattttcatgactaccgtagaaaacaacgcggcagctggcgcagaggcgttcgcatgtgcctgcggcacccagccgtgcagcggaataatcccggccagcaggccaaagccaatcactccgagcagccagatatcggaaccgagcggcagctgttgcatacgcatatccagcaggcgcagatccagcgtgccgtaacgctgccacagcagccagcaagcaatcgccagcagcagagtgccaagacgccccagcgcaaaccacagtttgccctctttgctgttgctggtgaggaacaccgcgcacagggccatgatttcggccattaccacgaacatgccgaggttgctggcaatgacggcgcagacggcggcagccatcaacatattgatctgcaagccgttgcacttcacctgcgcgtggcgatgccagtcaatgttgtagaggctgacaaacagaccgcacagaccgagcgtaatcagccaaatcgcgttaagcggagagatttgcacatcgtagcttaccagcgacagcgcaccgctcacgccaaccgcgccagtcagtacagtgaagcccgcggctgccgtatacagactaccaaccgcgccgccaattccagctatccagccacttaacgctttttgaaaagaaaagagaaatgccagaacagcggcggcgacaaaccacgccacgccgctattgatcagggaaattgcgctcatttagcctctccactttgagcctgctgaaacaaggtgagatcgccaaagtccgtgttaaaggtcagctcacgcttacgtttgctgacgcgggcgatatcggtgttatccaccagatgcagggctttagtcgggcacatccgcacgcaggccggaccttgttcatcaaagctacaaaggtcacatttgacggcgatcgcgcgaatacctggcacccagtcaagcaatgtgctgacacgcgccggagcaggcggtgccggtggcgctttcggggtattggcgtttgccggaatatccagcggacggctgccggaaaattcaattgcgccaaacgggcaggcgatgccgcacagcttgcagcttacgcacaggctttcattcaactgcacggccccatcgacgcgggtgatggcgttaaccgggcagaccaccgcgcagggtgcatcttcacagtggtgacagagctgcggcgcagattctttttcattcagcatcactctcaggcgcggcattgattgcaggccgtgctggcgatgcgtctctgaacaggcggcctcacaagtgtggcagccgatacagagcgtggagtcagcaattacaaaacgattcaccaggcattcctcaggtgattgtcatttttgacgaaaacatgccgatgaaatgtcattttcgacactcatcgacacgcccatccccaaacaggcgtaacgcctgcaaaacgggcaaagcctcagctcatgctgccgggctttgtccctttaccagttggcttaaattcaccggcacattgttttcaatagcggtgtataagctgtcgtaaacgccagcgattttttcgagatagtgttccagaacctgttcgcgatcgcggatgttgaccttgccatcaatcatgccgtcaatgctcagttgcgcctgcgcaatccgctgtttgtcttcgccatcttttgtttcgacgtaatactcgatggtgtggctgttaaagccatccgccagggtgacgtaaatgcgaaaatgttcaaaaaggacgaaacagagttctttgtccggcgcgcagctcatggcgtgatgcaggcgcgctttcgataacgtgatcccctgaaccagcgaattgcagtagatgtgccactggtcctgtaggcgacgatgccgctgtgcgatgtaatcggctttctcgcttatttcccaaatagtcattgtcaggttacccgtttaacagagatgccagctttaagcattttttgtgccaacttttaatttattgttattaaagagatttttaagctaaagatgaatttcgtcgccgtgtcgacgtgtcatttcgacatcatcgacattattcaccgcagggataatcaacactggcacaattattgcttgtagctggcaatagttaatgggaggcgatatgcacgaaataaccctctgccaacgggcactggaattgatcgaacagcaggccgcaaaacacggcgcaaaacgcgtaactggggtctggctcaaaattggcgcattttcttgtgtcgaaaccagctctcttgccttttgttttgatctggtttgccgcggcagcgtggcggaaggttgtaaactgcacctcgaagaacaagaggccgaatgctggtgtgaaacatgccaacagtatgtgacgctactgacccagcgcgtccgccgctgtccacagtgtcatggtgacatgctgcagattgtggcagacgacggtttacagattcggcggatagaaatagaccaggagtgagcgatgtgtacaacatgcggttgcggtgaaggcaacctgtatatcgagggtgatgaacataaccctcattccgcgtttcgtagcgcgccatttgccccggcggcacgcccgaagatgaaaatcaccggcattaaagcgcctgaatttacccccagccagactgaagaaggcgacctgcattacggtcatggcgaagcgggcactcacgcaccgggcatgagccagcgtcggatgctggaagtcgaaattgacgtgctggacaaaaataaccgtctggctgaacgcaaccgcgcgcgctttgctgcccgcaagcaactggtgctcaacctggtttccagccctggttccggtaaaaccaccctgctgacggaaaccctaatgcgcctgaaagacagcgttccgtgcgcagttattgaaggcgaccagcaaaccgtgaacgatgccgcacgcattcgcgctaccggcacaccagcgattcaggtgaacaccggtaaaggctgccatcttgacgcacagatgattgccgacgccgcaccgcgtctgccactggacgataacggtattctgtttatcgaaaacgttggcaacctcgtatgcccggccagcttcgatctcggtgaaaaacacaaagtggcggtgctttccgttaccgaaggtgaagacaaaccactgaaatatccgcatatgtttgccgccgcctcgctgatgctgctcaacaaagttgacctgttgccgtatctcaactttgacgttgaaaagtgcatcgcctgcgcccgcgaagtcaatccagaaattgaaatcatccttatttccgccaccagcggcgaagggatggaccagtggctgaactggctggagacacagcgatgtgcataggcgttcccggccagatccgcaccattgacggcaaccaggcgaaagtcgacgtctgcggcattcagcgcgatgtcgatttaacgttagtcggcagctgcgatgaaaacggtcagccgcgcgtgggccagtgggtactggtacacgttggctttgccatgagcgtaattaatgaagccgaagcacgcgacactctcgacgccttacaaaacatgtttgacgttgagccggatgtcggcgcgctgttgtatggcgaggaaaaataatgcgttttgttgatgaatatcgcgcgccggaacaggtgatgcagttaattgagcatctgcgcgaacgtgcttcacatctctcttacaccgccgaacgccctctgcggattatggaagtgtgtggcggtcatacccacgctatctttaaattcggcctcgaccagttactgccggaaaacgttgagtttatccacggtccggggtgcccggtgtgcgtactgccgatgggtagaatcgacacctgcgtggagattgccagccatccggaagtcatcttctgtacctttggcgacgccatgcgcgtgccggggaaacagggatcgctgttgcaggcaaaagcacgcggtgccgatgtgcgcatcgtttactcgccgatggatgcgttgaaactggcgcaggagaatccaacccgcaaagtggtgttcttcggcttaggttttgaaaccactatgccgaccaccgctatcactctgcaacaggcgaaagcgcgtgatgtgcagaatttttacttcttctgccagcacattacgcttatcccgacgttgcgcagtttgctggaacagccggataacggtatcgatgcgttcctcgcgccgggtcacgtcagtatggttatcggcaccgacgcctataattttatcgccagcgattttcatcgtccgctggtggttgctggattcgaaccccttgatctactacaaggcgtggtcatgctggtgcagcagaaaatagcggcccacagcaaggtagagaatcagtatcgtcgagtggtaccggatgccggtaacctgctggcgcaacaggcgattgccgatgtgttctgtgtcaacggcgacagcgaatggcgcggcttaggcgtgattgaatcttctggcgtgcacctgacgccggattatcaacgattcgatgccgaagcacatttccgcccggcaccgcagcaggtctgcgatgacccgcgcgcgcgttgtggtgaggtattaacgggcaaatgtaagccgcatcaatgcccgctgtttggtaacacctgtaatcctcaaaccgcgtttggtgcgctgatggtttcctccgaaggagcgtgcgccgcgtggtatcagtatcgtcagcaggagagtgaagcgtgaataatatccaactcgcccacggtagcggcggccaggcgatgcagcaattaatcaacagcctgtttatggaagcctttgccaacccgtggctggcagagcaggaagatcaggcacgtcttgatctggcgcagctggtagcggaaggcgaccgtctggcgttctccaccgacagttacgttattgacccgctgttcttccctggcggtaatatcggcaagctggcgatttgcggcacagccaatgacgttgcggtcagtggcgctattccgcgctatctctcctgtggctttatcctcgaagaaggattgccgatggagacactgaaagccgtagtgaccagcatggcagaaaccgcccgcgcggcaggcattgccatcgttactggcgatactaaagtggtgcagcgcggcgcggtagataaactgtttatcaacaccgctggcatgggcgcaattccggcgaatattcactggggcgcacagacgctaaccgcaggcgatgtattgctggtgagcggtacactcggcgaccacggggcgactatccttaacctgcgtgagcagctggggctggatggcgaactggtcagcgactgcgcggtgctgacgccgcttattcagacgctgcgtgacattcccggcgtgaaagcgctgcgtgatgccacccgtggtggtgtaaacgcggtggttcatgagttcgcggcagcctgcggttgtggtattgaactttcagaagcggcactgcctgttaaacctgccgtgcgtggcgtttgcgaattgctgggactggacgccctgaactttgccaacgaaggcaaactagtaatagctgttgaacgcaacgcggcagagcaagtgctggcagcgttacattcccatccactggggaaagacgcggcgctgattggtgaagtggtggaacgtaaaggtgttcgtcttgccggtctgtatggcgtgaaacgaaccctcgatttaccacacgccgaaccgcttccgcgtatatgctaataaaattctaaatctcctatagttagtcaatgaccttttgcaccgctttgcggtgctttcctggaagaacaaaatgtcatatacaccgatgagtgatctcggacaacaagggttgttcgacatcactcggacactattgcagcagcccgatctggcctcgctgtgtgaggctctttcgcaactggtaaagcgttctgcgctcgccgacaacgcggctattgtgttgtggcaagcgcagactcaacgtgcgtcttattacgcgtcgcgtgaaaaagacacccccattaaatatgaagacgaaactgttctggcacacggtccggtacgcagcattttgtcgcgccctgatacgctgcattgcagttacgaagaattttgtgaaacctggccgcagctggacgcaggtgggctatacccaaaatttggtcactattgcctgatgccactggcggcggaagggcatatttttggtggctgtgaatttattcgttatgacgatcgcccctggagcgaaaaagagttcaatcgtctgcaaacatttacgcagatcgtttctgtcgtcaccgaacaaatccagagccgcgtcgttaacaatgtcgactatgagttgttatgccgggaacgcgataacttccgcatcctggtcgccatcaccaacgcggtgctttcccgcctggatatggacgaactggtcagcgaagtcgccaaagaaatccattactatttcgacattgacgatatcagtatcgtcttacgcagccaccgtaaaaacaaactcaacatctactccactcactatcttgataaacagcatcccgcccacgaacagagcgaagtcgatgaagccggaaccctcaccgaacgcgtgttcaaaagtaaagagatgctgctgatcaatctccacgagcgggacgatttagccccctatgaacgcatgttgttcgacacctggggcaaccagattcaaaccttgtgcctgttaccgctgatgtctggcgacaccatgctgggcgtgctgaaactggcgcaatgcgaagagaaagtgtttaccactaccaatctgaatttactgcgccagattgccgaacgtgtggcaatcgctgtcgataacgccctcgcctatcaggaaatccatcgtctgaaagaacggctggttgatgaaaacctcgccctgaccgagcagctcaacaatgttgatagtgaatttggcgagattattggccgcagcgaagccatgtacagcgtgcttaaacaagttgaaatggtggcgcaaagtgacagtaccgtgctgatcctcggtgaaactggcacgggtaaagagctgattgcccgtgcgatccataatctcagtgggcgtaataatcgccgcatggtcaaaatgaactgcgcggcgatgcctgccggattgctggaaagcgatctgtttggtcatgagcgtggggcttttaccggtgccagcgcccagcgtatcggtcgttttgaactggcggataaaagctccctgttcctcgacgaagtgggcgatatgccactggagttacagccgaagttgctgcgtgtattgcaggaacaggagtttgaacgtctcggcagcaacaaaatcattcagacggacgtgcgtctaatcgccgcgactaaccgcgatctgaaaaaaatggtcgccgaccgtgagttccgtagcgatctctattaccgcctgaacgtattcccgattcacctgccgccactacgcgagcgtccggaagatattccgctgctggcgaaagcctttaccttcaaaattgcccgtcgtctggggcgcaatatcgacagcattcctgccgagacgctgcgcaccttgagcaacatggagtggccgggtaacgtacgcgaactggaaaacgtcattgagcgcgcggtattgctaacacgcggtaacgtgctgcagctgtcattgccagatattgttttaccggaacctgaaacgccgcctgccgcaacggttgtcgccctggagggcgaagatgaatatcagttgattgtgcgcgtgctgaaagaaaccaacggcgtggttgccgggcctaaaggcgctgcgcaacgtctggggctgaaacgcacgaccctgctgtcacggatgaagcggctgggaattgataaatcggcattgatttaactgcaaattgccggacagatctgcctgtccggcatactattcatgaggttttttcggacgatatttttccggcagttctggcaccggacgcttgtcatcgatgagatgacgcacggttaagatcggatgacgccacagcattctcggcccggcccaacgcataatctgtttcatctcttcacgctttgcaggctggtaacagtgcaccggacactgcttacaggctggtttctcttcgccgaacacacatttatccagccgcttttgcgcgtaaacaaacaacgcctcgtaatgctccggctccgctgacgcctgcgggcatttcgcttgataaagatcgatcatttttttaatcgtcagtttttcacgagagatacgcttgccggacatgctgcctccacctcattaagatgtatttatattacatcttaatcttaaagggcactatgactccaaagaagaagggttagccaaccgatacaattttgcgtacttgcttcataagcatcacgcaaaagctgcaaaacagcatctttcccggaaccagcatcaagaactcgccgttcgcttcttcccctgaaatgattaactccggtatcatgtgcgccttatgtgattacaacgaaaataaaaaccatcacaccccatttaatatcagggaaccggacataaccccatgagtgcaatagaaaatttcgacgcccatacgcccatgatgcagcagtatctcaggctgaaagcccagcatcccgagatcctgctgttttaccggatgggtgatttttatgaactgttttatgacgacgcaaaacgcgcgtcgcaactgctggatatttcactgaccaaacgcggtgcttcggcgggagagccgatcccgatggcggggattccctaccatgcggtggaaaactatctcgccaaactggtgaatcagggagagtccgttgccatctgcgaacaaattggcgatccggcgaccagcaaaggtccggttgagcgcaaagttgtgcgtatcgttacgccaggcaccatcagcgatgaagccctgttgcaggagcgtcaggacaacctgctggcggctatctggcaggacagcaaaggtttcggctacgcgacgctggatatcagttccgggcgttttcgcctgagcgaaccggctgaccgcgaaacgatggcggcagaactgcaacgcactaatcctgcggaactgctgtatgcagaagattttgctgaaatgtcgttaattgaaggccgtcgcggcctgcgccgtcgcccgctgtgggagtttgaaatcgacaccgcgcgccagcagttgaatctgcaatttgggacccgcgatctggtcggttttggcgtcgagaacgcgccgcgcggactttgtgctgccggttgtctgttgcagtatgcgaaagatacccaacgtacgactctgccgcatattcgttccatcaccatggaacgtgagcaggacagcatcattatggatgccgcgacgcgtcgtaatctggaaatcacccagaacctggcgggtggtgcggaaaatacgctggcttctgtgctcgactgcaccgtcacgccgatgggcagccgtatgctgaaacgctggctgcatatgccagtgcgcgatacccgcgtgttgcttgagcgccagcaaactattggcgcattgcaggatttcaccgccgggctacagccggtactgcgtcaggtcggcgacctggaacgtattctggcacgtctggctttacgaactgctcgcccacgcgatctggcccgtatgcgccacgctttccagcaactgccggagctgcgtgcgcagttagaaactgtcgatagtgcaccggtacaggcgctacgtgagaagatgggcgagtttgccgagctgcgcgatctgctggagcgagcaatcatcgacacaccgccggtgctggtacgcgacggtggtgttatcgcatcgggctataacgaagagctggatgagtggcgcgcgctggctgacggcgcgaccgattatctggagcgtctggaagtccgcgagcgtgaacgtaccggcctggacacgctgaaagttggctttaatgcggtgcacggctactacattcaaatcagccgtgggcaaagccatctggcacccatcaactacatgcgtcgccagacgctgaaaaacgccgagcgctacatcattccagagctaaaagagtacgaagataaagttctcacctcaaaaggcaaagcactggcactggaaaaacagctttatgaagagctgttcgacctgctgttgccgcatctggaagcgttgcaacagagcgcgagcgcgctggcggaactcgacgtgctggttaacctggcggaacgggcctataccctgaactacacctgcccgaccttcattgataaaccgggcattcgcattaccgaaggtcgccatccggtagttgaacaagtactgaatgagccatttatcgccaacccgctgaatctgtcgccgcagcgccgcatgttgatcatcaccggtccgaacatgggcggtaaaagtacctatatgcgccagaccgcactgattgcgctgatggcctacatcggcagctatgtaccggcacaaaaagtcgagattggacctatcgatcgcatctttacccgcgtaggcgcggcagatgacctggcgtccgggcgctcaacctttatggtggagatgactgaaaccgccaatattttacataacgccaccgaatacagtctggtgttaatggatgagatcgggcgtggaacgtccacctacgatggtctgtcgctggcgtgggcgtgcgcggaaaatctggcgaataagattaaggcattgacgttatttgctacccactatttcgagctgacccagttaccggagaaaatggaaggcgtcgctaacgtgcatctcgatgcactggagcacggcgacaccattgcctttatgcacagcgtgcaggatggcgcggcgagcaaaagctacggcctggcggttgcagctctggcaggcgtgccaaaagaggttattaagcgcgcacggcaaaagctgcgtgagctggaaagcatttcgccgaacgccgccgctacgcaagtggatggtacgcaaatgtctttgctgtcagtaccagaagaaacttcgcctgcggtcgaagctctggaaaatcttgatccggattcactcaccccgcgtcaggcgctggagtggatttatcgcttgaagagcctggtgtaataacaattcccgatagtcttttgctatcgggaatattaacgacaactgacgaataaaataaaaacaccctgtataataggaaagcttattttacagggtaaaaccatgccatctacacgctatcaaaaaatcaatgcccatcactatcgccatatatgggtcgttggtgatattcatggtgaatatcagttattacaatcccgcttacatcaactctcttttttccccaaaatcgacttacttatttctgtcggcgataatattgatcgtggaccggagagtcttgacgtcctgcgcctgctaaaccaaccctggtttacgtcggttaaaggcaaccacgaagcgatggcgcttgaggcattcgaaactggcgatggcaatatgtggcttgccagcggtggtgactggtttttcgatttaaatgattcagagcaacaagaggcaatagatctgttgctgaaattccatcaccttccacatattattgaaatcactaacgacaacataaaatatgccatcgcacatgcagattatccggggagtgaatatctctttggtaaagaaatagcggagagcgaattactctggcctgttgatcgtgtgcagaaatcgcttaatggcgagttacaacaaataaacggcgctgattattttatatttggacatatgatgtttgataacattcagacgttcgctaaccagatttatattgataccggatcgccgaacagcgggcggctgtcattttataaaataaagtagtctcatgcttcttctgtgaagcatgagtaacccggtgttattgcaggccattattcatttttcgctaccagcaaagagagatcctgcttcaccagcgcgcgactggcactctccggcaaaccgtcgtctgtaataatctgatcaaactcgcttaatggtaacgccagccatgtcgccacctgaccatatttcgtcgcatcacagaccaaaactcgctggcggctggcactggcaatcgcccgtttcaccgtgactttatcttccgctggcgtagaaatcccccgcacactccatgacgatgcagaaataaaagcctgatcaatcatcaggctgcgcagcatggtcgcagcggcttccccgacacaggaacggttttcccgacacactgcaccgccagtgtgaataattgtgcaattactgttgtcgagcaagtagtccgcaataacgaaatcgtttgtgaccacagtcagtgactccatgtgaatcagatgctgtgctatcgctaacgtggtcgttcccgcatccagatagatacaacttcccggctgaacaagacttgccgccagcttgccaatagccgctttttgcgtcattgccagcgcagtttttacctgatgagaaggttcatgcgccacgcgtcccggagactggacgcctccggacaccagcacaacggctccctgctgctccagtttttgtaaatcccgacgaatggtcatatgtgacacattcattctgtccgttagttcagcaatactgacaatgcctttttcagctaccatctcaaggatgatttggcgacgctctacgggtatcaacttttgctccttcctttgtcctgctgacattctacgctatttgcctgcgaaacgtgcgcggcgcaactaacgcttagttcacataaaataacacacaatgttaatttatgtgaatcagatcaccataccgttatcttccagcgcttatattcacaatatcaaacaaaatatcacttaaattaacaaggagagcagatgaaaacgggatctgagtttcatgtcggtatcgttggcttagggtcaatgggaatgggagcagcactgtcatatgtccgcgcaggtctttctacctggggcgcagacctgaacagcaatgcctgcgctacgttgaaagaggcaggtgcttgcggggtttctgataacgccgcgacgtttgccgaaaaactggacgcactgctggtgctggtggtcaatgcggcccaggttaaacaggtgctgtttggtgaaacaggcgttgcacaacatctgaaacccggtacggcagtaatggtttcttccactatcgctagtgctgatgcgcaagaaattgctaccgctctggctggattcgatctggaaatgctggatgcgccagtttctggtggtgcagtaaaagccgctaacggtgaaatgactgtcatggcctccggtagcgatattgcctttgaacgactggcacccgtgctggaagccgttgccggaaaagtttatcgcataggtgcagaaccgggactaggttcgaccgtaaaaattattcaccagttgttagcgggcgtacatattgctgccggagccgaagcgatggcacttgcagcccgtgcggggatcccgctggatgtgatgtatgacgtcgtgaccaatgccgccggaaattcctggatgttcgaaaaccggatgcgtcatgtggtggatggcgattacaccccgcattcagccgtcgatatttttgttaaggatcttggtctggttgccgatacagccaaagccctgcacttcccgctgccattggcctcaacagcattgaatatgttcaccagcgccagtaacgcgggttacgggaaagaagacgatagcgcagttatcaagattttctctggcatcactctaccgggagcgaaatcatgatcaagattggcgttatcgccgatgattttaccggcgcgacggatatcgccagttttctggtggaaaacggtctaccaacggtacaaattaacggtgttccaacaggtaaaatgccggaagcaatcgacgcactggtgatcagcctgaaaacgcgctcctgtccagtggttgaagccacacagcaatcgctggcggctctgagctggttgcaacagcaaggttgcaaacagatctatttcaaatactgctctactttcgacagtacggcgaaaggtaatattggcccggttaccgatgccttaatggatgctctcgacacgccgtttacggtcttctctccggccctgccggtcaacggacgtacggtttatcaggggtatttgttcgtaatgaatcaactgctggccgaatccgggatgcgccatcacccggtaaatcccatgaccgacagctatcttccccgtctggttgaagcgcaatccacagggcgctgcggcgtcgtttcggcacatgttttcgaacaaggtgtggatgccgttcgtcaagagctggctcgcttacagcaagagggctaccgctacgcggtgcttgatgcgctgaccgaacaccatctggaaattcagggagaagccttgcgcgatgccccactggtaacgggcggttctggtctggcgattggcctggcccggcagtgggcgcaagaaaacggtaaccaggctcgcaaagcagggcgtccgctcgctgggcgcggcgtagtgctctccggttcatgctctcaaatgaccaaccgccaggtagcacattaccgtcaaattgcaccagcccgtgaagttgatgtggcacgctgcctctcaattgaaactctggccgcttatgcacacgaactggcagagtgggttctgggccaggaaagtgtacttgctccactggtttttgccaccgccagcactgacgcattggcagcaattcaacagcaatacggtgcacaaaaagccagtcaggcagtagaaacactgttttctcaactagcggcgcggttagcagcggaaggcgtgacacgctttattgtcgcaggcggtgagacctccggcgtagtcacacagagcctgggaataaaagggtttcatattggcccaaccatttccccggcgtgccgtgggtaaacgcactggataagcctgtctcactcgcccttaaatctggcaacttcggtgatgacgcctttttttcacgagcccaaagagagtttttatcatgagcgatttcgcaaaagtagagcagtctttgcgagaggagatgacgcggattgccagttcattctttcagcgcggctatgcaaccggttcggctggcaatctgtcgctgcttttacctgacgggaatttactggcgacaccgacaggttcatgcctgggcaatctcgatccgcagcggctttccaaagtcgccgcggatggcgaatggttaagtggtgacaaaccctcgaaagaggtgctctttcatctggcgctgtatcgcaacaatccgcgctgtaaagcggtggtgcatttgcacagcacatggtcgacggcgctttcctgcctgcaagggctggacagcagcaacgttattcgtccgttcacaccatacgtggtgatgcggatgggaaatgtcccgctggtgccttattaccgaccgggcgataaacgcatcgcacaggatctggcggaactggcagcagacaatcaggcttttttactggcaaatcatggcccagtggtttgcggtgaaagcctgcaagaagccgccaacaatatggaagagctggaggaaacggcaaagctgatttttattctcggtgaccgcccgatccgttatctgaccgcaggtgaaattgcggaattaaggagttaatgcaatgcctcgttttgcagctaatttatccatgatgttcaccgaagtgccttttattgaacgcttcgccgcagcgcgaaaagccgggttcgatgctgtggaatttctgtttccctataactactccaccctgcaaatccaaaagcaactggagcaaaaccatctgacactggcgctgttcaataccgctcccggagatattaatgcgggggaatggggattatccgcccttcccggacgtgagcacgaagcacacgcagacatcgacctggcactggaatatgcattggcgctcaattgtgaacaagtccatgtgatggcaggcgtcgtgcccgctggcgaagatgctgaacggtaccgggcagtatttatcgataatatccgctacgctgccgaccgctttgcgccacacggcaagcgaatattagttgaagcactcagccccggcgttaagcctcattatctcttctccagccagtatcaggcactggctattgttgaagaggttgcgcgagataacgtgtttattcaactagatacttttcatgcgcaaaaagtagatggcaacctgacgcatttaatccgcgactacgccgggaaatatgcgcacgtacaaattgccggactacctgatcgacatgaaccggacgatggagaaatcaactatccgtggctgttccgcctgttcgatgaggtgggatatcagggctggatcggttgtgaatataaacctcgtggcctcaccgaagaagggcttggctggtttgacgcctggcgctaattcgttaaatccctaattacaacgtacccatacatccccccatctacggatggggtaggttaactataactttcagacagggtttcccatgtccacaattacattgttatgcattgcgttagctggcgtaatcatgctgttgctgctggtcatcaaggcaaaggtacaaccattcgttgctttgctcctcgtcagcctgttagtcgcacttgcggcaggtataccggcgggcgaagtgggtaaagtgatgatcgccgggatgggcggtgtgcttggttccgtcactattattattggtctgggcgctatgctggggcgtatgatcgaacactctggtggtgcagagtcactggctaattatttcagtcgcaagttaggtgacaaacgaactatcgctgcgctgactctggcagcgttcttcctcggtattcccgtcttctttgatgtcggctttattattcttgcgccaatcatttacggttttgccaaggttgccaaaatatcgccactcaaatttggcctgcctgtcgctgggatcatgctcactgttcacgtggcggtaccgccgcatccaggccctgtcgccgcagcggggttactccacgcagacatcggctggctaaccatcatcggtattgcgatttctattcccgtaggggttgttggctactttgcagcgaaaataatcaataagcgccaatatgcgatgtcagtagaagtactggaacagatgcaactggctccggccagtgaggaaggcgcgacaaaattaagcgataaaataaatccaccgggcgtcgcgctggtcacctcgctaattgttattcctatcgcgattatcatggcgggtacggtttccgcaacactgatgccgccttcgcatcccctgcttggtacgctacagctgatcggctcaccaatggtagctctaatgattgcgctggtgctggcattctggttattggctttacgtcgcggctggagcttacaacacaccagcgacattatgggctcagcgcttcctactgcggcggtagtgattttggttactggtgctggaggggtatttggcaaagtgctggtggaatcgggcgtcggcaaagcccttgccaacatgctacaaatgattgacctgcctctgttaccagccgcatttattatttcactggcgctgcgtgcatcgcaggggtcagcaaccgtagcaatactgacaaccggcgggttactctcagaagcggtgatgggattgaatccgattcagtgcgtattggtgacgctggcagcctgctttggtgggcttggtgcgtcacatattaatgactcagggttctggattgtgaccaaatatctggggttgtcggtagcagacggtctgaaaacctggacagtgttaacgaccattctcggttttaccggattcttaattacctggtgcgtatgggcggtaatttgaccttaataaaaaggtccgatgggcatcggaccttttattgtgcacagaaaaggccagcctcgcttgagactggcctttctgacagatgcttacttactcgcggaacagcgcttcgatattcagcccctgcgtttgcaggatttcgcgcaaacggcgcaggccttcaacctgaatctggcgaacacgttcacgggtgaggccaatttcacgacctacatcttccagtgttgccgcttcgtaccccagcaaaccgaatcgacgtgccagcacttcacgctgtttggcgttcagctcgaacagccatttgacgatgctctgcttcatatcgtcatcttgcgtggtatcttccggaccgttctctttttcatcggccaggatgtccagcaacgctttttcggaatcaccacccagcggggtgtctaccgaggtaatgcgctcgttaagacgaagcatacggctgacgtcatcaactggcttatccagttgctctgcgatctcttccgcacttggttcatggtccagcttatgggacaactcacgtgcggttcgcaggtaaacgttcagctcctttacgatgtgaatcggcaaacgaatagtacgggtttggttcataatcgcccgttcaatcgtctggcgaatccaccaggttgcgtatgttgagaagcggaaaccacgttccgggtcaaacttctctaccgcgcggatcagccccaggttgccctcttcgataaggtccagcaacgccagaccacgattgccataacggcgggcaatttttaccaccagacgcaagttactctcgatcatccggcggcgagaggcgacatctccacgcagtgcgcgacgcgcaaaataaacttcttcttcggccgttaacagtggtgaataaccaatctcaccaaggtaaagctgagtcgcgtccaacacacgctgtgtggctccctgcgataacagttcctcttcggccaaatcgttatcactgggttcctgttctactaaggccttttcgtcaaaaacctcaactccgttctcatcaaattccgcatcttcatttaaatcatgaactttcagcgtattctgactcataaggtggctcctacccgtgatcccttgacggaacattcaagcaaaagcctggttccgccgatttatcgctgcggcaaataacgcagcgggtttacggatttccccttgtaacgaatttcaaaatgcaagcgtgttgaactggttccggtgctacccatggtcgctattttttgccccgccttaacttcttgttgttcccggaccagcattgtgtcgttatgggcgtaggcactcaggtaatcatcattatgtttgatgataatcagattaccgtagccgcgcagcgcgttaccagcataaacaacgcggccatctgcggtcgcgataattgcctgtcctttgctgcctgcgatatcaatccccttgttgcccccctcagaagcgccaaaggtttcgatcactttgccctcagtcggccagcgccaggtggagataggcgtactggttgatgtactgctgacagtcggctcggttgtgcttgctgttggtaccgttacaggcgctgtgaccgtggtcgcagttggcttgttgttcggcaacattttgttagcactctgttcacccgaagactcagaatacgtaattgtcggttgcgacgcaacagcaacggtggaattttgtgcaggcttgatcacaactccttgctctgctgcgtcggcctgggtaatggcatttccgccagtgattggcgtaccggaagcattacccacctgcaaggtctgaccaacgttcagcgcgtatggtgcctgaatattgttgcgctgagcaaggtcacggaaatcgttgccagtaatccaggcgatatagaaaagtgtgtcgccttttttcacggtataggtactgccgctataactgcctttcggaatgttcccatactgacggttatagacgatgcgtccgttttccatctgtaccggctgctgagctactggctgcactggctggatttgcggttgttgagtagcctgaatttgtggctgctgcaccggctgaatttgcggttgctgcgctgtagacgtcgtccccattttcggcggcggcgtaatcaacataccagaattagtatttgcaggcgcattgccattaacggagctgaccggtgccggtggatttgaagtgtcagaacagcctgccagccatagcgaaaccagtgacaaagccgcaatgcggcgaacggtgaattttgggcttcccgcgctcatttatcccccaggaaaaattggttaataaccagtgacataattaccgtgcaaggcaccctactgaacactggaaaagatgttcacgatacgctgacctgcggcaaaataaccaggaaaaatccaggtatttcctcacgttttaagccagctcacccttcactaaagggacaaagcgcacggcctccacggtatcgataataaattcgcctccccgacgacgcacccgtttcaaatactggtgctcctcccctacgggtaagacgagaatcccgccttcgtccagctgcgtcattagcgcagttggaatttccggcggtgccgccgtaacaatgatagcgtcaaacggcgcacgtgcctgccaaccttgccatccatcgccatgacgggttgaaacattatgtaaatcaagatttttcaggcggcgacgtgcctgccactgcaagcctttaatccgttcaaccgagcaaacatgctggacaagatgcgccaggattgccgtttgatatcccgaaccggtgccaatttccagcacccgcgactgcggcgtcagctcgagtaattcggtcattcgcgccaccatatatggctgcgaaattgtctgcccctgacctatcggcaaagcgatattgtcccaggctttttgttcaaacgcttcatcaacgaatttttcacgcggcacggcggcaagtgcattcagcacctgctcatcctgaataccttgcgcacgtaattgatccagaagtgcttgtacgcgtctgcttaccattgcgtgccaactcccacgctgtttaaccagtctgaaaccacatcttgcgcgctatgcgcagttaaatccacatgcagcggcgtgatggagacatagccctcatctaccgcagcaaaatcggtccccggaccagcatcacatttaccgcccggcgggccaatccagtacagcgtattgccgcgcggatcttgctgcgggatcacctgatctgccggatgtcgtgtaccgcagcgcgtcacgcgaatacctttgatttgatccaagggtaaatccggaacgttaatattaagaatacgcccggtgcgcagcggctctttacacagtgcgcgcaaaattgaacaggttaccgccgcggcagtgtcgtaatgtttatgcccgtcaagcgagacggcaagcgccggaaaacctaaatgacggccttccatcgcggcggctaccgtaccggaataaataacatcatcccccagattcggcccggcgttaattccggacacaacaatgtccgggcgcggacgcatcagagcattcacgccaagatagacgcaatcggtcggggttcccatttgcacagcaatatcaccattttcaaaggtaaacgtgcgcagggaggattccagtgtcagagaatttgaagcgccgctgcggttacgatcgggggcgaccacctgaacgtcagcaaactcacgcaaggctttcgccagcgtttgtataccgggtgcatgtaccccgtcatcattactcagcaatatgcgcataatcacctgttgtgttgataagttccctgacaacgctggttgcaaaactacccgccggaagccagaaacggatctctacggtgacgtcatcccaccaattccagcttaattgttgcggatacagcagcatcgctctgcgcgcggcttcaactttttcgcgcaccagtaaagcttgtaattcagtttctgcggcgacagctgcttgttcgaatgccagcgcttcacgctgagttccccattcgccactgcctggcaatgcggcggttatcatcaactctttatcgttgacgcgacgctgtaattccgccagttcttcggtggttgcgacaaaccagctaccacgtccggctaattgtagcgcatcgccgtcaacaacttgattaacgtctgcttttttgaggcgctcagcaacaatctgattaaacaacgcactgcgggctgccgacaaccaaaaactccgtttattgcgatcgcgcaccggagtattggtttgcgcccagcgctgcgccccctgcaagttgctaccgccaatcccaaaacgttgggcaccgaagtagttcggtacaccttttacgcaaatatcgatcagacgttgttcaacgtcatcgcgattgctcacttcgcgcagaaccagggtaaaggcgttacctttcagcgcgcctaaacgcagcttgcgcttgtgccgcgcatactccagcacctggcagccttccagttgaaaggcgctcagatcgggcatttccttgcccggcacgcgagcgcataaccactgttccgtaacagcatgtttgtctttttgcccagcgaagctgacttcacgggcatgaattttcaggaatttcgccagtgcatccgccacaaaacgggtattgcagccgtttttgaggattctaaccagaatatgctcaccttcaccatcaggctcaaagcccaaatcttccaccaccacaaagtcttccggattggctttcagcagcccggtgccttgcggtttaccgtggaggtaagtgagattatcaaactcaatcattttgttgccttaatgagtagcgccaccgcttcacaggcaatcccttccccacgtccggtaaatcccagtttttccgtagtagtggctttcacgttaacatcatccatatggcagccgagatcttcggcaataaacacgcgcatttgtggaatgtgcggcaacatcttcggtgcctgagcgatgatagtgacatcgacgttgccaagggtataacccttcgcctgaatacgacgccaggcttcgcgtagcagctcgcggctatcggcacctttaaatgccggatcggtatccgggaacagcttgccgatatcccccagcgccgccgcgccaagcaatgcatcggtcaacgcatggagcgccacgtcgccatcagaatgcgccagcaatcctttttcgtaaggaatgcgtacgccaccaatgataattgggccttcaccgccaaaggcatgtacgtcaaaaccgtgtccaattcgcattatgtattctcctgatggatggttcgggtgaggtaaaactcggccagtgccaaatcttccgggcgcgtgactttaatgttatccgcacggccttcgaccaactgaggatggaatccgcaatattccagcgccgaggcttcgtcggtaatagtcgcgccttcatttagagcgcgcgtcagacagtcatgtaacagctcacgagggaaaaattgcggcgtcagcgcgtgccataagccgttgcgatcaacggtatgagcaatggcatttttgcccggttcggcacgtttcatagtatcgcgcactggtgcggcgaggatcccccccgtgcggctggtttcgctcaacgccaacaatcgcgcgaggtcatcctgatgcaaacaaggacgagcggcgtcatgcaccaatacccactgcgcgtcgccagcggctttcagacctgccagcacggaatcggcacgctcatcaccgccatctacaacggtgatttgcggatgattcgccagaggaagttgtgcaaaacggctatcgccaggacttatggcaatgacgacacgtttcacccggggatgcgccagcagcgcatgcaccgagtgttcaagaatggtttgattaccgattgagagatattgcttaggacattccgtttgcattcgacggccaaatccggccgccggaaccacggcgcaaacatccaaatgagtggttgccatgttaattcccgggctgatttatcgattgttttgccccgcagactgtgcgcgcttcgacgcgtcaggcaccagacgataaaaagtttcgcccggcctggtcatgctgagttcattacgcgcacgctcttcgagcgcctcctggccgccattgagatcgtcaatttcggcaaaaagttgatcgtttcgcgctttaagtttcgcgtttgtagcttgctgtgccgccacatcatcattgacgcgggtatagtcatgtataccgttcttaccgaaccacagcgaatactgtagccagaccagaatagccagcaacagcagcgttagtttacccatcctgccccctgaaaaacggcatcatcatcccatgcatccgaagacgactctacatcctctgttggggataccgcgacaacgcgggcaaatgtaccacatttgtccattgttacgtatacccagggcgtgcagaacataatctcattattagttacggtttgaattatgaacagaggagacgggaaagtacaaattagcccagtagccacataaacagtgcgccaaacataatgcctactgtcaccagggtgaaaacaatactgtagcgtagctttccgtccatcaatgaatgcagcgcaatccccaccactaccgcgacgggcatcagcgccagaaagaaaggccaggtgtagataaagaagaacagcgtgttagagccataaatcaacatcggcatcgccagcgcaaataaccaggagataaaaccgaccacggcaccaggcagtgaccatgtggtttcttcatcctcagtaaggctgtcgttatttgttagtgtaatgttatggctattacgcatatttgatcctgttactttgacgaaccgggcatggaaacccggtggtgtctcaggatctgataatatcgttctgtctcaacagatctaataattgctgtaccaaatttgttactaattgttcaccattgagatgaatttctgccgattcaggcgcttcgtaaacggaatctattcccgtaaagttgcgcagttcaccggcacgcgctttcttatataagcctttgggatcgcgggcttcgcaaatcgccagcggcgtatcgacaaacacttcgataaagcgcccttctcctacgcgttcgcgaaccatctggcgttcggcgcggtgtggcgagataaatgcggtcagcaccaccagtccggcttcaaccatcaaattcgccacttcaccgacgcgacggatattctctttacgatcggcatcgctaaaaccgagatcgctgcataatccgtggcgaacattgtcgccatccagcagatacgtactgacgccgagtttatgtaacgcctcctccagcgccccggcgaccgttgatttaccggacccggagaggccggtaaaccacagcactacaccacgatgaccgtggtgtagctcgcgttgttgcacagtgaccggatggctatgccagacgacgttttcgtcatgcagcgccattatttatcccccagcaaatcgcgcgcgccccagtgcggaaagtggcgacgaaccagagcattcaattccagttcgaatgcactgaattcagatggcgcagcagttgcctggctaactggctcgtgcaccataccggcacccacggtcacattgctcaggcgatcgataaaaatcagcccacccgtcaccggattttgttgataacgatctaacaccagcggctcgtcaaaagtgagatccacgaggccgatcccattcagtggcaggttttcaacttcacgctgggtaaggttattaatatcaacctgatagcgaatgccatcaacacgcgcgcgcgtcttcttaccggcaattttgatgtcgtaactctgccctggagaaagcggctgttccgccatccataccacatccaccgacgcgctctgcaccgccggtaacgcttcgtctgccgccagcagcagatcgccacggctgatgtcgatctcatccgtcagcaccagggtgatcgcttctccggcaaaggcttcttcgcgatcaccatcaaaagtcacgatccgcgcgacgtttgattccacaccagagggcagcactttgacacgttgcccgacttccacgcgaccggatgccagcgttccggcgtaaccacgaaaatcgagattcgggcgattaacgtactgcaccgggaagcgcattggctgagcatccaccactcgctggatctccacggtttccagcacttcgagcagtgtcggaccgctgtaccacggcatactttcactttgcgatgccacgttgtcgccttccagtgcagagagcggcacaaagcggatatccagattacccggcagctgcccggcaaaggtcaaataatcttcacgaatacgggtgaacgtctcttcactgtaatccaccagatccattttgttgatcgccacgaccagatgtttgatccccaacagtgtggagataaaactgtgacgacgggtttgatcgagcacgcctttacgggcatcgatcagtaagatcgccagttcacatgtcgatgcgccagtcgccatattgcgggtgtactgctcgtgccctggggtgtcggcgataataaatttacgcttctcggtagagaaatagcggtaggccacgtcaatggtgatgccctgttcgcgctcagcttgcaggccgtccaccagcagagccagatccagcttttcgccctgggtgccgtgacgcttactgtcgttatgcagcgatgagagctgatcttcgtagatttggcgggtatcgtgcagcagacgaccaatcagagtacttttgccgtcatcgacgctaccacaggtcagaaaacgcagcaggcttttatgttgttgcgcaatcatccaggcttcgacgccgccttcattggcgatttgttgtgcaagtgcggtgttcatcttaaaaatacccctgacgttttttcagctccatagaccccgcctggtcgcggtcaatcacgcggccctgacgttcactggtggtggaaaccagcatctcttcgatgatttccggcagtgtttgtgcatttgactccaccgcaccggtcagcggccagcagcccagcgtacggaaacgcaccatccgttttttaatcacttcgcccggttgcaggtcgatacggttgtcatcaatcatcatcaacataccgtcgcgttccagaaccggacgttccgcagcgagatatagcggaacaatgtcgatattttccagccagatgtattgccagatatcctgctcggtccagttagagagcgggaagacgcggatgctttcgcctttgttaatttgcccgttgtagttgtgccacagctccgggcgctgatttttcggatcccagcgatggaagcggtcacggaaagagtaaattcgctctttagcgcgggatttctcttcgtcacggcgcgcaccaccgaaggcggcatcaaaaccgtatttgttcagcgcctgtttcaggccttcagttttcataatatcggtatgtttcgcgctgccgtgcacgaatggattaatccccatcgccacgccttccgggtttttatgcaccagcagttcgcagccgtaggctttagcagtacgatcgcggaactcatacatctcgcggaatttccagccggtatcgacatgcagcaacgggaaaggcagcgtacctggataaaacgccttgcgcgccagatgcagcatgacgctggaatctttaccgatagagtagagcatcaccggatttgagaattctgccgccacctcgcgaataatgtggatgctttccgcctccagttgccgcaggtgagtaagtcgtatttgatccataaccgttcctttgcaataccgctattttcttgccatcagatgtttcgactatagggagcgtaagagaacgaatgaaattaccaattagaatgagtagttccttaacggaataacgatttggcaaagctaatatcaaaaagtgcttaaggcaccggatttcgggcgtttaggaagatttgaaattgttttagcgcagcggcagtttcatactatggcggtaaaaaaatttgcatggtatttaaggactcactatgttttccgcattgcgccaccgtaccgctgccctggcgctcggcgtatgctttattctccccgtacacgcctcgtcacctaaacctggcgattttgctaatactcaggcacgacatattgctactttctttccgggacgcatgaccggaactcctgcagaaatgttatctgccgattatattcgccaacagtttcagcaaatgggttatcgcagtgatattcggacatttaatagtcggtatatttataccgcccgcgataatcgtaagagctggcataacgtgacgggaagtacggtgattgccgctcatgaaggcaaagcgccgcagcagatcatcattatggcgcatctggatacttacgccccgctgagcgatgctgacgccgatgccaatctcggcgggctgacgttacaaggaatggatgataacgccgcaggtttaggtgtcatgctggaattggcagaacgcctgaaaaatacgcctaccgagtatggtattcgatttgtggcgaccagcggcgaagaggaagggaaattaggcgctgagaatttactcaagcggatgagtgacaccgaaaagaaaaatacgctgctggtgattaatctcgataacttaattgttggcgataaattgtatttcaacagcggtgtaaaaacccctgaggcagtaaggaaattaacgcgcgacagggcgctggcaattgcgcgcagtcacggaatagccgcaacgaccaatccgggtttgaataaaaattatccgaaaggcactgggtgttgtaatgacgcagaaatattcgacaaagcgggcattgctgtactttcggtggaagcgactaactggaatcttgggaataaggatggttatcagcaacgcgcaaaaacacctgccttcccggcgggaaatagctggcatgacgtaagactggataatcaccaacatattgataaggctcttcctggaagaatagaacgtcgctgccgtgacgttatgcggataatgctacctctggtgaaggagttggcgaaggcgtcttgatgggtttgaaaatgggagctgggagttctaccgcagaggcgggggaactccaagtgatatccatcatcgcatccagtgcgcccggtttatccccgctgatgcggggaacaccagcgtcaggcgtgaaatctcaccgtcgttgccggtttatccctgctggcgcggggaactctcggttcaggcgttgcaaacctggctaccgggcggtttatccccgctaacgcggggaactcgtagtccatcattccacctatgtctgaactcccggtttatccccgctggcgcggggaactcccgggggataatgtttacggtcatgcgccccccggtttatccccgctggcgcggggaactctgggcggcttgccttgcagccagctccagcagcggtttatccccgctggcgcggggaactcaagctggctggcaatctctttcggggtgagtccggtttatccccgctggcgcggggaactctagtttccgtatctccggatttataaagctgacggtttatccccgctggcgcggggaactcgcaggcggcgacgcgcagggtatgcgcgattcgcggtttatccccgctggcgcggggaactcgcgaccgctcagaaattccagacccgatccaaacggtttatccccgctggcgcggggaactctcaacattatcaattacaaccgacagggagcccggtttatccccgctggcgcggggaactcagcgtgttcggcatcacctttggcttcggctgcggtttatccccgctggcgcggggaactctgcgtgagcgtatcgccgcgcgtctgcgaaagcggtttatccccgctggcgcggggaactctctaaaagtatacatttgttcttaaagcattttttcccataaaaacaacccaccaaccttaatgtaacatttccttattattaaagatcagctaattctttgttttcaaacaggtaaaaaagacaccaaccttaaaccatccaaatctaccggggtacgcctgtttaacccaaatgtctggaactcaaatcccgtttccgtattcgttgcccatgccatcactacattgccttcttccgccagtccagctatttgttcccagatcatttcacgaatttttgcggatacatcacctacatatacccctgcacgtacctccaacaaccagatggctaatctgcctcgtaagcgcggaggtacattttcagtgaccacgaccaacatactcatttcagctactccgatggcctgcatctcccagtgaaacaggaagcggaatggcaacaggctgtgcatcttcaggtggggccggcggttgtatttctccagcggcaagcacgtcctctataagcggaatcaatttggctaatgttttactactgcgaaaaatatccctgcacgccaaacggacttcccggtccggctcaccagggttacgacgcgctatctcaaaagctttcggtacaacagtgtcaaatttaatgatgtctgcaatatcgtaaacaaaggaaagaggctttcctgtatgcacaaacccaatagctggtgcataaccagctgcaagtatcgccgcttcagttacgccgtataaacaggaagttgcagcgctaatgcattggttgatcgtatcgcccttttcccagtctttcggatcgtagcgacgtccattccatgtcacgccgtattgcttcgccagaagtgcgtaggttgcccgcacgcgactgccttctatacctctgagttgctctacggagcgccgggcaggcgcaggttctccaaaccgaagttcaaacattttacgtacgaccttcagacgcaaatcttcatccagagcaagttttgcctgatagagcagcttatctgaacgcgcacctccaggctgaccagaagcataaacacgaacgcccgcttcccccacccataccaacaatgttccaacttgcgcagccaggcgtacagctgcatgcgaaacccgtgtaccaggttccagcatgatgcaggcaaccgagccaacaggaatatgagtgcggatccctgtcttgtcgataagtacaaacgcgccatctattacatcgatctgcccatattgcagaaagatcatggagacgcgatctttgagtggaatgggattaaggggaagccaggtcattttattacacctcaatcacagtggagccaaagatagcaagccacatcccatcgatttagctggcccaataccttgctgtacaagatctattaacgctggcgcgtcgttgatggtgagcacaccttcaaagcaaaccgtttggatctttccacttttaccatcaccagaaaaatactgtggccgttccgatatgggatgcacatcttcaacgcgcgccgcattgcccaatttacgttgcaaccacgcgatttgttctgcttcttttattaacggaacccgacagcgtttaatattccctttactgtccaggcgcttttgattgtcgagaatagttttgatcggatttgcccgaagccgaaaatagagtggaacaccaacctgaagttgaaattcaacctgtttagttttaatgactgtcgcaacggcagttgaaacaggcatttgcgctgactgcaataaaacatgacagccttctggtgtgtttcgcttctcaacatgaaaaagaaaatcacgagcagcatccggtctgtttggaaataaatgccataatccctggtgaagttggtaaagatccctgctccaggccctggcaatgatgactttactgagatacatccatacctcctttaatcacataccattctcgggaagcaaattgtcgaggcaaggtgatcatcggttcgtcgcgcgccgtaaattttaaatgatgccctgtaactgattcctcactatatatatcgccgccaacgggctcataatttaatagcgccttctgaggatccgatgcctgacatgtccccaaaaaaagcgggtgtgttagtgggcaacttctccgccccaggtaaggtgtataccgaggctttaatactgctttttcaagttctgagataaccatcgttgcatggggtgttaaccagagagcgacggtaaaggaggcatcacataaatattcgcgccatgtttgaatcgtttcatgacttttcaaaccacggtaatcttctcgcgctccaaggactgtatggtaatcacgcaaccccgttacagacacacgacgatcgtcaagaatgagttcatcgcagcgcactgcaaattgcacactctctgataacgcctgtaatgaagaagtatcatcacgttggatcccaagacaagccccgagtagccctaataacccgcttcgggtcggaaatcttccggtaggtcgcgttccttcaaaggtcggctgcccccaggcttgcattggcccagcaagccgcaagatcaaataagatctcatgttcacgcctcgccattattacgaacccaggattttaactgttctaaagtaggcatttgtttaacttgagcagtaattgggtctacatcagataagctgaattgcgcagcagctccgttcagaccatatccattggcaacgcgatcccaatattgattaaacgcctgtatagacggttgcaaaaagccatctttcgctttaaccgctttttcaaaagcatttgccatagaaagtggcatatcggagaaattaaccattaccatatccgcagggttaaaagcggcataagtacgctgttttgctccagggacctctgttgccagcatatgaacaacatgggttgcaatttccagagcctgctccctggaggcaccacctaaattttcctgaagttgagcgaggttaatgttggcataacgataaaaaacacccgatgaaaattcctgagttcccagatgtgcagaaccttgttcctgtaaatcatctacagcggtgaaccagtcaatatcagaatcaacctgatgagtagtgatcgcatgcgcaatggacattgcaccatcaacttttcccaactcagtcatcatgccgctggttgccattcttccactaagcgcaatatcaacaccctgctgtaaattcacacgtatggcggcaatatcttccttaagaactttgagcagctttttatcatccagattatcagcctctgcttttgcaacctgctcacagaaccaggctatttctcccacaacccagggagtaaccgcatcggcagaaatcttttcggcttcatcaactgatttaccggagagcagcgctaatgtcttatcgatgattttttggtcaaaacgttcaccaagtttttgccgaagaacatcacgtaattgtgcaagatgaatggttctgagactggattcaccaatattttgtgcgtaataaccacttttacgcatcgcacgtttaaggctttgacttgaaattcttactcgtcttttgccgccgaaaatagcgtctttctgcatgttcatatcgtcgcggttcagacatgaagggctgtgagagatcagaacatgaatattgataaagttagacatagaaaggtttccttacgcatttttgtttgtggtcaatacaaaatcttccagaagttgctggcgttcgcgctttccccaccaggtcaacatcctggccattaatggccagtcaagtacgggttcggcgtgagtaagtaatcgacgtaactggaccatatcggctgttctgtcagcccgaattaattgaaagatacggcgctcgttaattcttccactattggctaaagctcttcccaacgagatacctgttgtttgctccgattttttgtcctgatgtcggatgacattctttcctgcgctcaggcaaaacaccatgcgcaaaagagcctgctggtgacgtgggttttcccaaccaaaaggttgcaccagcctataaaacgcagggatatcgcgtaattcatcaggttctgaaacacgtctaatttgcgcacatgatccattatccagttgttgccaggctcgatataaagccattgcatcaatttcatcagccatttgatggccctccttgcggttttaactcccgtaaatgtttgtatagcgtggcgcgggcaagcgctaatgtgcttattaatttaggatgatgtgcatagggagctacagattgattaaatagcatttcacacaattgatgaagtttgtctcgtaaatcagctattacctcatcagcctgggaaaaattaacattcgccagtacatcgggaattaataattcactctgtcgatagaaatgcctttctgcagtctcatgaacagagactccggcccctttgaagtctttatttttaaacccttctgcaaaggtatataacgccttgcgtaaggctgttttatatcccaaaccaacagtcactatttcgtttatcacattgccgtattgttgccacccctgattaaacatcaacacatcatgacgccgttcaagaatagatgcttgattattacgatatccccccataatcaattcaagaggactttgcggcgcaatatttctgaattgattcacaaccgccgccacgcgatttccattttcattttgaataatcttatctaccacaactcggctgatttgtgtccatgatggtgcggaggtggtgaaagcaagaaatttttcctcaacctcccctttcttgactgttaccagacaaggggaatgcggatggggccatagcccattaactgtaaaggtaaatttttccttaagaaaaccggtataacgcaaattgctttcctgtccacagcaagaacatttaccaatcccaatgggatcgcataattcaatatgcgctggttgccagaatagaccacggacaaacccaattgacgaagcaggtatagactcattggacttgataggtttaatccaggtaggttggttttccgtatgtgattcattaggaaattgtttttgaagacgaggtaatgtgaggacattgagtaacaccgttgaacgaagatcgatcccacgtacgaacgttgttacaggtgttcctccacgtaaaccgcttttaaaaccaccaccaaaacctggtgcctgattcgcctggttgaataacgcaatcgcagtgcatccaccacataatgcttcaccctgccccggttgattgacaaatgcacaattcgtcgcgccgcttaccccagccaacagtttttccattggagtcacatcatttgctttgacacctttggtctgcataaagggatgttctgcgtgattaaggtagaacatatctatccacggcgcgatgagttgttgaaactcatcttcagtgagcggattcattatgcgatgtcgaaattcaacgtcatcttttgccggggcgataatttgcccaatgcaaaccagcagtgctaaagcggccagttccatatcgtcacggggcaaacttaatcgccactgatctctactgcagtatagcgattgcagatttatgatttggactttccccccgtttcgcgggcgtacagggatccagttatcaataagcaaattcatttgttctccttcatatgctccgacatttctcctgcatttctatacgtcggcacacttccgttatcggtaaaaacaaagaaaaaatacggcgtaattaattcaataatcacattcactgcaaaaatatattcattggtttaatacaattaacctatacatatattaagatgtgttgaattgtttaaagacaataatgcatgcatttcaaatctgcaagttattcgttttattattaaagaaacttttagttataataattaccatgaattttattacataaaatattcatactgtgaatataaaatctcataccgggaaattaaaagaagatgtacattgtgcaccttccctacttaagtagggataaaccgttattggtcttattatcgtcattgataacaatcattcccgaagttatttgggatttgcagggatgactctggtcatcccttcatcccctgtataggtaataacaatactgttaccctgccagacccatccatccagattctgtttcccttccagccaaagtaacccatcttcatctactacttcagaaaaactacgtttccaggtgaagggtacattgacgcgattaagtgcaagcgcctcatactgctgttcatgacttaggtcctcgtagacctggccatcgagcagttgtttacctgaagacgtttgtacataaggcaataatggcaggctcatttccccatccctcgttaccgcaagaatggtttcatcgttatcctgcaagctatattcttcagcccactgcaggaccttgcgagccttgaaccttttttcacactcggcgctttcaaatttatccatgccattgccgacccattctggctcatccatttccgcatcatcgtaaatgctatccagccattgccggtaagcatcagggaaaaataaggatgctccattaagctcctcaatatgttgctgcgtccgccacatgactctaacgttgctataaatatgctcatgtcgtccgtaaccctcgccatcaggcagcaaaatggtggcaacaggaatctcaaaaccagcgggacgatatttgcgatgatggcgatgtaaacggcccaatcgttggaaaagcaaatctgcaggacaatgctgagtaattaaccaatcaaaatcaacgtcgagtgattgttccacgacctgggttgcgacaagtatccgtccaacatttcgcttcccatttttgccgaaattgctaataactcgattctctttttcacgacgatcgttcagcgtaaagcgcgcatgaaacaaatctatatctacttgcgtgttatttagctcctttagccgttggtagcatacttgtgcaacgtcaaccaaattgcaaataagacagacctgtgcacccgcgtttgccgctgcgatcattcgctctaacatcgtaaggtcaggtaacatgtcagctaaacaaataggttctggctgaatcgaaaagcggggcgggagttgttctggatgagctagcagatcaaaacgttgcgcaccattcacacctcgccagttaatgagtggatatgcggagttattttccactggatctgtatgcagaccataagtatccagaagtttctgtttttgtttcattggtagggttgcggaaagaagaataacactccctcccacatcagcctgagccttgagcactgcctccagcaagccgttcatataggtgtcgtaagcatgaacttcatcaacaattaaaacacttcgaccaattcccaaaccacggataaagcggtgtttaactggcaataccgatatcaacacctgatcaatcgtgcaaacgccgatttgcccaagaaacactttcttattgctttgtgacaaccactgacaacactgaacccacgcttcttcttgcccctgttcagtaatcgcgcgtgattttattgattgaaagaggtggttaaaccgtgaattgccatgagcaagaataagatttggggatgaaaataagtggctcgcgctcgcttccattctcgtaagcatagcattcgcggtagcttgtgttgggagggcaaaaataacactatccgcaatttgttgatcaataagtttccaagcataggccagcgctgtttccgttttaccggagcctgtaggtgcctctattaccgtcagcccgggagctactggaagagcatcaactaacacctgtaattgtctgggttgatagccattgtccagtagtgcatgaacaccttcataacatcgcttatttgatacaagtccactcaactccaatacccggctcgcatcctgctgtcggtcctggaaatacgttctcagagcatttatgtcggaaggcgcatcctcattaaacagaaaggtattcgttgtagtccaggagcctaaccagtcagcaagcgagcaaaaacctgctaacagtgatgaacaatcaggtggtatatcgtttatagataaccccgctggcgttaaaaataatgcttccagtacagatatccactcctcacgagcctgtttatcttgcgcagcataagatgccagagaagctggcatttcccaacgcgacttatcttgatcctgggaatgtaatataaaaccatgatgtcctgtaacggcctctacccatggaaaccaggactcataaggatgaggagcggcatcaaaaaaactgaaaaaatccccgagagattgctctgaaagtgaatcctggttaaaccaatacagaccggctgcaccatgattaaatttacggcacatttgtgttgatggaccattaagtgatggcgttgcaggatttaatttcagccaactttctgctgatttatattggaatcgtatatcaaactttccaatatcatgaagagcaatgaaaaataacagccaggccttcaccctctgttttgatagcatttcatttcggcaaaaagtattttgcagtacgactgattgatcccaccagcaatctgcaacagcagcaacatcaaggcaatgataaattaacagatgaatatcatttcctttcgtcaagctttttgaggattttccccagtaatggcatatatatttaaaaggttccattaatagcctccctgtttttttagtattatcgatgatatcagcgggctatttttcgatgctgctcataaatatcgaattacagtgatatacacatgtcttgcctccctgcaaagaagagactaacattcgaattgtttgggttcgaacgctggcctcaggttgatagaaatatcgcctggggcttttgtccatctggaacctcgcgaatgcttaacgccagacagcctcaagcacccgacgccattctatacctgataattcttcccgcggcgttcacgtttaaaatcaggaatgctgctcgcaaaataaaaacgcccccatcatttctgacagaggcgtttaatttgtccggcaatatttacccttcgtgtaacccacattccctttttaagccaaagaaacgcgtttcttcttccgccatgccgggttcccatttacgggttgtatgggtatcgcccaccgataaatatccttcatcccataatgggtgatatttcaggccatgtttttgcaggtactgataaatagttcggttatcccagtcgataatcggcagcactttaaatacgccacgctgaattgccagcaccggtaaattggcacgactgccggattgttcacggcgcaggccagcaaaccaggtttgcgcattcagttctttcagagcccggttcatcggttcgactttgttgatgtcattgtacttttcaatgccttcaacgccctgctcccacagttttccgtagcgtgcttcctgccaggctgcgctttcggtagcacggtacactttcaggttgagcttgagtttgtccgttaactcgtcaataaagcggtaggtttccgggaacaagtaacccgtatcggtgaggatcaccggaatatccgggcgaatttgattcaccagatgcaggctcaccgccgcctgaatgccaaagctggaagaaagtacatattcaccgggcagattatccagcgcccaggctacgcggccttcagcgtccagtttttccagttcggcgttagtttccgccagcgccagaatgcgatctaccttcggcagttcgttcagggcgtttagatcgagtttggacatagattcctcactgtttgccttgcctgatgcgacgctcacgcgttcttatcaggcctacaagaccgggctgatggttaatcccacaaatcacgcgccggatcgagcaccgggcgaatgatgcccgcacgcaccgtaaagtcgccgaagccttcacccgcttcgcgctctttcgcccagcgccctatcagttcatcaagcgacgccaggatttccggctcggtgatgttttctttatacatccgtgggatacgtgtcccaatgcggttgccgccaagatgcaggttgtagcgacccggcgctttacccaccaggcccacttccgccagcatcgcgcgaccacaaccgttcgggcagcctgttacacgcatcacgatatgctcatcgctgacaccatgtttcgccattaaattatcgatgttgtcgataaaagacggcaggaaacgctctgcttccgccatcgccagcgggcaagtcgggaatgacacgcaagccatcgagttttcacgctgcggcgtgacggcattcattaacccgctctctttggcgatcttctcgatcttcgctttctcgctttccggtacaccggcgatgatcagattctggttcgccgtaatgcggaaatcgcctttgtggatcttcgcgatctccagcaggccggttttcagcggacgcgccggataatcaaggatgcgaccattttcgataaacagcgtcaggtgccagttatcatcaatgcccttaacccagccaatacgatcgcctcgtccggtgaactcatatggacggatcggttcaaatttgatccccgcgcgacgctccacttccgctttaaacgtctcaacccccacgcgctccagcgtgtatttggttttggcatttttacgatcggttcggttaccccagtcacgctgagttgtcacgacggcttcggccaccgccagcgtatgctccagcggcagatagccaaactcactcgcggtgcgggcgtaggttttcttgttgccgtgttcgatggaaagcccaccgcccaccaacaggttaaagcccaccagcttgccgttttcggcgatcgccacgaagttcatgtcgttggcgtgcagatcgatatcgttctgtggcgggatcactaccgtggttttgaatttacgcggcaggtaggtctggccgaggatcggttcttcatcagtagtggcgactttttcctggtcgagccagatctccgcatacgcgcgggtacgaggcaacagatgctcagaaatcttcttcgcccactcgtacgcttccgcgtgcagctgcgactcgtaagggttcgaggtgcagagtacgttacggttcatgtcgttagctgtcgccagcgcatcaagaccgaccgagtgcagcatctggtgcaccggtttgacgttctttttcagaatgccgtggaactgaaacgtctggcggttggtcaggcgaatgctgccatagatggtgttttcaccggcaaatttgtcgatcgcctgccactgtttagtggtaatcaccccacccggcagacgacagcgaagcagcatcgcgtggcgcggctccagcttctgttcagcacgttcggcgcggatgtcgcggtcatcctgctgatacatgccgtggaagcgaatcagcaggaagttgtcgcccttaaagccgccggtcagaccgtcgtttaaatcttccgcaatggtgccgcgcaggtagttgctttcatgcttcatgcgctcggcgtctgtcagttttccttcgaccactaaaggccctggatgtttttcgctcattagtagacatctcgctgataacggcgctctacgcgcagctcacttaaaaattcatccgccgcttcggtgtccatgccaccaaattcggcaatcacttccagaagtgcctgctcaacgtctttcgccatgcgattagcgtcgccgcagacataaatgtgggcaccatcattgatccagcgccacagctccgcgccctgttcgcgcagtttgtcttgtacgtaaactttttctttttgatcgcgcgaccaggcaagatcgatacgtgtcagcacgccatctttgacgtagcgctgccactccacctggtacaggaagtcttccgtaaagtgcggattaccaaagaacagccagtttttacctggcgcttcgtcggcggcgcgttgctgcataaaggcgcggaacggcgcaataccggtgcctgggccaatcataatcaccggggtttctggattggctggcaggcggaagttatcgttatgttcgataaatacgcggacttcgccctcttcttccacgcggtcagcgaggaagctggaggcaccaccggcacgggcgcggccttccacgtcgtaacgcaccacaccaacggtgacgtgtacttcgttctcgacttccgcctgcgaggaggcgatggaatacagacgcggcgtcagcgggcgcagcagattaattagcgcttcggcatcaagctgtgccggggagaaacgcaccatgtcaacaatcggcgtcgtcgcggcgtaatgctgtaacttcgctttatcgcccaccagcggcagcagtgtttcactgcgggtaagcgtggcgtaattctcaacaatgttggcggtgttgacggtcagttcgaagtgccactgtagcgcttcgttcagaggcaacgttttgccctcgacggtgacaggttcatcgcctttcagccacagcagttcgacaagttctttcaccagtgccggatcgttctgataccagacgcccagcgcgtcacccggctggtaacgcatgcccgagtcacctaagtcaatttcgatatggcgaacgtctttttcagagttacgcccggtaattttctggttaacagagaggctagccaccagcggcgcgtctttgctgtacgggctggtgtggatttcatttaccgcgccagtagcgacggattgcgaaggtgccgcgacaggcgcacgcgatttaagcgcatcaaccacgcgggcgcgccactcgctggcagcagcctggtattcaacatcggcatcgacacggtcgagcaggcgttcaccacccagttccgccagcttgctgtcgaaatctttcccggactggcagaaaaattcataagagctatcgccgaggctaaacacggcaaacgcggtgttttccagctttggcgcttttttggagaacaggaacttatgcagcgcgacggcttcttccggcggttccccttccccttgcgttgacgtcactacgatgagcagtttttcgctggcgatttgtttgaatttatagtcgcccgcgttcaccagcttaacgttcagttttgctgctaataaatcatcacgtaatgcttcagcaacccggcgcgcattgccggtttgcgaggcggagataatagttatacccggcatttctgcggctggcgctggcgtcgctgcaagcgcagcaggctgctgattgagtacgccccagaaatagccagaaacccaggcaagctgggtgggagttaaatcggtcgtggccgcctgaaggcgtgccagttgctccgggttcaacggaagcaacgcggaaggtgggacctgtgtcgtcatgcgtcgttatgttccagtaagcaaagctgtttctgcgccctgtcagcgcccataaaacagaagagaaggtaaggttaacggggcaaacggtgtggattaaagacgggatagcgataactaataaccaaatcgactaacctgttttagcaatagtctttaacaacaaaatagattaaccaacctaatgaaaaacaaatgaatttagccaatcattaagataaatcagcgattttgcgcaacaaagtcgttttagataatgcgaaaaaacagcctttccggtactctacggcggttttatcgtcctgtagagaaattatgatgtccaccacgttatttaaagatttcaccttcgaagccgctcaccgcttaccacacgtcccggaagggcataaatgtggtcgcctgcacgggcattcctttatggtgcgactggaaattaccggggaagtcgatccgcatacgggctggattatcgatttcgctgaactaaaagcggcgtttaaaccaacctacgagcgcctcgatcaccattatctcaatgatattccaggtctggaaaacccaaccagcgaggttttagcaaaatggatttgggatcaggttaaacccgttgtgccgctgttaagtgcggtgatggtaaaagaaacctgcaccgcaggttgtatctatcgcggcgaatgataagagtgtgtcggcggtcaatttcccttaagtaacgctatgttagggtgttgtgttctggatatctggggcatgacatggaagacgactgcgacattattattattggtgccggtattgcaggcaccgcttgcgcgttacgctgcgcgcgagcgggtttatccgttttgttactggaacgcgctgaaatccccggcagcaaaaatctttccggcgggcggttatatacccatgcactcgcggaactcctcccgcaatttcatctgaccgcgcctcttgaacgacgcatcactcacgaaagcctttccctgttaacgcccgatggcgtaacgacgttttccagcttacagcccggcggtgaatcctggagtgtattacgtgcacgattcgatccgtggctggttgccgaagccgaaaaagaaggtgtcgaatgcatccccggagcgacggtggatgcactgtatgaagaaaacggcagagtctgtggcgttatttgtggtgacgatattctccgcgcccgttatgtggtgctggcagaaggtgccaacagcgtcctggctgaacgtcacgggttagtgactcgtcctgctggcgaagcgatggcgttggggatcaaagaagtgctgtcgctggaaacatccgctattgaagaacgttttcatctggagaataacgaaggcgcagcgttgctgttcagcggcaggatctgtgatgacttacccggcggcgcatttctttatactaatcaacaaacgctctcgttagggattgtttgcccgctctcttcccttacgcaaagtcgtgttccggcaagcgagctgctgactcgctttaaagcgcatccggcagtgcgcccgcttatcaaaaacacggaatcactggagtatggtgcgcatctggtgccagaaggtggcttgcacagtatgccggtgcaatacgccggtaacggctggctgctggtgggcgatgcgttgcgcagttgcgtcaataccggaatttccgtgcgcggcatggatatggcgctgactggcgcgcaggcggcggcacaaacgctgataagcgcctgccagcaccgcgagccgcaaaatctgtttccgctttatcatcacaacgtagagcgcagcctgctgtgggatgttctacagcgttatcagcatgttccggcgcttttgcaacgcccgggatggtaccgtacgtggcctgcgttaatgcaggatatttcccgcgatttatgggatcagggtgataaacctgttccaccgctgcgccagttattctggcatcatttacgtcgtcacggcctgtggcatctggcgggcgatgttatcaggagtctgcgatgtctgtagcccgtaatctctggcgcgttgctgatgcgccgcacattgttccggctgactccgttgagcgccagacggcagaacggttgattaacgcctgtccggcaggtcttttttcgctcacaccggaaggtaacttacgtattgactatcgcagttgcctggagtgtggcacctgccgtttgctgtgcgacgaatcaacactacaacagtggcgctatccgccttccggattcggcatcacctaccgctttggataaataataaggataatttatgcccctcttacacctgctccgccagaatccggtgattgctgccgttaaagataatgccagcctgcaactggcaatcgattctgaatgccaatttatttccgtgttgtacggcaatatctgcaccatcagtaatatcgttaaaaagattaagaacgccgggaaatatgcttttattcatgttgatttgctggaaggcgcgtcaaataaagaagtcgttattcagtttttgaaactggtgaccgaggcggacggcattatcagtaccaaagcctcaatgttgaaagcggcaagagcggaaggttttttctgtattcatcgcctgtttattgttgattcaatttcgtttcacaacattgataagcaagttgcgcaatcgaatccggattgtattgagatcctgccaggctgtatgcccaaagtgctgggctgggtgacagagaaaatccgccaaccgctgattgccggtgggctggtgtgcgatgaagaagatgcgcgtaatgcgattaacgcgggtgtcgtggcgctttccaccacgaataccggggtctggacgttagcgaaaaaattactttgacgggataatcgtaaccaattgaatttggtttgatttgtaggccgcacgccacatccgacattcagcgcctgatgcgacgcttgacgcgtcttatcaggcctacaagtccccaggccagaaccgtaggcaggatcatccggcaacacgttattggcaatctgcgtgaatgtttgtcaccagtgcctccagcaccactttccagtcatcaaccacgccaacatctgcctgtgaaaataccgcagcgctggcgtcatgattaatcgccaccacaaacttgctattgcgtacgcccgccattaacgctgctgcgccagaagcgccaacaacaatacacacctcaggtgccagcagatgtccggaaataccaatcactttttcagcatcaacgccaccgttcatcactcgcgcccgactgtagcccacttcggctcccagcttttctgccagcatagcgatttcctggttatctgcctctccgccctgccccaccaccagcacccgtctggcctcagctaatgggtcgcgggtaacatttttcagatcctctgtgctaaccagccagtccggaagcgcacccgggacaatgttcagttgttgcattccagagggcaacgtggcgtttttcgctgctcccgcctgacgcgccagggaaaggcatagcgggcgtttttctgtttgcagcgtcgccgttagcgcatttccccagtgggatttgcgcacgcttacggttggaatatctaacgaagtcacctggcagatgcttgcaccatgtaaacgccaggccagccgggtcgacagttcatcgccaaacgttcccggcggaaagagaacaacgtccgcaggcgttcgctgccactgttccaccaacgcatccagcacctgttccgccactacaggctgaggttcaatctgccagtgcgccagggtacaaccgctgaaatcctgcgccgccagccagcttgctattgcggcattctcctgatttattgtcacaattgcgatattcatggctgcatcctttggcgtaaatagtcctgccatagcttttgagctttttctgctaccgtttgcccatcaatcagcgtcgctccgcgtcgttgctctgctcttgccagttgcagacactgcatcgctggcatttcggcagcaacagttttacggataatttctgctttccccgcagccattcgctggcgcattcccggtactggcaaggccacttcaccgcactgacgcacggcaatcaccgcaggcaagcgaacccggcaacaacgcaacccatgttcagtacgctgttcgagggtgataaacagcgcgtcgagagtgaaacgctccacctgggtgaagcagggccagcccagcatttccgccagcaaaaatggcgtttgcccattctgcccttcgctgctttggcagccggtaattatcagatccagcggattctgatgctgccattcggcaatatggcgagcgacaaattccggcgcaaagcgcagatctgccgccgtctccagcaatacagcttcctcaaacccaagagccatgagatagcgcagccagtgcaatgcccgttcatcccccatgctcaacgcggttaaagacatcggcgtaccgttttttctctgcgccaacagcagcgcggcagcggcctgttcatcagcaccgagtaaacttcgcagtagcgaaatatccggtccgcttttaccctgagccgccgcctgccactctttttccgccagcattccggcatccggttcggctttaaacgctaacagaatgttcattcgcacctcctacatttcccgccgccaccagcgggagggctttagtttctggtgcccatagccaggtcacaacaaaaccaaccaacaacactgtcgccaggagcaataaggtgacttgcattccccactgcgccagcacccacggcagcaggccagtacttaccgccgcgccaagtcgactcatggcagtggcaaaaccgacgcccagcgagcgaatgtcagtaggaaaactttccgcaggcaaaatgcccaccagattactgactgccgaaatggtggtgctgaagagaacaaaaagcagcagcgttaatgaactgccggaaggcaaacaggccatgactaccagcgttgccgccagcagcaaaaaacttcccagcaaaaatttgcgatgtgccagcaggtgcgtcagaactaatcccagcagcgcgcccacaattaacaacgcattaagcatcaggctggcagtcagcgcatcttccagaccaatagtctgggcgatagttggcagccaggtataaatcacaaaccatgggattacgaggcagacaaagaagacgctgttaaacgccgtgcgccgccagtaacgcgaagagaacaaggttttgatgtgtttatgggtcgccgttaccacttcatcgcccagtaaaacatggggaccaaaatagcgatgcacgatagcgtgagcttctgcaaaacgcccctggcgcagtagccagcgtggtgattctggcgttccccagcgtaataacgtaatcaacaacgcgggcagagctgccgatgccagtagccagcgccaggcctccgggttttcggaaataaagtgatgtccggcaatacttgccagcacatagcctacggtccacaccacgctgaatgcgcccagcaaaataccgcgatggcggcgcggggaaaattcagccagcaaggtgtgacctactgaataatcgcctcccagaccaatgccaatcaaaatgcgcagtccaataagatgctctggcgtggtggcaaaaaattgtaaaaacgaagcaagcgtaatcagcaaaaagctgaaggtgaagattttttgccgaccaatatggtcggagatccacccaagaaccaggctgccaaggaacaaaccaaggagcgccgagccgccgatcattcccgccataaacggcgtcagttgcatggcgggcgtaagctgaataatggcgtaaccaatgacgccgagaacataaccgtcggtcaggtgtgcgccgaaagtgagcgcagcaatgcggcagtgaaaacggttaagcggtaaatcatccattcgcaccggtgaagtgttcatctttaccccttcattgtccggtaataagaacggcttctcgcctgagaagccgaaaaggcaacgccccgtcatcgcggaacgctgcctgacacattatttttcaatcggatagatagtacccgtattcataatgccattaggatcgaactgctttttcagcccttccagcaacgcccacgcgctgccgtgttccagtttgctccagtgaacgcgatgtttaccgataccgtggtggtgcaccatcgaaccgccgaggcgaatggtttcttcacagatgatcttgttgagcggattgtggtacttgtcgatttcctcttccggcttacagtcaacgacgttgtaatcgtagacgaagtacatgttggtgccgttctgatagctatgagaggaatgaccgcccagcatggtgatgtcgtcggcgtgcgggaactcagtacgaatacggttaataacgctttcgtagatttcgtggatgcagctccagcagccggatacttcggtggtaaagcccatgttgccggttttgaggatctgcacacgttcggcagccactttatccggtccccagttcaggttgttaaaccaggtttcgatcagcttgctgtccacgcgctggcattgcgggtagcgggcaacgatttccgcaatcccttcgcccgtcaccttcgcaatgcgagggttaccttcagccataaagatcagcacgcattttccgtcggcaaaatgggtgaagtgttgggtgccatcttcagcgtcatacaaacgagcgattgacggacgatacccttccaccatgatttcacgcaggatgttgaagccggttttcatgtcttccaggatatagccgtagaagaggttgttttccggggtgaatttaaagattttcactgttacttcagtgatatagcacaatgcaccttcgttgccgatgatgatgtgacgaatgtccgggccagccgcgcggcgtggcacgtttttaatgcgtgtgacggtgccatcagccaatactgcttccagaccaacgaccatatcttcgattgcgccgtagagtgtggagaactgcccgatacttcgggttgctaccaggccgcccatctgcgccagcggctttgactgcggagaatgccccgtggtgtaacctttttcacgcaacgcgttttccagcacttccagcggaacaccacattgcgccgtcgcctgcatattctcaatatcaatattaatgatttgattcatggcggagccgtcgagcaccaccgagttttctacaacagtttccagcccaccttcggtggcggaagcaccggtacgcggcacaccgttaattttgtgcgcattcataaaattcagcacacgggatacttgctctgtggaaccgagttttacgaccgctgccggaatcggcaaagtataaatgccatgaatatccggaaatttacgaaaacggtcaatactgtttttctttaatactgtttcatcggtaattacgcgatctgcaccaacaatttcctttagctggtcgacaatcgctgcgcgagataaagacatagtaattccttcctgataataaaaatggaataatcattaataagagaaaacagaaaccaccgttatgggttagcgcactaaataaccgccatcaaccactaataaatgcccgttgacataattcgatgccggacttgcgaggaatacggctgcgcccattaaatcctgagtatcgccccaacggtttgccggaatatgatcaagaacgcgctgattggtttctggattactgcgtgtcgccagcgtaatatctgttgcataatagccaggggcgataccatttacctgaatattatattgacctagttcatcacaataagctttggtgaacccggcaagagcatgtttagtggcagaatatgcaggtgaccattgtccacctaagtaagagaacaatgaacagatattaataattttgccgcttttctgcgggatcataatttttgcagcttcatagcttaactcgaatgcggcggtcaggttcacatcaatcatcggatcccagtcggcacgaccgaagtccagcaccttattcagcttacaaataccggcattgttaaccagaatatcaactgtaccgaaacgctcacagcaagcagcgataatcttctgcggcgcgccttctgcggtgatacccacctgcatgaagtccacctcaacaccctgtttttcaatcatttcctttgtttcgccgttatctttgacgaaactaggaataaagatatttgcgccagctttggccaacgccatggcaaatgcctggcctaaaccgctattcccaccggtaacaattgcggttttacctttcagggagaaaaaatccattgagaacgcattgagagattcgattgacatagttagctccaatttccgtaaggcaaaaaaaaagaaaggtaacttcccccgcgagagggaagttacctttctcattatctctggtaactggagataatttttagcataagggcataactgctaatgtgatcgtaatcacagtgtgatattcgtattgtcaaataattttaaaaagcagaagcgtgattactctcacacaacacctctgctttccatgttatttattatttcaattactagagacctgagaaaagtaatccacctgaaagggcggcttacttttctcttttttttgtctattacaaatgggaatacgatatgcaacacaactcatatcgccgttggataaccctcgcgataattagttttagcggcggcgttagtttcgacctggcttatttacgttatatttatcaaattcccatggcgaaatttatgggattcagcaataccgagataggtttaataatgagtacctttggtattgcggccattattctttatgcccccagcggcgttattgccgataaattttcacaccgcaaaatgattacttccgcgatgatcattaccggattactgggtctgttaatggcaacgtatccaccgctgtgggtaatgctctgtattcagatcgcctttgcgataacgacgattttaatgctgtggtcggtgtcgattaaagctgcatcgttgcttggcgatcatagcgagcaagggaaaattatgggctggatggaagggctgcgcggcgtcggtgtaatgtcgctggcggtgtttaccatgtgggtcttttctcgctttgcaccggatgacagcaccagcctgaaaacggtcattatcatctatagtgtggtttacatcttgttggggattctgtgctggttttttgttagcgataacaacaacctgcgcagtgccaataacgaagaaaaacagtcattccagcttagcgacatcctggccgttttgcgtatcagcaccacctggtattgcagcatggtgatttttggcgtcttcaccatctacgccattctgagttactccaccaactatctgaccgaaatgtatggcatgtcgctggtggcggcgagctacatggggattgtgatcaacaaaatattccgcgcgctgtgcggcccacttggcggcataatcaccacctacagcaaagtgaaatcccctacccgcgtgatccaaatcctttccgtactcggcctgctgacgttaactgccctgctcgtcacgaactctaacccgcaatcggtcgcgatggggattggcctgattttactgctgggattcacctgttacgcctcacgcgggctgtactgggcctgccctggcgaagcgagaacaccgtcttacattatgggcaccacggtaggtatttgttcggtgattggattcctgccggatgtcttcgtttacccaattatcggccactggcaagacaccctgcccgctgcagaagcctaccgcaatatgtggctgatgggcatggcggcgcttggcatggtgattgtctttacctttttgctgttccaaaaaattcgtactgctgatagcgcccccgcaatggctagcagcaagtaagccaggaaaattacaggagaaaaatcatgtcgaaaaaatacatcatagggattgatggcggaagtcagagcacaaaagtggtgatgtacgatctggaaggtaacgtggtttgcgaaggcaaaggcttattacagccgatgcacacgccagatgccgatactgcagaacatcctgacgacgatttatgggcatcattatgttttgccggtcacgatttgatgagtcagtttgccgggaataaagaagatattgtcggtattggtctgggatccatccgttgctgccgtgcgttattgaaagccgatggcacgcctgctgcgccgttgattagctggcaggatgcacgcgttacacgcccttacgaacacactaaccctgacgtggcatatgtcacctctttttcgggttatctgacgcatcgcttaaccggcgagtttaaagacaatatcgccaactattttggtcagtggccggtggattataagagctgggcatggagcgaagatgctgcggtaatggataagtttaatatcccccgtcatatgctgtttgatgtgcaaatgcctggcaccgtcctcggacatatcacaccacaagccgcactggcgacacatttcccggcaggactgccggttgtttgtaccaccagtgataaaccggtagaagctctgggggccggattactggatgatgaaacggcggtaatttctcttggcacttacatcgcattgatgatgaacggcaaagcactgccgaaagatccagtagcgtactggccgattatgtcttctattccgcaaacattgctgtatgaaggttacggtattcgcaaaggcatgtggacggtgagctggctgcgcgacatgctaggcgagtcgttaattcaggatgccagggcgcaggatctttcaccggaagatttactcaacaaaaaagcttcttgtgtgccgccaggctgtaatggtctgatgacggtgctggactggctgaccaatccgtgggaaccgtacaaacgcgggattatgatcggctttgattccagcatggattacgcatggatatatcgttcgatactggaaagcgtggcgctgacgctgaagaacaattacgacaatatgtgtaatgaaatgaatcactttgcgaagcatgtgatcattactggcggcggttcgaacagcgatctgtttatgcagatttttgccgacgtgttcaaccttccggcacgacgtaacgccattaacggttgtgcaagcctgggggcagcgattaatacagcggtaggtctggggctatacccggattacgcaacggctgtcgataacatggttcgcgtgaaagatatctttataccgattgagagcaatgccaaacgctacgacgcgatgaataaaggcattttcaaagacctaaccaaacatactgatgtgatcctgaaaaaatcgtatgaagtgatgcatggggaattggggaatgtggattcgatccagagctggtcgaatgcgtaagtgaggaaggccgggcgggaaactgcccggcctgaacatacctgaatggttatccccgctgacgcggggaacataagttcgacaacttaaaaaatgataacaagtccggtttatccccgctgatgcagggaacataataaaaactttaactagttcggtttatccctgtttttacaaggaatattaactacactcgatgtctttagaataaaagacaatacgaatcgcactttatcaattttcacttaaagtatgaactggatatctttattcataagaactattcatcaacagcgtatagaggcggttatgtaaaaccactcattagcctcaaaacaaagacaaacttccagatttattacttaaccaatgaataacaagcttaaaaaatatactgttattctaaagaaaaaattaacaggcattaattcaatattaaaaaaataatagattaaaatttcttaacgatttaagaatcatacaaataacactttgattaaatttaattttttgtatcgataattgtgaacctctctggcatggagaactattttgaacatgaggtgttacgtggatatgttgcttattacaagtactgctaatataaaaacttgagaaagagataacgggttatatggtggtttatccccgctggcgcggggaactcgacagaacggcctcagtagtctcgtcaggctccggtttatccccgctggcgcggggaacacctgttttcgcaaatctatggactattgctattcggtttatccccgctggcgcggggaacacgggcgcacggaatacaaagccgtgtatctgctcggtttatccccgctggcgcggggaacactggctctgcaacagcagcacccatgaccacgtcggtttatccccgctggcgcggggaacacgaaatgctggtgagcgttaatgccgcaaacacaggtttatccccgctggcgcggggaacacattacgcctttttgcgattgcccggtttttgccggtttatccccgctggcgcggggaacactctaaacataacctattattaattaatgattttttaagccagtcacaatctaccaactttatagtatcacacaaacaacacatccattatgttaaagagcacttaatccattgattaaaaaggtaaatatttaaaataactctatacaaactaaaatctaccaaactttaccgcaataattttcactccagcgaaaaattaatgccacagaatttgtagagaatgctaatgattagccctggatgggtaaaatggaggagttttcagaggcgacaaacaatataaatgagtagaagtctttacaggttccacccatttataacgcttataaatgtttaatcaggcaatatttagatatttatgtgtttgcatcgacaaacgccaattacgcgcaatgcaggtttcaatgcacaaacgtgtggcatcatccttttggctaatcggctgcagtgcaatgactcgcggtttatcatcggtcagcgttgccagtagttcatccagtgcttcaatatcgcgtacgcgccccactggatgcttgatttcgttggctcgctccagtgcctgtgacaacacttcatagccgccgcgcatgttcagctttggcgatacggtaacccaggtattcggtgtgcagcgtacctcatgagtaccactggtttcgatctggcagctaaaaccgttcttttcgagcagatcagtcagtggcagcaaatcatgaatgcaaggctcaccacccgtaatcaccacatgccgcgcggtgtatccctggcgaccaatgacagccagcaaatcttcactgctcgcagccccccacttatcactctctttggtcttcgccagaatgctgaaaagggagacttcccgatcctcaagcttttcccaggtgtgtttggtgtcgcaccaggcacagccaaccgggcatccctgtaaacgaataaaaatggcgggaacgccggtaaagtaaccctcaccttgcagggtctggaacatctcgttaatcgggtactgcatagcattctctgtgaagtggataattgttaattattgcagatcctgccacaacaatcatgtcttattaacattctgttacaggcaggtttaaagaaaaatgcgaaacatatcgttaataattaaagggagtaacgtattatgtcagaagaaaataaagaaaatggatttaatcatgtcaaaacattcaccaaaattatatttattttttctgtattagtttttaatgataacgaatataaaattaccgatgccgccgtcaatttatttatccagatttaatgagaaatttataatgcgctatttcatactaatgttcactttcgtatgttcctttgttgcagcccaaccaactattgtcccacaattacagcaacaagttacggatcttacgagtagcttaaactcacaagaaaagaaagaactgacgcacaagttagaatctattttcaataatacccaagtgcaaattgccgtattaattgttcccacaaccaaagacgagacaattgaacaatatgctacaagagtttttgacaattggcgtttaggagatgccaaacgtaatgatgggatactgatcgttgttgcctggtcggatcgcactgtccgcatccaggtaggttatgggctggaagaaaaggtaaccgatgctctggctggagatatcatccgtagcaacatgatacccgcatttaaacaacaaaaattagctaagggattagagctagctataaacgctttgaataaccaactcacttcacaacaccaatatccgactaatccttcagaaagtgaatcagcgtcttccagtgatcattattactttgctattttttgggtatttgcagtgatgttcttccctttctggttttttcatcaaggcagtaatttttgtcgcgcatgtaaaagtggagtctgtatttcagcaatctatcttttagatttattcctgttctccgataaaattttttccattgctgtattttccttcttttttactttcaccatatttatggtctttacctgtttatgtgtacttcagaaaagagcatctggtagaagttatcattcagacaacagcggttccgctggaggctcagatagcggcggatttagcggcgggggcggttcttctggaggtggcggcgcatccggccgctggtaactcaaccataaaaaatgccagcccggaggctggcatttttaaatcagataaagtcagtcttatgcctggcctttgatctctttacgaccgttgtacggtgctttttcgcccagagcttcttcgatacgaatcagctggttgtatttagcaacacggtcagaacggctcatagaaccagttttgatctggcctgcagcagtaccaacagccaggtcagcgatggtagcgtcttcagtttcgccagaacggtgagagataactgcagtgtagccagcatctttcgccatcttgattgcagccagagtttcggtcagagaaccgatctggttgaatttgatcaggatggagttagcgatacctttttcgataccttctttcaggatcttggtgttggttacgaacaggtcgtcaccaaccagctggattttgtcgcccagaactttggtctggtatgcgaaaccgtcccagtcagattcgtccagaccgtcttcgatagaaacgatcgggtactgtttggtcagttcttccaggaagtgagtgaattcttcagaggtgaacgctttgttgccttcgccagccagaacgtatttaccatctttgtagaattcagaagctgcgcagtccatcgccaaagtgatgtctttgcccagttcataaccagcagctttaacagcttcagcgataacagccagagcttcagcgttggaacccaggttcggcgcatagccaccttcgtcaccaacagcagtgttcatgcctttcgctttcagaacttttgccaggtgatggaaaacttcagaacccatgcggatggcttctttcacagttttcgcgccaaccggctgaatcatgaattcctggatatcaacgttgttgtcagcgtgctcaccaccgttgatgatgttcatcatcggaaccggcatagagtatttgcccggagtaccgttcagttcagcgatgtgctcgtacagcggcatacctttagcagctgcagcagctttggcgttagccagagatacagccaggattgcgttcgcgccgaatttggatttgttttcggtgccgtccaggtcgatcatgatcttgtcaatgccagcctgatctttagcatctttgccaatcagcgcctgagcgatcgggccgtttaccgcagcaacagctttggttacgcctttacccaggaaacgggatttgtcgccatcgcgcagttccagagcttcacgggaaccagtagaagcacctgacggagcagctgccataccgacgaaaccaccctccagatgtacttcggcttcaacagtcgggttaccacgggagtcgatgatttcacgaccgatgatttttacgattttggacattaggttttcctcaagtcactagttaaactgaaactccagacaaacaacgcgtacccagggtacgcgttgccgctctaacttttttacttacttcgcctgacgtttctggaactcgctggcggctttcacaaagcctgcaaacagcgggtgaccatcacgtggagtagaagtaaactccggatggaactggcaagccacgaaccacgggtgattcggaacttcgatgatctcgaccaactgatcatccccggaacggcccgcaacgcgcagacctgcatcttcaatctgtttcaacagcatgttgttgacttcgtaacggtgacgatgacgctcaacaattgtcggcgcattgtacagctggcgaaccaggctatcgtcaaccaactggcactgctgtgcgccgagacgcatggtaccgccgagatcgctcttctcgctacgaacttcaacgttgccgttttcatcgcgccactcggtaatcagcgccacaaccgggtacttacagtctggcacaaattccgtagagttggcgttctccatgttggcaacatggcgagcgtaatcaattaacgccacctgcatacccaggcaaatgcccagataaggaatattgttctcacgcgcaaaacgcgcggtcgtaatcatgccttctacgccacgatagccgaaaccgccaggtacgaggattgcgtccagacctttaaggatttcaacgccgcgcgtttcaacatcttgtgaatcgatcagtttgatgttgacgctgacacgattcttcagcccaccgtgtttcagtgcttcgatcactgatttataagcatccggcagttcaatgtacttgccgaccataccgatggtgacttcacttaccgggttcgcttcttcgaagataacctgttcccattcggacagattcgcttccgggcagtttaagctgaatcgtttacaaatataatcgtccagcccctgagatttcaacaggcccggaattttatagatggaatcgacgtctttcagagaaataaccgctttttccggaacattacagaacaatgcaatcttcgcacgttcgttcgccggaacagcgcgatctgaacgacaaatcaggatgtcaggctggataccgatggagagcagctcttttacagagtgctgagtcggtttggttttgacttcaccagacgctgccatgtacggcaccagcgtcaggtgcataaacagagtgtgctcacggccaatttcaacagccatctggcgaatcgcttcgaggaacggcaaggattcgatatcacctactgtaccgccgatttctaccagtactacgtcatgaccttcgccaccttccagcacgcgctctttgattgcgttagtgatgtgcggaataacctgcacggttgcgccgaggtagtcaccgcggcgttctttacgcagaacgtcagagtagatacgacccgtggtgaagttgttgcggcggctcattttggtacgaatgaaacgctcgtagtgccccaggtccaggtcggtttcagcgccgtcttcagtaacgaacacttccccgtgttggattgggctcatagtacctggatcgacgttgatgtacggatccagtttcatgatggtcacattgaggccacgggcttcaagaatggctgcgagggaggctgcggcaatgcctttacccagagaggatacgaccccgccggtcacaaaaatatagttcgttgtcatgctgaacctgagaagttaggttgaaaagacgatggaataaccaagacgggaaagcagtatacccgaacatgacctgtgccacaaactttcattatccctcctcttcgccagcgcactattgaaatcaggagtgagaaaatagcccctttggggtaaatgtttttgacgcaaatcaagcgcttgtcatttaaaaaatgacacaaatggcgcttgaccgcgtaattcccttagagatcaatttcctgccgttttacctgttgccagacttcttccattgtttcgaggtcaacacctgtcatttccagtccacgcgcggcaacaatacgctccacttcgcgaaaacgacgctcgaatttttcgttcgctttttgcaatgcgatttctgctttcgtccctaaatggcgagccagattaaccgtggcaaacagcaggtcccccatttcctcctccagtttagcctggtcgacaacagcctgccgcgcttcgtacatcacctcgtcgatctcttcgtagactttatcgactaccggaccaagcgtcgtccaatcgaagccaacgttggcgcaacgtttctggattttttgcgcacgcattaaagccggtaaactacgaggaatatcgtccagcgccgaatgctgcgctttctgcgcgcgctcttcggttttgatttgctcccaacgggcaagcacttcactactgttttcggcagaactatcagcaaaaacatgcggatggcgacgctctaatttatcgctaatagcagcgcaaatatcattaaagtcaaagcgcccttcttcctgagccatttgcgcgtaaaacaccacctggaatagcagatcgcccagttcaccgcgaagatcgtcaaaatcttcacgggcgatggcgtccagcacttcgtaggtttcttcaagggtgtaaggcgcaatggtggcaaatgtctgctctttatcccacgggcagccgttttccggatcgcgcaggcgctgcataatagtgagcaaacggtcgatttgattcattgaattgtcctgaaaattgcgggtctgtcaggtggaaacctgtgaccagaatagaagtgagttagtaacactacccaatcagtacgttaattttggctttaatgagttgtaattcctctggggcaactgttcctttcttcgttgctcctcttgcccgccaggcgatactttttacctgatcagctaacgctacgccatcacgttcctgaccggataaaacaacttcgaacggatatccttttgattgcgttgtacaaggaacacacagacacatacctgttttgttgttgtacatgaaaggactcaggacaacagctggacgatgtccagcttgctcgctaccttttgtcgggtcaaaatcaacccaaatcagatcgcccatatcgggtacgtatcggcttaccattaccagacttccttatctttcggctctccccagtcgatattctcgtggaggttttccggcgtgatgtcgttgaccagttcagcaagcgtaaatacgggctctttacgcactggctcaataattaatttgccatccaccaggtcaatcttcacttcatcatcaatattcagattgagcgcctgcattaacgtagccgggatccgcaccgccggtgaatttccccaacgctttacgctactgtggatcataaccctttcctcaaaccgctatcatatgtagatacagtatatatcaatctacattgtagatacgagcaaatttcggcctaactcccgtgcaaccgacgcgcgtcgataacatccggcacctggttgagtttacccagcacgcgccccagcacttgcaggttgtaaatctcaatggtcatgtcgatggtcgccagttgctgtttggtgtcgctacggctggcaacgccaagcacgttcaccttctcgttggcgagaatggtcgtgatatcacgtaacaacccactacgatcattagctaccacgcggaccaccagcgaatatccggcggagtagctctcaccccataccgcgtcaacaatgcgttctggcgcatgggagcgcagttccgccagttgttcgcaatcggcgcggtgtactgaaataccgcgcccctgggtaatgaagccgacaatctcatctccaggaatcggctggcagcagcgcgcgatgtggtgcatcaggttgccaacaccttcgactaccacgcgaccgttatctttactgcggttttgcggcgtgtagcttttttgctgaagttgcttcagcgcggcggcgtcctgctcttcggcactcggcttattaaattgcgattgcaggaagttcaccatctgattgagacggatatccccgccaccaatcgccgccagcaactcgtcgacatcattgaagttgtaacgcggcagcagatgtttttctgcttctttcaggctgatccccagatgttccagctcgtcgtcaaggatttgccgcccagccagaatgtttttgtcacggtcctgtttacggaaccaggcgtgaattttcgaacgcccacggctggttgtgacgtaaccgaggtttgggtttaaccagtcacggctggggttcggctgtttctgggtgataatttcaatctggtcgcccatctgcagctggtaggtgaacggcacaatgcgcccgccaatttttgccccgatgcagcggtgtccgacatcactgtggatgtggtaagcgaagtccagcggcgttgatcccgcaggcaaatcaacgacatcacctttcggcgtaaagacgtacacccggtcgtcaaagacctgactacgtacttcgtcgagcatttcgccggaatcagccatctcttcctgccacgcaatcagtttacgcagccaggcaatccggtcttcatgtcccgaacgtgcgccgccagcagccgcgccctctttatatttccagtgcgcagcaacacccaactctgcatcttcatgcatctgtttggtgcggatttggatctcaacggtttttccacccggccccagaaccacggtatgaatagactgataaccgtttggtttcgggttagcgacgtaatcgtcaaactcatccggcaggtggcgatagtgagtgtgcactatccccagtgcggcatagcaatcctgtaaacgctcggcgacaatacgtaccgcacgcacatcaaacagctcatcaaaggcgaggttctttttctgcattttacgccagatgctgtagatgtgtttcggacgaccatacacttccgctttaacgccttcagctttcatctcagcgcgcagatgaccaacgaactcttcgatgtagtgttcgcggtcgagacgccgttcatgcagcagtttggcaattcgtttgtattcggttggatggaggtaacggaagcagtaatcttccagttcccatttcagttgtccgattccgagacggttagccagcggtgcgtagatgttggtacactcttttgccgccagtacacgttcatcttccggcgcatcttttacttcgcgcagatgagcaatacgctccgccagtttgatgactacgcagcgaaaatcatcgaccatcgccaataacatccggcgaacgttatcgacctgttcggaggaaacagaatcagtgtgcgtcgctttcagctggcggatcgccgccatatcacgcacgccgtgaataaggttaacgaccgacttaccgacgctctcacgcagcacatcttcgctgactacgttggcatccgccagagggaaaagcagcgccgcccgcagcgtgtcaatgtccatacttaatgtcgagaggatctccaccatctcaacaccacgccacaataacagactggcatccggatgcccctgcgtctgttgcagacaatacgcccaggtttcggctaagcactcacacgacttctggctggtaatacccagacttgcgatccatttttccggatcaaattcaccagccttattgatatgtgcacttcttaccgcaaccatcgtcctctcctttagggaccagacctgccgaaatcggcaaatcgcaactatttaacgcgcgagaaaagtaccatcgattccagatgtcccgtgtgtgggaacatatccagcatcgccagtcgcgcaatggtatatcctgcttttaataacgcttcgctatcccgagccagcgttgcagggttacaggatacataaactatacgaataggttccagttttataatttgctgcataacacctgcggcacctgctcgcgccgggtccagcaacactttatcgaagccgtttttcgcccacggctgctttgtgacatcttcttcaagattttcgtgataaaacgtcacattctgtaagccattaagacgcgcattctgctggcctttttccaccagcgccggaacaccttctacaccgaccacactggcagcttgtgtcgccaatggcagtgtaaagttgcccataccgcagaacagatccagtacgcgatcttcaggttgcacatccagccattccaacgcacgcgctaccattttttggttcacacccgcattgacctgaataaaatcgcgcgggctaaaagttaagcgcaacccgtttgagtcataccagggcatctcaccagagacggtttcgagtatctcactatcgggggcgagatacagatccaggccttcagaatgcgaaaagcgttccagtttttcgcgatctgccgaacttagcggtgcggtatggcgcaaaatcatcagcgtgccgctggttgcctgtaccagttcaacatgaccaagatggcgcatagcttgtaagctgcccagacatgccctgactttgggcagcaatgcttcaagttggggcgctaaaatggggcattgtttgacgtcgacaatgtcactggagcccgctttgcgaaaccccatctgaagttgctgtgttttcggtaagtagttcagacttaaacgcgcgcgacggcgatagccccagggaacatcggcgatcacttcagagacatcgtgtttcattaatcgggcgagtgccgcacttttgcttcgctgctgtaaatccacgctggcgtgttgttgctgacagccaccgcatacgccaaaatgaggacagcgtggcgtttcgcgttccgggctatcgcttaaccggcgtacgactttagcgcgggcatactgttttttatcttcagtaacagtaacttccgcgttttcctgcggcaataatccggggataaatagcgttttgccgttatgtcgcgccacgccctgaccaaaagagtcgaggtcgttgactgaaacggttatgatctgacgcgtcgtcgtgcgtcgttttgcagagtagaattgcgccattggcgagactttctcaatttaacagtgtgaccttaattgtcccataacggaactccatgaccaactacagcctgcgcgcacgcatgatgattctgatcctggcaccgaccgtccttattggtttattgctgagtatctttttcgtcgtgcatcgctataacgacttgcagcgtcaactggaagatgccggtgccagcattattgagccgcttgcagtttctactgaatatggcatgagcctgcaaaatcgcgaatctatcggtcagttaataagcgtactgcatcgtcgccattccgatattgttcgcgcgatttcggtttatgatgaaaataaccgactctttgtcacctccaattttcatcttgatccctcatcaatgcagctcggcagcaacgtgccgtttcctcgccagctcactgtcactcgtgacggcgatattatgatcctccgcacgccgattatttctgagagttactcccccgacgaatcgcccagtagcgatgccaaaaatagtcaaaatatgttgggatatattgcgctggagctggatcttaaatcggttcgcttgcagcaatataaagagatctttatttccagcgtgatgatgctgttttgtatcggtattgcgcttatttttggctggcgcttaatgcgcgatgtaaccggtccgattcgcaacatggtgaataccgtcgaccgcatccgtcgcgggcaactcgacagccgggtggaaggatttatgctcggcgagctggatatgctgaaaaacggtatcaactcgatggcaatgtcgctggctgcttatcacgaagagatgcagcacaatatcgaccaggcgacgtccgatctgcgtgaaacgctggagcagatggaaattcagaacgttgagttagatctggcgaaaaagcgcgcccaggaagcggcgcgtattaaatccgagtttctggcaaatatgtcacacgagctgcgtacaccactgaatggtgttattggctttacccgcctgacgctgaaaacagaattaacaccaacgcagcgcgatcacctgaatacgattgaacgttcggcaaataatttgctggcaattattaatgatgttctcgacttctcgaaactggaagcaggtaagctgattctggaaagtattccattcccactacgcagcacgctggatgaagtcgttactctgctggcacattcttctcacgataaagggttagaactgacgctcaatattaaaagcgacgtgcctgataacgtgatcggcgacccgctgcgattacagcaaatcatcactaacctggtggggaatgcaattaaattcaccgagaatggcaacattgatattctggtagaaaaacgtgcgctgagtaataccaaagtgcagattgaagtgcagattcgggataccggcattggtattcctgaacgcgatcaatcgcgcttattccaggccttccgacaggctgatgccagtatttcccgccgtcatggtggcaccgggctggggctggtgattacacaaaaactggttaatgaaatgggcggcgatatttcgttccatagccagccgaatcgcggttcaactttctggttccacattaatctcgatctgaacccgaacattattatcgaagggccatccacccagtgcctcgcaggtaagcgcctggcctatgtcgaaccaaactccgcagcagcgcaatgcacgctggatattttaagtgaaacgccgctggaagtggtttatagcccaacgttctccgcgctgcctcccgcgcattacgacatgatgttgttaggcatcgcggtgaccttccgcgagccgctaacaatgcaacatgagcgattagcgaaagcggtatcgatgaccgatttcctgatgctggcacttccttgccatgcacaagtcaatgctgaaaaactcaagcaagatggtatcggcgcgtgtctgctgaaaccattaacacctacacgcctgttgcctgccctgacggaattttgtcatcacaaacaaaacacgcttttgcctgtaaccgatgaaagtaagctggcaatgacagtcatggcggttgatgacaaccccgctaacctgaaacttatcggcgcattgctggaagatatggtgcaacatgtggaactttgcgatagcgggcatcaggcggttgaacgggcgaaacagatgccgttcgatttgatcttaatggatattcaaatgccggacatggatggcattcgggcctgcgaactcatccaccaactcccgcatcagcaacaaacgccggttatcgcggtaacggcgcatgcaatggccgggcaaaaagagaagctgcttggcgcagggatgagcgattatctggcgaaaccgattgaagaagagcgattgcataatttgttgttgcgctacaagcctggcagcggtatttcctctcgcgtcgtgacgcccgaagtcaacgaaattgtggtgaacccgaatgcgaccctcgactggcaactggcactacgccaggcagcaggaaaaaccgatttagcgcgcgatatgctgcaaatgttactcgatttcctgcctgaagttcgcaacaaagttgaggaacagctggttggagaaaacccggaaggcctggttgatttgattcataaactgcatggcagttgcggctatagcggtgtgccacgtatgaagaatctctgccaactgatcgaacaacagctacgtagcggtactaaagaagaagatttggaaccggagctgctggaactgttggacgagatggataatgtcgcgcgcgaagccagcaaaattctcgggtaatggatgtcttgtcgagtagcaatcggctttttatgacgctggtttcagattggtgacaaagtgcctgtgtttatgccggatgcggcgttaacgccttatccggcctacaaaaccaattaaattcaatgaattaaaaaatgatgtagacctgatacatagcacaacaggctattttgcgtttagcatcagtctcaaaccggctccagatagagccggttttggttttctgtcttaacgcaccatgcacgggcgcttgttatcgaacgtccagccaggaatcagatactgcattcccatcgcatcgtcacgcgcgccaagcccgtgtttctgatacagctcatgggctttcatcacttgatccatatcgatttctacacccagccccggtttttctggcacctgtaccagcccgcctttgatctcaaacggttctttggtcaggcgctgattgccttcctgccaaatccagtgcgtatcaatagcagtaattttacccggtgcagcggcggcaacatgggtaaacatcgccagggaaatatcgaagtggttgttagagtgtgaaccccaggtcaggccaaattcatggcacatttgcgccacacgtaccgaaccttgcattgtccagaaatgcggatccgccagcgggatatcaacggattgcagggagagcgtatggcccatttgccgccagtcggtggcgatcatattggttgcagtcggtagacctgtcgcgcgacggaactctgccatcacttcacgcccggagaaaccttgctccgcaccacacggatcttctgcataagccagcgaacctttcaggtatttaccgattttaatcgcttcgttcagcgaccaggcaccgttaggatcgagcgtaatacgcgcctgcgggaagcgttgcgccagtgccacaatagactcggcctcttcttccccggccagtacaccgcccttcagtttgaaatcgttgaagccatatttttcatatgccgcttccgccaggcgcaccaccgcatccggcgtcatcgcttcttcatgacgcaggcgataccagtcgcatgagtcatccggctggctttgatacggcagcggcgtggctttgcgattaccgacgaagaacagataaccgagcatttcgacttcgctacgctgttgaccatcgcccagcagcgatgccacgtttacccccagatgctgccccagcagatccagcattgccgcttctatcccggtaactacatgaatagtggtacgtaggtcaaatgtctgcaaaccgcgcccaccagcatcacgatcggcaaaagtattacgcaccagcgtcagaacgtttttgtattcacccagcgttttacctaccaccagcggaatcgcatcttccagcgttttacggattttctcgccgccgggaatttcccctacgccagtgtgaccagaattatctttgataatcacaatattacgcgtaaagaacggtgcgtgtgcaccactcagattcatcagcatactgtcatgacccgccaccgggataacctgcatttcagtaacaacaggcgtcgtaaattgagaactcatatttatgtcctttttcagaatcaatgacggccgaaaacgggacgtttacggtcaaaggtccagccggggatcaggtactgcatcggacctgcgtcgttacgcgcaccgccaggcagacgtttataggcctcatgtgccttttgtacctgttcccagtccagttccacgcccagaccgggcgcatcaggaacggcaatttttccgtttttaatctccagcggattttgggtcaggcgacaatcgccctcctgccaaatccagtgggtatcgatagcggtaggattacccggtgccgccgcgcccacatgggtaaacatcgccagagagatatcgaaatggttattagaatggcagccccaggtcagcccccagtcgtcgcaaagctgcgccacacggactgcaccggaaagcgtccagaagtgcggatcggcaagtggaatatctaccgcattgagcatcaccgcatgacccatttcgcgccagttggtggcgatcatgttagtcgcgacgggcaagccggtcgcccgtcgaaattccgccatcacttcacgtccggagaagccctgttctgcgccgcatggatcttcggcataggtaagaacatcattcagccctttgcataaagaaatggcttcatcaagcagccatgcaccgttgggatcaacggtaatccgcgcatccgggaagcgtttcttcaatgcacgaacagtgtcgatttcttgctcgccaggtaacacgccgcccttaagtttgaaatctttaaagccgtagcgatcctgtgaggcttccgccagacgcacaacggcttcgctgttcattgctttctgatgccgcaactgataccactcatggttgcccggcgtattttccacataaggaagatcggttttggtccgatcaccgatataaaacagataaccgaggacggtaatagcctcgcgttgcttgcctggccctaacagttcgcagaccggaacattcagcgccttacctagcaggtcaagcaaagcggcttccagcgccgccacggcgttaacgcgtaattcaaaggtccaggcacctttaccgaaggtatcaaaatcggcggcctgattacctttatgcacctgctggaccactttattcagtcgcgcaacttcctggcccagaaccatcggaatagcatcgacaagcgtctgataaatcacatctccgcccggcgcttcaccaatgccggtatgcccggcgttatcggtgagtaccacaatattgcgggtgaaatatgcgttatgtgccccaccaatattaagcaacatgctgtcatgcccggccaccggaatgactttcatatcagtaataacaggactggattgtgtcgccatcttattgccccgcaacaggtttcaactcgatacgcttgatatcgcccaccagcaccaggtagctcagtaccgcgattaaggcatgaacaccaacataaatcagcgccccattaaacgagccagtcgtgccaacgatataaccaattgcgattggcgtgacgatgccagaaatgttaccgaacatgttgaacaggccaccggaaagaccgctgatctcttttggcgcggtatctgccattactgcccaacccagcgccccgatgcccttaccgaagaaggccagcgccataaagccgatgatcatccactcaacgttgacgtagttgcagaacaccatcaccatcgacagcaacatgcccattacgatcggtgttttacgcgcaatgttcagcgatcccgtgcggcgcatcagccagtcggaaataatcccacccagcacaccgccgataaaaccgcaaaccgccggaacggaagccacaaagcccgctttcagaatcgacatcccgcgtgcctgcaccagataaaccgggaaccaggtaataaagaagtaagtcagggcgttgatacagtactgaccgatataaacgccgatcatcatccgtgaccctagcagctgtttgatctgcccccacttcacgctgaacggcactttaactttggtgttttgctgatccatattgatcagcgcaccacccgcggcgatgtactccagctctttcttatttacccccggatgttgatttggctcgtggatgactttcaaccagataaagctgatgacaatccccagaccgcccataaagaagaagacgtgtgaccagcccacttcatgcgtcagccagcccataatcggcgcgaagatcaccgttgcgaagtattgagcggagttaaaaatcgacaccgccgttcccctttcctgcgccggaaaccaggccgcaacaatgcgactgttgccggggaaagatggcgcttcagcaagcccgaccaggaagcgcagcgtaaacagggcaacgataatgccgaatccactaaagatatcgacgaagccttgcagcaaggtaaacatcgaccagataaagatcgaccagaagtagacgcgttttgaaccaaaacggtccagcaaccagccaccagggatctgcccgataacataagcccatgagaaagcagagaacacatagcccattcccacgggatcaaggccgatatctttggccatttccgaaccggcgatagagagcgtagcgcggtcgccgtagttgaaggatgtgacgataaacaacatcaccactatccagtaacgagcatttgtgcgtttttccacactgctcgcagcctgacttaaagaactcattgttgcactcctgaaaattcgcgttagccacgctcactctggactgcgacatcgccaggaaatcagaggtgacgtagggtgttttttgccgtttttataggtcgttcgccgaatacggcgcgtgtttatatctggcaatagcagtataaaaagcgcgccatagcggctcaccgtgcaacaacacaacattaatgcgttcaatgaggcccgattttggcattagccctggacggtggaatccacttcacggaaatgaaaacaagaacaagaaaggaagggttaaaacgaagaaataaagaagagtatgaaatggatcgcttgactccaggcaaacgccagtaaaaatccgcgctatgaagcagtttttactggcatttgcctgaaaagattcgattcagcaccgctaaaacgacatttaccgctcgctgaacatatcaggacaacagcgtgccccactgttcgacccacggatttgattccgtttccggttccgggttctcactggcgtcaatcaacagcatttcgccaacccgctgagcgctctgttcctgcaacaaggcatcgaactgtttgccgccattgcagaaattcacataactactgtcgccgagcgcaatcacgccataacgcagattcggctggaagcccagactatctttgattccctgaaagagtggcacaatgctatcaggaaggtcgccctgcccggtcgtggacgtaaccaccagaacatacttatcctgatagggcagccagtcgcttaattcaggatcttcaaataccgttgctttgtggccctgcgcggtcagaatcgcttccgcttcttcggccactaacagtgaattcccgtacatggtgccgacaaaaataccaatttccgccataccgttttctccctggattaggaacttatctctccatcctgacccgatggcgcactgaactcaaccctttcattttcaggaagcagaccgcgccagccaaattgtgataacgcctgcatccaggtgtcgtccaggcccgcgtgaatagtcagcggctcgccagtaaaaggatgcgtcaatgacaactgactggcatgtagcattaaccgctggaggccaaaatgctcagcaccgctgcgattctggcgtaaatcgccatgtttgctatcgccaataatcggatgacgcaaatgggcaagatgtcggcgaagctgatgtttgcgtccggttttcggctccagttccaccaggccgtagcgcgtggtcgggtaacgtccggtcgctaccggcatttctacggtcgccagaccgcgataatgcgtcactgctggctgcgggcctttatcttcgcgggcaaatttatcagcgattttgtccagttcttccaccagtggataatccagcaccgcttcttccatcaaccagccgcgcacaatcgcatggtaacgtttctggatttggtgctgttcaaactgttgtgccagcagccgtccggcctcgctggataatcccatcaacaacacaccagaagtgggtcggtccagacgatgagcagtaaaaacatgctggcctatctggtcacgcacggtttgcatgaccactactttctcgtcgcgatccagccagctgcggtgaaccagccagccggagggtttatttaccgcaaccagccattcatcctgatagagtatttccagcattagctcgcatcatccgcaaaaagagcatccagtttttccagctcagccagaataagcgcgcgttgcggatggtccgtcgccagcgccatttcataatagggtgcaacggcaaaagcgcccggtaacggctgtttgttatctaacaaatcgtgcattcgcgggatcagcacccactgcaaccactccagtggttccatggtgtccataaagaacggttgggtactattaaattgatgcggctggggttcatcgtttcgccagtgctgatgttcacgcagtaacgcttcaagcgcctgcaactggagacgaacgcggtcatgagtggtcataaagcaacctcaataagaaaaactgccgcgaaggatagcaggaataaaaaaagggagcactgtattcacagcgctcccggttcgtttcgcagcattccagctacttttgttgctccctgctcatccttgacaacttttcctctggccttgcggccaatcgttcatcctgaactattgcttcctgctcacaccaccccgatgtgatacttcatcctgaagtgtccctggccttcctgacccaccgaatcatcctgaccggttctcattctccatcctggaggtgtcctttaacgcgtcctgcgtcatcctcttcgcttcatccagaagcctttccctgaaacaccatcctggtgtgtcctgcagaagtgtcatcatcctgatgttcacttcgttgtctgactccctgtcgacgaagatagaatcgtctttttcgcgaagtcttacaaggcgcttacagacaatgccttaaggaaaatttcatatgaaagttaagaattaacaatcaacattttgattttaaatgaaaataacgattcttatctttttaagtattcgcttatttcctggcgatctcctacagagtctgtaagagatctctcacaaccagatggggtatttggattacagaagaggcttaagttgattaaggaattccgcaagatttgaggctaaatgcgtccgtttacgtgttcccagcgtctctttgcacacttcaccggagagattacacaccgagatgacctctaactcttcttccagcgtcgcgataaatagtgtgggcggcagttttagccttttctgagtcaccagatgaccaatcagattttcctgcacccgacggaagtcgtcttcactccaggtttgcagcaatgtcagtttgatatcgccaaactgcgcgtgcatatccccggcaaactgagtcgtataaaaggtatgaattgtgggttgtatcacaatatcaaaagcgcgttcaaccgcgtttacattttgttccccggtaaacggctggggttgccagtatacggcatcttcggtagttgaaataatgcacggtgaaggaacaccgtacagttcctcacttaacggccagcttttatgctcttcatgccacgcatcgcagtagcgtgcagtaaaatctttcagggcttgtgcggtcaaatcgtccactaatttctctcttcacttaaaccagatacacttgtcgtttagtttatctggtttatgacggtgaaacatgtcttcttatgcaaaccatcaggcacttgcgggcctgactcttggaaaatcaaccgattaccgggatacctatgacgccagcctactgcaaggcgttccacgcagcctgaatcgcgacccgctgggtctgaaagcggataacctgccttttcacggtacggatatctggacgctgtatgaactttcctggctgaatgcgaaaggtttgccgcaggtcgctgtcggtcatgttgaacttgattacaccagcgtaaatctgattgagtcgaagagttttaagctctatctcaacagttttaaccagacgcgttttaataactgggatgaggtgcgccagacgctggagcgcgacttaagcacttgcgctcagggtaagattagcgtggcgttatatcgtcttgatgaactggaaggccagccgataggtcattttaatggcacttgcattgatgaccaggatatcactatcgataactatgaattcactactgactatctggagaatgccacctgtggtgaaaaagtagtggaagagacgcttgtcagccacctgctgaaatcaaactgcctgatcacccatcaaccagattggggttcgctccaaattcagtatcgtggacgccaaattgacagagaaaaactgctgcgttacctggtctcattccgtcatcacaacgagttccacgaacagtgcgtggaacgcatctttaatgacctgttacgcttctgccagccagaaaaattgagcgtttacgcacgttatacccgtcgtggcggtctggacattaacccgtggcgcagtaatagcgattttgtcccatcgaccacaagactggttcggcaataaattttttctcaattttgcgtgctggattcacgcagaaggttgtgaaaggtcatcaggcagggctattgtaatcaaagggaatgacgatattcgtcccataaggagtttttcttgattacacatattagcccgcttggctccatggatatgttgtcgcagctggaagtggatatgcttaaacgcaccgccagcagcgacctctatcaactgtttcgcaactgttcacttgccgtactgaactccggtagtttgaccgataacagcaaagaattgctgtctcgttttgaaaatttcgatattaacgtcttgcgccgtgaacgcggcgtaaagctggaactgattaatcccccggaagaggcttttgtcgatgggcgaattattcgcgctttgcaggccaacttgttcgcggtcctgcgtgacattctcttcgtttacgggcaaatccataacaccgttcgttttcccaacctgaatctcgacaactccgtccacatcactaacctggtcttttccatcttgcgtaacgctcgcgcgctgcatgtgggtgaagcgccaaatatggtggtctgctggggcggtcactcaattaacgaaaacgagtatttgtatgcccgtcgcgtcggaaaccagctgggcctgcgtgagctgaatatctgcaccggctgtggtccgggagcgatggaagcgccgatgaaaggtgctgcggtcggacacgcgcagcagcgttacaaagacagtcgttttattggtatgacagagccgtcgattatcgccgctgaaccgcctaacccgctggtcaacgaattgatcatcatgccagatatcgaaaaacgtctggaagcgtttgtccgtatcgctcacggtatcattatcttccctggcggtgtgggtacggcagaagagttgctctatttgctgggaattttaatgaacccggccaacaaagatcaggttttaccattgatcctcaccggcccgaaagagagcgccgactacttccgcgtactggacgagtttgtcgtgcatacgctgggtgaaaacgcgcgccgccattaccgcatcatcattgatgacgccgctgaagtcgctcgtcagatgaaaaaatcgatgccgctggtgaaagaaaatcgccgtgatacaggcgatgcctacagctttaactggtcaatgcgcattgcgccagatttgcaaatgccgtttgagccgtctcacgagaatatggctaatctgaagctttacccggatcaacctgttgaagtgctggctgccgacctgcgccgtgcgttctccggtattgtggcgggtaacgtaaaagaagtcggtattcgcgccattgaagagtttggtccttacaaaatcaacggcgataaagagattatgcgtcgtatggacgacctgctacagggttttgttgcccagcatcgtatgaagttgccaggctcagcctacatcccttgctacgaaatctgcacgtaatctccgctcccccggtgacgtttgttgccgggttttctcgtttttggtcacttactcatcaactcatttcatttgttatatgaatgtttcttaccaccctcacgcgacaaatatcatcacagttaatatgtcatacaatttatgttgcaacgcaaacgtttccctattttcataaaccgtattttatcgctatgaaaaagaaattatcgccatgattaactaaaagtattgattttttcagttcaacctacatatattgcgcgccccggaagaagtcagatgtcgtttaatgggcaaatattgcccttaaattctcttttacttttgatttacagagtaaagcgttgggataatctatcttccaagtagattattgtatttgagatcaagatcactgatagatacataacttgtgtgtatctttccgccctcaaattattacggcggtaaatgattaagccatcgccgatagacagatttcatttttacggtcaggcaccttcccgggctgaactggctaaaagctgaattatttgcattcctccaggagaaatagatggaaacgactcaaaccagcacgattgcgtcgaaagactctcgtagtgcctggcgcaagacagacaccatgtggatgctgggcctttacggcacggcaatcggcgcgggcgtgctgttcctgccaatcaacgccggtgttggcggtatgatcccgctgatcatcatggctatccttgcgttcccgatgacgttttttgctcaccgcggcctgactcgcttcgtactgtctggtaaaaacccgggcgaagacatcaccgaggttgtagaagaacactttggtattggcgcaggtaaactgattaccctgctctacttcttcgctatctacccgatcctgctggtttatagcgtggcaatcaccaataccgttgaaagcttcatgtctcaccagctgggtatgacgccaccgccgcgtgcgattctgtcgctgatcctgatcgtgggtatgatgaccatcgttcgcttcggtgagcagatgatcgttaaagcgatgagtattctggtattcccgtttgttggcgtactgatgctgctggctctgtacctgatcccgcagtggaacggcgctgcactggaaacgctgtctctggacactgcatctgcaaccggaaacggtctgtggatgaccctgtggctggcaattccggtaatggtgttctcgttcaaccactctccgatcatctcttctttcgccgttgcgaagcgtgaagagtacggcgatatggcagaacagaaatgctcgaagatcctggcattcgcacacatcatgatggtgctgaccgtaatgttcttcgtcttcagctgtgtactgagcctgactccggcagacctggctgcggctaaagagcagaacatctcgattctgtcttacctggctaaccactttaacgcaccggttatcgcgtggatggctccgattatcgcgattatcgctatcaccaaatccttcctcggtcactacctgggcgcacgtgaaggcttcaacggtatggtgattaaatctctgcgtggtaaaggtaagtctatcgaaatcaacaagctgaaccgtatcactgcgctgttcatgctggtaacgacctggattgttgccaccctgaacccgagcatcctgggtatgattgaaaccctgggcggtccaatcatcgcgatgatcctgttcctgatgccgatgtacgcaattcagaaagtaccggcaatgcgtaagtacagcggtcacatcagcaacgtattcgttgtcgtgatgggtctgattgcaatctccgcaatcttctactctctgttcagctaagtcctttcgcgccgctttcgggcggcgcttcctccgttttaacgcgatgtatttcctatgattagcgtattcgatattttcaaaatcggcattggcccttccagttctcataccgttggaccaatgaaagcgggtaaacaatttaccgacgatctgattgcccgtaacctgcttaaagacgtgacccgcgtggtggttgacgtgtacggctcgctctctctgaccggtaaaggccaccacactgatatcgccattattatgggcctggcgggtaacctgccggataccgtggatatcgattccatccccagttttattcaggatgtgaatactcatggtcgcctgatgctggcaaacggtcagcatgaagtggagttcccggttgatcagtgcatgaacttccacgccgacaacctttctctgcatgaaaacggtatgcgcattaccgcgctggcgggcgataaagtcgtttacagccagacttactactctattggcggtggctttatcgttgatgaagagcattttggccagcaggatagcgcaccggttgaagttccttatccgtacagttcagcagccgatctgcaaaaacattgtcaggaaaccgggctgtcactctctggcctgatgatgaaaaacgagctggcgctgcacagcaaagaagagctggaacagcacctggcgaacgtctgggaagtcatgcgcggcggtattgagcgcggtatttccaccgaaggcgtgttgcctggcaaactgcgcgttccacgccgtgctgcggcactacgccggatgctggtcagccaggataaaaccaccactgacccgatggcggttgttgactggatcaacatgtttgcactggcagtgaacgaagagaacgctgctggcggtcgcgtggtgactgcgccgactaacggtgcgtgcgggattatcccggcagttctggcgtactacgacaagtttatccgcgaagtgaacgctaactcactggctcgttacctgctggtagccagcgccattggttctctttataagatgaacgcgtcgatttctggtgctgaagtgggttgccagggtgaagttggcgtggcgtgctcaatggcggcggctggtctggcagaactattaggcgcaagcccggcgcaggtgtgcatcgcggcggaaatcgccatggagcacaacctcggtctgacgtgtgacccggtcgccggacaggtacaggtgccatgcatcgagcgtaacgccattgcggcagtaaaagcggtgaacgccgcacgtatggcgctgcgccgtaccagcgagccgcgcgtctgcctcgataaagttatcgaaaccatgtacgaaacaggtaaagatatgaacgccaagtaccgcgaaacctctcgcggcggcctggcaatgaagatcgttgcctgcgattaatcgctctccaaaggcctcgttttgcgaggcctcttcccgatttctcatccagccgtagcctgttccggcatcgaatgttacccttatcgcctgatctttaagggggttatcgtggctgttcatttgcttattgtcgatgcactgaatcttattcgtcgcattcatgccgttcaggggtcgccctgtgtcgaaacctgccagcatgcgctcgatcagctcattatgcacagccagccaacccacgcggtcgccgtttttgatgatgaaaaccgcagtagcggctggcgtcatcagcgtttaccagattacaaagcgggtcgaccgccaatgccggaagagttgcacgacgagatgcctgcattacgcgccgcctttgagcaacgcggcgtcccgtgctggtcaaccagcggcaacgaagccgatgacttagccgccacgctggcggtcaaagtgacacaggccgggcatcaggcaacgattgtttcgacagataaaggctactgtcagttactttcaccgacattacgtattcgtgattacttccagaaacgttggctggatgcgccatttatcgataaagaatttggcgttcaaccgcagcagttgcccgattactggggacttgcggggatcagcagttcaaaggtaccgggtgttgcgggaatcggaccaaaaagcgccacgcagctgctggtcgagtttcagagtctggaagggatatatgagaatctggatgcggttgccgaaaagtggcgcaaaaaattagaaacccataaagagatggcgtttctgtgccgcgatattgcccgcttacaaaccgatttgcatatcgacggcaatttacagcaattgcggttggtacggtaacggcgagccggatacgccgcaaacgtcgtatccggcattatcacatcagcgcatttaccaggcggtatggtaaagctctacaatatcctcaagcgttgcttcacgcgggttgccaccggtacaaacatcatccagtgccgcctgcgccagtgccggaatgtcttccttgcgtacaccaacatcacgcaaatgtggcggaataccgacatcacggttgagagcaaacaccgcttcaacagcggcattacgcgcctcttccaggctcataccttccactttcacgcccataacgcgcgcgatatcgcggtacttctcaccggtaaagtcagcgttataacgcatgacatgcggtaacaggatggcgttcgcaacaccgtgtggagtgttataaaacgcgcccagtggatgcgccataccatgcaccaaccctaacccaacattcgagaagcccatacccgcaacatactgcccgagcgccatttcttctccggcatccttatcaccagcaaccgatcctcgcagcgccccagcaatgatttcaatcgctttaatgtgcagtgcatcggttagcgcccacgcgccacgggtaatatacccctcaatagcatgagtgagcgcatcgacacccgtcgcagctttcagcgctggaggcataccatccatcatgtcagcgtcaataaacgccacctgcgggatatcatgcggatcaacgcaaacaaacttgcgccgtttctcttcgtcagtgatcacgtagttaatggtcacttctgccgcagtacctgctgtggtaggaattgccagaatcggtacactgggtttattggtcggggaaagcccttccaggctacgcacatcggcaaactccgggttgttgctgataatgccaatcgctttacaagtatcctgtggagaaccaccaccaatagcgatcaggtaatccgcgccgctattctggaatacaccgagcccttctttgacgacagtaattgttgggttgggcactacgccgtcgtaaatcgcccatgccagccctgcagcatccatcttatcggtcactttcgccaccacgccgcattgcaccagcgttttatcggtgacgatcagcgccttctgataaccacggcgtttcacctcatcggttaaagccccaacagcaccccgaccaaaccatgccgtttcgttcagaatcattctgttagccatcatccttctccttgttgctttacgaaattactcttcaattcgtaacccataggttttgaatttctccagcactacggcaatctcttcatcgctcagcactggcaccgggtccgtaatcgccagggtcgtcaggtaaagttgcgccagcacttcaacttcatgcgccagccataacgctttttccagattcacctcacaagcgataagcccatgatgttgtaacaaagttgccttacgatttttgagagccagcgcaacatgttcagaaagttcgcgtgttccaaaggtcgcataaggcgcgcaaggaatagaattaccgccagccgccgcaatcatgtagtgaatagcggggatcgatcggttaagaatggaaactgccgtgcaatgaacggcatgattgtgaacaaccgcgttggcatccggtctgctttgataggctgccatatggaaacgccattcgcttgaggggagctttccttcctcatgtttaccgttgccatcaataaagacaatatgcgactccgtcagtttttcatatggaatgcctgtaggcgtaatcagcatcccatcctgataacgtacactgacgttccccgctgtcccctggttcagtcccaggcgggtcatttccaggcaagtgtcaataatctgacgagcaagtttatttcgttccattagctacctctctctgattcaaaacagggcaataatgttgttcctttcacactattgaattagccgtttaattacccaccatcttcttcctgattaacaagaaagaaattcacaagcttatattttgtgacctggttcaactaatcacagtaaataactgcaagttctctttttataaccccattaaaaatgaccgctcttaaaaatatttatcaaaacggtcatttttctattcctccaagcccggaatgaccgttttcggcacaaacaattaatacggtcatctgatttgtgttttttatgatttattttctgaaacgggcatgaaatttcgattattaaagtgatggtagtcacataaagtcaccttctagctaataagtgtgaccgccgtcatattacagagcgttttttatttgaaaatgaatccatgagttcatttcagacaggcaaatattcactgatatgaagcccgaactcgctggttttgcacttttgaaaacataaccgattacgtgcttaagcttctgaacctaagaggatgctatgggaaacacatcaatacaaacgcagagttaccgtgcggtagataaagatgcagggcaaagcagaagttacattattccattcgcgctgctgtgctcactgttttttctttgggcggtagccaataaccttaacgacattttattacctcaattccagcaggcttttacgctgacaaatttccaggctggcctgatccaatcggccttttactttggttatttcattatcccaatccctgctgggatattgatgaaaaaactcagttataaagcagggattattaccgggttatttttatatgccttgggtgctgcattattctggcccgccgcagaaataatgaactacaccttgtttttagttggcctatttattattgcagccggattaggttgtctggaaactgccgcaaacccttttgttacggtattagggccggaaagtagtggtcacttccgcttaaatcttgcgcaaacatttaactcgtttggcgcaattatcgcggttgtctttgggcaaagtcttattttgtctaacgtgccacatcaatcgcaagacgttctcgataaaatgtctccagagcaattgagtgcgtataaacacagcctggtattatcggtacagacaccttatatgatcatcgtggctatcgtgttactggtcgccctgctgatcatgctgacgaaattcccggcattgcagagtgataatcacagtgacgccaaacaaggatcgttctccgcatcgctttctcgcctggcgcgtattcgccactggcgctgggcggtattagcgcaattctgctatgtcggcgcacaaacggcctgctggagctatttgattcgctacgctgtagaagaaattccaggtatgactgcaggctttgccgctaactatttaaccggaaccatggtgtgcttctttattggtcgtttcaccggtacctggctcatcagtcgcttcgcaccacacaaagtcctggccgcctacgcattaatcgctatggcactgtgcctgatctcagccttcgctggcggtcatgtgggcttaatagccctgactttatgcagcgcctttatgtcgattcagtacccaacaatcttctcgctgggcattaagaatctcggccaggacaccaaatatggttcgtccttcatcgttatgaccattattggcggcggtattgtcactccggtcatgggttttgtcagtgacgcggcgggcaacatccccactgctgaactgatccccgcactctgcttcgcggtcatctttatctttgcccgtttccgttctcaaacggcaactaactgaacatattttccgaataaagtgaggaatctgtaatgaaaaaaatcagcttaccgaaaattggtatccgcccggttattgacggtcgtcgcatgggtgttcgtgagtcgcttgaagaacaaacaatgaatatggcgaaagctacggccgcactgctgaccgagaaactgcgccatgcctgcggagctgccgtcgagtgtgtcatttccgatacctgtatcgcgggtatggctgaagccgctgcttgcgaagaaaaattcagcagtcagaatgtaggcctcaccattacggtaacgccttgctggtgctatggcagtgaaaccatcgacatggatccaacccgcccgaaggccatttggggctttaacggcactgaacgccccggcgctgtttacctggcagcggctctggcagctcacagccagaaaggcatcccagcattctccatttacggtcatgacgttcaggatgccgatgacacatcgattcctgccgatgttgaagaaaaactgctgcgctttgcccgcgccggtttggccgtcgccagcatgaaaggtaaaagctatctgtcgctgggcggcgtttcgatgggtatcgccggttccattgttgatcacaacttctttgaatcctggctgggaatgaaagtccaggcggtggatatgaccgaactgcgtcgccgtatcgatcagaagatttacgacgaagccgaattggaaatggcactggcctgggctgataaaaacttccgctatggcgaagatgaaaataacaaacagtatcaacgtaatgccgagcaaagccgcgcagttctgcgcgaaagtttactgatggcgatgtgtatccgcgacatgatgcaaggcaacagcaaactggccgatattggtcgcgtggaagaatcacttggctacaacgccatcgctgcgggcttccaggggcaacgtcactggaccgatcaatatcccaatggtgacaccgccgaagcgatcctcaacagttcatttgactggaatggcgtgcgcgaaccctttgtcgtggcgaccgaaaacgacagtcttaacggcgtggcaatgctaatgggtcaccagctcaccggcaccgctcaggtatttgccgatgtgcgtacctactggtcaccagaagcaattgagcgtgtaacggggcataaactggatggactggcagaacacggcatcatccatttgatcaactccggttctgctgcgctggacggttcctgtaaacaacgcgacagcgaaggtaacccgacgatgaagccacactgggaaatctctcagcaagaggctgacgcttgcctcgccgctaccgaatggtgcccggcgatccacgaatacttccgtggcggcggttactcttcccgcttccttaccgaaggcggcgtcccgttcaccatgactcgtgtcaacatcatcaaaggcctgggaccggtactgcaaatcgcggaaggctggagcgtggaattgccgaaggatgtgcatgacatcctcaacaaacgcaccaactcaacctggccaaccacctggtttgcaccgcgcctcaccggtaaagggccgtttacggatgtgtactcggtaatggcgaactggggcgctaaccatggggttctgaccatcggccacgttggcgcagactttatcactctcgcctccatgctgcgtatcccggtatgtatgcacaacgttgaagagaccaaagtgtatcgtccttctgcctgggctgcgcacggcatggatattgaaggccaggattaccgcgcttgccagaactacggtccgttgtacaagcgttaatacattactccctgatgtgatgcccggtcgctccggctaccgggcctgaacaagcaagagtggttagccggataagcaatgttatccggctatattgcaggagcgattatgaaacaagaagttatcctggtactcgactgtggcgcgaccaatgtcagggccatcgcggttaatcggcagggcaaaattgttgcccgcgcctcaacgcctaatgccagcgatatcgcgatggaaaacaacacctggcaccagtggtctttagacgccattttgcaacgctttgctgattgctgtcggcaaatcaatagtgaactgactgaatgccacatccgcggtatcgccgtcaccacctttggtgtggatggcgctctggtagataagcaaggcaatctgctctatccgattattagctggaaatgtccgcgaacagcagcggttatggacaatattgaacggttaatctccgcacagcggttgcaggctatttctggcgtcggagcctttagtttcaatacgttatataagttggtgtggttgaaagaaaatcatccacaactgctggaacgcgcgcacgcctggctctttatttcgtcgctgattaaccaccgtttaaccggcgaattcactactgatatcacgatggccggaaccagccagatgctggatatccagcaacgcgatttcagtccgcaaattttacaagccaccggtattccacgccgactcttccctcgtctggtggaagcgggtgaacagattggtacgctacagaacagcgccgcagcaatgctcggcttacccgttggcataccggtgatttccgcaggtcacgatacccagttcgccctttttggcgctggtgctgaacaaaatgaacccgtgctctcttccggtacatgggaaattttaatggttcgcagcgcccaggttgatacttcgctgttaagtcagtacgccggttccacctgcgaactggatagccaggcagggttgtataacccaggtatgcaatggctggcatccggcgtgctggaatgggtgagaaaactgttctggacggctgaaacaccctggcaaatgttgattgaagaagctcgtctgatcgcgcctggcgcggatggcgtaaaaatgcagtgtgatttattgtcgtgtcagaacgctggctggcaaggagtgacgcttaataccacgcgggggcatttctatcgcgcggcgctggaagggttaactgcgcaattacagcgcaatctacagatgctggaaaaaatcgggcactttaaggcctctgaattattgttagtcggtggaggaagtcgcaacacattgtggaatcagattaaagccaatatgcttgatattccggtaaaagttctcgacgacgccgaaacgaccgtcgcaggagctgcgctgttcggttggtatggcgtaggggaatttaacagcccggaagaagcccgcgcacagattcattatcagtaccgttatttctacccgcaaactgaacctgaatttatagaggaagtgtgaaatgctgaaaacaatttcgccgttaatttctcccgaactattgaaagtgctggcagagatgggacatggagatgaaattattttttccgatgctcactttcccgcccattcgatgggaccgcaggtgatccgcgctgatggcctgttggtgagcgacttgctccaggcgattatcccgttatttgaactggacagttatgcaccgccgctggtgatgatggcggcggtagaaggtgacactctcgatcctgaagtagaacgacgttaccgtaatgcgctttcactacaagccccgtgtcctgacatcatccgcatcaatcgttttgcgttttatgaacgggcgcaaaaagcctttgcgatcgttatcacaggcgaacgagcgaagtacgggaatattcttttaaaaaaaggggtaacaccgtaatctcataccggtacgcccgcatgacgcgggcggttatcgaatgatggggtgaaaaatatgaaagcggcacgccagcaagcgatagtcgacctgctgctgaaccataccagcctgaccacggaagctctctctgaacagctaaaggtcagtaaagaaaccattcgtcgcgatctcaatgaattacagacgcagggtaaaattctgcgcaatcatggacgcgctaaatatatccaccgtcaaaatcaagacagtggcgatccctttcacatcaggctgaaaagccattatgcgcataaagcagatatcgcgcgcgaggcgctcgcgtggattgaagaagggatggtgatagccttagacgccagttcaacttgctggtatctggcacgccagttgcctgacatcaacattcaggtcttcaccaatagccatccgatttgccatgaactcggtaaacgcgaacgcattcaactgatcagttccggcggcacacttgagcgcaaatatggctgttacgtcaatccctcgctgatttcccaacttaaatcgctggaaatcgatctgtttattttttcttgtgaagggatcgatagcagcggcgcactgtgggactccaatgcgatcaacgctgattacaaatcgatgctattaaaacgtgccgcgcaatcgttgttattgattgataaaagtaaatttaatcgttcaggggaagcccgcatcgggcatctggatgaggtaacgcacattatttctgatgagcgccaggttgcaacttctttggtaacagcctgacggaaagggtagcaggccggagacgacgccccggccttgcctgttatcgctcgtcgcgacgaccacccaccgcagcccagatgcggcggacgtgcaccgtcacttcttcgcgatcgtgatacaactgccgcgcctgaatctgagcatttatgccatgttcatcaagctgtgcctgaatatacgccagattgtgtgacacttcttcgtagcgttttttcatcggcagtttgaggttgaaaatggtttcacggcaccagccattaaccagccactgcgccatcaatgccgcaactttcgccggtttttcaaccatatcgcataccatccaggagatattgctgcgcgtcggacggaatttgaaaccgtcttcccgcagccacgtcacctgtccggtatccatcagactttgcgccatcgggccgttgtcgacggaataaacccacatgttgcgcttcaccagttggtaggtccagccgccagggcaagcgcctaaatccaccgcccacatcccgttcgccaggcgttcatcccactcatccgcaggaataaacacatgaaatgcctcttccagtttgagcgtggaacgactcggcgcatctgccggaaatttcaggcgcggaatgcccatatagaacggcgaattattgttgctgtatgagtaaccggtatagcagcagcctggtgcaataaagaatacatgcacaaccggacgcttcggcgtttcatagttcgccagcaccccggcatcgcgcaaggcagcgcgtagcggaacagtaaatttacggcagaatttcagtaactctttgctttcgttggtatcggcaacttcaacacgcagttcaccgcccttctctactacgccctgtaacatgccgacaatgggggtaatacgatcttctggcggcaaatgctgcaggagttcccccaccacaaaccactggcgggcaaaaattaatgaactgaacggcagctcacggattaacttatcgccatcatcaggttgataacattcataaatgacataacccgcattctctttcacgcgggcaaaaccgaaaatttcccgctggccggctttatcggtaatttctgcggcgcactctttttcaaagcccggacggcacagcaatacaaccttattcatgacttacgcccttgcgctttaaacggatagcaccaactaacattaacgcccagcccgcgaggaagctcacgccgccaaccggagtgacaaacgcccacaaacgcagatgggacagcgccaggcaataaaggctgccgctgaacaacaccgtgcctaacgcgaggaaaacgctactccagtaaaaccagatactgatgcgacgctgcattgccaccgccagacctaagatcgccagcgtatgaaacgcctggtattcgaggccggtctggatccagcccatctcaacggcccccatggttttacttaacacatgcgcgccaaaagcgcccagagccacaaaaatgaagccgctaatggcggcgaaaatcagcataaaacggctggtcatggtcgtaccctacgtaaattattgttcataacgaaagcggaatttttcttgttcagcagcggctttcgccaggatccattggcgaaaggcggctattttacccagttctgcctgactgtcatgacaaaccagataaaaagcatttttactgaccagaacatcattaaacgggcaaacaagacgtccggcctcgatttcagattgcgccatcacgttatttgccagcgccactccctgcccgtggatagccgcttgcagcaccatggcgctatggctaaaaattggcccttgctgaacgttgatatgatttaaccccaactgtcgggtatatgtctgccagtcacggcgcgaagcatcatgtaataacgtatgtttagccagatcttccggtgtcttcaagggtttttcgccagtcagcagtagcggcgaacacaccggcaataaatattcggcgtacagtttttccacccgtagccccggccagttgccccgaccataaaatatcgccacatcaacatcatccgccagcttatcttcctgacgatcaaccgcctggattcgaacgtcaattcccggataagctgaattaaagctggaaagtcgcggaaccaaccaatgaatggcgaaactggggagtaaactgaccgtcaacgcccccttggcgctacgggcctggagtttacgcgtcgcttcggttaattgcgaaaatatctctttgatatcgaggaaatagctttgcccttcctcggtcagcaggagtgaacgattacggcggcggaacagttttagccccaaaaaatcctcaagagacttgatttgatgacttactgcggcttgggtcacaaaaagctcttctgctgcgcgagtgaaacttaaatggcgtgctgcggcatcaaaaactcgtaaggcatttagcggtggtaatcgtttagacatggctattaaactttgatgttaaatgaatttaacaattagatcacactatgtaacctattagtttttttaatctgagccattataaattgtccgttgagcttctaccagcaaatacctatagtggcggcacttcctgagccggaacgaaaagttttatcggaatgcgtgttctggtgaacttttggcttacggttgtgatgttgtgttgttgtgtttgcaattggtctgcgattcagaccatggtagcaaagctaccttttttcacttcctgtacatttaccctgtctgtccatagtgattaatgtagcaccgcctaattgcggtgcttttttttaccttgcgatcgcgaattactgatccagttcgaccatctctttcacgtcagtacggttgatctgctgtttgttgccattagcgtctttatacgaaatcataccggtatcgttatcagtctgtggtttgccgtcagagacgatggtacgtccgtcattggtgtgcatcacatagttcgaaccggaacaggcgctcagggcaaaagtcagcatacaggcagaaataattgcggcagtctttttcatcatcttctccttaaagcgattaataaatcttaatagtattgattaacaggctaaaattaacgcctaacactattcagcatatgttacttacgcggcttcgccaggatatccagataattctgatggttagcactctccttgtatcaaagtgaattttgcgtcacgatcggtgcatcaagccgaggagtaccatgaacgtttttaatcccgcgcagtttcgcgcccagtttcccgcactacaggatgcgggcgtctatctcgacagcgccgcgaccgcgcttaaacctgaagccgtggttgaagccacccaacagttttacagtctgagcgccggaaacgtccatcgcagccagtttgccgaagcccaacgcctgaccgcgcgttatgaagctgcacgagagaaagtggcgcaattactgaatgcaccggatgataaaactatcgtctggacgcgcggcaccactgaatccatcaacatggtggcacaatgctatgcgcgtccgcgtctgcaaccgggcgatgagattattgtcagcgtggcagaacaccacgccaacctcgtcccctggctgatggtcgcccaacaaactggagccaaagtggtgaaattgccgcttaatgcgcagcgactgccggatgtcgatttgttgccagaactgattactccccgtagtcggattctggcgttgggtcagatgtcgaacgttactggcggttgcccggatctggcgcgagcgattacctttgctcattcagccgggatggtggtgatggttgatggtgctcagggggcagtgcatttccccgcggatgttcagcaactggatattgatttctatgctttttcaggtcacaaactgtatggcccgacaggtatcggcgtgctgtatggtaaatcagaactgctggaggcgatgtcgccctggctgggcggcggcaaaatggttcacgaagtgagttttgacggcttcacgactcaatctgcgccgtggaaactggaagctggaacgccaaatgtcgctggtgtcataggattaagcgcggcgctggaatggctggcagattacgatatcaaccaggccgaaagctggagccgtagcttagcaacgctggcggaagatgcgctggcgaaacgtcccggctttcgttcattccgctgccaggattccagcctgctggcctttgattttgctggcgttcatcatagcgatatggtgacgctgctggcggagtacggtattgccctgcgggccgggcagcattgcgctcagccgctactggcagaattaggcgtaaccggcacactgcgcgcctcttttgcgccatataatacaaagagtgatgtggatgcgctggtgaatgccgttgaccgcgcgctggaattattggtggattaatgacaaacccgcaattcgccggacatccgttcggcacaaccgtaaccgcagaaacgttacgcaataccttcgcaccgttgacgcaatgggaagataaatatcgccagttgatcatgctggggaaacagcttccggcattgccagacgagttaaaagcgcaggctaaagagattgccggatgcgaaaaccgcgtctggctgggatatacagtggctgaaaacggcaaaatgcatttctttggcgacagcgaagggcgcattgtgcgcggcctgctggcggtgttgttgactgccgttgaggggaaaaccgccgccgagttgcaggcacagtcaccactggcattgtttgatgagctgggattacgtgcgcagcttagcgcctcacgcagccaggggttaaatgcgttaagcgaggcgattatcgctgcgacgaagcaggtttaagcacagaaccgggtcggataagacgttcgcgtctcatccgacctgattgtttaaccctgacgcgccgctttcgccatcatcttcttcagcgcatgagaaaccgcaacaaacccaaaggtggcggtcaccatcgttgccgcgccaaatccagatgcacaatccatccgcttcggcccttctgccgtggctttcatcgcacacaccgtaccgtctgactgcgggtacaccagcgcttcagtagaaaacacgcaatccacgccgagcttacctttactgtttttcactacgccaaaatcgcttttcaggcgctcgcgcaacttcgccgccagcgggtcctgaatcgttttcgccagatcggtaacctgaatctgcgtcggatcaatctgcccacccgcgccaccggttgtgaccagtgggattttattgcgccgacaataagcaatcagcgccgctttgggccgtacactatcaatggcatcaatcacgtacgaataacccacgctcatatactgcgctacgttatccggcgtcacgaaatcatccaccaccgttacacggcactccgggttaatctggcgaatacgctccgccataacttccgcttttgccagcccaacgttatcgcgcagggcatgaatttgccgattggtattggtgacgcacacatcatccatatcgataagcgtgattgcgccaatccccgtgcgcgccagcgcttccgccgcccaggaaccgacaccaccgataccaaccacacaaatatgcgcgtcagcaaacagttgcaacgctttttcaccatacagacgcgctgtgccaccaaaacgctgacgccatgcatcactaattaccacagacatagcacctcagaattaaaaagggcgaggttatccctcaccctaaacgcataaatgcctgatgcgctacgcttatcaggcctacataactcctgcaatattttggatttgcatgatttgtaggccggataaggcgttcacgccgcatccggcatgaacaacgcgcacttagtcaataatcaggatgtgaggttacccctcaccctgtcatatccgtaaaaacggcatacagaatatcacatcagccgctaaagacgttacctgcgcccggggcggttttcagcacccagacacgtccatagtggttgtaccaacctgcgcggtgtccggcttccggcccgatcccttgatagatatcgaagtgttggcctttgattgcaccaccgacatccagcgccaccatcagacgcagttcgtactgaccattaaatttgccgttattatccagcaacggcacttctgccagcaaggtagtacctggcggaataatggaacgatcagaggcaactgacgcgcgaccaaccagcggcaccgcacttgcccctttcaccggagcaaaagattgcggtttaaagaagacgaaagacgggttctgttccagcagctcgcgaacctcggcttcactgtgtgtttcgccccagtgacgaatcgcctgcatcgacatatcttcttttttcacttcgccacggtcgatcagcaccttaccaatgctgcgataggcatgaccgtttttccctgcatagctgaaaaagttaagcggactgccatcaccaaagtcgatatacccactaccctgcacatccataatgaagttatccatcagggagttactgtaagcgagaatatatttatcactcaatgcccccgcgtagatctccgcacgagacggcagacgaccacgttttggcggcatacggtaaataggatactggaactcgccctggcgggtatggcgcgcctgaattaccggcgtgtaataaccggtaaactgcacgttaccatagttgtcggcaccttccatctgccaggcatcaatgccgaactggcgcatattgcgggtatcaccgcctgcgcgcagccactcttgcaccgcgttataaacattactctggttgccatacagacgcggtgacgaattacggatatggttaatttgctcggcaaaatcaccggcgttaatcggcgcgccaacggcatctggctggttcaccagagagaaaggctgggtaaatttcccgtctttatattgctgtccgcgatcggttggtttggaagagcaggcggcaagcattgccacaaccgtgcccataagaaggtactttacccaacgtcctttcattgttctcttcttcaggttaaaaaataaggcgcaacgaagataacaaaccgccgcgtttaatgaaatgagcagcctctccctgacgcaaattttgcacaaaaaataggctttagtgatttgtttttgttcaaaatcatgccaaatccgtgatcggggtaaaaaaaaggttgcatgaaaacgcgagcggagtatagtgcgcatccacggacgcggggtggagcagcctggtagctcgtcgggctcataacccgaaggtcgtcggttcaaatccggcccccgcaaccaattaaaatttgatgaagtaaagcagtacggtgacgcggggtggagcagcctggtagctcgtcgggctcataacccgaaggtcgtcggttcaaatccggcccccgcaaccaatcaaatttgatgaagtaaaagcagtacggtgacgcggggtggagcagcctggtagctcgtcgggctcataacccgaaggtcgtcggttcaaatccggcccccgcaaccaattattgaacaccctaacgggtgtttttttgtttctggtctcccataaaaaagcgccattcagcgcctttttatcatccccttctcgccagcgtcgccccatcggcaaaatacgctttaatccccgcaagaatagactccgcaacttcctgctggaaagtcgccgttttcagtttacgctcttcctcaacgttactgataaacgccgtttcgaccagaatggagggaatatctggtgcctttagtacggcaaacccggcctgttcaacttgatttttatgcagcttgttgattttaccgagcttattcagtaccgctttaccaaacttcaggctgtcggcaatggtcagcgactgtaccatatcgaacatggtgtggtcgacatagcggtcaccgcttttgctcacgccaccaatcaagtccgaggcgttctgggtttgtgccagatattttgccgcagtactggttgcacctttggttgagagcgcaaacacagaggaaccgctcggctgacgactggtaaaggcgtcggcatggatagagacaaacaggtcagcacgctgtttctgggcttttgctacgcgcacttgcaatggaatgaagatgtcttcattgcgcgtcatgtacaccttcatattgccctctttctcgatcagagagcgcaaacggcgagctatttgcaataccacatctttttcgcgcgttttgtatttccccaccgcaccggagtcttcgccaccgtggccagggtcaagcataatgacaatcggacgatcgcgccctgctttacccggttgtggaccactttgcgctggcggcacctgcttttcgaggtcgcctttgttgtaatcctccagcagcgccagcagcgggtcctgcatatcctgtgcattggccggatagaggtccatcaccagacgctctttaaacccggcgaccggcgcaagggcaaacagctgcggttttacgttttgctttaattcaaaaaccatccgtacggtttgcgggtcaaattgcccgacgcgcgccgacttgatgaacgggtcgtctgcacgaatttgtgccgccatccccttgagtaccgagttcaggtttacatcttcgatatccaccaccacgcgttcagggttactcaacgcgaactgcttatatttcagctgacgatttgattccaccgtcacgcgggtgtagctggacgcaggccagacgcgcaccgccacgacctggctgaccgcagccagactgacctgacttacgctcaatagccacatggcacccgcgccttgcagtaaacgacgacggctgattgcagtgttggatcctgacatgcctctcccgagcaaaagaaatctaagctgtgtaacaagtaaacgactaatttgaccggaaactttagcgaaagacgcataatctgtcatctaataaacggtaaacattctttttatattcacggcattactgataaaaaagtcgctctcgcataaaatttacacttgcaccctgcgaaaaaacagaataaaaatacactaatttcgaataatcatgcaaagaggtgtgccgtggtaaaggaacgtaaaaccgagttggtcgagggattccgccattcggttccctatatcaatacccaccggggaaaaacgtttgtcatcatgctcggcggtgaagccattgagcatgagaatttctccagtatcgttaatgatatcgggttgttgcacagcctcggcatccgtctggtggtggtctatggcgcacgtccgcagatcgacgcaaatctggctgcgcatcaccacgaaccgctgtatcacaagaatatacgtgtgaccgacgccaaaacactggaactggtgaagcaggctgcgggaacattgcaactggatattactgctcgcctgtcgatgagtctcaataacacgccgctgcagggcgcgcatatcaacgtcgtcagtggcaattttattattgcccagccgctgggcgtcgatgacggcgtggattactgccatagcgggcgtatccggcggattgatgaagacgcgatccatcgtcaactggacagcggtgcaatagtgctaatggggccggtcgctgtttcagtcactggcgagagctttaacctgacctcggaagagattgccactcaactggccatcaaactgaaagctgaaaagatgattggtttttgctcttcccagggcgtcactaatgacgacggtgatattgtctccgaacttttccctaacgaagcgcaagcgcgggtagaagcccaggaagagaaaggcgattacaactccggtacggtgcgctttttgcgtggcgcagtgaaagcctgccgcagcggcgtgcgtcgctgtcatttaatcagttatcaggaagatggcgcgctgttgcaagagttgttctcacgcgacggtatcggtacgcagattgtgatggaaagcgccgagcagattcgtcgcgcaacaatcaacgatattggcggtattctggagttgattcgcccactggagcagcaaggtattctggtacgccgttctcgcgagcagctggagatggaaatcgacaaattcaccattattcagcgcgataacacgactattgcctgcgccgcgctctatccgttcccggaagagaagattggggaaatggcctgtgtggcagttcacccggattaccgcagttcatcaaggggtgaagttctgctggaacgcattgccgctcaggcgaagcagagcggcttaagcaaattgtttgtgctgaccacgcgcagtattcactggttccaggaacgtggatttaccccagtggatattgatttactgcccgagagcaaaaagcagttgtacaactaccagcgtaaatccaaagtgttgatggcggatttagggtaagcgatgaaaatcgtcggatgcgacatgcgtaacactcgtacgtcgcatccggcaattacgtttattcccgtgaactaaacaacgccgccagaccactgcgccgctcagtacgagtggcgattgccgcacttaatatgcgctcatcggcatacagcgacagacggcgacgcgcgcgggtcaccgcggtataaaccagctctcgcgttactaccggcgtgcgttggctcggcaaaatcaacgccgcatggtcgaactccgatccctgcgatttatgtaccgtcatcgcccacgtagtttcgtgctctggcaagcgactcggttgcacagacttaatattgccgtccggcatcgcaaaccagacgcgcgtcccctgcccgcgatccagcgcaataccgatatcgccattaaacaacccaagcgcgctgtcattacgggcaatcatcaccggtcgaccttcgtaccaacgagagtgcggatgacgatgaattttgcgcttctgttgcataaactgctcaattcgctcattcagtccagccacgccaaacggcccttcccgcagggcgcacaaaagctggtactcattgaacgcctgaatgattaaatccggctcggcacgcgcttgcagcagatccagataacgtccgtaacccgcaagagcttcctcaagcatcgcaatataatcttcgccgctctgtaaaagccgtttttcgatatcagtaaaatcctgctgaaaaacggttttcactgccgttttatcaccacggttgatcgccgcagctaactgaccaatgccagaatcgctgccgaaacgatagcttttttgcagcaggcagagactgtcgcgcaaagatgccgcttctgtgccggttcctgccggaacgtgagtccccgtcaggcggcttagctgcctggcacgctcggcggtaaagcccgcgttggcataagcgcagatatcgcccagcacagccccagcctcaaccgaggccagttgatcacgatcgccgagaaagatcactcgcgcatgatcgggcaaggcgtcgatcagtctcgacatcataggcagatcgatcattgacgcttcatctaccaccagcacatcaagatgcagcgggttaccggcatgatgacgtaaacgctggctacccggctgcgcgcccagcaatcggtgcaaagtgctggcatcttccggaatgcgtttcttttgttcatcggtcagcggtaactgtcgcaaagccttgccgagagattcggttaagcgcgcggcagctttacccgttggtgcagccagacggatacggcagcgttcgccgtcggccatttgaattaacgctgccagcaacttcgctacggtggtcgttttaccggtgccagggccgccggaaatcaccgagatccgccgcgtcagcgccactgccgccgcaactttttgccagttaatttcatcgcttactggaaaaagtttgtccagggtttgcgccagtagagcttcatcaacctcaatggcatgattcacttcgttgaaaaagcgtgccactgtgcgctcgttacaccacatgcgattcaaataaagacgatcgccacagaggatcatcggcgtgggttcatctcccctgctgaccgcttgagaagccagcaagcattcttcccaattttgtagctcaccgatttcactgacacaggtcgccaacagcggatgcgacgcctcgttattttccagtcgtgaaagcggcaaacaaacgtgtccctctccggcatcatgacttaacagtgccgccgcgagggtgacggcaggatgttcatctcccgccacggtcagggcaaattgcacatccagcgggcgtagctgtttgtgctccacagcttccagtaattgcttttgcaatttcattacgcctcctccagggtcataccggcaaacatctcatccatcagggcaatcaacccggcgttgggtcgggttgtgtaaatcccctgttgcggatgttctttatcaacgccacgcaggaacagataaataacgccgccaaagtggtgctcatagtcgtaatcagcaatgcgatggcgcagataacgatgcagcgccagggtataaagctgatattgcagatcatagcggtgtgcctgcattgccgctgccatagcctgttgggtgtaagccgaactgtcttcacccaaccagttggatttatagtcgagcaggtaataacgcccttcgtggcggaacaccaggtcgataaagccttttaacatgccacgtacctgcatgaactccagcggcgggcagcctgcggatagcgggtcaaactggcggattaacgtatcaagctgactggcgataagcggttcactaatcggcagataaaactccatctccacctgtttattgcgggcggaaagttgactcaggcttacgccggtttcattgagaggtgcctggaggacagccgtgatccactcggtcaataccggttcccactgcgattcaaagccgccgagttccagtttttcccgcacccagttcgggtcaaccggctgggtaaaatccaggtcttcaaacaaactgtgcaagaacgtccccggtgacgcaccgcgcggaaactgatgtggtgttaacgtcggttcttcaacgacgctggcaacgcctgcagcatcgacatccagccgaggcatcaaatcctgggcgataccgtgaccacgctgttgcaaaccagagtagctggtgacgcgccagttatcgccgggcaatcgttgtaacgtcttcgcattcagctctgctgtagaaacatcattaacctgccagggttggttatcaccagtttgtgccgtttgccaggcaatatcatcatcgcataacgcttcaatacaggtgcgaagccctgccgcatcttgcggttcccctttttgcagcaaacgcccgagcgcactttggtggacgtcggtgtcaccttttttatcgccacgacggcgcaccagcggtgcaacgccgagactgcaatgccaaaccgaacgtgtcagcgccacgtaaagcaaacgcagatcttccgccagacgttcggcctccgcgaggtcgacgctttctggcgcagcattaagatccagaactgcctcaaacgagtggcgatcgtgataaaacgcctgctcctggacgcggaaattggtgataaacggcagccagaccaatggatattccagccctttcgatttgtggatcgtgacaatctgcaccagatgtttatcactttcgagacgcatttgttggctggaggcattactgtctggctcgaggatatgttgcgataaccagcgtaccagcgcatgttcactttccagctgcgttccggcttcttgtagcagttcgctgatatgcaagatatcggtaagacgccgctcaccgcctgccgttgccagcaagttttcagcaatgttacgcgccgacatcagcgcccgcagcatcggcataacgccacgtttgcgccagatttgccgataaccatcgaactcttcgactaccacatcccacgcatgttcgtcattgttcagcgtttcgatatccagcgcgttcagccccatcattgacgttgccagcgcactacgcagggtgttctcacgttcgggcgtcatcaccgcctgcaacaaccaaagcatttcctgcgcttccagagtttcaaaaacactgtcgcggttcgaaaggtaaacggaagggatttccagcaacgttaaggcatcgcgcacctgggcggcctcctggcggctgcgcaccagcacactgatgtccgaagcacgcaccggacgcgcgtcgtcgccgttcatcagcaacgcttcgccccgctgtccggcttgtagccagtcgcggatttgcgcagcacatacctgcgccatggtactttgataatcgccaacgccgcagctttcgccttccatcagccacattttcatcgcaggctgtgtttcacctttaaatacaaaacgtaacgcctgatttttcccggctgatttcactggaataaacggtatttcgcgaaacatgaacgcgtcatcagtctggctgaaaagcttattcacgctgttcaccattcctggtgcggaacgccagttggtgtctaaagtgtagtgggcgtgaacttcgctacgcgccttcatataagtgaagatatccgcaccccggaatgcatatatggcctgcttcgggtcgccaattagcaacaatgcggtttccggctgatggtgccagatacggcgaaaaattcggtactgctgggggtcggtatcctgaaattcatcgatcattgccaccgggaatcgcgtacggatcgccgctgccaacacctcaccgctttcgctacgcagcgcggaatcgagccgacttaacatgtcatcaaaacccaattcgccacggcggcgtttttcacgcgctactgtttcgcggatctcagccaatgcgcgggtgatcaccagatcgcggatcgacaatggttctgcaagcagttgatcgatcgcctcaaacagtggatgtcgcggggtttcccccccggccttcgtgcgatcttctaagaaacgctgggagaatttttccagcgactccggcaactgataactgtttgtctcttcttctgcccaggcgctgatcttgtcgatccatttagcctgattgctacggttaaacttgcgtcgatcaataccagaagattcgatcagcgcatccagttcacccactgcgtcgcgccactgctgttttaccgtatcaatacgcgccacaatttgcgcgtgacgggaagccagcgtttcatcatcgggcggcggtgctttgataaccggcgcttcgccttgcagataacgattaatatcgcgcagcaacgcctgcggccctttccaggtttcaaagacgacctgggctatttcacgcggcagcgggtagcagtggcgacgccagaaatcggcgcaggcctggtagcgtagcagagactcatcttcaatcagctgctgctcaaacagcatgccggattcaaaggcattcaggttgagcatgcgctggcaaaagccgtgaatagtaaagactgccgcttcatccatctgccgttcggctaacaacaaccactgcgcggcttgcgctttatcgtcgatctcttccagcaggcgttcgtacagtggattgtcggtggtttcacgcagacaggcgatgcgcaactcgtggatattgctacggatacgaccgcgcaattctgccgtggcagcctcggtaaaggtgaccaccagcagttcttcaacggtcagcgggcggggaaaggcggcggaaccgcctagtccaagtaacaggcgcaaatagagcgccgcaatcgtaaaggttttgcctgtgccggcagaggcttcaatcaggcgctcaccctgtaagggcaagcgcaaaggatctagtgtctcggcgacatcactcattcttttcactcatcaggggcattgtttgctgcaacgcgctgacgttctcccacactttccagccttcagggtgtacatattcggctttcccgttctggctgccggaaatctgcgacagaatagccatgccttgcggctcgaccaccgcctgatggaagaaatcagcaagtttttgcggcgtcagcagttttatctgggccacgattttatcacgcgaatcgaagcgcatattgccgcgatcgaaatctttacttaacttcgatgcttcttcgccgagcgtttgcggtgcctgcagcatctgggtaattaccgcctgctggatttgcgcaaactcatctggcttcatcgctcgcaattttgcctctgcggttgggaaaaacgccttgtaacgctcccacaagaatgaaggctgtttatcattgctttgcaaaaggaagcccatgccccactgacgccccacgctcattggaaacgcaaacacggcatagcccaattgttcttcggtacgcaactgattgtagaaccacggctgtacgatctgccccaacagagagctataggctgagctggtgtattcatcgtagccagtcggtacaaataccgctgccagtgcggagtcggtgctgttaccggctttttcaaagatgacggattgttttttatcgaccactacatctttgtttcgacaccactctgaaccatcagcgcccaactgtttttgcacatcgcgtgccagcgttgttgcctgggcctcggtcatgttgccgataaccataaactctggtcgagcccctgattttaaggcgtcgcgataggccagcacctctttcaacgtaatggagggcaaaattttacgccgttcatctcgcgagaagtacggcacttgcgagagcatctgcgcgggcataatcgcctgctcaaacgctttacccttttctgcggaatccatcatctggttataccaggacttcgcctgctcaagctgatcttccgtagcggtatagctaaagtacccctcgagcaatgcctggaacagctgcggcagacgctgggtgtaaccattagcattaaccataaggccgttgttagcgttggtggaaaaacttatgccaccaaccgacgcctggttgcttaactgatcaagcgccagccctgcgagataatcattgagcgcaaacatcacctgattgcgggcgctgtccatggctttcggattacgcaaaatcaggctgacatcagctttgggctcgctggcaaaataacggcttggcgcatacaccacgcgcagattcgactcatcaacaatcagctctggatggtcgtatttcttctctgacttaatcagcgagaaatcatcaggaatataagggttaagctctggcaaagagagcgcaatgtcggcggcttttttctgccagtcggcgaaagtttgtgcgctgattttatcgacctgatacggcgcatcgacaaagtaagccgttttgttgtgcggctctttcgggctgatataccagatacgcgcattctgcggcgtcatcatcgccagacgttcctttactgctttagcatcgtaccgatcggcaatattgactgcatccagcgtatgctcaacaggaacgcgaatcatggtatctgccagccattcgacgtaatccatatcacgggtgatcgacggataacggaagtcgatatccagcacattcgccagttcatcgaagtattgtttatcaatgcctttttcacgtaacagattgagatagctaaaaattgccgccacaacctgatcgcgattagccaggcctttatcggttaaagacgcagagatcgctaatacgccgctgttgccgttgacgataggatcggagttggcgctaatgccctcaactaatccctgcttttgcagccagtcagaaagtgtacctgggctgcgattgccaatcagataggtaatcaattcatcggttttactacggaacttcgctgagttgttatcgatgcgaaactcaacgcgcaacactttacgcggcagcgcagggacgtaatgaatgataatgcccttttgcgcgtcggtgactaccggcacggtgatttccggttttttgctctctttgttcggcacgcgaccaaaggtgtccgccgccatttttgccaactccggcagcggtttattactgtaaataaccgccttcatcaaattggcggaatagtacttctcgtggaaatctttcagcgcctgctgcaccggattaccaggtttgtcgcttaaagtttcgaggttaccaccagaaaactttgaaccggggtgtgccgggttaatggtttctgcgctgacctgtgccatgcgcatcccgtcacgcgtacgcgccatggttaattcagcgttcaccgcattacgctcacgttcggcatatttcttgtcgagcaaaggttcagcaatagcatcggccaggcggtctaccgcaccaggcaaggcgtcgttctcaacttccagatagaaagccgtgcgatacggcgcagtgctggcattgtgactaccgccgtgcattttgagatattcggccagactgtcagcctgcgggtactttttcgaccccatcagactcatatgttcaaggtaatgtgccagcccctggtacgcctcgggatcttccagcgacccaacgggcaccaccagcgccgagagcgatttaactgcctgcggatcagaaaccagcaagaccaccataccgttatccagacgtatagcctgatactggcggttatctttatcacttttacggatggtttcctgaatcggctgccatcccgtttctgcctgacttaagggtgcccaaagggcaactaacaacaataatgctttgaaccaggtgctgcggggcattcacggacctcataatcaacttaattttctgtccagattcaacacgttaacgcaaatcatctgccagaatttaatcttgtgctgcacgagtcagcctatgtttatataaccatcagtccgtgactggtgcgcatcataaagtaagcggatagattgcgcaatttttatacagcactcatgactgattaaagcgaaacagcggtaacaggaaacgttgcgactgttcaacgatggcctccattgtctctggtgttaattgccgccagagcctttgataccagatatcatcaccttcgccacgcaccatcatgttgccttcgtaagcctgaaggaatttcgtacgggctttttgcaacgtggaatcgtcatccagcatggcatcgttttgcgcgtcataacaggtttttagccacgcgccgccactttcaggtaacaccagcaatggcgcggacattccttcacgatacccctcaatcagttgtgagaggtaatgcaaagcctgttcggctgcaagcggcggaaaacgccactcgccgtctttgcgtagaaaaaggcgactttcaccattaccaccgctggcacagtagacaaggtgttccagccaaagttgcattccctgggccacacttaataaagagggacgccagcgcaacaggccatccggctgcacctgcggcaaccagccagttatctgcacaccgttgcaggcgagatcaatttccatactctgccccggctggcgacaggcaatgactctgtcggcaagctgctgcatctcctggcactgtgtttcccagaaaatttcaccaaaagcgccatacggtaaatcccctgccgctcggaagcggcggaacaagcgttcggcatcatcctgctcaaccagtgcattcaataactgctgattgatttgataacggctaagtccttccagaataaatggctcggtgtcggggatttcgctgtcttcagtacggaagttcacctgcaaacgcatctggaaaaatgcccgcaccggatgtgcccagaatcgttgtagcgtttccagcggcacggtttccggtaaggtaaacggcagcggctgaacaaattcagaatgtgctttaccagcctggctggccgcaggtagccattcacgagcatagctttgtcgttcgcctggctggtagttttgtggatcaaacggcatccgggtatggaggcaagtaagatgcgcttttacccttgcctcgctttcatcacagttgagcgcttcatcgcccggtagataatgactttgcccgatgtagtcgatcagttcctgcaccagtaccgacgggaaacgctcactgttatcctgaatggaacgaccgatatagctgatatagagtttttgctgcgcggaaattaacgcttccaggaacagatagcggtcgtcatcgcgacggctacggtcgccacgcttcggtttctggctcatcaggtcaaagcccaatggcgcaagctgacgtggataaacgccgtcgttcattcccagcaggcaaaccactttgaacggaattgaacgcattggcatcagagtacaaatgttaaccggtccggcgagaaaacgctggctgatacgttcttgatccagacgctgtgccagttcatcacgcaatagtgacagcggcaccgcgtcgccatactgcgcacctaaaccttcggcgataatcgcctgccattgttgttcgatcagcgtcatcgccgcttcggtttccgcatccggcaggaagaaggcgttgagcatatcgcgacaaaccggcaaccactcttccagcggacgctcctgtgccagcccgcgacgccagatgtttagctgcattagcagtgaagccagatgccccaccagttctgcaattaagccgctcgattcatcataaggtagaaccgattgccactcgccctgcgcgctctccatcgcgtagcccaacaacatacgcgtcaggccaaatcgccaggtgtgttgtccggtggcggggagttccagctcgcgaacgttgtcgtcatctatgccccaacgaatgccggattcgttgacccactggcgtaaataacgcagcccttcttcggtgatgtcaaaccgcgccgccagcaccggcacatccagcaacgccagcacatcctctgacacaaaacgactgtcaggcagtgataacaggctgataaacgcttccagtaccggatgtgactgccgcgcacgacggtcggaaatggcgtaaggtaggtaacgatccgcaggtgcgctaccaaacacagcctgaataaacggactgtagctgtcgatatcagccaccatcacgatgatgtcgcgcggagtaagtgtcgggtcttcctccagcatcgccagcaggcgatcgtgtaaaacttcaacttcacgctgcgggctatggcaaacgtggaaggtgatactgctatccagtggatcaagcgggcgtttgttatcgctacgggaaaactcttcgatgttcacaccagcaacggcgcggttttccagttccagaatgtcagactgaatgttatgcagcaggttatctggcgtgacatcgacaaaggcgtccagctcctggctgctctccaggtcagaaaggagataaatgtagtcgcgcccaagcttaccccatgaagccagcagcgggttgccgacatcctgttcaccatcgctgttaaagagctgcccggcattttcgctatcacgaaatagcggcaattcgcgatcttcaaaactgtgtcgacgctgacgggtcagcagtttcgccagataagcaggatctttaatatcgccccagtaataacggcaggggttggtaaacaggagatggatttcaatatgtttacccagcgcctgtagcgcctggagataaacaggcggtaacgcggaaataccgcatataaagacgcgcgaaggtaaccccggcgggcaggtcgtcgcggactccagcgtttcgataaagcgctgatagagattggcgcggtgccagcgcggttgcccgagttgatgggtatattccaccagcgccttccacaacggggcttgccaggcctgtgcttctcccagcccttcaaccaaatgtcctgtttcccactgtgccagccagtccggacgatagaccagatactggtcaaacaggtccgccgcttttgaggaaagctggaacagttttcgcttgtcgctatcgtcagtcagataatgccgcaacagggtaaagtcttcgcgctccagcaattgcggcagcagagtcatcagtttccagctcatgctctgtttgttaaaggcgctctctttggggatttccggtaacacccggacgaacatatcccagataaagctcgctggcagcggaaaatcaatgtttgccgcaataccaaacttttgcgacagggtcatttgcagccactgtgccataccggtactttgcaccagaatcatctctggttcgaaaggatcgtccagccgttcgcgttcgacaataaactccatcaacgcttccagcacgtccagacgattggaatggtagacccttaacatagcggctcctgactactgacgattcgggcaatgcaggcgggtcatctcgccttctctgcccccgggtgaaactagcgtaacgctgatgctgacacatcccgcctgcgatgtctgcattcggttgacctgccagttggcaggtggcgaaatcgcgcgcagttgcgtttgctgccagccatgccgccagagctgttggtactggtttctgctggcaagactgttcattaatgttcgctggaaacccgataacgcagtgacaatcatcaccatcaacaccatcgccaacattacctccggcaggctaaagccttgttgattcttcagggaagctgacataacgccctctctttcagcggacaaaaatcgctccagccgcgtggcgaaaaaacaatgtttccatcaatgacttcgcctgttcgccacaacgaaacgccttcataaccggcaatcaataaggcttcattatctgccagtaaacgcaaacaaacctgggcatcggtttcagcgtactgcgagcactgaactgctggctgcgtctgccagcagtgcatttttccccacgccagcgccgactgaacgatggcctggcggcgcaatgactgactttccatgctcacgcgagaggcaaaactgcgatcctgttggctcattccttgtaatagcaaactacccaaaaccagcagcatcaggaccagagccagtgacgaaacacccttttcgcggttcacaggttgaatcctgtcacgctatagctggcattcaccacggtttgcggttcagacttactggcagcacgcatattaaccgtcaacaccggcgagaagccgctgacatcctgacgtacgacctgaaaagtgtcgataatgatggcatccggattagtgactttatcccagcccttaccttcacaggatgtcgcaccgcgtagcgtttccagcacatgctccttcagacgaaatccaatctggtcggactcttttaccggttcgcgatcccagataccgttactgttcgcatcccactgcacaatgacacagtcaccctgtccgacaatttccagcccttcgccggtacagatgccatgacaataacccgccctctggagatgcttcgcgacggtaaatacccgcagccagatttcatcttccagcgccagcttacgggtgctcgttaaactttcacgctgtaacgcaggcagaaagcgtgccgcccccagcaacaatacgctactgatcgccatagcaatcaacacttccagcagagaaaaaccttgctcttttacaggcatccttctgtttctccttgctgacaaagccggagtcttccccacggcgaaaccaccagccaccactcgcccgttgagtttttgaagcgaatatgcccggcccatgcggtattgcgcaggccaaagaaagcaagcgaaggtgtcaggtcgctcatttcgacttcgggccagcgtggcacaaagaccaatggtgaactgccatgacaggtattggccccagcagcggaactcacaaggcaccataacgtcccctccctgataacgctgatactgtggtcgcggttatgccagttggcatcttcacgtaaatagagcaaatagtcccgcgcctggctggcggtttgccatagccgttgcgactgctgccagtattgccagccatagagtccacttgcgcttagcatgaccaaaatcagcatcgcgaccagcgtttcaatcagcgtataaccacgttgtgttttcatgccggcagtatggagcgaggagaaaaaaagacgagggccagtttctatttcttcggcgcatcttccggactatttacgccgttgcaggacgttgcaaaatttcgggaaggcgtctcgaagaatttaacggagggtaaaaaaaccgacgcacactggcgtcggctctggcaggatgtttcgtaattagatagccaccggcgctttaatgcccggatgcggatcgtagccttcaatctcaaagtcttcgaaacggtagtcgaagatggattcgggtttacgtttgataatcaacttcggcagcggacgcggttcgcggcttaattgcagatgagtttgatccatatggttgctgtacagatgcgtgtcgccaccggtccagacaaaatcacccacttccagatcgcactgctgcgccatcatatgcaccaataacgcgtagctggcaatgttgaacggcaggccgaggaagacgtcacaggagcgctgataaagctggcaagagagtttgccgtctgccacatagaactggaagaatgcatggcacggtgccagcgccattttatccagttcgcctacgttccacgctgaaacaataatgcggcgcgaatccgggtcgtttttcagctggttcagtaccgtagtgatctggtcaatatgacgaccatctggcgttggccaggcgcgccactgtttaccatacactggcccgaggtcgccgttttcatcggcccattcgtcccagatggtgacattgttttcgtgtagataagcaatgttagtgtcgccctgcagaaaccacagcagttcatggatgatggaacgcaggtggcaacgtttagttgtcaccagcgggaatccatcttgcaggttaaaacgcatctgatgaccaaaaatggaaagcgttccggttccggtacggtcgtttttctgtgtgccttcgtcgagcactttttgcatcagttctaaatactgtttcatggttcctcaggaaacgtgttgctgtgggctgcgacgatatgcccagaccatcatgatcacacccgcgacaatcatcgggatggaaagaatttgccccatgctgatgtactgcacccaggcaccggtaaactgcgcgtcgggctggcggaaaaactcaacaatgatgcgaaacgcgccgtaaccaatcaggaacaaacctgagacagctcccattgggcgtggtttacgaatatacaggttgaggataataaacagcaccacaccttccagcagcagctcgtaaagctgtgatgggtggcgcggcagcacaccgtaagtgtcgaaaatggattgccactgcgggttggtttgcagcagcaaaatatcttctgtacgggagccagggaacagcatggcaaacgggaagttcgggtcaacgcggccccacaattcaccgttaataaagttgcccagacgcccggcaccaagaccaaacggaatgagtggtgcgataaaatcagagacctggaagaaggaacgtttagtacggcgggcgaagataatcatcaccacgataacgccaatcaggccgccgtggaaagacatgccgccgtcccagacacggaacagatacagcggatcggccataaactgcgggaaattgtagaacagaacataaccaatacgtcccccgaggaagacgccgaggaagcccgcatagagtaagttttcaacttcatttttggtccagccgctgcccggacgattcgcccgtcgtgttgccagccacattgcaaaaatgaaacccaccagatacatcaggccgtaccagtgaagcgccacgggtcctattgagaaaatgaccggatcaaactccggaaaatgcagatagctactggtcatctgtcaccacaagttcttgttatttcgctgaaagagaacagcgattgaaatgcgcgccgcaggtttcaggcgctccaaaggtgcgaataatagcacaaggggacctggctggttgccggataccgttaaaagatatgtatatgatccgcgctataaccctccgcgaatcagcccgcccatgccgcgacgctccataaaggctgcaacctgatggcgaacttcggtcgccagttgcgcttccagactacgctgcgcaagattttctgcttcggcataatcaatgcgccgcagcaggtattttgcccgcgctacagaacgtccgttcatagacagatggcgatacccaagcccaatgaggattgccacgcacatgggatcgcccgccatttcaccgcacaaacggagatcgattccatgtatttccgcttcccgggcgatcatcgccagagctcgtaacattgcaggatgaagactgtcataaatgttcgccacccgggtattgttgcgatcaacggccagaatgtattgagtcagatcgttggtgccaacagagatgaaatcgacccgctttgccagatgcggcagcataaataccattgacggcacttccagcatgatgccgatacgtggtttgggaatttcgtaaccgatcatctcctcgacttcacgtccggcacgttcaatcaggcggcgtgcttcatcaacttcatcgaggcttgtgaccatcggcaacagaatattcaggttgcccgtagcggcattagcacgcagcatcgcccgcacctggatcaagaagatctccggctgatcgagcgtaatgcgaatcccacgccaacccaggcatggattctcttcgctgatcggcatgtaaggcagctgcttatctgctccgacatccagcgtacgcaaggtgacgggtttatcattgaacatttgcagcatcccctgatactgcgccacctgttcttcttccgacgggaaaccactttgcagcatgaatgggatttcagtgcgataaagaccgatgccatcaatacggctgcccagtttttcttcatgttccgggcttaaaccagcattgagcatgacttttatacgctcaccgctttttaactgcgcgggtaaattgacgtcatcttccgccagacggctaagctcaatctcttcactaattagccgctgatattcttgcagcagtaccggctccggatcgaccagcaattcaccgcgatagccatcaacgatcagcgtcctacgatgcagcaccgaaggctgaatatccgcgcccatcacggtagggatccccagcgcacgtaccatgatcgcagcatgggagttggctgcgccatctcgcacgacaacaccgactaagcgatcctggggcagctcagcaagcgttgtcgctgacagttcatctgccaccagaatgaaacgttccggccaggcgttcggcccttgattagcgtcatcaagatgaaacagcaatcgctgacccagcgcacgtaaatcgccagcccgctctttgagatagttatcacttagcgcggcaaactgttcggcaaatttttcaatgaccgtttttaccgcccactctgccaccgagcctttatcaacctcggcaaacaattcgcgacgcagccgggtgtccgaaagcaggtgcgagtaaagatcgaaaatagccgccgtttctttttgtgcaccggcggcaaagcgtttgctgtagcggcgaaactcgtttgccgcttcttccagcgccccggtcagtcgttcgcgttccagagccggatccagcgttgatgcctgatacacctgttccattaaaggtaacgtggcatcctgccagccttcggcaatcgccacaccaggtgctgccggtaatgcgcggattcgcgtctggcgatattgcccaaacaaggcagtcaactgcgactgagaaagaatagctgccatctgggtggcaagcgtcaccaggaaggattcttcactttcgtcatactggcgcaactctcgttgctgtaccaccagtacaccaagcaactggcgacgttgaataattggtacgcctaaaaacgcgcggaaacgttcttcttttacggaggggatgtatttgaagctggggtgcttttgcgcatctgcaaggtttatcggttccgccagcctgccaaccaggccgacgatcccttcatcaaacgcgagcgttacagtgcgaccgcgtggttttttcagcccccgggtcgccatcaggtagtaacaacgtcgatcatgatcggccaggtagaccgaacagacctcggtatccatcgcaagacagatgtcggtaaccagaatatttaacgcctcattcaggcgtggtgcgctggctaccttttcgactatttcgcgcaggcgagtgagcataattggcgtgacttaacctcttttacgtcgataagcagatgcgttttgtggttttggcgtattttcctgcagtgacatcaccacactcgcgaactctttcattaccctacggtagacatcacgtttaaatgacaccacctgtctgaccggataccagtaacttacccatcgccagccgtcaaactctggtgtactgctggtttgcatattgatttctgcatcgccgctcaccagctgcaagagaaaccatttttgtttttggccgatacaaaccggcttcgtgtcccaacgcaccaaacgtttcggtaatttgtagcgcaaccagttacgcgttgaagcaaggattcgaacgtctttgcggcttaatcctacttcttcaaacaattcacggtacatcgcctgctctgcggattctccggggttgattccgccttgcggaaattgccaggagtgctgaccaaatcgccgggcccacattacctgcccctggcgattacaaatcacgatacctacgtttgggcggtagccatcgtcatcaatcaccggactacctcaaaataaagctttatatacgaatgattgtttcatactccaggaagacggtaaaccactctctgcagggcattacacactaataacaattgaataactcacagttatgtgcagagttataaacagaggaaggggtggatagccgtttttattcaccttttctgtggatagagttgtgaagaactacggaattactacgggaaaacccggagcattctgaataagcccgatatagacattttaaaatattcattatcagtcaatgcattacatgtaattttagtaatgaaaaagagtaattcgtgacccaggtcacacctctcatttacgggttggcgaaagatcaaccaatgccgtatttatccacagaatgtgccactaagttaagcactgaaccactaaaaactggagtttcgtcgcacgtcaaggctgtaaatggaaacagtagtggaggtttttcacagttatcccagctttctgtggataacatggtgtaagatcctgtttattttcagtgaccagatttggaaaacccgttgcagtgttgcgcaactcgattaccggcaacctaaaaagcaatataaatcagagaattgaacaacgcatgtggaaaaagttacactgcgaatattcggcacataattgctgtttgttttttaatcaaggtatcatgacatgtcccaacctcgcccactgctctctcctcccgaaactgaagaacagttgttagcgcaagcacagcaactttctggttatacattgggagaactggcggcacttgtcgggctggttacgccagagaatttaaaacgcgataaaggctggattggcgtgttactggagatctggctaggtgccagcgcagggagtaaacctgagcaagattttgctgctctgggcgtggaacttaaaactatccctgtggatagtcttggtcgtccgctggaaacaacattcgtttgtgttgccccgttaacgggcaatagcggggtgacctgggaaaccagccacgtgcgccacaaactcaaacgcgtactgtggataccggttgaaggcgagcgcagcatcccgctggcgcagcgtcgcgttggatcaccgttgctgtggagcccgaatgaagaggaagaccggcagctacgcgaagactgggaagaattaatggatatgattgttctcggtcaggttgagcggattaccgctcgtcacggggagtatttacagatacgaccgaaagcagcgaatgcgaaagcgcttaccgaagccattggtgcccggggcgaacggattctgacgctgccacgcggcttttatttgaagaagaatttcaccagtgcactactggcccgtcattttctgatccagtagccatcgctttgacctgccgctttccgggcatataattaccgcttcatttttttggcagggctttttagatgttatttgcatggataaccgatcctaacgcctggcttgcgctcggtacgctgacgctgctggagatcgttcttgggatcgacaatattattttcctttctctggtggtggcaaagcttcccacagcacaacgtgctcatgcgcgccgtctggggttggcgggagccatggttatgcgtctggcgctgctggcatcaatcgcctgggttacgcgcctgacaaatccgctttttacaatattcagtcaggaaatttctgcccgtgatttgattctgcttctgggtggcttgttccttatctggaaagccagcaaggaaatccacgaatccattgaaggtgaagaagaagggctgaaaacacgcgtttcatcattcctcggcgctatcgtgcagattatgctgctggatattatctttagcctcgactcggtgattacggctgtgggtctgtcagatcacctgtttattatgatggcagccgtggtgattgccgtaggcgtgatgatgttcgccgcgcgctcgattggtgattttgtcgaacgccatccttcggtaaaaatgctggcgctctctttcctgattctggtgggctttaccctgattctggaaagtttcgacatccacgtaccgaaaggttacatctacttcgcgatgttcttctctattgcggttgaaagcctcaacttgattcgcaacaaaaagaatccgctctgatactccgtacgctctcctgcgggagggcgtactcactccttttaccctcacagtttaagattttcctgctttcaagatatataacgtcggtttataaacagactattatcataggtaggccaaatgaggataaccggatgaaaaaatgggcagtaataatttctgcagtcggactggcgtttgctgtttccgggtgttccagtgattacgtcatggcgaccaaagatggccgtatgattttgaccgatggaaaacctgaaattgatgatgataccgggctggtgagttatcacgatcagcaaggtaacgcgatgcaaattaaccgtgatgatgtttcgcaaattattgaacgttaacaaataaggtcagcatccggctggccttaagatttttctctttcccttttcccttccctctgccatttttatattccttatgtcgtgattataaaaaggaaacggctatgcaatatcaccgtataccccacagttcgctggaagtcagcacgctggggcttggcacgatgacgtttggtgaacagaacagcgaagccgacgcccacgcacaactcgactatgccgtcgctcagggcattaaccttatcgacgttgccgaaatgtacccagtacctccgcgccccgaaacgcaagggttaaccgaaacctacgtcggcaactggctggcgaaacatggcagccgcgaaaagttaattatcgcctccaaagtgagcggaccgtcgcgcaataatgacaagggcatccgcccggatcaggcgctggatcggaagaatatccgcgaagcgctgcatgacagcctcaagcgcctacagactgattacctcgatctttatcaggtgcactggccgcagcgcccgaccaactgcttcggcaaactcggttatagctggacggattctgcgcctgcggtttcgctgctggatacgctggacgcactggcagagtaccaacgcgcgggaaaaattcgttatatcggcgtgtcgaacgaaactgcatttggcgtaatgcgctacctgcatctggcggacaaacacgatctgccgcgtattgtcaccattcagaacccttacagtctgttaaaccgcagttttgaagtaggtctggcagaagtcagccagtatgaaggggtcgaactgctggcctattcgtgcctgggtttcggcacgctgaccgggaaatatctcaatggtgcaaaacccgctggcgcacgtaatacgctctttagtcggttcacccgctatagcggtgagcaaacgcaaaaagccgtcgcggcgtatgttgatatcgccagacgtcatggcctggaccctgctcagatggcgctcgcgtttgtacgccgtcaaccgtttgttgccagcactctgctgggcgcaaccacgatggatcagctgaaaactaacatcgaaagtttgcatctggagttaagcgaagacgtattagctgaaattgaagcggtgcatcaggtttatacttatccggcaccataagattaacgccggttaaaaccggcgttaaatattaatgacggcgctgccagatccacagcgccgttattgccagcgcaaacagcgcaccgaagccaatgccaatgggcacgaccgggatgcctatcattaccgccagcgagtaaatgcccagcatcaacaacatggcgctgttttcgccaaggttttgtactgcaatcgcattccccgccccgacgctttttttaccccgctcctgtagcaacgcattgagcggaacgacaaaaaagccccccatcacgccaatcagcatcaacaaggcataggctggcagcagctcgtgttgcagggaaaaaatcagtaccaccacgccaatcaaaatcccggctggcatacagcgtgacacggtttccagcgtaactaacttcgctgccgcacctgcgccaaccacgataccaatcgctaccatcgcgttgagataggtgggcgtagcgttatcggtaatgcccagcgccaccggtacccacagcaccaacaggaaacgcagcgtgacacccgctccccagaataaactggtgcccaccagcgaaaaacgcgtttcaccattgcgccatagcgaggtgcaggcattcaggaaactgcgggtcatgttgatgagattccaggactgccccggacgcgccgccgccagtttgggaatgtagatattggcaacgaccgcaccaccgtaggccagtgcgcatgcggccagggcgacgaggacatgccagtcagccagcacaccaccggctacggaaccgagcaaaatcgccgctatggtagaagcttccattaaaccgttagctttcactaacttactacccgtggttaattcgccgagaataccgtatttcgccggtgaataggctgcagcaccaacacccaccagcgtatagccgagaaacggattgataccaaagcagatactggctgcgcccagcagcttcaggccgttggcaaacatcatcacccggcctttggcgaagctatccgccacctgcccgacaaacggcgcaaaaagaatgtaagcacctacaaacaccatttgcaggatgggctggctccactccggatagaactgcgctttcagtaacgccagagtggcaaacagtagggcattatcgccaaacgcagagagaaactgcgccacgataaccgctttcatccccttcgaccacaacgaagtgttagtgtgcactgactcactcatcgtgttgttccgcttcgtctacccagcttttcaacgtgacaaagtcaggtttgccgctgccaagtaatggcatctgtttcagatagcgaatatcgcgcggtacagcaagctccggcacgccgtgctcgcgggcatactgttgcaacttatcgcgcgtcagttcgttatctgtggtgaaaagcaccagtgcctcgcctttgctggcatcgctcttaatcgcagtggcatggactttatctggcgaaacaccaagtgccagttgttccaccatttccagcgacaccatttcgcctgcaattttggcaaagcgttttgcgcggccctgaatctgcacaaagccctgctcgtcaaaacgcacaatatcgccagtgtcataccagccgcgctccatttcgccgcgaacattctcggcggtgggcacttccagtacacctggcttctccacccgcagatagccgttcattatgttcggccctttcagttgcaggcgtccgccctcttcgataccagggaccgacaacaggcgcgcatccattcctggtagaatacgccctaccgtaccgggtttcgccgccatcggtacgttgatagaaacgacaggcgcgcattcggtcacgccgtagccttcaaggatgcgcaggccaaatttatcctgccaaagctgtttggtactttcttgtaatttttctgcgcctgccaccacatagcgtagacgatagaagtcatacgggttggcgaaacgcgcgtagtgaccgaggaaagtcgaggtgccgaacaacacggtgcaactgcggtcatacaccaactccggcacaatgcggtaatgcagcgggcttggataaaggaacacttctgcacctgtaagcagtggcgtaaacaggcctaccgtcagcccaaaggagtgaaacagcggtaacgccgacataaagcgatcgttggtggtgaagtcggcaatcgttttaatctgctcgacattcgccagaatgcttttatggctatggacgacgcctttcggatggccttcagaaccggaggtaaaaaggatcagcgcctcttcttccggctgctgtttaacctgtgccagacgcggcatcagcaaatgagcgaagatccatactttgtcggcagtggtgacatctgcttttaaatcttccagatagacccagcgcacctgagtaagttgctccggcagatgccagagtttgcctttatcgagaaactggcgggaagtgaagatggttttgatttcagccgccgtaatagcactggtcagcccttttaccccggcagtgtagttcatcattgcgggcatgcggcgacgggcgatggccccaaaaatcactgccgcactgatgcctgcattgggcagcattaagccgatgcgttcgccttcaacactgtatttttcaaggatgcgtccaacaaacagcgttttcgtaagcaatttgcgataggagtctggggtaaagttgacgtcttcgacacatttcttcccggctccgaagcggtacattgcactcagtaaagattcgtacagcgtttcacgcgggcgcaccgccattcgcgcttccatcattatttgatgcagcatttcgccagcgattttgcgacggtcacgggcacgcggcgcatccggcatcgccacctgcgttggtggcaaaatatgcagagtaatttgcgggaacaagcgacgtttaaccagacctttcaggcggctgaagtgcgtaagttccgccccttcaatacgcacaggaataaccgttgcaccagacttcgccgcgacaaaacccgcgccatcgtagattttcatcagcgagcctgtcgtggtgatgcgtccttcagggaaaatcaccactggtcggccctgttccaccagacgtaccagatgtttaatagccataggttgcgtcgggtcgagaggaacaaagtcgataaatgatttcagccaacgcatataccactgttggcttattgaggtgtaaacggcaaacactggacgcacaggtaaaaacagtccaagcaaaatgccatcaataaaagagacgtgattaggcgtaattagaacgcgctcgcccttcagtgcctgggtgtcacccgtaacgcgaacgcgatacaaaacacggcacaaatttcgaaaaaagctaaaaagcattccaactccctttgctctgattcagtaaaagcgaatggagggagattacacgagataaagaacgcgagcgacagtaaattaggtgcgaaaaaaaacctgcgcatccgcgcaggttggtgcaagagacagggtacgaagagcgtaccgaataatctcaccaatcaatacctctgggatcttgattgtggtctgcacgacgactcttcgccagcgagaaaacgcaaaggaatgaagggaaatgcaacgaggtgtgtaaattgtcggttactgttacagattgatgaccggcaaaaaaaacctgcgcatctgcgcaggctggtgtaattcatgtgctcaacccgaagttgacttcacctatcaatacctctgggatcaccactttagcaacctgaagccaaacgccaccagcggtcaatcgcaacagcgtttcgcaaagtgtaaccaaaggtttgcaatctctttttttgtcttacttatttgcgtttggctcacattcccacgatgaaaacacgccaccccttgaaccaacgggcgttttccgtaacactgaaagaatgtaagcgtttacccactaaggtattttcatggcgaccataaaggatgtagcccgactggcaggcgtttcagtcgccaccgtttcccgcgtcattaataattcacccaaagccagcgaagcttcccggctggctgtgcatagtgcaatggagtctcttagctatcacccgaacgccaacgcccgtgcgctggcgcagcagaccactgaaacggtcggtctggtcgttggtgatgtttccgatccgtttttcggtgcaatggtgaaagcggtcgaacaggtggcttatcacaccggtaattttttattgattggcaacggttaccacaacgaacaaaaagagcgtcaggccattgagcaactgatccgccatcgctgtgctgcgttggtcgtccatgccaaaatgatcccggatgctgatttagcctcattaatgaaacaaatgcccggtatggtgctgatcaaccgtatcctgcctggctttgaaaaccgttgtattgctctggacgatcgttacggtgcctggctggcaacgcgtcatttaattcagcaaggtcatacccgcattggttatctgtgctctaaccactctatttctgacgccgaagatcgtctgcaagggtattacgatgcccttgctgaaagtggtattgcggccaatgaccggctggtgacatttggcgaaccagacgaaagcggcggcgaacaggcaatgaccgagcttttgggacgaggaagaaatttcactgcggtagcctgttataacgattcaatggcggcgggtgcgatgggcgttctcaatgataatggtattgatgtaccgggtgagatttcgttaattggctttgatgatgtgctggtgtcacgctatgtgcgtccgcgcctgaccaccgtgcgttacccaatcgtgacgatggcgacccaggctgccgaactggctttggcgctggcggataatcgccctctcccggaaatcactaatgtctttagtccgacgctggtacgtcgtcattcagtgtcaactccgtcgctggaggcaagtcatcatgcaaccagcgactaaccgcagttaaagcaattccagcgccagtaattcttcgatggtctggcgacggcgaatcaaccgcgcctgaccattatcaaacagaacttctggtaacagcggacggctattgtagttggatgacattgatgcgccatatgcccctgtatcatgcagtaccagataatcacctgccttcacttccggcaaggcgcgggtttcaacatttcccccttcctgctgggtaaagacatcgcccgattcacataacggtccggcgacgacggtttccaccgttggcgcgtgttccagagaacgaccatcagctgccagggcactgatatggtggtaactaccgtacattgccgggcgcatcagatcgttgaacccggcatcaaccagcacaaagtggcggctccccatttgtttgacgctccgcacctgagtaattaatacgccagactgcgctaccaggaagcgacccggttcaatttccagtttcacagggtggcccaaatggcgggcgatttgctcacgcgcggcattccacagaccataataatgttcggtatcaaccgcctcttcaccctgttgataaggaacagaaagcccaccgcccgcagaaatagcctgtaaatcctgaccgaattcgatgacctgacgcaccatagcaccacacacctgttccagatgggcataatcaacgccagaaccaatgtgcatgtgaatgccgaccagctgcagatgatgacgttgtatcacgtccagtgcggcgggcagatcggtgtaccagataccgtgcttgctgttttcgccaccggtattggttttttggctatgtccgtgaccaaaccccggattaacgcgcagccatacccgatgccctggcgaaacctggcccagttggtcgagcatatcaacagaacccgcattcaccggaatttgcaattcactgacgcgttcaagcgtcgcctgatcgataacatctgccgtaaaaacaatatcatcggggtgcgtttgcggattgtaacccgccgccaacgcacgctctatttcgcctaacgagacggaatccactttcacgccctgctcacgcattaagcgcaaaatatgaatattggaacaggctttctgtgcaaagcgcaccacatcaaactgtttcagcgctgcaatctgccgacgaataatttgcgcatcgtagacccacaccgggcagccaaattcagcgggcaaacgcagcagattttcggcggtgagatcggtatcggtgctgaacagtgaatgtggcataacaaactccagataagtgcttttttatgattacgccacatcataaaaagaataaaaaatatcgatttatgtcgagtctatgcaaaaatgatatggattaccggattgcgagagagcgctaatggccgccgttaacttacgtcatattgaaatttttcatgcggtaatgaccgccggaagcctgactgaggcggcacacctgctacacacctcacagccaaccgtcagccgcgaacttgcgcgctttgagaaggtgatcgggctgaaattgtttgagcgcgtacgtgggcgattacatcctaccgtgcaaggactgcgtctgtttgaagaagtgcaacgatcctggtacggactggatcgcattgtcagcgccgcagaaagtctgcgcgagtttcgccagggagaactgtctattgcctgcctgccggtcttttcgcaatcttttttaccgcagctcctgcaaccctttctggcacgttatcccgatgtcagcttaaatatcgtgccccaggaatcaccgctacttgaagagtggctctcggcccagcgtcatgatttaggactcactgaaacgctccatacgcctgcgggaacagaacgtaccgaattactctctttagatgaagtgtgtgtgttacctccgggtcatccgctggcggtaaaaaaggtattaacgccggatgattttcagggtgagaactacatcagcctttcccgtactgacagctatcgccagttgctggatcagctatttactgaacatcaggttaaacgacgcatgatcgtagaaacccacagcgccgcgtcagtctgcgcaatggtacgggcgggggtaggtatttcggtggttaacccgctcaccgcactagattatgcggcaagcggtttagtggtgcggcggttcagtattgcggttccgttcaccgtcagcctgatccgccccctgcaccgcccgtcatcagcgctggttcaggcgtttagtgggcatttacaagcggggttaccgaaactggtcacttctcttgacgctattttgtcgtcagctacgacagcataaaagcgacagcatcctcggcatggatcgccgcggtatcaaacacaggcaaaacactgcgctcttctggcaccagtaaaccaatttctgtgcagccaaaaatgacgccctgtgcgccctgttctgcaaggcgagcaatcacttgcgcacaataagcgcgtgacgcttcggtaaattgccccagacacagttcttcaaaaataatctgattaattttcgcccgttcatccgcttcaggaataagacaattgatggaaaattgttccgtcagccgcccgcgataaaaatcctgttccatggtgtaacgcgtacccagcagcgccacacgagtcattccggccccggtaattgcacgtccggtggcatccgcaatgtgtaagaaaggcagagtgcaacgtgactcaatggcatccgccactttatgcatcgtattggtacatagcacaataccttctgcgcccgcccgctgtaagccaagcgccgcctcagccagaatgtccccggttttatcccattccccgcgacgctggcactcttctatttcatgaaaatcgacgctatgtagcagcacttgcgcagagtgaagcccaccaagccgctgtttaatgccttcatttatcaaacgatagtaaggaatggtggattcccagctcattcctcccagcaaaccaattgttttcattcctctctcctgatgtgtgttaccgcaacaaggctgaataaggaacgagacaaacgcctcaacggccaagtgcccaatctctattaacgaaaaaagggccggatgtacagcacatccggcccgtgaaatcagacgccgatatttctcaacttctcgcctgccatcagtttgcgttcgatatgttccagcgtgacatttttggtttccggaatgagccagaaagtaatgcccacaaacgcaatgttcagcgcagtgtagagccagaacgtaccggcagcgccaatgctatcaagcagtgtcaggaaggtcgcgccgataatcatattcgacacccagttcgtggtggtcgaacaggtaataccgaaatcgcggcatttcagcggctgaatttcagagcacaggatccacaccactggcgcggcgctcatcgcataaccggcaatacacatcatcgtcatgccaacagagagccaggacaagccactggaagccgtaccgttatcaaactgcatcaggcaatagcccagcaccagagtgcctaacgccatcacgctgaaaccaattttcagagccggtttacgccctgctttatctaccgtaaacaccgcaataaaggtggcgaacataaaggtcagccctacgaccagagtcgcaatcatctgttgttctgtggtcgtaaagcccgccattttgaagatacgcggcgcgtagtacatgatgatgttcataccggtaaactgctgcatcgcctgcaacaacataccgagaaacacagcacgacggacgttacggttgatcttaaacagtgcccaaccgccctgttttaacttcaggctttcacgaatttcgttgagttcttctcgcgctttttccgacgtatcgcgcagcatacgcaatacttcttccgcctcaatatgacgccccttttccgccagccagcgcgggctatttggcaggaagactaccagaataatcagcagaactgctggtaaagcaagaacccccaacattgcgcgccagttaccgctataactgaacgctgtatcggataaaaacgccagcacgatgccgagtgtgaccatcaactggtacatactgatcatcttaccgcgaacgttttcacttgccatttcagaaagatacagaggagcggtgtaagacgcgatcccgacagcaatgcccagcaccacacgagcggcgattaacatctctacgctggtcgcaaaagcggaccctatagaaccgagtacaaacaggatggcccccgccatcaggctgtatttacgccccaggcggaacgacagccaaccattaaacagcgcaccaattgctgcaccgagcatcatgctactaaccacccattcctgcaaacgactggtcagcacaaagtgatcggtaatgaacggcaacgctccggcgattacgccgatatcaagaccaaataacaatcctgcgaccgcagcagctaccgaaacaaacatattcatacgccgcgtatcccgcaaagaacgtggcgttaaagcagattccgtattgatagtaaccattttttcctgccagcagagagtaagacatagtgaaaaaatacgtgaacaactcacgcaggtgtcaggtcggaaacagcataaatatggattaaattgctgcgacatgtcgttatgtgatggatattccaattttcaaattaagttgaattattgagattattattaaccacctaattttacagcagataaaattcataaagttcattaattgataattaatatggattatttcataaccatgatatggattatgatgatctacaggtataaaaaaccctgccatgcggcagggtcataaaagtaagaagaatgaattaacgcgccagccaaccgccatccacggcaatggtataaccattcacataatctgaagcgctggaggcaaggaacactatcggccccatcaggtcactcggcagtccccaacgaccagctggaatgcggtcgagaatttccgcgctacgttgttcatctgcccgtagttgttgagtattgttggtcgccatgtaacccggggctatcgcattaacattaatgttgtgtttagcccattcgttcgccatcaatcgcgtcacacccatcacgccgctttttgatgcggtataagaaggcacacggatcccgccctggaaggagagcattgacgcgatattgataatcttgccgccattgccttgcgcgataaagtgtttcgccgctgcctgagacatgaagaatacgctcttgatattcaggttcatgacatcgtcccagtccttttcgctgaactcgagagcatcttcgcggcgaatcaatccggcgttattcaccaggatatcaatatgaccaaactccgctaccgcgcgatccagcagtgctggaataccatcaatctttcgcagatcggcggtcaggcttaaaaaacgacgccccagcgctgtgacctgctcgatggtttcagtcggttcaacgatgttaatgccaacaatgtcacagcccgcttgcgccagccccaacgccatcccctgacccagtccagtatcacaaccagtgacgaccgcaactttaccttcgagagaaaatgcacttaaaatcataacaataccttattcgtttatgcccacaactagcgcaaatctttaacggccacatggtccatatcatcaaagacctggttttcaccgaccatgccccagataaaggtataagctttggttccgacaccggaatggatcgaccagctcggggagatcaccgcctgctcgttatgcatcacaatatgacgcgtttcttgcggctgccccatcatgtggaaaacgcaggcgtcatcatccatattgaaatagaaataaacttccatccggcgctcgtgggtgtgacacggcatggtgttccacaagttacccggagccagctccgtcagccccatactcaattggcaggtttccagtacatccgggacaaaatatttgttaatcgtgcgacggttactggtgaggttatcgcctaacgtgactggagatacttcgtccggtgtgacttttttggtgggatacgtcgtatgcgcgggtgcgcaattgtaataaaacttcgccggagtgccggtatcaatactggcaaagacaacttcttttgcacctttaccaacatacagggcgtcgcggtgaccgatttcatagcattggccatcgacagtaatcgtaccggcaccgccaatattgataacacctaactcgcgacgttcaaggaaatagcttacgccgagttgtttaccaacttccccgccaacggaaaccgttttagttatcggcataatgccgccaacaataattcggtcaatgtggctgtaaaccatggtgtactcatcggcgacaaataccttttcaaccaaaaattcattgcgcagcccttgggtatccagcgtttttgcgtgcgcactgtggatgctctgtcttacgtccacatcaacctccgataatcagtgaagcgtgaaaatagaaaacgatagtgaaacactgtttcgttttctctataaagggatgatatgcccatgggctagggttttcaattaaaaataaaacaatgtttcatttttaagttaaggattaaaaaaagtgcagtgtcgatcacgaatatgtcatgagaatggaaaaatgagggagcccagaaaatgtatgtcgacttgccagccatcattattcaacagattaatgacggcagatatttatcggtaaggaggaaatgcagagctattcgtcacgttcaatggtcaatgccacaccctggcccccgccgatacaaagcgttgccagtcctttgcgggcattacgtttcaccatttcatgaaccagagaaaccaggattcggcaaccggaagcgcctatcgggtgaccgagtgcgatcgcgccaccattgacattgacccgacgctcatcccactcaagcatcttgccaaccgaaagcgcctgtgcagcaaacgcttcattagcctcgataagatcgacttcagccaactgccagcctacacgctccaggcaacggcgggtcgcatacaccggcgcaattcccatcaatgccggatctacaccaacgctggcaaatgcgcgaatgcgggccagcacgggtaaattcaacgctcgtgctttggcttcgctcatcatcattaccgcagctgcgccatcgtttatggatgatgcattacccgctgtcacagaaccgagactatcaaatgaaggatttaaacgggctaagccttctgcgctggcgtcagtgcgtggctgttcatcggtatcaacaaccaacgtctgcccgttactttgggtcattaccgggacgatctcatctttaaatcgtccggcgtcaatcgccgctcgcgctttttgttgcgagctaagtgcgtaagcatcctgcaactgacggctgatgccatattcgcgagccagattttcggcggtgacaccaatatgataatcattgaaggcatcccacaacccatcatgcacaagactgtcaaccaactggctattgccaagctgtgcaccggtgcggctatcagtcagaacatgtggtgcgcggctcatgttttcctggccaccggcgatgacaatatcagcctcgccacactgtatcgcctgagtagccagatgcagtgctttaagcccggaaccgcaaacgtcattaatagtgattgcagaaacgctattaggcagaccacctttaatagccgattgccttgccggattctgccctgcccctgcagtcaacacctgaccaagaattacttcatccaccgcatatgcaggaacgccggtacgttctattaacgctttcacgaccagactaccaagttccacggcggaatgacccgctaacgcaccacgaaagcagccgataggtgtccgtaacgccccgacaatcacaacgtctttcatcacaacctcgcaccaattaacagtgcaatagtaaatgattgttaattacagttatcttaattgtttaaaaaaagtgatttttatcacaaaggaaatatgcctgagcagcagtcagagacataactggcacgtaaggtttgcaaccactaacccaccaatagaggggtagatagggcgttaatctcccatacttaacctggtttatggtaaattgccctccattttgtttaatttgtagatgatacgttcagataatgtctaatatttggtctaaagaagaaactctgtggagtttcgcgctctacggcacagccgttggtgcaggcacgctcttccttcctattcagttaggttcggcaggggctgtggtcctgtttattactgctctggtcgcctggcctttaacatattggccacataaagccttgtgccagttcatcctctcatcaaaaacatcagcaggtgaagggataacgggcgcggtaacacactactatggcaagaagattggtaatctgattaccacgctgtacttcatcgccttttttgtcgtcgtgttgatatatgcagtggcaattaccaactcacttacggaacagctggcaaagcatatggttattgatcttcgcatccgtatgttggtgagtctgggtgttgtattaattctgaatctcatttttctgatgggacgtcatgccactattcgggtaatgggatttttggtattcccattgattgcctatttcttatttctttccatttaccttgtcggtagttggcaacctgatctattaacaacccaggtagagttcaatcagaatacccttcaccagatatggatatcgattcccgtgatggttttcgcctttagccatacgcccattatttctacgtttgccatagacagacgtgaaaaatatggcgaacacgctatggataaatgcaaaaaaattatgaaagtcgcttatctcatcatctgcataagtgtactgttctttgtctttagctgcctgctttctattccaccttcgtatattgaagctgctaaagaagaaggggtcaccattttatcggcgctttctatgctgccgaacgccccagcatggttgtcaatttccgggattattgtcgcagtagttgcgatgtcgaaatcattcctgggtacgtactttggcgttattgaaggtgccacagaggtcgtcaaaacaacactacagcaggttggtgtaaagaaaagtcgtgcatttaaccgcgcactatcaattatgttggtatcgctgattaccttcattgtttgttgcattaacccgaacgcgatttcgatgatttacgcgatcagcggcccgctcattgccatgatacttttcatcatgcctacgctgtcaacgtatctcatcccggcgcttaaaccctggcgttccatcggaaatctgattacgctgatcgtgggtatcctgtgcgtatcggtaatgttctttagctaatatcagttgtggatggttcaaaattgctacaattttgaaccattccatttttcataatattcatttgttattattccaccctatcacttctctcgtcatatcctagtattatcagttagttaaacacacaaagagatctgaacatcttaaataagactatttaagatgcataacttagattcgcaagatatcttctggtcattcaaaaacaatttgcgatatagatattcttataccatgagatagttatctggaccgctctcaaccatgcaagattaaatcagtgaaacataatcatatttgataacgagaaatgcatttttaaatgccttactcagaattatagcaaatacagattaatcgcaatttttcccggcaaaattacaaaatcatggtgtattgacatcatcaataaccaatgaaattatgcaattatatacggatagggaggttcttaacatggggctttgtagtcgttataaaagtcttacatgcaatagttgctcaatgcattgccaaataatgccagaagagtcaccgcgtttgcagtattgcgcaaactcgtgtttttgtatgtggcccgaagaaagttcatattttaatcgtggtgtggtagaaggtatcttaacaaaaaaccacaatgcgagattaagcggatatatttttgtcgatttttcagtaagttttttacgtctattccttgaaaaagactggattgactatcttgcaagtactgacatggggattgttttagtcagcgaccgcaatatgcaatcgttagctaattactggcgaaaacacaactcagcaatatctgctgtcatatataatgatgatggtcttgatgttgccaatgaaaagatcagacaactatttattggtcgttatttatcatttaccggaggtaacacattaactcagatggaattcaccataatggggtatatggtttctggttataatccatatcagattgctgaagttctggatatggatatccgtagcatctacgcgtacaagcaacgaatcgaaaagagaatgggtggtaaaataaacgaattatttattcgttcacattcggtccaacattgatactcaacgaccagccagaatcatactctgtttatacgggcatttattgaaatgtccgtattttataaataggccgtcccctcaagagtaaacaccatagtatttaaaaccatcacacgaaaaattcagaagcattacgaaatatgaatttacaaacaatagtggcataaatgttaaccatgttaatttacgtaaagttttacgttgcaacattaaagcctcatttcaatcatcatgataaatataaaattaatatatatttatgccgtaaataccaatatacttagcaaactatgtgatctccatttcgattgatttagtgtttattgacgtatgtactggattattaacgataatatcgagttctggcctgagcaccgaaaattaatatcggtacataacgccgatcttaacgtcgttctgacaacgccagccagtcgatgtttatcacttctacttgaagcttttcctgatgtggttgcacaacaagattttttcaccagagtctgggaagaagaaggtatgcgtgtgcctactaacacgttatatcagaacatatccattatcagacgcggatttcgcgctgttggtgatactacccactcgctaattgcaaccgtgccgagaagaggattcaagatccataatgacattaacatacaaaatcatgtaataaactcgtcaacagacgcacatacacacaatgccccacctgccataaaagttaatgcgggatacaaagagagcattggtggcgcaaagaatttcaataacaaaatcctcaaacatataaaaagtcatctaattatgttgagcgcatttgtcataggcgcatattctgcatattggctatggaataataatcaaccgaagccatttttcaaggattacaagactgttgcggaaattaatggctgccattttaatgtaacagaagatacaattgatgggttgaaagagttcgataaatataaaacacggatactggattcggggattaactgtaaaaaacatccgtggttatacttccctcttgcaaaatcctcaccggggatgattgttatggcatgcaataaaaactataaccaacatgaagtggcaaactgtttaaccctgtcttaccgtgaggttaatcgtgattgattataaaaaaaacttattatttattttagtttttatcagtgggtttattctcttcactgtctattcttacactgcagaaaaaatgatatataacgaaacatgcactgcaaattgggtaatttttaatgaccagggacgagcaaatcttaccatcgactttatgtataacaaaaaaaataaaacaggaactgttgcgttgagtggaacctggcaacaaggtaacagagaaagtaaatcaatacggcgaaatattgaatacacatggattgaaaactatgacacagcccatttaacatcaaagaaagttaataagtttgagattatggatcaagttgatgatgatagacttgcacaacttattcctgatttttatgtctttccagaaaaaagtgtaagctataatatactaaagcaaggtaagcatgcttttattttgagcattggtaacagagcaataatgcattgtgcaaggtaaactaaaatagataacaaaaagatggaacctcgttaatcataaaacaataaaattaaatattctcgcagtatatggcagtctaaagcatcaaagatttgatcaacatctttcattttagacatctccttgcaatgtaaaatatcatgtatcaacaacatctggtgcaaatccatgagtcgaactcgacattcatcttagctcgattattattccttcgtacagtcgatgtaaacaatacagaaagaggattattaagaaccagtttactcagtgaatcaatagaggaaaggactaacgtttctttaaaagaattgatttcatcatctgttaaactaaactcatcattgacagatcgtgagatataactgtttttaactttactctttacgttgactttattgacagaattaacattcacatatcttgaatttaatgtccatgatgttgtttgcgtgagaacattctcagcattaaggaatttttttaacggaatccttggtttctttttcgagtccgaatttacaatatcatgcatatagaccatttcatgaatctgcgaaaattcaatgtccattgtatacctcacatttttaccgtgactcgatgttactgttcaataatcaccttccatcaatactaaaattaatacccctaatgtgccgataacaaatatagtcattctacgtaacgtctccataaggtgatatttgacattatcagaagctgcgaattcggattttgctctaatcaaatgagagaaatgtaaaatgaagccacgaaatattaataatagcctaccactgcaaccattagttcctgatcaggagaacaaaaataagaaaaatgaagagaaatccgttaatccagttaaaatcacaatggggtctggtttaaattatattgaacaagaatctcttggaggaaaatatctaacacatgatttgtcaataaagatagcggatatttctgaagagataattcagcaagcaatattatctgctatgagcatatataaattttcgataacagatgatttaatgagtatggctgtaaatgaactcataaaactgaccaaaatagagaataatgtagacctgaataaattcactactatatgcacagacgttctatccccccgcgtcaccagacataataaagaaaaaaacaaacgacattctacccttctcaaaaatcccctttttaattttcattgaaaaaatggcaattgatactatgaatccaggtcatacacattaaggcatttatgtaatgtcgtaattaagataactaataaggtgaatattagtaaaacaactaatgatgttattagtttgtagtgaacagtacttttaccaataatgaaaaatataccataagcaatgcaagcttaaaactcataatttaaaaaagataaatataaaaatatcaatgagtcaatcaataataatttggcatcacgagacacatcacagaggaatattatgagcacagaaacaattgaaatattcaataatagtgatgaatgggcaaatcaactaaaacacgcattatcgaaaggagaaaatctggcattactacatggtttaactcctgatatccttgatagaatatatgcatatgcattcgactaccatgaaaagggtaatataacggacgcagaaatttattataaattcttgtgcatttatgcgttcgaaaatcatgagtatctaaaagattttgcatcagtatgtcagcccaaaaagaaatatcaacaagcatatgacctttacaaactaagttacaattacttcccgtatgatgactattcagttatttatcgtatgggtcaatgtcagattggggctaaaaatatcgataacgcaatgcaatgtttctatcacattattaacaattgtgaggatgatagtgttaagagtaaagcgcaggcatatattgaactcttaaacgataattcagaagataatggctaagcattacaatcatttggttaaatttgctggttatagtgcagttaaccactataaccagcacctcttatgttttcttaaatcagcatcttaaaacagttaagagcatactataaatcattatttttcaatgcgttagagaacaatctactttatcaaaattgaataaggctatttcagattacatcactgaattcctaagataaattagtgaacacaaccatagatatgtcaaatgtaatttcctgtagcgttaatgacacataaatatgaatagccataatttctattgcttaagcaggatgcaagaaaccaattttttcatagaggttaactaatggacttagaaaataaattctcatatcattttcttgagggattaacgctcacggaagatggaattcttactcaaggaaatgagcaagtttatattccacagaaagagttaggtgtattaatagtattacttgaatccgctggtcatgttgtactgaaagatatgatcatcgaatcagtatggaaaaatattattgttagtgacgagtccctgacaagatgtatctattctttgcgctgcatttttgaaaaaattggctatgatcgttgcatagaaacaatctaccggaaaggttatcgtttcagcgggcaggttttcaaaactaaaattaatgaagataatacttcagactattccatagctatattccctttcactacttcattgaatacactggatccattaatacttaatcaggaattagtgcaaatcatttcaaataaaaaaatcgatggtctctatacctatccgatggctgcgacaaatttttgtaatgatcacatatctcaaaattcattcttgagcagattcaagccagattatttcgttacaggaagaataaaccagaataatgcagtgaacactttatacattgagttgatcgacgctaaaaaccttttcctcatcgccagtaatcatctccctgttgatgaactacataatacatcacaatttattatagataatatccttcaaacggtacataaaccagaacgatctgtaagattagctaagcaggaccaaggatataagaatcattatttatcagatgaaatgttagccggaaagaaagaactttacgacttcacccctgaaagcatttacagggccatgactatatttgatagattacaaaataaaagtgatatacagacgctaaaaacagaatgttattgccttctagcggaatgccatatgtctttggcacttcatggaaaaagtgaacttgaacttgctgctcaaaaagcattagagcttttagattatgtatcagacataaccactgtcgatggaaaaattttagctattatgggactgataactggtctgtctggacaagcaaaagtatctcatatcttatttgaacaggctaagatacactcaactgatatagcctctctctactactatagggcactagtccactttcataatgaaaaaattgaagaggcaaggatttgtatagacaaatcactacaactcgaacccagaagacgaaaagcagttgtgataaaagaatgtgtagatatgtatgtgcctaacccgctcaaaaacaacattaaactctactataaagaaactgagagtgaaagccatcgagttataattgacaacattttgaaattaaagcagctgacgagaatttgtatgcgataaatttttattgacgcaattttattatttagatgtatgcaacttgttatttaaacaacagagataaaaatatctaagatattcaccttattgcaagatatttaaaatgctctagagttaaaagtatgatgtaaagaccattggcctggacaattaaaaaagggagctttatgactaatccaatcggtatcaataatttatctcaaagttcaaatatagcgaatgcaacgggtgatgaagtcgtatcattagataaacacatcaacaccagtgctactgatacagatcaaatacaagcatttatagtttcaacatggatggcgccttttcaaaatgatatgtattcagaagataatcctatctcaccttactataaaattgagtggtagacgattgaccaaataaatcataacgagatacttttataatagtatctcgttcctttcattcaatcctcacacatgaaaaaatatgcgctcaccaaaagttaaattcttaaccatcttcacgttttgtatatttattacaaaaatgtctttcgccagcaactcttgctctaatgaagcaggaacaatgttcagaatcgaaccaaatttaattaaagctatcgctcttgttgaaagcaatctaaaaaaggatagcataggcaagaacagagataagaataacaatataaagagtttagattattggttaatgcagataaaccagatgcatattcccctgttaaaaaaacgtggaataataaaagatgaacgagatttgttagataacccttgtctgaacattaaaataggaaccgagattttatataaccatttttcacgttgtggagtaacgtggcaatgcctggggacttataatgcgggttttgcaatggataaccaaaaaaagagacagcaatatgccccaaaatatatattgtatataccaggcttaatgaactagacaatcgtaaggcttcagcaaaatgagcctaaagcctcttttttttatatagtgcaaacacccatacgtaaagctgttttgatcaactcgataccactgtgaacatctaatttcttcatgatattgagtctatgagtttcgactgttttcctgcttaactgcaagaaattagcgatttctttgtttgttttaccatcagctatgagttgtaatatttctgactcacgatttgtaagttgattatcagaggaatacctggaagatattttttcacaatccatatgtacactatcaaaataagtgtaaccattactaatcgaatcaatagcacgatttagtttcgccgggtgactggttttccatacgcatcctttcgcacctgcttcaagcaattttattgaatcaatatacggcatctttgctacaaatgtaataatatgagcatctatcttatgcgatttaacccattttacgagttcggcccccatcattccacctgcaaattctcctaaaataaatatttaggctgtagatttgttacactccgctatagctttcttcagatctttatagcccccaacaacctcatataaatcaggataatgtccgagaaatccaattatcccatcaatcataaacggctgctgatctgaaactacaattttaatttttcccatatattcatcctgagtgtaaatgctttaacgcattcatttataatcatcccttccattattattataagcaaaatccaaagaatacattgatgaaataataatgaaatataattaaaaataaaatttttgcgtaaaaaaataccacaggcattaaaaaatcatgagatgattaaaatattacaattagattatattcaaatcattaaacttgagccagggagctataagtcctcagggcttgccaaaacagaattattcatatccaaagaatgtgtttcaaacattttttcaactaaataatgtctggcttgttcgcagatttcgttaaccttgtcaggggagaaacaatgattattaattaaatattgctcacaattatccacaaattcctgcggactaaattcagcaataaattgatcggtaaaaaacacaaaacgcttatcatcatgaaatgtaatatggacattccatattgatttgtcgacaaaatatgactctacttcaagagacttatctttgaaactggtaggtatatggagatttacaggacctgatattgatggtaattttgttacccaactttcaaaaattttgataaaaacatcaacttcttctgaaggttttaacaatatactcttcagatcgtttatcatgtttattcttttttttcaagttctgagcatagcaagcttatcaagggtataaaattatccatctcatcaataatgccttttgtatagccatcataataaccttgaataaatttttcttctctcttttcctcaatactctgaatttttgcggtggtttcaagaaggattttttctttaagagaaactatttctttcaatccatcagaaatttttcttttaatcacaacaccatttgcaggagattttatcaagctcatctctattttttttcgcataaaatgtaattctctctaaaagtgttgatgcaagtggtaacggcgattgtatgtggtcaacaaaatcaggaaataataaattaaatcgttgctgcattgccaatggttgttgccttatatagggtaacaacgttgaaaaaccacatgtgatgatattgtgatagttagcgatgccgggtttgtatcgtgccttttcatttatttccagcggtatagctgataaataatcccttagtacatcaggaaccttataaaaaaacccgcgttctgcaaacctttctcgataaaagtgacaaccactgagtaaacagatcaatggaagtaaattccaattgtttattggatttgcccctatatttccagacatctgttatcacttaacccattacaagcccgctgccgcagatattcccgtggcgagcgataacccagcgcactatgcggatgccattcgttataatgctcgaacgcctctgcaaggttctttgctgccgttaacccgtctggtttgggcatgatactgatgtagtcacgctttatcgttttcacgaagctctctgctattccgttactctccggactccgcaccgccgtgttcttcggttcaagtcccaacatccgggcgaactggcgtgtttcattagcccggtagcatgaaccattatccgtcagccactccactggagacgacggaagatcgttgccgaagcggcgttccaccgctcccagcatgacgtcctgtactgtttcactgttgaagccgccggtagtgaccgcccagtgcagtgcctcacgatcacagcagtccagcgcgaacgtgacacgcagtctctctccgttatcacagcagaactcgaacccgtcagagcaccatcgctgattgctttctttcacggccactctgcctgtatgtgcccgtttcgatggcggtacagcaggttttcgctcaagcaacagcgcattctggcgcatgatccggtaaacacgtttggcattgatcgcaggcataccatcaagttctgcctgtctgcgaagcagcgcccatacccgacgataaccatacgttggcagctctccgataacatggtgtatacggagaagcacatccgtatcatcagtgtgacgactgcggcggccatccatccagtcatcggttcgtctgagaatgacgtgcaactgcgcacgcgacacccggagacaacggctgactaagcttactccccatccccgggcaataagggcgcgtgcgctatccacttttttgcccgtccatattcaacggcttctttgaggagttcattttccatcgttttcttgccgagcaggcgctggagttctttaatctgcttcatggcggcagcaagttcagaggcaggaacaacctgttctccggcggcgacagcagtaagacttccttcctggtattgcttacgccagagaaataactggctggctgctacaccatgttgccgggcaacgagggagaccgtcatccccggttcaaagctctgctgaacaattgcgatcttttcctgtgtggtacgccgtctgcgtttctccggccctaagacatcaatcatctgttctccaatgactagtctaaaaactagtattaagactatcacttatttaagtgatattggttgtctggagattcagggggccagtctaaacttgctcttttcttctggtgtttatctttgaaagatttgtaggataaataacattaagtaaagccgcatcggcttctctgtaatgtttatctttttccagataacctggggattctccccctaaatcaagctgtaacgttattctttcataacctttatctatgaggtggttcaacctcgttgttgaaagagtttcatccagttcattgactttagcttcgcgtagtaaatcagagacaaaaacagagtctttcttcgagagtaggtttgacaaacgttccagtccagaggtcaccagtgcaacggaagatgtgtttaatcgggcatcttcttcccatgctcaggaatcttccataacatagaaattggctttatccagataagcaatcagcagcgcaaccgactttaatcggtcacctttttgccaatcttcagcgttaatagtaccagtgttgattgcttgtataaggagatcaaggtaaagacctaaagcatcattttgtttatggttccacagctgcggcttgccttcttcctgcacatctgccatcacgggggagttgctgtcaaatcggatatgcacagcattcatttgcacgggaattccatccagtcgttttgggttgctaatgacgtcctgcatccgcttaatctggtcgggcgtagacatataatcccacagggtgagcagaaccttttttgcggctacactatttccctgatctgatactaatgccatatagccccataaactatccctcaaccagacagcatcatagtgggtttctgccgctgttttgtcatcttcgaaagtagaagcaagaataaacgttccccagggtttctccgtcaacgttaactttcgtgtgttttctgttaatgttagcaatccttgaatttcgtctttggtatagtggctctttatttcattttgtaatttggctgagtgaatcagaagacgataattaggatacttatctggatttaacgataaataacttttatctgttgctgcccccgtggaattaagaatgttaaatacagattcactcgtcacttctgcccctgtcgcctggcatgtgccgcacgaaaatataccagcgagcagaagagttaatgcagatttccctttcataaaatattccatcaatcgtttgttaaaagcgtagataaccacttatttaacaacttgaaaataaggtgttttacctgggttgttacaaaaggattgcattgcgtaaacgctttttatttacaacaaaatggggaagtattacggcgaagataaattggagcgggcgaagggaatcgaaccctcgtatagagcttgggaagctctcgttctaccattgaactacgcccgcttcgagatgcgtaaggcattataaaccttacgctctccttagcaagtgccacgctgctgactgctgattaattcgccatcagcattttggcttgctgccctgaggcggcaagtaacgtagcggatcaattgccgttgcacggtaacgaatctggaaatgcaggcgaacagatgccgcatccgtgctccccatagtggcgattttttgcccagccttcacgctttgcccattatttaccagcatcgtgtcattatgggcgtaagccgtaatgtaatcttcactgtgtttaatcatgatgagattaccgtagccacgcagctggttgcccacatacaccacctttcctgcacccgcggcgtaaataggtgtaccccgtggagctgagatatcaatccctttattgccgccatctgctgtcgaatacggcatgataactttccctgtcgttggccataaccaacaacgttgccctactggcggccaggatgatttcggtaccgctgatgacggtgtaaccgatgcggttttggtcgttgatttggcggttgatttacgtgtaatactgctacttttcgccccacccagttttagtttctgaccaacttcaatggtgtaagggggggaaatgccgttcagtcgcgccagttcttttacgctggttcccgtggtgcgcgaaatacgatatagcgtatccccccgtttcacggtgtaaacggagccggaatacgttcctgtatcggatgatttgctacccgaacagcccgccaaaagcagtccaaccgataacaacatcacgatacccagagattttttattcaggcgtcccgcactcaaaatctttcctcgcttaaaaaacaagacgccttatcatagcagccagcctcttgatacccaatctcttgcttctggaaaaacgtggtaatagagaaagaggttaatttcatttggcaaagggaagtatcatcagcaaaatattcgctgtagaggtatcgaacttcctgactttttaccctatttcccatcctgatgcgtaataatcccaatttatcacattgattttatcgccactcatattgatacgtatcactgcccctattcagagtcctgtttcgtatcatatctgtgtttttttaacgtcatcacacttcctacctcccctaacgcttatcgtcgtttctggcgtaaatcttgcctgcttagactaaatctttgccataagaaccaaatgttcaaatcgaggggatttctatggaagcgcgggaagcaaccgctacgggtgaatcatgcatgcgcgtcgatgccattgctaaggtcaccgggcgggcacgatatactgacgattatgttatggcgggcatgtgttatgcgaaatatgtacgtagccctatcgcacatggttatgccgtaagtattaatgatgaacaagccagaagtttgccgggcgtactggcgatttttacctgggaagatgtgcctgatattccattcgctacagctgggcatgcctggacacttgacgaaaacaagcgcgataccgccgatcgcgcactgctaactcgccatgttcgtcatcatggtgacgccgttgccatcgtcgtggcccgcgatgaactcacggcagaaaaagcggcgcaattggtcagcattgagtggcaagaattacccgttatcaccacgccagaagcggcgctggcagaagacgctgcaccaatccataacggtggcaatttactgaaacaaagcacgatgtcgacgggtaatgtccaacaaacaatcgatgccgccgactaccaggtacaggggcactatcagacccccgttattcaacattgtcacatggaaagcgtaacatcgctggcgtggatggaggatgactcgcgaattaccatcgtttccagcacccagatcccgcacattgttcgccgcgtggttggtcaggcgctggatattccctggtcatgcgtacgagtcatcaaaccatttgtcggtggcggttttggtaataaacaggatgtactggaagagccaatggcggcattcctgaccagcaagcttggcggcattccggtgaaagtttcccttagccgtgaagagtgtttcctcgcaacccgtacccgccacgcttttaccattgacgggcaaatgggcgtgaaccgcgacggaacattgaaaggttatagtctggatgttctgtctaacaccggcgcttatgcatctcacgggcactccatcgcttctgcgggggggaataaagtcgcttacctttatcctcgttgtgcctacgcttacagttcaaagacctgctataccaacctcccctcggctggtgcgatgcgtggttatggcgcgccacaagtcgtatttgccgttgagtctatgcttgatgacgccgcgacagcgttaggtattgatcctgttgaaattcgtttacgcaacgccgcccgcgaaggagatgctaatccgctcacgggcaaacgtatttacagcgcagggttgccggagtgtcttgaaaaaggccggaaaatctttgaatgggaaaaacgccgtgcagaatgccagaaccagcaaggcaatttgcgccgcggcgttggcgtcgcctgttttagctacacctctaacacctggcctgtcggcgtagaaatagcaggcgcgcgccttctgatgaatcaggatggaaccatcaacgtgcaaagcggcgcgacggaaatcggtcagggtgccgacaccgtcttctcgcaaatggtggcagaaaccgtgggggttccggtcagcgacgttcgcgttatttcaactcaagataccgacgttacgccgttcgatcccggcgcatttgcctcacgccagagctatgttgccgcgcctgcgctgcgcagtgcggcactattattaaaagagaaaatcatcgctcacgccgcagtcatgctacatcagtcagcgatgaatctgaccctgataaaaggccatatcgtgctggttgaacgaccggaagagccgttaatgtcgttaaaagatttggcgatggacgctttctaccaccctgaacgcggcgggcagctctctgctgaaagctccatcaaaaccaccactaacccaccggcgtttggctgtacctttgttgatctgacggtcgatattgcgctgtgcaaagtcaccatcaaccgcatcctcaacgttcatgattcagggcatattcttaatccactgctggcagaaggtcaggtacacggcggaatgggaatgggcattggctgggcgctatttgaagagatgatcatcgatgctaaaagcggcgtggtccgtaaccccaatctgctggattacaaaatgccgaccatgccggatctgccacaactggaaagcgcgttcgtcgaaatcaatgagccgcaatccgcatacggacataagtcactgggtgagccaccaataattcctgttgccgctgctattcgtaacgcggtgaagatggctaccggtgttgcaatcaatacactgccgctgacgccaaaacggttatatgaagagttccatctggcaggattgatttgaggataacatcatgtttgattttgcttcttaccatcgcgcagcaacccttgccgatgccatcaacctgctggctgacaacccgcaggccaaactgctcgccggtggcactgacgtactgattcagctccaccatcacaatgaccgttatcgccatattgttgatattcataatctggcggagctgcggggaattacgctggcggaagatggctcgctacgtatcggctctgcaacgacatttacccagctaatagaagatcctataactcaacgtcatctcccggcgttatgtgctgcggccacgtccattgctggaccgcagatccgtaacgtcgctacctacggtggaaatatttgcaacggtgccaccagcgcagattctgccacgccaacgctaatttatgacgcgaaactggagatccactccccgcgcggtgttcgtttcgtcccgattaatggctttcacaccgggccgggcaaagtgtctcttgagcatgacgaaatcctcgtcgcctttcattttccgccacagccgaaagaacacgcgggcagcgcgcattttaaatatgccatgcgcgacgcaatggatatttcaacgattggctgcgccgcacattgccgactggataacggcaatttcagcgaattacgcctggcatttggtgttgccgcgccaacgccgattcgctgccaacatgccgaacagactgcacaaaatgcgccattaaacctgcaaacgctggaagctatcagcgaatctgtcctgcaagatgtcgccccgcgttcttcatggcgggccagtaaagagtttcgtctgcatctcatccagacgatgaccaaaaaagtgattagcgaagccgtcgccgcggcggggggaaaattgcaatgaatcacagcgaaacaattaccatcgaatgcaccattaacgggatgccttttcagcttcacgccgcaccaggcacgccgctctcggaattactccgcgaacaaggactgctaagtgtcaaacaagggtgctgcgtgggtgaatgtggtgcctgtacggtgttggtcgacggcacagcaatagacagttgcttataccttgccgcctgggctgaaggaaaagagatccgcacgctggaaggtgaagcgaaaggcggaaaactttctcatgttcagcaggcttatgcgaaatccggcgcagtgcagtgcgggttttgtacgcctggcctgattatggctaccacggcaatgctggcgaaaccacgcgagaagccattaaccattacggaaattcgtcgcggactggcgggaaatctttgtcgctgcacggggtatcagatgattgtaaatacagttctggattgcgagaaaacgaagtaaaaggatatccggcctgaattcaggccggattcactgaggttatgtgtttaacaactcatatttcttaatcttgcgatagagcgtagcaatgccgatgcccagttcatcagcaacttgcttcttgctgttatgacgtgaaagcgcctcgcggatcatttgcttttccatctcctccagcgccgtgccgcccgcatcatcgagtgacaggtgcgcctcactgacctctgttacatcactttgctccgttgtgccattattcagcagatttggcggcaatagcgtgctgtcgataacttcacctgaaggaaccacgttaaccagatattccatcaaattgcttaactcgcgcaggtttccgggccaacgatgcttacgcaatatttcgacgacatcgggagcaatgccaggataaaccgatcccagacgacgggtatgcagatgtaaaaagtaatgcaccaatagttcaatatcttcctgacgttcacgcagcggtggcagagttatcgggataacattaagtcggtagaagagatcttcgcggaatttaccttcggcaatgaactgggccaaattctgattagttgcagaaatgatgcgaatgtcgacttgtattgggctactggcaccaatcggcagaatttcacgtgcctcaatagcgcgcagtaatttagcctgcaacattaatggcatatcacctatttcatcgagaaacagcgtgcccgtattcgccgcctgaatcaaccctgttttaccgttggcagaagcgccagtaaatgcacctttaacataaccgaacagttcgctctccagaagctgctccggaatcgcggcacagttgatagcaataaagggtttattccgtcttccgctcaacttatggattgcacgggcgacgacttctttacccgtgccgctttcaccaaccaccataacgctggatgggctgggtgcaatacggctaatgagtcgttttaattgccgcataacacggcactcgccaaccaattgttcaatatgcggttcatcaggtgcatttgctacagaaaaactggtatgcgattggtgaaacgccattaaaaataattgtcggccctgaatgttatgcaattgaccaatgattaattcacttttatcgtcccatgaaacaatatgctgcatatgtccatgggtaaaattactctcaaatgttaatggtctgaaacggataggtttcccaataatattattttgcacaacaccaagtgtttttaaggcagtctgattaacaaactgaacccgattttcatcatctacaactaatacgccctgatccatattatcgatcatggtcgcaaatattttactgatgttatctcctggcccctgatcctccagaagtttcgaaacaaaaatggtggatatatggcgaacataatcagaaaattcgcgtaaattatcactgatatgctcttgttgctcgtgggtaacggcaatcaaacttatcaccccaacacaacgatcctgtaaaatgacaggcgtacccagaaatgctttttcgcggcaattttctttactatcgcaaccttcgcaaaggggatcgaagcgagactgtgtcacaactttttcagttttcgtttccaggacgtggcggagcaggcgtgagttgccgctcaactggcgaccaagaaacttcccatacgcgcccgttccggcaacgcgacacaagttttcatcaacgatctcaacctcaagctgcaaaacgctggcaagcattctggcaaaacgctgaattgtcggttgaatttgcatcaatactgactgcgtagtagcaagctccatagctttaccttccagacttacttaaaagtcgatcattgaagacgttgatggttcacagatcatgatgatattaactcaggcgaaattggctttgataaaaacataagatttttatcattttctaatgaaattatggaagagatatcacatttctatatcaatatgagaattacggcggtgagtttatcaaactgaagagagatagcctgcccctttatcttatttctgatacttagcagcaaataaataacgcgataaaaaaagccaaacgttttcgtattttacaaacaaccagaagctggcatcaatttgtgatcaaccccacacattatccgtcaaattagtcttttgcagccgcgcggataattctggcacacttattgttagtcccaggtatagctgtgaaaacaccaatcactttggcaagtcacagtgaaataaaccactttgcctgtcattccactaccgggactttatgatgaaaactgttaatgagctgattaaggatatcaattcgctgacctctcaccttcacgagaaagattttttgttaacgtgggaacagacgccagatgaactgaaacaagtactggacgttgccgcagcattaaaagcactgcgtgctgaaaacatctcaaccaaagtctttaatagtggattaggtatttccgtattccgcgacaactccacccgtacccgcttctcttatgcttccgcgcttaacctgctcggccttgcacaacaagatctcgacgaaggcaaatcacaaatcgctcacggcgaaaccgtgcgtgaaaccgccaatatgatctccttctgcgccgacgctattggtattcgcgacgatatgtatctgggcgcaggcaacgcctatatgcgtgaagttggcgctgcacttgatgacggttacaagcagggtgtactgccacagcgtccggctttagtgaacctgcaatgcgatattgaccacccgactcagtcaatggctgacctcgcgtggttacgtgaacactttggttcactggaaaacctgaaaggtaaaaaaatcgccatgacctgggcctactctccaagctatggcaaaccgctctctgtaccacaaggcatcatcggtctgatgactcgcttcggtatggatgtcaccctggcccatccggaaggctacgacctgatcccggatgtggttgaagtggcgaaaaacaatgctaaagcctccggtggtagcttccgtcaggtcaccagcatggaagaagccttcaaagacgcagacatcgtttatccgaagtcatgggcaccttacaaagtgatggaagagcgtactgaattgctgcgtgcgaacgatcacgaaggcttaaaagcactggaaaaacagtgtctggcacagaacgcgcaacacaaagactggcattgtactgaagagatgatggaactgacccgtgatggcgaagccctgtacatgcactgcctgccagctgatatcagcggcgtatcctgtaaagaaggtgaagtgactgaaggcgtattcgaaaaataccgtatcgctacctacaaagaagccagctggaagccttatatcatcgccgcgatgatcctgtcccgtaaatacgccaaaccaggtgcactgctcgagcaactgctgaaagaagcgcaagaacgcgtgaaataacccctcgggccgatcagctggtcggccctctatttccagaggccaaaaggataggatatgtccgttttctcattgaagattgatatcgccgataacaaatttttcaacggcgaaacatcaccgctcttttcgcaaagccaggccaaactggcgcgccagttccaccagaaaatagctggttatcgcccaacaccgctttgtgcgctggacgatctcgcaaacctttttggtgtgaagaaaattctcgtcaaagacgaatcaaaacgattcggtctgaacgccttcaaaatgcttggcggtgcgtacgccatcgctcaattattgtgtgaaaaatatcatcttgatatcgaaacgctgtcatttgagcacctgaaaaatgccatcggcgaaaaaatgactttcgcgaccaccaccgacggcaaccacgggcgcggtgtggcgtgggcagcacagcaactcggacagaatgcggtgatttacatgccgaaaggttctgctcaggaacgcgttgacgccattctgaacctcggtgccgagtgcatcgtcacggatatgaactatgacgataccgttcgcctgaccatgcaacacgcgcagcagcacggctgggaagtggtacaggacacggcatgggaaggttacaccaaaatcccaacctggatcatgcaaggctacgcaaccctggcagatgaagccgtcgagcaaatgcgtgaaatgggcgtaaccccgacgcacgttctgctgcaagccggtgtcggagcaatggccggtggtgtgctgggttatctggtcgacgtctatagcccgcaaaatctgcacagcattattgttgaacctgacaaagctgactgtatttatcgctccggcgtcaaaggcgacatcgtcaacgttggcggtgatatggccaccatcatggcaggcctggcctgtggcgaacctaacccgctgggctgggaaatcctacgtaactgcgccacccaattcatctcctgccaggacagcgttgccgcattaggtatgcgcgtgctgggtaatccgtacggcaacgacccgcgcatcatctccggtgaatccggcgctgtcggtttgggcgttctcgcagcggttcattatcacccgcaacgtcaaagcctgatggaaaaactggcgctgaacaaagatgccgtggtgctggttatcagcactgaaggcgacaccgacgtgaagcactaccgcgaagttgtctgggaaggcaaacacgctgtagcaccttaatcaccctattggaactgctccctgcaaaacggggagtaaaaaatctggagaaaaataatggctaagaatattccattcaaactgattcttgaaaaagcaaaagattaccaggcggatatgactcgcttcctgcgcgacatggttgctattcccagtgaaagctgcgacgagaaacgcgtagtacatcgtattaaagaagagatggaaaaagtcggcttcgataaagttgaaatcgacccgatgggcaacgttctcggttatatcggccacggcccgcgtctggtggcaatggacgctcatatcgataccgtcggcattggcaacatcaaaaactgggacttcgatccgtacgaaggcatggaaactgatgaactgattggtggtcgcggtacttccgaccaggaaggtggcatggcctctatggtttatgccggtaaaatcattaaagacctcggtctggaagatgaatataccctgctggttaccggtacggtgcaggaagaagactgcgacggtctgtgctggcagtacattattgaacaatccggcattcgcccggaatttgtggtcagtaccgaaccaaccgactgccaggtataccgtggtcagcgcggtcgtatggaaattcgtattgatgttcagggtgttagctgccacggttctgcaccagaacgcggtgataacgccattttcaaaatgggtccgattcttggcgaattacaagaactctcccaacgtctgggttatgacgaattcctcggcaaaggcaccctcaccgtttctgaaatcttcttcacatccccaagccgttgcgctgtagcagacagctgcgcagtttcaatcgaccgtcgtctgacctggggcgaaacctgggaaggcgcgctggacgaaatccgcgccctgcctgcagtacagaaagctaacgcggttgtttctatgtacaactacgaccgtccgtcctggactggcctggtttacccaaccgaatgctacttcccgacctggaaagtggaagaagatcacttcaccgttaaagcactggtgaatgcctacgaagggctgtttggcaaagcgccggttgttgataagtggaccttctcaactaacggcgtatctatcatgggccgtcacggcattccggtgatcggctttggcccgggtaaagaacctgaagcgcatgcacctaacgaaaaaacctggaaatctcacctggtgacctgtgccgcgatgtacgctgcaatcccgttaagctggctggcaacagagtaattactcttcacttattcccctccggttcgccggagggtttttggagtttgctatgcgcgtattgatcaaaaacggcactgtcgttaacgcagatggacaagccaaacaggatttgctgattgaaagcgggattgttcgccagttgggcaacaatatttcgccgcagctcccgtatgaagaaattgatgccactggctgttacgttttccctggcggcgtggatgtccatacgcatttcaatattgatgtcggcatcgcgcgcagttgtgatgatttttttaccggtacccgcgcagctgcgtgtggcggtacaacaaccattattgaccatatgggatttggcccaaacggctgtcggttacgccatcaactggaggtttatcgtggttatgccgcccataaagcggtcatcgattacagctttcacggtgtgatccagcacattaatcacgcaatcctcgacgaaatcccgatgatagtcgaggaaggactgagcagttttaaactctatttaacctatcaatacaaactcaacgatgacgaggttttgcaggcattacgccgcttgcatgaatccggcgcgctgaccaccgtgcacccggaaaatgatgcggctatcgccagcaagcgggcggaatttatcgccgcagggttaaccgcgccgcgctatcatgccttgagtcgccctctggaatgcgaagcggaagccatcgcccgcatgattaacctggcacaaattgccggtaacgccccgctctatatcgtgcacctgtctaacggcttaggtctggattatctgcgtcttgcccgtgcgaatcaccagccagtctgggttgaaacctgcccacaatatctcctgttggacgaacgcagttacgatacagaagatggcatgaagttcattcttagcccaccgctgcgtaacgtacgcgagcaggacaaactgtggtgtggcatcagcgatggtgcgattgacgtggtggcaaccgatcactgcaccttctcgatggctcaacgcctgcaaatttctaaaggcgatttcagtcgctgcccaaatggcttacccggtgtggaaaaccgcatgcagttactgttttccagtggcgtgatgacgggacgtataacaccggaacgctttgttgaattaaccagcgcaatgcccgccaggttgtttggcctgtggccgcaaaaaggattattagcgcccggttccgacggcgacgtggtgattatcgacccacgtcagagccaacaaattcagcatcgccatctccacgacaacgccgactactcgccatgggagggttttacctgtcagggcgcgattgtcagaaccttatcccgtggtgaaacgattttctgtgacggcacctttacaggcaaagccgggcgaggtcgtttcctgcgacgcaaaccgtttgtccctcccgtgctctaaccactgccagggatctatacacaatcaagaatgatgagtgaggaaaaatgagtaagaaaattgttctcgccctgggcgggaatgcgctgggcgatgacctggccgggcaaatgaaagcggtaaaaattacttctcaggcaattgttgatttaattgcccagggacatgaagttatcgtcactcatggtaacgggccgcaggtgggcatgattaaccaggcctttgaagctgccgcaaaaactgaagcgcactcgccaatgctgccgatgtctgtctgtgttgcattaagccagggttatattggttacgatctacaaaacgctttaagagaagaactgctttctcggggcattaataaacctgtagcaacgctggttactcaggtcgaagtcgacgctaacgatccggcattcctcaacccgaccaagccgatcggttcgttctttaccgagcaagaagcagagcaactgacaaaacagggttacactctgaaagaagatgctggtcgcggctatcgccgtgttgttgcctcgccaaaaccggttgatatcattgaaaaagaaacggttaaagctctggtagatgcaggtcaggtggtgatcaccgttggcggtggtggtatccctgttattcgtgaaggtaaccatctgcgtggtgccagcgcggttatcgataaagactgggccagcgcccgtttagcagaaatgattgatgccgatatgctgatcattctgactgcggtagaaaaagtggccattaacttcggtaaagagaatgaacagtggctcgatcgcctgtcattaagtgatgctgaacgctttatcgaagaaggtcattttgcgaaaggttctatgctgcctaaagtggaagctgccgcctcgtttgctcgctctcgcgcaggtcgtgaagcactgattaccgtattgagcaaagcgaaagaagggattgaaggcaaaacaggaacggtgatttgtcagtaatttaaaggccgggtgggtaataccatccggccaaagattgtcaagtaagtgcgctttgttgatgccggatgcggcgcgagcgccttatccgtcctacaaaacatcgcaaattcaatagattgcaatgcacttgtaggcctgataagcgtagcgcatcaggcaatttggcgtttgtcatcagtctcaggccgggtgggtaataccatccggccattttcatttaagccacttccagcacttcttttgtcgctttcacgccctgatgcatcaacatcattaacgcctcaagtacgccgccgccaatcgcccgggctttatcagaaacgctggtgaaatcagcggtttcaccacgaggatcgatatcaccaattttaaaaccaccaaccactgccaggccgtcgttcaacaagccacgcaccatccccgtcaacggtgctttaatttcatgctcaccaatccaggcaatcacatcgccctctttcaccagatcgcctaatttcacgttggatcgcataatgcctgcagcaggagcacggatcacccgtcgggtggtatgccccataatattgccaggaacaccggtattctcctgcgcacaaccagagtaaatcacctgaccgagccagtgcccgcgatttgtttcaattaccgcatgacaatccttcccagcagtaaagcccggcccaagcgcgattgttactggtgccatatctgcccgcgttcccaaattctgtttcgccagaatagcgtccaccacgcaaagcggtttcagttcatcaagcaatgaacaggcgggatctaccatcacaggaatgaatccgcgttcggtaagtttcatcgcttccgcagagctggttgccaggcgagcagtgacgccttcgaccgtcatttcgccatcgaacacggcctgggcaaacgccacggtacaacgaatcactgtcggtttttccacttccagcatgatcactttaaaacccgcatgatacagacgtagcgccacaccactggcgatatctcccgcaccgcgaatcaccaccagctggtgtccggaaggatgagaaggtttcatcatcagcccacccggcgcgttatttttcacctgtaatatttctgccagcacgctgatggcgatctcctgcggcgtttccgcacctatgttgtaaccaacgggcgcatgtaaacgggcaatatgttcttcagccacgcctttctcacgcaattgacgcaggaaaagctgaaccttgcgacgacttgccagcaaccccaaccatgcaatgggctgttcaatgagtttgtcgagggcttcacgatcctgattattcgtggcaatcaggacaaaattatcagggcgaatatccagtgcttccactgccgcaccaaacgactcagcatggagaagcgtggttgatggtgggaatagttcaggattgaggctttcgcgataaatatcagcaacggcaatatcaaatcctaatagcgccgcactctgggctatcgcccggttgacatgccccgcgccaatcaacaccagacgtggacgcataccatggacgctgataaatactgacattgcacctccacaatctgacccgacagcatccgcaccgttacgagccatacgtccatggaataatcgcggcttacgttcctgcaatgcctgaagcgactcttcaatcaccttccgctcaaccattccgccaccaattgtaccgacgatagaaccatcggcgcgcactaacatttgtgcagaatggcggggagtcgagcctcggctatcaacaatttgcgccatagcaaacggacaattttgctcttcgagttttgcagcctctgtgaaaatattcataccaacctcaatggatatcctttcagtaacccggaatacccgggccgctaattcacaaatctgcgcgcgattgcaggatgttcttgtatatcgcccagccagattgcctctacgtcgtgttgttgcagcggttgaaggagctcgctttgtgcaatcgcattctcacattgagaaaaacggttaatgaaccagactcgccgacaaccttgcggtacgtttttaaacgccccctgagggtggcgaaccagcgcaacgagatcgctcagttgcaaggttgcatcaggtgttaacccggtaatatcagcaaactgcgaccagcgatggacattttctgtgctcactttcgcgcccaaagtatgtcctcccatcacagcaatcacgcagcaactgcttttgggtatgcaaggttcgtgctcatcaggcgcttttaacggcattccacgcgagccatctgcttcaatgagaattacgtcacactctggtcgttgcaccagtgcatcaatcgcttctggcgtaaatccctgcacttttccctggttcgctttccagctgtgaaaacaaaatgaaatgggggatgtaagagacgcatgaggaagcatggcgggatcacgacagaaaaccacgggccagtgagacgttggcataaacatatgtgtcgtcgtcgtgattaacacacgcctgccgctagcctggagcagttctgccagccaaaaaagcaagctggttttccccccagcaccaacaacagaaatcacagtgggacgtttctgcgcacctaaatcaatgactaatgccgatgggtcaactatacttttcacgagtctttatgacctctctgggataaattatccccaacttaatccatcaggaagtaacgcaattatcaggcgttattagcccctataaataatggaaccactatgtcagccatcgactgtataattaccgctgccggattatcatcaagaatggggcaatggaaaatgatgttaccctgggaacagggaacaattcttgatacaagtatcaaaaatgcgttgcagttttgtagccgaattattttagtcaccggctatcgtggtaatgaactgcacgaacgttatgcgaaccagagcaatatcactattattcacaacccagattatgcgcagggtttactaacatccgtcaaggccgcagtacccgcagtgcaaacagaacattgttttctcacccacggtgacatgccaaccctcaccatcgatatttttagaaaaatctggtcgttacgaaatgatggcgcaatactgccactccataatggcatccccggccatccgattttagtgtcaaaaccatgcctgatgcaggcaatccaacgacccaatgtcaccaatatgcgtcaggcactccttatgggagatcattattccgtcgaaatagaaaatgcagaaataattttagatattgatactccggacgactttattacagcgaaggaaaggtatactgaaatttagaaaacgtagttaaacgattgcgttcaaatatttaatccttccggcactcattatcataatgataaggaatcactgattttgagaaaagagaaaaattgataaatgggctggcaataataattttcaggagtgattttaattctcatttagcacctgtgagttcattcacaaaaagcccttaagtttcgagccgcctcacatttttttatatttcccgccaaacctggcaagagtggtgcgattgttgctctatccccctaaaccaccggatttctcaacaccggtcactcaatgatatctgtataagctaaggagagggttatgggggatattatgcgtcccattccgtttgaggaacttttgacgcgcatatttgatgaataccaacaacaacgctcaatctttggtattcccgagcaacagttttactcacctgtaaaaggtaaaactgttagcgtcttcggtgaaacctgtgccactcccgtcggccctgccgctggcccgcacacgcagctcgcgcaaaatattgtcacttcctggctgactggcggacgcttcatcgaactaaaaaccgtccaaattcttgaccgcctggagctggaaaagccctgtatcgatgccgaagacgagtgctttaacaccgaatggtctaccgagtttaccctgcttaaagcctgggatgaatacctcaaagcctggtttgccctgcaccttctcgaagcgatgttccagccttctgattccggtaaatcgttcatctttaatatgagcgtcggttacaacctcgaaggtattaagcaaccgccgatgcaacagttcatcgacaatatgatggacgcatctgaccatccgaaattcgctcaatatcgcgatacgctgaataaattactccaggatgacgcatttttagctcgccacggattgcaggaaaaacgcgaaagcttgcaagccttacccgctcgcatccccaccagtatggtgcatggcgtcaccctctccaccatgcacggctgtcctccgcatgaaatcgaagccatttgccgctacatgctggaagaaaaagggctcaacacctttgtgaaacttaacccgaccttactggggtacgcgcgtgttcgtgagatcctcgatgtctgcggtttcggttacataggcttaaaagaagagtcatttgatcacgacctcaagctgacgcaagcactggaaatgctggaacgcctgatggcactggcaaaagaaaaatcactcggctttggcgtaaaactgactaacactctcggcaccatcaacaataaaggcgcactgcctggtgaagagatgtatatgtcaggccgtgcgctgttcccgctctccatcaatgttgcagcagttctctctcgcgcctttgacggcaaactgcccatttcttattccggtggtgccagtcagctgactatccgcgatatttttgatacaggtattcgccctattactatggcaaccgacctgctgaaacctggcggctatctgcgcttaagtgcctgcatgcgcgagctggaaggctccgacgcctggggacttgaccatgttgacgtcgaacgactgaacagactggcagcagatgcgttaaccatggaatacacccagaaacactggaagccagaagagcgtattgaagtggcagaagacctgccgctgaccgactgctacgttgccccctgtgttactgcctgcgctatcaagcaagatattccggaatacatccgtctgcttggcgaacaccgctatgccgacgcgctggaactcatctaccaacgcaacgctctgcccgccattaccggtcatatttgcgatcaccagtgccaatacaactgtacccgcctggattacgacagtgcgctgaatatccgcgaactgaaaaaagtcgcgctggaaaaaggttgggatgaatataagcaacgctggcacaaaccagccggttctggttcacgccatccggttgccgtgattggtgcaggtccggcgggtctggcagcaggttacttccttgccagagcgggccatccggttacgctgtttgaacgcgaagccaatgcgggcggcgtggtgaaaaatatcattcctcagttccgtattcctgcagagttaattcagcacgatatcgattttgttgccgctcacggcgtgaaatttgagtatggctgctcacccgatttaaccattgagcagttaaaaaatcagggcttccactatgttctgattgccaccggcactgataaaaatagcggtgtgaaactggcgggcgacaaccaaaatgtctggaaatcactccccttcctgcgtgaatacaacaagggtacagcgctcaagctgggcaaacatgtggtcgttgtcggggcgggtaacaccgcaatggactgcgctcgtgcggcgttacgcgttccaggcgtagaaaaagcaacgatcgtttaccgtcgttcactacaagagatgcccgcatggcgcgaagagtatgaagaagcgttgcacgacggcgtagagttccgtttcctgaataatccggaacgtttcgatgctgatggcaccttaaccttgcgcgttatgtcgcttggcgaaccggatgagaaaggtcgtcgtcgtccggttgaaaccaatgaaacagtaacactgcttgtagacagcctgatcaccgccattggtgaacagcaggatactgaagccctgaatgcgatgggcgtgccgctggacaaaaacggctggccagacgtcgaccataatggcgaaactcgtctgactgacgtctttatgatcggcgacgtacagcgcggaccatcctccattgtcgctgctgtcggaaccgcgcgtcgggcgaccgatgccatccttagtcgggaaaatatccgttcccaccagaacgataaatactggaacaacgtcaatccagcggaaatctatcaacgtaaaggcgatatctctatcacgctggtgaacagtgacgatcgtgacgcgtttgtcgcccaggaagccgctcgctgcctcgaatgtaactacgtttgcagcaagtgtgtggatgtctgcccgaaccgcgccaacgtctccattgcggtcccaggcttccagaaccgtttccagacgctgcacctcgacgcttactgtaacgaatgcggcaactgcgctcagttctgtccgtggaacggtaaaccgtacaaagacaaaatcaccgtcttcagcctggcgcaagactttgataacagcagcaacccaggcttccttgtggaagattgccgggtacgagtacgtctgaataaccaaagctgggtgttaaacatcgacagcaaaggtcagtttaacaacgtaccaccggagctgaacgatatgtgccgcatcatcagccatgtccaccagcatcatcattatctgctgggccgcgtggaggtgtaatcatgttgattctgaagaatgtcactgcggtacagctacacccggcaaaagtgcaggaaggcgttgatatcgccatcgaaaacgatgtgattgtcgctatcggcgatgccctgacgcaacgctaccccgacgccagcttcaaagagatgcatggccggattgtgatgccagggattgtctgctcgcacaaccatttttactcggggctttcccgcggaattatggcaaacatcgccccttgcccggatttcatctcaacgctgaaaaatctctggtggcggctcgatcgcgcccttgatgaagagtcgctctattacagcggactgatttgttccctggaagcgattaagagcggatgtacatcggttatcgatcaccatgcctctccggcgtatatcggcgggtcgctctccacattgcgcgacgcatttttaaaagttggcctgcgcgcgatgacctgttttgaaactactgaccgtaacaacggcatcaaagagttgcaggaaggtgtagaagaaaacatccgtttcgcccgtttgattgatgaggcgaagaaagcgacaagcgagccgtatctggtggaagcacatatcggtgctcacgcgccgtttaccgtgccggatgccggtctggagatgctgcgtgaagccgtgaaagccacaggccgtggtttgcatattcacgctgcggaagacctttacgacgtttcctacagtcaccactggtacggcaaagacctgctggcacgactggcgcaattcgatctcatcgacagcaaaacgctggtcgctcatgggctgtacttgtcgaaagatgacatcaccctactcaatcagcgcgatgcgttcctggtgcataacgcccgttcaaacatgaacaaccatgtcggctacaaccatcaccttagcgacatccgcaatctggcgttgggaacggacggcattggttcggacatgtttgaagagatgaaatttgccttctttaaacatcgcgatgcgggtggtccgctgtggcctgacagttttgccaaagccctgactaacggtaacgaactgatgagccgcaactttggcgcgaaatttgggcttctggaagccggttacaaagctgatttaaccatttgcgattacaactcgccgacgccgctgctggcagacaatatcgccgggcatatcgctttcggtatgggctcaggcagcgttcacagcgtgatggtcaatggtgtgatggtctatgaagaccgtcagtttaacttcgattgcgattccatttatgcacaagccagaaaagccgctgccagtatgtggcgtcggatggatgcgctggcataaatgacagatgccctcttcccgcagggaagagggttaaataaggaaagaagatgattgaacaatttttcaggcccgactctgtcgaacaggcgctggaactgaagcgccgctaccaggatgaagccgtctggttcgccgggggcagcaaactcaatgctacaccaacccgtaccgataaaaagattgccatttccttacaggatctggaactggactgggttgactgggataacggtgcactgcggattggcgcaatgtctcgcttgcagccactgcgtgatgcgcgatttattcctgcagcgctgcgtgaagccctcggttttgtttactcacgccatgttcgtaatcagtcgaccattggtggtgaaatcgccgcccgccaggaagagtcggtgctgcttcccgtcctgttggcactggatgctgaactggtttttggcaacggcgaaacgctgtcaatcgaggactacctggcctgcccatgcgatcgcctgctaaccgaaattatcattaaagatccgtatcgcacctgtgcgacccgcaaaattagccgttctcaggcaggtttaaccgtcgtgacggcagccgttgcaatgacagaccacgacggtatgcgaattgcgctggatggcgtcgccagtaaagcactgcgtctgcatgatgtcgaaaaacaaaatctggaaggcaatgcacttgaacaggctgtcgccaacgccattttcccgcaggaagatttgcggggcagcgtggcctataaacgctatatcacgggagttctggtagccgacctgtatgccgactgccaacaggctggggaggaagccgtatgatcatccactttactttaaatggcgcgcctcaggagctaaccgttaatccaggcgaaaacgtgcaaaagctgttgtttaacatgggaatgcactctgtacgcaacagtgatgatggtttcgggtttgccggttctgacgcaataatctttaacggtaatatcgttaacgcgtccttgcttattgccgcacagttagagaaggcagatattcgtaccgcagaatctctgggcaaatggaacgagttaagtctggttcaacaggcaatggttgatgttggcgtggtgcagtctggttataacgatccagctgcagctctgattatcaccgatcttctcgatcgcatcgccgcacctacccgcgaagagatcgacgacgcgctttctggtttgttcagccgcgatgctggctggcagcaatactatcaggtcattgaactggcggttgcacgtaaaaataatccgcaggccaccattgatatcgctccgactttccgtgacgacctagaagtcattggtaagcattatcctaaaactgatgccgcgaaaatggtgcaggcgaaaccctgctatgttgaagaccgcgtaacggctgacgcctgcgtcattaaaatgttacgtagcccacacgctcacgcactgattactcatctggatgtcagcaaagctgaagccttaccgggcgtcgttcacgttattactcacctgaattgcccggatatctactataccccgggtggtcagagcgcaccggaaccgtcaccgcttgaccgccgtatgttcggcaagaaaatgcgtcacgtcggcgatcgtgttgctgcggtcgtcgcagaaagtgaagaaattgcgctcgaagcactgaagctcatcgacgttgaatatgaagtgcttaagccggtaatgtcgatcgacgaagcaatggcggaagatgcgcctgtcgtgcacgatgaaccggtggtgtatgttgctggtgcgccagatactctggaagacgataacagccatgcagcccagcgcggcgagcatatgatcatcaacttcccgatcggttctcgccctcgcaaaaatatcgccgccagtattcatggtcatattggcgatatggacaaaggctttgccgatgccgatgtgatcattgagcgaacctataactcaacgcaagcgcagcagtgcccgactgaaacacatatctgctttactcgtatggacggcgatcgtctggttatccacgcctccacccaggtaccatggcacttacgccgccaggtcgcgcgcctcgtgggcatgaaacagcataaagttcatgtcattaaagagcgagttggcggcggttttggttccaaacaggacatcctgctggaagaagtgtgcgcctgggcaacctgcgtgaccgggcgtccggtactgttccgctacacccgtgaagaagagtttattgctaacacctctcgtcacgtcgcgaaagtcaccgtcaaactgggagcgaaaaaagatggtcgcctgacggcagtgaagatggatttccgcgccaacactggcccttacggcaaccactcactcaccgtaccgtgtaacggaccggcgctgtcgctgccgttatatccgtgcgataacgtcgatttccaggtcaccacctactacagcaacatttgcccaaatggtgcttatcagggttatggcgcaccgaaaggtaacttcgctatcaccatggcattagcggaactggctgaacagttacagatcgaccaactggaaattatcgaacgtaaccgggtacacgaagggcaagagctgaaaattctcggtgcaatcggtgaaggtaaagcgccgacctccgttccttccgccgccagctgtgcactggaagagatcctgcgtcagggtcgcgagatgatccaatggtcgtcaccgaaaccgcaaaatggtgactggcacatcggtcgcggcgtcgccattatcatgcagaaatcgggtatcccggatatcgatcaggctaactgcatgatcaaactggaatcggacggcacctttatcgttcattctggcggtgcggatattggtactggtctggatactgtagtgacgaaactggcagcagaagtgctgcactgcccaccgcaggacgtgcatgttatctccggtgataccgatcatgcgttgtttgataaaggcgcatatgcctcgtccggtacttgcttctcgggtaacgcggcgcgtttggcagcggaaaatctacgggagaaaattctgttccacggcgcgcaaatgttgggtgagccagtggcagatgttcaactggcaacgccgggcgtcgtgcgcggcaagaaaggcgaagttagtttcggggatattgcccataaaggcgaaaccggcaccggctttggttcactggtgggaactggcagttatatcacgcctgatttcgccttcccgtatggcgcaaacttcgctgaagttgccgtcaacacgcgtacgggtgaaatccgcctggataaattctacgccttgctggactgcggtacaccggtcaatccagagttagcgttgggacaaatctacggtgccaccctgcgtgctatcggccacagtatgagcgaagagatcatttatgacgccgaaggtcacccgttaacgcgtgatttacgcagttacggcgcaccgaaaattggtgacattccgcgtgatttccgcgctgtgctggtgccgagcgacgataaagtcggcccgttcggggcgaaatcgatctcggaaatcggtgtaaatggcgcagctccggcgattgctaccgcaattcacgatgcatgcggcatctggttacgcgaatggcatttcacaccggagaaaatactcactgcgctggaaaaaatataaataataaatggccgcttcggcggcctgtttctctgtttgaacgatgactaaatagtgactgcgaaaatgagataagccgttctcaaggcgtcctgcgccccaaattcgtgggaatttattttactaattcagatgatcaaatttactttaaaaggagtgaagggatgtctgatataaaccatgcaggttctgaccttatatttgaactggaggatcgccctccctttcatcaggctctcgttggtgccattacccatctgttggcaattttcgttccgatggtaacccccgcgttaatcgtgggtgcggccttacagctttccgctgaaacaactgcctatcttgtttctatggcgatgatcgcctctggtattggtacctggttacaagtaaaccgctacggcatcgtcggttctggcctactctcaattcagtcagtcaatttttcatttgttacggtcatgattgcgctgggcagcagcatgaaaagcgacggttttcacgaagagttaatcatgtcgtcgcttctcggcgtctccttcgttggcgcatttctggttgtcggatcttcatttatcttgccctatttacgtcgggttattacgcctaccgtcagcggtattgtggtactgatgatcggcttaagcctgattaaagtcggcattatcgattttggtggaggatttgcagccaaaagcagcggtacgttcggcaattacgaacatctcggcgttggtttattggttttaattgtggtgatcggctttaactgctgtcgcagtccgttgctacgcatgggagggatcgccattgggctatgtgtcggctatatcgcatcgttatgcctgggcatggtggatttcagcagtatgcgcaatttgccgttaatcaccatcccgcatccgttcaaatacggctttagttttagcttccatcagttcctggtggttggcacgatttatctgcttagcgtgctggaagcagtcggcgatatcaccgccacggcaatggtttcccgccgccccattcagggggaagagtatcagtcccggctgaaaggcggcgtgctggcagatggtctggtttctgttatcgcctccgctgtcggttcattaccattaaccacgtttgcgcaaaataatggggttattcagatgactggcgtcgcttcacgttatgtcgggcgaaccatcgcggtaatgctggttatcctcggcttatttccgatgattggcggcttcttcacgaccattccctcggcagttctgggaggcgcaatgacgttgatgttttccatgattgccatcgcagggattcgcatcatcatcaccaacggtttaaagcgccgtgaaacacttattgtcgccacttctttaggtttagggcttggcgtctcctacgatcccgaaatttttaaaatattgccagcctctatttatgtattagttgaaaaccctatttgtgctggcgggttaactgcgattttattaaatattatcctccctggtggctaccgacaggaaaacgttctgcctggtattacctcagcggaagagatggattaacagtaaaggagtcaatgatgtcaggagaacacacgttaaaagcggtacgaggcagttttattgatgtcacccgtacgatcgataacccggaagagattgcctctgcgctgcggtttattgaggatggtttattactcattaaacagggaaaagtggaatggtttggcgaatgggaaaacggaaagcatcaaattcctgacaccattcgcgtgcgcgactatcgcggcaaactgatagtaccgggctttgtcgatacacatatccattatccgcaaagtgaaatggtgggggcctatggtgagcaattgctggagtggttgaataaacacaccttccctactgaacgtcgttatgaggatttagagtacgcccgcgaaatgtcggcgttcttcatcaagcagcttttacgtaacggaaccaccacggcgctggtgtttggcactgttcatccgcaatctgttgatgcgctgtttgaagccgccagtcatatcaatatgcgtatgattgccggtaaggtgatgatggaccgcaacgcaccggattatctgctcgacactgccgaaagcagctatcaccaaagcaaagaactgatcgaacgctggcacaaaaatggtcgtctgctatatgcgattacgccacgcttcgccccgacctcatctcctgaacagatggcgatggcgcaacgcctgaaagaagaatatccggatacgtgggtacatacccatctctgtgaaaacaaagatgaaattgcctgggtgaaatcgctttatcctgaccatgatggttatctggatgtttaccatcagtacggcctgaccggtaaaaactgtgtctttgctcactgcgtccatctcgaagaaaaagagtgggatcgtctcagcgaaaccaaatccagcattgctttctgtccgacctccaacctttacctcggcagcggcttattcaacttgaaaaaagcatggcagaagaaagttaaagtgggcatgggaacggatatcggtgccggaaccactttcaacatgctgcaaacgctgaacgaagcctacaaagtattgcaattacaaggctatcgcctctcggcatatgaagcgttttacctggccacgctcggcggagcgaaatctctgggccttgacgatttgattggcaactttttacctggcaaagaggctgatttcgtggtgatggaacccaccgccactccgctacagcagctgcgctatgacaactctgtttctttagtcgacaaattgttcgtgatgatgacgttgggcgatgaccgttcgatctaccgcacctacgttgatggtcgtctggtgtacgaacgcaactaataataaaactttaacatcctcgtgaggacatcattatgtctggagacatcctacaaacaccggacgcaccaaagccacagggcgcgctggataattattttaaaattaccgctcgtggcagtaccgttcgtcaggaagtactggctggcttaacgacctttctggccatggtttattccgttatcgtcgttccgggaatgctgggcaaagcaggttttcctcccgcagctgtgtttgttgccacctgtctggtcgcgggcttcggctcgttgctgatgggattatgggctaatttgccaatggcgattggttgcgcgatttccttgacggcgtttaccgcattcagtctggtactcgggcaacaaattagcgttcctgtcgcactgggcgcggtatttctgatgggcgtcatcttcaccgccatttccgtaaccggtgtgcgtacctggatcttacgtaatttgccgatgggtatcgctcacggtacaggtatcggtatcgggctgtttctgctgctgattgctgctaacggtgtgggtatggttatcaaaaacccgattgaaggcttgccagtggcgctcggtgcgtttacctccttcccggtgatgatgagcttgctggggctggcggtcatcttcggcctggagaagtgtcgcgtacccggcgggatcttgttggtgattattgcaatttcgatcatcggcttaatctttgacccagcggtgaaataccacggtctggtggcgatgccaagcctgactggcgaagatggtaagtctctgattttcagcctcgatattatgggtgcactccagccaactgtacttccgagtgtactggcattggtgatgaccgcagtgttcgacgctactggcaccatccgtgccgtcgccggtcaggcgaatttgttggataaagacaaccagatcatcaacggcggcaaagccctgaccagtgactcagtaagttcaatattctccggcctggtgggcgcagcgcccgcagcggtttatatcgaatcagcggcaggaaccgccgccgggggtaaaacaggtttaaccgcaaccgtagtgggggcgttattcctgttaattctgtttttatcaccgctgtcatttttgatccctggttacgccactgcacccgctctgatgtacgtaggtttgctgatgttaagtaacgtctcgaagctggatttcaatgattttattgacgctatggctggcctggtgtgtgccgtgttcatcgttctgacttgtaatatcgttaccggtattatgctgggctttgtgacactggtcgtaggccgcgtctttgcacgcgaatggcaaaagctgaatattggtacggtgatcattactgccgcactggtcgcattttacgcgggtggttgggcaatctaatagattctccgcgcctttcagcgcggagatttctttcagagaggattctcaccgctggcaacaatacgctgctggcggactcgcctgagttctctttcagtaagcaactgcagcgcctgtgttgggcaagattcaacgcaggctggcccctcttcccgctgttcacagagatcgcatttcacaatttgttgtcgggtatcccccggcaacgactgaatggtgatcattccaaacgggcacgcactgacgcaactctgacagccaatacaacgggcagaattggtctgcaccacctgctcgcccatcgtcagcgcccccacggggcaagcgccaacacaaggggcgttttcacactgatggcacatcaccggcgcactgatgctgtccagtcgctgtaccttcagccggggtaaaaagacatcggcattcaactcctgttctgaagggtgagcgaccacacaggctacttcacaagtacggcagccaatacagtcagccggattaacgataattaacgatttcatcacgatgccttcgtatcaaacagagttaacatatcgcgcgccgcctgccttcctgcggccattgcagtgacaaccagatccgcgccatgaactgcatcaccaccagcaaagacttttttcagatgcgtctgggtaggtaaatacccgacgtcaccggtttgaatcaggccccatttatcgagtttaattccgctgccctgcaaccacggcatggcatgcgcctggaaaccaaaggccataatcagaacatcggcgggcaattcaaactctgaacccgctaccggacgaggacgacggcgaccatccggccccggctcacccatggcggtacgaatcaggcccaccgcagttaaacgcccatcttcgtcacaagcgatatattgcggttgaacattgaactgaaactcgacaccttcctcgcgcgcattaaccacctctttgcgcgagcccggcatactgacttcatcacgacgatacgcgcaggtcacgctggcggcattgaggcggatggaagtccgcaaacaatccattgtcgtatcgccaccgcccaataccacgactcgcttaccttccacgtccgtcagcggatactcttcagactccggcaatcccatgagctggcgggtatgggcagtcaggaacggtagagcctgaatgacaccgggcgcatcttcatgcggcagatctgctcgcatcatcccgtaagtccccacgccgatgaaaactgcatcatattcagaagttaaatcgctaaaggtaatatcgcggccaatttcacagttaagatgaaagtcgattcccattgcggtgaatatctctcgccgctggcttaataccgttttatcgagtttgaaaggaggaatgccaaaagtcagcataccgccaatttctggatggcgatcaaagacatcgacctgaactcctgcgcgcgccagaatatcagcacaccctaaccctgcaggcccagcgccaatcaccgccactttttcgctacggggaacaactttgctgacatcgggacgccagcccatcgccagcgcggtatcggtgatgtagcgttccagattaccgatagagactgcgcccgagtgatctttcaaagtacatgcgccttcacaaagacggtcctgtggacataccctgccgcaaatttctggtaaggaactggtctggtggcaaagttctgccgcttcaataatctttccttcctgtaccagacggatgtaatccggaatagcgttatgcagcgggcaatgccagttgcagttagctttttcggcacaataaacacagcggtcactctcataagtcgcttgttgtggatccagcccgcaatatatttcgccaaagtgggttttccgttcactcgctgaaattttatctgcgcctttacgcgagttaacggggagcaacgctgcactgcgagatggctgagcgtctgatgacgcttttcctgctgccgttttgcgctggcgggccacctttatctgctgcaaccctttatcgtccatcagtcgtaacgcctgtgttgggcaaacttcaatacaggcttgcgtgccggaactgcgctggttacaaaggtcgcatttctgcgcaatcgtatcgaccatctcaacgacgccaaaggggcaagcgattgcgcatcttttacaaccaatacatttttgctcgtccagttgtacgctatcggactggaaagtcagagcattaaccggacaagccgtaacgcaaggggcattgttgcagtgatggcaggccaccggattcgcagcctggcctttccctacaacgtggatacgcggtcgaaagtcactgtgactcagcggccagttttcttgattgtgtgccaccgcacaggcaatttcacaagcatgacagcctatacattccgcagcttcagcagcaataaacttattcatttgcatccctttcatttaatgagttatgtcttctcaaatttcgcgatgcaataaacgggcatatattaggtagcatgaccgttttaattataattttgcgactgagttcaaattattgcccctcaatctatgccgctttcattatttcaacattgccgatcaaaagagcgctatccagataaaaacgattaaatgcgagagtgcgacatgccagaatgattaatgaaatatcaatatgagaaaattacagataattccattgtcaggttctcttctcattttcgtggtttaaccacgattatgtgattgcctccgcaattcctgtctctaactccccttcctcgcaaaaactggcactccacgagcatgtgtttagacagtttcattaacgtaaacggttgctttttactctggcgggcgaaaggagaaacactgatgagcgccatagattcccaacttccctcatcttctgggcaagaccgcccaactgatgaggttgaccgcatattatcaccaggaaagctgatcatactcggtctgcaacacgtccttgtcatgtacgcaggtgcagtcgctgttcctcttatgattggtgaccgactgggcctctcaaaagaagctattgcgatgctcattagctcggatctcttttgctgcgggatcgtcacattattgcaatgtatcggtatcggccgctttatggggatccgcctgccggtgattatgtcggtgacctttgctgctgtaacaccaatgatagccattgggatgaacccggatatcggcctgctggggatatttggtgccactatcgccgcgggttttatcaccacattattagcgccacttatcggtcgcttgatgcctttattcccgccactggttaccggtgtggttattacttctatcgggcttagcatcattcaggtgggtattgactgggccgccggaggtaaagggaatccgcaatatggtaatcccgtttatttaggtatctcctttgccgtcttaatttttatcttgctcattactcgctatgcgaaaggatttatgtccaacgtcgccgtattactggggattgtatttggctttttactttcgtggatgatgaatgaagtcaatttatccgggctacatgatgcttcatggtttgcgattgttacgccgatgtcgtttggtatgccgattttcgatcccgtttccattctgaccatgactgccgtgttaatcatcgtgtttatcgagtcaatggggatgttcctggcactgggtgaaatagtcggtcgtaaactctcttcgcacgatattattcgcgggctgcgtgtcgatggcgtagggacaatgataggcggcacgtttaacagcttcccccacacgtcattttctcaaaacgttggcctggttagcgtgacgcgcgttcatagccgctgggtgtgtatttcttcgggaattatattaatcctgtttggcatggtgccaaaaatggcggtgctggtagcctccattccgcaatttgtgctgggcggcgctggtctagtgatgttcggcatggtactggcgacagggattcgaattctgtcgcgctgtaactacaccaccaaccgttacaacctctatattgtggcgatcagtctcggcgttggcatgactccgacgctctctcacgatttcttttctaagttaccggccgtactgcaaccgctgctacatagcggcattatgctcgcaacccttagcgccgttgtgctgaacgtcttctttaatggctatcagcatcatgctgacctggtgaaggaatccgtctctgataaagatttaaaagtcaggacagtacgtatgtggcttctgatgcgcaagctgaagaaaaatgagcatggagaataatatgaattttttaatgcgcgctatattcagtctgttgttgctttttactctctctattcctgtcatttctgactgtgttgcaatggccattgaaagtcgcttcaaatatatgatgctacttttttaaatggtttttacctgtcggcatccgctcaaaacgggcggttgtcgataaacgctcacttggttaatcatttcactcttcaattatctataatgatgagtgatcagaattacatgtgagaaattatgcaaacggaacacgtcattttattgaatgcacagggagttcccacgggtacgctggaaaagtatgccgcacacacggcagacacccgcttacatctcgcgttctccagttggctgtttaatgccaaaggacaattattagttacccgccgcgcactgagcaaaaaagcatggcctggcgtgtggactaactcggtttgtgggcacccacaactgggagaaagcaacgaagacgcagtgatccgccgttgccgttatgagcttggcgtggaaattacgcctcctgaatctatctatcctgactttcgctaccgcgccaccgatccgagtggcattgtggaaaatgaagtgtgtccggtatttgccgcacgcaccactagtgcgttacagatcaatgatgatgaagtgatggattatcaatggtgtgatttagcagatgtattacacggtattgatgccacgccgtgggcgttcagtccgtggatggtgatgcaggcgacaaatcgcgaagccagaaaacgattatctgcatttacccagcttaaataaaaaaaccccgacatttgccggggttgtgagcataacgtaatgcttattttaccggacgcatcgccgggaacagaataacgtcgcggatggtatggctgttggtgaacagcattaccatacggtcgataccaattcccagacctgctgtcggcggtaagccatgttccagtgcggtgacgtaatcttcatcgtagaacatcgcttcgtcgtcacctgcgtctttcgcggcaacctgatccaggaagcgttgcgcctgatcttccgcgtcattcagctcgctaaagccgttaccgatttcacgaccaccaatgaagaactcaaagcggtctgtgatttccgggttaacgtcgttacgacgcgccagcggagaaacttctgccggatattcagtaatgaaggtcggctgaatcagatgtgcttctgccacttcttcgaagatctcggtaacgatacggcccagaccccagctcttctcaacgtggatgccgatagattcagcaattgctttcgcagagtcgaagttgtccagatccgccatgtcggtttccgggcgatatttcttgatcgcttcacgcatggtcagtttttcgaacggtttaccgaagtccagcgtcacgtcgccgtaggtcacttccgtcttaccgagaatatcctgtgccagagtacggaacagcgattcggtcagctcgatcagatctttgtaatctgcgtaagccatgtagagttccatcatggtgaactctgggttatgacgtacggaaataccttcgttacggaagttacggttgatttcgaatacacgctcgaagccaccaaccaccagacgcttgaggtacagttccggcgcgatacgcaggtacatgtcgagatccagcgcgttatggtgggtgataaacggacgcgcagcggcaccgccagggatcacctgcatcatcggcgtttcaacttccataaagccgcggttcaccatgaactggcgaataccagagaggatctgcgagcgcactttaaaggtgttgcgggattcatcgttggagatgagatcgagataacgctgacgatagcgcgcttcctgatcctgcaagccgtggaatttatccggcagcggacgcagtgctttggtcagcagacgcaactcggtgcagtggatagacagttcgccggttttggttttgaacagcttacctttcgcgccgaggatgtcgccgaggtcccattttttgaactgctcgttataaacgccttccgggagatcgtcacgggcaacgtacagctgaatgcgaccgccaacgtcctgcagggtaacgaaagacgctttacccataatacgacgggtcatcatgcggccagcaacggcgacttcgatgttcagcgcttccagttcttcgttctctttgccgtcgaattctgcgtgcaattggtcagaggtatgatcgcgacggaaatcgttcgggaaggcaatcccctgctcgcgcaggttcgccagcttctcacgacgcgttttcagttcattgttaagatcgactaccgcgtcagcgccctgtgcgtgttgttcagacatgttggttcctcataaccctgctttcaaacttgcttcgataaattgatccaggctgccgtccagcacggcctgcgtgttgcgggtttctaccccggtgcgcagatctttaatgcgggagtcatcaaggacataagaacgaatctggctgccccagccgatgtcggatttgttatcttccatcgcctgtttctcggcatttttcttctgcatctccagttcataaagcttcgctttcatctgcttcatggcctgatctttgttcttgtgctgggaacggtcgttctggcactgggtcacgatcccggtcgggatgtgggtaatacgcaccgcagattcggtacggttaacgtgctgaccgcccgcgccggacgtgcgataaacgtcaatgcgcagatccgccgggttgatttcgatatcaatatcatcatcaacttccggataaacaaacgcggagctgaacgacgtgtggcgacgaccgccggagtcaaacgggcttttacgcaccaggcggtgaacgccggtttctgtacgcagccagccgtaagcgtaatcgccggagattttgatcgtcacggatttaatacccgccacttcaccttccgactcttcgatgatttcagttttgaaaccacgcgattctgcccagcgcagatacatacgctcaagcatgctcgcccagtcctgtgcttccgtaccgccagaccccgcctgaatatcgaggtagcagtcggcgctgtcatattcgccagagaacatacggcggaactcaagctgcgccagtttttcttccagggcgtcgagttcagcaacggcttcgttaaaggtttcttcgtcgtcagcttctacagccagttccagcagaccagaaacatcttccagcccctgtttcatttggtcgagggtgtcgacaacggcttcgagggaggaacgctctttacccagcgcctgtgcgcgttcgggttcgttccagacatccggctgttccagctcggcgtttacttcttccagacgctctttcttggcgtcgtagtcaaagataccccctaagaacgtcggagcgttccgtgaggtcctgaatgcgattatttaccggattaatttcaaacatggtctgatttcttttattgagctagtcaaaatgcggtgataagagcgggattgtacccaatccacgctcttttttatagagaagatgacgctaaattggccagatattgtcgatgataatttgcaggctgcggttgccgcgaaactcgttgatatcgagcttataagccagttgcacttcgcgcacgccgttatccggccagagggcggtatcgacattaaaagcaataccatccagcagtggaccgccgccgaccggttcgaccatcaccttcaaatgacgttcgcccaccagccgctgttgcagcagacggaaatgaccgtcaaacagcggctccgggaacatctgcccccacgggccagcatcgcgcagcagctgcgccacttccatggtcatttcggccgggcttaacggaccgtctgataccacttcgccttgcaatagcgaagggtccagccactcagtaaccagttcgccaaaccgttgttgaaagagtttgaatttatcctcttccagcgacaaacccgccgccatcgcatgaccgccaaacttcagcatcatgccagggtagagtgtgtctaatcgctccagcgcatcacgcatatgcagcccctgaatggagcgaccggaacctttcagcgtaccgtcacctgctggcgcaaacgcgataaccggacggtgaaaacgctctttgatgcgcgaagccagaataccgacaacgccctgatgccattcggggtgatacattgccagcccgccgggtagcgtgtcacggctgcgctccagtttctcgcacagggtcagggcttcaatttgcattccttgttcgatctcttttcgcgtctggtttagcgcatcgagttcatttgccagcacgcgcgcttcgccgatgttgtcgcacaacaacagcgccacaccgacggacatatcgtccagtcgtccggcagcattgagacgtggccccagcgcaaaacctaaatcgctggcggcgagtttttgtgcatcacggtttgccacttcaagcagcgctttaatccccggacggcactttccggctcggatgcgactcatcccctgccaggtcagaatgcgattattagcgtccagcggcacgacgtccgccactgtccccagcgcgaccagatccagcagttctgccaggttaggaattgcgatgttacgctcatcaaaccagccctgatcgcgcaaaaaggtgcgcagcgccagcatcagataaaacgccacacccacgcctgccagtgatttcgacgggaaattacagtcgcgcaagttagggttaatgatcgcttccgctgcgggtaatgtgtcgcctggcaaatggtgatcggtaacaataaccgggatgcccaacgagcgagcgtgctcaacccccgcatgggaggaaataccgttatccaccgtgacaattaactgcgcgccacgggcatgggcctgatcgaccacttccgggcttaagccgtaaccgtcttcgaaacggtttggtaccaggtagtcgatattgctgcaaccaagcgagcgcatcgccagcacgcttagagccgtgctggtcgcgccgtcggcgtcgaaatcaccgaccacaataatccgcgttccttcgcgaaaagcgttgtaaaggatctcaacggccttttcgacgccgctcagttgctgccagggcagcatacctttaacactgcgttccagttcttgcgcactgcgtactccccggctggcgtataaacggcgcagcaagggaggcaattcagcgggcaagtctgccgtttcatcgacttcacggcgacgaagttgtatctgttgtttcacgcgaattatttaccgctggtcattttttggtgttcgtcgaggaattctttcatctctttcggcggctggtaacccggaacaagtgtgccattgctcagcacaactgccggagtaccgctaacgccaagctggacgccaagtgcgtaatggtcggcaatatccacgtcgcaactggctggtgcgacgcttttacctgccatcacatcatcaaacgctttgtttttatctttcgcacaccagatagctttcatttctttctctgcatcgctgtccagcccctggcgcgggaaagcaagataacgcacggtgatccccagcgcgttgtagtctgccatttgctcatgcagtttgtggcagtaaccacaggtaatatcagtaaacacggtgatgacgtgtttttcctgcggcgctttataaacgatcatctctttttcaagcgcattcaactgctttaacagcatcttattggtgacattgaccggagccgtgccactaacgtcatacattggcccctgaatgatatgtttaccatcatcggtgatgtacaacacgccgctgttagtcagaactgtcttcatgccagctacaggcgcgggctgaatatcgctgcttttgatgcccattttggctaacgtttgttgaattgccgcgtcatcagcctgagcaaagcctgaaaacgccgctaacaaagtaaacaacataaaacctttcttcataaatcttcccgttcttttcagacatcacgcccgcgggtgatgctgttgatgaagttgccgcagacgctcggtagcgacatgcgtataaatttgcgtggtggagagatcgctgtggcccagtagcatctgcaccacgcgtaaatccgcaccatgatttaataaatgagtggcaaaagcgtgacgcaacacatgcggtgacagcttttcgctgtcgatacccgccagcacagcataatgtttaatacggtgccagaaggtctgtcgcgtcatctgctgcgcacgctggctgggaaacaacacgtcaattgacacaccattcagcagccacggacgcccatgttccagataggtttccagccagtaaaccgcctcttcacctaacggcaccagacgctctttgttgcctttaccaatgacccgtaccacgccctgacgcaggctgatatcactcattgtcagtccgaccagttcagagacacgcagcccggtagcatacaacacttcaagcatggctttatcgcgtagctccagtggctgatcgattaatggtgcctgtaataaacgttcgacctgcgcttcgcttaaatcttttggcaaacgctggggcaatttcggtgaagcgagatgcgcactgggatcgtcttcacgaaacttttcgcgataaagatactggaacaatcggcgcactgcactcagcaaacgcgctgagctggtggctttatacccgccctccagccgttctgccagtaatgcctgcaaatcgtcactttgcgccgtcgccagcgtcaacccgcggtgatgcaaccactccaccatcattgacagatcgcgacggtaagcgttcaacgtattttcagccagatttttttccagccacagagcatcaagaaactgctcgatgcgtgccagatcctgtttcacttgcgccccttatggtcactcatttgatccattatgccttattgtgccgtgactaaagcgattctgatacactagccgcaaaagccacagcagaatcgagaagcttacgttatgaatatgggtcttttttacggttccagcacctgttacaccgaaatggcggcagaaaaaatccgcgatattatcggcccagaactggtgaccttacataacctcaaggacgactccccgaaattaatggagcagtacgatgtgctcattctgggtatcccgacctgggattttggtgaaatccaggaagactgggaagccgtctgggatcagctcgacgacctgaaccttgaaggtaaaattgttgcgctgtatgggcttggcgatcaactgggatacggcgagtggttcctcgatgcgctcggtatgctgcatgacaaactctcgaccaaaggcgtgaagttcgtcggctactggccaacggaaggatatgaatttaccagcccgaaaccggtgattgctgacgggcaactgttcgtgggtctggcgctggatgaaactaaccagtatgaccttagcgacgagcgtattcagagctggtgcgagcaaatcctcaacgaaatggcagagcattacgcctgatctcactgacggcttagcgcatatgctttgccgtcatctttatctttgcgtctcttgttgcaacaaaatccgccgtaaatcccgccattcagcttcgtccatgctgtcggctgccagccataaatgttgccgtttaccgccatcagaacgtaaacgcagcatcatgccgctcttaatcatccacggtgctttgacgatgctccactcctgcccttgccaacgcaaacgcccgtccatcaacaagcgaatttccccctggcgagcattaatacgccgctggctgcgaacgcaatcaaacaccaccagcgaaagtaacaccatccataacggggtgtaactgagtggccagggcatgagtaaaataacagcggcaaccagcccatgaatcagcaaggaaagccactgtgcgcgccaggagacgcgcaaatcagattgccacaggaccacgttcccggttccgtgtctggatgagtcggaccatcatttccagttctgcatcggccggtttaccgtgattcatcagccagttaaacaggtccggatcgtcacattccagcagacgaataaagatgcgtttttcgtcatcgcttaagctgtcgtactcatgttcgaaaaacggcatgattgaaatatcgagttcgcgcataccacggcggcatgcccaatgaatgcgggctttgttgttaatgtccatcttcttcctgtctcacgaaaatccagtacccggctattgtaacgtgtttttcgccttcttttacgggaatatcagtaaacaccatcgcgatcgcgaaattaattcacaacaattcaatggcttcatttttttggaagtcgcctcgcagaaggcacagatcgcgtagtgaaagcacttgcattgcctcatagctcttttaccattagtcattaatacgccgttaagcaactcaggactctattatggcttttacaccttttcctccccgtcagcctacggcttctgcccgtttaccgctgacgctgatgacgcttgatgactgggcgcttgccaccattactggcgcggacagcgaaaaatatatgcagggtcaggtgacagcagatgtcagccagatggcagaagatcagcacctgctcgccgcccattgcgacgccaaaggtaaaatgtggagcaatttacgtctgttccgcgacggcgatggctttgcatggattgaacggcgcagcgtgcgtgaaccgcagctgactgaactgaaaaaatatgcggtattctctaaagtgaccatcgcgccagacgacgagcgtgtgctgcttggtgttgccggttttcaggcgcgcgccgcgctggcaaatctctttagcgaactgccttcgaaagaaaaacaggtagtcaaagaaggcgcgaccactttgctatggtttgaacacccggcagaacgtttcctgatcgtaaccgatgaagctactgctaatatgctgaccgataaactgcgcggtgaagcggaactgaacaatagccaacagtggctggcattaaacattgaagcgggtttcccggtgattgatgccgccaacagcgggcagtttatcccacaggcgaccaatctccaggcgctgggcggtatcagctttaagaaaggctgttataccggacaagagatggtggcgcgagcaaaattccgtggtgccaataaacgtgcgctctggttgctggcaggtagcgccagccgactgccggaagctggtgaagacttagagctgaaaatgggcgagaactggcgtcgtaccggtacggtactggctgcggtaaaactggaagatggtcaggtcgtggtacaggtcgtcatgaataacgatatggaaccggatagcatcttccgcgtacgcgacgatgcgaatacattgcatatcgagccgctgccgtattcgctcgaagagtaaatctctttatcgcatcaggcatttatcgcctgatgcgacgctggcgcgtcttatcatgtctgggatttgatgcctttatcacaacagggacgaggcccgtagatcggataaggcgttcacgccgaatccggcagttgtgctccgatgcctgatgcgacgctggcgcgtcttatcaggcctacaaaggcatacccattacgcctgcccaatatacaaatagatcgccagaaagtggcacacactaccgccgagcacgaagccgtgccagatggcatggttgtatggaatgcgtttgcagacgtagaaaatcaccccgagcgaataaaccacgccgcctaccgccagtaaggtaacgctgcccgccgcgagcttaactgccatttcataaattaccaccagcgacagccagcccatcgccagataggtcaccagagataaaattttgaatcggtgcgcgatggtcagtttaaacagaatacccagcaatgccaggctccagataacaatcatcaacccgcgcgctaacggagaatccagccccaccagcaaaaacggcgtgtaggttccggcaatcaacaggtaaatagcgcaatggtcaaatttcttcagccacatttttgcccgttgatgaggaatggcgtgatagagcgtcgaagcgaggaacagcaggatcatactgccgccatagaggctgtagctggttatcgctgtggcgctggcattaagatccaccgcctgaaccagtagcaacaccagcccaacgataccaaacaccaacccaatgccgtgactgacgctgttggctatttcctctgccagtgaatatccctgcttaatgaggggcttctgaaccataacttactccggagaaacgtacacgcacatgtatacctctccagcgtaactgagaatagttccagtgaacacctgttagctaaaataaattctgatttgagactaatctcctaaaaatcatgaaattaaatgcgaaatttcaactaacaggcgtgagttcaatttaaagacatttaaattcaatcacataaaattgtgtctgaccgggatagatgtcagcaatgacttttttcagttcagtcagggtcatattttcctgctctgcatgtttttcagtcagcgtatccagcgttacggttgaggttgcggtgacttcaatcgtgcaaaaataaccgtcatcttcaaaacgtccgacacgaagcacatcacccgttttgaagtgcgattcagactcgtcgcggatggtgatggttttacgcccagccagaatgtcatcctggaaacgttgaaaaaaagtgatgtcgtttggctgcatggtactatttcctgtaagaattgactcatctggagcctatgatagtgaaaaaactcaccttaccgaaagatttcttatggggcggcgcagttgccgctcatcaggtcgaaggcggctggaacaaaggcggaaaagggccgagcatttgtgacgttctgaccggtggcgcacacggcgtgccgcgcgaaatcaccaaagaagtcttgccaggaaaatactatccaaaccatgaagccgttgatttttatggtcactataaggaagacatcaagctatttgccgaaatgggcttcaaatgttttcgtacatccattgcctggacgcgcatttttccaaaaggcgatgaagctcagccaaacgaagaagggctgaagttctacgatgatatgttcgatgaactgctgaaatacaacatcgaaccggtgatcaccctctcccactttgaaatgccgctgcatctggtgcagcaatacggtagctggaccaaccgtaaagtggttgatttctttgtacgtttcgcggaagtggtatttgaacgctataagcacaaagtcaaatactggatgaccttcaacgaaattaacaaccagcgtaactggcgtgcaccgctgttcggttactgctgctccggcgtggtgtataccgagcatgaaaacccggaagagacgatgtatcaggtgctgcatcaccagtttgtcgccagcgccctggcggtgaaagctgcgcgtcgcattaacccggagatgaaagtcggctgtatgctggcgatggtgccgctctatccttactcctgtaacccggacgatgtgatgttcgctcaggagtcgatgcgcgaacgctacgtctttaccgatgtgcagctacgcggctattacccgtcctatgtgttgaacgagtgggagcgtcgcggatttaacatcaaaatggaagacggcgatctggatgtgctgcgtgaaggcacctgcgattatcttggtttcagctattacatgaccaatgcagtgaaggccgaaggcggcaccggcgatgcgatctctggttttgaaggcagcgtaccaaacccgtatgttaaagcatctgactggggctggcagattgatccagtaggtctgcgctatgcactttgcgaactgtatgagcgttatcagaggccgctgtttattgtcgaaaacggttttggcgcttacgacaaagtggaagaagatggcagcatcaacgacgactaccgcattgactacctgcgcgcccatatcgaagagatgaaaaaagcggtgacttacgatggcgtggatctgatgggctacacaccgtggggctgcatcgactgcgtgtcgttcaccaccgggcagtacagcaaacgctacggctttatctatgtgaataaacatgacgacggtactggcgatatgtcgcgttcacgtaagaagagctttaactggtacaaagaggtgattgccagcaacggcgagaagctttaagtcgatgaagtaccggatgcaatacttgttgcatccggtcagacaacttccctgttttatttcccgcccgccaaatcgataaaacttcccgtgacgtaagaggctttatcacttagtagccagacaatggcctgcgcgacctcttctgcctgtccaccacgctgcatggggatgttcgacttaacgcgatcgacgcgtccaggctcgccgccgctggcgtgcatttcggtataaataaaccctggccgcacgcagttaacgcggatcccctgcgcggcgacttccagcgatagtccggtggttaacgtatcaatcgcccctttcgatgccgcgtaatcaacatattcccctggcgaacccaaccgtgaggccaccgaagagacattgacgatagcgccgccactgccaccatttttaagcgccatgcgttttaccgcctcgcggcagcagagaaaatatcccgtcacgttggtggaaagtactcggttgattcgctctgcggtaaggttttcaacggtgcactgggtaaacaagatcccggcgttattgaccagcgctgctagcggttcatcgtgctgatcgattgctgtaaacatcgcaacgacctggttttcgtcgctgatatccgcctggagcacgaatgctttgccaccggcttgcgttattaagttcatcacttcctgcgccgcgtggaggttttgctgataattaaccgccaccgtatacccttcttgcgccaacagtaatgcagttgcccgcccgatgccgcgactgccaccagtcacaagtgctatagccatttgtttttccgagaaaaattaattcgttgacgtatctttgagattgctaacaaactggctcaatcttcaatgttggcacgcttttccccctcgccctttcagggagagggccggggtgagggtaaatattcgcgccagtgccggcctgttcccctcaccctaaccctctccccaaaggggcgaggggactgtctgagcacttttgtactttgtcatctgactaaaaaggcgccgaagcgcctttagaaaatagtcgaatcagtgaattactggtattcgctaatcggtacgcaggagcagaacaggttacggtcgccgtaaacatcatccagacgtttcactgtcggccagtatttgtctgccacacctgccgggaataccgcaacttcacggctgtacggatgcgcccactcggcgaccagttcgctctgaatgtgcggcgcgttcaccagcgggttatcttccagcggccagacaccggctttcacctggtcaatttctgcgcggatagccagcatcgcgtcgataaagcgatccagttccactttgctttcagattcagtcggttcaaccatcagcgtacccgccaccgggaacgacatcgtcggcgcgtggaaaccgtagtcgatcaggcgcttggcaatatccagctcgctgatgccggtttcttctttcagcgggcgaatatcgagaatacattcgtgcgccacgcgaccgtcgcgaccggtatacagcaccgggaaggcatcctgcaggcggctggcaatatagttggcgttgaggattgccacctggcttgcttttttcagcccttctgcgcccatcatgcggatgtacatccagctgattggcaggatagaggcgctaccgaacggtgccgcagaaaccgcgccctgacgggttaacatgccttcgatttgcaccacgctatgacccggtacaaacggtgccaaatgcgctttcacgccgatcggtcccatacccggaccaccaccgccgtgcggaatgcagaaagttttatgtaggttaaggtgtgaaacgtccgcaccaataaagcccggcgaggtgatgccaacctgggcgttcatgttcgcgccatcaaggtaaacctgaccgccgaactgatgcacgacttcacacacttcacggatcgtttcttcatacacgccgtgggtagaaggataagtcaccatgatacaggagaggttatcgcccgcctgttccgctttcgcgcgcagatcagtcagatcgatgttgccgtttttatcacacgccacaaccaccacctgcattcctgccatatgtgcagaagcggggttagttccgtgcgcagaagccgggatcaggcagatatcgcgatgcccttcgttgcggctttcatgataatgacgaatcgccagcaggcccgcgtattcgccctgtgcgccagagttcggctgcatacaaacggcgtcgtaaccggtcagtttcaccagccagtcagccagctgcgcaatcatctgctgataaccttcggcctgctccggcgggcagaacgggtgcagttcggcaaattccggccaggtgattgggatcatctcggcggcggcgttcagtttcatggtgcaggaacccagcgggatcatcgcctgattcagcgccagatctttacgctccagcgagtgcatatagcgcatcatttcggtttcgctgtggtagcgattaaacaccggatgggtgaggatttcgtcgtcgcgcagcatcgcaggctggatagagcggctgtcgtgagccacgtctttgtccagcgtgtcgatgtccaggccgtggttatcgcccagcagcacgttgaaaagctgcattacgttttcacgcgtggttgtttcatcaagggtgatcccaaccgcgttcagaatatcgctacgcaggttgatttcagccgcttcggcacgcgtcagtacgcccgctttgtcggccacttccacacacaaggtgtcgaaatagtgcgcatggcgcagtttcagacctttttgttgcaggcccgccgccaggatatcggtcagacggtgaatgcggttagcgatacgtttcaggccaaccgggccgtgataaacggcatacaggctggcgatgtttgccagcagtacctgggaagtacaaatgttggagttcgctttctcacggcggatatgttgctcgcgagtctgcatcgccatgcgcagcgcggtattgccagctgcatctttcgatacaccgataatacggcccggcattgagcgtttgtattcatctttcgccgcaaagaatgccgcgtgtgggccaccgtagcccatcggcacgccgaagcgttgcgccgaaccaaaaacaatatccgcgccctgtttacccggcgcagttaacagcaccagcgccataatatcggcggcaacgctgaccacaattttgcgtgatttcagttcgctaataagcgcagtgtagtcgtgaatttcaccggtagtgcctacctgctgtaacagcacgccgaagacgtcctgatggtcgagcactttttgcgcgtcatcgacaatcacttcaaaaccaaaggtttcggcacgagtacggaccacatccagcgtttgcggatgcacatcggaagccacgaagaagcggttggcatttttcagtttgctgacgcgtttcgccatcgccattgcttcggcggcagcggtggcctcgtccagaagagaagcagaggccatatccagtccagtcaaatccagcgttacctgctggaagttgagcagtgcttcaaggcggccctgggagacttcaggttgatacggagtgtacgcggtataccagcccggattttccagcatgttacgcaggataaccggcggtagctgcacggcggtgtaacccatgccgatgtaagacgtgaagcgtttattgcgactggcaatagccttgagttctgccagtgcggcgtattcggtcgccggtgcgccaacctgcggtggtgtcgcaagttgaatatctttcggcacaatctggccggtcagcgcgtttaacgattgtgcaccaacggcattcagcatttcttgctgttgcgcggcgtccggtccgatatggcgttcaataaaagcgccgctgttttcaagctggcttaacgtctgtgtcatgagcgatggttcctgaaacgtgcagtgaattgtgaacctctctccttacgaagagagtgagggtgaggcataaattttcctcaccctgatcctctcccgcagaagaggaataaagccgttactcgtcttctaacaatgcttcgtatgcggtcgcatccagcagtgattccagttcgctttcatcgctggctttgattttaaagatccagccgcctgcatacggttcgctgttcaccagttccggggaatcgctcagtgcgtcgtttaccgccacgatttcaccgcttactggcgcataaatgtctgacgccgcttttaccgattcggcaaccgcgcagtcatcgcccgcgctaaccgttgcgcccacttccggcaggtcaacaaacaccatatcgcctaacagctcctgagcatgttcggtaataccaacggtgtaagtgccgtcggcttctttacgcagccattcgtgttctttgctgtatttcagttctgctggtacgttgctcatcaatcaatctccaaaaaagtaaatcacgcgacggctttgccgttacgcacaaaaacaggttttgtcactttaaccggcatttcacggttgcgaatttgcacaatcgccgtttcgccaataccttccggcacgcgcgccagcgcaatgctgtaacccagcgtcggggagaaagtaccgctggtgataatgccttcatgctggttgccctgcgcatcggtaaagcgtaccggcagttcattacgcagcacgcctttttcggtcatcaccagaccaaccagtttttctgtaccatgctcacgctgcacttccagggcttcacgaccgataaagtcacgatctgccggttcccaggcgatggtccagcccatgttggcggctaaaggagagatggtttcgtccatctcctgaccataaagattcatgcccgcttccagacgcagcgtgtcacgcgcgcccaagccacatggcttaacacccgcttccaccagcgcacgccagaaatcggccgctttttcattgggcagcgcaatttcatagcccgcttcaccggtataaccagtggtggcaataaacagatcgcccgcctgcacgccaaagaacggtttcatcccttccaccgcctgacgctgggcgtcattaaacagtgtggcagcttttgcctgcgcattcggcccttgcacggcaatcatggaaaggtcatcacgaacggtaatttcgatgccgaaaggttcagcgtgttgggtaatccaggagaggtctttttcgcgggtggcggagttaacaacgaggcggaagaaatcttcagtaaagtagtagacgatgaggtcatctatcacaccgccagaggcattcaacatccccgagtaaagggctttgccgcttttggtgagcttcgccacatcgttcgccagcagataacgcagaaactcccgggtgcggctgccgcgaagatcgacgatggtcatatgtgacacatcaaacattccggcatcggtacgtaccgcatgatgttcgtcgatttgcgaaccgtaatgcagcggcatcatccagccgtggaaatccaccatgcgagcgccgcaaagcgtgtgttgttcgtacaaaggagtctgttgtgccatcttgtcctcattgaataagcggggctgacaactttttcatggtgaaattatcaccacgaaacccagcatcggagccactcccggtccccaacgcaatcgttctcttttgcctgaacttaccaccgaaacagactgttaaccataaggtaaaattgatcatcacattagcttatggttaaaaaatgcaaaaatcgcgacagaataaaaaaccaaaaaatacaccagtttctatacaaagatgatgtgatgagaaagtcaatttgaataagacaatattaagagctaaaaaaatgtcaaaaaacactaaatcaaaaaataatggcattagaaaatataatgcgaaaacggaggtgaaattagtttatttcaaatgaggaaaatctcccggcgaaaaaaccgggagatgaaagtgtgatgggtatcaaataaacaacagaggagaaatttttaacgcagccattcaggcaaatcgtttaatcccattgcctggcggataagttgcggcttaacgccaggaagcgtgtcggccagtttcaaaccaatatcacgcagcagttttttcgccggattggtaccggaaaacagatcgcggaatccctgcataccagccagcatcaacgccgcactgtgcttgcggctacgctcatagcgacgcagataaatgtactgcccgatgtctttcccctgacgatgcaaccgtttcagttcggcaatcagctctgcagcatccataaagccgagatttaccccctgccccgccagcgggtgaatggtatgtgcggcgtcgcccaccagcgccagacggtgcgaggcaaactggcgcgcataacgccccgtcagtgggaacacctgacgcgcgctctcaaccttgcataagcccaggcgattatcaaaagcgatatttaacgcgcgattaaattcgtcttcacttgcctgctgcatccgctgcgcttcctctggcgacagtgaccagacaatcgagcaaagatgcggatcgctaagcggtaaaaaggccagaatgccttcgccatggaaaacctgccgcgccaccgcatcatgcggttcttccgtgcgaatggtcgctaccagcgcgtgatgctgataatcccagaaagtcagcggaatatcggctttgttgcgcaaccaggaattagcgccgtccgcgccaatcaccagacgcgccgttaacatgctgccatctttcagcgtcaggaaggtttcattttctccccaggcgacctgctgtaattctgcgggggctaacagagtgatatctgacgactgatgcgctttgttccacagcgcgtagtgaatcactgaattttcaacgatatgcccaagatggctatagcccatgctttgatcgtcaaacgaaatgtgaccaaagctgtctttgtcccacacttccataccgtgataacagctggccctacgagagagaatgtcctgccagacgccaagacgggtgagtaatttttcgctggcggcattgatagccgaaacgcgcagttgtggtggtgcattcgccgccagaggttcctgtacgcgctgctccagtacggcaacgcgtaagccgctcccctgtaagccacaggcaaccgccagccccaccatgccgccgccaacaatggctacatcaacactttgcattgtttattccttaaaaccgccttcaacgcgccacccaaccgagggtgcgctgcgccagcacatcgcgtgccggggtgaataattccatcgtcatcagcccgatgttgcgcccgacaaccagcggtgcccaacggttggcaaaaagatgtacaaggctgtccgtgacgccaatggttgcttcgcgatcgctctgtcgacgctgctgataacggcacaatacgccgtaatcccccatgtcttctccgcgctcctgcgcctgagtcagggtttccgcaagactcatcacatctcgcataccgaggttaaacccttgcccggcaatcgggtgcagagtttgcgccgcattgcccaccagcacggtacgatgggtaatagatctggcggcgtgggttaacgccagcggataagcactgcgtttaccagcgtgggtaattttcccaagtcgccagccaaaggccgactggagttcacggcaaaacttctcgtcactccacgacaacacctcttcgcgccgttccagtggatgacaccagaccagcgaacagcgtccgtcagacatcggcaacatcgccagcgggccatgttgcgtaaagcgttcaaaagcgcgcccttcatgcgcaacggaagtagcaacgttggcaatcacggccagttgttcgtaaggctcctgctgccagtcaacgccgcacgcggtggctaacgctgaatgggtgccatcagctgctaccagcacgcggcccgtcagcgtctcgccactctccagcgtcacttcaacgtgactctgagtacgggcaacgttagccacgcgatcagggcaatgcagcgttacgccaggtgctttacgcagcaatgcaaacagccgttgcccgacattgtgcaattcgacaacctgtcccagcgccgccagttggtaatcttctgcggcgagggtgacaaatccagcgtgaccacgatcgctgacatgcacggtggtgatggcagttgcgcaatccgccagagattgccagacgccgatgcgcgccagttgctgacaggtacccgccgccagcgctatcgctcgtccatcaaagcccggatgagcatgtgactctggcgcagtcgcttcaatcaaatgtaccggcagcgccccgtgacttaaccgggaaatagccagcgccagcgtcgcgcccgccatgccgccaccgacgatgattacgctcattgctttctcgcagcaaccatcaacgcttcgatttcttccggctttttcaccacgctggcggtgaggttttcgttaccggtttcggtaatcacaatgtcgtcttcaatacgaatgccgataccgcgatattgttctggcacttctgcatccggcgcaatatacagccctggctctacggtcagtaccatgcccggttccagaatgcgcgagcgatcctgaccataaacacccacgtcatggacatccagtcctaaccagtggctaaggccatgcataaagaaaggacgatgggcgttctgagcgatcagttcatcaacatcacctttcaggatgccgagttttaccaggccgctaaccatgatgcgcaccacttcaccagtgacttccagaatggaagttcccggacgatacaggcgcaggctggtttcgagagactccagcacaatgtcgtagatttcacgctgggcctgggtgaatttgccgttgaccgggaaggtgcgggtaatatcgccagcgtaacctttgtattcacaacccgcgtcaatcaacaccaggtcgccgtcgcgcatttcacactcgttttcggtgtagtgcagaatgcagccgttttcaccgctgccgacaatggtgttataggacggatagcgcgcaccgtggcggttaaattcgtggtgaatttcgccttccagatggtactcgaacattcccggacggcatttttccatcgcccgtgtatgtgccatggcggtgatttctcccgcgcggcggagtacggcaatctcttctggcgatttgaacaggcgcatttcatgaacaacaggacgccagtcgatcatcgttgccggtgcggtgagattttgccgcgaacctttacgcagtttttccagcgcactgttcacgattacatcagcatatgcatattcgccctgggcatggtaaaccacatccaggccgttaagtagttgataaagttgctgattgatttcgctgaatgccagtgcgcggtcaacgcccagtttctctggcgcggcatcctggcctaagcgacggccaaaccagatctccgccgtcaggtcgcgaacgcggttaaacagaacgctgtggttatgagtgtcatcgcttttaatcagcaccagcaccgcttccggttcgttaaagccggtgaagtaccagaagtcactgttctgacgataggggtattcgctgtcggcgctacgtgttacttctggtgcagcaaaaatcagcgcggcgctgccgggttgcatttgctccaccagggcctgacggcgacgctgaaactcttgccgggatatctcactcataacactctccttacgttttttgtttttagtgtagagtcggtttttgtacttctggcgcggtcggttgcggatgagtaaaggtgtcgtggcataacagcgcggcaacacgaacgtattcgatgatctcttcaagcgacatttcaagctcttcctgatcttcgtcttcgtcgtaacccagttgcgcaatgttacgcagatcgtcgatagcttcaccggtttcgccggtcactttatccagcttcggttgcgtaacgccaagaccaagcaggaagtgattgacccaacctgccaatgcatcagcccgatcgaaaacgctgacatcatcgccatcaggcagataaagctgaaaaaggaagccgtcatcctgcagggcatcgctggtggcagagtgcattttacgcagtgcctgtgccagctcatgaccgaaagccatgccttcgttcgtcaggtcgtgaagtagcggtagccatgagctgtcatcgttaccgccacatatcatcccgctgattaaaccatgcatctcagctggggtcagacccgtcccttgttggttcagatactggttcatttcgttgtaaccaggcatttcgttctgtatagacataagcattcgtcgtcaaagggaggaatattcatgatatgctaccactttgggccctggtggaccagaaaagggcttgtctcttctcatcagggtagctatagtgtcgccccttcgcagaccatgggtctaaagacgaaggcagcgcagtcaatcagcaggaaggtggcatgtctgcacaacccgtcgatatccaaatttttggccgttcactgcgtgtgaactgcccgcctgaccaaagggatgcgttgaatcaggcagcggacgatctgaaccaacggttgcaagatctgaaagaacgcactagagtcacaaatactgaacagttggtcttcattgccgcattgaatatcagctatgagttagcgcaagaaaaagcaaagactcgtgactacgcggcaagtatggaacagcgtattcggatgctgcagcagaccatagaacaagcgttacttgaacaaggtcgcatcaccgaaaaaactaaccaaaactttgaatgacacttttcggtttactgtggtagagtaaccgtgaagacaaaatttctctgagatgttcgcaagcgggccagtcccctgagccgatatttcataccacaagaatgtggcgctccgcggttggtgagcatgctcggtccgtccgagaagccttaaaactgcgacgacacattcaccttgaaccaagggttcaagggttacagcctgcggcggcatctcggagattcccttcttatctggcaccagccatgacgcaactaccagaactcccactgacattatcccgacaagaaatccgcaaaatgattcggcaacgtcgtcgtgcgttaacgccggaacaacagcaggaaatgggtcaacaagccgctacccggatgatgacttatcccccggtggtgatggcacatacggtcgctgtattcctctcttttgatggcgaactcgacacccagccactcatagaacaactctggcgcgccggtaagcgcgtatatcttccagttttgcatccctttagtgccggtaatttgctgttcctgaattaccatccgcaaagcgaactggtgatgaacaggttgaagatccatgagccaaaattggatgtgcgtgacgtgctacccctttcccgattagacgtgctgatcacaccgctggtcgcctttgatgagtacggtcagcgcctgggaatgggcggtggtttttatgatcggaccttacaaaactggcagcactataaaacgcaaccggtgggttatgcgcatgattgtcagttggtggaaaaactccccgttgaagagtgggatatccctcttcctgcggtggttacaccgtcgaaagtctgggagtggtaagggcgatacacccgcatcgccctgattgacatcgttgattctttgacctaatttagtgagtaagggtaagggaggattgctcctcccctgagactgactgttaataagcgctgaaacttatgagtaacagtacaatcagtatgatgacaagtcgcatcataacccttctccttcaagccctcgcttcggtgagggctttaccgttacagccccatgctgccctgccatcgtaaatccccattaaataaacacaacgcattgatctgactttgatttattttctggagcagactcgcaaagtagaatgcgcaacgcggcaacggtgtggagaagggataaaaaaacgggcaagtcagtgacctgcccgttgattttcagagaaggggaattagtacagcagacgggcgcgaatggtacccggaatagctttcattgcctgcagcgctttttcggcaacgtcttcgtcggcttcaatatcaataaccacataacccatctgggcggaagtttgcagatattgcgcggcgatgttgacgccctgctcggcgaagattttgttcagcgcagttagcacgcccggacggttttcgtggatgtgcatcagacgacgcccaccgtgcagtggcagcgagacttccgggaagttcaccgcagagagcgttgagccattgtcagaatacttgatcaatttacccgcaacttccaggccgatattctcctgcgcttcctgagtcgaaccgccaatgtgtggcgtcagaaggacgttgtcgaattcacacagcggagaggtaaatggatcgctattggtcgccggttccgtcgggaatacgtcgattgccgcccccgccagatgtttgctcgccagcgcatcacacagcgccggaatatccaccacagtaccgcgcgaagcattaatcagcagcgagccgggcttcattagtgaaatttctttcgcgcccatcatatttttggtggacggattctctggtacatgcagactcaccacatcgctcatattcagcaggtcagaaagatgctgtacctgagtggcgttgcccagcggcagtttattttcaatatcataaaagtaaacatacattcccagcgattcagccagaatgcccaattgcgtaccaatatgaccgtagccgatgatacccagctttttgccgcgcgcttcaaaagaacccgccgccagtttgttccacacgccacggtgcgctttagcattggcttccggcacgccgcgcaatagcagcagcagttcgccaatcaccagctccgcaacagagcgcgtatttgagaacggtgcgttaaataccgggatcccgcgctttgccgccgcatccagatcaacctggtttgttccgatacagaaacagccaatagcgaccagtttttctgcggcgttgatcacgtcttcagtcagatgggtacgggatcgcaggccgatgaagtgggcatcgcggatggattcttttaattgttcatcatccagcgcgcctttgtgaaattcgatgttggtgtaaccagctgcacgaaggctttccagcgccttttggtgcacgccttctaccagcagaaacttaatcttgtctttctccagcgatacctttgccatttacccaatcctgtcttttgaaatgttgtgtgcggatttgcatccgcctttcaacatatcaaaaaataatattgcggcaatatgaacgtttgcgtcgcgatgttgaggaaatatcacgcaaaggtaattcttggatgaatatgctggtttagaggatttatttagagcaatcgacaattgcctggtaaaagcgtgacacatgtcaccaaatttaatgaagagaatttttttaacgggggaggttcccccgtcagatcatttcacaatggttttgacaccgtcaggtgtgccaatcagcgcaacgtccgcgccacggttagcaaacaagccaacagtcaccacgccaggaatcgcatttatggcgttttccatcgctatcgggtcaaggatttccatgccgtggacgtcgaggatcacgttgccattatcggtcaccacgccctgacggtattccggacgaccgcccagtttcaccagctgacgcgccactgcactacgtgccatcgggataacttctactggcagcgggaatttacccagaatatcaacctgcttggaagcgtctgcaatacagataaatttttctgcaaccgaagcaatgattttttcacgggtcagcgccgcgccgccgcctttgatcatttgcatgtggccgttgatttcatctgcgccatcaacgtagatgccaaggctgtcgacttcgttgagatcaaaaacgtgaatgccgaggcttttcagtttttcagtggaagcatctgaactggaaacggccccttcaatctggcctttcattgtaccgagcgcgtcaataaagtgtgcggcggtggaacctgtacctacaccaacaatggtgccgggctgaacatactgaagtgccgcccatcctactgcttttttcaattcatcctgcgtcatgatcgtttcgcctgtggtatgaaatttcacacgcattatatacaaaaaaagcgattcagaccccgttggcaagccgcgtggttaactcatccataaaatatcgcgcaatggcaggcatcccctttcgccccgcaaataaagcatacaacggtctgggtatgccgctccacggtgcaaacaggcgcaccagttcaccgttcgcaagcccctgtttacaggcaaattgaggcaataacgccacgccattcaacacaaccagggcgcgaactcgctgagcgaaatgcattagcgcaaatccctgatcttttaagctgcgcttttaaccacggatacaaatgttacccgccgacggcttcggtatatgcaacctgacacaaaattgtgtcatagtgcaggaaaaagcatttaccaggagcagacaacagcaatgaaacgcccggactacagaacattacaggcactggatgcggtgatacgtgaacgaggatttgagcgcgcggcacaaaagctgtgcattacacaatcagccgtctcacagcgcattaagcaactggaaaatatgttcgggcagccgctgttggtgcgtaccgtaccgccgcgcccgacggaacaagggcaaaaactgctggcactgctgcgccaggtggagttgctggaagaagagtggctgggcgatgaacaaaccggttcgactccgctgctgctttcactggcggtcaacgccgacagtctggcgacgtggttgcttcctgcactggctcctgtgttggctgattcgcctatccgcctcaacttgcaggtagaagatgaaacccgcactcaggaacgtctgcgccgcggcgaagtggtcggcgcggtgagtattcaacatcaggcgctgccgagttgtcttgtcgataaacttggtgcgctcgactatctgttcgtcagctcaaaaccctttgccgaaaaatatttccctaacggcgtaacgcgttcggcattactgaaagcgccagtggtcgcgtttgaccatcttgacgatatgcaccaggcctttttgcagcaaaacttcgatctgcctccaggcagcgtgccctgccatatcgttaattcttcagaagcgttcgtacaacttgctcgccagggcaccacctgctgtatgatcccgcacctgcaaatcgagaaagagctggccagcggtgaactgattgacttaacgcctgggctatttcaacgacggatgctctactggcaccgctttgctcctgaaagccgcatgatgcgtaaagtcactgatgcgttactcgattatggtcacaaagtccttcgtcaggattaatccatcaaataatgcctgatagcacatatcaggcgttgtcctcacttctttttgtattccttgaatcacatcacaaaatagacaaatctcaggcggcaaaaaacgacgtctgaatgcattttttttgctggcgacaaacccacgtaaaaagctcaccgtaggcgcaaataccctcattttgattgcgttttacggagcaaataatgtctaacgtgcaggagtggcaacagcttgccaacaaggaattgagccgtcgggagaaaactgtcgactcgctggttcatcaaaccgcggaagggatcgccatcaagccgctgtataccgaagccgatctcgataatctggaggtgacaggtacccttcctggtttgccgccctacgttcgtggcccgcgtgccactatgtataccgcccaaccgtggaccatccgtcagtatgctggtttttcaacagcaaaagagtccaacgctttttatcgccgtaacctggccgccgggcaaaaaggtctttccgttgcgtttgaccttgccacccaccgtggctacgactccgataacccgcgcgtggcgggcgacgtcggcaaagcgggcgtcgctatcgacaccgtggaagatatgaaagtcctgttcgaccagatcccgctggataaaatgtcggtttcgatgaccatgaatggcgcagtgctaccagtactggcgttttatatcgtcgccgcagaagagcaaggtgttacacctgataaactgaccggcaccattcaaaacgatattctcaaagagtacctctgccgcaacacctatatttacccaccaaaaccgtcaatgcgcattatcgccgacatcatcgcctggtgttccggcaacatgccgcgatttaataccatcagtatcagcggttaccacatgggtgaagcgggtgccaactgcgtgcagcaggtagcatttacgctcgctgatgggattgagtacatcaaagcagcaatctctgccggactgaaaattgatgacttcgctcctcgcctgtcgttcttcttcggcatcggcatggatctgtttatgaacgtcgccatgttgcgtgcggcacgttatttatggagcgaagcggtcagtggatttggcgcacaggacccgaaatcactggcgctgcgtacccactgccagacctcaggctggagcctgactgaacaggatccgtataacaacgttatccgcaccaccattgaagcgctggctgcgacgctgggcggtactcagtcactgcataccaacgcctttgacgaagcgcttggtttgcctaccgatttctcagcacgcattgcccgcaacacccagatcatcatccaggaagaatcagaactctgccgcaccgtcgatccactggccggatcctattacattgagtcgctgaccgatcaaatcgtcaaacaagccagagctattatccaacagatcgacgaagccggtggcatggcgaaagcgatcgaagcaggtctgccaaaacgaatgatcgaagaggcctcagcgcgcgaacagtcgctgatcgaccagggcaagcgtgtcatcgttggtgtcaacaagtacaaactggatcacgaagacgaaaccgatgtacttgagatcgacaacgtgatggtgcgtaacgagcaaattgcttcgctggaacgcattcgcgccacccgtgatgatgccgccgtaaccgccgcgttgaacgccctgactcacgccgcacagcataacgaaaacctgctggctgccgctgttaatgccgctcgcgttcgcgccaccctgggtgaaatttccgatgcgctggaagtcgctttcgaccgttatctggtgccaagccagtgtgttaccggcgtgattgcgcaaagctatcatcagtctgagaaatcggcctccgagttcgatgccattgttgcgcaaacggagcagttccttgccgacaatggtcgtcgcccgcgcattctgatcgctaagatgggccaggatggacacgatcgcggcgcgaaagtgatcgccagcgcctattccgatctcggtttcgacgtagatttaagcccgatgttctctacacctgaagagatcgcccgcctggccgtagaaaacgacgttcacgtagtgggcgcatcctcactggctgccggtcataaaacgctgatcccggaactggtcgaagcgctgaaaaaatggggacgcgaagatatctgcgtggtcgcgggtggcgtcattccgccgcaggattacgccttcctgcaagagcgcggcgtggcggcgatttatggtccaggtacacctatgctcgacagtgtgcgcgacgtactgaatctgataagccagcatcatgattaatgaagccacgctggcagaaagtattcgccgcttacgtcagggtgagcgtgccacactcgcccaggccatgacgctggtggaaagccgtcacccgcgtcatcaggcactaagtacgcagctgcttgatgccattatgccgtactgcggtaacaccctgcgactgggcgttaccggcacccccggcgcggggaaaagtacctttcttgaggcctttggcatgttgttgattcgagagggattaaaggtcgcggttattgcggtcgatcccagcagcccggtcactggcggtagcattctcggggataaaacccgcatgaatgacctggcgcgtgccgaagcggcgtttattcgcccggtaccatcctccggtcatctgggcggtgccagtcagcgagcgcgggaattaatgctgttatgcgaagcagcgggttatgacgtagtgattgtcgaaacggttggcgtcgggcagtcggaaacagaagtcgcccgcatggtggactgttttatctcgttgcaaattgccggtggcggcgatgatctgcagggcattaaaaaagggctgatggaagtggctgatctgatcgttatcaacaaagacgatggcgataaccataccaatgtcgccattgcccggcatatgtacgagagtgccctgcatattctgcgacgtaaatacgacgaatggcagccacgggttctgacttgtagcgcactggaaaaacgtggaatcgatgagatctggcacgccatcatcgacttcaaaaccgcgctaactgccagtggtcgtttacaacaagtgcggcaacaacaatcggtggaatggctgcgtaagcagaccgaagaagaagtactgaatcacctgttcgcgaatgaagatttcgatcgctattaccgccagacgcttttagcggtcaaaaacaatacgctctcaccgcgcaccggcctgcggcagctcagtgaatttatccagacgcaatattttgattaaaggaatttttatgtcttatcagtatgttaacgttgtcactatcaacaaagtggcggtcattgagtttaactatggccgaaaacttaatgccttaagtaaagtctttattgatgatcttatgcaggcgttaagcgatctcaaccggccggaaattcgctgtatcattttgcgcgcaccgagtggatccaaagtcttctccgcaggtcacgatattcacgaactgccgtctggcggtcgcgatccgctctcctatgatgatccattgcgtcaaatcacccgcatgatccaaaaattcccgaaaccgatcatttcgatggtggaaggtagtgtttggggtggcgcatttgaaatgatcatgagttccgatctgatcatcgccgccagtacctcaaccttctcaatgacgcctgtaaacctcggcgtcccgtataacctggtcggcattcacaacctgacccgcgacgcgggcttccacattgtcaaagagctgatttttaccgcttcgccaatcaccgcccagcgcgcgctggctgtcggcatcctcaaccatgttgtggaagtggaagaactggaagatttcaccttacaaatggcgcaccacatctctgagaaagcgccgttagccattgccgttatcaaagaagagctgcgtgtactgggcgaagcacacaccatgaactccgatgaatttgaacgtattcaggggatgcgccgcgcggtgtatgacagcgaagattaccaggaagggatgaacgctttcctcgaaaaacgtaaacctaatttcgttggtcattaatccctgcgaacgaaggagtaaaaatggaaactcagtggacaaggatgaccgccaatgaagcggcagaaattatccagcataacgacatggtggcatttagcggctttaccccggcgggttcgccgaaagccctacccaccgcgattgcccgcagagctaacgaacagcatgaggccaaaaagccgtatcaaattcgccttctgacgggtgcgtcaatcagcgccgccgctgacgatgtactttctgacgccgatgctgtttcctggcgtgcgccatatcaaacatcgtccggtttacgtaaaaagatcaatcagggcgcggtgagtttcgttgacctgcatttgagcgaagtggcgcaaatggtcaattacggtttcttcggcgacattgatgttgccgtcattgaagcatcggcactggcaccggatggtcgagtctggttaaccagcgggatcggtaatgcgccgacctggctgctgcgggcgaagaaagtgatcattgaactcaatcactatcacgatccgcgcgttgcagaactggcggatattgtgattcctggcgcgccaccgcggcgcaatagcgtgtcgatcttccatgcaatggatcgcgtcggtacccgctatgtgcaaatcgatccgaaaaagattgtcgccgtcgtggaaaccaacttgcccgacgccggtaatatgctggataagcaaaatcccatgtgccagcagattgccgataacgtggtcacgttcttattgcaggaaatggcgcatgggcgtattccgccggaatttctgccgctgcaaagtggcgtgggcaatatcaataatgcggtaatggcgcgtctgggggaaaacccggtaattcctccgtttatgatgtattcggaagtgctacaggaatcggtggtgcatttactggaaaccggcaaaatcagcggggccagcgcctccagcctgacaatctcggccgattccctgcgcaagatttacgacaatatggattactttgccagccgcattgtgttgcgtccgcaggagatttccaataacccggaaatcatccgtcgtctgggcgtcatcgctctgaacgtcggcctggagtttgatatttacgggcatgccaactcaacacacgtagccggggtcgatctgatgaacggcatcggcggcagcggtgattttgaacgcaacgcgtatctgtcgatctttatggccccgtcgattgctaaagaaggcaagatctcaaccgtcgtgccaatgtgcagccatgttgatcacagcgaacacagcgtcaaagtgatcatcaccgaacaagggatcgccgatctgcgcggtctttccccgcttcaacgcgcccgcactatcattgataattgtgcacatcctatgtatcgggattatctgcatcgctatctggaaaatgcgcctggcggacatattcaccacgatcttagccacgtcttcgacttacaccgtaatttaattgcaaccggctcgatgctgggttaatgactcgtcccgtcacgatcttcagcaatatgctgaagcatcgtggcggtataacgatgatttctgattgaataaagatattcctgcatatacatcggcctgtgcggtgcatcaaaatatttcagcgttgccggattcaccagtcgccaggcaaaatgcgggatcaccgtcagaaaatgtccgcgctccacggcgctgattttggccataaaactgtagggacgataaataatggttggattgatcccacaaggtcgcatattcgcatcaatcattgcttcgaagttggcccggttctgaaagcgcatttgtagccagggcagctcctgaagcagctcttgctcttgtcgctcttcataacggcgagaaacgagaaagcctaatcgcagcggtggtagttcactgatagtcaggttttccagttcctgaactcgtgcagatacatgctgtggggagataataaaatctaactggcggtcaaaaagattatcgataacgccattttcgctgaactcaactggctgggcggtcacgccttcatacttatctccgagactaatcaactgatcgaaaataattgtcggataagtattatctatgccaatcacaatttctcgtgaacgacgccctgagttatggatttcattatcaatcgcagaaagccgttgataaaccgggaacagtttttgatacagttcctgtccggctttattgaggctgatattattatctttgcgggtaaatagcgtatagccaatttgttcttccagcgcggcaatgcttttaccaaatggcgaagccgtcatatggattttttctgccgcccgggcaatattattggtttgcgctaataaaatgaaattgcgcatctttttcgaaataaaaatgtccatccccctcccccgcatccttgtccgcttaaccgtttcagtcagcctatccttgatgaaaccgcgagcaaagataggtgattacgtcatggttttacagaaaattacagaaaaaggaggcaatatcgggtaaaggcattagcccgacgaatacgtcgggctacaaatattattgtgctgcaggtgttttagcgggttgttgatccacaggttctaactggaagaccacatcgacctgatcatcaaactgaatagcggcctgctcgtaagtttcctgggcggacaccggcgcggcatcggctttcatcatccgcaccattgggctgggctgatagttggaaacatggtagcgcacgctatataccggccccagtttacgatgaaagccgttcgccagttcctgcgcctgatgaatcgcgttatcaatcgctgccttacgcgctttgtctttataggcatccggctgcgccacgcccagcgacacagaacgaatttcgttaagacccgccttcagcgcgccatccagcaaggaattcagtttgtctaactgacggagcgtgacttccaccgttctcacagcgcggtagcctttaaggatacttttaccatcctgataatcataatctggctgggtgcgtaagttcgctgagctgatatcttttttcgcgatctgattgagttcaaggaaggaaatgtattgtgcgacgcgctcatctgcctgtttcttggcagtagcggcatccttcgcggccacgttaacttcaatcgcaagagtggcaatgtctggcaccgcatccacgcttgccgtaccggaggtgacaatatgcggtccatccggcaattcgttagcctgcgctgccatcccgctaatacccattaatgccgccagggcgataactttgaacttcacgttagtctctccgtgttaattgacttgcccaaaattcaggacctctggaggcaagcttagcgcctctgttttatttttccatcagatagcgcctaactgaacaaggcttgtgcatgagcaataccgtctctcgccagctgcaaggcaataaaccacataacacatcccacaaccagattgataatgcgctgtgcttttgccgtgcgcagacgcggtgccagccaggctgcgagaagagccagaccaaagaaccacaggaaagaggcgctaattgtcccgagtgcaaaccagcgttttggttccacatcaagttgcccgccaaggctgcccagtacaacaaaagtatccaggtaaacatgcggattcagccaggtcactgccaacatggtggcgataattttccatctgccttgcttcatgacttcggcgctggctaactcaatattactgctcattgctgttttaaaagcgccaaaaccataccacagcaagaaggctacgccgccccaggtgaccagcgccagcaaccacggcgactgcatcaataacgcgctgccaccaaaaatcccggcgcaaatcaggaccaaatcgctgatagcacaaagtaaggcaatcataatgtggtactgacgacgtatgccctgattcatcacaaaagcattttgtggaccgagcggtaggatcatagccgccccaagtgcaagaccttgaaagtaataagaaaacacgttggatattccgaattaagtatctgatgcagagactatatcgcgggattgttattagcggaaattgataatattaattggcaatcagaaaaactaataagagagaggccagagagtattatctggcctcagcgttgattacgcagctttgtcttctttcacccgcttaaagttcacatccatttgcgggtacgggaagctgataccggcggcatcaaattcacgtttaatacgctccagcacatcccagtacacgttttgcagatcgccgctgttgctccagacgcggaccacgaaattaatcgacgatgcaccaagttcgttcaggcgcacagtcatttcgcgatctttcaaaatgcgatcttcagactggataatattggtcaggatctgcttaacctgatcgatatcggaatcatacgccacgccaataataaattcgttacggcgaactggctcgcgggagaagttaataatatttccggcaataattttaccgttcggaataacgataattttaccgtctgcagtacgcatggtggtggagaaaatctgcacactcagcacagtaccggctacgccgcccaggtcaacatattctccggcacggaacgggcggaacatgacaagtaacacgccagcggccaggttagacagtgacccctgcaaagccagaccaacagctaagcctgcggcaccgagtacagcaatgactgacgcggtttgtacacccacgcgtcccagtgcagcgattagcgtaaaggcgataataccgtaacggactaatgcagaaagaaaatcagcaacagtggcatcgattttacgggagatcatcaggcgattcaccgcgttggaaatcatccgcgcgataatcaaaccaacgatgatgatcgcgagtgccgccacgatgtttactgcataacttagcagcagcgcctggttagctaccagccagcttcccgcgccgtttatgctatcgacaacattcaaatcttccattcaatattccttttcaactgactcaaaatggagaaatacactccgccgccttatgacgggcagtctgacaagggtaaacaataaagcataattttgccaaatagatcacagatttctcatctgaatcaccttgcttttggcgaaaaaatccccgcagagcggggctcagacagatatcaatgtgcgctttgtcatgccggatgcggcgtgaacgccttatccggcctacaaaaacctgcaaattcaatatattgcaggatacgtgtaggcctgataagcgtagcgcatcaggcaattttgcttttggcgaaaaaaagacccgcagagcgggccttgagataagcagaaaggaatatcttacagaacgtcgatcgcgttcagttcctggaatgctttctccagacgagcgatcatcgaagtctgaccggcacgcagccatacgcgcggatcgtagtatttcttgttcggctgatcttcgcctttcgggttacccagctgaccctgcagataagcttcgttcgctttgtagtagttcagaacgccttcccaggttgcccattgggtatcggtatcgatgttcatttttactacgccgtagcttacggagtctttgatttcctgagcagtagaaccggaaccaccgtggaatacgaagttcaggctgttgtgcggcaggttgtgtttcttggaaacatattcctgagaatcacgcaggatggtcggagtcagaaccacgttacccggcttgtaaacaccgtgtacgttaccgaaggacgctgcgatggtgaaacgcgggctgattttgctcagttcggtgtatgcgtaatcaacgtcttccggctgggtgtacagtgcagaagcgtccatgtggctgttgtccacgccgtcttcttcaccaccggtgcaacccagttcgatttccagagtcatgccgattttggacatgcgctccaggtatttagagcagatttcgatgttctcttgcagagattcttcagacaggtcgatcatgtgagaagagaacagcggcttaccggtagctgcgaagtgtttttcacccgcgtccaacagaccgtcgatccacggcagcagtttcttcgcgcagtggtcagtgtgcaggataaccggaacaccataatgttcagccatctggtgaacgtgatgcgcaccagagatcgcgcccaggatagcagcaccctgcggaacgtcagatttcacgcctttaccagcgataaaggaagcaccaccgttggagaactgaacgataaccggcgctttaactttagcagcggtttccagtacggcgttgatggagtcagtaccgacgcagtttactgctggcagtgcgaagttgttttcttttgctacctggaaaactttctgtacgtcatcaccagtgattacgccaggttttacgaaatcaaaaatcttagacatgtctcttgtcctgtatcgtcgggccttatactcgtcatacttcaagttgcatgtgctgcgtctgcgttcgctcaccccagtcacttacttatgtaagctcctggggattcactctcttgtcgccttcctgcaactcgaattatttagagtatgaaaaattgcgtgctctaaaagcgcgctgaaacaagggcaggtttccctgccctgtgattttttacttcttagcgcgctcttcgagcatcgctactgcaggcagtactttaccttccacgaattcgaggaatgcgccgccgccagtggagatgtaggagattttgtcagcaatgccgaacaggtcgattgctgccagagtgtcgccgccgccagcgatggagaacgcttcgctgtctgcgatagcgttagccacgatttcagtacctttgcggaagttcgggaattcgaacacgccaaccggaccgttccacagaatggttttcgcattcttcaggatttcagccagttcctgagcggaagcatcaccgatatccaggatctgctcgtcagctttcacatcgttaacagatttcagggtagccggtgcagtttcagagaactcggttgctacgcgaacatcagacggaaccgggatgttgcaggtggtcagcagacgtttagcttcgtcaaccaggtcagcttcgtacagggatttacccacatcgtggccttgtgccgcgataaaggtgttagcgataccaccaccaacaatcagctggtcagcgattttagacagggagtccagaacggtcagtttggtagatactttagaaccaccaacgatagccaccatcgggcgagcaggttctttcagtgctttacccagcgcgtccagttcagctgccagcagcgggcctgcgcacgcaacgtcagcgaatttaccgataccgtgagtagaagcctgcgcgcggtgagcagtaccgaatgcgtccattacgaacacgtcacacagtgcagcgtattttttggacagggtttcgtcgtctttcttctcgcctttgttgaagcgaacgttttccagaacaaccagttcaccttcagcaacgtcaacgccgtcgaggtaatctttaaccagacgaaccgggttagacagtttgtctttcaggtagttaacaaccggcagcagagagaattcttcgttgtactcgccttcggtaggacgacccaggtgggaagttaccatcacttttgcgccttgtttcagggccagttcgatggtcggcagagaagcacggatacgcgcgtcgctggttactttcccgtcttttactggtacgttcagatccgcacggataaatacacgtttcccagcaagatccagatcggtcatcttaattacagacatggtgaatcctctcgttgattctaaaagttttgcagacgctgcttgcgtcttacctgaaagcaacagtagccatagctaacgtcgtgtcgagcattcggttagcaaagccccattcgttatcgcaccagaccaacgttttgatcaggtgtgcgccactgacccgggtttgggtgccatcgacaatggcactgtgcggatcgtggttaaaatctacagagaccaacggcaattccgtatagtcaactataccatgaaatgcaccttgtgctgctttttgcagcaacaggttgacttcattggcttttacaggtttcttcaccgtcacgcttaaatcgattgccgtcacatttatggttggcacacgtaccgcaatcgcttcaaagcgatcgttaaattgcggaaaaaatcgtgtgataccggcggccagtttagtatcgaccggaatgatcgactggctggctgcccgggtgcgacgcaggtcaggatggtatgcatcaataacctgttgatcgtgcatggcggagtgaattgtggtcacagtgccggactcaataccgtacgcatcatctaacaatttgatgacgggaattatgcaattcgtggtacaggaagcgttagaaacgatgcggtgttccgcacgaagttgatcctgattgacgccgtaaacaacggtcgcgtcgagatcgttactgccaggatgtgaaaagagcacttttttggccccggcggcaatatgcgcttcgccatgctcgcgggagccatatacgccggtgcagtcgaggactacatcaacgccaagttcacgccaggggagcgattgcagtgaacgttcatgcaatacgcggatggcgtcatcaccaacaaaaagttgatcgcgttcctgtcgtacttcccatgcaaaacggccatggctggtgtcatatttcaacaaatgcgccatgcccgcagcatccgccagttcgttgattgccaccacggtaatttccgcccggcgtccggattcatacaaagcacgaaccacattacgcccgatgcgaccgaagccatttatcgctacgcgtacggtcatagatctcctgcaaggttttccctgagcaaatttgccagacagagtaatccagcaaatcgtccggggaaaccttacctgtcgcaaactgcgactgattggttaattgtcgaacatttaatcgactgaaacgcttcagctaggataagcgaaacgtggaataaaaggaatgtttgtccagccgaagaagacatttatctgactcacatcacacttttatccccttttgtgggaagctttattccaggctggcgtaataataaccctacaataactggaataaattgtcagcttgtgaagtgataccggccttcttcagtcatctctactatcagattggcctgacggctattcatcagcacacgctcgacattggggccatcggtgcgggcataaaatgcttcggctacttgccgcgttaatcctcccgcaattttacgactaatcaagcgctcccgcagaatttgagcaggtgcatgaataaaaatagaaaaatcgcagaaagatgccaactccagccacttttcatcatccagtaacaaccagtttccttcgacgatgacgagtggtgcggtaacgtgcaacgcatcttcaacaggatcatgcttttgtcgatcgtactgcggccacgtacaatccccttccacgacctggcgcagattttccgtcagtttcgcaacgtcaaatgtctctggtgcgcctttgaaggggcgcaattgatgcgcatccagccagctattgtaatggtgaaaaccatccatcgggagcgtctgaatagcgggcagttccgggtcttgttgcgcgagatattcccagaaggtggttagggttgatttacccgtccccggcggagcgcaaagaaaaaccaccgtacgccgctgcggatttaccgtctgtaaggccgccaacatgtgcagcaacggtttatgtacattttcaatctcttcgttctggtactgtgcctgtatcttcagcccattcaccgttaattcaattttcacggcgttaattcctttaaggtggtcgttactgccagcgtcagcgccgttttgaccattccgctaaaacgcgcctctgaccagacggagaaatcagcgaacttcatcgcttttaacgcgtcatagagcatcgcattgcgggttatgctattgacgttgctgataaaatcccaggtcatgtcatcggcaaatccgggcgtttcatcctgttcgttcaggtaatgccagaactgggaaaaatgcgtgatatcggcgtacaaccatttatccattttccccaacgcataaatcaaacgcagtgcaacatcaatatcgtcaagcgggccgctttgggcgagtaacggcttcactgcatattccacgatctcttcatcgttatcgacaaacagcgacggcagaaactggcgtatcccctggagcaaaatggtatgcgcagttttcataaatgaaaataaattgtcctgtgcatccagttgctcaagcacatcatcttctgtcagcgtcgccattggtcttccgatagatcaccatcaatgcagggagtctattatattacacgtttggtccgcgccgccgatcagtaatgtctgcgtccgcaccccattcgccgtctgttggataccgttcaccagctcaccgcccgtcacgcccgtagcgctaaagaggatatcgttccccctcaccagttcatcgagcgagtacacacggttaacgtcaacgcccattgccttgcaacgcttgcgctcctgctctgcaatctgccgattttccgtgtaatcccctttagcctggcaaaagtcaatcagctcggcctgcatatccccgcctaatgctttaacggcacaggcagaaatcacgccttctggcgcaccgccgatggtgtacatcacatcgtaaggattatcctgccagcaggtcagcacgctggcggcgacatcgccatccggcagggcaaaaaccttcacgcccagctgtgttgcttcctcaatcgcggcactcaggcgcggtttatccagcgtaaccatgcgcagcttatccagcggtttgcctaacgctttcgccacgttgcgcaggttgtccgtcagaggcaaagacagatcaatcgcgcccgccgccagccgattaacaaccagctttttcatatacatatcgggcgcatgtaacaggctatctcgaggggcgaaagccatgaccgccagcgcattgctctgccccatcgccaccatccgcgtgccttcaatgggatcaaccgcgatatcgacttctggcccatcgcctttgcccacctcttcgccaatccacagcatcggcgcatggtcaatttctccttcgccgataaccactcgtccacgaaaagcgacgtcgtttaatgcctggcgcatcgcggtgaccgccaggccatcaattttatttttgtcgccacatccggtttgcggccaggcagccaacgctgcctgttccgtaacgcgaaataatggccacgccagggacatcattgcgcggcctccccgatatcaacgccaaattgtgccagcagatatttctcggcctgttcattccagatgccgtgcgtttcctcaaccagccgcgccaactctttaaacagcggatcggttttgcctttttcggcaaaatcggcaatggcagtgagcggcatggtcacgccgttataaatgagttttttaccgccagggatatccggcagattgagcacggtttctggcaccgcatccaggccaccgatatgggtcaccataaacgacggctgtaactgcccagtggcgctaagggcaatcgcctctttcatgtcgtccgttgaaccgccagatgtaccgacgacgtgcgtgctgttgtaatggacgttgtagaaattaaacggcactttgaagtttttatccgtcggcccggcaaagaagttcagacagccatcttccgccagtaattcatcagccatctcaacgacagcaggcaccgccgcataaacaaaaatgtcatcgaacccggcatctcctgtcagcgcccgcagcatctggacaggatcgctcatccctttggtattcacatacaccagctcaatgcctttactggccgccagttccaccggcagcagcttctgtacctgcgccagacgtttgtcgtcgatatcgaccaccaccacccgcgacggttgtatgccgccgttaatggcgtaatcgatagcgccaatgcccatcggacctgcacacgccagcagtgcaatattgccgccaggtttgacgcccatgcgatgctcataaacatattgcgtggtgtgataattggcatgataagcaccaataatgcagcacataggctctgccagcgacgccgcagcaaaataagagccgtgatacggtaatacgcagcccaaattaatggcgatttcgggaataatcatataagtggcattgccgccaaaatattcgtagctgtagcccgctgaatatccgcttggtaaccccatcgccggttgcaatacaaaacgctggccttttttatatttgccagtgagatttttacccacttcgacaataaccccggcacattcatgcccggtaatgaccggatgattttctaaatcgtcgggtacgcgtttatgttcactaccgagtaacgccgctttccaggtcgataaacagacgctgtcagaaattacactcaccagtaattcattatcggtaatttctggcagttcaaatacgcgcagacggacatcccgcttgccataaatagcagcaactttggttttcatttttacctctgtaatcagtgtttatgttcggcggttaattgattaaataaagtgtcgagttttggatcgccaatatagttattaatcaatatcagtggtttatccgtcacacgtttcacgcgcccttccagactggcatgagtaacgacgatatccgcatccgcaggcacgttttctatggcgtaatgttttacttcaattgccagccccgctttttccaggcgtttacggaaggtggtcgcgcccatcgcactggagcccatccccgcatcgcaaacaaaggcgatacgcttaaccctgcttaacgagaatgcaccctcttgtttcatcgccttaaccgcattggctgactgagcaaactcatcttcgctctccgtttccaccgttttttccatcttcagtatcagcgaagtaatagcaaaggacaccagggtacctaccgtaacaccggcaattgtcgccaggaacgagcctttcggcgtcagtgccaggtaagcaaagatagaccccggacttgggccagccaccagaccaccgtccagtaagttaaacatccaggtgccagacataccgcccgcaatcatggcaataatggtcagcggcttcatcagcacatacgggaaatacagttcgtggatcccaccgaggaagtgaataatcatcgccccgggcgcagaacgtttactcatccctttaccaaacaaggtaaacgccagcagcagccccaggcccggacctgggttagaggccaccataaagaagatggatttaccgttaaccgaagcctgttgcattcccagcggataatagacgccctgatcgatcgcattattgaggaaaagcactttcgccggttcattgatgactgacaacaatggcagataacccgcatgtaccagcgcctcaatacactctttgacgaaagtattggcaattaacaccgccgggccgataacttcaaaacccagcagacaaaggagcatccccgcgatacctaatgagaagttattgataaccatctcaaaaccggcaggtatgcgtttttccagtgccttatcgacatattttatgaccaacccaccgagcggccccatgatcattgagccaaggaacatcgggatctctgcgccaacgatcacaccaatagtacctattccgcccatgaccgccccgcgtttaccgccgaccagatgaccacctgtagaaccaatcatcacgggcaataaataggtaatcatcgggccgacaattttggcgaaatgttcgttaggcagccaaccggtgggaataaataacgcagtaataaaaccccaggcaataaaagcaccaatattggggatgaccattgcagtcaaaaagcccccaaaagcctggacctttgcacgagcagacttgttttccataatattatcctgtagaggagagagtaattatccgcggctgataatgtccgctaattgtttttctgatgatgctgttaagagttgttcgagtatttcttcttcgcacagtaattcacttaacgcctgaatagcgccaatgtgcgaatcggcatcggcagcagagagtccgatgagtaatttaattggttcgtcattccccggaaaataaacaccttgttcaagtaatgtcaaagacatcccggttttaagcgccccacattccggtcgcgcatgaggcattgccacgcctggtgcgagaatataataagggccattgttaatggtggaatctttaattgcctgaatgtaattctcgctgatatagtttttatccagcaatgataccatcgagaaatcgatagcttcctgccaatcttttgctgaatgtataactgagattgatgattctggaaaataatcactaagccgcataaattatccttattttatttttagggtaccgtccggcggtaaaaataaaatactcgtgcggtttaatgaaagcaattgagcagggaaaccggtgttttgaaaacagtgaattattaatttcttatataacattgagttatagatataacaacaaatgtcaatacgcatatcgtgatgcatattacataattgatatttattgcatataaatatttgtgatctacaacacgccttatctattgcttgtccgcaaacggacatatcaaggtaataaaaaaggtcgccgaagcgacctttttacccgaaatgctaattacagcagttcttttgctttcgcaacaacgttatcaacagtgaagccgaactcttcaaacagcagctctgccggagcagattcaccgaaggtggtcataccgacgatagcaccgttcaggccaacatacttgtaccagtagtcagcaatacccgcttctacagcaacgcgtgcagtaaccgctttcggcagtacggattcacggtaagcagcatcctgcttgtcaaatgcgtcggtagacggcatggacaccacgcgcgctttcacgccttcggcagtcagtttttcgtaggcagcaacagccagttcaacttctgaaccggtagcgatgaaaatcagttccggctgaccggcgcagtctttcagcacataaccaccgcgcgcgatgtttgccagttgctcttcagttcgttcctgctgcgccaggttctgacgggagaggatcagtgcggtcgggccgtcctgacgctcaacaccgtatttccacgcgaccgcggattcaacctggtcacacggacgccatgtagacatgttcggggttacgcgcagagaagcgacctgctcaaccggctggtgagtcgggccgtcttcgcccagaccgatggagtcgtgggtgtaaaccatcacctgacgctgtttcatcagcgcagccatacgtacggcgttacgtgcgtattccacgaacatcaggaaggtggaggtgtacggcaggaagccaccgtgcagggagataccgttagcaatcgcggtcataccgaactcgcgaacaccgtagtggatgtagttacccgcagcatcttcgttgattgctttagaaccagaccacagggtcaggttagacggcgccaggtcagcagaaccgccgaggaattccggcaacagcggaccgaacgcttcgatagcattctgagacgctttacggctggcgattttcgccggattagcctgcagtttagcgatgaactctttcgctttagcgtcgaagtcagacggcatttcgcctttcatacggcgggtaaattcagcggcttcctgcggataagctttcgcgtaagcagcgaatttctcgttccatgcggattctttcgcctggcctgcttctttcgcatcccactgagcatagatttcagacgggatttcgaacggcgcatatttccagcccagttgttcgcgggtcagggcaatttcagcgtcgcccagcggcgcaccgtgggagtcgtgggtaccggctttgttcggggaaccgaaaccgatgatggttttgcacatcagcagggaaggtttgtcagtcactgcgcgcgcttcttctactgcgcgtttgatagatgccgcgtcatgaccgtcgatgtcgcgaataacgtgccagccgtaagcttcgaaacgcattgcggtgtcgtcggtgaaccagccttcaacgtgaccatcgatagaaataccgttgtcatcgtagaatgcaatcagtttacccagcttcagcgtacccgccagagagcaaacttcgtgggagatgccttccatcatgcagccgtcgcccatgaaggcgtaggtgtagtggtcgacaatgtcgtggcccggacggttaaactgcgccgccagcgttttttctgcaatcgccataccgactgcgttggcaataccctgacccagcggaccggtggtggtttccacaccagcggtgtaacccacttccgggtgacccggagttttagagtgcagctgacggaagtttttcagttcttccatcggcagatcgtaaccggtgaggtgcagcaggctgtagatcagcatggagccgtggccgttggacagcacgaagcggtcacggtcagcccaggacggattctgcgggttgtgtttcaggaaatcacgccacaggacttcggcaatgtcagccatacccataggggcacccgggtgaccggatttggctttctgtactgcgtccatgctcagcgcacgaatagcattggcaagctctttacgtgaggacattttgactccagatcggatgatgaagggcacgcccttaacgacttgacgacagcgcgttttgggctacgccggaaaatttgccaacaatttaccgcaagccgcgcgtcatgtacatggaacatccttttgccgcttcagaaatctctggatcatgctcgcatgttgcgcaatctactcgcccgtccgctgcgcttttccttatactgagactgagcgtcgattcacctgcaaacggcgcatttttagaataatcctgaccttgtgcggaagagaaaacatgaaaattcgcgccttattggtagcaatgagcgtggcaacggtactgactggttgccagaatatggactccaacggactgctctcatcaggagcggaagcttttcaggcttacagtttgagtgatgcgcaggtgaaaaccctgagcgatcaggcatgtcaggagatggacagcaaggcgacgattgcgccagccaatagcgaatacgctaaacgtctgacaactattgccaatgcgctaggcaacaatatcaacggtcagccggtaaattacaaagtgtatatggcgaaggatgtgaacgcctttgcaatggctaacggctgtatccgcgtctatagcgggctgatggatatgatgacggataacgaagtcgaagcggtgatcggtcacgaaatggggcacgtggcgttaggccatgtgaaaaaaggaatgcaggtggcacttggtacaaatgccgtgcgagtagctgcggcctctgcgggcgggattgtcggaagtttatctcaatcacaacttggtaatctgggcgagaaattagtcaattcgcaattctcccagcgccaggaagcagaagccgatgattattcttacgatcttctgcgccaacgcggcatcagcccggcaggtcttgccaccagctttgaaaaactggcaaaactggaagaaggtcgccaaagctcaatgtttgacgaccatcctgcatccgccgaacgcgcccagcatattcgcgatcgcatgagcgcggatgggattaagtaaagcctggtggtgtcgaacgtaggtcagataaggcgttcacgccgcatctgacatgaatggcacatttgttaccttgtgcgcattgccggatgcgatgctggcgcatcttatccggcctacgggtgccgaacgtaggtcggataaggcgttcacgccgcatccgacattaatggcacgttttacccgtgcgcatcgcatctggtgcttactcgccctttttcgccgcctgaatatacagcatttccagcgccagcgttgccgctgccagagcagtgatttccgactgatcgtatgccggagccacttccactacgtccatcccaacaatgttgagatctttcaggccgcgtaccagtttaatagcgcgatcggaggtcaggccgccaatcactggcgtaccggtgcctggtgcaaaagcaggatccaggcagtcgatatcaaaagtcaggtaaaccggcatatcacccacaatctgtttcacttgggcgataacgtcatccacgctgcgatcgttcacctggcaggcgtccagcacggtaaagccgttgtctttatcaaactcggtacgaataccaatctgcacggaatgattcgggtcgatcagaccttctttcggcgcggtatagaacatagtgccgtggtcaaattcacaaccgttcgcataggtatcggtgtgggcgtcaaagtgtaccagcgccattttgccgaaatgcttcgcatgagcacgcagcagcggcagcgtaacaaagtggtcaccaccgaaagagagcatacgcttaccggcagccagcagcttctcggcgtgcgcctgcagcttttcgctcatctcacgggcatcgccaaaggcatataccagatcgccgcagtccacgacgttcagacgctcacgcatgtcgaaattccacgggaagcggttgtgttcccaggccagattcgtcgaaacctgacggatcgctgccggaccgtggcgaccacccgcacgaccagaagtggccatatcgaacggcacgccagtaatcacccagtctgcatcgctgtcatacggctggaagttcatcggcaggcgtaaaaaaccaaaggcattggaaaccagtgagttatcgtattgatgacctaaggtgctcatggatggactcctattacaaagtcgatataaaaaaacccttccgcgtcgttaggcccgacgaggaagggttggatttgtcacaataaattgtggcggattatcaccgctaaattaagcggattcaagtaacacaggacttactcatcttcaagataagtataaccgtacaaacctgcctcgaactcttcaaggaactgttgttgcagttcagcatcaagatcggttttcttcacttgatcgcggaactgggttaacagcgttttcggatcgagctgtacatattgcagcatgtccgccacggtatcgccttcgtcagacagttctacttctacgctaccgtcagggaagacgaacacgtcaaccgcttcggtatcaccgaacaggttgtgcatgttgccgaggatctcctgatatgcgccgaccataaagaaaccgagcatcggcggattctctggatcgtactccggcattggcattgtcgtggcaataccgtcaccatcaatatagtggtcgatagcaccgtcagagtcacaggtaatatccagcagcacagcgcgacgttccggcacttgatccagcccttccagcggcagaaccgggaacaactggtcgatcccccatgcgtccggcatcgactggaacagcgagaagttgacgtacattttgtccgccatacgttcctgcagctcgtcgataatcggacgatgagcacggttttgcggatccagctgcttttgcacttcatggcacatgctcaaataaagctgctcagcccatgcacgttcttgcaggctaaagatgccggaagagtagccgatatgaatgtcgtgcagatccatctgactgtcgtgtaaccattcacgcagagaacggcgagttcccggttcgtgcatctcctgccaggtttcccacatgctttgcagcgcgcgcggcgcatcttctgcaggcgcggtcggcaccgtgtattcgttacgttccacgccgatgatattagacaccagcacggtgtgatgcgcagtcaccgcacgacccgattcggtgattaccgtcggatgcggcagaccgttttcttcacacgcatcgccaatcgcccagataatgttgttggcgtattcattgaggccgtagttcaccgaacagtcggactgcgaacgagtaccttcataatccacgcccagaccgccgccgacgtcgaagcactgaatattgacgcccagcttgtgcagttccacatagaaacgcgcggattcacgaacgcctgtcgcgatatcgcgaatattcgccatctgcgaaccgaggtggaagtgcagtagttgcaggctgtcgagacgcccggcttcacgcagggtttcaaccagttgcagtacctgagtcgcagccaggccgaacttcgatttttccccgccggaggactgccatttacccgaaccctgcgaagccagacgtgcacgcacgcccagacgaggaacgacattcagacgttctgcttcatccagcacaatggcgatttctgacatcttctcaatgaccagatagaccttgtgccccatcttctcgccaattaatgccaggcggatatattcgcggtctttataaccgttgcagacgatgacgctacgggtcatgccagcatgtgccagtactgccatcaactcggctttggaaccggcttccagacccagcggttcgcccgaatgaatcagggactcaatcacgcggcggtgctggttaactttgatcggataaacaaggaagtaatcgccgttatagccgtaggattccctcgcacgtttgaacgcggcgttaatggaacgcaaacggtgctgcaggatctgtgggaaacagaacagtgcaggcagacgctggccctgtgcttcacgagttttcactaactgcgcgagatcgacgcgagcttccgggacgtccgggtccgggcacacgctaatgtggcccagctcgttaacgtcatagtagttattgccccaccaggcaatattgtaagtacgcagcatcttgctggcttcctgggagctcattgcaacctcctgcatggagcgtagtacaccgtgttcgcccgctgacgaaggcaaacccatagacatgtcgtcagacatagcgaacctcaaattattttattaagtgtaaaacagttaacgactatcgcagcctggaactgcgataacaacccataagcacatggattttccagcagtgaatgctgacgctccaactgcgcaaccggtttctttttcataacattattaagcacataaccgaacgtaagtgtgaaagttcggcgaaaccacgagaaaactcttgtttttacaagagcgcccttgttcagtcctcagtaactgtaaccagctcttgaatcctgagaagcgccgagatgggtataacatcggcaggtatgcaaagcagagatgcagagtgcggggaacgaatcttcaccagaacggtgagacaggttaagcagcagacaacggttcattatttcgtatcacctccacggccgcctgttaagacgaacccacaagccaaaactctgatttcaacccggctggaagtggcaacacgaaagaaacgtcgtgtgctttttatttaagccgcgcgccgcgttttataccccacaatggcagaaaattgcaaaagataaatacgcagaatgccggcattgtcaggaaaaatttccagccacgtttttaacagaatgagacacgattcaaaaaaaagtggaaatagggtgaagaattgacctaaaatagccatccagatgttaatccatccataccgattaacactcagactgccagtgtttttaacctgcagagtcgtggtaggatccgctaccacagaaaatccacacaacagtttgagctaaccaaattctctttaggtgatattaaatatggcaaaacacctttttacgtccgagtccgtctctgaagggcatcctgacaaaattgctgaccaaatttctgatgccgttttagacgcgatcctcgaacaggatccgaaagcacgcgttgcttgcgaaacctacgtaaaaaccggcatggttttagttggcggcgaaatcaccaccagcgcctgggtagacatcgaagagatcacccgtaacaccgttcgcgaaattggctatgtgcattccgacatgggctttgacgctaactcctgtgcggttctgagcgctatcggcaaacagtctcctgacatcaaccagggcgttgaccgtgccgatccgctggaacagggcgcgggtgaccagggtctgatgtttggctacgcaactaatgaaaccgacgtgctgatgccagcacctatcacctatgcacaccgtctggtacagcgtcaggctgaagtgcgtaaaaacggcactctgccgtggctgcgcccggacgcgaaaagccaggtgacttttcagtatgacgacggcaaaatcgttggtatcgatgctgtcgtgctttccactcagcactctgaagagatcgaccagaaatcgctgcaagaagcggtaatggaagagatcatcaagccaattctgcccgctgaatggctgacttctgccaccaaattcttcatcaacccgaccggtcgtttcgttatcggtggcccaatgggtgactgcggtctgactggtcgtaaaattatcgttgatacctacggcggcatggcgcgtcacggtggcggtgcattctctggtaaagatccatcaaaagtggaccgttccgcagcctacgcagcacgttatgtcgcgaaaaacatcgttgctgctggcctggccgatcgttgtgaaattcaggtttcctacgcaatcggcgtggctgaaccgacctccatcatggtagaaactttcggtactgagaaagtgccttctgaacaactgaccctgctggtacgtgagttcttcgacctgcgcccatacggtctgattcagatgctggatctgctgcacccgatctacaaagaaaccgcagcatacggtcactttggtcgtgaacatttcccgtgggaaaaaaccgacaaagcgcagctgctgcgcgatgctgccggtctgaagtaatctttcttcacctgcgttcaaaggccagcctcgcgctggcctttttcttttggataggcgttcacgccgcatccggcaaaaaaaccgcccgcacaataacatcattcttcctgatcacgtttcaccgcagattatcatcacaactgaaaccgattacaccaaccacaacagacaaagatttgtaatattttcatattattattcggttttcacagttgttacatttcttttcagtaaagtcttaattgcagataacagcgtttaatctatgatgatataactcaattattttcatgcacttaaatcataactaagataaatgttagtgtaagcgattacactgatgtgatttgcttcacatctttttacgtcgtactcacctatcttaattcacaataaaaaataaccatattggagggcatcatgcctgacgctaaaaaacaggggcggtcaaacaaggcaatgacgtttttcgtctgcttccttgccgctctggcgggattactctttggcctggatatcggtgtaattgctggcgcactgccgtttattgcagatgaattccagattacttcgcacacgcaagaatgggtcgtaagctccatgatgttcggtgcggcagtcggtgcggtgggcagcggctggctctcctttaaactcgggcgcaaaaagagcctgatgatcggcgcaattttgtttgttgccggttcgctgttctctgcggctgcgccaaacgttgaagtactgattctttcccgcgttctactggggctggcggtgggtgtggcctcttataccgcaccgctgtacctctctgaaattgcgccggaaaaaattcgtggcagtatgatctcgatgtatcagttgatgatcactatcgggatcctcggtgcttatctttctgataccgccttcagctacaccggtgcatggcgctggatgctgggtgtgattatcatcccggcaattttgctgctgattggtgtcttcttcctgccagacagcccacgttggtttgccgccaaacgccgttttgttgatgccgaacgcgtgctgctacgcctgcgtgacaccagcgcggaagcgaaacgcgaactggatgaaatccgtgaaagtttgcaggttaaacagagtggctgggcgctgtttaaagagaacagcaacttccgccgcgcggtgttccttggcgtactgttgcaggtaatgcagcaattcaccgggatgaacgtcatcatgtattacgcgccgaaaatcttcgaactggcgggttataccaacactaccgagcaaatgtgggggaccgtgattgtcggcctgaccaacgtacttgccacctttatcgcaatcggccttgttgaccgctggggacgtaaaccaacgctaacgctgggcttcctggtgatggctgctggcatgggcgtactcggtacaatgatgcatatcggtattcactctccgtcggcgcagtatttcgccatcgccatgctgctgatgtttattgtcggttttgccatgagtgccggtccgctgatttgggtactgtgctccgaaattcagccgctgaaaggccgcgattttggcatcacctgctccactgccaccaactggattgccaacatgatcgttggcgcaacgttcctgaccatgctcaacacgctgggtaacgccaacaccttctgggtgtatgcggctctgaacgtactgtttatcctgctgacattgtggctggtaccggaaaccaaacacgtttcgctggaacatattgaacgtaatctgatgaaaggtcgtaaactgcgcgaaataggcgctcacgattaatctccccaagcttcctcccatcgcggaggaagccacctcttgcagtcatcttttcttcgctctatcctctgccgctatgaaaacatcccgtctccctatcgccatccaacaggccgttatgcgtcgcctgcgggaaaaactcgcccaggccaacctgaagctagggcgtaactacccggagccaaaactctcttacacccagcgcggaacctccgccggaacggcctggctggaaagctatgaaattcgcctcaatcccgttttgctgttggaaaacagtgaagcttttattgaagaagtggtaccgcacgaactggcacatttgctggtatggaaacatttcggccgcgtagcgccacatggcaaagagtggaagtggatgatggaaaacgtgctgggtgttcccgcccgtcgtacgcatcagttcgaactgcaatccgtgcgtcgcaacaccttcccctaccgctgcaagtgccaggagcatcagcttaccgtacgccgccataatcgcgtagttcgtggcgaggccgtctatcgctgtgttcactgcggtgaacagctggttgcgaaataaccatctgaactatcaggaactttcctgatctggctgattgcataccaaaacagctttcgctacgttgctggctcgttttaacacggagtaagtgatgtaccgttatttgtctattgctgcggtggtactgagcgcagcattttccggcccggcgttggccgaaggtatcaatagtttttctcaggcgaaagccgcggcggtaaaagtccacgctgacgcgcccggtacgttttattgcggatgtaaaattaactggcagggcaaaaaaggcgttgttgatctgcaatcgtgcggctatcaggtgcgcaaaaatgaaaaccgcgccagccgcgtagagtgggaacatgtcgttcccgcctggcagttcggtcaccagcgccagtgctggcaggacggtggacgtaaaaactgcgctaaagatccggtctatcgcaagatggaaagcgatatgcataacctgcagccgtcagtcggtgaggtgaatggcgatcgcggcaactttatgtacagccagtggaatggcggtgaaggccagtacggtcaatgcgccatgaaggtcgatttcaaagaaaaagctgccgaaccaccagcgcgtgcacgcggtgccattgcgcgcacctacttctatatgcgcgaccaatacaacctgacactctctcgccagcaaacgcagctgttcaacgcatggaacaagatgtatccggttaccgactgggagtgcgagcgcgatgaacgcatcgcgaaggtgcagggcaatcataacccgtatgtgcaacgcgcttgccaggcgcgaaagagctaacctacactagcgggattctttttgttaacccctaccccacgcgtacaaccgcgtggggagacgacgcggatttttaactatgcgtatcccccgcatttatcatcctgaaccactgaccagccattctcacatcgcgctttgcgaagatgccgccaaccatatcgggcgcgtactgcgcatggggccggggcaggcgttgcaattgtttgacggtagcaaccaggtctttgacgccgaaattaccagcgccagcaaaaaaagcgtggaagtgaaggtgctggaaggccagatcgacgatcgcgaatctccgctgcatattcacctcggtcaggtgatgtcgcgtggtgaaaaaatggaatttactatccagaaatcgatcgaactcggtgtaagcctcattacgccacttttttctgagcgctgcggcgttaaactggatagtgaacgtctgaacaagaagcttcagcagtggcagaagattgcaattgctgcctgtgagcagtgtggtcgtaaccgggtgccggaaatccgtccagcgatggatctggaagcctggtgtgcagagcaggatgaaggactgaaactgaatcttcacccgcgcgccagtaacagcatcaatacgttgccgttaccggttgaacgcgtccgcctgctgattggcccggaaggcggtttatcggcagatgaaattgccatgactgcccgctatcaatttactgatatcctgttgggacctcgcgttttgcgtacagagacaactgcgctcaccgccattaccgcgctacaagtacgatttggcgatttgggctaacggagaagaataatgatcaagctcggcatcgtgatggaccccatcgcaaacatcaacatcaagaaagattccagttttgctatgttgctggaagcacagcgtcgtggttacgaacttcactatatggagatgggcgatctgtatctgatcaatggtgaagcccgcgcccatacccgcacgctgaacgtgaagcagaactacgaagagtggttttcgttcgtcggtgaacaggatctgccgctggccgatctcgatgtgatcctgatgcgtaaagacccgccgtttgataccgagtttatctacgcgacctatattctggaacgtgccgaagagaaagggacgctgatcgttaacaagccgcagagcctgcgcgactgtaacgagaaactgtttaccgcctggttctctgacttaacgccagaaacgctggttacgcgcaataaagcgcagctaaaagcgttctgggagaaacacagcgacatcattcttaagccgctggacggtatgggcggcgcgtcgattttccgcgtgaaagaaggcgatccaaacctcggcgtgattgccgaaaccctgactgagcatggcactcgctactgcatggcgcaaaattacctgccagccattaaagatggcgacaaacgcgtgctggtggtggatggcgagccggtaccgtactgcctggcgcgtattccgcaggggggcgaaacccgtggcaatctggctgccggtggtcgcggtgaacctcgtccgctgacggaaagtgactggaaaatcgcccgtcagatcgggccgacgctgaaagaaaaagggctgatttttgttggtctggatatcatcggcgaccgtctgactgaaattaacgtcaccagcccaacctgtattcgtgagattgaagcagagtttccggtgtcgatcaccggaatgttaatggatgccatcgaagcacgtttacagcagcagtaacccaccttagcgagaaggatctcgttgagactctgagtgacagcgcccttctttccacgcatactgggcgctgttgcttttttgaaccaggaaacagaacctctgacaatgaatttacagcatcactttcttattgccatgcctgctctccaggatccgattttccgtcgttccgtggtctacatttgcgaacataataccaatggtgcaatggggatcatcgtcaacaagccgctggaaaatctcaaaattgaagggattctggaaaagctgaagatcacgccggagccgcgtgatgaatcaatccgtctggataaaccggttatgctcggcggtccgctggctgaagatcgcgggtttattttgcatactccgccctccaattttgcttccagcattcgcatttcagacaacacggtaatgaccacttcccgcgatgtgctggaaacgctcggcaccgataaacaaccgtctgacgtattggtggctctgggttatgcctcctgggagaaaggtcaactggaacaagaaattctcgataacgcgtggctaacggccccggcagatctgaatattctgttcaaaacgccgattgccgaccgctggcgcgaggcggcaaaactgattggtgtggatattctcaccatgcctggtgtggcaggacacgcctgatgagtggaaccttactcgccttcgacttcggcaccaaaagcattggcgtagcggtcggccaacgcattaccggcaccgctcgccctttgcctgcaattaaagcacaggacggtacgccggactggaacattatcgagcgtttactgaaagagtggcagccggacgaaatcatcgtcggtttgccgctgaatatggacggcaccgagcaaccattgactgccagagcgcgtaaatttgccaaccgtattcatggccgtttcggtgttgaagtaaagctccatgacgagcgtcttagcactgtggaagcccgttccggtctgtttgaacagggcggctatcgggcgctcaacaaaggcaaagttgactctgcctctgcggttattattctcgaaagctatttcgagcagggatattaaggcgatttaaacgcctggcggagtgtaaataatatcatcgcgtcttattgccggatgcggcgtgaacaccttatccagcacacatctggcagcggctataggtctgataagacgcgttagcgtcgcatcagacatttattgcctttgtaggcccgataagcttgcgcatcgggcatggcaacgtcacaaacgcccttcccccacccggtgctgataactctgctgaaacgttatcatccccacctgctgcccggtttgaataacatgcggtaactggtgggttttcccttcgcgaatcaaattccccaccgcgggtgtgttaatcagcaattcaaatagcgccacgcgtccttcctgtttatccacttccagcttttgtgacagcactgcccgtaaactacctgccagttgattacgcacggggtctttttcctgcgccggaaatgaatccaccagtcgctcaactgcctgcgcggcaccacgcgtatgtaatgttgccagcaccaaatgcccggtttctgccgccgtcagtgccagacggattgtctcgctgtcacgcagctctccgagcaaaatcacatcaggatcttcccgcaatgcggcccgcaatcccgatgcgaacgtcatacagtgcaaaccaatttcccgctgctggatcaaacatcgctggctggcatagagatattcaacaggatcttccagcgtcagaatatgcgcatcggcatgttgattgagatagccaaccatcgccgccagcgtggtagatttgccactccccgtcgcccccgtcaccagaatcaggccattctcgctcttgagtaattccggcaataccgttggtgcgccaagctgttcgagctgcgggcagtgcgaaggtaacagccgtaacgccagcgaaatgccatgccgttgcgcgaatgcgctgccacgcaatcgctggttttccgccagcgacacggcaaaatccagctgaccattctccagcaatattgcccgctgatcgtcatccagccactcccgcagtagctcttcgacgtccggcgtatcaaacggcgcagcttccattctgccgcgaatgcgccatcgtgcgggccaggcgctgcacaggtgtagatccgagacgttatgctttacactaagggccacaatttcttccatattcatactaagatcctcggaaaatgaacgatattgcgcataacctggcacaggtccgggacaaaatctcagcggctgcaacgcgttgcggccgttctccagaagaaattacgctgcttgcagtcagtaaaacaaaacctgcgagcgccatcgcagaagccattgatgccgggcagcgtcaatttggtgaaaactacgttcaggaaggggtagataaaattcgccactttcaggaactgggcgtaacaggattagaatggcattttattggcccgttgcagtctaataaaagccgcctggtggcagagcatttcgactggtgtcataccatcgaccgtttgcgcatcgctacccgtctcaacgaccagcgcccggcagaacttccccctcttaacgttctgattcaaattaacattagtgatgaaaacagtaagtccgggattcaactggctgaactggacgagctggcagctgcggtcgctgaactaccgcgtttacgtctgcgcgggttgatggcaatccctgcgcctgagtcagaatatgtaaggcagtttgaagttgcacgccaaatggctgtagcatttgccggactgaaaacgcgctacccgcatatcgacacgctctctctgggaatgtcggacgatatggaagccgccattgcggcaggtagcacgatggttcgtatcggcactgcaatttttggtgcgcgtgattactctaaaaaataaggaattaaaggaacgccatgaatacgttgactttcctgctttcaacggtcattgagctgtataccatggtgctgttattacgcatctggatgcagtgggctcattgtgatttttacaaccccttctcacagtttgtagtgaaggtaacgcagccaattatcgggccactgcgccgcgttattccggcaatggggccaattgacagcgcctcgctgctggttgcctatattctcagttttatcaaagccatcgtgctgtttaaagtggtgaccttcctgccaatcatctggattgccggtttactgattctgctgaaaaccatcggcctgctgattttctgggtcctgctggtgatggcgattatgagctgggtaagccaggggcgtagcccgattgaatacgtgctgattcagctggccgatccgctgctgcgcccgattcgccgcctgctaccggcaatgggtgggattgatttctcgccgatgatcctcgttctgctgctgtatgtcatcaatatgggtgtcgcagaagtattacaggcaaccggaaatatgctgctgccagggctgtggatggcgttatgaatgccgtaacagttaatgatgacggtctggttttacggctctatattcagccgaaagccagccgtgattctattgtcggtttacatggcgacgaagttaaagtcgccattaccgcgccgccggttgacggccaggccaacagtcatctggtgaagtttctcggtaagcaattccgggttgccaaaagccaggtggtgattgaaaaaggcgaacttggccgccacaaacaaattaaaatcattaatccgcaacaaatcccgccagaaatcgcggcgttaattaattaggtatcctatgcaaaaagttgtcctcgcaaccggcaatgtcggtaaagtgcgtgagctggcgtcgctgcttagcgacttcggtcttgatatcgtggcccaaacagacctcggcgttgattccgctgaagaaaccggcctgacctttatcgaaaacgcgattctgaaagcgcgccatgcggcaaaagtgaccgctttaccggcaattgccgacgactctggtctggcggtagatgtgcttggcggcgcgccgggcatttactccgcgcgttattccggtgaagacgcgaccgatcaaaagaatctgcaaaaactgctggaaacaatgaaagacgtaccggacgaccaacgtcaggcgcgtttccactgcgtgctggtatatctgcgtcacgcggaagatcccactccgctggtatgccacggtagctggccgggcgtgattactcgtgaaccagcgggcactggtggctttggttatgatccaatcttcttcgtaccttccgaagggaaaaccgccgccgaactgacccgcgaagaaaagagcgccatttcccaccgtggtcaggcgttgaaactgctgctggacgctttacgtaatggttaaattacctccgctgagtctctacattcacatcccgtggtgcgtgcagaaatgcccgtactgcgatttcaactctcacgcgttgaaaggagaagtgccgcacgacgattatgttcagcatctgcttaacgatctggacaacgatgtggcttacgctcagggccgtgaagtaaagacaatctttattggcggtggtacgccgagcctgctttccggcccggcgatgcaaacgctgctggacggcgtgcgtgcgcgtttgccgctggcagcggatgcagaaattactatggaagcgaaccctggcacggtagaagccgatcgctttgtcgattatcagcgtgctggtgtgaaccgcatctctattggtgtgcagagttttagcgaagaaaagctgaaacgacttgggcgtattcatggcccgcaagaagcgaaacgcgcggcgaagctggcgagcggtttagggttacgtagctttaaccttgatttgatgcatgggctgccggatcaatcactggaagaggcgcttggcgatctacgccaggccattgaactgaatccgccgcatctttcctggtatcaactgaccatcgaacccaatacgctgtttggttcgcgaccaccggtgctgccggacgatgacgcgttgtgggatatattcgaacaggggcatcagttattaaccgcagcgggttatcagcaatatgaaacttccgcttacgccaaacccggttatcagtgccagcacaatctcaactactggcgctttggtgactacatcggtattggctgcggcgcacacggcaaagtgaccttcccggatgggcgcattctgcgtaccaccaaaacgcgtcatccgcgtggttttatgcaaggaaggtatctggaaagccagcgtgatgtcgaagccacagataagccgtttgagttctttatgaatcgcttccgtctgctggaggccgcgccgcgcgtggagtttattgcgtataccgggctttgcgaagatgtgattcgcccacagttagacgaggcgattgcccagggttatctcaccgaatgtgcggattactggcagataacggaacatgggaagctgtttttaaattcgctgctggagctttttctggctgagtaaacttgtattgccggatgcggcgtgaacgccttatccagccgacatgtggcagcggttgtaggtctgataagacgcgcaagcgtcgcatcagacgttgattgccggatgcggggtcaacgccgcatcctgctacaaatcgtgcactatatcaaacttacttaatcaccccattgcgccgcagttgttcggtatcttttttccagcgttcattagcttggttgatatcgtcaattttcatcaaaatcgcgacttttttactgtttatttctgaaactttcatcgttaacggatattgccctttttcgagcgttacccagtcatcctgcaatttacggctaagtttttgtgattgcagaaaagtctgtcgccgttgttcgttgatatcgaaatctcgtttctgctgaatcggcacttcataacactcttcactctgtttatgacatgccgcaatcgccggttgataaacctctttgtcatatttaaccgcgaacgcctcgctatcgttctgtttattaaactcatcacgctgttggtgaatttttttaaaggcgtcttcgcgggtcatttgcttaccgtttgcatcttttccccaatatgcatccgctgctttctgcgccgccaccatttgcttatcaagcgctttcacttccttttccagcgcaggaatcgagttcttctgggtattcaacgcagattcaagctgactaaagcgataattgaaatcttcgctattcacgatcagatatttattattcgttttgatatcgtcgaccacccgcccacgatcgctggctgccgcctgaaaagagtaaaagttcaccgaccagccagacgcgggcgttcctttactggttaacatcgccgagaattttaccggtttatctttcgtccaggtctgttcgagcagttcgtaatctgccaactgaccgacccaggtatagagatcgtcactggaagagacatcgccttccgctgaccaggtggcctgattacccttagcatcaagattttttaaggtgatagcatcaagcttgagaatgccgtgatactgctttttgaattgatcttttaagatattttcagttggcggttcgccatctgcccaggcattaccagtcatcaacataagcagtgccgtgccaacaatccattgctttttcacccgaaaaacctcacgcggaataatttattccggtgattatcattagggtaattaaaattggcaatggacgtgagtctgaagtgaaaaagccccggcacgataccggggcgaggcgattagtactgattgaagatctgctggatctgctgcggatctttggtttgcgtcagagccagttgcagcagaacgcgcgctttttgcgggttcagcgtgccagaggcgacgaagccgtatttcgcatcatccacttcggcatcctgagtggtagcgcccgtcggtacgcgggaagaacgcacgactgcagtaccggttttcgcggcggtcgccagcgtgtcgaacacagatttatacaggttgccgttacccacaccagcgctaacgatgccatcatagcccgcatctaccagtgctttagccggaagatcggatgcgttagcgtagttataaacaatgccgactttcggcagttcattcagcttagagacatcgaatggcgtgtcgctggtatgcttacgtgccggggtacgctggtagtcaatcttaccgttgtgaatgtaacccagaggaccgtagttaacagacttgaaggtcgctacgtcggtggtgttggttttggtgacgtcacggccatcaagcacggtgtcattcatcactaccagcacgccacggttggcggaggctttatcagctgcggtcactaccgcgttatacaggttgaatggaccgtctgcgctcatagacgtggacggacgcattgcgccgaccatcaccaccggtttgtcgcatttcaccgtcaggtcgaggaagtaagcagtttcttccatcgtgtcggtaccgtgggtaatgacgaagccgtcggtcttatcgcagtcggtgttaatttttttcgccagtgtcagccagacattatcgttcatgtcctgggagccgatattcactacctgctcgcctttaacgttcgcaatgtcttttagttgcggcaccgcattaaccagattttctacgccaactttacccactgtgtagttagatttggttgcggagtcaccaccaccggcaatggtcccgccggttgctaaaatggtgatattgggtaatgccaatgctgcaccactaaaacccataaccagtgcggcaagtgccgtctttttgaaaaactccatttcattcctccagttacgtgaacgctacgcattatcccttagctctgtatgggaaatttgacgttaaacaatttacaacgtgaatatattttggagatctacaaagttagaggcaggtaacaaaacgaagaattaaacggcataaaaaagtattatgccgtcttaaaatagaggattattttaaattcccgaccagggctttgcggctatcttccagagtcacaacgcggctacaaacatctttgccaaactgctggaaatctttttcctgctttttccactcggtttggattgaggattgcagcccccccaggcttcccagcacattctgtaatgggttaccgccgcttttcagcaccgctttcgcgcccatttcattaatgctgtcctgtaaaattccacccattgcctgattcactaattgctggccttcggcgcgaacctgatcaatggctttatagtgaaacgtcaggccatcgctgcgcgtttcaataatgcggttcatctgctctttcagctgcgcatcaagtttggtcagacggctgcgcattttgctgctttcgcccatctcctgaacgataattttatccagagcaatacgggctttctcgacgcggcttttcgcgccttcatcaatccacggcagcgtgctgcgtagttcagcctgataatccttcgcctgctcgcgctgggcggcattcagggaatattgcttaccgttatacatcacgttgccgtctggcgtgatcaccagattgccgttttcgcccttcacctgcacggtttgcgggctgacaatcacatcgtcacgcggcgtgacgctgcactggtagtcggcgtgagcggtcattgccgtcactgaaagtgctgccgccagcagcattttgcgcatcatagtcttccctcaagaaaaaatcaggccagcatttgctggccccagattgataacaaagtacgcgttttccatgccggatgcggcgtaaacaccttatcccgcctactcgatcgtgcatctttccaggcctgataagcgtagcgcatcaggcagttttgcatttgtcatcgcccgtatgctttcttagtcccaccaaacgtcgaaaagttcgctggtgcgtacctcatccagtttgcgctcttccagccacttacgcacaatcgcctgatgttcttcggtgcatttgccgatttcctgcatgcagatcagaccttcccaggccagataaccgctgccgtcaaaggccagtttgttcggttcgataacctcgttaataaaatcatcaacggttttatcaatctgttcttccgatgtaccttccgggaatcgccatgccaccgaaaatcctaattcctggaattcgtcgatgtgcatttttttacgcagacgacggctacggttctttgccattatttcaccctctcgaacattaagtcccatactccgtgaccaagacgatgaccacgttgttcaaatttcgtcaccggacgtgatgccggacgcggtacgtaatcattgctctctgacaggtttttataaccgtcaatagaagacatcacttcaagcatatgttccgcataaggttcccagtcggtcgccatatggaatacgccccccagctgcagtttgctttttaccagttcggcaaacggcacctgaacgatacggcgtttattatggcgcgctttgtgccacgggtcagggaaaaagagctgcaccatgcgcaatgaattgtcaggaatcattttatgcagcacttcaaccgcatcgtgacacatcacgcgcaggttgcttaaaccttcttcatgcgcagaagccaggcacgcaccaacgcccggtgaatgcacttcaatgccgaggaagtcctgctcagggcgatctttagccattgccaccagcgacgcccccatgccaaaaccaatctcaagcgtcaccggcgcttcacggccaaaaagcgcggggaaatccagcatatcttcgctgaactcaacgcccatcaccggccagtagttttccagcgcatgttcctggcctttggtcagtcgcccctggcggcgcacaaaactacggatacggcgcagtgggcggccgttttcatcaaattccggtgaaatgacgtcgtttttcataaaggtttagtcgcttgtgaaagtgttctgaaaacgggcattatccaaagttagttgccggatgcaagcatgataaggccgtggctgcggaaagttccggtttacaccctgccgtcgctgtgctgcaatcttgcccccaacaacagtgaattcggtgaccatgcaagcgtcgcaattttcagcccaggttctggactggtacgataaatacgggcgaaaaactctgccctggcaaattgacaagacgccctacaaagtatggctctcagaagtgatgttgcaacaaactcaggttgcgaccgttatcccctattttgaacgctttatggcgcgcttcccgacggtgaccgatctcgccaatgcgccgctcgacgaagttctccacttgtggaccgggcttggctattacgcccgcgcgcgcaatctgcataaagcggcacaacaagtggcgaccttacacggcggtaaattcccggaaacctttgaggaagttgcagcactgccgggcgtcgggcgttccaccgcaggcgcgattctctcgctttctctgggtaagcactttccgattctcgacggtaacgtcaaacgcgtgctggcgcgctgctatgctgtaagcggctggcctgggaaaaaagaggtcgagaataaattatggagtttgagcgagcaggtgacgcccgcggttggcgtggaacggtttaatcaggcgatgatggatttgggtgcgatgatttgtacgcgctcgaaaccgaaatgttcgctctgtccgctacaaaacggatgtattgccgccgccaacaatagctgggcgctttatccgggcaaaaaaccgaaacagacgctgccggagcgcaccggctactttttgctattacagcacgaagatgaagtattgctggcgcagcgtccgccgagcggattgtggggcggtttatactgtttcccgcagtttgccgacgaagaaagtttgcggcagtggctggcgcaacggcagattgctgccgataacctgacgcaactgaccgcgtttcggcataccttcagccatttccacttagatattgtgcctatgtggcttcccgtgtcgtcattcaccggctgcatggatgaaggcaatgcgctctggtataacttagcgcaaccgccgtcagttggcctagcggctcccgtggagcgtttgttacagcagttacgcactggcgcgccggtttagcgcgtgagtcgataaagaggatgatttatgagcagaacgattttttgtactttcctgcaacgtgaagcagaaggtcaggattttcagctgtaccccggcgagctgggaaaacgcatctataacgagatctccaaagaagcctgggcgcagtggcagcacaagcaaaccatgctgattaatgaaaagaaactcaacatgatgaatgccgagcaccgcaagctgcttgagcaggagatggtcaacttcctgttcgagggtaaagaggtgcatatcgagggctatacgccggaagataaaaaataaaaacagtgccggagcacgcctccggcaacttgcataaaaacaaacacaacacgcacccggaatgatgaaaaaatatctcgcgctggctttgattgcgccgttgctcatctcctgttcgacgaccaaaaaaggcgatacctataacgaagcctgggtcaaagataccaacggttttgatattctgatggggcaatttgcccacaatattgagaacatctggggcttcaaagaggtggtgatcgctggtcctaaggactacgtgaaatacaccgatcaatatcagacccgcagccacatcaacttcgatgacggtacgattactatcgaaaccatcgccgggacagaacctgccgcgcatttgcgccgggcaattatcaaaacgttattgatgggtgacgatccgagttcggtcgatctctattccgacgttgatgatattacgatttcgaaagaacctttcctttacggtcaggtggtggacaacaccgggcagccgattcgctgggaaggtcgcgcaagcaacttcgcggattatctgctgaaaaaccgtctgaagagccgcagcaacgggctgcgtatcatctacagcgtcaccattaacatggtgccgaaccaccttgataaacgtgcgcacaaatatctcggcatggtccgccaggcgtcacggaaatatggcgttgatgagtcgctgattctggcaattatgcagaccgaatcttcctttaacccgtatgcggtcagccgttccgatgcgctgggattaatgcaggtggtacaacatactgccgggaaagatgtgttccgctcgcaggggaaatccggcacgccgagccgcagtttcttgtttgatcctgccagcaatattgataccggcaccgcgtatctggcgatgctgaacaatgtttatctcggcggaattgataacccaacatcgcggcgttatgccgtcatcaccgcctataacggcggcgcaggcagcgtgctgcgagtcttttcgaatgataagattcaggctgccaatattattaacaccatgacgccgggcgatgtttatcagacgctgacgacccgccatccctctgcggaatctcgccgttatctttataaagtgaataccgcgcaaaaatcctaccgccgccgataattccattaaccgcccctgacgatgctcaggggcaaaaatgttatccacatcacaatttcgttttgcaaattgggaatgtttgcaattatttgccacaggtaacaaaaaaccagtccgcgaagttgatagaatcccatcatctcgcacggtcaaatgtgctttttcaaacactcatccgcatcacgatgtgaggaaattaacatgaatcttaagctgcagctgaaaatcctctcttttctgcagttctgtctgtggggaagttggctgacgaccctcggctcctatatgtttgttaccctgaagtttgacggtgcttctattggcgcagtttatagctcactgggtatcgcagcggtctttatgcctgcgctgctggggattgtggccgacaaatggttaagtgcgaaatgggtatatgccatttgccacaccattggcgctatcacgctgttcatggcggcacaggtcacgacaccggaagcgatgttccttgtgatattgattaactcgtttgcttatatgccaacgcttgggttaatcaacaccatctcttactatcgcctgcaaaatgccgggatggatatcgttactgacttcccgccaatccgtatctggggcaccatcggctttatcatggcaatgtgggtggtgagcctgtctggcttcgaattaagccacatgcagctgtatattggcgcagcactttccgccattctggttctgtttaccctgactctgccgcatattccggttgctaaacagcaagcgaatcagagctggacaaccctgctgggcctcgatgcattcgcgctgtttaaaaacaagcgtatggcaatcttctttatcttctcaatgctgctgggcgcggaactgcagattaccaacatgttcggtaataccttcctgcacagcttcgacaaagatccgatgtttgccagcagctttattgtgcagcatgcgtcaatcatcatgtcgatttcgcagatctctgaaaccctgttcattctgaccatcccgttcttcttaagccgctacggtattaagaacgtaatgatgatcagtattgtggcgtggatcctgcgttttgcgctgtttgcttacggcgacccgactccgttcggtactgtactgctggtactgtcgatgatcgtttacggttgcgcattcgacttcttcaacatctctggttcggtgtttgtcgaaaaagaagttagcccggcaattcgcgccagtgcacaagggatgttcctgatgatgactaacggcttcggctgtatcctcggcggcatcgtgagcggtaaagttgttgagatgtacacccaaaacggcattaccgactggcagaccgtatggttgattttcgctggttactccgtggttctggccttcgcgttcatggcgatgttcaaatataaacacgttcgtgtcccgacaggcacacagacggttagccactaattacgcaaagaaaaacgggtcgccagaaggtgacccgttttttttattcttacttcaacacataaccgtacaaccgtttcacgccatccgcatcggtttcgctataaacaccttgcagctccggcgaaaatcccggcaacaaattcaccccttcttccagtgcaaggaaataacgttgaaccgccccaccccagacttccccgggtaccacgcaaagcacgccaggtggataaggcaacgccccttctgccgcaattcgcccttcggcatcacgaatccgcaccaactccacgtcaccgcgaatataagcgctatgcgcatcctgggggttcatcaccactgacgggaaactctgctggcggaacatcgctttttgtaggtctttgacgtcgaaactgacatacagatcgtgcatctcctgacacaactggcgcagggtgtagtcgcgatagcgcaccggatacttgttataaacgctcggcaacacctcaaccagcggcgagtcatcctcaatatgctgttcaaattgcgccagcatcgccaccagttgtgccagcttctcgtggctttccgccggagttaataaaaacagaatggagttgagatcgcacttctccggcacaatgccgttctcacgcagatagtgcgccagaatcgtcgccggaacgccaaagtcgctatattcgccggtttcggcatcgatacctggtgtagtgagtaacagcttgcacggatcaacaaaatactgatccgcggcatatccttcaaagccgtgccacttcgcccccggctcaaaactgaaaaaacggcggtcgctggctaacactgatgtcggataatcctgccacaatttgccatcaacaacgggcgggataaacgggcggaacagcttacagcgcgcaagaatagccttgcgcgcttcaatccctatctcaacacactcagcccacagccgacgcccactctccccttcatgaattttggcgttaacatccagtgcagcaaacagcggatagaaagggctggtagaagcatggagcataaaggcgttattcaaccgcttatgcgggcaaaaacgcgcctgtccgcggatatggttatcttttttatggatctgcgacgtctgtgagaatcccgcctgctgtttgtgcaccgactgagtcacaaagatccccggatcgttttcgttaagttctaacagcagcggcgagctatccgccatcatcgggataaattgttcataaccgacccacgcggaatcaaacagaatgtaatcacacagatgcccaacggtatcgatcacctgacgggcgttatagacagtgccgtcataggttcccagctgaataatcgccaggcgatacgggcgcggcaggtcggctttttctggcgcaacgtcgcgaatttgctggcgcagatactcttcattaaaacagtgcgcatcaataccgccaatgaaaccaaacgggttgcgtgaagcttccagatagaccggcgtcgcccccgcctgaatcagcgcgccgtgatgattcgacttatggttgttacggtcgaagagcaccagatcgccacgcgttaacagcgcattcgtcaccactttattcgctgccgatgtgccgttcagcacaaaataggttttatcggcatgaaagactttggctgcgaatttctgcgcatctttcgccgatccttcatgaataagcagatcgcccaattttacgtcagcgttacacatatcggcgcgaaagacgttctcaccaaagaaatcgtaaaaatggcgtccggcaggatgctttttaaaaaacgcaccatgttgatgtccagggcaagcaaaggtgctgttgcccatctcaacgtactgcgtcagcgtgtcataaaacggtggcagcaaattctcttcatactgacaggctgcggattccagctccagccactgctgctcgttgccgttgattaccgccgtaacgcccgcaggtaattcaacagcatgttcggaatacaaaaacaccggtagatgaaaaccggtgcgcttaagcaacgcaagaatgccactgcgactatccgcagcggtaatgacgactgccgcgacgtccgtaaaatcagtatctcccaacgccaccacgcgacgatgagaagaaagtcgggataccagttcactactggcggcaatattcattgatttcataagcgcaaacccgtttcggggaagtaagaataccggacaaggtggaaaaccctgccccatgagatatgggtcaaactggtcaccagctccgaccgccagacatcagtaaaagcagaaacgctctgattttactgttgtcctgcagtgagcgtgcgttaacttcaccgcatgagcagtaacatagaaagggaaacgtttcgcgcgaaacggcgataagcgagagaatgtaaggagatggcgtgcatcgggcaaactccgtacagagaggagaaaattcgcgcaatcatggcacctttcgctaaagcgtgcaagccaggactttgcgaacaaacaagccatcgacggcaccaaacggtcataataagaaaatcaaacaatacagctaacaggaactcttgtggtcatcggcccttttatcaacgctagtgcagtcttactgggtggcgttctcggcgcactgctcagccaacgcttaccggaacgtatccgcgtctccatgacatcaatttttggtctggcatcgctggggattggtattttactggtggtgaaatgtgccaaccttccagcgatggttttagctacgctacttggcgctctaattggcgaaatttgtttgctggagaaaggtgtcaatacagcagtcgccaaagcacaaaatctgtttcgtcactcacgtaagaagccagcgcatgaatcttttattcagaattatgtcgcgattattgtcctgttttgcgccagcggcaccgggatcttcggggcgatgaacgaagggatgaccggcgatccgagtattttaatcgccaagtcatttcttgatttctttacggcgatgatcttcgcctgctcgctgggtattgcggtatcggtgattagtatcccattactgatcatccagttaacgctggcgtgggctgccgcgctgattttaccgctgaccacaccgtcgatgatggcagacttcagcgccgtaggcggtttattgctgctggcaaccggattacgcatctgtggcattaaaatgttcccggtggtcaacatgcttccagcactccttctggcaatgccgctttccgccgcctggaccgcctggtttgcctgacaatgcgtgcaatatcggcaaagtgatgatagattgtgcagtctgcagtaaattgaagaaatttgattgacgagacgaggcgaatcaggtttaatgcgccccgttgcccggatagctcagtcggtagagcaggggattgaaaatccccgtgtccttggttcgattccgagtccgggcaccactaattcttaagaacccgcccacaaggcgggtttttgcttttggatctgacaataaccttcacgaaaaaaattagcttataaagtctgggggaattactctcgccacgttaacgagagtaattttattgatattaatctcctgatactttacccccgtccaaactccagccgctgcacattcaccatcccaggcttctcagcagcactgacatcaatttgtgtcacccgcagcgcatatttttcatccagtgcgtttaaccatttcagcaggtcattaaacaccacaggttctatccagacctgaatattctccccacgatcggctatccgcctgatgaccaccgagtgcgcggaagcactgtcactgatgacccgcgatacctgcgcaggcgttgttgtggcagattttcgcgctgcaataatatccggcgcggcgttcttcagtcgggtgttcatcgccaccagctgctgcaatattgtctcctgttgctcaatccgttcgctcaacggctgccagatgaggacgtaatatccgacgctaaacaggaacaccaccgctgccagtaacatgcccttttcacgcggagaacgccccgccaggtgttgtgccagccagtgttcgccacggcttaactggcgttcacgccattgctgaaaatagtgaataaatttatcgcgtaacatgttatttcctccgcaacgttacgccgccggaaaccgcatcaccctctttctgtaacgcgtcctgttgcacaacataatcggttgccagtacactacgcagtttgtcgaaactggcaaagttcgcggcccgtagctggaggtgaagtatctggcgtttttgatcaaaggtaaaaccacgcatttcgatgtcggaaagtgacgctgatttcagggtgctggctatcgctgacaactcggcgagcagccgggtatcgtcggcctgtgggcgatattttttcagcgccatcgtcacctgagagcgtaaattcacaatccgcttctgctccgggaacaacgttaagaactgttcctccgcctgggtgcggctttgcgccacctgttcgctgacgctccataacgtcacgccccgctccactgccagcgcaaccagaatcagcaatatcggcagaatcatcacccgccagcgcgcccactgttttcggtagctgacgcgaggctgccacggccctgtcagcaggttcccttccggttcgccataagtggtaatggcgggcagagctgtaacggtcaggcgttcagcgtctgcgccagcccatgctgatagcttttccggtgcaatgccgactacggttagcgaaagcggtaaatcctgctcattgagctgggcgcggaacatgaccggagccagcgccagcccggcgctccatccccggcattcatcgatgcggcagataacccgttgcgcatcgcaagccataaacccacaaggaatggacatccagtccggcgcgacggtagcgcgggtgatgccgttttcctgcaaccactgcgcaatgttgcgcatatgctgttggtgaatcactgctacggttgccagttgctggtcgatattcaacggggcgaaatgcagttcatcgatatcctggttcagctcttcttccagtaaggcgggcagaatagtcggtagcgcagcgcgatggaaatgtcgtggcgcgcacccttgcgtaaaaccgtaagttgaatggaatccattgaaggtaactgccgcatcagagcaatcattgctcgtggatcagtgaaatcctgctgatttagcgcaatggcgatatcgccttccttgaaaccgctggcatcgaacagagaacgatctgcccccggcttcgctgcataaccgacaatcccctccttacgcacaggcgtaagctggatatagttaaaaattttctgcggatctttcgccagtgcctgacgcacggcagccgggatctcaactggcacactgacagcaggctcagcaacagcttgctttgcttcgtcactgacggcttttttgttggtcacagcaacagtggaacgttcctcttctgccagactcagacgctctatttttccctgataacgcagcatcacatggtcgcggttgatttcctcaatcaccgcgttgtgagagccaagcgtttcaccctgcaaatagacctgctgtttaccgccttcttcaataaccgcgccgggtctggcaccaaaggcgatcccacgcagcaccacattaagacgcgtttctgccacaggcacaggttcgggttgttttacctgcgcggcgacaggctgatatttgccaaaccagttttgctggctgattaattgcacgtcatttttatcgaacgtttttgcatccacacggctcggtttattcaccggttgagaaaccgccgtatattccgcagaaaaggagatatagcgccagagtgaatgcgccatttttgcagaaataataagcagcatcagccagaacatcccgcgtgcaatttttcgcagatgctctttgtctgtattaagagattgtctctggttaagagtgtgacgaatttttgtcagccattgaatgagataaattcgtgcgtcacgaaaaacaacccgcgccaatttatatctacccgacgttatgctttgactattccacaggtggtacgatccagtttccgctgatactggttacctgtacgtgtatcattaatcgttatgctgtaattaattccctcagtgatcattaatttcaccgtcgggtcagcgcacatttgtcgttgatagctggttaaaaaggcgtcaggcgtctgcgtggtttgtgtacccgcttcgctgataatggtcatttttaccgttgtgccgctactttgcgccagcactaaggtatatcccgcagatttaatcggcaggttttggctgatattttgcgcctgttttttcgccagtaaactggcattttcattatggctggcacagccacttaataatcctgtaacgctcaacaatagcgatattaataccctccctggcatttgttttatcgacatggtaaataatctctaaggttattaataagagttaaaatgtcactttgataatgacgtggttatcattaaaacaatgcctgtagataaagtgttgctataccgcccagacttaaacacggtccaaaaggcagtgtggttgatcctctttttgtaataacggcatatatcaggccgcagcatgaggcgattaaagcaacattgggcagcgacaatgcccccacccagccacctaacgcggcgaaaagtaatacatcgcccatgcctaatgcttctttacgcagaactattccggctatccaacgcagagagtaaaaagtgataaatcccaccaggacgccggtgactgcatcttgtagcgtgagcggactctgctgcgcccatgccgcaatcagtcctgtccacaatacgccctgagtaaaaacatcgggcagccattggtgatcgaggtcgatgacactcgcggcaatcagccaggcggataatatcatcaccgccagcccccatccactttctggccagaccagactcgccagcaaaaaagcaagtgctgtcaataactccaccagcggataacgcttgctgattttcgcctgacagtcgcggcagcgccctttgagcatcagccaggagaacagcggaatattgtcacgtatccggatggtctgctgacaatgtgggcagtgcgaacgcggtagcgcaaggcttatttttgactgcgcactcgacatttcaccgtgaaactccgccatttgttggcgcagcatgattgggtaacgccaaatcaccacattcaaaaaactgccgatgatcaatcctccgacggttgccaggacgggcatcgccgtggggtattgctgaaaaacatcaaaaagcatggttaaaggttgtttgttgtaacttgctggatgcggcgtaaaacgccttatccgtcctacgggtgtctgccagcgcaaataatcgcggctttccccgtctgtaggcccgataagcaggcgcatcgggcaaatgtgttaacccggtgcgccttatttcatgccggatgcggcgcgagcgccttatccggcctacgggcttactcggcagacatcttatgctcggtaacctgattaatggtttccggtccctgttccggtttcggcagatcgagtgacgcgagcgtgttgtaagccgactggctcacaccgccctcgaagctcatctcgctcgcccccggcagctggtaagcattcgcgcccggattccatttcttaaagaactccgaaagatccgtctgggcgacccaggaggcacacagcatcagcgtgtccgctgcgttaccgttggattcagcacagtaattcttgccgccaaacttgtcattgctgacctcatcgccgcgtgctttacgatgcatcaactggaacaggttccagcctttcatcccttcacgctcgctgtaaaactctggcagaggagtgccatctggataccatttcttgatatcaaagtttttctctgcccattccttcagctgtgcgtacatcagcagacggtcacccgcaccgccgcgtgcccatgcctggttgttgctctcctccagatattccggtgcgacggtaatatcgtcagcgacacggttcatcttgccgagataacgatcctgcatgtacagcgccagcacgttgttagcgacttcagttgcacccggtacagtcaacggcgtttctgcggcgttatgaccgacttcatgccagatcagccagtcgttcagcggcgtcgtcggcagcgtggtgctgttcggcgagaagctgctgttcattaccggataacccgaatgcgcatcaccgatggagatctgcacatcgttggtgaaacgatgtttgtggcccggcaagtttttataggtaaacatccggtgcttaccgtcttcgctatcacggccgtagaagtcattcatcgagctggcaaaggtatccagatcgttagcgaattgctccagtccgccagtgtaattgctggcattcaggttcttcttcggtgtggtatagacgaaagcgtctgattccagctcacccagcggagccggtgagttcagatcgtttttccatgcgccgtctttatagaacggtgcttttaccacgccagtaaaggtgaagctggcagattcattggtagagctattgcccttgatataaatcaggccaccgtaaggcaccttgaacttcaccgtaccgctagcgtccagagagtacgttttagtcactcttggcggacggttcagcgcaacttcatgcttctcacgtccggtcaggtcgtcagccagcgccacggtgacggtcacaggaacgttcgcattggacttaatggtgacctctttctgagccggtgcccacaggccagttgactgcatgttacctgcaaaccatttggtcggattcgagtacaggctgatggtttcagtaacgttctgtccctcttccgatactgctcccggatacttctcgacatcaactttgatgttcagatcccaccaggaacggcccagcatcaggcgtgtcagcggtttttccatatagttgagcgggtagctcgggttcatcatgcccgctttgctgctaccgtcaccgtagatcatgttgttatcgaccagcgattttttcagatctgcagaacacttggtgccgcctgcataggcatcattggcgtagcagttcaggaactcggtgaacgttttaaagcccagctcgtcatttttgccttcttcataacgatagctcgtatcgttccacagccagaccgacatgttctggtacagacgttccagatcgacgctgctcagacgctcacctttgcgaccattggtccggaagtagagctcatgctgatacagacgctgaatgttggtgcctaaatccgcagcctgcaccatcgcttttgcagtgtcggcgttaaggcttagttgcgtatactgtggaacatacatgccaccagtaaccggaacccccgtgccaggacgatattccaggcagttgacctcatagtgatatgccggattagtacactctttcagccccgggaacgcggcgaaaattttctccttcgcagccttcagagaatcctctgttttatgatcggcctcatcaataaaggcataacgcgtttcctgtttgccatctacatcttccagccagctggcaacttccagcttcggtttgtcatcaggtttgttttctacctgatatttccacttaacttcccctgtcttactatcgatggtgtacggcagcgcaccatctacggcaggataacgttcatagacccaaatgcccgttgcgcgctgctgacgaacgcggttcggatacccttgcggatcgttatttactaccgacttgttcagtgccatcgacagacctgcggcatccaacagacgcacaaaaccagacgcgctctcttccttaagattgctcatcacgttttccatgatcagcaccgatccacctttgttcagataggcgatcagatcggtcacatcctgctgagtcagcttcggtttgctggtatctgcacgcagcgggattgcataaggatcgttacccacctgagtcacatattcaaagccgttaaggatcagcagcggcatttcctgcggatcgagatcgccatagctacttaaatgctcaacagagatgcccgcaaaatccggatggaagtcgaacgcagcgctgtttcctgtaacctgaccatgacgtttaaaatagacagtatccaggttggtgcctacggtcatgctggctttcgcgtccggcttccatttatcgtcggacagatagcgcagcacgttctccatgaagttcttcatgtcatccgggtcgctgttgagcgtacactgcccatctttattaacgcccccgttccagctgtaaccgttcgggcaacgcaaaatgctgttgtagtgtgggttaccgataaccatcagtttgccctcaccgacttgccccagcgaaataaacggcaggttaaaggtggcggtatcgcgcgtaacgttttccggctcaacaagagaaggcgcttccgtaatgtacgccagctcgtttttatcccaggcgcgtttttcgccgaaggccagccagtagtttttatcattacgcgccatcagaatcgggaaggccgcgttggagatattcaccaccgcctgaccgcgcgcattacccgtgctgccatagaagttggtggagtcatggaatacatggaacttgctgacagatttgtagttcgtatccacgccccacagcttgttgataacgccctgaatctggccgtcattaacattgcgcgtcgtcagcgagaaccagcgagcctcgttacaaccatcggttttcgcacaaatcgcggtatcgatctctttggcctgacccgtattaaactgctcaataaattcgttaggcagattaacgacttgctcaccttcccccagcgtcgcaccgttggataacgagagattgataatctcgttgatcacgttgggatattcggcaaagaccttgcgtacatcgtccggaacaacacgggtattattttgcccggtcgtcgaatagcgatgaataagctgatcaatattcgccccgcgaacttcatcacccagttcagtcagcgcaatggtcgacttattgccgcgcactgaacccagttcaaaggtatcgataccaaaggagatggtttcgccccagctaaaggaaaattcaccattttcccctgtcacgccacggcctgaattggtgtagtagttgacgccagcaacaccatatccctggctatcgaccagtcgaccttcagagagaatgatttcagtgggttgatactgataaaactgttccgcgttagccgacacgaaggaagcgttcagatccggttttgttcccggcgtggtgacgggcacgaccggtgaagtatgagtggatggcgctttatcggtcgcagcattgttttccacctcttcattgaccagctttttgaactcttccggtgccagatcgatttgcttatacagcgagtcgaagcgtttactctcgatcaccgaggagaacgtcagacaaacctgttctgtattcgccggacagctgttactggacgttaccagcgaaaccgcattgcttttcttgtcatcggagcccgccagttcttgcgcgtcctcaaggctaaacgacactttttcaaccgcacgcaagctacgcgcagcttctgactgagtgttgaaggtggcaattgtcgtgttacccgccacgcaagtaacgtcctcgccaggtttaaatgtaaagccatcgctggattcaccattacaggtagcaccagttacccgctggcttccgcccagggtcagataacccgttttcgtaggaacaggttctggctccggttctggtgttggttcaggatcaggtatcggttctggcgtaggctctgggtccggcgttggctcaggcgtcggctccgggtttggtgttggatcaggtttcacttccggcaaagaccctgttccagaatctacaggcggcgtatcggaggaagatccggaaccaccgccatcacaaccggctaacagggttgcgctcaaaatagccgctaaaagcgatttcttatatttaaatttcttattcattaataacgcaagtgacaaaacaatgttaaaaaattcgtaactgggagaaatagttttatgctttatcttctctaataacttcctccattcttaagaaaacgacatcattgatagaaaacaggtgaaatttataagaataacccctatacgatgtctatctggctatttttacgaaatttcaacaaacaaaaaattaacaacatttcacaacgtaactatataaatttgttggtagttttaacgattaagattgcaaaagcaacagatagaacggtgtttgctcatcaagcgaacataattaatacagacttgttttgcgtgataaaaaaatagatgttctcacgctcttaattatttagcaggttatctgaacgcaaaacattattgctgcatggataataaagcgagaaatgattttcaattaataagacagaataatgtaaatgaagccggatgatattaacgatcatccggctttattgatttacgagactaacatcccggtaaacacatacgcctgcagcagggtgataatgccgataacgctggcaaaaatcagactgtgcttcacggtgtagcggaacagttcagattctcggcccaccatgcccgtcgcggcgcaggccacggcgatagattgcggggagatcatcttgccagttacgccgccgctggtgtttgctgccaccagcagggtgtcagagacgttgatttgctgcgccgtggtcgattgcagtgaaccaaacagggcgttagaggaggtgtccgagccggtaaggaatacgcccagccagccgagaaacggtgagaagaacgggaacatcacgcctgtacctgccagtaccagcgccagcgtggtggacatgccagaatagttggtgacgaaggcgaacgccagcaccatgccaatcgacagtatcggccacttcaagctaattagcgtttcggcaaagacgccaatacctttcttgatccccacaccgaggatgaagatagagataatcgccgcaataaaaatagcggtgccgccagccgagagggggtcgaatttaaacaccgcatccattggcgttggttgggcgacaatgggtgccgctttcaacacttgttgatgcaaatgagggatctggaaattaatcaccagtgaataaaacgcgccgcccggagcaaataacgctttaaacggcttcatggtccagatggtgaccagcaccgttaagattaaaaacggtgaccacgctcgaatgatttgccccagactatattctgaaggcacgggaccgccagaagatggcttatttaccaccatcgcacctgcggattgtcccatgctgattgccgtttcggtatttttcggccgccagactttaaggaataaagcgagtgagacgatactcaccagcgccgaagtaatatccggcagttccggaccaatatagttagaggtaaagaactgagtgacagcgaagcttcccccagcaaccagcgccgctggccacgtctctttcacccctttccagccgtccatcattgctaccagccagaacggcacaagaaccgacaggaacggtaactgacgtcccgccattgcgccaatgtggaacggatcgattcccgttacctgaccggcgaccagaatcggcacgcccaacgcaccaaacgccaccggcgcagtattggcaatcagacacagccccgccgcgtataacggtttgaagcccaggcccaccagcagcgcaccggtaatcgccaccggcgcaccaaagccagccgctccttccagcaacgcaccaaaggagaaaccaatcagtaacacctgcaaacgctgatcgtcggtgatggagataaccgagctgcggataatatcgaactgcccgctggcaacggttaatttatacaggaacaccgccgcgacaataatccacgctattggccataatccataaataaagccatagcccgcagcagcaaatgccatatcaatcggcattttaaaggcgaatattgcaatcaggatagataatataagggttattgctccagcgacatgtcctttcagacgtaataccgcgagtgcaacgaagaagaatattatcgggatcagggcgaccagagcggatagccccagtcctcccatcggcatatacatttgggtccaggtaaccatattgttcagtctcttattatctttatatgcttgatatacttaaggttgtaataagcaaaagaggactgaactgtaaaatataggcgttatactttacagcaacagtacgccgctaacgcaattgctacctctggcataacaagtatatcgggtaagggtttctgttccgcacacgcagacgcagagtatcgttaagatgtccatattgttgttttaggcccgctagtaatgcgctacgggtatttaatattgttaaaccctgataatcgctccggttatttccgggataaatgtactaccgcagttactatcatagccccgacaataaaacttgccggggcttttttgacgctattaatgactttctttttcgcgtaaacgccaggcgtgtaataacggttcggtatagccgtttggctgtttcacgccgaggaagattaaatcgctggcagctttaaaagcacacgagttagcgaaattccccgccatcggacgataagccggatcgccagcgttttgctgatcaaccactttcgccatattctccagcgacgcctgcacctgttctttggtcagaataccgtgacgtaaccagttggcgatatgctggctggagatacgcagcgttgcgcggtcttccatcaacgccacattgtgaatatccggcacttttgaacaaccaatcccctgctccacccagcgcaccacgtaccccagaatcccctgcacgttgttatccagctcttgttggatctcttgcgccgaccagttagcgttttcagcaaccggaatagtcagcagatcgtccagcagcggttcaaattcagcattgaactcggtctgggcaatgttggcttgtacgctctgtacgttggtttggtggtagtgcagcgcatggagcgtagcagcggttggtgacggaacccaggctgtgtttgccccggcacgcagttggtcgcccttctggctgtacatgtctgccatcaggtccggcattgcccacatgcctttaccaatttgcgctttaccgcgcagcccacagaacagaccggaaagcacgttattacgctcgtaggctttgatccaaggcgtcgatttcatctgatttttacgcagcatcgggccagcttccatcaccgaatgcatttcatcgccggtacggtcgaggaaaccggtattgatgaacgccacgcggttgcgcgcctgagcgatacagctacgcaagttcagcgaggtccgacgttcttcatccataatgcccattttcagggtattcggtgccataccgagcattgtctcaatgcgggtaaacagtttgttggcgaacgccacttcctgcggaccgtgcattttcggtttcacaatatagacgctgccagtgcgcgagtttttctgcacttttaaatcatagagggcaatcgcgccagtcatgacgccatcaagaatgccttccgggatttcattgccttcgctgtcccaaatcacaggaatggtcatcaaatgacccacgttgcggataaacagcagcgagcgtccgtgcagagaaatttcagagccatcggcggcggtgtaatgacgatcgtcattcagtttacgcacgatttgccgaccgtttttctccattttctcttgcagagtcccctgcatcaggcccagcaggttgcggtacagcaggattttatcttccgcatcaaccgccgcgaccgaatcttcgcagtcgagaatggtactgatagcagcttcgacgataacatcgttgatgtgcgccggatcgtctttgccaatccgcccattggcatcgatttgcagctcaatatgcaggccgttatttttcagcaaaatgcaggtcggcgcagcggcatcgccacggtaaccgacaaactgtgctggagtacgtaacgtggtttctttaccatttttcaactggatgcgtaattgtttatcaaccaccttaaacgccaccacatcctgatagctgccgttttccagcggtagagattcatcgaggaaacgccgaacccaggcgataacctgctcaccgcgttgcggatcgtagccgctgaccatcgccccttcctgcgggatgatgtcgctgccgtataacgcatcgtacagtgagccccagcgagcgttcgccgcgttcagcgcgtagcgggcgttcattgccggaaccaccagctgcggccccgcctggctggtgatttcgctgtcaatgcccgtggtttccaccgtcacgcgctccggttgcggcaccaggtagcccagttcacgcaggaaagatttataggccgctttatcttttaccggccccggattgctgcgatgccactcatcaagcgctgcctgaatgcgatcgcgttctgccagcaactgacgattttctggtgccagatcatgaacgatctcatcaaaattgcgccagaacgccgcagcgtccagccctgttcccggtaaaacttcttcatccacaaaacgtttaaaattggcgtcaatgcgtaaacggctctgggttatggtttgactcattgtttatctcctcgttttcgcttatttcgccaacaccgctgctgccgctttcgcgacctgcgcatcctgtgctccggttaaaccagaaacgcccacggcaccaataatttgcccatccacaacaaccggtacgccgccttccagcgacgttaataacggcgcagtcacgaacgcggtacgtccgttgttcaccatctcttcatagcccttagtttcacgacgccccagcgcggcggtacgcgctttctcctgggagatataagccgcaatcggcgcgcaatcgtccatgcgacttaacgccagcagatgaccgccgtcatcggcaacagcaatggaaacagaccagttatttttctgcgcctcttcctgacctgcggcaataattgcactcgccatttgctggctaagaatgactttagttttcattttgttattccttttcaagggcttgttctacaatttcaatccagtgacgcacagaggtacgaccggcgctcgccagatgcgtctggcaaccaatgttggcggtgacgatcatttccggtttgccgctttccagcgcattcattttgttatcccgcagctggcgtgccagatcgggatgcgttaacgcatatgttcccgctgaaccgcagcacagatggctgtcgggaacgtccgttaaggtaaatccaagacgaagcaacactttttccacttcgccgttcagcttttgcgcatgttgtagggtacacggacagtggaaggccagctttttatcgccgcgaattgccagtttttccagcggttcctcgcgcagaagttcgactaaatcgaccgccagttcactgacctgacgtgctttatcggcatataacgcatcgtttttcagcatctgcccatactctttgacaaacgcgccgcagccgctggcggtttgcaaaattgcctcggcacctgcttcaatcgcgggccaccaggcatcaatattattgcgcgcccgtgccagccctttctcctgcgcattaagatgatagtccaccgcgccacaacagcctgcttcgttagctggcatgacgctgatccccagacgatccagcactcgcgcagttgccgcgttggtgttgggcgaaagcgtaggctgggcgcagccttccaacattaaaacccgacgcttatggcgcagcggcggacgcggtttagctttcaccgtttcagcaggcagttttgctctgacctgttccggtaaaaacggtcgcagcaccagccctacctgcgtcagcgcacggaagaccgccggacgcggcactacctggcgcaatccttcgcgcagtattcgctccggcagtgggcgtttcactttctgctcgacaatatcacgcccgatatccagcaaattgtgatagcgcacaccagaaggacaggtggtttcacaattacggcaagtgaggcagcgatcgagatgctcctgtgttttaagcgtgacttcgttgccttccagcacctgtttaatcagatagatgcgcccgcgcggcccgtccagttcatcgcccagaagctgataggttgggcaggttgcggtacaaaatccgcagtgaacacaggcgcgcaggatgctgtcggcttccagcgcgcgcgcgttctgccgcatctcttcagttaattgggtttgcatagcctgctcctcaaagttccgcgtacatgcgaccggggttaaacacgccgcaagggtcgagctgctgtttaagctgctggtgatagcggaataaaggagccgatagcggggcaaagccaccatctccggcactaaagcgggtcgcatgaccgccagcgttgcgggcgatgcgatggatttgattgtcctcggctgtcgatttcagccagcgtaacgccccgccccagtcgatcagttgctcgccgggtaaatccatcatcggcgcatcactgggtaatgaaatgcgccataaggtacctggtaacgagaagaacggcagttgttgttcacgcaattgctgccagaactgaccggcaacctcttcgccacccagcagttcacgcgctgcttttaccgatccttcgccgccctcaaggcggatccacaacgcattgtcgaagtaacataagccactaatgggtaatggctggagttgccactcggcgatttcactcatggcttcttgcaggctgatttcccgacgcaggctcagggaggcgcgcggtcgcggtaacactttcattgagatttcagtgagcacgccaagacaaccgtagcttccgaccattaaccgtgagagatcgtatccggcaacgtttttcatcacttcgccaccaaaacgcagatgttttccagcgccggtaatgatgcgcgtgccgaggacaaaatcgcggaccgaaccgctccacgggcgacgcggccccgccagcccgcaggcgaccatcccgccccaggtggcttcttcaccataatgcggcggctcacaggggagcatttgccccgcgctttccagcgccgcttcaattgtcaccagcggcgttccgacacgcgcggttatcaccagctcggtcgggtcgtaattaacaatgccgcgatgacaacgaacatccagcgtttgcccggtgacagggcgacctaaaaaggctttgctattgctgccctgaatcaccagcggcgttttatcgctaatcgcctgattcacctgctccagcagcgcctggctgtaatcacactcgcgtagcatcagaaacgctccagttcagggaaaggtaaatgaccgtgatgcacatgcatggcaccaaattcagcacagcggtgtagcgtgggaatgtttttcccagggttcagcaaaccatcggggtcaaacgccgccttgaccgcatggaaggtcgtgatttcatcgctgttgaactgggcgcacatttgattgattttttctcgcccgatgccatgttcgccactgatgctgccgccaacttcaacgcagagttcgaggatcttcccgcccagctcttccgcgcgggcaaattcaccgggttcgttggcatcgaaaaggattaacgggtgcatgttgccatctccggcatgaaagacgttggcaacacgtaaatcatattgctgcgataaacgggcaatgccttccagtacgccaggcagggcgcgacgcgggatggtgccatccatgcagtagtaatccggggagatacgtcctaccgccgggaacgcatttttgcgaccggcccagaaacgtacgcgctctgcttcgtcctgtgccagacggacgtcagtcgcgcccgctttcaacaagatgtcgttaacccgctcgcagtcttcctgtacgtcagactccacgccgtccagctcgcataacaaaatcgcttcggcgtcgacgggataaccggcatgaataaaatcttccgccgcgcggatcgacaggttatccatcatctccagcccgccggggataatgccattggcgatgatgtcaccaaccgcaagtccggctttttctaccgagtcaaagctggctaacagaacccgcgccacgggcggcttcggcagcagttttaccgtcacttcggtggtcacgccgagcataccttccgatccggtgaacagcgccagcaggtcaaaaccaggtgaatccagcgcgtccgatccaagcgtcagtgcctcgccgtccagcgtttgcacttcaattttcagcaggttatgtacggtcagaccatatttcaggcagtggacgccgccggcattttcagccacattgccgccaatggaacaggcgatttgtgaggaagggtccggtgcgtagtagagattatgcggtgcaacggcctgggagatcgccaggttacgcacgcctggctgcacgcgcgcgcggcgaccaacggggttaatgtcgaggatctctttaaagcgcgccatcaccaacaacacacctttttccagcggcagcgcgccaccagaaagcccggtgcctgcaccacgggtcaccaccggtacacgcaggcgatggcagacagccagaatcgctgtcacctgttccatttgcttaggcagaacaaccagtaatggacgcgtgcgatacgcgctcaacccgtcacactcgtaaggaatgatctcctcatcggtatgcaggatctcaagtccagggacatgctcacgcagtgccatcagtaccgatgtgcggtcgacatcgggtaaagcgccatcaagacgctcttcgtacaagatgctcatgagtaggcttcgctttgttgtgttgtgtggcagctgatttttgcgcgctgcttctgtgaacagttattaagcgggcttttcgttttcgtctatctctttagctaccggtcagaccattttttttccagctctgtgaccttgtcttggttaactcaatgttaaattgatgtaacataatcacttacgtgatgtgcgtgttttgcgagttaagaacagaaaaattggtcctacctgtgcacgaggtccgggaatgaaagatgaacgtcgccctatttgcgaagtggttgcagagagtatcgaacggttaattatcgacggcgtactgaaggtcggtcagccgcttccctcggaacgtcgactgtgtgaaaagctcggcttctcacgctccgcactgcgtgaagggctgaccgtgctgcgcgggcgcgggattattgaaacggcgcagggtcgcgattctcgtgtcgcacggcttaatcgggtgcaggacaccagcccgctgatccatctgttcagtacgcagccgcgaacgctgtacgatctgctcgacgttcgcgcattactggagggcgaatcggcaaggctggcggcaacgctgggaacgcaggctgattttgttgtgataacccgctgttatgaaaaaatgctcgccgccagtgagaacaacaaagagatttcgctgatcgaacatgcgcagttggatcacgctttccatctcgccatttgtcaggcttctcacaatcaggtgctggtgtttacgctgcaatcattgaccgatctgatgtttaattcagtgtttgccagcgtaaataatctctaccatcgaccacagcaaaaaaagcagatcgatcgccagcatgcgcggatctacaacgcggtgttgcagcggctgccgcacgtcgcccagcgcgcagcacgcgatcatgtgcggaccgtgaaaaagaatctccacgatatcgagctggaaggccaccatttgattcgctcggcggtgccgctggagatgaacctgagttagctggtattaaatctgcttttcatacaatcggtaacgcttgtacggctccgccccaatgcgttccagcatgttattcatgcctgtattggtttcgaggatccatgacatctccagcgcatcgatcttccggcgggcaaacggatcgcgtaaggcttcaatcaataacagcgcaatcaccgggccgatgcggctgaactgatactcgtcgcgcacgcccatcagcggtactcgcgcagttcgcacaccgctgactttcaaacgccacagcaattttgcccagccgaagggaaagagcgatccgttcagatcggcaatcgcctcgttgatgttcggcaagccgacaataaacgcgcagggtgcagaatcaatctcagcgatatagatcatatcgtccggcaccagatatttaagttgatcgcccatggtcgcgaattcatgttcggtaaacggcacaaatccccagttgtgctgccagccagagttgaaaatctcacgcaggatctgcatctcttcggcaaaccgctgacgattgatgcagcgaatggtcacctttttgcgcacctgatccatcagtttttttagcgccggagagaaagtgagatcggttcgctgcatccaccacgccagtaaatcaatgcctttgtgataacccagttgttcaatatgcgcggcataccacggtttgccgtgtggcatcatcgcacagggtggtgtgtcaaaaccttcaatcagtaatccgctttcctgattgatattcaggctgaaaggaccgctgatcttacttgcaccttgtgacttcaaccacgcttccgctgcgccaaacaacgcggcaaaaacctgcggatcatcaatggcgtcaatcatgccgaaatgaccggtatctttgccgtaacgctcgcggtgcaaggtatctatttgcgcggtaatacgcccaactatctgccccgctttttttgccacccacgcctgccagatgatatggtccgtccccggatttttcgcagacaaatgctcgttgcgttcaatgaataaagggggtatccagtttggatcgtcgggataaagtgatgacggaaaagcgataaatgccttaaggtcatttttattaaggaaggtgcgaacaagtccctgatatgagatcatgtttgtcatctggagccatagaacagggttcatcatgagtcatcaacttaccttcgccgacagtgaattcagcagtaagcgccgtcagaccagaaaagagattttcttgtcccgcatggagcagattctgccatggcaaaacatggtggaagtcatcgagccgttttaccccaaggctggtaatggccggcgaccttatccgctggaaaccatgctacgcattcactgcatgcagcattggtacaacctgagcgatggcgcgatggaagatgctctgtacgaaatcgcctccatgcgtctgtttgcccggttatccctggatagcgccttgccggaccgcaccaccatcatgaatttccgccacctgctggagcagcatcaactggcccgccaattgttcaagaccatcaatcgctggctggccgaagcaggcgtcatgatgactcaaggcaccttggtcgatgccaccatcattgaggcacccagctcgaccaagaacaaagagcagcaacgcgatccggagatgcatcagaccaagaaaggcaatcagtggcactttggcatgaaggcccacattggtgtcgatgccaagagtggcctgacccacagcctggtcaccaccgcggccaacgagcatgacctcaatcagctgggtaatctgctgcatggagaggagcaatttgtctcagccgatgccggctaccaaggggcgccacagcgcgaggagctggccgaggtggatgtggactggctgatcgccgagcgccccggcaaggtaagaaccttgaaacagcatccacgcaagaacaaaacggccatcaacatcgaatacatgaaagccagcatccgggccagggtggagcacccatttcgcatcatcaagcgacagttcggcttcgtgaaagccagatacaaggggttgctgaaaaacgataaccaactggcgatgttattcacgctggccaacctgtttcgggcggaccaaatgatacgtcagtgggagagatctcactaaaaactggggataacgccttaaatggcgaagaaacggtctaaataggctgattcaaggcatttacgggagaaaaaatcggctcaaacatgaagaaatgaaatgactgagtcagccgagaagaatttccccgcttattcgcaccttccctaaatcaggtcatacgcttcgagatacttaacgccaaacaccagcgaaatgagcggcttgccgacgatcaacaccgcgagcgccaccagaataccgattccgcccgccagtaaaccggacttcacacctaacaaccacggtctggtggtgcgcggatctaaacgcatcacctctgggtaaaaacttttacccagcaaacccgctggcgttccggcggcgtcgaagaatgtcatggcgattttaaataacccggcggcagcgggtcctaacacgatccccaccaacactgtgctgcacgagttacgcgccgaccagatggagtgggcaatgttggttgaccagacaaaactccacgcgcctttaatgtatcgggcagactcaaacagattcaatttgaaggcgttatggatatttcggcggcgtaattcgcgcgcggcaaaccaccagtacatggtgccgccaaccagattcgacacgtaccaggcaataacaaaacccgcaaaaccaaagtcaaaataccaggctacgacgctccccgctgcgcgcagaaaaggtttcgtcgcctgctgtacagcaattaaatcgaagcgatctaccgcacgcagaatgccggtcggcgtggaggaagccattgaaggaatgagcgtgcaatagagcgctgccagccaaaaactttggtcatccagacctaatgaatgggaaaggaatggcagtaaggcaatgccaccgacaatcgccaccgcgccgctgacgatatccagcgagaaggaaaatgagacgacattgcggaattgctgcggattattgttggttaatgctggtgttccgtactgaaccaccagttgccatgtctgaaacttaataaaatcgctgatcgacttggcgtacgattgcacaatcaccagtacgccaaacatggcgggcgtcatccctttaccggcacacgagagcgccaacagacccagcaaggcgctcacgacattactggagcctaaccaggcgctattgcgaataatggtgcgaaacgcgccatctgcaaaccaatgtttgatgttaaaacccgccaattcagcctgaccttatcgttgatagtaaaaagtatcccgccagccttaagttaaacttcggcggtcagaaacgatggcaaccagagaaaccgccttctgtgcctgttccagcacttcgctgtagggcgctctggaatcaatctcaagaatttttgtgccgttatagccaatcttcgacatgacaccgattttgtcctgcagctcggcatagtcatggtcaggcttgcgggagatggcagtctcaatatcaatgcccaggcgaataattaattccgggcgatattgcgccatttgttggtataaacgccgttcgcgctgcgccagaaacatgctgattttcccggtcgcacgttcgacgccaatccccggtccatcataataaaagcccgaaatttcagcctgcgggaagcgatcgctgaccaccagaacgccactttgcgccagtcgctgaaccttgcgtagattcgccattcttcgcagcgagaagcagtacataatcaccgccgcccatagcgccggagatttggttttcatgctttgggttttcgaggatttggccgccagtcgccgttccagccagacgccaaccaacggcaatcgtttgattttgtcgccgtcttcgccggagagcagccccagatagcgccgctcggtttgccagtgttgttgcagcgatttcaccaggtcggtggtcagtgtggatttaccggtgccatcacacccgaccaccgcaatcagccccggaatgtagttgggctgcggcgcggttgtactattaacagtttgagtttgtagtgcatccattcgttaaatcatcccctatccattttggtgatcaggaaagcgcggcgtgaattgcgcgtagtgacgcttgcagaatttcatcggcggggtgtcgcccatccagttcaaggatctttgcgccattgaatgtcagttgcggcgtaacggcgattttttcctgtaacgctgccagttggtggtcaggtttacgcgcaaacgcggtttgttcatcaatgccaagacgaatcaacaatacgggcaaataagatgccatccattggtacagcttcagctcgcgctgccttaacatttttatccaaccgttaccgcccgtggtttttgccaattgcgggccatcaaagcgaaaccccggcacttcaacctgcgggtagcggtcggtgatgagcagaaagccttgctggcttttacacaacattttgcgaaacttgtacgcccgccagcaggaaagcagatagataaccagtgcagtaatattgccaggcggtgttgagggcttttcgtgcacatgtgccgctttacttcgcagataacgcccaaaaggtgcgccaataacagggagctgtgaaatccattcgccaattcgcccggacgattgcccgagataaatgtgttctgttggcattcttgctgccagttcatttaccaggcttgccgtgagggtcgatttacctgaaccatcacatcctacaatggcaataacacgcactggcgtggaattaattattgacatattacgttgattcacgaaaaacccggcagtaaataatgtattgaatattacgtggtccgtgctcagaatatccgttcaaccttattgtgacaatggttaattgtgacattgacctgaattacgctttcataaaaacatattaaccaaataaatatttttaatggatatttaaattaaaggatatattcatgcagtcaataacacctccattaattgccgttattggtagcgatggttcaggcaagtcaacggtgtgtgaacatcttattaccgttgtcgaaaaatatggtgctgccgaaagagttcatttaggaaaacaggccggaaatgtcggtcgtgcagtgacaaaattaccgttgatgggaaaatccttacataaaacaattgaacgaaatcaggtgaaaacagcaaaaaaattgcctggaccagttccggcgctggtaattacagcgtttgtcgcccgtcgcttactgcgctttcgtcatatgcttgcctgtcgtcgtcgcgggttaattgttctaaccgaccgttatcctcaggaccaaattcctggcgcttacgatggtacggtgttcccacctaacgttgaaggtggtcgttttgtctcatggctggcaagccaggaacgtaaagcgtttcactggatggcgagccataagcctgatctggtcatcaaactcaatgttgaccttgaagttgcctgtgcacgtaaacccgaccataaacgggaatcgctggcgaggaagattgccataacgccacagttaacctttggtggtgcacaactggttgatatcgatgccaatcagccactggaacaggtgttggttgatgcagaaaaagcgattacggattttatgaccgcgcgtggttatcactagtcaaaaatggaaatgcccgatcgccaggaccgggcattttcaggaaggttaaatcaactgcaatgctatccagtacagcccaccagaaagaaaaattgccgccggtaaagtaaatacccacgccatcaggatgctggttaccgttttacgctgtaacccaccgccgtccaccaccatcgtccctgcaactgcagacgagaggacgtgtgttgtggagacgggcatcccaatataactggcaagaccgatagacactgccgccgtcatttgtgccgccatgccttgcgcatacgtcatgccgcgcttaccaatcttctcaccgatggtcatcgctacacgacgccagccaatcatggtgccaatgccgagcgccagtgctaccgccatgatgatccacaccggagcgtactcaatggtgcttaacatatcgctgcgaagttttttcagcaggttctggtcttctttactgacgcctggcagtttcgctagcttcgcggaggtatcagagatgcacagcataatgcggcgcagctggctgcgctgactcacgcttaacggctcgtaactttccatattgcctggcagcatcgttttaacgcgcgcaatagcatcaaaggtatttgccggatgacagtgaaactctgttacttgcgtgccatcagtcgatgctgcaggcaatggaggttccatcgcaatcaacttctgcggcagttcaggatgctgttgcaggtagtgttcgaagttggtaacggcatcgcgggtacgggtaatttcatagccggacgcattcatattgacgacgaagccagcaggggcaatccccaccagtaccagcattaccaggccgatccctttttgtccgtcgttcgcgccgtgcgaaaacgccacgcccgcagcggaaacaatcagcgcaatacgcgtccagaatggcggtttacgtttgccttttttctttttgcgatcttccggaatgcggtgaatacggtcacgctttttcgtcccgctccagtagcgtcgcagcaggaatatcaggcctcccgcaatgaccaggccgacgataggggaaacaatcagcgaggagaaaattttggtcacttcacgcaggtttaacgcatccatcaccgatgagccggttaacagcgcgttggttaaaccgatgccgataatcgcaccaatcaaggtgtgcgaactggaggccggtaaaccgaagaaccacgttcccaggttccagataatcgccgccagcagcatggaaaagaccatcgccaggccgtgggttgaccccatattcagcaacaaatcggttggcaacatatggacaatggcataggcaacgctaagtccgcccaataacacgccaaaaaagttaaaaaatgccgccatcaccacagcaagttgtggttgcatggcacgagtataaataacggctgccaccgcattcgccgtgtcatgaaaaccattgattgcttcgtagaacaacacaaatgccagagcaagcaataacaaaagccctgtgtatatatcaaggccaacaaataaatttagcatatattagattacgccattttgaatttacgaacggacgcattatcagtgactttaacggcatgggcaaagtgaaatatcattttttaacgataaaaagagtgttatttcttgtgtatcagacaataagcattcattcaaaacctttagaaataatcaaaacacaggtattccactggttaatatattcacatatgaaatgaataaatattggaatatataaatattgaatattttgattaatccccgtactgattattcttcataatcagtacggggttgctacaacatgtattactttttcaccacaattaacggttcaatatcactctcttttttgatgaccagtgattcatcaccgcgcaaacacgtcccaccgtagttgccgccaacggtgaaggtacatacctgaatgtatttaccgtccactttcggcaaacaccacagttgctgatagatgtttttctgctcggcaaatttaccgctggttttgtccagcacctcttcatgatggctgacgaggtcgatattgctgccacagcgaccggcgatcggtttcactgcgtaacctgttttcaccagttcatcattaacagtgaaatcggtatccagcaggtaacgatggtgcgggaacagcgaccagaggatcggcagaatcgctttgttgccggggatcaccgtccacagcggctcaaagaccagcacttccgggcgcagcaatacgtcgataagacgcacttcgttttgcggatgaccggtacggattggcaccgcagcaaactcacggtcgctaacttcacgaatctgatcaaacgcggtttcccacgcccaggttttccacacgcagttaaccagtcgcccttccccatcaatcagttgcccggcagcatcccagcccagttcatccaatccacgcaagatacgcgtttcaaagcccgcctggtgcagcgcctgctccataaactgcgcgtgatagttttcctcgatatctttgtcctgcatgatatggacaaacggacgtgcacgactgtgtttccaggcaccagccaattcgttaatcagcccttccgccggattgaagccgttgcctttatagccctgctccgcccaacgttcgaggatcaagcccgcttcggtatgacaggaggcggagtcggcgttgtactcgtaaaccttcaggccacgctcatccatgcagaaatccatacgaccagtgatcatatggtgacggcgacgctgccaggagagacgcaaacgtggccagaggattttcgggatgtcgaacagcgccagcaggttgtcatctttcagcaccttgtcggttgcgtgaagatacatcaggtgcagctcgttggtggctttaattagctcctgctcggcactctcggtaatggtgtagtaatgataaggatcctgattgatcacctgaccgttggcctgcacataggcgttttgcagcggatctttttcatccagccatttaccgtcaaactggcctttgttttccaggcgcgctccgctgattttcagcagctcgcctgcaatttccggctgcggtaagctgtattcagtatcttccgtctggatcatccagcccagaatggtggtgtcatcaaaagtgtctttcagggtatagcagccgttttcgaccaccatctccagctcgcgcgtccactgttgcccttgcggcaacggggaatgaatcacgttctgttccgcaatacggactttgttgccatgcaattgggtaatgatggcgacatggccagtgtctttaaattcaccgcctttatcccagataagaagcgcacccgcgaccggcgcacgcggcgagccgttaggaaatgcctgcaatggcaggatgttgtcattaaccacttctcgcaggaagcgcagcgagaaaatctcccacgccatacccacgtcagtaaagaccacaccgtaattcagaaagagaaaacggcgagcaaattcaacgcattgccacttgtggcccatatattcgtcgtcgatatagctacggaatacggcgtcatcttcgtattcctgcggatcgagagaactgtaatctgaagagtagattgctaccccacctggggcgtagcccaataatgtcccgaacggggcatcctggctggtcgttcctttgctcatcactttacctttaacaatacaacctaagcagttggcgtaattgttgtgctctgattacctgctcagcgacattaaccggacagaggtcagactaatcatacacctcatcgcagcggctggcgcaaagggttaaaaaattcacattctgtacagcaagtgacctgctacactgcttcaacactaccactcagaaggcaactcactatgacagacaatacttatcagcccgcgaaagtctggacgtgggataaatccgctggcggcgcgttcgccaatatcaatcgcccggtttctggtccgacgcatgaaaaaacgctgcccgttggcaaacacccattgcaactttattcgctgggaacgccgaacggtcagaaagtaacgattatgcttgaggagctgctggcgctgggcgttactggtgcagagtacgacgcctggctgattcgtattggcgatggcgatcaattctccagcggctttgtcgaagtgaacccaaactcgaagatcccggcgctgcgcgatcatacgcataatccgccgatccgcgtgtttgaatctggttcgatcctgctttatctggcggagaaatttggctacttcctgccgcaggatttggcaaagcgtactgaaacgatgaactggctgttctggttacagggcgcggcaccgttcctcggcggtggttttggtcacttttaccattacgcaccggtaaagattgagtacgccatcaaccgctttaccatggaagccaaacgtctgctcgacgtgctggataagcaactggcgcagcataagtttgttgcgggcgatgagtacaccattgcggatatggcgatttggccgtggtttggcaacgtggtgttaggtggtgtgtatgatgccgctgagtttcttgatgcgggcagttataagcatgtacaacgctgggcgaaagaagtaggcgaacgtccggcggtgaaacgtgggcgtattgttaaccgcaccaacggaccgctgaatgagcagttgcatgagcgccatgacgccagtgatttcgagacgaatacggaagataagcgtcaggggtaagggttggtgttcgtcgcagcaagccatccaggccggataaggcgttcacgccgcatccggcaatcgtgcacaatgcctgatgcgacgctgccgcgtcttatcaggcctacgaaagctaatcatcacgcgctggtaatgtcgtaatccatttggcgcagtgcgtctaatgtggctttggcttcatcttcgtcgatgatgctcatggcaaatccgacgtgtaccagcacccactggcccagtagatcggcagggttaccttcacaaatcagggcgatattcacatcgcgcttgataccacatacttcaacctgcgcaagctggtgaatatcttcaccgacagccagcacctggcctggaacgccaatacacattattaactccggttattcaacttcaatacttttgacgatcagcgaatcgccggtatcgacacgcaaccgctcgccgtgacagagcggacactgcgcatcgtgctgatgaatctccaccacctggctgcaatcccagcaccaagcctgggcgggtttatagacgatatgtaaatcgcacccttgcgccaccgttccgtggcagacaatttcaaaactaaaacggacggcgctctcctcaacgcaggagagcgcgccaatttccagccacacggcggtgacgcgcttaacatcgtgctgctccgcctgccgttggataatttcaacggcgctctggcaaagagacaactcatgcattttcgccactcctgcgaccaaacagcagggcgcgacgccctgcgtgtggtacatccggattcgtgactggcagcgaaaggatcattcgtgcgcagtcatccgtcaggcgttggccctcttcaatcgacatgctgtgcgaaagcggcgacatcagcgaacaggagagatattgcgaaacaccgtccagttcgccaacggtaaaggtcatagtgccatacggcagttgcagaccaattttttcactcactttgcgcagcggccagagttgatccgggccggggaagataactgcactcagcatccacggggtgatcacacaccccgtccactgaccttcgaacagcgtaaaatcagaaacatacaccggcattgaaggatgcagaaaagagagatcgtgcatcgaacgccgggcaatttcttcaaacgctgcctgtacttgcgccttcggggaggtctggaaacctgctatctcttcagtcatgaatcgcctcccgtgggatggcttccacgccagattcacgcagcgcagccagaacctgctcaagcgcaggttcaatcattgcttcaaccgtcggcgttaagccgatgtgtggctccagcgattccgggatcacgccgaccagggtcagctttttcggaaactcgccggtgaagcgcagggccgacaagacgtcggccaggccaagctgatgcggagagattttgttggtaaacaacgccggaacttcttcatcccgcaggatcatcatcgttcccggcgcgttctttttcgagacaatggcatccgcaataatcaaatgatcgcgatttgccatgtcgccaagcagctccattcccgccgtgccgccatcgaggatctcaacataatccggcagaatgtatcgttgctctaacgcttcgacaatccgcacaccgatggcttcatcggtcagcaaaatattgccgacccctaagactaaaatacgcattacagaaccttcactgaaaccacttcgttgccgtcagcatccactacgtgtaccgcacaggccatgcacgggtcaaaggagtgaatggtacgcaccacttccagcggtttattcggatcggcaaccggtgtacccaccagcgactgctcgtaaggaccgacgtcatcattgaagttacgcggaccagagttccaggttgatggaacaaccgcctggtagttgctgatgataccgtctttaataaccatccagtgagagagcataccgcgcggcgcttcgaggaagccaacacctttgaattcacccgttgccggaatgttcggcttcacaaaggtggtgtgatcgcctttgccgatattggtgatcagtgcactgtattggttttgcaggatatcctgcaattcacagcagtgaacggtacgaccaataatacggcccagcgtggagtgcagctgtgccacttccagcgtgttgccagtcagtttctgataaatcgcaacgatttcattcagtttgttctgggtagattcgcgacctgccgccagtttcaccagcatattagccagtggccccacttctaccgttttgccgtagaaagtcggtgatttcacccaggaatatttcccgtcgtcagaccaaccatcataagccggaatggtggtgccttcccacggtgcctgcggcgcttcgtctttataccaggagtgcttcgcgctttcctgaatgcctttgatcaggtattcatcggaatgagaagtgatcggacgatacgaggacagatccgcattctcaatgtagccgcccgggaacaggaagctgccgtttttactgtcggtcgggaattccggcacgctcaggtagttcaccgcacctttaccgcgtgtcagccattccgggtagaacgcggcaataactgcggtatcaaccttataaacctgctcaacaaagtcgctcagtttgtcgatgaaagacttgatgtacatcaggcgctcaaggttcagcacgcccaaaccgtcgaggttgatcgggttcgcgacaccacctaccgccaggttctgaatgtgcggcgttttaccgcccagcagcgccacgacgcggttagcgtcacgctggcactccaacgcttgcaggtagtgcgctaccgcaatcaggttcacttccggcggcagtttcatcgccggatgaccccagtagccattagcgaaaatacccaactgaccgctggcaaccagatctttgatcttgttctgaactttggtgaactcttccggactgttcaggtgccaggtcgaaacgcctttcagcatttcggaggctttggttgggtcagcttgcagtgcagaagtgatgtccacccagtccagcgccgaaagctgatagaaatgaacaatatggtcatgcgtggtgtgcgcagccagaatgatgttacggatgtattgcgcgttaaccggaacgtcgatattcagcgcactttctgccgcacgaacggaagacagcgcgtgagtggtagtacatacgccacagatacgttgcacaatcatccatgcatcgcgcggatcgcggtttttcacgatctcttccatgccgcgccacatggtaccggaagcccatgctttcgaaacgacgccattttcgatttcgcaatcgatgcgtaaatgcccctcaatacgggttaccggatcaatagtaattctctggctcatgctttgctcgcctcatgacgattatgatcgttttgttttaaaggaggaagtatcggcagtagacgaatgagtacgatgtaagcgcaaatctcaatagccacaaaaccaatagaaatcaacagttcttcccaggtcgggaagtaggcgtaaccgccgcccgggttgaatgccaccagcgaataggtcagacgccaggttgcacaacctaacagtgcgctcagtgctgacaggaacagcatgcgggaatcattacgcagcttcgccacacgcagaacgaccagcgggaagagcatcagcaggacttcaatccagaacatcacggagtagaagtcaccggcaaacgctaacgacagcttgtcgcgatagataagctcgccaaagcgcagcacgatgaaaatcgccagcaacacactgatggtgttggtcagcttaacaaacagactcttttcatccggaccgttgccacgcagacccgcctgcaccagcgaaccttcaaagatgacaatcgagaagcccatgatgaacgccgtcagcagcgagaacagcggcaacatttcatagctctgccacaacggatgcaccttgtagcccgccgagatcatcagcgaccccattgaagactggtgcatggtcggcagcagcgcaccgagcgcgatgatgaagaacatcaccttgtttagtcgctgtagcgacaccttccaccccagacgttcaaacagtgccggagcaaactccagtgccatcacgccgatatagatggtcatacagaccgccgtctcgaacagtaccgagttcacgttgaagtgacccggaatgtagaagtacggcaggttccagtagcgacccacgtcgatagtgatcgacaagccacccagtgagtaaccaaacagactcgccaacagcgccggacgcaccagcggatggtattgcccacggttaaagacgtataccgcccacgccagcgcccagccgccacaggcaaagccggtgccaatcagcaggtcaaacgcgatccacacgccccacgggaagccgccgttcaggtcagagacagagcccagaccgaacaccagacgcttcacaatcaggagcatacagatgacgattaacggtccaaaaatcatgaccggtttactgatgattttgccgcccagcggttgtggatcatgactcatgatcgtctcctccgtcgtgatggtcgtttttggtgttgcgacgaaccagcacggttaagcccgccagcacagccagtggtagcatcatgcctttatacagggtgtgttgaatattttcggaacgcgcaccggtagaaagatcgtccagtttcggcaggtcgagattttcataaggcacacccgtcagtaccagaacctgagtaccgccgccctctttctcgccgtacagatgcggataatatttcggcaccgtatgcaggtaagtgtcgccagatttcagcgtctgacgcggatagtggtattcgctgccaggcttcagcgccagacgttttttcgcctccgccatcagctcttcacgcgtaccgaaaatcaccgcgcccgccgggcacacttctacgcagccaggtagaccgcctttatcgagacgttccacacctttctggttgcacagctcgcacttatgcagcgcaccaaacgggttgttgtagtcgtacttcggcacgttgtacggacaggcgaccatgcagtaacggcagccggtgcacacatctttgtcgtaatggacaatgccggttttcggatcttttttcagtgcagagaccgggcacacagagacacagttcggatcgacgcagtgcatacactgtttcttaatgtacgcgtagccgttctcctcctggtctttgttgacccctgtgccgctggtccacacctgaatgatgttattggtatacggcgacagtttgtcgttgttcgaccaggtctgttccccttgcgggttacgttcagggaaattgatatcctgacacttggtgacgcaagcctggcagcctacgcacaaggtcgagtcgtacaacatccccagcgatcccggaattggcgggcggttttcagcagccgcatgactgacagacggcagcgcgcccgtcagcaatgccccgcaggaggctgctttaataaaattacgtctgttcacggttattctccccgtgagtcagcgttatctttcttttgctgacgacccagttcacgcaccgccatcacgctgacaccggcaaccaacccaaccacaccgccgagcaaaccaatagcgcctgcagagacgttgccgccctctttagcgttaacatccggtttctgtgaacgcggagtttgattttcgacgttggcaagctgatggatgcctttatggaagccgataccttcttcgttacagccatagcaagggtgaccaatcgccaccggccacacaccgccaacatcgcagaattgcagcgttgagcagttgccgtaagtttctggccctttacagccgaggtggtacaggcaccagccttcgcggtggccttcatcaccgaactctttggcaaaacgaccagcatcgaagtgcgggcgacgttcgcagtgttcgtgaatcagacggccataggcgaaggtcggacggtttttgtcatccagtttcggcggtttgccgtaagtgatgatgtgcgcaacggtcgcgaggaagttgtgcgggttcggcgggcagcccggaatattgataacggttttgcctggcagaacttcttgcaggctgactgcgccagttgggttaactccagctgcggcaacaccgccccacgcagagcaggaaccgatagcgataatggctgctgcgccttccgccgctttgcggatgtgatccacaatcggctcaccggcaaccatgcaataaataccgttatcttttaatgggatggaaccatccaccactaacacatactgccctttgtacttctcgagagcgttatgtttgttctcttcgacctgatgaccgaaggcggcggaaagcacttcgtgatactccagagagatagtctccagtacgaggttttctaccgttggatgcgttgcacgaagcagagattccgtacaaccggtgcactcctgcgcgccaatccagataactggcggacgctgcgggttagtaaccgattcggccatctctgcagcggctttgctacttaaccccatggtggcggctaatgctgcacaaagcttcatgaaatcacgacggttaatgccgtgagaatggatgagggtgttatctccagtcatttatagttattccgttgcgaagacctggcatatattttgcctcaatcgcaaaatcaataatgcgatcgatgcgccatttaccacacatttattatggttatcgatatcatgatactgcggcggggcgctaaaacgaagggaagaagcattagtgtaattaattaaagcaagataatacgtatgtttgatcaattttcgaggcgataaccggccataaaaaagcgcaacgtagaacaggaattattctcacgaaagaaatccattaccatctctttatccagtccatagcggcgcgtcagaatacccgcttcccaggcgctaagctggcgatctccggtcttttcgtacatccggtgtgagtagcctaatacaaaaccgcgtttataatcggcacagaattttgtcacattaaccgcactgtcggcatgcgttgcttttaatcccgccattaagcctttaccaaaatggttattcatcgttcacctcattcgctatatattgtcatatatagcgatattttaggcaaagaacgacttttgcgcacgctattttttcatgcttgtttaagacgtaatcccgtaagagataaacctatcaggagagatatttatcgaaccatttcagtgtcctttgccaggcaagatcggcggcagatttgtcataacggggcgtggaatcattatggaatccgtgattaacccccggatagatatacgcctcataaaccttattattggctttcaacgccgcctcgtaagcaggccagccctcgttgattcgggtgtccagttccgcgaagtggagtagtaaaggcgcttcaatcttcgccacatcggcagtgggtgcctgacgaccataaaacggcaccgcgcaggccagttccggatacgcgacagccgccgcgttcgatacgccaccgccatagcaaaatccggtaatacccactttgcctgtcgcttgcggatagcgttgcataaactcaattgcggcaaagaaatcattcatcagtttgttggatcaacctgctgttgcagctcacgacctttatcatcatttcccggataacctccaacggaacttaagccgtcaggtgccagggcgatataccccgccttcgccactcgccgtgccacatcttcgatatacggattcagtccacgattctcatgcaccaccactacggctggcgttttgccgctcatctttgcgggcttcaccagataaccccgcacctcgccgtgaccatttggcgaaggatacgtgatgtactcagcaacaatttccgggtcggtaaactctacctgagtcgccagcgcataatttggcttgagcaaatcaaacaacgctaatgccgtcatcccgcctaccgcacttcgccgcaaggttgaggaactcacgtttcgagattttcccgtgagcgtaatagtcatagtaatccagcaactcttgtgggaaatctttggcggttaaacgcggcatcgttgcactcctcagttggtgtttttttaagcaaagcataagcacgtatttttgcccagtttttcgtcactctgtgagccagactacgggatacgcgctggcgaatcgctaaactagaaacattgtttcgaaattgaacggtggaaaggagaggtcatggtctggttagcgaatcccgaacgttacgggcagatgcaataccgctattgcggaaaaagtggtttacgcctgcccgcgttatcgctcggtttatggcacaatttcggtcacgttaacgcgctggaatcacagcgtgcgatcctgcgtaaagcgtttgatttgggcattacgcactttgatttagccaacaattacgggccgcctccaggaagcgcagaagagaactttggtcgcctgctgcgggaggattttgccgcttatcgcgatgaactgattatctctaccaaggctggctacgatatgtggcccggcccttacggctctggcggttcacgtaaatacctgctcgccagcctcgaccaaagcctgaagcgtatggggcttgagtatgtcgatatcttttactctcatcgcgtcgatgaaaatacgccgatggaagaaaccgcctctgcgctggctcatgcggtacaaagcggtaaggcgctgtatgtcgggatctcctcttactcgccagagcggacgcaaaaaatggtcgagttgctgcgcgagtggaaaattccgctgttaattcatcaaccttcgtacaatttactgaaccgctgggtggataaaagcggcctgctggataccctgcaaaataacggcgtgggctgtattgcctttactcctctggctcagggattgctgaccggaaaatatctcaacggcattccgcaagattcacggatgcatcgtgaagggaataaagttcgtggtctgacaccgaaaatgcttaccgaagccaacctcaacagcctgcgcttattgaatgaaatggcacagcagcgtggacaatcaatggcgcaaatggcgttaagctggttgctgaaagatgatcgcgtgacgtcggtattgattggtgccagccgcgcggagcaactagaggagaacgtgcaggcgctgaataatctgacatttagcaccaaggagctggcgcagattgatcagcatatcgccgatggcgagctgaatctgtggcaggcgtcttccgataaatgacctgttaataacgggcgcgcgaaccgcgcccgaatcagatcagtgattatgacgagtcagtcggtcaagatagcccatcacaaatgcagaaagcacaaacgtcagatggataatgacgtaccacatcagtttgttatccgggacatttttcgcatccataaagacgcgcagtaagtgaatggaagaaattgccacaatcgacgctgctactttgtttttcagcgacgttgcgtccattttccccagccagttcagcttctctttgttctcggagatatccagctgtgagacgaaattctcataaccggaaaacatcaccatcaccagcaaaccgccaaccagcgtcatatccaccagcgacagcaacacgaggatcaaatctgattccgccatcgagaagatattcggcagtacgtgaataatctcctggaagaacttcagcgccagggcaactaacgccagcgaaaggccaaagtacacgggggcaagcagccagcgagaagcatacattgcattttcaagaaaacgttccatacattcctgtcgtgtagttaaaacgggcaacagtatatcgcaattgagtaaacagcacgcaacagcaaatcaacatatacgttaaacctttgtcgcataattctgaggtttagggatcttcctggttcccttatcaacgcatcgagaacgtctacccttaaaggacgttgaacctgaagggagaaaaacgatgtctcatttaaaagacccgaccacgcagtattacactggtgaatatcccaaacagaaacaaccgacgccaggcatccaggcgaagatgacaccggtaccggattgcggcgagaaaacctatgttggtagcggtcgcctgaaagatcgtaaagcactggtgacagggggcgattccggaataggtcgcgctgccgccatcgcttacgcgcgtgaaggggctgacgtggcgatcagttatcttcccgtggaagaagaagacgctcaggatgtgaaaaagatcattgaagaatgcggacgcaaagccgttctgctgccaggcgatttaagcgatgagaaatttgcccgttcgctggttcacgaagcgcacaaggcgttaggcgggctggatattatggcgctggtcgccgggaaacaggttgccattccggatattgcagacctcaccagcgaacagtttcaaaagacctttgccattaacgttttcgcgctgttctggctaacccaggaagcgatccccctgctaccgaaaggtgcaagtatcatcaccacttcgtcaatccaggcataccagccaagtccgcatttactggactatgcggctacgaaggcggcgattctgaactacagccgtggcttggcaaaacaggtcgcggagaaaggtattcgggtgaatattgtcgcgccaggcccgatctggacagcactgcaaatttccggcggacaaacgcaggataagatcccgcagtttggtcagcaaacgccgatgaaacgtgcggggcaaccggcggaactggcccctgtatatgtttatctggcaagtcaggagtcgagctacgtcaccgcagaagtgcacggcgtgtgcggcggcgagcatttaggttaaaaaaatgcccggttgtgaaaagcaaccgggcatcattgtgaattcactcttacctgatgtggcgaaaacgccttatccgcctacaaacgcatgaagattcaacatgttgcaatagattttgtaggcctgataagcgtagcgcatcaggcattgagcacctaatgccggatgcgtcgtgaacgccttatccggcctacaaacgcacgaagattcaacatgttgcaatagattttgtaggcctgatgagcgtagcgcatcaggcaattctactttacttcgctttggcggtttcttcgccgaccagacctatcttcaggtaacccgcctgatgcagcgtatccattaccttcatcaacgtctcgtaatcgacggttttgtccgctcggaagaagatggtggtgtctttcttgccttcggttaacgcattcaacgccgtaatcattgtttcatcggtgaccggatcgttaccgataaacatcgagttgtctgccttcaccgacagataaaccggtttttccgggcgcggctgcggcgtgctggtagaagcaggcaagttcaccttcacatctaccgtcgctaacggtgccgccaccataaagataatcagcagaaccaacatcacgtcgataaacggcgtcacgttgatatcatgcatttcgccgttatcgtcgaggttttcgttaagatgcattgccatcggatattatcctgcgcgtaatttttgtgcgacacgaaccggatgcgcagcggcgctggcttccagatccaggtcacggctttgcagcaacaatacctgcgctgcaacatcacccagcatcgctttaaagccgccaatctggcgtgcaaatacgttatagataacgaccgcaggaatcgctgccacgaggccgattgccgttgctaacagagcttctgcgatacccggcgcaacgactgccaggttagtggtctgcgtttgcgcgataccaataaagctgttcatgatgccccagaccgtaccaaacagaccaacgaacggagaaatcgcgccgatggttgccagatagccgttaccgcggcccatttgacgacccactgcggcgacccgacgctccagacggaagctggtacgttctttaataccttcgttatcgtcgctgccttctgacagttccagctcattctgcgcttcattgagcaaatgcaggcttaagcttttgctaccaaaatcagcggcgatatcgttggcctggtttaaggaacgcgcttcagccagcagttgctgctcgcgcttaaggcgacgcttctgattgaagaactctacgctcttactgaagaagattgcccaggtgactacggaggccaaaataagcccaatcatcacgcacttaacgacaatatcggcgtgctgatacataccccagacggaaaggtccgtctgcattaaattattacccactgtgtatctccaggacgcaagtcacaaaatctgcgcataataatatcaaaacgacgtcgaattgatagtcgttctcattactatttgcatactgccgtacctttgctttcttttccttgcgtttacgcagtaaaaaagtcaccagcacgccatttgcgaaaattttctgctttatgccaattcttcaggatgcgcccgcgaatattcatgctagtttagacatccagacgtataaaaacaggaatcccgacatggcggacaaaaagcttgatactcaactggtgaatgcaggacgcagcaaaaaatacactctcggcgcggtaaatagcgtgattcagcgcgcttcttcgctggtctttgacagtgtagaagccaaaaaacacgcgacacgtaatcgcgccaatggagagttgttctatggacggcgcggaacgttaacccatttctccttacaacaagcgatgtgtgaactggaaggtggcgcaggctgcgtgctatttccctgcggggcggcagcggttgctaattccattcttgcttttatcgaacagggcgatcatgtgttgatgaccaacaccgcctatgaaccgagtcaggatttctgtagcaaaatcctcagcaaactgggcgtaacgacatcatggtttgatccgctgattggtgccgatatcgttaagcatctgcagccaaacactaaaatcgtgtttctggaatcgccaggctccatcaccatggaagtccacgacgttccggcgattgttgccgccgtacgcagtgtggtgccggatgccatcattatgatcgacaacacctgggcagccggtgtgctgtttaaggcgctggattttggcatcgatgtttctattcaagccgccaccaaatatctggttgggcattcagatgcgatgattggcactgccgtgtgcaatgcccgttgctgggagcagctacgggaaaatgcctatctgatgggccagatggtcgatgccgataccgcctatataaccagccgtggcctgcgcacattaggtgtgcgtttgcgtcaacatcatgaaagcagtctgaaagtggctgaatggctggcagaacatccgcaagttgcgcgagttaaccaccctgctctgcctggcagtaaaggtcacgaattctggaaacgagactttacaggcagcagcgggctattttcctttgtgcttaagaaaaaactcaataatgaagagctggcgaactatctggataacttcagtttattcagcatggcctactcgtggggcgggtatgaatcgttgatcctggcaaatcaaccagaacatatcgccgccattcgcccacaaggcgagatcgattttagcgggaccttgattcgcctgcatattggtctggaagatgtcgacgatctgattgccgatctggacgccggttttgcgcgaattgtataacattgccacttttggacaattttgcagacattttattgtgaaaagtcttaaattgttgcgtccgggatcaaggcgtcccggacgattcaggagtacaataggcagataaaggcttaaacgctgttccacaggaaagtccatggctgttattcaagatatcatcgctgcgctctggcaacacgactttgccgcgctggcggatcctcatattgttagcgttgtttactttgtcatgtttgccacgctgtttttagaaaacggcctgctgcccgcctcatttttgccaggcgacagcttgttgatactggcaggcgcattgattgcccagggggttatggattttctgcctacgattgcgattctgaccgccgcagcaagtctgggctgctggctaagttatattcaggggcgctggttagggaataccaaaacggtgaaaggctggctggcacagcttcctgctaaatatcaccagcgcgccacctgcatgtttgaccgccacggtctgctggcgctgctggctggacgttttcttgcatttgtccgtacgctgctgccaaccatggcgggaatttccggtctgccaaaccgccgcttccagtttttcaactggttaagtggattgctgtgggtcagcgtggtaaccagttttggctatgccttaagtatgattccgttcgttaaacgccatgaagatcaggtaatgacgttcctgatgatcctgccaattgccttgttaaccgctggcttgttaggcacgctgtttgtggtgattaaaaaaaaatactgtaacgcctgacgattttccccgttcccggttgctgtaccgggaacgtatttaattcccctgcatcgcccgcattcttgccgcatcttcccccggcgtcacaccgaagtaacgtttaaactcacggctaaattgcgatgcgctttcatagccgacgcgcatcgctgctgcgctggccttcatgccgtcatggatgatcatcatccgcgccttatgcagacggtaattcttcaaatactgcaacggcgaggtactggtgacagacttaaaattatggtggaacgccgatacgctcatgttggcttctgccgccagttgctcgacgctcaggttttcggtgtatttattctcaatccgtttcagcacgcggctaatcagactgaagtgagtctggcgactgaccagcgccagtaacgcgccgccgcaaggtccggtcagcacgtagtacagaatttcgcggatgatctgtttgccgagaatacgcgcatccagtggtcgctccatcacgtcgagtaaccgctccgccgcgcataaaatctcttctgataacgtggcggagttaatcccgctggctgccatcgacggctggaaatgctcatcttcgccaatgtccatcaacagttcctgtaactgcaaaatatcgacattgagacgcaaccctgccagcggcacctctgacgtggcataggtttcgcactcaaacggcaacggcaccgtcagcagcaggtattcattggcatcataacgaaacacgcgttcattgatataaccgattttatgcccggaaaagagaattatgatgccaggctcgtacatcaccggtgtacgtgcgaaaggcgtctcgccatacaacaaacgcacatcgggcaacagtcctgacaaactattttctttatttttcagtttattaactttatccgccagcaagcggcaaatctcttcacgtttcatatcgcgtaatttcttaggaataatgcggcaatttgattgtgcgcaattttgtagcatttctccagcactctggagaaataggcaagacattggcagaaatgagcattgagagccagggcgctggcgatcacaatgaaaaacatcaggcagatcgttctctgccctcatattggcccagcaaagggagcaagtaatgaacaactttaatctgcacaccccaacccgcattctgtttggtaaaggcgcaatcgctggtttacgcgaacaaattcctcacgatgctcgcgtattgattacctacggcggcggcagcgtgaaaaaaaccggcgttctcgatcaagttctggatgccctgaaaggcatggacgtgctggaatttggcggtattgagccaaacccggcttatgaaacgctgatgaacgccgtgaaactggttcgcgaacagaaagtgactttcctgctggcggttggcggcggttctgtactggacggcaccaaatttatcgccgcagcggctaactatccggaaaatatcgatccgtggcacattctgcaaacgggcggtaaagagattaaaagcgccatcccgatgggctgtgtgctgacgctgccagcaaccggttcagaatccaacgcaggcgcggtgatctcccgtaaaaccacaggcgacaagcaggcgttccattctgcccatgttcagccggtatttgccgtgctcgatccggtttatacctacaccctgccgccgcgtcaggtggctaacggcgtagtggacgcctttgtacacaccgtggaacagtatgttaccaaaccggttgatgccaaaattcaggaccgtttcgcagaaggcattttgctgacgctaatcgaagatggtccgaaagccctgaaagagccagaaaactacgatgtgcgcgccaacgtcatgtgggcggcgactcaggcgctgaacggtttgattggcgctggcgtaccgcaggactgggcaacgcatatgctgggccacgaactgactgcgatgcacggtctggatcacgcgcaaacactggctatcgtcctgcctgcactgtggaatgaaaaacgcgataccaagcgcgctaagctgctgcaatatgctgaacgcgtctggaacatcactgaaggttccgatgatgagcgtattgacgccgcgattgccgcaacccgcaatttctttgagcaattaggcgtgccgacccacctctccgactacggtctggacggcagctccatcccggctttgctgaaaaaactggaagagcacggcatgacccaactgggcgaaaatcatgacattacgttggatgtcagccgccgtatatacgaagccgcccgctaagctttttacgcctcaaactttcgttttcgggcatttcgtccagacttaagttcacaacacctcaccggagcctgctccggtgagttcatataaaggaggaacgtatggctaatccaaccgttattaagctacaggatggcaatgtcatgccccagctgggactgggcgtctggcaagcaagtaatgaggaagtaatcaccgccattcaaaaagcgttagaagtgggttatcgctcgattgataccgccgcggcctacaagaacgaagaaggtgtcggcaaagccctgaaaaatgcctcagtcaacagagaagaactgttcatcaccactaagctgtggaacgacgaccacaagcgcccccgcgaagccctgctcgacagcctgaaaaaactccagcttgattatatcgacctctacttaatgcactggcccgttcccgctatcgaccattatgtcgaagcatggaaaggcatgatcgaattgcaaaaagagggattaatcaaaagcatcggcgtgtgcaacttccagatccatcacctgcaacgcctgattgatgaaactggcgtgacgcctgtgataaaccagatcgaacttcatccgctgatgcaacaacgccagctacacgcctggaacgcgacacacaaaatccagaccgaatcctggagcccattagcgcaaggagggaaaggcgttttcgatcagaaagtcattcgcgatctggcagataaatacggcaaaaccccggcgcagattgttatccgctggcatctggatagcggcctggtggtgatcccgaaatcggtcacaccttcacgtattgccgaaaactttgatgtctgggatttccgtctcgacaaagacgaactcggcgaaattgcaaaactcgatcagggcaagcgtctcggtcccgatcctgaccagttcggcggctaacatgcaaattctcccggtggcggtaatgttccgctaccggacttttcagaaatcatttattcccctcgcgtcccgcccgttgttactcttccttgttcaggaatgccaaatataaggacatcatcatgcagagccggaagctcttaaaagaacaactcatctatatccgggataaacgcaacggagaggtgaaaaacagatgaaaataatacttctgtttttagcagccctggcaagttttaccgtacacgcacagcccccctcacagaccgtagaacaaacagtccggcatatttatcagaactataaatcagatgccactgccccttattttggtgaaaccggagagcgggcgataacttctgcgcgtattcaacaggcgcttaccctgaacgacaatcttacgctgccgggcaatattggctggctggattatgatccggtttgtgattgtcaggattttggcgatctggtgctagaaagcgttgcgataacccaaactgacgccgatcatgccgatgccgttgtgcgctttcgtatctttaaagatgataaagaaaagaccacgcagacactgaaaatggtggcggaaaatggtcgttgggtcattgacgatattgtcagcaatcatggcagcgtcttacaagcagttaatagcgagaatgaaaaaacgctggccgctttagcttcgttgcaaaaagaacagccggaagcctttgttgccgaactctttgaacatattgctgattatagctggccgtggacgtgggtggtttccgactcttaccgccaggcggttaatgccttctataaaaccaccttcaagacggccaataatcccgatgaagatatgcaaatagaacggcaatttatttacgacaatccgatctgttttggcgaagagtcgctattttcacgcgttgatgaaattcgagtcctggagaaaaccgccgattccgcccgcattcatgttcgttttacgctgaccaatggcaacaacgaagagcaagaactggttttacagcggcgcgaaggcaagtgggaaatcgctgattttatccgcccgaacagcggcagcctacttaagcagattgaggcaaaaactgccgccagattaaagcaatgagctgaattaaataacaattagccggaacaataaataaaagggaacactatatgaaaacgattttcaccgtgggagctgttgttctggcaacctgcttgctcagtggctgcgtcaatgagcaaaaggtcaatcagctggcgagcaatgtgcaaacattaaatgccaaaatcgcccggcttgagcaggatatgaaagcactacgcccacaaatctatgctgccaaatccgaagctaacagagccaatacgcgtcttgatgctcaggactattttgattgcctgcgctgcttgcgtatgtacgcagaatgataaaaaaatccccggtagcgtgtcagttgccggggatattttttaacgtccaaccgccgctttaggccgtttcttcgcaccagcattcaccggacgagattgcgtagacgacgctttttttgccgtagcaggcgtctgacgctgggtcgccatcggcgtatgtttcgtcaacgccggacgggtattgcggttctggcgacgagcttcacgcatctcttcaatggttggcgcaggcactaagcaatcgcgacggctgccaatcagatgctttttgcccatcgcttccagcgcctggcggattaacggccagtttgccggatcgtggtaacgcaacaacgctttatgcaaacgacgctgtttgtcgcccttcggtacgaagacgtcttcgctcttataaccaatcttcgccagcgggtttttcccggtgtaatacatggtggttgagttcgccagcggcgacggatagaagttctgcacctggtcgaggcggaagcggtgctttttcagccacagcgccagattcaccatatcttcatcacgcgtaccggggtgcgcggagatgaaataggggatcagatactgctctttacctgcctgttttgagtaagtatcgaacagctctttaaagcggtcatagctgcccatgcccggcttcatcatcttcgataacggcccttcttcggtatgttccggggcaatcttcagataaccgccgacgtgatgggtcgccagttctttgatatagcgcggatcttctacggctatgtcataacgcacaccagaggcaatcaggatctttttaatgcctttcagatcacgcgcacggcgatagaggttgatcgttggttcgtggttcgtgtccatgtgcggacaaatatccggataaacgcacgacaaacggcgacaagtttgttcagcgcgtggcgatttgcagcgcaacatatacatgttggcagttggcccaccaagatcggaaatcacgcccgtaaaacctggaacggtgtcgcggatcgcttcgatctcattaatgatcgaatcttcggaacggctctgaataatgcgcccttcgtgctcggtgatagaacagaaagagcagccgccaaagcagccacgcataatgttgaccgaaaaacggatcatttcgtaagccggaatacgggcattgccataggccggatgtggcacgcgcttgtatggcagcgcaaaaacgctgtccatctcttcggtagaaagcggaatagcaggcgggttgatccacacatagcggtcgccgtgtttttgcatcaatgcgcgggcacagcctgggttggtttcgtggtgcagaatacgcgaagcatgggcgtacagcactttatcgcccttcactttctcgaaagaaggcagcaacacgtaggttttttcccacggtttcgggcgcggtggctgcacggttacggctttggcttcctgctttttcggtgccaccggtttgttatccgcgcacggcaaatcttcaccatacggatgcgggattgggtcgatttttccaggggtatcaagacgggtggaatccacgccgctccagccaggcagcgcctctttcacgataatcgcggtattacgcacatcgcggatttcactaattggctcgcccatcgccagacgatgcgccacttccaccagcggacgctcaccgttaccaaacatcagcatgtcggctttcgaatccaccagcacggaacggcgcacggtatcggaccagtaatcataatgcgcggtacggcgcagactagcctcaataccgccgaggatcaccggtacatctttccacgcctctttacaacgctgggtataaaccagtgtggcgcgatccgggcgcttacccgcgacgttatccggcgtgtaggcatcgtcatgacgtaaacggcgatcggcggtataacggttgatcatcgaatccatgttgccagcagtaacaccgaaaaacagattcggtttacccagacgcataaagtcgtctttgctgctccagtccggctgggcgatgatcccgacgcgaaagccctgcgcttccagcatacgaccgcaaatcgccatcccgaagcttgggtgatcgacatacgcgtcgccagtaaccaaaatgatgtcgcagctatcccagccaagttgatccatctcttcacgagacatcggcaaaaacggtgccggtccaaaacaggcggcccagtactgcggccaggagaacaggtcgcgatccggttggatcagggagatagagctcattttgcttccagaaatgataaaaaaataatcaaaggccggggattataagccggaacgaaagagaaatcgaaaggtattccatactcgccctcctcgggcgagtatgaagattacggtaccggattgaccaacagttgcccaatcgagccacggtccgccatttccagcgtctgactgttgaagtagaacgggaagtgcgcccaggaaggctgaccgaaataaacaagcagctccacttgtccgtcaacccaaacggtatctttccagcctctgtcttccgggaacggcatcgcgccattcacgttacggatctggaacattacgccttcaatatggaacgcttgcggctcgtccgcgcgtaccgtccagcgttcccacgttccttgctgcgcggtgacatcaatacggttgacgtcccacagctgtccattaatacccgggtcatcacccagactgatatcgcgactgcgaattggcgaaccagccatgatttcagttggcagcaagcgcatcggaagactgtctgtgaccagcggcagaaggccggttgggcgcagcgttagcaccagggtagaaaccagaatactggatggctcaaagaagccacgaatacgatcaacaatgctcgccgcttcgccacaggtgatcgacacttcatcgccgttgctcatatccaccagaatctcgcggcgctcgcccggtgccagcgaaagttgcttcaccgatacaggagcaggcaggaatccctgatcgccagaaatcacatgtaacgggcgaccatcgttcatctgtagttgatagcgacgagagttcgacgcgttcagcagtcgcaagcgcacccagccacgcgagacttcaacgtacgggctttgtacaccgttaaccagcagcgtatcaccaacaaagccgccgcttcccggttcgttgtattctggcgtaccaaagttatccagccgtttatcctggataatgaccggaaaatcatccacaccataatggttggggataggcagcgacttgctgacttcatcttccaccagccacattccggcaaggccgttatagacctgctgagccgtgcggttgggagtattggcgtgataccacagagtagctgcgttctggcgaatgggcagtacgggtgcccagtcagcgtttggcgacatcatccgtgccggaccgcccatcagcgggcctggtacctgtagcccggccaccgtcattgagacattttctgtcaggcggttgctgtaaataagcttaacatcgtcgcccttccagacgcggatagtcggccccaggtaacgaccattgattccccagaccgacgcgcgtgtccctggcgtaaatgaccagtgcgcacgttgtacagtcataaacagcggttgcccacggcgagattcaagtagcggcggaacgggtagcggttgctgttgcccggctgcgctggccttcaggggaacagcgcctgcacaaagtgcaatccccgatgcctgaatgaactgacgccgactgagtgacatatttgctccatgtaaaactggctaaagtaataccgtgcaggaaagtgttccccgcaaaaatacagattgccgacttaaacttttccggcggcttcgcgttctgcgacttctttatcgagctcggcgattttttgttccattatcgaacgacaatgggcagccagctcacgaacctgatctttgccatactgactgacgtcaattggcggcagcatttcgacaatcaccagaccgttgtgcagtcgattaagattaatcttattcgaagttgtagagacgcacacgggaataatcgggacgcccgccgcaattgccgcgtgaaatgctccagtcttgaacggtagcaggccgcgaccacggctgcgggttccttccgggaacatccagatggaaatacggcgttttttgaagtgattcactacttccgcaatggtgccgtgagctttagtgcgattgtttctgtcgatcaataagttgccggttaaccagtacaactgcccgaagaaggggatccacagcaagctctttttacctaccgtcaccgtcggcggttgcacgatgttcgatgctgtcaccatgtcatagttgttctggtggttagcgatatagatagcattgccgtagctttcagcgtctgtaggtttacggcactcaactttcaggccaaacagcggcgcaagacggccaaacatatgcccaaaggtggccacatgtttcgggttacgcgggctgaaaaggcagtaaatggagccgaatacacagactaagatgctgtaaatcacggtaataataagacgaaagatatatagcataacaccctctgaaggtctgagagactggcattgtacgtcacctgaaatcaggttagggcattgttaaaagccgctctctggaaaagcgtattgttaatcgcaacgcatgaataaacaacggtttcaagggaatttttatcgtttccgggggttgaatacgctgccggatgacgacttaacgtttcatccggcgttccttgcaagcgggaggaaacagcgccctccccggcatattactcttcgctatcaccgctgctggcacggcgaggagagtcgatctcaacacgatcgatacgctgcaaaccgcgcatcaacgtaccgcggcgtccacgttcgccagtgactttctgtaactcttccgggcgcagtttaattttgcgtttcccaacatgaatggtcagcgtgctttgcggcggcagaacgtacaattgcgccagaccatcttctccacgcgcggcttctgccgatggaatgttgataatcttgttgcctttgcccttcgacagctgcggcagatcacttaccgggaacatcaacatacggcctgcctgagtgattgccagcagcatatcggaagcatcttcaatcaccaccggcggcataacatgggcattttccggtaaggtgatcaaagccttacctgcacggttacgcgccaccagatcgttaaaggtgcagacgaaaccgtaacccgcatcggaagccatcagcagtttctgatcgtcgctttccatcagcatatggtcaacggtcgccccaggcggcaacgttaatttgccggtgagcggctcgccctgaccacgcgccgacggcagcgtaatcgggtcaatggcatagctacgaccggtggaatcaacaaacactaccggttggttgctcttacctttcaccgccgctttgaagctatcacccgctttataattcaggcccggcgcgtcgatatcatggcctttagcgctgcgtacccagcccatctgcgacagcacaatggtgacaggttcagacggcagcatgtcgtgctcgctcatcgctttcgcttcttcgcgttcctgcaacggcgaacgacgatcgtcaccgtaggcttgcgcgtctgcctgcagttctttcttcagcaggttattcattttacgctcggaagccaaaatgccctgcaactggtcgcgctctttttccagttcactctgctcaccgcgaatcttcatctcttccagtttggcaagatgacgcagtttcagttcgaggatcgcttccgcctgggtttccgtaaggccaaaccgcgacatcagcgccggtttcggttcatcttcattacgaatgatctcaatcacttcgtcgatattgagaaacgccaccagcaaaccttcgaggatatgcaggcgcttgaggactttctccagacgatagttcagtcggcggcgcacggtatcgcggcggaacaccagccattcggagaggatttccagcaggtttttcaccgccggacgaccatccagaccgatcatattaaggttaatacgatagctcttttccagatcggtggtagcgaagaggtggttcatcacctgatccatatccacgcggttggaacgcggcacaatcaccaggcgggtcgggttctcgtggtcagattcatcgcgcagatcgtcaaccatcggcagctttttgttgcgcatttgcgcagcaatttgctccagtacgcgcgcacctgaaacctgatgcggcaatgcgctgataaccaccgcgccatcttctttcttccacaccgcgcgcatacgcactgaaccacgtccgttctcgtagattttacggatctcggcgcgcgaagtgataatttccgcttcagtcggataatccggcccctgcacgatatccagcagctgatcgagcgtggttttcggctggtcgattaatgcgattgccgcctgagccacttcacgcaggttatgcggtggaatatcggtcgccatgccgacggcaataccggtggtgccgttaagcaaaatgtttggcagacgggcaggtagcattttcggctcctgcaaagtgccgtcgaagtttggcacccagtcagccgtcccctgccccagctcgctcaatagcagctcggaatatttcgacaaccgggattcggtgtaacgcattgccgcgaacgatttcggatcgtccggcgcgccccagttcccctgaccatcaaccagcggataacggtaagagaacggttgcgccatcaggaccatcgcttcataacaggcgctatcgccgtgcggatggtatttacccagtacgtcaccgacggtacgggccgattttttaaatttggcgctggcattcaggcccagttcagacatcgcatacacaatgcggcgctgaacaggtttcagaccatcaccaataaacggcaacgcacggtccatgatcacgtacatggagtagtttaagtaggcgttttccgtaaattcatgtagcgcaaggcgctctgccatatcgctcattaattctgattcctcaacttattcgccagccttcaaaggggcaatattgccggagatactacattatctgccgcgtcgagtcacaggagatcaacgtgaatagcgccgccggacgtgctccgacggcgataaaggcatcaatgtgccttgatatacaactctttgctgtagacataatcctggggattatgcagcggaaaaccgccaacgtagggtttaagcagtttgattaacggctgatagtagataggaatcagcggtgcctgttggttgatgatcacttctgcctgctgatacaacgcattacgctttgtcgcatcagtgatctgcgtggcctggtttagtaaggcgtcatactgcgcatttttccagtgaccgacgttttcttcactatcgcttttgagcgtgttcaggaagctggaagcatcattgtacgtcgcatcccacgactgccgagacagcatgaaatcaccggctcgtcgggcatcaagataggttttccactccattgtgcgcagcgtcacctgtgcacccagccattttttccattcggaagacaacgctatcgcggtcttttcatgcagatcgtacttgttgtagaacagctcaaagcgtagcggatgagaggcgtcgtatcccgcctgtttcagcaaggcttttgccatcgcgacgcgctcactcattggcttttgcagttcatcgaacgtcgtcgcgctaaagccttttacctctggcggcgtcagcgtggttgcgggcgttctcaaccccagtaccttttgcgcaataagctgtcgatcaaccgtaagatatagcgcccgacgcactcgcacatcgttaaatggcggtttctcaaggttgaagttgtaatattcgctgttcagacgcggaataattcgtagctcgccaggcagtgatttttcaatggcgggaatttgctgcgccggaacccaggtgagatcgacctctcccgcgcgatagcggttatagccggtgaccgaattatctagcgccagatactcaacctgttgcaatactgtatgttgcgcatcgcggtactttggatttttgcgtgcagtaatcttttcgttaactacccactgatcaagcacaaaggcaccgttgtaaaccatgttctctggcttactccagctatcgccatgtttagcgatgacatgatgaggaaccgggaacagcgtcggccaggcgagcatcgtcgtgaaccaaggaaccggctgctcaagcgtaacttcaagagtacgatcatccgtcgctttgacacccagcgatgtaacatctgctttacccgcaacaatagctgcggcattgttaatgtgcgcctgtgccagatagccagcaaaagggcttgccgttttcgggtcaaccgcgcgctgccagccgaggacaaaatcctctgccgtcagaggctgaccgtcggaccactgcaaaccgctacgcagatggaaaatatagcgcttgccgccgtccagtatctcccagcgttcagcctgagcgggctgcacctggccttcaccgtccatccataccagaccttcaaacagatccagcacaatctgcgcggcagtattctcctccaccttttgcgggtcgagcgtacctgggtcgctatgattgttgtaacgaaagacttgttgcggggcgagcggtgtgttggcgggaacgtcagcagcgtagagaggagccgcacttaccaggctgaccagccataataaatttcgcgtatacatggtattccttaccggagaaattataagcccaacaacaatacgcctgtggcattgttcgctcaaacttatcgcgagtgatttggctcacactccggtaaagaaaaaagcgagttgcccccgcttttccattaattaacggatttcattcaatagttctggatgcttatccagaacacgtaaaagtttgattgtggaaggatgaggttgggcattgcctttttcgtaacgcgaaaacgcatttacacctcccccaaaaatttcgcttgcctctttttgggtaagagagagcttttttcgaaccttcactataaattcaggtgccactgtttcggcattcaccgaagcccgaaatgcctttacttgcgccatgaaagcatctgactcttctttattcatgatgctctcttcgcaatggacacaatataaaccgtggatacctttcaatactgtttttcgtccacggaaggtgtatggaatatctttaatgccagaaaccatttctccctggtggcaaaccggacatttcatattacttctccttaaacgagacgatcagtacgtcatgaattaccgtaattttaagataaacctggcctgtaacaagcctgggtctgtaaacatcctgccagatagtatgatcagagtaggtggtcatgcttttataaaagtcgctctctgataatccaatgataacattacacataccatcaaaatccaaacctaactcatctgcatttaacagggcactacgtgttgtacgaacttgcccggcattgacaagttttttaacctgactcaaacgtgtatgtggtgtgcgtttttccataacccccgcctccctgttactttagttataacctaaaaggttaattacagcaatgaaaaagcacctaaaaggttagttagatgtacggagatagtgaccacacaaaacgtattctttaaggaaagtgattgaccatataagaaagtggcgcattagtagcgccagtttgaagcaggaatttataagggaagctggagtcaggcatcacgccaacggcacataaacatccgtttccagtcgctgctctgtcaccccttcggcaagattggtgtagtgaaacagaatcggtgctttacgcattttctcgccgcttgcaggcagccagtggcgaatgatgccccataccgtgtgtgaaatatcgtccagctcgccaacgtggcgggccacggcataacgtccaccggtaagttcaccattgctcacaccataacgattatcgggaatcggttcgctaacgctgccgcagatatcaaagcgaaacgcttccggtgcggtggtggcagggtcgtcccaggcgacgccaaaagtctggctttggttaacaggagaaagccccgtctctttacgccacatgataaatttcgccacgctgtagttgagcaattcagggctacagcggtgcggcaacatcgccacaggtattgatgggaaatcgataatgtttacatccagtgtcaggtttgtcattttgcctccctgcgaaattattcccgggaacgcgtcccgggagcggtaacaattacggatttactttgcggatctgtttgacgtcaatttcaacagaattccagtctttatcgacttcaccctgaatctcaaccgtatctttcggcgtcaccgtcacgccgttccagcgtttgtggtcgatatcaacattgatagtaccgctggcatctttgaacacgtagagatcgtcagagatgcgttcaacgatattgccgcgcagggttacccaggtgtcgtcacgcagggattttgcgctttctacagtcgttacgctgccgttcggcccctggaatcctccggcctgactttgcgttgccgatgggccagaaaaaccgccctgctctgctgccatcaccggtgcgctgcacagggccattactgcgattactgctgcgaattttttcatgtttattactccctttaatgtctgtttccgagcatttaacaagatagtccttaacaacttcttaagggaaaaaaataaaatttagtgctgtacagagcgcgttacaacacggtttactggcagcaaatacggttatcgcagggatgaaaaaatgcgaattttactgatagaagatgacatgctgattggcgacggcatcaaaacgggccttagtaaaatgggttttagcgtcgactggtttacacaaggtcgtcagggaaaagaggcgctttatagcgcaccttatgatgcggtgatcctggatttaaccttaccaggcatggatggtcgcgatattttgcgcgaatggcgagaaaaaggtcagcgtgagccggtactgatcctgaccgcgcgcgatgcgctggcggaacgtgtagaagggctgcgtctgggagctgacgattatctgtgtaaaccttttgcgttgatagaagtcgccgccaggctggaagctctgatgcgccgaaccaacggccaggccagcaacgagctgcgccacggtaacgtcatgctcgaccccggcaaacgtatcgccacgctggctggcgaacccttaacactgaaaccaaaagaatttgccctgctggaattactgatgcgtaacgctggtcgggtactgtcgcgcaaactgattgaagagaaactgtatacctgggacgaagaggtcaccagtaatgccgttgaagtgcatgtgcatcatctgcgacgcaaactcggtagtgattttattcgtaccgtgcatggtattggttacacattaggtgagaaatgaaatttacccaacgtcttagtctgcgcgtcaggctgacgctaatctttttaattctggcctcggtgacctggctgctttccagctttgtcgcctggaaacaaacaacggataacgtcgatgaattgttcgacacccaactgatgctgtttgccaagcggttaagtacgctcgatctcaacgaaatcaacgcggcggatcgcatggcacagacgccaaatagattaaaacacggtcatgttgatgacgatgcgctgacctttgccatctttacccacgacggcagaatggtccttaatgatggcgataacggagaagatattccctatagctatcaacgggaaggttttgctgacgggcaactggtcggtgaagacgatccttggcgttttgtctggatgacctcacctgatggcaaatatcgcatcgttgttggccaggaatgggaataccgtgaagacatggcgctggcgattgttgccgggcaattgatcccgtggctggtcgcactgccgattatgttaatcatcatgatggtactactgggtcgtgaactcgcgccgctgaacaaactggcgctggcactacgtatgcgtgaccctgactcggaaaaaccactaaacgcgactggcgtacccagcgaagtgcggccactggttgagtcgctaaatcaactgttcgcccgcacacatgcgatgatggttcgtgaacgacgctttacctccgacgcagctcacgaacttcgtagcccgttaacggcgctgaaagtgcaaaccgaagttgcgcagctctctgacgatgatccgcaggcgcggaaaaaagcactgctccaattacattccgggatcgatcgcgctactcgtctggttgatcaactgctcacgctatcgcggctggactcactggataaccttcaggacgtcgcggagatcccgcttgaagatctcctgcaatcgtcggtgatggatatttaccacacggcgcagcaggcgaaaattgacgtgcgactgacactcaatgcccacagcatcaaacgcaccgggcaaccgctattgctaagtttgttggtgcgaaatttgctggataacgccgtgcgctacagtccacagggcagcgtggtagacgtcacgctgaatgctgataatttcatcgtgagggataacggccccggtgtgacaccagaggcactggcgcgaattggcgaacgcttctatcgcccacccggacaaaccgctaccggcagcgggcttgggctatcgattgtccagcgaatcgccaaattgcatggcatgaatgttgaatttgggaatgcggaacaaggtggatttgaggcgaaggtaagctggtaacttctctgtctatgagagccgttaaaacgactctcatagattttactaatagcaaaatataaaccgtccccaaaaaagccaccaaccacaaaccagacaaataccgagcgagaatacatatacccaaaactcgaacatttcccgcataaagagttttcttaagataagaataataagtggcgtaagaagaaaaaatgctgcaatcattgcttgcaatatacgatcttcgcctgaaacggaaggtatactgcaaatatttcctcccgactcaagcatccagtcatacttattgaaagcaaaaaaagaatctattaaccaataagtaagcattatatatagcaatgcttcaaatattgttttaattttctgctttaacatatatcagtacgctcataaaaatccatttataattatcaacatgacacgttgatactttcatcttttacttattcaaagccatattttcaatccccaaaaaaaccgaaccaaacgtgtaaattattccggtgcgagtaagaattatgaggaatggctatcagtattgtcattttcagaaaatatttatcctgcatcggtgagtcagagtaagatcagacttttgctaaattcgcaaaagactttgcacattttgctaatttcaccgtaccgctctgtgacgtactatagtcggcaaacgtctcaccttgaggttaaaaaatgagcaacatcctgattatcaacggcgcgaaaaaattcgcccactccaatggtcaactgaacgacaccctgaccgaagtcgcggatggcacactgcgcgaccttgggcatgatgtccgcatcgttcgcgccgacagcgactacgatgtcaaagcggaagtacaaaactttctctgggctgatgtggtgatctggcagatgccaggctggtggatgggcgcgccgtggacagtgaaaaaatacattgatgatgtattcaccgaaggtcacgggacgctgtatgccagcgatggtcgtacccgcaaagatccgtcgaaaaaatacggttccggcggcctggtacagggcaaaaaatatatgctttctctgacctggaacgcaccaatggaagccttcaccgaaaaagatcagttcttccacggcgttggcgttgacggtgtgtatctgccgttccataaagcaaaccaattcctcggtatggaaccgctgccgacatttatcgctaatgacgtgataaaaatgcctgatgttccccgctatactgaagaatatcgcaagcatcttgtggaaatttttggttaactagagctcaggctttagaaggagttaaccatgcttaccgtaatcgcagaaatccgtactcgtcctggtcaacatcaccgtcaggcggtattggatcagtttgctaaaatcgttccaaccgtactgaaagaagaaggttgccacggctatgcgccaatggtggattgcgcagctggcgtgagtttccagtctatggcaccggattctatcgtgatgattgagcagtgggaaagcatcgcgcatcttgaagcgcatctgcaaaccccgcacatgaaggcgtatagcgaagccgtaaaaggtgacgtgctggagatgaatatccgtattctgcagccagggatttaatcctgccttgtttgcccggccatcctgaccgggcaatgttctttcctttaaacctcaatctccgccatgtcgcctttctcttgcaaccagttgcggcgatcttccgagcgtttcttcgccagcagcatatccatcatcgcgtcagtacgctgatcgtcttcatcatcgatagtcaactgcaccagacggcgagtgttcggatcaagcgtggtttcgcgcaattgcatcgggttcatttcccccagacctttaaaacgctggacgttcggcttgcctttcttgcgttttaattgctcaagtacgccctctttctcttcttccgtcagcgcgtaataaacctctttcccgagatcaatacggtagagcggtggcagtgcgacgtaaacgtgaccgtgtttcaccaacgcgcggaaatgttttacgaacaaagcgcagagcagcgtggcaatgtgcagaccatcagagtccgcatccgcgaggatacagattttgccataacgaagctggctcagatcgtcgctgtcaggatcgataccgatcgctaccgaaatatcgtgcacttcctgcgaagccagcacttcgtcggaagagacttcccaggtgttaaggatcttacctttcagtggcatgatcgcctgatattcgcgatcgcgcgcctgcttggcagatccgcctgcggagtcaccttccacaaggaacagctcggtacggttaaggtcctgcgcggtacaatcagccagtttgccaggcaacgccgggccgctggtcagctttttacgcaccacttttttggccgcacgcatacggcgctgggcgctggaaatcgccatctccgccagcagttcagccgcctgaacgttctggttcagccacaggataaaggcatctttcaccacgccagaaacgaatgccgcgcattgacgcgaagagagacgctctttcgtctgcccggcaaactgcggatcctgcatttttactgacagcacataggcgcagcgatcccagatatcttccgccgacagctttacaccgcgcggcagaatattgcggtattcacagaactcacgcatcgcgtccaacaggccctgacgcagaccattaacatgggtaccgccctgcatcgttgggataaggttgacgtagctttcggtcagcagttcaccgccttccggcagccacagtagcgcccagtccacagcttcagtatcaccagcgaaattaccgataaacggtttttccggcagcgtcggcagaccatttaccgcttccgccaggtaatcattcagaccgtcctgatagcaccagcgttgttcggtattgttgatctcatctttaaaagtgatctcaacgccagggcacaataccgctttggctttcagcacatgcgtcaggcgtgaaacagaaaatcgcgggctgtcaaagaaggtttcatccggccagaagtgcacactggtaccagtattgcgtttaccgcaagtgccgacaacctgtaaatcctgcaccttttcgccattttcaaaggcgatgttataaacctgaccatcgcggcgcacgttaacttctacgcgcttcgacagggcgttaaccaccgaaatccccacgccatgcaggccgccagagaactggtaatttttgttagagaatttaccgcctgcatgcagacggcaaagaatcagttcaaccgccggtacaccctcttccgggtgaatatccaccggcatcccgcgcccatcgtcaataacttctaacgactggtcagcatgtaaaataacgtccacgcgttttgcgtgacccgccagtgcttcatccacactgttatcaatgacttcttgccccaaatggttagggcgagtggtatcggtatacatccccggacggcggcgaaccggctcaagcccggtgagtacctcaatggcatcagcgttataagtttgcgtcatggtttaagttagtaattcgagttgatcgtcagagatggtgcagaccaagaaaatcgacgatcgggttgaaataatcttcgaagcccgtgaatgcgtggttgccgccttctatgacagtctggcggcaggaagcgtagtacgccaccgcctggcggtaatccagcacttcatctcccgtctgttgcagcagccagatcaaatccggcgcttccagcgggtcaatctgcatgactttaagatcgtaaatatggcgtgactctagcacatattgctgcccggtgtaggggttctcgttctgaccgagatagtccgtcagcagttcaaacgggcgcaccgccgggtttaccaccactgcgggcagcataaaacattgtgacaaccaggtggcgtaatatccccccagtgacgaaccgacaatacccagcgaatcaccgccatgttccaggacaatggattccagcagctctgccgcgtcggaaggatacggcggcaactgcggaatgatcatctcaacgtcagggtgatgttccgccagccagttttttaacaagctcgcttttgcagagcgcggcgagctgttgaaaccgtgtaaataaagaagcgtagacatcagtagccttctgaagcggtatcaggttggaaacgtgtgtccgccaggcgatgcacctcggtggtcagcgtgccatcagcatgtaactcgagagtacgccagccgggcgcgatggtatccagcgtaaagttggaacagtgcggcttaaactgcacacaggtcgacggcgttgccagcaggcggcgaccattccagtcgagatccagctcctgatgaatatgaccgcacagcaagtatttgacgtgcggaaacttcgccagcacggtatccagttcgcccgcgttacgcagactgtgttgatcgagccaactacaacccgcaggtagcggatgatgatgcagcagcagcaacgtatggcgttctggcgcatcggccagtttacgttccagccactcaagctgaaactcgctcagctcaccgtgcggcacgccaaacacctggctatccagcaacaggatttgccattgctcaccaataaacacgcgcttcgccggggagatacccgcatcctgtaacgcgctgtacatcgcgggctggaaatcgtggttgcccggcagccagacgcagggcgcacgaaaacttgcgatgccttcagcgaaatgctgataggccgcagaggattgatcctgcgctaaatcacctgtcgcgacaatcaggtcgaattcgtgctggtgtggccgaatcgcctccagcaccgcctggtaactctcccaggtgtttacccctaacagggcttcgtgcttttgtgcaaacaggtgagtgtcggtaatttgtaaaatcctgactctggcctcaccagccagaggaagggttaacaggctttccaaatggtgtccttaggtttcacgacgctaataaaccggaatcgccatcgctccatgtgctaaacagtatcgcaaccagtccgctaaaaactgattaatttgatgcttttcgtcgcgttgatgcaactttttattaggataatcataccgcgctttgaagcgaaaaatctgctggcttgaacacacttcagccaccatcgcgtcatgatacagacgcaccgtcattgacggaaggctccagtaactgatcgcgggcgcagtctgttctattgtcaccagggtagtgtatcgggtcgattccacaatcgtcagccgatattgtgcgtttgccacctgatagcttacagtttcgccgggtgcgtcattgcgcggtaacaaacggcgcaattgtgaaaagttcatctcgcacaggcgcatcatttcaggaaagtcaggtgtgtaacgcttcatttatgcccactcattttttaacgcttgatgatgcagctgcagccattgcaaagcgatgaccgacgctgcgttgtcgattttcccctcttctacccactggtatgcctgttcccggcttaccacatgaacgcgaatatcttcgttttcatcagccagaccgtgaataccgcttgcggtcgtggcgtccacttcgcccaccataattgacgaacgctcactggtgccccccgggcttgccaggaaacttaacaccggtttggtccgtttgactatcagtcccgcctcttcaatcgcttcgcgacgggcaacatcttccacactttcaccctcttcaatcatcccggcaaccatctccagtagccaaggggtttcgctggtgtcgtacgcggcaatccgaatctgctcaatcagcacaacttcatcacgcactgggtcaaagggtagcaagactgcggcgtgaccgcgctcaaaaatttcccgccgcacctcatgactcatttgcccgttgaatagacgatgacgaaatctataaagatctaatgaaaaaaagccgcgataaagtgtttctcgtgcaataatttctacatcgtttttgccaaatgtaacgggcaggttgtctggcttaagcattgttaatgtcctggcactaatagtgaattaaatgtgaatttcagcgacgtttgactgccgtttgagcagtcatgtgttaaattgaggcacattaacgccctatggcacgtaacgccaaccttttgcggtagcggcttctgctagaatccgcaataattttacagtttgatcgcgctaaatactgcttcaccacaaggaatgcaaatgaagaaattgctccccattcttatcggcctgagcctttctgggttcagttcgttgagccaggccgagaacctgatgcaagtttatcagcaagcacgccttagtaacccggaattgcgtaagtctgccgccgatcgtgatgctgcctttgaaaaaattaatgaagcgcgcagtccattactgccacagctaggtttaggtgcagattacacctatagcaacggctaccgcgacgcgaacggcatcaactctaacgcgaccagtgcgtccttgcagttaactcaatccatttttgatatgtcgaaatggcgtgcgttaacgctgcaggaaaaagcagcagggattcaggacgtcacgtatcagaccgatcagcaaaccttgatcctcaacaccgcgaccgcttatttcaacgtgttgaatgctattgacgttctttcctatacacaggcacaaaaagaagcgatctaccgtcaattagatcaaaccacccaacgttttaacgtgggcctggtagcgatcaccgacgtgcagaacgcccgcgcacagtacgataccgtgctggcgaacgaagtgaccgcacgtaataaccttgataacgcggtagagcagctgcgccagatcaccggtaactactatccggaactggctgcgctgaatgtcgaaaactttaaaaccgacaaaccacagccggttaacgcgctgctgaaagaagccgaaaaacgcaacctgtcgctgttacaggcacgcttgagccaggacctggcgcgcgagcaaattcgccaggcgcaggatggtcacttaccgactctggatttaacggcttctaccgggatttctgacacctcttatagcggttcgaaaacccgtggtgccgctggtacccagtatgacgatagcaatatgggccagaacaaagttggcctgagcttctcgctgccgatttatcagggcggaatggttaactcgcaggtgaaacaggcacagtacaactttgtcggtgccagcgagcaactggaaagtgcccatcgtagcgtcgtgcagaccgtgcgttcctccttcaacaacattaatgcatctatcagtagcattaacgcctacaaacaagccgtagtttccgctcaaagctcattagacgcgatggaagcgggctactcggtcggtacgcgtaccattgttgatgtgttggatgcgaccaccacgttgtacaacgccaagcaagagctggcgaatgcgcgttataactacctgattaatcagctgaatattaagtcagctctgggtacgttgaacgagcaggatctgctggcactgaacaatgcgctgagcaaaccggtttccactaatccggaaaacgttgcaccgcaaacgccggaacagaatgctattgctgatggttatgcgcctgatagcccggcaccagtcgttcagcaaacatccgcacgcactaccaccagtaacggtcataaccctttccgtaactgatgacgacgacggggcttcggccccgtctgaacgtaaggcaacgtaaagatacgggttatctgccgcattcttcccccttctcgcttcaatttcgaccagccatcctctattctgatgggtatttaccactggtcccggaagacaaaaatgaaacggacaaaatccatacgccacgcatcgttccgcaaaaactggagcgcacgccatctgacaccagtcgctctcgcggttgccactgtttttatgctggctggctgtgaaaagagtgatgaaacagtgtctctctatcaaaatgctgacgactgttcagctgcaaacccaggcaaaagcgccgaatgtaccaccgcgtacaacaatgcgctgaaagaagccgaacgtactgcgccgaaatacgccacccgtgaagactgtgttgctgaatttggtgaaggtcagtgccagcaggcaccagcccaggctggcatggcaccagaaaaccaggcgcaggcccagcaatccagcgggagtttctggatgccgctgatggccggttacatgatggggcgtctgatgggcggcggcgcgggatttgcacagcagccgctgttctcctcgaaaaacccagccagtccggcttacggtaaatataccgacgcgacgggtaaaaactatggcgcagcccagccaggccgcaccatgaccgtaccgaagacggcaatggcaccaaaaccggcgaccaccactaccgttacccgtggcggttttggtgaatctgttgccaaacaaagcactatgcagcgtagtgcaaccggtacctcttctcgttcaatgggtggctgataccgatggaaagagtcagtattaccgagcgcccggactggcgtgagaaagcccacgaatacggtttcaattttcacaccatgtacggcgagccgtactggtgtgaagatgcttactacaagttgaccctcgcccaggttgaaaagctggaagaagtcaccgccgaactgcaccagatgtgcctgaaagtggtggaaaaagtgatcgccagcgatgagctgatgaccaaattccgcattccaaaacacacctggagttttgtgcgccagtcatggctgacgcaccagccatcgctttattcgcgtcttgatctggcgtgggatggcactggtgaacctaaacttctggaaaataacgccgatacgccaacgtcactatacgaggcggcgttctttcagtggatctggctggaagatcagcttaacgccggtaacttgccggagggcagcgaccagtttaacagtctgcaagaaaaactgatcgatcgcttcgttgagctgcgtgaacagtatggcttccagttgctgcatctcacctgctgtcgcgacacggtggaagatcgcggaaccattcagtatttgcaggactgcgcaacggaagctgaaattgctactgagttcctctacatcgatgatatcgggttaggtgaaaaaggtcagttcacggatttacaggatcaggtaatttccaacctgttcaaactgtatccgtgggaatttatgttgcgtgagatgttctcaaccaagctggaggatgcaggcgtacgctggctggaaccggcgtggaagagcattatctccaacaaggcacttctaccgctactgtgggagatgttcccgaatcacccgaacctgctgcccgcttattttgcggaagatgatcatccgcaaatggaaaaatatgtggttaaaccgatcttctcccgtgaaggcgcaaacgtgtcgatcattgagaacggcaaaaccattgaagcagcggaaggtccgtatggcgaagaagggatgattgttcagcaattccacccgttaccgaaattcggcgacagctatatgctgattggtagctggctggtgaacgatcaacccgccggaattggcattcgtgaagaccgtgcattgatcacccaggatatgtctcggttttatccacatatttttgttgaataagccacgataccggatggcactcgccatccggtaattgttagcctatctgcaccgacagcatactcaggctgcccatttctataccctcaaccggaatggtaattggctcctgcccatcccacgcacctaacacatacaacaacggcaaataatgctctggcgttgggttcgataacgtgccaccttcatggtcgaggtaattcaccagaggatgttgttccactggcccttgccacgtcagattcgctttcacatactcattaaacgacgtcgcccacggatacggtgaactatcaccgtgccacttcactgtgcgcaggttatgcaccacgttaccgctggcgaccaacattattccttcatctcgcagcgctgccagtttgcgccccatttcgaaatgccaggcggcaggtttgctactgtcgatactcaactgcaccatcgggatatcagcgtcaggatacatcttaatcagcacgccccacgagccgtggtcaaagccccaggcttctttatccagcgtcaccgggatcggcgctaacagctcaaccagacgctgtgccagcgcaggcgaacccggagcaggataatgcgtatcgtacagcgcctgcgggaagccaccaaagtcatgaatcgtgggcggcgtctccatcgcggtcactcctgttccacgggtaaaccagtgagccgaaaccaccacaatcgcttgcgggcgtggcaatgtcatccccaacttctgccagctgcgggtatacaaattatcttccagcacgttcatcggactaccgtgacctaaaaacaatgctggcatacgtgttgaagacatgatgatatccttaactaaaggtgtcattttgatatcctcacaatacgcttgttcggcggagtaagaacccggataacaatgatgatgatcatcagttattttgacgatctgcctgaaggtgaagatttataaggagttgtcgatgtcagtacctctcattctgaccatactggcgggggcagccacgtttattggcgcgtttctcggcgttctcgggcaaaaaccctcgaaccgcttactggcgttttcgctaggttttgcggcggggatcatgttgctcatctcattaatggaaatgcttcctgccgcactagcagctgaaggaatgtcgcctgtgttgggttatggaatgtttatcttcggtctgcttggctattttggcctggaccgcatgttgccacatgctcatccgcaggatttaatgcaaaaatcggtgcagccgttgccaaaatcgatcaagcgcacagccattctgctcactctcggcatcagtctgcataacttcccggaagggattgccacctttgtcacggcgagcagcaacctggagctgggatttggcatcgcactggccgtcgcgttgcacaatatccctgaaggtctggcagtggcaggcccggtttatgcggcaacggggtctaaacgcaccgcgattctgtgggcggggatttctggactagcagaaattcttggtggtgtgctggcgtggttaatcctcggtagcatgatttccccggtggtcatggcggcaatcatggcggcggttgcaggaattatggtggcgctctcggttgatgaattaatgccgctcgccaaagagattgaccctaataataaccccagctatggcgtactatgtggaatgtcagtgatgggattcagtttagtgctgctacaaacggcgggaattggttaaaaacaacatcagaagttgtccagcgcatggacaacttctgccagcttcacgaaagccttattctaccttttcggctgtctcttctctcgtactgtttaagtatttgttccgcgcttcaagcagtgcgtctctgtcctggcgaaacgcccgacaataacgtttcaaatgcaggaaataacccaccacaaccagagcaatcaatacaatccagtaccaggcgataaacatccttttacccttaatatttaacaatactaaacatttagcgtataaatttcacatatcctttttcggatatattcatatggtcgcataataacggaacaattatatgattttgatcataatgaaaaagaatgcctgatattaatgaaattttctcatagaaagagaagcggaattaacatcttgcatagcagggaaaaataaaaaccgaagcctgctacaacttcggtttcttgattaaggcagtaaattaagcagcggttttcagctggctttacgctcatgtgcctgacggtatgccaccaggtcttcaatagtcacgagcgccatattgtgtttattggcaaactcaatacactctggtgcacgcgccatcgtgccatcgtcattagtcagctcacacagtacaccagccggtttaaagcctgccagcgtcatcagatcaatagttgcttcagtatgaccgccacgcgtcagtacaccacctgcctgagcgcgaagtgggaaaacgtggccaggacgattcagatctgacggttttgcgccatcggcaatcgctgcgcgaacggtcgtaatacggtcagcggcagaaacaccggtagtcacaccttcagctgcttcaatggtcacggtaaaaccggtgccataggcgctggtgttattttctaccatcattggcagatcgagttgtttacggcgatcttcagtaatgcacaggcaaacaataccgctaccgtggcgaatggtcagcgccatctgctcaacagtcatggtttctgccgggaagatcatatcaccttcgttttcacggtcttcatcatcaagcaccattacaccgcgtccttcacgcagcgcagccagtgcattttcaacacgttcgaaaggcgtaccaaaagaggaaagtagcgtctgattcatggtaaaaaaacctcactaaaattatggttaccagaatcagggcagtcttaggagtggcggcatatagccaaaataacgtgagcgggtccatgcccgacagaatcgttactctctcccatccggactctaaccgtcggccccggaattacaccggatctgctgtcctttgagttcgcacccaaagcgctcgcgggctttcaactgagttgatttaccgccggtggggaatttcgccccgccctgagaataagcggattcactataacgctaatgattagcggcagcaacgcatagcttcacataattctggtttatgacttacccttatcgcactacaatggcactcaacacctatcagtacagggaaactacaatgattgacccgaaaaaaattgagcaaatcgctcgccaggttcacgaatcaatgcctaaaggaatcagggagttcggggaagatgtggagaaaaaaatccgccaaaccctacaagcgcagctgacgcgcctcgaccttgtaagccgtgaagagttcgacgtccaaacgcaagtcctgttacggactcgtgaaaaactggcgctgcttgaacaaagaatcagcgaactggaaaatcgcagtactgagatcaaaaagcagccagatccagagactctccccccaacgctgtaaacattcgtctttaatgcactgtaaattatgaattaatcctctaatttatagtgctttctattaccttatcgcgtaatcccattcagaaaaccatcacaaaaatgaatgagtacaattgaaagtataattgcaatgtattttttaagttttacttaatcgatatttagataaactaattttataaaaaacacaaaataaaatatcatatttcaatgattagtagtccttaaataacagttactaatcattctcttttctacttatctttatataaaggaatattatgtccgcttttaaaaagtcacttcttgttgctggcgtagcaatgattctttccaataacgtgtttgctgatgaaggtcacggtattgttaaatttaaaggtgaagttatctctgctccatgttctattaaaccaggtgacgaagatttaactgtaaatctgggtgaagtagcagataccgtactgaaaagcgatcagaaatctttggctgaacctttcactattcacctgcaggactgcatgctgagtcagggtggaactacttattcaaaagcgaaggttactttcactacagcaaataccatgacgggtcagtctgatcttctgaaaaataccaaagaaactgaaatcggcggcgccactggcgttggcgtacgtattctggacagccagagcggcgaagtaactttaggtactccggtagtaattacgttcaacaataccaacagctatcaggaactgaatttcaaagctcgtatggaatccccaagcaaagatgccaccccgggcaacgtttacgctcaggctgactacaagattgcttacgagtaatcgcatttggccgggttcgcccggccacatcattaacggattaatgataagtggatcagatgtataaaaaattaaaattaaccacaataagcgaattgattaaaaatatttattgttcattatccgttattagactggccccctgaatctccagacaaccaatatcacttaaataagtgatagtcttaatactagtttttagactagtcattggagaacagatgattgatgtcttagggccggagaaacgcagacggcgtaccacacaggaaaagatcgcaattgttcagcagagctttgaaccggggatgacggtctccctcgttgcccggcaacatggtgtagcagccagccagttatttctctggcgtaagcaataccaggaaggaagtcttactgctgtcgccgccggagaacaggttgttcctgcctctgaacttgctgccgccatgaagcagattaaagaactccagcgcctgctcggcaagaaaacgatggaaaatgaactcctcaaagaagccgttgaatatggacgggcaaaaaagtggatagcgcacgcgcccttattgcccggggatggggagtaagcttagtcagccgttgtctccgggtgtcgcgtgcgcagttgcacgtcattctcagacgaaccgatgactggatggatggccgccgcagtcgtcacactgatgatacggatgtgcttctccgtatacaccatgttatcggagagctgccaacgtatggttatcgtcgggtatgggcgctgcttcgcagacaggcagaacttgatggtatgcctgcgatcaatgccaaacgtgtttaccggatcatgcgccagaatgcgctgttgcttgagcgaaaacctgctgtaccgccatcgaaacgggcacatacaggcagagtggccgtgaaagaaagcaatcagcgatggtgctctgacgggttcgagttctgctgtgataacggagagagactgcgtgtcacgttcgcgctggactgctgtgatcgtgaggcactgcactgggcggtcactaccggcggcttcaacagtgaaacagtacaggacgtcatgctgggagcggtggaacgccgcttcggcaacgatcttccgtcgtctccagtggagtggctgacggataatggttcatgctaccgggctaatgaaacacgccagttcgcccggatgttgggacttgaaccgaagaacacggcggtgcggagtccggagagtaacggaatagcagagagcttcgtgaaaacgataaagcgtgactacatcagtatcatgcccaaaccagacgggttaacggcagcaaagaaccttgcagaggcgttcgagcattataacgaatggcatccgcatagtgcgctgggttatcgctcgccacgggaatatctgcggcagcgggcttgtaatgggttaagtgataacagatgtctggaaatataggggcaaatccagttatcatcattggttgtgcgtcagcttatgccgttgaattcaacaaagatttaatcgaagccgaagatcgtgaaaacgttaacctttcccaatttgaaactgatggccaattacccgtcggcaaatattcactaagcactctgattaataataagaggacgccaatccaccttgacctccaatgggtattaattgataaccaaactgcagtttgcgtgacaccagagcaattaacattattaggatttactgatgaatttattgaaaaaactcagcaaaacctgatcgatggttgttaccctatcgaaaaagaaaaacaaattacaacttatctcgataaagggaaaatgcaattatccatatctgcacctcaggcatggttaaaatacaaagatgcaaactggacgcctcctgaactttggaatcatggtattgctggggcatttcttgactacaatttatatgcctctcattatgcaccacatcagggcgataattcgcaaaatataagttcctatgggcaggctggggttaatcttggggcctggcgcctgcgtactgattaccagtacgatcagtcatttaacaatggcaaaagccaggcgaccaacctggattttccgcgtatttatttgtttcgcccaatcccagcaatgaatgcaaaactaactataggtcaatacgatactgaatcctctattttcgactctttccatttttctggcatttcgttgaaaagcgatgagaatatgttaccgccagacctacgtggttacgcaccgcaaatcacgggtgtcgcacaaacgaatgcaaaggtcactgtctcacagaacaaccgtattatttatcaagaaaatgttcctccaggcccatttgctattaccaatttattcaatacattacaggggcaacttgacgtcaaggttgaagaagaggacggacgcgttacgcaatggcaagttgcatctaatagtattccttatctgacgcgtaaagggcagattcgctacaccactgctatgggtaaaccgaccagcgttggtggtgattccttacaacaacccttcttctggactggtgaattctcatggggttggctgaacaatgtatccctgtatggtggttcagttttaacaaaccgtgattatcaatctctggctgccggcgttggttttaatcttaactcattaggttcattatcttttgatgtcacacgatctgatgctcagttgcataatcaggataaagaaacgggttatagctaccgcgctaactattcaaaacgttttgaatctaccggtagccagctcactttcgctggttaccgtttctctgataaaaactttgtgacaatgaatgaatatatcaatgacactaaccattacacgaattatcagaatgaaaaagagagttatattgtcacgtttaaccagtatcttgaatcattaaggttaaatacatacgtaagtttggctcgtaatacttactgggacgccagcagtaatgtgaattattcattatcacttagccgcgattttgatatcgggccattaaaaaacgtctccacttctctaacatttagccgaataaactgggaagaagacaaccaggatcaactgtacctaaatatttcgattccctggggaactagtagaacattgagctatggtatgcaacgaaatcaggataatgagatttcgcatactgcttcgtggtatgactcttccgatcgaaataattcctggagcgtttctgcttcaggcgacaatgatgaattcaaagatatgaaagcgtcactacgcgccagttatcagcataataccgagaacggtcgactctacctctccggtacatcacagcgagacagttattattctctgaatgccagttggaatggttcattcactgcgactcgccacggtgccgctttccacgactatagcggtagtgctgactcgcgttttatgatcgacgcagacggcactgaagatattccgttgaacaataaacgcgcggtaactaatcggtatggcatcggagttattccatcagtcagcagttacataacaacatcattaagtgttgatacccgaaatctgccagaaaatgtggatatcgaaaactcggttatcaccaccaccttaaccgagggtgctattggctacgccaaacttgatacccgcaagggctaccaaatcataggggttattcgcctggcagatggtagtcatccaccactggggattagcgtaaaagatgaaaccagccacaaagaattaggactggttgctgatggcggctttgtatacctcaacggcattcaggatgataacaaacttgctttacgctggggtgacaaatcttgttttattcaaccacccaatagcagcaacttaaccaccggaacggctattttaccgtgtattagccaaaattaattcaggatgaaactaatgcgctacttaaatacaaagaatatcattgcagcaggagtattactctcctgtatgagcagcattgcctggggtgccatcatcccggatcgtacccgtatcataatgaatgagtcagataaaggcgaagcattaaaacttactaatcaaagtaaaaacctgccctatctggcccaaacatggatagaagatacgaaaggcaataaatcgcgtgactttattgtcactgttcctccaatggtgcgtttaaatcccagtgagcaaattcaaataagaatgataactcaggaaaaaattgctcaacttcctaaagacagagaaacgctcttctattttaacgtgcgagaaataccgcccaaaacagataaaaaaaatgtgatgcaagtcactatgcagcacgcattgaaactattctggcggccaaaagccattgaattagaagacgatggggtaatgacttacgaaaaagttgaaatcattcgtagaaatgacggttcgatccgctttaacaataagatgccttatcacgttacgctgggttatatcggaacaaatggggtaacgatgttaccacaaacgcaaagcttaatggtaaccccttttagctatgcaaatacgcagtttaaaaatgttccgtcaacttttcaggtgggttatatcaatgactttggtggattaagtttttatgaaataaactgccctgtagtaaataacatttgtaatatttctgtagccaaccgagatcaataatatgcgctacttgttaattgttattactttttttatgggttttagttcattacctgcatgggcaatggactgctatgctgaacatgaaggtggaaataccgttgtcattggttacgtaccaagaatctctatccccagcgatggtaaaaaaggtgataaaatctggcaaagcagtgaatattttatgaatgttttctgtaataatgcactaccaggcccatctccaggagaagaatacccatctgcatgggcaaatataatgatgttgttagcatcaggtcaagacttttataatcaaaactcttatactttcggtgtaacttataatggggttgattatgattctacatctccactacctattgcagcacctgtatgtattgatataaagggagccggaaccttcgggaatggctacaaaaagcccgcagtctgtagtggcggtcctgaaccgcaattatcagtaacttttccagtacgagtgcagctatatattaagctagctaaaaatgccaataaagtaaataaaaaacttgtattacctgacgaatatatagcacttgaatttaaaggtatgagcggagcaggtgctatagaagtagataaaaatctgaccttcaggattcgcggattaaataacattcatgtccttgactgctttgttaatgttgatctggaaccagctgatggcgttgtcgactttggtaaaataaattcccgaacaattaaaaataccagcgtgagtgagacgtttagcgtagtcatgaccaaagatccgggtgcggcctgtactgagcagtttaatattttagggagttttttcactacggatattttgagtgattatagccatctggatataggtaatggtctgctattgaagatatttcataacgatggaacagcaacggaatttaaccgcttctcacaatttgcttctttttcatcgtctagtgcgccttcggtcaccgcaccattcagggcagaactgagtgcgaacccggcagaaacggttgttgagggaccgtttagtaaagacgtaatcctgaaaatcacctataactagtatctaatacaaacactaaaacgggccatcaggcccgttatatcagtgctctaactccagctctcttgcctgcatcatctgttgacaataccaggcataacgtgcgcaaaaccaggttctatgttcttcatccatgttaccagtaacggccagaatatcgaccgggcgaccttctgcgtgcattctggcaaaactacgcgccaggaaatcgaaattatttaaagaattaagactatgatccataagcacatcctccggttatcgcataccttttaaggccatatgctttttctgatttcagtattccccaatcagtgtagtgcctttaaacataacgtgcgtaaatatattgtccccgatcacactttttagtgaaaaataaaaaaccatattaaaagactttctcttccagaacttctctaacctgtgttattattaacacagataaatgtaagcaaggaaactattacaaagtaaatattgcgtcactaaatggacattggagtgatatatgattttattcgccgactataacaccccttatcttttcgctatttcctttgtactgttgatcggcctgttagaaatttttgcgcttatctgcggtcacatgctctccggtgctcttgatgcacatcttgaccattatgattctataaccacaggtcatattagccaggcacttcattatctcaatattggaagattgccagctctcgtcgttctctgcttactggctggtttttttggtcttattggcatcctgttgcagcatgcctgcatcatggtctggcaatcaccactgtcgaacctgttcgtggttcctgtcagtttactgtttacgattattgcggtgcattataccggtaaaatagttgcgccctggattccacgcgaccatagttcagctattacagaagaagaatatattggtagcatggcgttaattaccggtcatcaagccacttcaggtaatccctgcgaaggaaaactcaccgatcaatttggccaaatacattatttactactggagcctgaagaaggaaaaattttcactaaaggagacaaagtgttaattatttgccgactttctgcaacgcgatatttggcggaaaataatccctggccccaaatattgtaatttattaatcaaaaggaaatttaataatggatgatattgttaattctgtgccctcctggatgtttaccgcaattattgccgtatgcattctgtttattattggaattattttcgccaggctctatcgtcgcgcttcggcagagcaagcttttgttcgtactggtttaggtgggcaaaaagtggtaatgagcggtggcgcaatcgtgatgccgatctttcatgaaataatccccatcaatatgaatactctgaagctggaagtcagccgctcaaccattgatagcctgattacgaaagatcgtatgcgcgtcgatgtagtagtcgctttctttgtgcgggtaaaaccttcagtagaagggattgccaccgctgcccagacgctggggcaacgcaccctgtcgcctgaagacttacgtatgttggttgaagataaatttgtcgatgccctccgtgcaacagctgcgcaaatgaccatgcatgagttacaggatacccgcgagaactttgtgcagggggtgcaaaatacagtggcagaagacctgtcgaaaaacggtctggaactggagagcgtttcacttaccaactttaaccagacctcgaaagaacatttcaatccgaacaatgcctttgacgccgaaggtttaaccaaactgactcaggaaacagagcgccgtcgccgcgaacgtaacgaagttgaacaggatgtagaagttgcggtgcgtgaaaaaaatcgcgatgcgctatcgcgcaagctggagattgaacagcaagaagcgtttatgacgcttgagcaggagcagcaggttaaaacccgtactgccgaacagaatgcacgtattgcggcttttgaagctgaacgtcgtcgtgaagcagagcagacacgaattctggctgaacgacagattcaggaaacagaaatcgaccgcgaacaggccgtccgctcaagaaaggttgaagctgaacgtgaagttcgcattaaagagatcgaacagcagcaggtcaccgaaatcgctaaccagacgaaatcgatcgctattgccgccaaatcggaacaacagtcccaggcagaagcgcgtgctaatctcgcacttgcagaagcggtaagcgcccaacaaaacgtagaaaccactcgccagactgccgaagccgatcgtgctaaacaagttgccctaatcgctgccgcgcaggatgcagaaaccaaagcggttgaactgaccgtgcgggcgaaagcagaaaaagaagccgcagagatgcaggcggcggctatcgttgagttagccgaagctacacgtaaaaagggtctggcggaagcagaagcacaacgtgcgctgaacgatgctatcaacgtactttctgatgaacaaaccagccttaaattcaaactggccttgttgcaggcgctgcctgcggtaatagagaaatccgttgagccgatgaagtcaatcgacggtatcaagattattcaggtcgatggtctgaatcgtggcggcgctgcgggtgatgcaaacacgggtaatgtggggggcggaaacctggcggaacaagcattatcagccgctctctcttaccgcacacaggcaccgctgattgactccttgctcaatgaaattggcgtttcaggcggctcactggcggcattgacttcacccttaacctcaacaactcccgtcgaagaaaaagcagagtaaaccctcttccaggaataatccctggcccaaaaagccggggattttttatatctgcgttccgctaaaaagtgcaaatgatcaggttgttgcagcattttgcgtgacggctcggggaaggcaaaactgcatcagagaaagcattgcgtggggtctggcgctcatcaacaatcggggagtcagcagggggctgaaacgggaaagcccctcccgaagaagggggccttacagaaggaaagggttatgatgaagctcgtcatcatactgattgtgttgttactcgtaagtttcgcagcttattaacagccaatcagaggggggagaaatcctccctcacccttgttcctttactttaggttgaaaaaaaatcagcgtcaagaaggtttcattaacacatatccctggcccaaaaagccggggattttttatatctgcgttccgctaaaaggtgcaaatgctcaggacgttgcagcgttttgcgtgaccgctcggggaaggcaaaattgcctctgggaaagcattgcgcggggtccggcgctcatcaacaatcggggggcagcaaggggctgaaacgggaaagcccctcccgaagaaggggccttgtataaggaaagggttatgatgaagctcgtcatcatactggttgtgttgttactgttaagtttcccgacttactaacaactcatcagaggggggagaaatcctcccttacccttgttcctttactctaggttgaaaaaacaacagcgtcaataggcctgccatgtacgaagcgagatctgtgaaccgctttccggttagccttttttatcctgttggatcttcttgatgatgttggtcgtcgagcaaccgtcttcaaagttgagcaccaacacttcgccaccgttggcccagacttctttactcccggcaatctcttctggtttatagtcgccgcctttcaccagcagatctggcaagatcccggcgatcaagcgctgcggcgtgtcctcttcaaacgacactacccagtcgaccgcttccagtgcgcccagcacaatcatacgctgttcgagtgggtttaccgggcgggaatcccctttcagccgtttggtggaggcatcgctgttgacggcaacaatcaagcggtcacccagcttgcgggcatttgccagataagagacgtgcccggcgtgcaggatgtcaaagacaccgttggtcatcaccactttttcaccacgtttacgcgctgccgctacggccagcttcagttcctcttcggtcatcacgccaaagcctgtatctgcacgtccacgtacagcattttccagctcgatcggcgaaaccgtggaggttcccagtttgccgaccaccacgccagccgccgcattggcaaagaagcaggcttcttccagcgaattacccgctgccagcgttgccgccaggacgccaatcaccgtgtcgcccgcaccggtaacgtcatacacttcctgcgcttgggttggcatatgcagcggcgctttacccggttgcagcagcgacataccctgttcggaacgggtcactaacagagccgagagttcgtaatcggcaatcagtttcatgccgcgctcaacaatctcttcttcggtcttacatttaccgacaacagcttcaaattccgagagattcggcgttaacagcgtagcgccgcggtagcgctcaaaatcggtaccttttggatcaatcagcaccggaacacccgctttacgcgccagttggatcatctgctgtacgcttgccagcgcacctttggcgtagtcagaaagcaccagcgcgccaatcgaactcagcgcctgattaatccgctcgtgcagcggctgcggatcaacaccttcgaaaccttcttcaaaatccagacggatcagctgttggttgcgggaaagtacccgtaatttggtaatggtcggatgcgtcggtacagaaacgaagtcgcatttgacgttgacgtcggccagagatttactcagcgcgcgcgctgcatcgtcaatgcccgtcaacccgaccaggcgtgcattagcaccgagagaagcgatattcatcgccacgttagccgcgccgcccggacgttcttcgatggtattcactttaaccacgggcaccggcgcttccggcgagatacgactggtggggccgtaccagtaacgatccagcatcacatcaccaaccaccatcactcctgcacgttcaaactctggcagcgttactttcattcctgtctcctgagagattcaaaatttgcgcgcgataataccatacttcattcttccaccagccacttctgccagcttgcccgcaccagttcacgctctgcggtgaagcaatcctccgacacatggcccggcaattcctgtaatgccagatgatgaagttcatcgcgaagcgtagtgtaagcacgggtcagcgccatcgcttcctgctcttccataatgtcgttttgcgccagtagttccagaatacgcacgttgtctgaccagcgcgttaacttcggtttttcatgagcgtagcgcaacaccagatattgggtaataaattcgatatcggtaattcccccttcatcagctttgatatcaaagcgatcgcgatgtttattgccgagatgagcgcgcattttctcgcgcatttcccgcacttccgtttgcagagttttaccttcacgcggcagcgtcataatctcgcgacgcactgcgtcaaagtgcgcggtgagctgcggatcgccgtacactacacgcgcacgcaccagcgcctgatgttcccacgtccaggcctcgtttttctgataatcggcaaatgcttctgcggatgtcaccagcattcccgccgccccggacggacgcagtcgagcatccacttcatacaaaatgccggaagaggtacgcgtactgaacagatgcataatgcgttgcgccagacgcagataaaactgccgcccgtcgatttcccgctcaccgtcagtcatcgcatccattgggcaatcatggaggaagataaggtcaagatcggaactgtagcctaactcccagccgcccagcttgccgtagccgaccaccgcaaaaccacgcccttcgcgttcgttcaggtgattcggcttaccgtagcgggcaaccatttgaacccacgcctgctgaacgacggcatctatcatggcttccgccagccaggttaagtgatcgctcactttcatcaccggtagcgtaccggcgatatccgctgcggcgatgcgtaacagctgcgcctgtttgaactgacgcagcgcctcaagctgttgctcttcgtcatcttccggcacgcgcagcaaatactggcgcaactcatcgcggtaggcatcggtcgccgtcggctggtaaagggtgtttggatcgagcaattcatccagcaataatggataacgcgccagctggctggcaatcatcggcgacgcggcacacagagaaatcaaatgtttaagcgccgcggggaattcactgagcaattctaaataggtggtgcgggtaacaatccccaccagcaaggcggtaatgcgcgacagcgtaacggcagcgtcttcacgcgcacagacatcacttagcagatgcggcatcagatggtcgagcacctgacgtcctcgcggcccgatggtgcgcttatccagctctttgcggaaatcggcaatcagcgttagcacctgtttgcgatcatcctcgctaagatgcgccagcactggcgtagtgtcatcttcctgcaacgcatcctgccacagctcacgccactgttccgacagcgactcttcctgagtttcactttcatcgtcgccaatcaattcattaaacacccggcgcacattggtcatatgtgcggtcagcgccccggtcagttgcggccagtcagcaaagtccatcgcccacgccagccgcgcacgattaagctcatcagaaggaagcgtctgggtttgttcgtcgttaatgctttgcagcaggttttccagacgccgcaggaacagatacgccactcgcaattgttcagcatcgttttcagaaagcagatgcagctcggcaatggcgctgagcgttggcagtaaagagcgcgattgcagcgacggttcgcgtccgccgcgaatgagctggaacacctgaacgataaattcaatttcgcgaatgccgcctgcgccgagtttgatattgtcggtcaaaccacgtcgacgcacttcacgggcaatcatccctttcatgttgcgcagcgactgaatcacgctgaaatcgatgtaacgacggaaaacaaacgggcgcagcatcgcacgcaactcgttagcatagacgccttcgctatcgcccataatccgcgccttgaccatcgcgtaacgctcccagtcgcgcccctgctcctggtaataatcttccaacgcggcaaagctcagcaccagcgggccactttcgccaaacggacgcagccgcatatccacgcgatagacgaagccatcctgcgttggttgatccagcactttaatcagccgctgccccatgcgggtaaaaaactgcgcgttatccagttcccggcgtccaccctgcgtacaaccatgttccggccaggcaaaaatcagatcgatatcagaggagaaattcagctccccaccgcccagcttacccatgcctaaaatcagcagcggttgcgcttcgccctgcgcattgcacggcgttccccactcgcggcagcaggcgtcatacagccagtcacgcgccgcaacaatcagcgtctccgccagatagctgagctgctgcaatatgctctcttcagtaaccagtgccagcgtttgcgcccaggcgatgcgcaccataatgcgccgccggaatagccgcagctcgcgcattaacccggcttcgtcactcacattacagagcgcctcctgcaaccatgccgcgtaatgctgccattcgtcggcctgcggcggttggctttccagttccgtcagccactctggatgcgcaatcacgctgtcctgcacaaaatcactaaaagtaagtactgacttcgcctgtgcgctaagtgattcctcggctaaaggctctggcagccgctcaacaacggtctgccagtactgctgtaacggtgaagagagcggcttcataagcgattttatccttgcctgattaacgttttccgctgtgcaaccagaacggttcctgattgtttgcctcattacggaaatgttcaatttcgatgcgttgcccggtcgcaatagcgtgatgcagcccctgccagttctccagccaggcttgcgcgacgacaggatcatagtaacccgccagcaacagtattgagtcaatatcacgcgtcaggcgtggcaactggtcacggtagcgatcgcctaacggctggcagaaaacgcttttcagttcagcggcatggcgggaaagatggatatcggcaaagcgtttgaaggagtcgctgattttgccctgcgctttggcatctaaaaatggctgccatgctttgcttaccaaccattcggtcaacgccagcttcgccattgccgtttcggtagagtagaccgccgtcacggcagacaccgcagaagcaatggtcgcctcgcattgagtcagcagatcacgtaagtgagtgctcgctttacgcggcacaataccaccgaacagcatcagcgtatgacggaccaggctaatggctgccagcacctgttctttcgccgcatcgttgccgcgtacccacagttcttcatgatactgccattgcgctaacgccagctcgagcgccgcttccagcccctgttccacatcggcttttgccgcaacatgcaaaatggtggtcggtttgatttcacgcgccggattgccctgcgccagatgatagccacgcgccgctttgctcaggctgccctggcgtaatccggtttgcgataccagttggttcgccagtttcagcaccgcgcgcgtgtcgccgctaagcagttccagttccagctcacagataggttcagcaaattcacccgctttcacttccccctggtcgagggcgatttcaatttggctaccatcgaccgccaccagccatttttcgcgataaaaatcggtgctgaacagcggctgcacgcgggaggcgagatcggcgggcaattcgccgttcggccagacttccgtcggtaactgcgccaggtcgagcgtcggttcgctcaacgccacgttatattccgggcgctgatgtaagccgcctgtcactcttcctgcaactttcatggtcatctcatagcgaccgttttcgccacgaatacgtaagcccatatcgtgcccacgcagccagttatccggcgtttcgtagtaaatattcagcaactgcacggggtcatggtgctcgccgcccagcgtattgagatggtcacgcaacgcctcaacggcactgtgattaacaataaactttaattcgatttcctgagccatggcctttacttatcggttatgtcacataagtgacgatgaacggcgaacttaatgcgatcttttttgtcagtagatagtattttgcgccaaattgccatgcaacgggcaatttgacgggcgtaaaagtttgaagcagtggcaagacctgacacagaggattccgattgatgtcgaatgctttgcgtagcgacactgatgccactactatcgttccactttccatgacaataacgacagcctgatgccaaaattacgcctgatcggattaactttactcgcacttagcgcgactgccgtctcacacgctgaagaaacgcgctatgtttccgacgaactgaatacctgggtccgcagcggtccgggagatcattatcgcctcgtgggcacggttaacgccggcgaggaagtgaccttattacaaactgacgccaacaccaattatgcccaggtgaaagacagctctggccgtaccgcctggatcccgttgaaacaacttagcactgagccaagcctgcgctcccgtgtgccagatctggaaaatcaggtcaaaaccctgaccgataaactcaccaatatcgataacacctggaatcagcgcaccgcagaaatgcagcaaaaagtggcgcagagcgacagcgtgatcaacgggttaaaagaagaaaatcagaaactgaaaaacgagctgattgtcgcgcagaaaaaggtcgatgccgccagcgtacagctggatgacaaacagcgcaccatcatcatgcaatggtttatgtatggcggtggcgtgctggggcttggcttgctgctcggtctggtactgccgcacctgatcccaagccgcaaacgcaaagatcgctggatgaactaaatcgccttcttcgttgcactgtcttattattaggaattgtgtatttgacgaagggatgatggcgtgaagatttatctggtcggtggtgctgttcgggatgcattgttagggctaccggtcaaagacagagattgggtggtggtcggcagtacgccacaggagatgctcgacgcgggctaccagcaggtaggccgcgattttcctgtgtttctgcatccgcaaacgcatgaagagtatgcgctggcacgtaccgaacggaaatccggttccggttacaccggttttacttgctatgccgcaccggatgtcacgctggaagatgatcttaagcgtcgcgatctgaccattaatgcgctggcccaggacgataacggcgagattatcgacccgtacaacggtctgggcgatctgcaaaatcgtctgttgcgccatgtttcccccgcttttggcgaagatccgttacgcgtattgcgcgtggcgcgttttgctgcgcgttatgcccacctcggttttcgtattgccgatgaaactctggcgttgatgcgcgagatgacccatgcgggtgaactggaacacctgacgcctgaacgggtatggaaagagacggaaagcgccctcaccacccgcaatccacaggtgttcttccaggtactgcgcgattgcggcgcactgcgcgttttattcccggaaattgacgcactgtttggcgttccggcccctgccaagtggcatccggaaatcgatacgggtattcataccttaatgacgctctcaatggcggcgatgctgagtccgcaggtcgatgtccgtttcgcaactttatgccacgatctcggtaaagggctgacgccgccagaactctggccgcgtcatcatggtcatggcccggcgggtgttaagttagtggaacaactatgccagcgtctgcgcgtgccaaatgaaattcgcgatttagccagactggtggctgagtttcacgatctcatccacaccttcccaatgctgaacccaaaaaccatcgtcaaattatttgattccatcgatgcctggcgtaaaccgcagcgtgtcgagcaactggcgctgaccagcgaggctgacgtgcgcggcagaaccggttttgaatcagcggactacccgcaaggccgctggttgcgcgaagcctgggaagtggcgcagtcagtgccgacaaaagccgtcgttgaagcgggatttaaaggtgtggagattcgcgaggagctgacccgacggcggattgcggcggtagccagctggaaggaacaacgttgcccaaagcctgaatgagtattgggcattttgccggatgcggcgtaaacgccttatccggctacatgtcaacgacagttgtaggcctgataagacgcgcaagcgtcgcatcaggcgttgattgccggatgcggcgtgaacgccttattcggcctacgcaatcgttgacaacgccaagcatccgacactattcctcaattaaaagaacacgacatacaccgcagccgccacaataaagcgataaatggcgaacgggataaacgaaatgcgcttaatcaattgcaggaaggttttaatcgctatcagcgccaccacaaaagcggtgataaacccaacggcaaacatcgggatatcgccgcttgtcaggaagccccagcttttgtagagatcgagcgccgttgcgcccatcatcatcggcaccgccagcaggaacgaaaactcggaagcagcgtaacggctcacccccatcagcatcccacctgaaatggtcgccccggaacgggagaaacccggccacagcgccagacactggaaacagccaatcataaatgcctgacgataggtcatatcatcaagacccggcgcacgcggctctttcggcttcaggcattcggcggcaatcagcaacaaaccgccaacgaccagcgcatacatcacatttatcgggttaaacaatgacttaatcgtgtcgtggaacaacagccccaataccaccgccggaatcatccccagcaaaatgtggatcagcgttaaacgacctttgctttcaccttcgtgctgcaacgggcggccaaagtggatgccaatcaggccaaacagacgccgccagaacatcactactaccgccagaattgatcctaactggatcacaacttcaaaggttttcgccgtgtcgccctcaaaccccaacaagtgaccgacaataatcatatggcccgtgctggataccggcagaaattctgtcaatccttcgaccacacccaatattgccgctatcagcagcgagtgcatatcgctcatcaataaacccctaaattattaaaatgtaccgcttgtccgaactactgcgtatgaccaggttataaccgtttggtttaacagctgtaaaattaattattttctttcagattattgccacgctcaatgattacgccaacattcgccgcccgcgccactgcgcctggcttgctgagtttgatacgcacccacggcgagttgaagcgtgctaacagcagctccgccacctcttcagccacgcgttccaccagcgcaaaacgcgccccctcgacgtggctgaccaccgtttctgcaatgtcagcgtaactgaggcaatccgccacatcatcacttttcgccgctttacggttatcccacgccatttcgatatcgaacactaacttctgttcgatggtctgttcccagtcgtaaacaccaatagtggtgattaccgaaagttgctctataaatacaatatccatcacgtcctgcctgctttttggctaaccggataccacttccggcgaaatgtgcgtattatccacagattcatcgttgaacacgaattttcaaaacggaacagcttatgagtgcaatcgcgcctggaatgatcctcatcgcgtacctctgcggctccatttccagtgccattctggtttgccgcttgtgtgggctgcccgatccgcgaaccagcggctccggcaatccaggcgcaaccaatgtgttacgtatcggtggcaagggagcagccgtagcagtactgattttcgacgttctgaaaggaatgttgcccgtctggggcgcgtatgaattaggtgtcagccccttctggctaggcttaattgccatcgccgcctgtcttggacacatctggcccgttttcttcggatttaaaggaggaaaaggcgttgctaccgcttttggtgccatcgcacccattggctgggatctcaccggagtaatggcgggaacctggttactgaccgtgctattgagcggatactcgtcgctgggagcgattgtcagtgcactgattgctccgttttatgtctggtggtttaagccacaattcaccttcccggtttcgatgctctcttgcctgatcctgctgcgtcatcatgacaacatccaacgtctgtggcgtcgtcaggagacaaaaatctggacgaaattcaaaagaaagcgcgaaaaggatcccgagtgatttctggtggatctacatgacctgatagccttcatcgggcttgcccagccgttgctggcaccatgccgccagaaattccacgcagacacgtaatttcatgctgcgatagagcggctcccggtaaacagcccagatattggcgctttgtgcatactctggcaatacttgcaccagtttgccactctccagaaacggcaacacatcccactcggaacgcagcataatccctttgccctccagcgcccattgcagcacaatctcgccgctattggaggaaagatgcccgcttaccttcaccgattttttctcctgaccgttccccaactcccatattccatgggtcatatcgcgctctttggtcaccagacagtcatgacgacttaattcctgtagggattgtggctgcggatatttttgcagatactcaggtgctgcgcataatattcttttattttttgtcaaaagatgcgcaatataataatcaggaatttcgtcattaatacgaatatccagatcaatattatcctgcactaaatcaatttgccgatcgaacaattcaaaatgcacctgtaactcaggataattgcgcatcagttcggtaatagctggcgcaatatggctgcgcccaaaaccaaaactgcaaccaatacgaatcatcccctccgggcgcgttttgatttgcgtgacgtcatcgaccagtcgctgatattgggtgaggatttccaacgcatgttcgtaacaacgttggccactttcagtcagcgccacgccgcgagcggagcggttcagcagcgttgttgccagcgtattttcaaggatttggatccgcttggtgacaaatgcaggcgtctgcccaagcgtcgccgctgcggcgctaaaactcccgctgtgaacgatttctaccagtacctgcaagtctttggctaaaggccagctattcagcatcgttaattatccgcagttgtgataagcgcagtgtatttcgcaaaacattgccattccctgctctggcgcaatattcattcttattttcgcgttgattcacgaactgttaattacatattcacggtggcaaaaaatataaaaccacatttttagtggtagtttgtggcggtgaatttttccagacaaatacaaaaactggagttgccatgatgagcgaaagtaataagcaacaggcagtgaataagttgacagagattgtcgctaactttaccgccatgatttctacccgaatgcctgatgacgtggtggataaactaaaacagctaaaggatgccgaaacgtcgtcgatggggaaaattatctaccatacgatgttcgacaacatgcaaaaagcgattgacctgaatcgtcctgcctgtcaggacaccggggagattatgttcttcgttaaagtcggttcccgcttcccactgcttggcgagctgcaaagcatactcaaacaagccgtggaagaggcaaccgtcaaagcgccactacgtcacaatgcggtagaaatttttgacgaagtaaacaccggcaaaaataccggtagcggcgtaccgtgggtcacctgggacatcatccccgacaatgacgatgcggaaatcgaagtttacatggcaggcggcggctgcacgctacctggccgctcgaaagtgttaatgccgtcagaaggctacgaaggcgtggtgaaattcgtcttcgaaaatatctccaccctcgccgtaaacgcctgtccaccggtactggtgggcgtgggcatcgccacctcggtggaaaccgccgccgtactctcgcgtaaagccattttgcgcccgattggcagccgccatcccaatccaaaagcggcagaactggagctacgcctggaagaaggactcaaccgtctggggattggtccacaagggctgaccggcaacagttcagtgatgggcgtacatatcgaatctgccgcccgccatccgtcaaccatcggcgttgctgtctctaccggctgctgggcgcatcgtcgcggcacgctgctggttcatgccgatctcacctttgaaaatctgtctcacacccggagcgcgttatgaaaaagatcctgacaaccccgatcaaagctgaagatctgcaagatattcgcgtcggcgatgtgatctacctgaccggtacgctggtgacctgccgcgacgtttgtcaccgccgtttgatcgaactgaaacgtccgatcccttacgatctcaacggcaaagcgattttccacgctggccccatcgtgcgcaaaaacggcgacaaatgggagatggtctccgtcggcccgacaaccagtatgcgtatggaaagttttgaacgtgaatttattgagcagaccggcgtgaaactggtggttggcaaaggtggtatggggccgctgaccgaagaaggctgccagaaattcaaggcgctacatgtgattttcccggcaggctgcgcggtgctggcggcaacccaggtggaagagattgaagaagtgcactggacagagctcggaatgccggagtcactgtgggtctgccgggtcaaagagttcggcccgctgattgtctctattgatacccacggcaacaacctgatagccgaaaacaaaaagctgttcgccgaacgccgcgatcccatcgtggaagagatctgcgagcacgtccattacatcaaataaccctcccggagaggctcacccctctcctttttcgcaggcataacacgatgaaaccttccactgaatggtggcgatatcttgcgccgctggcggtcatcgccattattgctctacttccggttcccgcagggctggagaaccatacctggctctactttgccgtttttactggcgtgatcgttggactgatcctcgaacccgtgccgggtgccgtggtggcgatggtgggtatatccatcatcgccatactctctccctggctgctgttcagcccggagcagctcgctcagccaggctttaaattcactgcaaaatccctctcgtgggccgtttccggtttttctaattcggttatctggctgattttcgccgcctttatgtttggcacaggctatgaaaaaaccgggcttggacgccgcattgcgctgattctggtgaaaaagatgggacatcgcacgctgtttctcggctatgcggtgatgttctccgagctgatcctcgcacctgtaacaccgtccaactcggcgcgtggtgcggggattatctatcccatcatccgtaacctgccaccgctctatcaatcacaaccaaacgacagcagttcgcgcagcattggctcgtacatcatgtggatggggattgttgccgactgcgtgaccagcgccattttcttgacggcgatggcaccaaacttgctgttaattggactgatgaaaagcgcatctcacgccacgctgagttggggcgactggttcctcgggatgttgccgctcagcattttactggttctgctggttccctggctggcttacgtgctgtacccgccggtactgaagtctggcgatcaggtgccgcgctgggcagagacggaactgcaggcaatgggcccgctctgttcgcgtgaaaaacggatgctggggctgatggtaggcgcgctggtgctgtggattttcggcggtgattatatcgatgccgcgatggtcggttacagcgtggtggcactgatgctgcttctgcgcattatcagttgggacgacattgtcagtaataaagcggcgtggaacgttttcttctggctggcctcgcttatcaccctcgccaccggactcaacaacaccggttttattagctggtttggcaaactgttagcaggcagcttaagcggttattcgccaacgatggtgatggtggcgttgattgtggtgttttatctactgcgctactttttcgccagcgccacggcgtatacctccgctctcgcaccgatgatgattgctgctgcgctggcgatgccggaaatcccgctgccggtgttctgcctgatggttggtgcggcaattggtctggggagcattcttacaccatacgccaccggccccagtccgatttactacggcagtggttatctgccaacggcggattactggcgactgggggcgatttttgggctgatattcctcgtattgctggtgattaccggcttactgtggatgcccgtggtgttgctttaagtgaggacggtgccggaaattgctctccggcacccaatagttttacgcagccggtaactccgccagcggccagcgcggacgcacgctaacgccgagatccgccgtcgcgcctgctttaaaccgcaccattccggcataggcgatcatcgcgccgttatcagtacaaaattccggacgcgcgtagaacacttcgccgcggcgttttttcatcatttcagccagcttcgcccgtaacgtacggttagcactcacgccgcccgccatgaccagtcgcttaaagcccgtctgatccagcgcccgcttgcacttaatcatcagcgtatcgaccaccgcatcttcaaaggcgcgggcgatatcagcacgcgtctggtcgtcggtgccgttgtcacgaatggtatttgccgcgaaggttttcaggccggagaagctgaaatccagccccggacggtcggtcatcggacgcgggaagacaaagcgcccggcagtaccctgagccgccattttcgacagtaacggcccgccaggataatccagccccagcagcttcgcggttttatcaaacgcttccccggcggcatcatcgatagactcgccgagcagctcgtactgaccaatgccagtcacgctgattaactgcgtatgaccgccggaaacaagcagcgcaacaaacggaaattccggcgggttatcttccagcatcggcgctaacagatgcccttccatatggtgtacagggatcgccggaacgtcccaggcaaacgccagagaacgccccacggtcgcgccaaccagtagcgcgccgactaatccagggcctgcggtataggccacagcatcaatgtcttttgccgttaaaccagactcctttagcgccgcctggatcaacggtacggttttacgcacatgatcgcgggaggccagttcaggcacgacgccgccgtagtcagcgtgcaatttcacctgactatacaattggttggctaacaaacctttttcatcgtcgtaaatggcgatgccggtttcatcgcaggaagtttcaatacccagtacacgcatgacttgttttacctcgctttattaccgcgcagtgtaggaccaatgcgggttgatgtaaaactttgttcgcccctggagaaagcctcgtgtatactcctcacccttataaaagtccctttcaaaaaaggccgcggtgctttacaaagcagcagcaattgcagtaaaattccgcaccattttgaaataagctggcgttgatgccagcggcaaaccgaattaatcaaaggtgagaggcacatgccggtaattaaagtacgtgaaaacgagccgttcgacgtagctctgcgtcgcttcaagcgttcctgcgaaaaagcaggtgttctggcggaagttcgtcgtcgtgagttctatgaaaaaccgactaccgaacgtaagcgcgctaaagcttctgcagtgaaacgtcacgcgaagaaactggctcgcgaaaacgcacgccgcactcgtctgtactaattccccgagagcgttgctctccgatcagaccgagttgtagttgtaaggccgtgcttccgaaaggaatgcgcggcttattttcgtttatgaattgctaaaaatcggggcctatggctggacgaatcccacgcgtattcattaatgatctgctggcacgcactgacatcgtcgatctgatcgatgcccgtgtgaagctgaaaaagcagggcaagaatttccacgcgtgttgtccattccacaacgagaaaaccccgtccttcaccgttaacggtgagaaacagttttaccactgctttggatgtggcgcgcacggcaacgcgatcgacttcctgatgaactacgacaagctcgagttcgtcgaaacggtcgaagagctggcagcaatgcacaatcttgaagtgccatttgaagcaggcagcggccccagccagatcgagcgccatcagaggcaaacgctttatcagttgatggacggtctgaatacgttttaccaacaatctttacaacaacctgttgccacgtctgcgcgccagtatctggaaaaacgcggattaagccacgaggttatcgctcgctttgcgattggttttgcgccccccggctgggacaacgtcctgaagcggtttggcggcaatccagaaaatcgccagtcattgattgatgcggggatgttggtcactaacgatcagggacgcagttacgatcgtttccgcgagcgggtgatgttccccattcgcgataaacgcggtcgggtgattggttttggcgggcgcgtgctgggcaacgatacccccaaatacctgaactcgccggaaacagacattttccataaaggccgccagctttacggtctttatgaagcgcagcaggataacgctgaacccaatcgtctgcttgtggtcgaaggctatatggacgtggtggcgctggcgcaatacggcattaattacgccgttgcgtcgttaggtacgtcaaccaccgccgatcacatacaactgttgttccgcgcgaccaacaatgtcatttgctgttatgacggcgaccgtgcaggccgcgatgccgcctggcgagcgctggaaacggcgctgccttacatgacagacggccgtcagctacgctttatgtttttgcctgatggcgaagaccctgacacgctagtacgaaaagaaggtaaagaagcgtttgaagcgcggatggagcaggcgatgccactctccgcatttctgtttaacagtctgatgccgcaagttgatctgagtacccctgacgggcgcgcacgtttgagtacgctggcactaccattgatatcgcaagtgccgggcgaaacgctgcgaatatatcttcgtcaggaattaggcaacaaattaggcatacttgatgacagccagcttgaacgattaatgccaaaagcggcagagagcggcgtttctcgccctgttccgcagctaaaacgcacgaccatgcgtatacttatagggttgctggtgcaaaatccagaattagcgacgttggtcccgccgcttgagaatctggatgaaaataagctccctggacttggcttattcagagaactggtcaacacttgtctctcccagccaggtctgaccaccgggcaacttttagagcactatcgtggtacaaataatgctgccacccttgaaaaactgtcgatgtgggacgatatagcagataagaatattgctgagcaaaccttcaccgactcactcaaccatatgtttgattcgctgcttgaactgcgccaggaagagttaatcgctcgtgagcgcacgcatggtttaagcaacgaagaacgcctggagctctggacattaaaccaggagctggcgaaaaagtgatttaacggcttaagtgccgaagagcgatcgggaagcccccgacagccgcactgagaggcagcggcaaatatataagtacgccctcgtaattatcgttggcggtaaacaaccgttggatttcagcgttaacggctgaaggacatcgggtcaatcgcccaacaccaacctcatgaaataagtgtggataccgtcttatggagcaaaacccgcagtcacagctgaaacttcttgtcacccgtggtaaggagcaaggctatctgacctatgccgaggtcaatgaccatctgccggaagatatcgtcgattcagatcagatcgaagacatcatccaaatgatcaacgacatgggcattcaggtgatggaagaagcaccggatgccgatgatctgatgctggctgaaaacaccgcggacgaagatgctgccgaagccgccgcgcaggtgctttccagcgtggaatctgaaatcgggcgcacgactgacccggtacgcatgtacatgcgtgaaatgggcaccgttgaactgttgacccgcgaaggcgaaattgacatcgctaagcgtattgaagacgggatcaaccaggttcaatgctccgttgctgaatatccggaagcgatcacctatctgctggaacagtacgatcgtgttgaagcagaagaagcgcgtctgtccgatctgatcaccggctttgttgacccgaacgcagaagaagatctggcacctaccgccactcacgtcggttctgagctttcccaggaagatctggacgatgacgaagatgaagacgaagaagatggcgatgacgacagcgccgatgatgacaacagcatcgacccggaactggctcgcgaaaaatttgcggaactacgcgctcagtacgttgtaacgcgtgacaccatcaaagcgaaaggtcgcagtcacgctaccgctcaggaagagatcctgaaactgtctgaagtattcaaacagttccgcctggtgccgaagcagtttgactacctggtcaacagcatgcgcgtcatgatggaccgcgttcgtacgcaagaacgtctgatcatgaagctctgcgttgagcagtgcaaaatgccgaagaaaaacttcattaccctgtttaccggcaacgaaaccagcgatacctggttcaacgcggcaattgcgatgaacaagccgtggtcggaaaaactgcacgatgtctctgaagaagtgcatcgcgccctgcaaaaactgcagcagattgaagaagaaaccggcctgaccatcgagcaggttaaagatatcaaccgtcgtatgtccatcggtgaagcgaaagcccgccgtgcgaagaaagagatggttgaagcgaacttacgtctggttatttctatcgctaagaaatacaccaaccgtggcttgcagttccttgacctgattcaggaaggcaacatcggtctgatgaaagcggttgataaattcgaataccgccgtggttacaagttctccacctacgcaacctggtggatccgtcaggcgatcacccgctctatcgcggatcaggcgcgcaccatccgtattccggtgcatatgattgagaccatcaacaagctcaaccgtatttctcgccagatgctgcaagagatgggccgtgaaccgacgccggaagaactggctgaacgtatgctgatgccggaagacaagatccgcaaagtgctgaagatcgccaaagagccaatctccatggaaacgccgatcggtgatgatgaagattcgcatctgggggatttcatcgaggataccaccctcgagctgccgctggattctgcgaccaccgaaagcctgcgtgcggcaacgcacgacgtgctggctggcctgaccgcgcgtgaagcaaaagttctgcgtatgcgtttcggtatcgatatgaacaccgactacacgctggaagaagtgggtaaacagttcgacgttacccgcgaacgtatccgtcagatcgaagcgaaggcgctgcgcaaactgcgtcacccgagccgttctgaagtgctgcgtagcttcctggacgattaatcggtaggccggatcaggcgttacgccgcacccggcactaggccctctgcacaaacgccaccttttcggtggcgttttttatcgcccacgcactaccagcgcctggtccagctcgcgatacgcttcaaccagtttctccagtgaaacgcgacttaaaccgctgggatttggcagcacccaaatctgcgtcgaaccaatggtgagcgtttgtttcccccactgtgcaccgcgctggctgaatccctgttcatatgcttgtttgcccagaatcgccaacgcctgcggctgataatcttcaattttttcaatcagcttacgcccgcctgcgtgtagctcctgctttgaaacttcattggcttgcaccgttggacggtctaccagtttggtgacgccacaacgataatccagcagatgctgtgcctcctgcggcttcaactgacggtcggtaaacccggcctgatatatcaccttccagaagcgatttgccggatgagcaaagggaaaaccagtcccggcggatgaaagcccagggttgataccgcaaaacacgacccgtaaccctggagccaaaatatcctcaaccatatttactcctttctaacatcaccaggaaaagtataacggattgaaaatacattgtttataaaaacagcaggcgcgcggtaatggctggattgcgacacggagttactttataatccgctaccatggccccttagctcagtggttagagcaggcgactcataatcgcttggtcgctggttcaagtccagcaggggccaccagatatagcaaaggctgacgagaaatcgtcagcctttttctttttatatatcagttactttgcgtgccagtaagccgctgcacgtacccgctgtgggtcatactgttccgcttcaaagcggcggcttaaattcttaacgactttaccttcgccggttatccagatgaagtaatcatcggcagggatttgcatctgcgccagacgcgcatctaccgcctgctcatcatgtgccagccattcgatattaaaaccatcaaggtgcgcgagataatcctgacaggcgttatcccgcacgctaaccagcgcactaacttgcggtttaacggcaagtttgctcaacgtttccaggcggcggcgcaatgcaggcattccggattcatcgcagacatacagctgatacgcgtaatcttccggcaccaccagcgaaccgcgcggacctgccaccgtaagtttatcgcccggttgcgcctgcatcgcccagccgctggcgaccccaccgtcgtgaataaagaaatcaatcgccagttcatggcgtagttcgtcatacagcggcgtatagtcacgcgacggtgggcgtggtccttccggccagacgatgccctcttccgttaccgttggcggcacaaagtgagcgtcaggttgaggaaagaagagtttgctgtgatcgtcaaagccacgcgatgtaaaaccgtccagcgcctcgccgccgaggacaatgcgctgaaaaccggcgctgatgcgctcaacgcgtaacacagtcagttcacggaagcgcagatcattgcgaacgcgctgcgggtagcggggggtgttattcattgttatcgccttcgtgatggtaatcagatatatctaaataaaactcgcaaatgataatgattgttaatcatgataaatgcaagcgatttgtagaactgatatgtctatagtctgataagacgaaccgcctcttctcaggcatcattactcaacgccggatgcggcgtgaacgccttatccggcctacgtgtgagatgagtccacgtttaaaaatcatttttacacttgcaagaacgctcatatcagatataaattagatatatctaattaagcaaaaggaggctgatatgagccatcatcacgaagggtgttgtaaacatgaaggccagccacgccatgagggctgctgcaaaggtgagaagtcagaacacgagcactgcggacacggtcaccagcatgaacacggtcaatgctgcggtggtcgccacggtcgcggcggcggtcgtcggcaacgtttctttggtcacggtgaattacgtctggtgattctggatattctctcgcgcgatgacagccacggttacgaattgattaaagcgattgagaatctaacccaggggaattacaccccaagcccgggcgtcatctacccaacgctggattttctgcaggagcagtcgctgattaccatccgcgaagaggaaggaggtaagaagcagattgcgctgaccgaacaaggcgcgcagtggctggaagaaaaccgcgaacaggtggagatgattgaagaacgcatcaaagcgcgttgcgttggcgcggcgctgcgccagaacccgcaaatgaagcgggcgctggataattttaaagcggtgctggatttacgcgtcaaccagagcgatatcagtgatgcacaaataaaaaagatcattgcggtgatcgaccgcgccgcttttgatattacgcaactggattaatcgccgcatccgccagtggcgcggtgcaattgccggatgcgacgcttgacgcgccttatccggcctacacccgctacacaccccgcaggcctgataagatgcgccagcatcgcatcaggcattgtgctccaaccgccggatccggcataccgattaatgcagtaccgtcaccgcgtcttccagtcggctggcgcggtgtttcaccatcgccgacacctgcgcactctcttccaccagctcggcatttttctgggtgatcaggttaagctcatccactgcacgggtcaggctggaaagcccatcggcctgttccagcgttgaatggctaatctgggcgatcaactgggtgacgtttttcacctgtgccacaatatcttccatcgtccgtccggcggcgtgtacctgctgcgaaccggattgcaccttatcagcactggcatcaatcagcttgcgaatatcgttggcagcattagcgctgcggctggctaaatgacgcacttcccctgccaccactgcaaaacctttgccctgttcgccggcacgcgccgcttccaccgccgcattcagggccagaatattggtctgaaacgcaatatcgttaatcagcgaagtaatggtgccaatgcgctgggtactgtcggcgatatcgtccattgtcttgatcaccgtggtcatcgcctccccaccctgcactgccgcattactggcagtgattgacagtttatcggcagccgacgccgtggcagagttctgtttcaccgacgccgccatttggttcatggtcgccaccgtttgctgaacgttatcaactgtctgctgggtatgttcgttcagttcatcggtgcctttcgccagcgtctcactgccatttctgacactggacacctggcttgagacatcgttaattagccaacggcacatcaggccaagttgccctaccgcacgtaatgtcagccccagctcatcgctgcgattcagatgctcaacactattacgttctccggtcgccaccttcagtgcctgatgggcaacattttctatcgggcgcacaatctgccattcaaaacaggcgcttgccaacaataccactaacgcacagaggatatacgtcaccaccggggcagcaacaaaccaaagcatggccgccagcaagataaacatcagggtcatcactccacgcgcccgccagcgaagcggtaatgaaggcagtttacccagccagcctttacgcaccaccaggcctttatgaatacgcttactggtacgtccggcgttcaacgctttgtacagcggctccaccgccgcgatctcttcatccgtcgcccgggtacgaatcgacatatagccactgatttttccctcgcgcaccatcggtaccgcattggcccgcacccaataatggtcaccatttttgcggcgatttttcacgatgccgctccagggctccccttttttcagggtgaaccacatatccgcaaacgccgcttttggcatatccgggtgacgcaccatgttgtgcggctgcccttgtaactcttgcaaggtatagccgctcacctgcacaaaagtgtcattagcatgagtgatatagctttgcagatcggtagtggacatcagagtggtatcgtccgccagcggggtattttgctgggtgacatacggatgagaagacatgttcgcgtcctgtgcaggttatatggttgttaacttcttgtcagagtttatgtcggccccgctgcggttatctttaaccgattaatttgatttagatcgcaatttgcgatttaaacacaaatctaattccttgatttaaaatactttcactctgttactatacgaaaacgttaattatcttgcccaaaaatcaggcaattattgccctgaaaacgtgcatttgcgcagcaatcatcaaatccatacccgacaaaaaccgtgcaaaataacaacaaatgttaacagatagcattaaatattgcacaaatgataaccgaatttgtgtttatcccgattttcgcgatcgcagccggagtggcgcaatccctgcaatacttaaatcggtatcatgtgatacgcgagcctccggagcatattttgaacaggttaccttcgagcgcatcggctttagcgtgcagcgcccacgccctgaatctcattgagaagcgaacgctggatcatgaggagatgaaagcacttaaccgagaggtgattgaatacttcaaagagcatgtcaatccggggtttttagagtatcgcaaatctgttaccgccggcggggattacggagccgtagagtggcaagcgggaagtttaaatacgcttgtcgacacccagggccaggagtttatcgactgcctgggaggttttggaattttcaacgtggggcaccgtaatccagttgtggtttccgccgtacagaatcaacttgcgaaacaaccgctgcacagccaggagctgctcgatccgttacgggcgatgttggcgaaaacccttgctgcgctaacgcccggtaaactgaaatacagcttcttctgtaatagcggcaccgagtccgttgaagcagcgctgaagctggcgaaagcttaccagtcaccgcgcggcaagtttacttttattgccaccagcggcgcgttccacggtaaatcacttggcgcgctgtcggccacggcgaaatcgaccttccgcaaaccgtttatgccgttactgccgggcttccgtcatgtgccgtttggcaatatcgaagccatgcgcacggctcttaacgagtgcaaaaaaaccggtgatgatgtggctgcggtgatcctcgaaccgattcagggtgaaggtggcgtaattctgccgccgccgggctatctcaccgccgtacgtaagctatgcgatgagttcggcgcactgatgatcctcgatgaagtacaaacgggcatggggcgcacgggcaagatgttcgcctgcgagcatgagaacgtacagccggatatcctctgccttgccaaagcgctcggcggcggcgtgatgccgattggcgcgaccatcgccactgaagaggtgttttcagttctgttcgacaacccattcctgcataccaccacctttggcggcaacccgctggcctgtgcggcggcgctggcgaccatcaatgtgttgctggagcagaacttaccggctcaggctgagcaaaaaggcgatatgttgctggacggtttccgtcaactggcgcgggaatatcccgatctggtacaggaagcgcgtggtaaagggatgttgatggcgattgagtttgttgataacgaaatcggctataactttgccagcgagatgttccgccagcgcgtactggtggccggaacgctcaataacgccaaaacgatccgcattgaaccgccactgacactgaccattgaacagtgtgaactggtgatcaaagcggcgcgtaaggcgctggcggccatgcgagtaagtgtcgaagaagcgtaatatcaaatcggatggcgatacgacgtcgccatccgatctttttatacgacgcgtacgcccgcaggcatcatccgctccggcgttaacagcacgctttcactgccgtcatcggtttccgcacacaacagcatgcattccgacgtttcaccacgcattttcgctttttgcagattgcataagaccaccaccgttttccccatcagctcttcttcgctgtagtacggcaccaggctggtcacggtttgcagcgttttttgccccacatcaacctgtacgatgtacagcttgtcggcgttttcatggcgtttcacttccacaatctttccgacgcgcatttccagacgtgcaaaatcagcgtaagccacggtttccattgcttcctcccttagggtaaaattttactaaactatagcaaaagtttttctcaatcctgtaggctaaaaatggagaatgcaggcgtgatcacattcgtgagccgctgtgttaccgttacagcgtcaaagaaacgcgctttatttactgaaaacaggtgacccgataagcacttcctctacaatgggggcgcacatcagggaaagtaaaaaaggtaaacatggcaacactaaaagacatcgcaatcgaagctggcgtatccctggcgacagtatccagggtcttaaatgacgatccgacattgaatgtgaaagaagagacgaaacatcgcattctcgagatcgccgaaaagctggagtacaagaccagtagtgcccgtaaactccagacaggtgcagtcaaccaacaccatattctggctatctacagctaccagcaggagctggagatcaacgatccttactatctggcgatccgccacggcattgaaacccagtgcgaaaagctgggcatcgagctcaccaactgttatgaacacagcggcttaccagacattaaaaacgtcaccggtattttaattgtcggcaaacccacgcccgccctgcgcgccgctgccagcgcgttgaccgacaatatctgttttatcgactttcacgaacccggcagcggttacgatgcggtggatatcgatctggcacgcatcagtaaagaaatcatcgacttctatatcaaccagggcgttaatcgtattggttttattggcggtgaagatgagcctggcaaggcggatattcgtgaggtcgcctttgcggaatatggccgactgaaacaagtggtacgcgaagaggatatctggcgcggcggtttttccagttcgtcgggttatgaactggcaaaacaaatgctggcgcgggaagactatccgaaggcactgtttgttgcttccgattccattgctatcggcgtactgcgggcaattcatgaacgaggcctgaacatcccacaggatatttcgcttatcagcgttaacgatatccccaccgcgcgatttacctttccgccgctctccaccgtgcgcatccattccgagatgatgggaagtcagggcgttaacctggtgtatgaaaaagcccgcgatggtcgcgcgctgccgctgttagtcttcgttcccagcaaattaaaactgcgcggcacgacccgttaaatccccttacacactgtccggcaatcgtttttgccggacagtgctgccgtttattttcgtgatccagttaaagtaaatgcatttacctgctactttttagtaaaaattttactaaactccccagcaattacacaaactaccatcaccatgaatggttccgatttctctctaccgggaggccctatgaatcgctgggaaaacattcagctcacccacgaaaaccgacttgcgccgcgtgcgtactttttttcatatgattctgttgcgcaagcgcgtacctttgcccgcgaaaccagcagcctgtttctgcccttaagcggtcagtggaatttccacttttttgaccatccgctgcaagtaccagaagccttcacctctgagttaatggctgactgggggcatattaccgtccccgccatgtggcaaatggaaggtcacggcaaactgcaatataccgacgaaggttttccgttccccatcgatgtgccgtttgtccccagcgataacccaaccggtgcctatcaacgtattttcaccctcagcgacggctggcagggtaaacagacgctgattaaatttgacggcgtcgaaacctattttgaagtctatgttaacggtcagtatgtgggtttcagcaagggcagtcgcctgaccgcagagtttgacatcagcgcgatggttaaaaccggcgacaacctgttgtgtgtgcgcgtgatgcagtgggcggactctacctacgtggaagaccaggatatgtggtggtcagcggggatcttccgcgatgtttatctggtcggaaaacacctaacgcatattaacgatttcactgtgcgtaccgactttgacgaagcctattgcgatgccacgctttcctgcgaagtggtgctggaaaatctcgccgcctcccctgtcgtcacgacgctggaatataccctgtttgatggcgaacgcgtggtgcacagcagcgccattgatcatttggcaattgaaaaactgaccagcgccagctttgcttttactgtcgaacagccgcagcaatggtcagcagaatccccttatctttaccatctggtcatgacgctgaaagacgccaacggcaacgttctggaagtggtgccacaacgcgttggcttccgtgatatcaaagtgcgcgacggtctgttctggatcaataaccgttatgtgatgctgcacggcgtcaaccgtcacgacaacgatcatcgcaaaggccgcgccgttggaatggatcgcgtcgagaaagatctccagttgatgaagcagcacaatatcaactccgtgcgtaccgctcactacccgaacgatccgcgtttttacgaactgtgtgatatctacggcctgtttgtgatggcggaaaccgacgtcgaatcgcacggctttgctaatgtcggcgatattagccgtattaccgacgatccgcagtgggaaaaagtctacgtcgagcgcattgttcgccatatccacgcgcagaaaaaccatccgtcgatcatcatctggtcgctgggcaatgaatccggctatggctgtaacatccgcgcgatgtaccatgcggcgaaagcgctggatgacacgcgactggtgcattacgaagaagatcgcgatgctgaagtggtcgatattatttccaccatgtacacccgcgtgccgctgatgaatgagtttggtgaatacccgcatccgaagccgcgcatcatctgtgaatatgctcatgcgatggggaacggaccgggcgggctgacggagtaccagaacgtcttctataagcacgattgcattcagggtcattatgtctgggagtggtgcgaccacgggatccaggcacaggacgaccacggcaatgtctggtataaattcggcggcgactacggcgactatcccaacaactataacttctgtcttgatggtttgatctattccgatcagacgccgggaccgggcctgaaagagtacaaacaggttatcgcgccggtaaaaatccacgcgcgggatctgactcgcggcgagttgaaagtcgaaaataaactgtggtttaccacgcttgatgactacaccctgcacgcagaggtgcgcgccgaaggtgaaacgctcgcgacgcagcagattaaactgcgcgacgttgcgccgaacagcgaagcccccttgcagatcacgctgccgcagctggacgcccgcgaagcgttcctcaacattacggtgaccaaagattcccgcacccgctacagcgaagccggacaccctatcgccacttatcagttcccgctgaaggaaaacaccgcgcagccagtgcctttcgcaccaaataatgcgcgtccgctgacgctggaagacgatcgtttgagctgcaccgttcgcggctacaacttcgcgatcaccttctcaaaaatgagtggcaaaccgacatcctggcaggtgaatggcgaatcgctgctgactcgcgagccaaagatcaacttcttcaagccgatgatcgacaaccacaagcaggagtacgaagggctgtggcaaccgaatcatttgcagatcatgcaggaacatctgcgcgactttgccgtagaacagagcgatggtgaagtgctgatcatcagccgcacagttattgccccgccggtgtttgacttcgggatgcgctgcacctacatctggcgcatcgctgccgatggccaggttaacgtggcgctttccggcgagcgttacggcgactatccgcacatcattccgtgcatcggtttcaccatgggaattaacggcgaatacgatcaggtggcgtattacggtcgtggaccgggcgaaaactacgccgacagccagcaggctaacatcatcgatatctggcgcagcaccgtcgatgccatgttcgagaactatcccttcccgcagaacaacggtaaccgtcagcatgtccgctggacggcactgactaaccgccacggtaacggtctgctggtggttccgcagcgcccaattaacttcagcgcctggcactatacccaggaaaacatccacgctgcccagcactgtaacgagctgcagcgcagtgatgacatcaccctgaacctcgatcaccagctgcttggcctcggctccaactcctggggcagcgaggtgctggactcctggcgcgtctggttccgtgacttcagctacggctttacgttgctgccggtttctggcggagaagctaccgcgcaaagcctggcgtcgtatgagttcggcgcagggttcttttccacgaatttgcacagcgagaataagcaatgaggatcatcgataacttagaacagttccgccagatttacgcctctggcaagaagtggcaacgctgcgttgaagcgattgaaaatatcgacaacattcagcctggcgtcgcccactccatcggtgactcattgacttaccgcgtggagacagactccgcgaccgatgcgctatttaccgggcatcgacgctattttgaagtgcattactacctgcaagggcagcaaaaaattgaatatgcgccgaaagagacattacaggtagtggaatattatcgtgatgaaactgaccgtgaatatttaaaaggctgcggagaaaccgttgaggtccacgaagggcaaatcgttatttgcgatatccatgaagcgtatcggtttatctgcaataacgcggtcaaaaaagtggttctcaaagtcaccatcgaagatggttatttccataacaaataacaactacggcggcaaaaggagtttgccgccaccgctaccctactcattttcggagatgtgttatgtctgataccaaacgtaatacaatcggcaaattcggcttgctctcgctgacttttgccgccgtttacagctttaacaacgttatcaataataatattgagcttggactggcctcggcaccgatgtttttcctcgcgacgattttttattttattcccttctgtctgatcatcgcagaatttgtttcgttaaataaaaactcagaagccggtgtctacgcgtgggtaaaaagttcgctgggcggacgttgggcatttattactgcctatacctactggttcgtaaacctgttctttttcacctcactgttgccgcgcgttattgcttatgcttcgtatgccttcctcggatacgaatatattatgacgccggttgccaccaccattatcagtatggtgctgttcgccttctccacctgggtttccaccaacggggcgaaaatgttggggccaattacctccgtcacttcaacgctgatgctgctgttaacgctctcctacattttactggcaggtacggcgctggttggcggcgtacagcctgctgacgccatcaccgttgacgcgatgatcccgaacttcaactgggcgttcctcggcgttaccacctggatctttatggccgcaggtggcgcggagtccgtcgctgtgtacgttaacgacgtcaaaggcggttcgaaatcgttcgttaaagtgatcatcctcgccgggatttttatcggcgtactgtattccgtctcctcggtgctgattaacgtcttcgtcagcagcaaagagttgaaatttaccggcggatcggtgcaggtattccacggcatggcggcgtattttggtctaccggaagcgttgatgaatcgctttgtcggtctggtgtcctttaccgcgatgttcggttccctgctgatgtggaccgcaacgccggtgaaaattttcttctccgaaatcccggaaggcatctttggtaagaaaaccgtcgaactgaacgaaaacggcgttccggcgcgcgcagcgtggatccagttcctgatcgtcatcccgctgatgattatcccgatgctcggttccaataccgtgcaggatctgatgaatactattattaatatgaccgccgcagcgtccatgcttccgccgttattcatcatgctggcttacctgaatttacgcgccaaattagatcacctgccacgcgatttccgtatgggctcccgccgcaccggtattatcgttgtttcaatgctgattgcgatatttgccgtagggtttgtcgcttcgacattcccgactggcgcgaatattctgaccatcattttttataacgtcggcggtattgttatcttccttggctttgcgtggtggaaatacagtaaatatataaagggattaacggctgaagagcgccatattgaagcgacgccagccagcaatgttgattaagcagaataataaaaaatgagcaggcattttccctcttcctggatgaggagagggaaaatagtttctgcctttatatttttataattacaacgataaaaggctgtactttttctttagctcatggattaacacaatgaaattaatcactgcaccatgcagagcattacttgctctgccgttttgctacgccttttctgcggcaggagaagaagcacgtccggcagaacatgacgacacaaaaacacccgcaattacctcgacatcttctccttcatttcgtttttacggcgaattaggggttggtggatatatggatttagagggtgagaataaacataaatacagcgacggtacctatattgaaggtggcctggagatgaagtacggctcctggttcggcctgatttacggcgaaggctggaccgtgcaggccgaccacgacggcaatgcctgggtgccagaccatagctggggtggtttcgagggcggaattaaccgtttctatggcggttatcgtaccaatgatggcaccgaaatcatgctcagtctgcgtcaggattcctcgctggatgacctgcaatggtggggcgatttcacccccgatctgggctacgtcattcccaatacccgcgacattatgactgcgctgaaggtacagaacttaagcggcaactttcgttatagcgtcaccgcgactcctgccggacatcatgatgaaagcaaagcctggctacattttggcaaatacgatcgctatgacgacaaatacacctatccggcaatgatgaacggttacatccagtatgaccttgccgaaggcatcacctggatgaacggtctggaaatcaccgacggcacaggacagctctatctcacgggcctgctaactcctaactttgccgctcgcgcctggcaccataccggacgcgccgacgggctggacgtaccgggaagtgaaagtgggatgatggtgagcgccatgtatgaagcgttaaagggcgtttatctctccaccgcttacacctacgccaaacatcgccctgaccacgctgacgatgaaaccacctctttcatgcagtttggtatctggtacgaatacggcggcggacgtttcgccacggcttttgatagccgcttctacatgaaaaatgcctctcacgatcccagcgaccaaatcttcctgatgcaatatttctactggtaataaggactgtaatttcatgaaaataaaaactattttaacgccagtaacctgcgctctgctgataagtttttccgcccatgccgctaacgccgacaattataaaaacgtgattaaccgtactggcgcgccgcagtacatgaaggattacgattacgacgatcaccagcgttttaatccgtttttcgatctcggagcctggcatggtcatctgttgccagacggccctaacaccatgggcggctttccgggcgttgcgctgctgacggaagagtacatcaactttatggccagcaatttcgaccgcctgaccgtctggcaggacggcaagaaagtcgactttacgctggaggcatacagtattcccggtgcgctggtgcaaaaactgacagcaaaagatgtgcaagtcgaaatgactctgcgcttcgccacgccgcgcacgtcactactggaaaccaaaatcaccagcaataaaccgctggatctggtgtgggacggcgaactgctggaaaaactggaagcgaaagaagggaaaccgctttccgataaaaccattgctggcgaataccctgactatcagcgcaaaatcagcgccacccgtgatggcctgaaagtcacctttggcaaagtgcgcgccacctgggatctgctgacctccggcgaatcggaatatcaggtgcataaatccctgccggtgcagactgaaatcaacggtaatcgctttaccagtaaggcgcatatcaacggttcgaccacgctctacaccacctattcccatctgctgaccgctcaggaagttagcaaagagcaaatgcagatccgcgatattctggcgcgtccggcgttttatctcaccgcctcgcagcaacgctgggaagaatacctgaagaaagggttaaccaatccggatgcgacgccggaacagacgcgcgtcgcggtgaaagcgatcgaaacgctcaacggtaactggcgctcaccgggcggtgcggtgaaatttaacaccgttacaccgtcggtgaccgggcgctggttctccggcaatcagacctggccgtgggatacctggaagcaggcgtttgcgatggcgcatttcaatccggacatcgccaaagagaatatccgcgcggtcttctcctggcagatccagcctggcgatagcgtgcgtccgcaggatgtgggctttgtccccgacctgatagcgtggaaccttagccccgagcgtggtggcgatggcggcaactggaacgaacgtaataccaaacccagccttgccgcctggtcggtgatggaagtgtataacgtcacccaagataaaacctgggtggcagagatgtacccgaaactggtggcctatcacgactggtggttacgtaaccgcgatcacaacggcaacggcgtgccggaatatggcgcgacccgcgacaaagcccacaacactgagagcggcgagatgctgtttacggtgaaaaaaggcgataaagaagagacgcagtctgggctgaacaactacgcccgcgtggtggagaaaggccagtacgacagtctggaaattccggcacaggttgctgcatcgtgggaatcggggcgtgatgatgccgccgtctttgggtttatcgacaaagaacagttggataaatatgtcgctaatggcggcaaacgtagcgactggacggtgaaattcgccgaaaaccgcagtcaggacggaacgttgctgggctactcgctattgcaggagtcggtggatcaggccagctatatgtacagcgataaccattatctggcggagatggcaaccatcctcggtaagccagaagaggccaaacgctatcgccagttggcacagcagctcgcggactacatcaacacctgtatgttcgacccgactacccagttctactatgacgtacgtattgaagataaaccactggcgaacggctgcgcgggcaaaccgattgttgagcgcggtaaagggccggaaggctggtcgccgctgtttaacggtgcggcaacgcaggccaatgccgacgcggtggtgaaggtgatgctcgatcctaaagagttcaacacctttgtcccgctgggaacggcggcgttaaccaatccggcttttggcgctgatatctactggcgtgggcgcgtatgggtggatcagttctggtttggtctgaaagggatggagcgttacggttatcgtgatgatgccctgaagctggcggatacgttcttccggcacgccaaagggttaaccgccgatggaccaattcaggaaaattacaacccgctgacaggcgcacagcaaggcgcaccaaatttctcctggagtgccgcgcatttgtatatgttgtataacgattttttccgtaagcaataatttgcaactgctggcggatgcggcgtaaacgccttatccgccctacatgtgcaatcctcctggccggataaaacgcggcaagcgttgcatccggcaactgcaccgcgccactggcggatgcggcgtgaacgccttatccgccctacatgtgtgttcccgtaggtcggataagacgcgacaagcgtcgcatccggcatctgcaccgcgccactggcggatgcggcgtggacgccttatccgccctacatgtgcaattccgtaacctggataaaacgcgacaagcgtcgcatccggcgttatcaccgggcgtattctttttgaatcccatcacaaaccccgcactccccttttcccttttctccggcgacggctaaattagaactcatccgaccacataacaattattttacatactggacaattttatgagctacccgtcgctgttcgccccgctggatttaggttttaccacgttaaaaaaccgcgtgttgatgggctcaatgcacaccgggctggaggaatacccggacggtgccgagcggctggcagcgttttatgccgaacgcgcccgtcacggcgtggcgctgattgtcagcggcggcattgcaccagatttaacaggcgttggcatggaaggtggcgcaatgctcaacgacgccagccagatcccacaccatcgcaccattaccgaagcggtacatcaggaaggcggcaaaatagccctgcaaattttgcataccgggcgctacagctaccaaccgcatctggtcgccccgtccgcattgcaggcccccatcaaccgtttcgtgccccatgagttaagccatgaagagatcctgcaactgatcgacaatttcgcccgctgcgcgcaactggcgcgggaggcaggatacgacggtgtagaggtgatgggttccgaagggtatttgatcaacgaatttctgacgctgcgcaccaatcagcgtagtgaccagtggggcggcgattaccgcaaccggatgcgatttgccgtagaagtagtgcgtgcggtgcgcgaacgcgtcggcaacgacttcattattatctaccgactgtcgatgctcgacctggtcgaagacggcgggacttttgccgaaacggtagagctggcgcaggccattgaagcggcgggcgcgaccattatcaacaccggcattggctggcatgaagcacgtattccgaccattgccacgcccgtgccgcgcggcgcatttagctgggtcacgcgcaaactgaaaggccacgtctcgctgccgctggtaaccaccaaccggattaacgatccgcaggttgccgacgatattctctcgcgcggcgatgccgatatggtatcgatggcgcgaccgtttcttgctgatgcggagctgctgtcaaaagcgcaatcgggacgagccgatgagatcaacacttgtattggctgcaatcaggcctgtctcgatcaaatcttcgttggcaaagtcacctcgtgcctggtgaatcctcgcgcctgccacgaaaccaaaatgccaatccttcccgccgtgcagaaaaaaaatctggcggtggtcggtgcgggacctgctgggctggcgtttgccattaacgcggcggcgcgtgggcatcaggtaacattgtttgacgctcatagcgagattggcgggcagtttaatatcgccaaacagatccccggcaaagaggagttttacgaaacgctgcgctattaccgccggatgatcgaagtgacgggcgtgacgctaaaactcaatcacaccgtgacggcggatcagttacaggctttcgatgaaacgatcctcgccagtgggatcgtgccgcgcactccgcccatcgacgggatcgatcatccgaaggtattgagttatctcgatgtactgcgcgacaaagcgccggttggcaacaaagttgccatcatcggttgtggcgggattggttttgatacggcgatgtatttaagtcagccgggcgaatccaccagccagaatatcgccgggttctgtaatgaatgggggatcgacagtagcctacaacaggctggtggcttaagcccgcagggaatgcagatcccccgtagcccacggcagattgtgatgctccagcgcaaagccagcaaaccaggacaggggttaggcaaaaccaccggctggatccatcgcaccaccctgctctcgcggggtgtgaaaatgatcccaggcgtaagttatcagaagattgacgatgacgggctgcatgtggtgatcaacggcgaaacgcaggtattagcagtggacaatgtggtgatctgcgcagggcaagagccaaaccgcgcgctggcgcaaccgctgattgatagcgggaaaacggtgcatttaattggcggctgcgatgtggctatggagctggacgcacgacgggcaattgcccagggaacacggctggcgctggagatttaaatcgttatttgaagcgccggatgcaacgcatccggcacgtcgcgttaatcaataaacaaggcgggagaaatgccgaatcgcgttgccaattttttagcgtgttccagcgttaatttcctcttcccgctcaaaacgcgtgacaccatagatttactgccaatttccggcagatcggaaagggttaaaccatattgatccataagggtacgaatcacggctataccgccaggcatggcttgagccatggcattaaattccgcaaattcgggcgctgattcttcccacgcggttattttggcacacaccagatccagcaaggggttttcaggatcgttgagcagcagatgatctaccagttccagcgcctgggtgtattgttcctcgttctgaatacccgccagaaaaggtgccacagcagttagcttttctcctgcttgcaagatgtcggcaatcgcaatcattttttccccttagtacgatgaacagcggtaaagaaatcgtattctttatgcgtcataacttcacgtatgtagcacttttgcgattcaaaaaagaccattgctacaacacgtaattcattgcccccaacattgaaaacataatgcttatccagatatttgaagttatccagagatgggaatactgcttttaatgactcaggttttttgaaatatcccttagcaatcgtgttccccagagccaccaactccgttttatgttgcgggtatttttccgcagcatctttcaatgctttttgagttatcaggtgcattcttcatcacgtccgttgacaaattggcaatatgataacatccgttgccagattggcaacggatgaatttatctgtgtgacggaagaataaacgtagaaaaacgctaaacaagagaatgtagacgatggtgacagggattttttgttttatggaagcgcgattccagaactgggcagacattgccggatgcgacgcttgccgcgtcttatccggcctggagtaacgtgctgaacgtaggccggataaggcgtttacgccgcatccggcaggtaactcccaatcttaccgacgacgtcccagcttcaccgctttcagtaccacaaatttattattcgtcgcaatagtggtgcagttgccgaaaatcttcttcagtttatggaagtaatccaggtgacggttggcaacgatatacagctcgccgttgattttcaggcagcggcgggcgtggtggaacatctcccaggcgacgttatcggtcagcgcatgttgttggtgaaacggcgggttgcagagcacagcattaaagcggaaaggctccacgccggagagcgcgttgttgatcataaactcgcagcgatccaacgcctctggcatgttggtttcaacgttcaaacggctggaagcaaccgccatcggcgattcatcgacaaacaccactttcgcctgcgggtttttatcaagcagcgtcagaccaataacgccattaccgcaaccgagatcgacaatctccccttcgagattctctggcagatgttgcataaagaagcgcgcgccgatatcaagcccggtgcgggagaagacattcgcatggttgtggatagtccagtcagtaccttccagcttccagctaacggtctgcggcgcatcggccagctgcggttcattgaaagtgcaattaatcaggcgcgcttttttccatgccagcgtggtggtggttgggccgagcactttttcgaacagttccagcgtggaagtgtgaatgtcacgggccttggcaccggcaataatacgtgtatccgacgtgaccactttgcgcagcgcacgcagttgctgttccagcaatgccagtgttttcggcactttgatcagcaccacacccggctgttgcgggtagtcggcggtgctgtcgagaaacttcacgctcgactcatcaatcccgttgaggcgtaaattctcgcgcgtcgccagttcactgatgtatgagtcgccaatgctgtacggcttatgttccgccagtgcgcagcttaacgcaccaaaggcatcattcaggatcaacaccgggccgcggatttctgtgtcgtccaactgttgcagcaaatattcatccgccgcttcccacgcctgtagcgggttaacgtcatccgtcgccggaaaacgttgtagtgtcagtgaacggaaaccgttgtctaagtggctcatcggccctcctgaatgataaaatttcgacattgcccctgaaaagggtgcgtgagtataccctttttctctttttcgtgggcggttatgagcaatcttacttatcttcagggttatcccgagcagctactttcccaggtgcgaacactgattaacgaacagcgtctgggcgatgtgctggcaaaacgctatccgggaacacacgactacgccaccgataaagccctctggcaatatactcaggatctgaaaaatcagtttctgcgtaatgccccgccgatcaataaagtgatgtatgacaataagatccatgtgctaaaaaacgcgctcgggttacataccgctgtttctcgtgtgcagggcggcaagctgaaagcaaaggtggagatccgcgtcgctaccgtgtttcgcaacgcgccggaaccgtttttgcgcatgatcgtggtgcacgagctggcgcacctgaaggagaaagagcataacaaagcgttttaccagttgtgttgtcatatggaaccccagtaccaccagcttgagttcgacacccgactgtggctaacgcagttgtcgcttgggcagaacaaaatctgaaaatgatgtcaggcgttatcttttctttctttagcgcctaaaatcgacctcccccctttcgttaaggataacgaccatgctgcgcgcatttgcccgccttcttctccgtatttgtttttctcgccggactctaaagattgcctgcttactgttacttgtggcaggagcgaccatccttatcgccgatcgcgtaatggtcaacgccagcaaacagctgacctggagcgatgtcaacgccgttccggcgcgtaacgtgggtttattgctgggggcgaggccgggtaatcgctactttacccgacgtattgataccgcagcagcgttgtaccacgccggaaaagtgaaatggctgctggtaagtggcgataacggacgtaaaaattacgatgaagcatcaggtatgcagcaggctttgatcgctaaaggcgtaccagcaaaagtgatcttctgcgactatgccggattctcaacgctggattcggtagtgcgtgccaaaaaggtttttggtgaaaaccatatcaccattatctcgcaagaatttcataatcaacgcgccatctggctggcaaaacagtacggcatcgacgctatcggttttaacgcgccagacctcaatatgaagcacggtttttatactcaactgcgggagaaactcgctcgtgtcagcgccgtgattgacgccaaaatcctccatcgccagccgaaatatctcgggccttcggtcatgattgggccgtttagtgagcatggctgtccggcgcagaaataatgcgtatctgcgcacgtcgaagatgaaaaaggcgtgctacattgacgacagaatccctttatggagtatccacgcgttatgatacgtttcgctgtgattggtacgaactggatcactcgccagttcgtcgaggccgcccatgagagcggtaaatacaagttaaccgccgtatattcccgcagccttgaacaggcccagcacttcgccaatgatttttctgtcgagcatctgtttacctcgctggaagcgatggcggaaagcgatgccattgacgcggtgtatattgccagcccgaattccctgcatttttcccagacacaacttttccttagccataaaattaatgtgatttgcgagaaaccgctggcgtcgaatctggcggaagtggatgccgccattgcctgtgcgcgggaaaatcaggtggtgctgtttgaggcatttaaaaccgcctgcctgccgaactttcatttgttgcgccaggcgctgccgaaagtcggcaaactgcggaaagtctttttcaactattgccagtattcctcgcggtatcaacgttacctggatggtgagaatcccaacacctttaatccggcattctctaacggttcaattatggatatcggtttttactgtctggcgtcggcggtggcgttatttggtgagccgaaaagcgtgcaggcaaccgccagtttgctggcaagcggcgttgacgcccagggcgtggtggtgatggattacggtgatttcagcgtcaccttgcagcactcaaaagtcagtgattctgtcctggcgagcgagattcagggcgaagcaggatcgctggtgattgaaaaactgtctgaatgccagaaagtgtgcttcgtgccgcgtggcagccaaatgcaggatctcacccagccgcagcatattaataccatgctctacgaagcagagctgttcgctaccctggtggatgagcatctggtggatcatccagggctggcggtcagtcgcatcaccgccaaactgctgaccgagatccgccgccagactggggtgatttttccggcagatagcgtaaaactataattgccaaagtaaaacagtgtaaaaggtatgtaacagaccattgactggctgaatggtctgtcatactttgttacctgcaaaggggagtaacttcattgccggtcgatcgtcattacgatgtgtgaaaaaacacatccggtcaccgggcaacccgaaaggaatacgcagacgtattccttttttgttgtaagtgagaccttgccggaaggcgaggtctatgcataaaaagcagcggctgacgtcttccgacgttggccgtttttttatgtgtaaggaacttctatgaatactgtcggcacgccgttgctatggggcggattcgctgttgttgtcgccattatgctggctatcgacctgttgttgcaggggcgtcgtggggcacatgccatgaccatgaaacaggctgcggcctggtcgctggtctgggtgacgctgtcgttactgtttaacgccgctttctggtggtatctggtgcaaaccgaaggtcgcgccgttgccgatccacaggcactggcctttctcacaggttatctgattgagaaatcgctggcggtcgataacgtctttgtctggctgatgttgttcagctatttctctgttccggcggcattacaacgccgcgtgctggtgtatggcgtgctcggggcgattgttctgcgtaccatcatgatcttcactggcagctggctaatttcgcagttcgactggatcctgtatatcttcggtgccttcctgctgtttaccggcgtgaagatggcgctcgcccatgaagatgaatcaggcattggcgacaagccgctggtgcgctggctacgcggtcatttgcgcatgaccgacaccatcgacaacgagcatttctttgtgcgtaagaatggattgctgtacgccacaccgctgatgctggtactgattctggtggaattgagcgacgtgattttcgccgtggatagcattccggctatcttcgccgtgaccactgacccgttcattgtgctgacctcaaacctgtttgcgatcctcggcctgcgtgcgatgtatttcctgctggcgggcgtagcagagcgtttctcgatgctcaaatatggcctggcggtgattctggtgtttatcggtatcaagatgctgattgtcgacttctaccatattccaatcgccgtctcgctgggcgtggtgtttggcattctggtgatgacgtttattatcaacgcctgggtgaattatcggcatgataagcagcggggtggataatttttaatctgcctaagccgtgtaccctgtcattaacatgagcaccgttttctccctctcccttccagggagagggtcggggtgagggtaatttttcgcaccgatgctggcctgttcccctcaccctaaccctctccccaaacggggcgaggggactgaccgagtccttttttgatgttgtcatcagtctggaagccgcacgttggctttatttttatgtcaaagaaatgtaaccattaagtttcaaaatatgacctctctttaaaatccagcatttttcgcttcccgaagctgtaactttccttatactcgaccttgcaaacactttgttacatcctgaaagatgcgtcgacagaacgcaccagggatgtgcgacaacacaatgaaaggatcgaaaaatgactacgcaacgttcaccggggctattccggcgtctggctcatggcagcctggtaaaacaaatcctggtcggccttgttctggggattcttctggcatggatctcaaaacccgcggcggaagctgttggtctgttaggtactttgttcgtcggcgcactgaaagccgttgcccccatcctggtgttgatgctggtgatggcatctattgctaaccaccagcacgggcagaaaaccaatatccgccctattttgttcctctatctactgggcaccttctctgctgctctggccgcagtagtcttcagctttgccttcccttctaccctgcatttatccagtagcgcgggtgatatttcgccgccgtcaggcattgtcgaagtgatgcgcgggctggtaatgagcatggtttccaaccccatcgacgcgctgctgaaaggtaactacatcgggattctggtgtgggcgatcggcctcggcttcgcactgcgtcacggtaacgagaccaccaaaaacctggttaacgatatgtcgaatgccgttacctttatggtgaaactggtcattcgcttcgcaccgattggtatttttgggctggtttcttctaccctggcaaccaccggtttctccacactgtggggctacgcgcaactgctggtcgtgctggttggctgtatgttactggtggcgctggtggttaacccattgctggtgtggtggaaaattcgtcgtaacccgttcccgctggtgctgctgtgcctgcgcgaaagcggtgtgtatgccttcttcacccgcagctctgcagcgaacattccggtgaatatggcgctgtgtgaaaagctgaatctggatcgcgatacctattccgtttctattccgctgggagccaccatcaatatggcgggcgcagcaatcactattaccgtgttgacgctggctgcggttaatacgctgggtattccggtcgatctgcccacggcgctgctgttgagcgtggtggcttctctgtgtgcctgtggcgcatccggcgtggcgggggggtctctgctgctgatcccactggcctgtaatatgttcggtatttcgaacgatatcgccatgcaggtggttgccgtcggctttatcatcggcgtattgcaggactcttgcgaaaccgcgctgaactcttcaactgacgtgctgttcactgcggcagcttgccaggcagaagacgatcgtctggcaaatagcgccctgcgtaattaattgtttaacccctttcgtctacggcggaaggggttttctcaactttaaacggatcaattccccttttctgcatccgccagaaacgaatgatattcaggccattcataagcagaaaactaccctcaatcatcgtgccgcctatcgaccccgcccagaagttgtgaatcacccagcaacacgttgaaaaccacattacgcagcgcatggtcagccctttacagcagaatagcgcccaggtactgacaatcgtgccgataaccggcaatagttcgacaggatgatggaacttcgcgaggccaattccgccagtcagcacaataaaaatcgccattacccataagctgcgcgtgcgtaaggtaatcaatgtacgaatggcattaaggatggcactggcaccagcgggataggtgcccagaagaaaaaaatgtacgccaataacggcgctatagaccgaaagctgctttttgaagcgacgttcgtcacgattgaaaaatgttgtgataccaatcagaaaggcgatgacacccacgccctgggccagccaatacgcggtcatgataaatccttagcaggtatggaaaagcaaacggcgcttcacattatgaaacgccgttttttattaacaactcatttcgactttatagcgttacgccgcttttgaagatcgccagttcgcggaagtcgttacgctcgttacaggtttgcttaccgttggcaaactcaacgatggtgtcgataaattcttccagcaactgcggcatcgctttaccgtggatcaactgacccgcgtcaaagtcgatccagtgttttttcttcgccgccagttcactgttggtggcgattttcaccgtcggcacaaatccaccatacggcgtgccacgaccagtactgaacagcaccatatggcagcccgcacccgccagggcgctggtcgctacggcatcgttacccggcgcacttaacaagttcagccctggcgttttcagacgctcgccgtaacgcagcacgtcaaccacgacgctggaacccgctttctgggtacagccaagtgatttgtcttccagcgtggtgataccgcccgctttgttccccggcgatgggttttcatagatcggctgatcatgggcaataaagtactgtttgaagtcgttgaccatggtgaccagtttttcaaacgttgcttcgtcgcggcaatggtccatcagcaactgctctgcgccaaacatctccggcacttcggtcagtacggtagtaccgccgttagcaatcacgtagtcagagaaacgccccagcatcgggttagcagtaataccagaaagaccgtcagaaccaccgcactccagaccaaacttcagttcgctgagtttgcctggctcgcgtttatcgttgcgcatcacgttatacagctgatgcaaatgctcgattccggcttcgatctcatcatcctgctgttggcagatcatgaaatgaacgcgttcaggatcgatatcgcccagcgtttcacggaatgcggcaacctggttgttttcacagcccagaccaatcaccagcactgcgcctgcgttcgggtggcgcaccatgttttgcagcatggtgcgggtattaatgtgatcgtcgcccagctgtgagcagccgtaggtgtggctgaagaggaacacgccgtcagtaccttcggcgttgttggtctctttcagaaaacggttctggatctgccgcgcgatgccgttgacacagcccacggttggcaggatccacagctcattacgcaccccgacatcgccgttagcgcgacgatagatctgcacttcacgatctgccgcttgcgcaggcagatcctgaaaatcaggttgatagcgatactgatccagatcgctcagattcgtgcgcgtattgtgggcgtgaacgtgaacacctgccgcaatatccgccaatgcataaccaatcggcaggccatatttgatgacattggccccttttgcgatatccgttaacgcaaatttatgtccacgagcaacatcctggcgcagcgtaacagtctggttatcgacactgacttctgtgccttcagccaaatctgctaaagcgaccgcgacgttatccagcgcatggatcttgatgtattgcatatcaaccccagaccttagttcagttcaatggcgaagtagtcacgcgcattgttaaagcaaatatttttcaccatctcgcccagcaggttgatgtccgccggtgcttcgcccgcttccacccagcgaccgatcatctggcacagaatgcggcggaagtattcgtgacgggtgtatgacaggaagctacggctgtcagtcagcataccgacaaagcggctcagcagaccgagctgcgccagttgggtcatctgacgttccataccgtctttctgatcgttaaaccaccagccggaaccgaactgcattttgcccggcataccttcgccctggaagttaccgatcatggtgcccagcacttcgttatcgcgcgggttcaggcagtacagaatggttttcggcagcaggttttcttcattctgcttgctcagcaacttagacagctcttccgccatcggacggtcgttgatggagtcaaagcctacatccggccccagcagtttgaactgacgcaggttgttattacgcagcgcgccaatgtggtactgctgtacccagccgcgacgtgcatattcggcaccaaggaacaccagtaccgcagttttgaactgcgccacttcgtgctcgctcagggtttcgccagccagacggcgcgccagaatgctgtccagttccgcttcgttcgcttcagcaaacatcaccacatccagcgcgtggtcagacactttacagccgtgagcggcgaagtgatccagacgtttggtcagggcagtttgcaggtcagcaaagcggcgaatgtcggtatcggaaacttcgcccagcttcgccatgtagtcgttaaaggtcgcctgttcgatgttgaaggctttgtccggacgccagctcggcagcactttgatggtgaaagagccgtctttggcgatctctgcgtgatgctccagagaatcgatcgggtcatcggtggtgccgaccattttcacgttcatctgctgcatgatgccgcgcgcggagaagttatcctgcgccagcagttcgttacattcgttccagatttcatcggcagttgacggagaaagcaatttgccagtgataccaaacggacggcgcagttcgaggtgcgtccagtggtataacgggttgccgatagtgtgcggaacagtcgccgcccaggcgtcaaatttttcacggtcagacgcatcaccggtacacagacgctcggccacaccgttggtacgcatagcgcgccatttgtagtgatcgcctttcagccagatgtcatacaggtttttaaaacgatagtcttccgcaatctgctgcggcggcaaatggcaatggtaatcgaaaatcggctggtcttttgcgtagtcgtgatacagacggcgggcaaattcggtatctaacaggaaatcttcagtcataaacggagtcattttcgtcttcctctcaacgagtgagctagcttgcttatggtgcgatgctgacaaagttatcacaccaatttccagagtccgaagatattttcgtgagttagatcaataaacgtagttaaaaaaattactctcaaagtggtaaatctcgctgcaggccgcgccagtactggccttgctgtcgtcaggtaatgtccctacaaatattcccacatttgtgatggctctcaccttttaaagttgtatgacaagttatctttctgccgtcgcaaatcataagtcgacggaatgcaaattgccgattcattcatttgttagatgaatcgggttaaccggtacggaagccgaattagcacgaaactttcatggcaacgttcggggcgtgccggttttttttcggttacccggtcgtaactaacatcttcagcctctggcgggatgatggccgcgcttcctgcggatataacaaaacgatgaggttttacatgcgtaaaattaaagggttacgttggtatatgatcgcactggtgacgctcggcaccgtgcttggttacctgacgcgtaacactgtggcggcagctgcgccaactctgatggaagagttaaacatctccacccaacagtattcctatatcatcgcagcctattctgctgcttatacggtcatgcaaccggtagcaggttatgtactggatgtgctgggtacgaaaatcggttatgcaatgtttgctgtgctgtgggccgtgttctgtggtgcaaccgcgctggcaggtagctggggtggcctggctgttgctcgtggtgcggtcggtgccgcggaagcagcgatgatcccggcgggtctgaaagccagctccgaatggttcccggcgaaagagcgttccatcgcagtaggctactttaacgtaggttcttcgattggtgcgatgattgcgccgccgctggtggtatgggcaatcgtaatgcacagctggcagatggcatttatcatctccggtgcattgagctttatctgggcgatggcatggctgattttctataaacatccgcgcgaccagaagcatctgaccgatgaagaacgcgactatattattaatggtcaggaagcccagcaccaggtgagcacggcgaagaaaatgtccgttggtcagatcctgcgtaaccgtcagttctggggtatcgcgctgccgcgtttcctggcagaaccggcctggggtacttttaacgcgtggatcccgctgttcatgtttaaagtttacggctttaacctgaaagagatcgcgatgttcgcctggatgccgatgctgtttgctgacctcggttgtatcctcggtggttacctgccgccgctgttccagcgttggtttggtgtgaacctgatcgtttcccgtaagatggtcgtaacgctgggtgcagtgctgatgattggcccgggtatgatcggcctgttcaccaacccgtatgtcgcaattatgctgctgtgtatcggtggttttgcccaccaggcactgtctggcgcgctgattacgctctcttccgatgtgtttggtcgtaacgaagtggcaacggcaaacggtttaaccgggatgtccgcatggctggcaagtacgctgtttgcgctggttgtcggtgcactggctgacaccatcggcttcagcccgctgttcgcagttctggcagtgttcgacctgttaggtgcgctggttatctggaccgtgttgcagaacaaaccggcgattgaggtggcgcaggaaacacataacgatcccgcaccgcaacattaacgtttcgtgtaagttttagtttcccttcaaagccgccttctcaggcggctttttcatcactgcgagtagagctaaactcgcaaaagtggtataacaaatatagtctgccgtatcatgcctggagcgcatatggaaatcactgaaccacgccgtttgtatcaacaacttgccgctgacctgaaagagcgcatcgaacagggcgtctatctggtgggtgataaactgcctgcagaacgctttattgccgatgaaaagaacgtcagccgtacggtagttcgtgaagccatcatcatgctggaagttgaaggctatgtcgaagtgcgtaaaggttcaggtattcatgtggtttccaaccagccgcgccatcagcaggcggctgacaataatatggaattcgccaattacggtccgtttgagttgcttcaggctcgccagctcatcgaaagtaatattgccgaattcgcggcaactcaggtaacgaaacaggacatcatgaaactgatggccattcaggaacaggcgcgcggcgaacaatgcttccgtgattccgagtgggatttgcagttccacattcaggtcgctctggcgacgcagaactccgccctggcggctatcgtggaaaaaatgtggacccagcgtagtcataacccgtactggaaaaaactgcacgaacacattgattcccgtaccgtcgataactggtgtgatgaccacgatcaaatcctcaaggcgctgattcgcaaagatcctcatgctgctaagctggcaatgtggcagcatctggaaaacaccaagatcatgttatttaacgaaaccagcgacgacttcgagttcaatgccgaccgctatctattcgccgaaaacccggtggtgcatctcgatacagccaccagcggcagtaaatgaaattcctgtccgacaggcgctgcaatgcgcctgtttgtctcgtcggtaagcgaaaagtataaagtgtcagcctgtgtaaatcctctcgccaccctcccctgcattcagcaaaatcagactccacggacatgtaattttgataacgaacaacgttgacctttgttacaattagattcaatttgaatttatgtttttgaatgctttcttatctcacgatttaacagggaatagttcaggctgtgttgatgtatcaaacccgcagaacataccaaaacagcaataacattgcggtagtgcatcttttaaaaccagcgtggcgttaaccgattcaccaggaataatgaatggaacttttgacccaattgctgcaagccctgtgggcgcaggattttgaaaccctggccaatccatcgatgattggcatgttgtattttgtcttgtttgtaattttgttccttgaaaacggcttgcttccggcggcctttttaccgggcgacagtttactggtattggtcggcgtgttgattgcgaaaggcgcgatgggctatccgcaaacgattctgctgctgaccgttgccgccagcctcggctgctgggtcagctatattcaggggcgatggctgggcaatacccgcaccgtacaaaactggctatctcatttacccgcgcattatcatcaacgcgcacaccatctttttcataaacacggtttatcggcgctgttaattggtcgctttattgcgtttgtcagaacactgctgccgacgattgccgggttatcagggctgaataacgcgcgctttcagtttttcaactggatgagcggtctgctgtgggtattgatcctgacaactctgggttacatgctcggcaaaacgccggtatttttaaagtacgaggaccagctgatgtcatgcctgatgctgctcccggtggtgctgctggtgtttggcctggcaggttctctggtcgtgttatggaaaaagaaatatggaaatcgggggtaagggatgcaaatacctcgcatgtcgcttcgccagctagcctggtccggcgctgttttacttctggtcggcacgctgttgctggcctggtccgcggttcgccagcaagagtctacgctggcgattcgtgccgttcatcaaggcacaacgatgccagacggtttttcaatctggcatcaccttgacgctcatggcattcctttcaaaagtatcacccccaaaaacgacactctgttaattacatttgactccagcgaccagagcgccgccgcaaaagcggtcctcgacagaacattgccccatggctacatcattgcgcagcaggacaataacagtcaggctatgcagtggctgacccggttacgggataactctcatcgcttcggataacttcctgttatccgaaacatatcactcactttggtgatttcaccgtaactgtctatgattaatgaggcggtggttaacactaccgcttcgttgtctggacaatcgttcctttgtaataggtccgaatcacaatggaaggttcaagaatgaaataccgcatcgctttagctgtttctctctttgctcttagtgccggtagttatgccactaccctgtgtcaggaaaaggagcaaaatatccttaaggagatcagctatgccgaaaaacaccaaaaccagaatcgtattgacggtctgaataaagccctgagtgaagtccgggccaactgttcagatagccagctgcgtgccgatcatcagaagaaaatcgcaaagcagaaagatgaggtggcggaacgccagcaagatttagccgaggcgaagcaaaaaggcgatgccgataagattgccaaacgcgaacggaaactggcagaagcgcaggaagagctgaaaaagctggaagcgcgcgactactaactcacaatagtcactacttactcacctggagaaaactatgtcgaaagaacacactacggaacatctgcgtgctgagttgaaatccctttccgatacgctggaagaggtgcttagctcatctggcgagaagtcgaaagaagagttgagtaagattcgtagcaaagcggagcaggcactgaaacagagccgttatcgcctgggtgaaaccggtgatgccattgccaaacaaacccgtgtcgcggcggcgcgtgccgatgagtatgtgcgcgaaaatccgtggacgggcgtgggcattggcgctgcaatcggtgtagtgctcggcgttctgctgtcgcgtcgttaattatggcggacactcatcacgcacaagggcccggtaaaagcgttctgggcatcgggcagcgaattgtttctatcatggttgaaatggtagagacacgtctgcggctggcggtggtggagctggaagaggaaaaagcgaatctctttcaacttttactgatgctgggcctgacgatgcttttcgctgcatttggtcttatgagcctgatggtgctaattatttgggcggttgacccgcaatatcgcctgaatgcgatgattgccaccaccgtggtgttgctgctactggcactgattggcggtatctggacgctacgtaaatcgcgtaagtctacgttgctgcgccatacacgccatgagttagcaaacgatcggcagctgctcgaggaggagtcccgtgagcagtaaagtcgaacgtgaacgacgtaaggcgcaactgcttagccagatccagcaacaacggctggatctttccgccagtcgtcgtgaatggctggagacaacaggcgcttacgatcgtcgctggaatatgctgctaagtctgcgctcctgggcgctggttggcagtagcgtgatggcgatctggacgattcgccatcctaatatgctggtccgctgggccagacgcggttttggcgtatggagcgcctggcgtctggttaaaacgaccctcaagcagcaacagcttcgcggttaacttccctctggccggagccattccggccttatccctcaaattttttgaagatttttgacagttttccttgctaacaatcatcattcaccacgtttatgattctctccatcgacagcaacgacgctaataccgcgccattgcacaaaaaaacaatcagcagcctgagtggcgcagtggagagtatgatgaaaaaattagaagatgttggtgtactggtagcgcgcattttaatgccgattctgtttattaccgctggctggggaaaaattactggctacgcgggtacccaacaatatatggaagcaatgggcgtcccgggttttatgctgccactggtgattctgcttgagtttggtggtggtctggcaatcctgttcggtttcctgactcgcaccacagccctgtttactgcgggctttacgctgctgacggcatttttatttcacagcaactttgctgaaggcgtcaactcgctgatgttcatgaaaaacctgacaatttctggcggattcctgctgctggcaattaccggtccgggcgcgtatagcatcgaccgcctgctgaataaaaagtggtaagcacgcgctatacttaacgataaaaaacgaggaggaagctcctcgtttttgctattggaggagagaaaaatgggtcaactgattgacggcgtctggcatgacacctggtacgataccaaatctaccggcggtaaatttcaacgttcagcttccgcatttcgtaactggctcactgccgatggcgctcctggccccactggcacaggcggttttatcgcagagaaagatcgttatcatctctatgtttcactcgcctgcccgtgggcgcaccgcacgctgatcatgcgcaaactcaaaggactggaaccgtttatttccgtttccgtagtgaacccgctgatgctggaaaacggttggacctttgatgacagttttccgggagcaaccggagacacgctctatcaaaatgaatttctgtatcagctttatctccacgccgatccacactacagcggacgagttactgttcccgtgctgtgggacaaaaagaaccacaccatcgtcagcaacgaatcagcagaaatcatccgcatgttcaataccgcgtttgatgcgctgggcgcgaaagcgggtgattactaccctccagccctgcaaacaaaaattgacgaacttaacggctggatttatgacaccgttaacaacggcgtgtataaagctggttttgccaccagccaggaagcttacgacgaggcggtggcgaaagtgtttgaatcgctggcacgactggagcagattttaggccagcatcgttacctgaccggcaaccagctaaccgaagccgatattcgcctgtggactacgctggtgcgttttgatccggtgtatgtgacccacttcaagtgtgataagcaccgcatcagcgattacctgaatctgtacggttttctgcgcgatatctaccagatgccggggatcgccgaaacagtcaatttcgatcatatccgtaatcattacttccgcagccataagaccatcaaccctacggggattatttcaattggtccgtggcaggatctcgatgaaccgcatggacgagatgttcgcttcggttaaaaaaaggcaccttacgaggtgcctctgataattagctaagtgcatgttgttcatgtcggatgtggcatgaacgccttatctgacatacaaaacattgtacattcaatagattgcataacccgcgcagaccagataagcgtagcgcatctggcgattttgcgcttgtcatcagtcttagcgcgccttcacggcactttattaattccttgaacgaatatttactgccatttcattcacgtctattcttaatttgctgctttaaaaacaagtgattgagcaaaattgaggcaaaaatggactggtatctgaaagtactaaaaaattatgtcggtttccggggtcgtgcgcggcgcaaagagtactggatgtttattctggtcaacatcatctttacgttcgtgctggggctgctggataaaatgttaggctggcaacgcgctggtggcgaaggcatcctgacgacaatctacggtattctggtgtttttaccgtggtgggcggttcagttccgccgcctgcacgacaccgaccgctcggcgtggtgggcactgctattcttaatcccgtttatcggctggcttattatcatcgtctttaactgccaggcgggtacgccaggcgaaaaccgctttggaccagatccaaaactggaaccttaaaacaaatctgctcgccggatgtctgactcatccggcttttatcattatgttgatgaatgaataatttactaatgtttatttaaaatatttcaatgtcgttatataaattacctataaaaaataaccatgtatttatcttaaatatcaaaacctttataacatccgaaaaagaaagatacgaatagcatttacacaatacccggaatagactttcgtcacttttaattaaagggatgtttttatgcagtggtatttgtccgtattaaaaaattatgttggtttctctggtcgcgcacgtcgtaaagagtactggatgtttactctgattaacgccatcgtcggcgctattatcaatgtcattcaattgattttaggtctggagcttccatatctgtctatgctttatttgctggcaaccttccttcccgtccttgcgcttgctatccgtcgcttacacgataccgaccgttcaggtgcctgggccttgctcttttttgttccgtttattggctggctcgtgcttctggtttttttctgcacagaaggtacttctggcagcaatcgttacggaaacgatccgaagtttggttcaaattaatcttagaattggggcgatatttcgcccctttttattaacaataataaatattattttccgttaaaaagtttgggaatttcccgcagacaccaggatttcgcttcccccatactgtcacgacgccaggccataataatatcgatctcgctggtcgattccgggctgacgacacgcaaccgcccttccgcaatatctttttcgaccataggatacggcatcgtcgccacgccaagccccgccagtaatgcctgacgtttatcttcaatcgtgctcaccgttaagcgcggctgtttgtccagcagctgtacggtcaacaccgggcgctcacgagcggtatccgccaccgcaattccacgatatttcacacgcgtcacttcagataacggttccggctcctgatgaatcgggtgatcaggcgcggcaacgtagacgttcattaacgtatagagcttgcgcgagttgatctccgacgaggaacgaaaatgcatatccggcgcgataacaatatccgcccgcccctgctccagccgttcccacgcccccgccagcacttctgtgatgattgccagttgggtattggcttttgccgccagtttgtcgattaacgggaaaaaggcaggtgtcggtaccagcgcttcggtcacaatggtgagatgcgtttcccaaccgcgcgcgagagcttccgcatcagtagtcagtttatctgcggcttccagcaaaacgcgccctcgctccaacaacatcctcccgacattggtgaatttggtacgatggcccgagcggtcaaacagcaccacatccagctcttcttccagtttttgcatggtgtagctaagtgcggaaggcacgcgtcccagctcatccgccgccgccgcaaaactgccccggcgatcgatcgcatccataacccgtagtgcttccagcgttaatgccctttctttggccatttcgttctcattcaggaaatttgaacataccgggcagaatatctggctaacaatgtagcgtccagccccttaccataaaaggaagtaaagagaggtcaagaattatgattactacccgaactgccaggcagtgtggacaagcagactacggatggttgcaggcccggtatactttttcctttggacactacttcgacccgaaattgttaggctatgcctccctgcgtgtgcttaaccaggaagtgctggccccaggtgccgcctttcagccgcgaacctatcccaaagtcgatattttaaatgtgattctggatggagaagcagagtatcgcgatagcgaaggcaatcatgttcaggccagcgccggagaggcgttgctgctctctacccagccgggtgtcagctatagcgaacacaatctcagcaaagacaaaccgttaacgcgaatgcagctttggctggacgcctgcccgcagcgagagaatccgctgattcaaaagctggcgcttaatatgggcaagcagcaattaatcgcctcgccagagggtgcgatgggaagcctgcaattacgccagcaagtgtggctgcaccatatcgtgctcgacaaaggcgaaagtgcgaatttccagttgcatgggccacgcgcgtatttgcaatcgattcacgggaaatttcatgcgcttacgcatcatgaagagaaagcggcgctgacctgcggtgatggggcgtttattcgtgacgaggctaacattacgctggttgccgattccccactgcgcgctttgctgatagatttgcctgtctagttgtttttacagggagatgatgatgagtaaaaaattggccaaaaagcgccagccggtgaagcccgtggtggcgaaagaacctgctcgcaccgccaaaaattttggctatgaagagatgttgagcgagctggaagctatcgtcgcggatgctgaaacgcgtttagccgaggatgaagctaccgcgtaaagacaggttgccggatgcggcgaaaacgccttatccggcctacaaaatccaacaacattaacgaattaaacaacccgtaggccggacaagatgcgccagcatcgcatccggcacgatccccaaaacctggcgtttatctggccttgctcgccataatctcgataatctgccgatccgtttgctgcatcgaatggcttgctaacgcacacaggttggcaatcgactgctcaacatcatgcgccacaatcccttcattgccggtcacggcggtatcatccagcgccattaacaccgctttccacgcagccgaagcactggtcgaaaccttcatcgcgcagctgttcgacgcaccatcgcaaatcatgccgctgacatcgccgatcatactgctgatcgccatcgagatggtttcataacgcccatccaccagccatgccatcccggcggcggcccccattgctgcggtcgttgcggcacacagcgcagacaaacgcggtaactggttatggatgtaaattgcgctcaaatgcgaaagcatcagcgcacgcgccagccgttcatcatccgctccgaagtgttctgctaccaccaccacaggcattgttgcggtaatcccctggttacccgagccggagttactcatagccggaagcgtagcgccgcccatacgcgcatcggatgccgcgctggtacgaatcacaatggatgaagagagatctttcgccagcaaaccgcgctcgcactgtttttccagcgtcgcgccaatatgcagcccccacttaccgctcaaaccttcctgcgataacgcacaatttagcttcgcggaatcgagaataaagcggatcgccgcaaacgggacttcattgacgaacttcaggatctcagccagcgtcgttctggaaagcaccgtcagcggagactcttgctcgccctctgccacacacgcctgctgggtaaacaccacaccatcgtgcgtctcgatatgcacaatgttggtatgcccgccgacgatggtgacacacgcccacttctcaccgttccagactttggcgcgtgagaagaggatttcatcgcaaggttcctggatcttaacggagactttccccgccgccagcagtgctttggcatcggcaattgcctgcgctgttgcgtctttcagcacttccagcccggcgttggcatttccacctaacgcccccagcgccgccgcaatcggcagccccaccattcccgtgccgggaacggtgacgcccagaccgttcttcatcagatttggcgaaacccaggcttctacacgttcaaccggaccttccagttctgccgcagcaaccgccgccgccagcgccagtgaaatcggttcagtacatcccagcgccggttttacttcctcctgaacggcgaggatgtaacgctgccataacggatttaaagtcgaatcaaacatattaaaaaccttaaaatttcaggtaaatcaagaaaatgccaggaacggagaaacacacagcaacaaaccagtgacgataatcaggtacagagacatccctttgtatttgtgcaatgctggtactttgtaaaccagccacgccgggatcaggcaccctaccatgccgaaaatcgggctacagatagaggtgaagctcaacaccggtgcgttcagtacgatggcgctccaggccagcaaaatggcgaaaatcatgatgccgcgctgaacgagattttcgttaatcttctcggcaggcatcttgcgacgcaggatgttcattacgatcccttgcgttgcttcgcgaaagcctaaatagacgccaaagaatgcagtcatgacagcaaagatattgagaatgacgctgaccactttcacccacgctgcgccgtcaccgctaataaactgtgcggcaatcgccagcgcggaaatattctgctcataggcttttaccgcttcgtcatgtcccatcgccagcgtgaacgacacggcgtagaaaaagacggtgacaaacaaaatgccaaacgcgatattcattgcccgcaatgctttatgccgcgccacttcaattgatttttcccgcgagcgataagagatcaccatcggacttaacgtctggataaacagaatcgacgtcagggtaaacggcagcgtaataatggcgtttttcaccagcagccccagcggcggtagcgaaccgacgttatacagatgccacattcccaccatcgacacgcccagcgccgcgaccaccagcagcttggtcagcaccatgccggtcgaaattttgaataacaatttctcgccgcgtgaggagatcgccaccagaatgcaaatcagtaccagaccataaaagggactgtctgacagcaacccttccgtcacgccgaaggtatgcaggtaggaagcactatcgttggtgatggcggtggaatagacgaacatccaaatcaccagcattacgaaatagagcgcacctaacaggatgccccagtttttacctaaataaccgctaatgacgctcgggtaatctttacattctggtgattctgccagcgtattaataaacaatcgctgaaacagatacattgccgggtaaccaatcaccgatgagagcaaaaatacccacaatcccatcaaaccgacctgcaccgggagaaaaacaatccccgcgccaatcgccatcccgatactcataatcacccagccggtgtcagtactgtcgaatttgatcgcttctcgccactcgctctcactcattccagcacgacccgccggggtcgaagcgtctgcaatgacgcctttattcgatgcaatttccataatttctcgctcaatattttgtagggcttattatttttttccgagccgcatcaaggcgatatgcggtctacgtttttgcaggcgagttattagaataaagaaatgatacgcgcgaggtcagagaaaatcttcacaatcaagactttgaaataacggagatggataagaattttctactaaattaatcgcaggagaatattcattctctatttgcggcagatcacaaaaaaaaggtgcacatttgtgcacccaaggatgaaagctgacagcaatgtcagccgcagaccactttaatggccagtcctccgcgtgatgtttcgcggtatttatcgttcatatctttgccggtttcatacatcgtctcgatcactttatcgagtgaaacacgcggtgccgaggtgcggcgcatcgccatccgcgcggcgtttactgctttcacggcattaatggcattacgttcaatgcacgggatttgtacctgtccggcaaccggatcgcaggtcagcccaaggttatgctccatcgcgatttccgccgcattgcatacctgcgccggactgccgcccagtagttcagttaaccctgccgccgccattgaacaggccacgccaatctccccctgacagccgacttccgcgccagagatggaggcgttcattttatacagcgcgccaatagcccccgcggccagaaaatagcgggcaattgaccgctcgtttaccggacgacggaacttatcgtaataagccagtactgccggaataatgccgcacgcaccgttagtcggtgccgttaccacgcgcccgccagctgcgttttcttcactaaccgccagcgcgtacatgttgatccagtcgatgacattcatcggatcgttagagatgttatcgctggaaaccagctgacgacgcagcgctacggcacggcgcggcacattgagcggaccaggcagcacgccttcagtgttcatcccacgttcaataccgtcatgcatcacttgccagatacgggcaaaaccggcgtcaatttccgctttgctgcgcagcgctagctcgttgtgcatcatcagaccagatatagacaggccgttgtaatcacacattttcagcagttcacctgctgagtggaaatcgtaaggtacggacgtttcgacatcgtgcgacaggccgaagtgttcttcttcgacaataaacccgccgccgacagagtaataggttttacttaatagctcttcctgtcccttccaggcagtgatccgcattccgttctcatggcgaggcaacatttcgggatggaagataatgttctttgctacaggaaaatcaacaatatgcgcaccagatgccactggcagccgcccgctgcgcgttactaactctataaatgcagggatctcatcaatgacaacatcctgcggactgtttcctgccagtcccatgatgatggcgacatccgtggcatggcctttgcccgtcagtgacaacgacccgtacagatcgaccacaatatggctcgtcgcggttaataagccgctactttccagccgatcaataaaactttttccggcattcattggccccacggtatgcgaactggagggaccaatcccaattttgaaaatatcgaatgcactaatcatatccacaccctcggattgccgttcagtgaagtggagcggaacgaccttacgaccgtcccgctcacgaggctttacgcactacgtactgcgatggcttcaatttccagcttcacatctttcggcaaacgcgcgacctgcacacagctccgggtcggataggtcgcctgatgctcatcgaagaactgcttatagacttcgttgatggtggcaaaatcattcagatcggtgataaacacggtcatcttgatgatatcgcccacgctcagcccggcagcaaccacgatcgctttgacgttttcgaggcttaaacgcgcctgatcttgcacatcagccgggatctcaccggtctgtgggcaaaccggtatttgcccggaggtgaagaccatgctgcctaaatcaacgccctgaacataagggccgattgcgcctggggcacgttgcgtttcgataatctttttcatacatcctccggcgtcagagcgcctgggtaaaggtacgtgaaataacatcctgttgctgttcacgggtcagtgcgttgaagcgcacggcgtagccagagacacggattgtcaggttaggatatttttccgggtgctcgatggcatccagcagcatttcccgattcattacgttgacgttgaggtgttgaccgccttcgacatccgcttcgtggtggaaatacccatccagcaggccgacaaggttggttttacgtactggatcttctttgcccagcgccgcaggaacgattgagaaggtgtacgagatcccatctttggcgtaggtgaacggcagtttcgccaccgacgtcaatgaggccacggcacctttgcggtcacgaccatgcatcgggttagcgcccggcgcgaacggtgttccggcgcgacgaccgtccggcgtattaccggttttctggccgtacaccacgttagaagtgatagtcagaatcgactgggtagggacggcgttgcgataggttggcagcgctttaattttcttcataaagcgttcaaccaggtcgcaggcaatgctgtctacgcgctcgtcgttgttgccgtactgcggatattcaccgtcgatttcaaagtccaccgccaggccgttttcgtcacggattggtttcacgcgggcatatttgatggcagacagggagtccgtcgccaccgacaggcccgcgatgccgcatgccatagtgcgatagacatcacgatcgtgcagcgccatcagcgaagcttcgtagctgtacttgtcgtgcatgtagtgaatgatattcagcgcgctgatgtactgcaccgccagccagtccatgaagtgatcgaggctgtccatcactttgtcgtaatccagcacgtcgtccatcagcggtgctgttttcggcccgacctgaatcttcagcttctcgtccaccccgccgttaattgcgtagagcagcgttttcgccaggttagcgcgtgcaccaaagaactgcatttgcttaccaatcaccattgggctgacgcagcaggcaatcgcgtaatcgtcgctgttgaagtcagtacgcatcagatcgtcattttcatactgcaaggaagaggtgacgatcgacacctgcgcggcatattttttgaaggcaatcggtaattcttccgaccaaagaatggtcaggttaggttccggtgccggccccatagtgtgcagggtgtgcaaatagcggaaggagtttttggtcaccagcgtacgaccgtccagccccatcccgccgatcacttccgtcgcccagattgggtcgccggagaacagcgaatcaaattccggtgtacgcaggaagcgtaccatacggatcttcatgatgaagtgatcgatcagttcctgtgcctgctgctcattgagtacgccagctttaaagtcgcgctcaatgtagatatcgaggaacgatgccgtgcggcccagcgacatcgcgccgccattttgcgatttcactgccgccagataagcgaagtagagccactgcaccgcttcctgcgcattctgcgccgggcgagagatatcaaagccatatttcgccgccatttcctgaatctgcaacagcgcatgacgatgctctgccagctcctcacgcagacggatggtggcttccagatcctcgcctttttccagacgagactggagatcggcaaattgcagttcgcgttcacgtaccagataactgatgccatacagcgctacgcggcgatagtcaccgataatgcgcccacggccatagccatctggtaaaccggtcagcacgccagatttacggcagcgcagcatatccggtgagtaaacatcaaatacgccctggttatgggttttacgcagatcggtaaacagatattcaaattcactgtccatttctcggccataggcgtggaatgaacttttaatcatattaatgccaccgaacgggtgtagcgcacgtttcaacggcgcatccgtttgcaggccaacaattttttccagcggctggttaatatatcccgcatcatgagcggtaattgtggtggcaatattggtatcgaaatcaaccggcgcgtgggttgcattttcgatacggatgccttccattactttttcccacaattccgtggtggcaggcgtcgcttcggcgaggaaagattcatcgccttcatacggtgtatagttatgttgaataaaatcgcggacattaatttcgtttttccagtccgtacctttaaagccaagccatgcgtcggcgtacagcttatcgctggtatcaatatctaccttcatgaaaaataatctctctacaatacttcaactaaattatgcaaattctgcgggcgcgttaactttgcctaaatgaatggcatccaaagcaatcattttttcttcgttagtcggaataacggcacaaatgacacgcgcattttcactggaaacaattcgctcaccacaggagttagagcgattattcatttctgtatcaatctctaagcctaatacagccaaatgttccatgaccagacgacgaattaagcttgaattctctcctattccgccggtgaatataattccatccaggcgacgtaatgaagctgcgtgtccggcaatatgacgggcaattcggtgaacaaaggttttaattgccagttgcgcgcgttcgtgaccttcatgccaggctttttccagaacacgtaaatccgaagaaagaccggaaatacctaataatcccgactctttattcactacgcgttccaggtcacccaggctctggttggtttggctggcgacccaggacatcgcaccaaagtcgacatcgccactgcgggtacccatcatcaagccttccagcggcgtcattcccattgaggtatcaacactctgaccgttgcgaaccgcgcagattgacgcgccattgccaagatgcgccacaaccaggccggagtcatcttccgccagattcagcagcgaatgtgcgcgctgggaaacatagcggtgcgacgtgccgtggaaaccataacggcgtacacctaactcttcataatatttccacggcaggccgtataaataagcttccggagccatcgtctggtggaaactggtatcaaataccgccacctgagttacgcccggaaataattgctgcgccgattcaataccacttaaattggcgtaattatgcaggggtgccagtggagaaacgcgacggatattatcaatgacttcatcggtaataatggcggactcggtaaaaatactgccgccgtgagcgatgcggtggccaattaaggccacactgtcatttaaattccgtttttccagttcaaatgcaattgccttcaatgcaccttcgtagctgtggtgagccagcggtgctggctctcccccatttacggataagaatgcattttccgagttaataccgtcggcaatacctgacattaatacttcacagtcgctggcatcgagcacggaaaacttaatcgaagacgaaccacagttaataaccaaaacaaccggaaattcattcatctcttttctcatcctgagttacggattaaaacagtttgtatacgatgttcaggatggtcagcagaccaatcacggtaacaaacacgttatccagacgaccacggtatttcgccagagacggcgctttacggatggcatacatcggcaacaggcacagcagggatgcgataatcggtgcgcccatggcttcaatcaggtcaaggatgttcgggttggcgtaggcaacaacccaggtggagcccatgatgaagatcatgctgatagtgttcagtttacccagcgacactttagttttgtcgcctttataaccaaacttcaggaccaggccattcagaccttccagcgttcccagatagtgaccgaagaaagatttgaagatagccacgagtgcgatgatggaagccgcatattccagtgtaatcgcgaacgttgttttggtaccggtcatggacgcaaagtggttagccagataagaaagcactggaatattctgcgctttggcttccgccatgttggccggagacagagtaaacaggcagctaaaggcaaagaacatcaccactgcaaccatcagcatgctggcacgagaaatgatttgggaacatttacgttcggtgaagtcgcgaccgaagtctttctcatactcttcacgcttagaaaccacgaaggaagagacgattggcgagaagttaaaggagaaaaccatgatggaaatccccagccagacagtgatcaggataccgtcatgaccggttaacgacagcgaaccgaggtcaacctggtcgataactgcagagttccagtaagggatcagcgacaaagaaatcagcaccaggctggcgataaacggccataccaggtagctcatcactttaaccatcagatccttaccaaaccagatgacgaaagccatcagcagcaacaggaacagcgccacaaagccgcgattcagcggtgcaaagccgagctggttttcccagaacgtcataaaggtattggtaatagtaacgccataaatccacagcagtgggcaaatcgcgaagaagtacaggaacgtgataaccacgccgccagttttaccaaaatgctcttccaccgtttccgtaatgttgccggaagggttagagccagaaagacacagacgcgccagcgcccggtggcaataaaacgcgatggggtatgccaataccaacatcagaagaatcgggatcagtccgccaaaacctgcgcggatagggaagaacagcaccccggcgccgattgccgtaccaaacaagcctaacgtccatgtggtatctgatttacgccaggacgattgttttgtctggctggatacaatgctatctgaagtactcatatcctatcctcaacgaattaattaagcgtcaacgaaaccggtgatttgagagacgcgagaaagatcgatattgccgccggaaataatactgacggtttttctgttttgaatatattggtctaatttaccgcttaataatgcagcacatgccagagcgcctgcgccttcggtgacgactttattgcgctgaattaaggcaatcatactgtttctgatttcgtcttcgctgaccagcacgatgtcatcgactaattcacgaacgatttcgtaagttaaattacccgggcgggagacatcacaaccatccgccagggtgccggtagttcggtgcgtggttatttctccggagtggaaagaagccgccatgccgtgaacgttttcagactgtacgccaataacacgaatggtcgggttaatagatttaattgccaccgcaataccagcaattaaaccgccaccaccaattggcacaatcacgttatcgacatcatagagatcttccataatttccagaccaatcgttccctggccagcaatcactttcggatcatcgtaaggtgggataaaaatacggccttccatttcgacaatttcgctcactttagcgatagtgtcgttgaagttatcaccatgcagaacgacttctgcggagtagtcgcacgttgccgctactttggattttggcgcaccttttggcatcaccactttaccgtcgatacccagcatcgcgcaggagagggaaaccccttgcgcatggttgcccgcagaacaggccaccacgcctttgcgtttttccgcatcggtcagtgaacttaatttattaaatgcgccacgaattttaaatgaacccgtacgctgcatattttcaaacttcaggaatatttcacctttgcaacgttcactaaaatagttggagcgaggcatgcctgttttataaattcgcccagccagtcgttgtttcgcttcaataatgtcatcaatagcaaccggcagatcgtatgtaatatgcattataaaacctcttcgcctgaattaaatatgtaggtaaccgtaaccgacacctgcaagacagacaggtggattatttatgtttaaataaaaacaaataactaaccaacttctattaattgccttcgtctacacccattataagatgaatactctttggctaattccaccaaaaccgatgctgcttttttaatacgataatttttcgaccataccgcggcatattgtgccacaggtaatgtttcttcaaccggaatagtaataaattgattagaaccaaaaggtgacgtcatatcacaaggaattacagttaagaaatcagcattgagaacaagattataaattgtcacgactgagtcggttttaacgatgttttcaatactgatgccatttctttgtaacgtagtaagcagttcgctgtagtaccccatattagtttgtggcaacacccactgttcgttcttcaacgactccagcgtggtggtgccggtgcatgttcgggacttactggctaccagcacaaactcggactcgaacagcggctcaacatgtaaatcctgaagcttcatttctgcacttaacgtaccaatcgcaaaatccagtcgaccgtcgcggattgccggtaagaacgaagacagttgcgcttcatacatagaaacctgcgctttcgggaacacctctttgaacttgttgatcatccctgacataaaagtaaaaccaatcaatgaaggaaaaccaaatgagacttccaccaccgcctcagaagacataccgcttatctcattaaccatatttttcatttcacgggtaatggattcggaacgggagagtaacaattgaccggcaggtgttaatgttacaccggtatttttccgcaccactaattccacaccaaaataatcttcaatatcgttaatgattttactgacggccggttgagttaaccctaattcttttgcagccgagccgatagaaccacttctaatgacttcctgaaagactaccaggtgctgcgttttcggaagaagaatagtgctcataacgacctacgttaattacctcattgacggcatgaagtgtatcaaaatgaaatgaacaggatatgtgcgaccactcacaaattaactttcaatactttccagagtatcgttattacaattaaatacctttaaatatcaacaagttaaagtataaaaatcagcataaaccctgatttttgtcaaaaaaaatgacggggataaccatattttatggcgataacatcattcgttatgtggttaatacaaaaaaggggctgagaccatatttcaagcaattaccggataattaccaggcaaaatttgagttaaatttaatgagcaagttctcaaattttattataaataaaccattttcagtgataaataatgcggcatgtcacattttttcacgctatttgttggagaacaaacatttattttatcaatattttaaaatttcgaatacatgtattgatcatctcgaacaattgattaacgtcaactttttctcttctgacaggacgtcattttgtgaatgcaatcgttttccataaattcttctcccctcataggcgacgaatagcattttgtgttgaggatcacaaaacgaataattgctgatcgccgcgataaggtcagacaaagacaacaagggaaattttcacagagcttttgatcggcgtaggccacagaatgttgcttcgtttactgtaacgccgggtaaatgagcgttttttgatagtgcgaaagaaccctgcgaggaaaataagcatctattattgtttgtcatgatgacaaggcaggcatcaatgaaaggcttcccaattgcgcatatttttcacccttcaatcccgccaatgcacgcagtggttaacaatcacaatagaaatattgattattggacggtaaaaagaaagtttgcagaaattgtctccaccaatgacgttaataaaatttacagtataagtaatgaactgcggagagtattatctgcaataactgcattgaatttctatcatggcgatgttccttctgtcatgatccgaatccaaccggaaaatatgagtccattcattatagatatttctacaggagaacatgatgattatatcatacaaacattagatgtaggcacttttgcaccttttggtgaacaatgtacttgctcagccgtcaataaaaaagagctggaatgtattaaggagacgatttctaagtattgtgcaaaattcacccgaaaagaagccatcttaaccccccttgtgcactttaataaaaccagcattacttcagattgttggcaaattctctttttttcacccgatcattttaataatgatttttattgattatttataaaggataaaataatgttccctgtttcatcaattggtaatgatattagtagtgatttagtccgtcgaaaaatgaatgaccttcctgaaagcccaacaggaaataacctcgaagcactagcaccaggtatagaaaaactaaaacagacctctattgaaatggtcactttacttaacacgttacaacctggtggaaaatgcattatcactggtgattttcaaaaagaattagcgtacttacaaaatgtaattctttataatgtctcgtctcttcgtctggattttttaggttataacgcccaaattattcaacgatcggacaatacttgtgaacttaccattaatgaaccgttaaaaaaccaggaaatatccacaggtaatatcaatattaattgcccattaaaagatatttacaatgaaatcaggaggttaaacgtaatttttagttgtgggactggagatatcgttgatctatcctctctggacttacgtaatgtcgatttagattattatgatttcacagataaacatatggctaatactattttaaatccttttaaattgaattcaacaaattttactaatgccaacatgtttcaggttaattttgttagttcaacacaaaacgccacaatctcctgggattatttactaaaaataacgcctgttttaataagcattagcgatatgtattctgaagaaaaaatcaagtttgtcgaaagttgtttaaatgagcctggagacattaccgaagaacaattaaaaattatgagatttgcaattataaaatctataccaagggcaactcttacagataaattagaaaatgaattaacaaaagaaatatataaaagctcatcgaaaatcatcaattgcttgaacagaattaaattaacagagatgaaagaattctcatcagaaaaaatatatgattacatcgatataatcattgaagattatgaaaataccaaagaaaatgcttatctggtcgtcccccaaattaattatactatggatttaaacatagaagactctagctcagaagagttactttcagataataccctcgagaaagacgaaaattctccggacaatggctttgaggtcggggaatataacacatatgaagcatataactcagagaagcaatattttaccagagaggactatacgtatgattacgaccttttaaatgcaatatagacttaataacttcttacaaagtctattattaataccgtagatatttattcatcttaccctgtgcaccaaaagcaaaaactcactgacgcgggtttgaaactgatggcaaccgcaaaaatgcctgatgcgctacgcttatcaggcctacgccatctctgcaatatattgaatttgcgtgcttttgtaggcaggataaggcgttcacgccgcatccggcatgaataaagcgcactcaacaatctgaaacccgccggaacggtttattacgtacatcaggtaaaactgaccgataagccgctttcttttgggtatagtgtcgtggacagtcattcatctttctgcccctccaaaagtaaaaacccgccgaagcgggtttttacgtaaaacaggtgaaactgaccgataagccgctttcttttgggtatagtgtcgtggacagtcattcatctttctgcccctccaaaagcaaaaacccgccgaagcgggtttttacgtaaaccaggtgaaactgaccgataagccgctttcttttgggtatagcgtcgtggacagtcattcatctttctgcccctccaaaagcaaaaacccgccgaagcgggtttttacgtaaatcaggtgaaactgaccgataagccgggttctgtcgtggacagtcattcatctaggccagcaatcgctcactggctcaagcagcctacccgggttcagtacgggccgtaccttatgaacccctatttggccttgctccgggtggagtttaccgtgccacggactgttaccagccgcgcggtgcgctcttaccgcaccctttcacccttacctgatcccgcttgcgcgggccatcggcggtttgctctctgttgcactggtcgtgggtttcccccccaggcgttacctggcaccctgccctatggagcccggactttcctcccctccgcccgtctcccccgaagaggacgacgacgaagcggcgactgtctggtcagcttcggcgcgcagtatagagggtttgcgcgcccttgtcaccccgcgttgcgcattccaatcgccagtgtcgcggcgatattacgtgaagcacggcagatattgtcataagccccgcggaatgcttcgtccaacgtacctatgctggtcaatacgctgaagaccgcatcaatgccatgctgatgtacaacgccaacatcatcggtcaggctacccgcaatgccaatcaccggtttatggtacttcttcgccacgtttgcgacaccaatcggtaccttcccgtgaatactctggctgtcaatacgcccttcaccggtgatcaccagcgtacaatcgtgaatatgttcctccagattcagcgccgtagtgacgatttcaataccacttttcagttccgcaccaagaaacgccattagcgccgcgcccataccacccgcagctcctgcaccggggacatctttcacatcaacatgcagcgcttttttaatgacctcggcatagtgagagaggttattgtccagctcaacaatcatcgcttcactggctcccttttgtgggccaaagatgcgcgatgcgccgttatcgcccaccagcggattggtgacatcacaagcgacgcgaatgacgcaatcttttaagcgcggatcgaggccggaaatatcaatatcattcagagtattaagactaccgccgccaaaaccaatttcattgccgttggcgtcgcataatttcgcccccagcgcctgtaccatgcctgcgccgccatcatttgtagcgctgccgccaatgccgataataatgtttgtcgcaccgctctccagcgcctgcaggattaactcgcctgtgccgcgtgaagtggtcacgagtggatcgcgtttttccgcaggtaccagctccagcccactggccgccgccatttcaataaacgcggttttgccatcgccggagatcccccaactggcattcactttctcgcccagcggccctgtaacccaggcgtgacgttcagccccctgggtggctgcaatcatcgcttccaccgttccttcgccaccgtcggcaaccggaacagaaacgtactgtgcatcaggaaaaatttcccgaaatcctttttctatcgcctgcgcaacctcgctggcagataaactttctttataagagtctggggcgattacgattttcatacctatgcctgttaccacatgacgccggagggcgtttctcttattcggcctggattccaggcccggattgcaatacgccatccgggcacgacgtcattaacgagtaacttcgactttcgccagtttttcgtagtagcacgccagggcgctatgatccgccgttcctaaaccatctgctcgcagtgcctgcatcatctccataaccgcagctgtgagcggcagttgtgcgccgacgccgtgagaagtatccagcgcattcgccagatccttaatatgcagatcaatacggaagcccggcttgaagttgcggtccatcaccatcggcgctttggcatccagcacggtactgcccgccagtccaccgcgaattgcctgataaaccaggtccgggttaacgcccgctttagttgccagcgttaacgcttctgacatcgcggcaatattcagcgccacaatgacctgatttgccagtttggtgacgttacctgcaccgatttccccggtatgcaccacggaacccgccatcgctttcatcaaatcatagtatttgtcgaaaatagccttgtcgccgcccaccatcactgacagcgtaccgtcgatggctttcggttcaccgccgctcaccggagcatccagcatatcaatgcctttcgctttcagcgcttcgctgatttcacggcttgccagcggtgcgatagaactcatatcgatcaataccgtacctggcttcgcgccttcaataatgccattctcacccagcgccacctctttcacatgaggggagtttggcagcatggttatgatgacgtcgcactgttcagcgatcgctttagccgtagacgctgtttctgcacctgcagcaatcacgtcagcaatagcttctgggttacggtcagcaaccaccagcgagtaacctgctttcagaaggtttttactcattggtttacccataatccccaggccaataaaaccaactttcatagtcatatcaatcatctctcttgttgcggtggtggttattttttaaaggtatcagccagtttctgagtggcagagcggaagacgccgagatcgctgccgacagccacaaacgtcgcgccccattccagataacgacgcgcatcggcttcgaccggcgcgaggataccgctgggtttgccgtgcgcgctggcacggttaaaaatgtgctgaattgctttttgtacatccgggtgtgatgcattgccgagatggcctaatgccgcggccagatcgctggggccgacgaagatgccgtctacgccttcggtagcggcaatggcatcgacgttatctacgccctgctgactttctatctggaccagaatagtgatgttcttgttcgactgagcgaaataatccgccacggtgccaaacatattggcgcggtgagaaacggagacgccgcgaatgccttccggtgggtaacgggttgatgccaccgccagctctgcttcctcttttgtttctacaaaaggaatcaggaagttatagaaaccgatatccagaagacgcttaataattaccggctcgttggtcggcactcgcactactggcgcgctggcgctgcctttcaaggccattaactgcggaataaacgtggagatatcgtttggcgcatgttcgccatccagcaccagccagtcaaacccagccaaaccaagaacttcagtgctaatcgggttagagagtgctgaccagcaaccaatttgtacctgtttcgcagccagtgcggctttgaatttattcgggaaaacatcgttattcatcgcttatacctttgcttatttctgcaattccatacgtttaatgtcgccaactacgaagaggtagcagaccatcgccatcagcgctgaacatcccacgaaaaccagtgctgcattgaaggagtgcagttcacttaccaggtagccaatcaccagtggagtgacaatggaggcaacattgccaaagacgttaaagacgccgccgcagaggccaacaatctctttcggcgcggtgtcagaaatcaccggccagcccagcgcaccaaatcctttgccaaagaaagccagcgccatcagcatgaccaccagcgtggtgttgttggtgtagttacataagatgatggtggaagccagcaacattcccagcacaatcggtagcttacgtgccagggtcagggataaaccgcgtttgatcagataatccgagaagacacctcccagcacgccgcccgcaaaaccacacagtgctggaatcgaggcgaccagacccactttcagaatcgacatgcctttttcctgcaccagataaatcgggaaccaggtgaggaagaaccaggtgatggtgttgataaaatattgtccgaaaaatacgcccagcatcatgcggttagagagcaattgcttgatgtaatgcagtttgggtccgcttgctgccgcactgcccggctttttgtggtccatatcgaccaccgcgccattttcagagataaacttcagctcttccgcagacatacgtgggtgatctgtcgggttatgaatcaacttgatccacagcgccgtcagcacaaaaccaatcacccccataacggtaaagacgtgctcccagccccaggcgaaagtcagccagccaagcagcggcgaaaagagcgccagcgagaaatattgcgccgagttaaagatggcggaggcagtaccacgttctttcgtcgggaaccaggcggcgacaattcgggcgttcgccgggaatgatggcgcttccgagaagccgagcataaagcgcataaagaacatggagatccctgcccaggccagcgggaacatatcaacaaagccttgcaggaaggtgaatagcgaccagaaaaagaggctgtaggtgtaaacttttttcgagccaaacttatcaagcagccagccgccggggatttgcatcagcaagtaggcccagccaaaagcggagaagatgtaacccatcgaaaccgcacttaactgcaactcttttgccacttcggtaccagcaatagacagcgttgcacgatcggcgtagttaacggcggtaacaataaaaataatcagtaatattaaatagcgggtatgcacgcctttctttttttcgtcaacggtgtccagaatcattttatttacctcgggtacttatgctgatttttattattatggggaaggtgttatttatgagtttcatttatgccgtaacgacaatgaactcgggaattagtataagcagcgcgagaataataatcattgtgcaaatgctaatttaattaatactatttaaatattattttgagcatatgcacataaggttgcgcgctaaagcacagatttgcgctttaccttaccgggcggcactgcaatccctgaaatgattgacattgatcacatttctgcgtttaaactcctgacattcttatttcacccaatgaagtcatttatttttaaatgagaccaggtcctcattttaataacccctggctggagaatattgcacaatggccaacatcgaaatcagacaagaaacgccaactgcgttttatataaaagttcacgacacagataatgtggcaattattgttaatgataatggcctgaaagcaggaacgcgttttccggatgggctggaattaattgaacatattccccaggggcataaagtcgcattgctggacattccggctaatggtgaaattattcgttatggcgaagtgattggttacgccgtgcgtgcaatcccacgcggaagctggatcgacgaatcaatggttgtactaccggaagcgccgccgttacacacgctgccactggcaaccaaagtcccggaacccttaccgccgctggaaggatacacctttgagggctatcgcaatgccgatggcagcgtgggcaccaaaaacctgctcggtatcaccaccagcgtccactgtgtggcaggcgtggtggactatgtagtaaaaatcattgaacgcgatctgctaccgaaatacccgaacgtcgatggcgtggtggggctgaatcatttgtacggttgtggcgtggcgattaacgcaccggcggcagttgtacctatccgtaccattcacaatatttcgctgaatcctaactttggcggcgaagtaatggtgattggcctgggttgtgaaaagttgcagcctgagcgcctgctgactggaacggatgatgtgcaagctattccagtagaaagcgccagcattgtcagtttgcaggatgaaaagcatgtcggttttcagtccatggtcgaggatattttgcagatcgccgaacgccatctacaaaaactgaatcaacggcagcgagaaacctgcccggcttcagaactggtcgttggtatgcagtgcggtggcagcgatgcgttttctggtgtaacggcaaacccggcggttggctatgcgtctgatctactggtgcgctgcggcgcaacggtgatgttttcagaagtaacggaagtgcgtgacgcgatccatctgctgacaccacgcgcagtgaacgaagaggtcggcaaacggctgctggaggagatggagtggtacgataactatctcaatatgggaaaaaccgaccgcagcgccaacccttcgccgggcaacaagaaaggcggtctggcaaacgtggtagagaaggcactcggctccattgctaaatcgggtaaaagcgcaattgttgaagtgctgtcgcccggtcaacgcccgactaaacgcggattaatttacgccgcgacgccagccagcgattttgtctgtggcacgcaacaggtggcttcgggtatcacagtgcaagtgtttacgaccggtcgtggtacgccgtacggcctgatggcggtacccgtcattaaaatggcaacccgcaccgagctggcgaaccgctggtttgatttaatggatattaatgcgggcaccatcgctaccggcgaagaaactattgaagaggtgggctggaagttgttccactttattctcgacgtcgccagcgggaagaagaaaaccttctcggatcaatgggggctgcataaccagctggcggtgtttaacccggcaccggtgacctgatttcttttggaacgtccctcgcaaaacatggccttagtgccatgtttttattgtttaaagcccccacgtccattaataatgcatttgcattaccttagttcaagcttataatttgagcagaaaacaggctgtaaaaggacagtgaatcatgcccgctaatgctcgctctcacgctgtactgaccactgaatcaaaggtcacgatacgcggacaaacaactatccccgcgccagtgcgtgaggccttaaaactgaagccaggccaggacagcattcattacgaaattctgcctggtgggcaagtatttatgtgccgactgggagatgaacaggaggatcatactatgaatgcatttttgcgttttctggatgcagatatccagaacaacccgcaaaaaactcgtccattcaacattcaacaaggaaagaaacttgtcgctggcatggacgtcaacattgatgatgagattggcgacgacgaataatggattttccacaaagggttaatggttgggcgctatatgctcatccctgttttcaggaaacctacgacgctttagttgccgaagtcgagacattaaagggaaaagatcctgaaaattatcagagaaaagccgccacaaagttattggcggtagtccataaagtgattgaggagcatatcacggtcaatccatcatcaccggcattccgtcatggcaagtcgttaggctctgggaaaaataaagactggtcacgggtaaaatttggtgctggtcgttatcgtctcttctttcgttatagtgaaaaagagaaagtcatcattctgggatggatgaacgatgaaaacactctgcgcacctacggtaaaaaaacagatgcctataccgtattcagcaaaatgttaaaaagaggacatcctcctgccgactgggaaaccctcacccgagaaacagaagaaacccattgatggtgttcacaatgcccgccgaacgcattcgtgttgaccagcgggcatcctttctcactccccgaccagaatcacttcaaccccagcctttcgcagtccttccaggctatccgcaggaatgccttcatcaacaatgatcatgtcgatacgttgagtatcaatgatcttatgtaaactggaacgattgaacttactggaatcggtgaccacgatgatccgttccgcaacttcgcacatccgacggtttaaacgagcttcatcttcattatgtgtgctgacgccgcgctccagatcgatcgcatctacaccaagaaacagcatatcgaagtggtaattttgcagcgattgctcagcctgatcgccgtaaaaagattgcgactgacggcgcaaatgcccgccggtcatcagcagctcaacgccttccgcttccagcaacgcattagccacgttcataccgttggtcatcgcaattacgtcagtgtgcttgcgcatcagacgagcaatctcaaaagtggtggtcccggaatcgaggataacccgatgacctggctgaatcaactcaacggcagctttcgcaacgctgcgtttcatcgcggtgttcagtgcgcttttatcttccactgatggctcgactgacggcgtcgtgctatcgcagatcaacgcgccaccataggcacgcacagcgatcccctgcttttccagaaacgccagatcgttgcggatcgtcacagtagatacgccatacaatgccgacagatcgttaacctgcacactcccttgctgtcgcagacgctgaatgatctgttctcgtcgctcgctggtgccagtcactcgcttctcacctgaagcgtcggtattactcatagtaagtcctttcgtaaaactttcgtttcatttcgttttgcctattaacgcctttctattaagcaaatgcaagcccaccttgcccattgacgcaagctactctcgtttcagtgactttcattatgtttcttttgtgaatcagatcagaaaaccattatctttcgttttatttttatctcaccatgacgcagtatcaactgaaacaaaacgaaagattaatatcgcagtaatctgaactggagaggaaagtgaaacatctgacagaaatggtgagacagcacaaagcgggcaaaacaaatggaatttatgccgtttgttccgcacatccgctggtgctggaagctgcaatccgctacgccagtgcaaaccaaacgccgttactgattgaagcaacctccaatcaggtagaccagttcggcggttataccggaatgacgcccgccgattttcgcggctttgtttgtcagctcgccgactcgttgaatttcccgcaggatgcgttgattctgggtggtgaccatctggggccaaaccgctggcaaaacctgccggccgctcaggcaatggccaatgccgatgatttgattaaaagctacgttgcggcaggattcaaaaaaatccaccttgattgcagcatgtcctgtcaggacgatccgattcccttaactgatgacatcgtggctgaacgcgccgcccgtctggcgaaagtggcggaagaaacctgtcttgaacactttggcgaagccgatctggagtatgtcattggtaccgaagtgccggtacctggcggcgcgcatgaaaccttaagcgagctggcggtcaccacgccggatgccgcccgcgccacgctggaagcccatcgtcacgcctttgaaaagcaaggtttgaatgccatctggccacgcatcattgccctggtggttcaacccggcgtcgaattcgatcacaccaacgttattgattatcagcccgccaaagcgagcgccttaagccagatggtcgaaaactacgaaacgctgattttcgaagcgcactctaccgattatcaaacgccgcaatcgctgcgccagctggtgattgaccactttgccattctgaaagttggcccagcgctgaccttcgccctgcgtgaagctctgttctctctggcggcgattgaagaagaactggtgccagcgaaagcctgttctggtctgcgtcaggtgctggaagacgtgatgctcgaccgcccggaatactggcaaagccactaccacggtgacggcaacgcgcgtcgtctggcgcgtggttatagctactcggatcgcgtgcgctattactggccggacagccagattgatgacgctttcgctcatctggtacgtaatctggcggattcaccaattccgctgccgctgatcagccagtatctgccgctgcagtacgtgaaagttcgctccggcgagctgcagccaacgccacgggaactcattatcaaccatattcaggacatcctggcgcagtaccacacagcctgtgaaggccaataagcaaaacaaagaggaacacgctatgccaaatattgttttaagccggattgatgaacgcttgattcacggtcaggtcggcgttcaatgggtcggatttgcgggggcaaatctggtgctggtagccaacgatgaggttgccgaagatccggtacaacaaaacctgatggaaatggtactggcagaagggatcgccgtacgtttctggacgctgcaaaaagttatcgacaacattcatcgcgccgccgatcgacagaaaatcctgctggtttgtaaaacacccgccgatttcctgacgctggtgaaaggtggcgttccggtgaatcgcattaacgttggcaatatgcactacgccaatggcaaacaacaaatcgccaaaacggtttctgtggatgcgggcgatatcgcagcatttaacgacctgaaaaccgctggggtggaatgcttcgttcagggcgtcccgacagagcctgctgtggacctctttaaattactttgagggattcatcatggaaatcagcctgttgcaggcatttgcgttgggcattatcgcctttatcgctggcctggatatgtttaacggcctaacccatatgcaccgcccggtggtcctcggcccgttggtcgggctggtacttggcgatctgcataccggaattttaaccggcggtacgctggaactggtgtggatggggctggccccgctggcgggcgcacagccgcctaacgtgattatcggtactatcgtcggcacggcgtttgccattactactggcgtgaaacccgatgtcgcagtaggtgtcgccgtacctttcgctgtcgcagtacagatggggattaccttcctgttctcggtgatgtccggcgtgatgtctcgctgcgacctggcaacaaacccgcgccgcatttgatgctggtgccgacggcctggtgcattgctataacgggatgacaggtttacatcaccgcgaaccgggaatggttggcgcgggattaacggacaagcgcgcctggctggaactgatagccgatggtcatcatgtgcatccggcggcaatgtcgctgtgttgttgctgtgcgaaagagagaatcgtactgatcaccgacgcgatgcaggcagctgggatgccggatggtcgctatacgttatgtggtgaagaagtgcagatgcacggtggcgttgtccgtaccgcgtctggtgggctggcgggcagtacgctgtctgttgatgcggcagtgcgcaatatggtcgagttgacgggcgtaacgcctgcggaagccatccatatggcgtcgctgcatccggcgcgaatgctgggtgttgatggtgttctgggatcgcttaaaccgggcaaacgcgccagcgtcgttgcgctggatagcgggctacatgtgcaacaaatctggattcagggtcaattagcttcgttttgatagtttgctcctttattgggccttcacttcccccgtaaggcctttctttttctttcgttttgatctgtgcagcggtgtcggatgcgacgctaacgcgtcttatccgacctacagttggtgaccgcaaggccggataaagcgtttgcgccgcatccagcaatcccttttgcttcctttatcttttctttcaacgatcacaaatttcgttttatttcttttttctccattgaactttcagtttcttttctatagattttaatcaacgaaagacatcaccaagtgaaatgaaacgaaaggcaagtgaaagcgacaacgcccgacgtcaagttcatcagactaaggattgagttatgccagaaaattacacccctgctgccgccgcaaccggtacatggactgaagaagagatccgccatcagcctcgcgcatggatccgttcactcaccaacatcgacgcgctacgttccgcgctcaataacttccttgaaccgttactgcgcaaagagaatctgcggatcatcctgaccggagccggaacgtcggcatttatcggtgacatcatcgcgccgtggctcgccagccataccggtaaaaacttcagcgccgtaccgaccaccgatctggtcaccaatccgatggactacctgaacccagctcatccgctgctgttgatctccttcggtcgatccggcaacagcccggaaagcgtcgcagccgtggaactggcaaatcaatttgtaccggaatgctatcacctgccgatcacctgcaacgaagcgggcgctctttaccaaaacgcgatcaacagcgataacgcgtttgccctgctgatgcccgcagaaacgcacgatcgcggctttgcgatgaccagcagcattaccaccatgatggccagctgcctcgcggttttcgcacctgagacgatcaacagccaaaccttccgcgacgtggcggatcgttgccaggcgatcctgacctcactgggcgatttcagcgaaggtgtgtttggttacgcaccgtggaaacggatcgtttatctcggtagcggtggcttacagggcgcagcacgcgagtcggcgctgaaagtgctggaactgacggcgggtaaactggcggccttttatgattctccaaccggattccgtcatggaccaaaatcgctggtcgatgacgaaacgctggtggtggtatttgtctccagccacccttacacccgtcagtatgatcttgatctgctggctgaacttcgccgtgacaaccaggcaatgcgtgtaatcgccatcgccgcggaaagcagcgacatcgtcgctgccggtccacatatcatcctgccaccgtcacgtcactttatcgacgttgagcaggcattttgcttcctgatgtacgcccagacgtttgcactgatgcagtcgctgcacatgggcaatacgccggataccccatcagccagtggcaccgttaaccgcgtggtgcaaggcgtaatcattcatccgtggcaggcataagaggatcgcattatgagcattatctccactaaatatctgttacaggacgcccaggccaatggctacgcggtgcctgcttttaacattcataacgccgagacgatccaagcgatcctcgaagtgtgcagtgaaatgcgatcgccggtgatcctcgccggaacgccggggacctttaaacacatcgcgctggaagagatctacgccctgtgtagcgcctattccacaacctacaacatgccactggcgctgcatctcgaccaccacgaatcgctggatgatattcgccgtaaagtccacgcaggtgtgcgcagtgcgatgatcgacggcagccacttcccgtttgccgagaacgtgaagctggtgaaatcggttgttgacttctgccactcacaagattgcagcgtggaagcagaactgggccgcctgggcggtgttgaagatgacatgagcgttgacgccgaaagtgcattcctgaccgatccacaagaagctaaacgctttgtcgaactgactggcgtcgacagcctggcggtagcgattggtacggcgcacggcttatacagcaaaacgccgaagattgatttccagcggctggcggaaattcgtgaagtggtggatgttcctctggtgctgcatggtgccagcgatgttccggatgaatttgtccgtcgcactattgaacttggcgtcacaaaagtgaacgttgccacagaattaaaaatagccttcgctggcgcggttaaagcctggtttgcggaaaatccgcagggtaatgatcctcgttattatatgcgcgtcggaatggatgcgatgaaagaagttgtcagaaataaaattaatgtctgtggttcagcgaatcgaatttcagcataatcattagttttttatgatttatcccaatgtacttcccgattaatatcggggagtgccttaatggaaaaggagataactaaaccttaataaatacatcactacaatatcgcaacaataatatatttaaaaaaattatattattcaactttatggtgaggattacacaatgaccagtccaaatattctcttaacccgtattgataaccgtctggttcacggtcaggttggcgtgacctggacatccaccatcggtgcaaatctgctggtagtcgtggatgatgttgtcgctaacgatgatattcaacagaaattaatgggtattaccgcggaaacctacggctttggcattcgtttctttactatcgaaaaaaccattaacgtcatcggcaaagctgcaccacatcagaagatcttcctgatttgccgtacgccacaaacggtacgtaaattggtagaaggtggtattgacctgaaagatgtcaacgtcggcaatatgcatttctcggaagggaaaaagcaaatcagcagtaaagtttatgtcgatgaccaggatctcacggacttacgttttattaaacaacgtggcgtgaatgttttcattcaggacgtccctggcgatcaaaaagaacaaatccctgactaaatctaaaatcgccttaatattggtttgaggtaataaaaatgcatgaaataaccctacttcagggattatccctggcggcgttagtttttgttctggggattgatttttggctggaagccttatttttattccgcccgataatcgtttgtaccctaactggcgctattctcggtgatattcagactggcttaattaccggtggtctgacagagttggctttcgccggattaacccctgcaggtggtgttcagccgcccaacccgattatggcgggtctgatgaccaccgtcattgcatggtctacgggcgttgatgccaaaacagcaattggtcttggcctgccgtttagtttgttaatgcagtacgtcattctgttcttctattccgctttctcattatttatgaccaaagccgataaatgcgcgaaagaggcggatacggcagcgttttcccggcttaactggacaacgatgctcatcgtcgcttcagcgtatgcggtgattgctttcctctgtacttacctggcacagggggcgatgcaggcgctggtgaaagcgatgcccgcctggctgacccacggctttgaagtggctggcggtattctgcctgccgttggttttggcttgctgctgcgcgtaatgttcaaagcgcaatatatcccttacctgatcgccggtttcctgtttgtttgctacatccaggtcagcaacctgttgccggttgccgtactgggcgcaggctttgcggtgtatgagtttttcaatgcgaaatcccggcagcaagcgcaaccgcagcccgttgccagtaaaaatgaagaagaggactacagcaatgggatctgaaatcagtaaaaaagatatcacccgtctgggctttcgttcgtcgctgctgcaagcgagctttaactacgaaaggatgcaggcgggcggttttacctgggcgatgttgccgatcctgaaaaagatttataaggacgacaaaccgggcttaagcgcggcgatgaaagataacctcgaatttattaatacccacccgaatctggtcggattcctgatggggttattaatttcgatggaagaaaaaggagaaaaccgcgacaccattaaaggcctcaaagtggcactgtttggcccaatcgccgggattggcgatgcgattttctggtttactttgttgccgattatggcgggaatttgctcatcatttgccagccagggaaacctgctggggccgattctatttttcgccgtttacctgcttatctttttcctgcgcgtcggctggacccacgtcggttattcagtcggcgtgaaggcgatcgataaagtgcgagagaactcgcagatgattgcccgttcggcaaccatcctcgggatcacggtaatcggcgggctgatcgcttcgtatgtgcatattaacgtggtgacatcgtttgccatcgacaatacccacagcgttgcgctgcagcaggatttcttcgataaagtcttcccgaacattttaccgatggcctacaccctgctgatgtattacttcctgcgggtgaaaaaagcgcatccggtgctgttaatcggcgtgacttttgtgctctctattgtttgttccgcattcggcattttgtaaatggaacgaggcactgcgtctggtggtgcctctttacttaaggaatttcatcctgtgcaaacccttcagcaagttgaaaactatacggcgttaagtgaacgtgccagcgaatatttattggccgtgatccgtagcaaaccgaatgccgtgatttgcctggcgaccggagccacgccattactgacgtatcattatctggtagaaaaaatccaccagcagcaggttgatgtcagccagctcaccttcgtgaagctcgacgaatgggtggatctgccattaacgatgccaggcacctgcgaaactttcctgcaacagcatatcgtgcagccgctggggctacgtgaagaccagctcatcagctttcgctccgaagagataaatgagacagagtgcgaacgggtaacgaacctgattgcgcgcaaaggcggtctggatttatgcgttctcggattggggaaaaacggtcatcttgggctgaacgaaccgggagaaagcctgcaaccggcctgccatatcagtcaacttgatgccagaacacagcaacatgagatgttaaaaaccgcgggtcgccccgtgactcgtgggatcaccttaggcctgaaggatattctcaatgcccgcgaagttttgttactggtgactggcgaaggaaagcaggatgcgacagatcgttttctcacggctaaagtctctaccgctatcccggcttcatttttatggctgcacagtaactttatttgtttaattaacacctaaccagatgaaaaatttgctcaaaatgtttaaattaacttatgtaacagtcacgcattatattaaataacatttgactgggttgaacataacgccgatagcaaaaggagttatgttcaacaatttaattttagatatacatataacttgttctattaataaatcacctcgtattctgactcgccccctggcgcagcaaagtcaggcatttatactcttttgaatacatagaaaattgatatcaatataatgaaaatatcaaatatttgcatataaatataatcttaaagttcagtctatttaatgttcaatgaaatatttctgcctgtataatctttaaagatgttgaacatatattcacattaaatatgattatgtacttgttacaaggataaggttatatatgaataaagttacaaaaacagctattgcgggcttacttgcgcttttcgcaggtaatgccgctgcaaccgatggtgaaatagtttttgatggcgagattttaaaatccgcttgtgaaatcaatgactctgataagaaaattgaagttgctcttggtcactataatgccgaacagtttcgtaatattggcgagcgtagcccaaaaattccattcactattcctttagttaactgcccaatgactgggtgggagcacgataacggcaacgttgaagcgtctttccgtctatggctggaaacgcgagataatggcaccgtccctaacttccctaatctggcaaaagtaggctcttttgctggcatagcggcaacaggtgtgggtatccgtattgacgatgcggaaagcggaaacattatgccactgaatgctatgggcaatgataacacggtttatcagatcccggcggaatccaatggtattgtcaatgttgacctcatcgcttactacgtatcaaccgtagttccatcagaaatcaccccaggggaagcagacgctatcgttaacgtaacgctggattaccgttaatacgttagggcgttatctgacctgtcagataacgcccttttccttcctctttctcgttgtatcaggttgaaaaataactatgtcaaaacgaacattcgcggtgatattaaccttgttgtgtagcttctgtattggccaggcgcttgcaggaggaatcgttttacagcgaacgcgagtgatctatgatgccagccgcaaagaggctgcgttacctgtcgcaaacaaaggcgcagaaacgccttatttactgcaatcatgggtagataatatagatggtaaaagccgtgccccatttattataaccccaccgctatttcgtcttgaggctggcgatgactcatcactgcgaattattaaaacagctgataacctgcctgaaaataaagagtcgctgttctacattaatgttcgtgccattccagcaaagaaaaaatcagatgatgttaatgctaacgagttgacgctggtatttaaaacacggatcaaaatgttttatcgccccgcacacctgaagggacgggtaaacgatgcgtggaaatcactggaatttaaacgtagtgaccattcactcaatatatataacccaactgaatattacgtcgtatttgccggactggcagtcgataaaaccgatctcacaagcaaaattgaatatatcgcgcccggagaacataaacagttaccacttcctgcatctggcggaaagaacgtgaaatgggctgcgatcaatgattatggcggcagttccgggacagaaactcgtccactgcaataaaaaatataaaaacacaggtcatcagggaatgccacaacgacaccaccagggacataaacgcacaccgaaacagttggcgctcatcatcaaacgttgtttgccgatggtgctcactggcagcggcatgctttgcactaccgctaacgccgaagagtattatttcgaccccattatgctggaaaccacaaaaagtggtatgcaaacaaccgatctgtcgcgtttttcaaaaaaatatgcacaactaccaggaacttatcaggttgatatctggctgaataaaaagaaggtttcacagaaaaaaattacatttaccgccaatgcagagcaacttctgcagccacagtttacggtagaacaactacgtgagctgggtattaaggtggatgaaatcccggcgctggctgaaaaagatgacgatagcgtgatcaactcgcttgaacaaatcattcccggtacagctgctgaatttgatttcaatcatcagcaacttaatttgagcattccccaaattgcactgtaccgtgatgcaagaggttacgtctccccttctcgttgggacgatggtataccaacgctgtttaccaactactcgtttacaggttctgataaccgttaccgccagggcaatcgtagccaacgacagtacctgaatatgcaaaatggtgctaattttggcccctggcgattacgcaactattccacatggacacgcaacgatcagacatcaagctggaataccatcagtagttatttacaacgtgatatcaaggcgttgaagtctcagttgcttctgggagaaagcgccaccagcggcagtattttttccagctacacctttactggcgtgcaactcgcttccgacgataatatgttgccaaacagccagcgcggatttgccccaacggtacgcggtatcgcaaacagtagtgcaatcgtgactatcaggcaaaatggttatgtgatctatcaaagcaacgtgtcagcgggtgcctttgaaattaacgatctctacccctcttccaacagcggcgatttagaagtcacgattgaagaaagtgacggtacacaacgtcgctttatccagccttattcttcattacccatgatgcagcgacctgggcatctaaagtatagcgcgaccgctggacgctatcgcgctgatgcaaacagtgatagcaaggaacccgaatttgctgaagccacggcaatatatggtttgaataatacttttacgctgtatggcggcctgctcggttctgaagattattatgcgctggggatcggtatcggcggcacacttggcgcactgggcgcgttgtcgatggatatcaacagagctgacacccaattcgataaccagcactcttttcatggctatcaatggcgtacgcagtacatcaaagatatcccggaaaccaacaccaatatcgctgtcagctactatcgctataccaacgatggctattttagttttaatgaagccaatacccgcaattgggactataacagtcgccaaaaaagtgaaattcaattcaacatcagccagacaatatttgatggggtaagtctgtatgcctccggttcgcagcaagactattggggcaataacgataaaaacaggaatatctctgttggggtttccggccagcaatggggagttggttacagcctgaattatcaatacagccgctacactgatcaaaataatgaccgcgcactctctttgaatctcagtattccgttagaacgctggttaccgcgtagccgggtttcctatcagatgaccagccagaaagatcgcccaacccaacatgaaatgcgtcttgatggctcactgctggatgatggtcgcctgagctatagcctggaacaaagtctggatgacgataacaaccataacagtagcctgaacgccagttaccgttcaccttatggcaccttcagtgccggatacagctacggtaatgacagcagccaatacaattacggcgttaccggcggcgtggttatccatcctcatggcgtgacgctctcgcaatatctgggcaacgcttttgcgcttatcgatgctaacggagcatctggcgtgaggatacaaaactatccggggattgctaccgatccttttggctatgcagtggttccttatctcacaacttatcaggaaaaccgtctctcggtagatactacgcagctgcccgataacgtcgatcttgaacaaacaacacagtttgtggtgcccaacagaggtgcaatggtagcggcgcgtttcaacgccaatatcggttatcgcgtacttgttacagtcagcgatcgcaacggtaaaccgttgccctttggcgctcttgccagcaacgatgatacggggcaacaaagtatcgtcgatgagggcggcatactatatctctctgggatatcgagtaaatcacaaagctggactgtacgctggggaaatcaggcagatcaacaatgtcagtttgctttcagtacaccggattcagaacctacaacctctgtattacaaggcacagcgcagtgccattaaggataaaaaaatgaaaagagcgcctcttataacaggtcttttgttgatatccacatcctgcgcttatgcctcctcaggagggtgtggagccgacagcactagcggtgcgacaaattacagcagtgtggttgatgatgttacggtgaaccagacagataacgtgacaggacgggagtttacctctgcaacgctaagtagcactaactggcaatacgcctgttcctgctctgcgggtaaggcagttaaacttgtctatatggtcagccccgtacttaccaccactggacatcagacaggatattacaaactcaatgacagcctggatattaaaaccacattacaggcaaacgacattccaggactcacaaccgaccaggttgtctctgttaacacccgattcacacagataaaaaacaacacggtatattctgctgcaacccaaacgggtgtttgccagggtgatacgtctcgttatggacccgttaatattggtgcgaacaccacctttaccctgtatgtcaccaagccatttctcggctcgatgaccattccgaaaacggatattgccgtcattaaaggcgcgtgggtcgatggaatgggaagcccgtctacaggtgacttccatgatttagtcaagttatcgattcagggaaatctcaccgccccacagtcgtgcaaaattaatcagggcgatgttattaaggttaattttggattcatcaatggtcagaagtttaccacccgcaatgccatgccagacggttttactccagtagactttgatatcacttatgactgtggtgatacttcaaagattaaaaactcgttgcaaatgcgcatcgacggtacaactggggtagtagaccagtacaacctggtcgccaggcgaagaagttcagacaatgtgcccgatgtcggtattcgtattgaaaatctcggcggcggagttgcaaatattccttttcagaacggtatccttcccgttgatccttccgggcatggcaccgtcaatatgcgcgcctggccagttaatctggtcggtggtgagctggaaacaggaaaatttcagggcacagccaccattaccgtcatcgtgcggtaaaagaagacgttgcgttttgattaacgcaacgcttcggcactgttacccctgctgctccagcgcatacttatacagcgcatttttcttcacgccgtgaatttctgcggccagcgccgccgcttttttcagcggcagttctgcctgtagcagcgccagcgtgcgcagggcatcggcgggtaagtcttcttcctgtgctttatgaccttcgacaatcagcaccatttcgcctttgcgacggttttcatcttcctttacccacgccagcagctcgccaacgggcgcgccgtgaatggtttcccaggttttggtcagctcacgcgccagaaccacgtagcgggattcgcctaataccgcaacgatatcttccaggctatctaacagacggtgggtagattcataaaaaatcagcgtgcgcggctccgcttcaatggcttttagcgcatcacggcggccttttgatttggcaggtaaaaagccttcgtaacagaaacggtcagagggtaaacccgctgcgcttaacgcagtgatagcagcacacggcccgggtagcggcaccacgcggatccccgcttcacggcaggtacgcaccagatggtagccaggatcgttaattagcggcgttccggcatcggaaaccagcgcaatgttttgcccctcttgcagcttcgccagcagcgtttcagctttttgttgttcgttatggtcgtgcagcgcaaacaaccgggcattaatcccaaaatgttgcagcaataaaccggtgtgacgagtatcctcggcggcaatcagatcaacggcctgtaatacctctaacgcacgctgggtgatatccgccagattgccgattggcgtcggtacaatgtaaagctggccctgagaattatccgccgattggtgttgtttcattgtgtcgtccgtattgccgatttaatattgagcattgcgtaaaaaaaatatcactggatacattatggtaccctcaacattttctcgtttgaaagccgcgcgttgtctgcctgttgttctggcagccctgattttcgccggttgtggcacccatactcccgatcagtccactgcttatatgcagggcacggcgcaggctgattctgccttttatcttcagcagatgcagcaaagctctgatgataccaggatcaactggcaattactcgccattcgtgcactggtgaaagaaggtaaaaccgggcaggcggttgagttgtttaaccaactaccgcaagaactgaacgatgctcagcgtcgcgagaaaacactgctggcggtagagattaaactggcgcagaaagattttgctggcgcgcaaaacttgctggcgaaaatcacacctgccgatttagaacaaaaccagcaagcgcgttactggcaggcaaaaatcgatgccagccaggggcgtccttccattgatttactgcgcgcgttaattgctcaggaaccgctgcttggcgcgaaagaaaaacagcagaatattgatgccacctggcaggcgctctcctccatgactcaggaacaggcgaatacgctggtgatcaacgccgacgaaaatattctgcaaggctggctggatctgcagcgcgtctggtttgataaccgtaacgatcccgacatgatgaaagccgggatcgccgactggcagaaacgttatccgaacaatccgggcgcgaaaatgctgccaacgcagttggttaacgtaaaagcgtttaaaccagcctcgaccaacaaaatcgccctgctgttgccactgaatggccaggcagcggtatttggtcgcactattcagcaaggctttgaagcggcgaaaaatatcggcactcagccagtggcagctcaggtagctgccgcacctgccgcagacgtagctgaacaacctcagccgcaaaccgtggatggcgttgccagcccggcacaagcctcggttagcgatctgaccggtgaacagcctgcagcccagccggtgcctgtaagcgccccggcgacaagcaccgcagcggtaagcgcacccgcaaatccatccgcagagctgaaaatctacgatacctcatcacaaccacttagccagatcttaagccaggttcagcaggatggcgcgagtattgtggtcggtccgttgctgaaaaataacgttgaagagttgctgaagagcaacactccgctgaacgtactggcactgaaccagccggagaatatcgaaaatcgcgtcaatatttgttacttcgcgctttcaccggaagacgaagcgcgcgatgcagcgcgtcatattcgtgaccagggtaaacaagcgccgctggtgctgatcccacgcagttcattgggcgatcgcgtagccaatgcgtttgcgcaagagtggcagaaactgggcggcggcaccgttctgcaacaaaaatttggttccaccagcgaattacgcgcgggtgttaacggcggttctggtattgctttaacgggtagcccgattactctcagagcgacaaccgactccggcatgacgaccaacaatccaacgctgcaaaccacgccaaccgatgaccagttcaccaataatggcggtcgtgtcgatgcggtgtacattgtggcaacgccgggtgaaatcgcttttatcaaaccgatgatcgccatgcgtaacggtagccagagcggtgcaacgctgtacgccagctcccgcagtgcgcaagggaccgctggcccggatttccgactggagatggaaggcttgcagtacagcgaaatcccgatgctggcaggcggtaatctaccgttaatgcagcaggcactcagcgcggtgaataacgattattcactggctcgcatgtatgcgatgggcgtcgatgcctggtcgctggcaaatcatttctcacaaatgcgccaggttcagggttttgaaatcaacggtaataccggaagcctgacggctaacccggattgcgtgattaacaggaacttatcatggctacagtaccaacaaggtcaggtagtccccgtcagttaaccaccaaacagaccggcgatgcgtgggaagcacaagcgcgtcgctggctggaaggcaaaggactgcggtttatcgccgctaacgtgaacgagcgtggcggcgagatcgatctgataatgcgtgaaggccggaccaccatttttgtcgaggtacgctatcgccgctctgcgctttatggcggcgcggcagccagtgtgacccgcagcaaacaacacaaattattacagactgcccgcttgtggctcgcgcgtcataatgggagttttgatactgtggattgccggttcgatgtggtagccttcaccgggaatgaggttgagtggattaaggatgcctttaatgaccactcataattaaggtttaaggattagcgtgcaagaaagaattaaagcttgcttcactgaaagcattcaaactcaaattgcggcggcagaggcgcttccggatgccatctcccgtgcagccatgacgctggttcagtctctgctcaatggcaacaaaatcctctgttgtggtaatggaacttccgctgccaatgcacagcattttgctgccagcatgatcaaccgtttcgaaacggagcggcccagcttacctgccattgcactaaatactgataatgttgtcttaacggcgattgccaacgatcgcttacatgatgaagtgtatgcaaaacaggtgcgggcgctgggtcatgcgggagatgtattgttagccatttccacccgtggcaacagccgcgatattgttaaagcagttgaagccgccgttacgcgtgatatgaccattgtggcattgaccggctatgacggcggcgaacttgcaggtttgttagggccacaggatgtggagatccgcattccttcgcatcgtagtgctcgcattcaggaaatgcatatgctgacggtaaattgcctgtgcgatctgatcgataacacgcttttccctcaccaggatgattaaggagaatacatgaaggcattatcgccaatcgcagtccttatttccgcgctgctgttgcaaggttgtgttgccgctgccgtagtgggtaccgctgctgtgggtaccaaagccgcaactgacccacgcagtgtcggcacccaggtggacgatggtaccctggaagtgcgcgtgaacagcgcattgtcgaaagacgaacagattaagaaagaagcgcgcattaatgtaacggcctatcagggcaaagtgctgctggttgggcagtcaccaaatgctgaactttcggctcgcgccaaacagattgctatgggcgtagacggtgccaacgaagtgtataacgagattcgtcagggccagccgattggtctgggcgaagcatctaacgatacgtggatcaccaccaaagtgcgttcgcagctcttaaccagcgacctggtgaaatcgtccaacgtgaaagtgaccaccgaaaacggtgaagtgttcctgatggggctggtgactgaacgtgaagcgaaagcggcggcagatattgccagccgggtgagcggcgtgaagcgggtaactacggcgtttacgtttattaaatagcagccccttgtaatgcctgatgcgacgcttgccgcgtcttatcaggcctacaacgatacaaaccgtaggtcagataaggcgtttacgccgcatccgacatgttttccctcaaatcagaacaacagcgccagcccgccgacaatcacaccagacactgccaccatcgcccctgtcagccataaggctttcgccgggaacgctttgcgcagcataatcagtgacggcaaactcactgccgggagcgtcatcaacaatgccagcgccggagcggttcccatacctgccagcatcatcgtttgtacaatcggaatttctgctgccgtgggaatgacaaacaagcatcctgctaccgccatcgccaccacccacatcaggctgttatcgacagcaccatcggcatgggggaataaccagacgcgagcggcacccaacaccagtactgcaaggatgtaaaccgggatcgtactccagaaaagcgtccatagcgccctgccccagcggctaaaaaacccgccctgtgcttccggtatgtcaatttcgaccggtgcctgcgtttgcggtgtttcacgcacccatttttgcaccagcgtcgcaatcagcaacaccatcaccagcccggccaccagacgaatcgccgcaaaaccccagccgaggacaaagcccataaacaccagcgtcgccgggtttaacaccggattgcccatccagaatgccagcgcaccgcccatcgacacctgttggcgacgcattcccgccgcgaccggagccgcacagcaggtacacatcatgcccggcaacgaaaacagcgttcccagcagcgtgccgcgaaagcgcgattgcccaagcgtacgcaacaaccagtcacgcgggatcagcacctgaatcaacgaaccgaggatcacccccagcaccgccgctttccataccgcgaggaaatagatcatcgcgtaatccaacgccgcctgccatgggttagcatccgcctgcgcaaggatagatttaccgatactgtgggtttcggcagcagtaaacgctttgccgtagtaaggttcccatttcacataccagagaccggcaatgacaacgagaaagaaaagcgcgggtttccaccactgaatgggcgttgccgcctgagatgaagactgaccagtcatagcattccccaggaataagttatgataattgagcgcgtgaatattacgctcactatcaattcttgggaataattattcagctcttttgcgtaattctgaagagcttaaaatcgtcacgccttcatgctcaggccgcatcgactctgccagcatgacccgcgccacgtctctcgcatcaatggatttccagttacctggtaacaaacggaacagcggcgcaaaaagcgtttcgttcatccgctgtttgctacgatcgcccagtaacatcgacgggcgagcaatggtcaatttcggccagttctgggcgattaatgcttcttccatctcccctttgacgcggttatagaaaaacggcgagtgggcattggcacccatcgcactgactaccaacatatgctgcgcgcccagtcgccgcccggttaatgcggtatccactaccagcgtgtaatcggcatgaataaacgcctctttgctccccgcttctcgccgcgtggtgccgagacaacaaaacacaatgtcgatgggatcggtgacctgcgccaacgcgtcactcagttgcggatcatggggattaaacaccccgggcatatcgcccaacggacgtcgcgtcggcgcagcaatggcgttaactttcggttcgttaatcaacatccgcagcaggtgaccgcccaccagccccgttgcgcctgtaatcagtacctgactcatcttcgctcctttacagaattgtctgccttgcgctccacggctcatgcaccaggcttaatagaccatgaggtaattatccccgattgtgggaaattcgcctcatccaatgcaacaacgcggaggaagcatgagtaagaaaattgccgttttaatcactgatgaatttgaggattcagaatttacttcacccgcagacgagttccgtaaagccggacacgaagtgattaccattgaaaaacaagcgggtaaaacggtgaaaggcaaaaaaggagaagccagcgtgaccatcgataaatccatcgatgaagtgacgcctgcggagtttgatgccctgctgctaccgggcggccattcaccggattatctgcgtggggacaaccgttttgtcacctttacccgtgattttgtgaatagtggcaaaccggtgtttgccatctgtcacggcccgcagttgctgatcagcgccgatgtgattcgggggcgcaaactgaccgcagttaaaccgatcattattgatgttaaaaatgcgggcgcggaattttacgatcaggaagtcgtggttgataaagatcagctggttaccagccggacaccggacgatctgccagcgtttaaccgcgaggcgttacgcctgctcggtgcctgagtcgcgtagccaaatcatttttttaccaaagcccagcgtgttgtcggtgaatttgatttcatcgagccggatttcccacaccggggccgacagcattctggcaaccggaaagcgacgattgtacgccttgcgcgcgaggtcgctttcctcaccttccagcctgcggatctcacctttaaactgcacaccgcgaattaacgctaccgttttcggctgaccgtttaccgttccggcaaccgcagcctgcggcccactcatctgcgcgtggcgcgttttttcttccgtcaaaatgtagaaggcgactttctgcgcatcaaaaagataaaaggcattagcgcaccagagttccccttcctgctgcacacaccaagtgacaacatgttgttttgccagccaacggctgatggcgatgagtgtttccattgctgttctcttttatactgtgggcctgaccttaacatgcgacgcagacgatgacaccctggtttctttacttgatccgtaccgccgacaataagctttataccgggatcaccacggatgtcgaacgccgctatcagcagcaccaaagcggcaaaggggcgaaagcactgcgcgggaaaggagaactaacgctggtgttttccgcgccagtgggcgatcgttcgctggcgttacgggcggaatatcgcgttaagcaactgaccaaacggcaaaaagagcgtctggtagcggaaggcgcagggtttgcagagctgttaagcagtctgcaaaccccggagattaaaagcgattgaaatgctcgtgatactcaaccaggccggtaacgccattcagcgcgtcatccgctaaacgatgtacctggaaggcgctttcagtgcccggccagcggcaacgcagatcgtgatgcgccgccagttcaaagccgaaacgactgtacagcgccggatcgcccagcgtcaccactgcggcatagccgaactcattaagcgaatcgagtccttcatagaccagttggcgtgccagcccctgtccacggtatttttcatcaaccgccaacggtgccatgccgacccattgcaggtcttcgccctgcacatcaaccggactaaatgccacatagccaatgacctgaccttcgtcatctgtcgccaccagccccagcgtcagaaagccatcttcacgcagatcgtgaaccagcttcgcttccgcatcactttcgaatgagcgacgcagcagggcatcaatacccggcgcatcaatgggaatttctactcgaattagcatggttcacctaccgatgtctgtttggtttcaggcgcggttttcattcccgcctcaacaaaatccgccagttgcagcagcatcatgcgtaaggctttcggcatttgctccagttcaatggcgtccatcaggtttttcacatacagccccagctccgtatcgccttcaatcaccagccgacgctggaagaagagcgtatccggatcttgtttacgcgccgcaatcatcagcagatcgctggcgtcggcactaaaactcacatcagcttgcgcgttctggctaacgaccagtttgccattcaccaccgaggtaaaccattgcaggtcaatatcacgcacatgaatacttaaccagcggccttcaagaaactccagctcgccatcatccagcgcctggcggaattgccagcttaagacctgctcaagaacctggcgttttagcgcaaatggcgtcagttttaccggtacactcaacagagatggccccaaatgcacaatacgggaacgcagtttatccaacacgagttttactccctgtttcaacaatcatcctattttgccatatcagaaaaataacatagcggtataaatcaacaattccatatgaaattgctgctaccaccaatacaactttaactgccttaaatcaaaaattgtcgcagcaaggttaactaaaatcccagttcgttaacatttttgcgttttgatagcgcaaccttcaggaaaaattatggagctgctctgccctgccggaaatctcccggcgcttaaggcggccatcgaaaacggcgcagatgctgtttatatcgggctaaaagatgataccaatgcccgtcacttcgccggccttaactttaccgagaaaaaattgcaggaagcggtgagttttgtccatcaacatcgccgcaaacttcacatcgcgattaacacttttgcgcatccggacggttacgcccgttggcagcgcgccgtggatatggcggcgcagctgggtgccgacgcgctgatcctcgccgacctcgccatgctggagtacgccgccgagcgttatccgcatattgagcgccacgtatcggtgcaggcttcggcgaccaatgaagaggcgattaacttttatcatcgccattttgacgttgctcgcgtggtgctgccgcgcgtgttgtcgattcatcaggtgaaacaactggcacgggtcacacctgtaccactggaagtctttgctttcggcagcctgtgcattatgtcggaaggtcgttgctatctgtcgtcgtatctgacgggtgagtcgcccaacaccataggcgcgtgttctccggcccgtttcgtgcgctggcaacaaacgccgcaggggctggaatcccgcctgaacgaagtgctgatcgaccgttatcaggacggcgaaaacgcaggttatccgacgctatgtaaagggcgttatctggtggacggcgagcgctatcacgcgctggaagaaccaaccagtctcaataccctggaactgctgccggagttaatggcggcgaatattgcttcggtgaaaattgaaggccgccagcgtagcccggcgtatgtcagccaggtggcgaaagtctggcgtcaggctatcgaccgttgtaaggccgatccgcaaaactttgtaccgcaaagcgcgtggatggagacgctcgggtcgatgtccgaaggcacgcaaaccactcttggcgcatatcaccgtaaatggcagtgagaaaagcaatgaaatattccttagggccagtgctgtggtactggccaaaagagacgctggaagaattttatcagcaggccgccaccagcagcgccgacgtgatttatcttggtgaagcggtatgcagcaagcgtcgggcaaccaaagttggcgactggctggagatggcaaaatcgctcgccgggagtggtaagcagattgtgctctccacgctggcgctggtgcaggcatcatctgaactgggcgaactgaaacgctatgttgagaacggtgagtttctgattgaagccagcgatctcggcgtggtgaatatgtgcgctgaacgcaaactgccgttcgtcgccgggcacgcgctgaactgctacaacgcggtgacactgaaaatattgctcaaacagggcatgatgcgctggtgtatgccagtggagctttcccgcgactggctggtgaatctgcttaatcagtgcgatgagctgggcattcgtaaccagtttgaagtggaagtcctgagctacggtcatctgccgctggcctactccgcccgctgctttaccgcgcgttcggaagaccgcccgaaagatgagtgtgaaacctgctgcattaagtatccgaacgggcgcaacgtgctgtcgcaggaaaaccaacaagtgtttgtactcaatggcattcagaccatgagcggctacgtttacaacctcggtaacgagctggcatccatgcagggcctggttgatgtggtccgcctgtcaccgcagggtactgacactttcgcgatgctcgacgccttccgcgctaatgaaaatggcgctgcaccactgccgttgacggcgaacagcgactgtaacggctactggcggcggctggcaggactggagctgcaagcctaagtaaatagctcactttgttaacaactttaactactctttaatgcagtattaaagattaatcggtaacaaagtgagctgttatgactgataaaaccattgcgttttcgctactcgatctggcccccattcccgaaggttcttcagcgcgagaagcattctcccactctctcgatctcgcccgtctggctgaaaagcgcggctatcatcgctactggctggcagaacaccacaatatgactggcattgccagtgctgccacgtcggtattgatcggctatctggcggcgaataccaccacgctgcatctggggtctggcggcgtgatgttgcctaaccactcaccgttggtcattgcagaacagttcggcacgcttaatacactctatccggggcgaatcgatttggggctgggtcgtgctccgggtagtgaccaacggacaatgatggcgctacgtcgtcatatgagcggcgatattgataatttcccccgcgatgtggcggagctggtggactggtttgacgcccgcgatcccaatccgcatgtgcgcccggtaccaggctatggcgagaaaatccccgtgtggttgttaggctccagcctttacagcgcgcaactggcggcgcagcttggtctgccgtttgcgtttgcctcacacttcgcgccggatatgctgttccaggcgctgcatctttatcgcagcaacttcaaaccgtcagcacggctggaaaaaccatacgcgatggtgtgcatcaatattatcgccgccgacagcaaccgcgacgctgaatttctgtttacctcaatgcagcaagcctttgtgaagctgcgccgtggcgaaaccgggcaactgccgccgccgattcaaaatatggatcagttctggtcaccgtctgagcagtatggcgtgcagcaggcgctgagtatgtcgttggtaggtgataaagcgaaagtgcgtcatggcttgcagtcgatcctgcgcgaaaccgacgccgatgagattatggtcaacgggcagattttcgaccaccaggcgcggctgcattcgtttgagctggcgatggatgttaaggaagagttgttgggatagtgtgtcttaacgcgggaagccttatccgagctggcaacgctgtcctacatagacctgataagcgaagcgcatcaggcattgtgtaggcagcagaaatgtcggataaggcaccgctgattactgatacaccggcagtaaattaaagctcgataaaatatgcaccagtgcgttgccgacgccaaacaccagaatcagcgcaatcatcggcttgccaccccagacgcggaatttcgggctgccaaagcgtttacgcgatgcacgggctaacagcgccggaacaattgccgcccagatggtagccgctaaaccagcataaccaatggcgtacaggaatccgttcgggaacaacagcccccccacaactggcggggcaaaggtcagcaatgccgttttcaagcggcccacagccgagtcgtcgaaaccaaacagatctgccagatagtcaaacaaacccagcgttacgccgaggaacgaactcgctaccgcaaagtttgagaacacgaccagcagcagatccagactacggctgttcagtacgccgcttaacgcctgtaccagcacatcaatattaccgcccttctctgcaataccgataaactccggacgcgggatgttacccatcgtcgccagcaaccagatggtatacagcgccagcgccatcagcgtaccgtacaccagacatttcacgatggttttcggatctttgccgtaatacttcatcaggcttggcacgttaccgtgataaccaaacgatgccagacagaacggcagggtcatcaacagatacggtgcataagacgcattgctttcggcgacgttgaacaatgtcgcaggctgcacatgccccagcaggctaccaaaggtgaggaagaaggtaatgactttcgcccccagcacaatcgctgtcatgcgactgacggctttagtgctcaaccacaccacaaacgctaccagcaatgcaaaaccaaaacccgccgcccgtgccgggacgtttagtgacatctctgcgaaggtgtgatgcagaatcgaaccactggcagaaatataggcataggtcaggatatagagcacaaaggcaatggaaatgccgttgaccacgttccagcctttgcccagcaaatctttggtgatggtgtcaaaactcgaaccgattctgtaattcaggttagcttccagaatcatcaagccggaatgcagcatacagaaccaggtaaagatcagcgccgccattgaccagaaaaaccacgccccggacatgaccactggcagagaaaacatccctgcgccaataatggtgccgccgataatcaccacgccgccaagcagcgacggtgacgtttgggtggtggttagtgttgccatgagggcttctctccagtgaaaaatagtgcgactgcgttgttatgcattgcactgtaccagtacacgagtacaaaagacagaaaaaaagccccgatggtaaaaatcggggctgtatatattattttacagattgtgttcgctgttcagcgatgattacgcatcaccaccgaaacgacgacgaccggtagaatcatcacgacgcggagcgcggccttcacgacgttcgccgctaaaacgacgaccatcaccacggccaccttcacggcgttcaccgctgaagttacgaccgccttcacgacgttcgccaccgaaaccacgaccaccgccacgacgctcaccgccagtatgcggctgtgcatcgcccagtaactgcatgttcatcggcttgttgagaatgcgagtgcgcgtaaagtgttgcagcacttcacccggcatacctttcggcagttcgatggtggagtgagaagcaaacagcttgatgttaccaatgtaacggctgctgatgtcgccttcgttagcaatcgcaccaacgatatgacgaacttcaacaccatcatcgcggcccacttcaatgcggtacagctgcatatcgccaacatcacgacgttcacgacgcggacgatcttcacggtcaccacgcgggccacggtcgttacgatcgcgcggaccacggtcatcacggtcacggaattcacgtttcggacgcatcggcgcatctggcggtacgatcagagtacgttcaccctgtgccattttcagcagtgccgcagccagagtttcgagatccagctcttcaccttcagcagtcggctgaattttgctcagcagtgcgcggtattgatccagatcgctgctttccagctgctgctgtactttagcggcgaatttttccagacggcgtttgcctagcagttctgcgttcggcagttctacttccggaatagtcagcttcatagtacgttcaatgttgcgcagcagacgacgctcgcggttctcaacgaacagcagcgcgcggccagcacgacccgcacgaccggtacgaccgatacggtgaacgtaagactcagaatccatcgggatatcgtagttaactaccaggctgatacgctcaacgtccaggccacgggctgcaacgtcggtcgcaatcaggatgtccagacgaccatctttcaggcgttccagtgtctgttcacgcagcgcctggttcatgtcaccgttcagcgcggcgctgttgtagccgttacgctcaagagcttcagccacttccagagtcgcgtttttggtacgaacgaagataatcgccgcatcaaaatcttccgcttccaggaaacgtaccagtgcttcgtttttgcgcataccccagacagtccagtagctctggctgatgtcaggacgggtagtcacgctggactgaatgcgcacttcctgcggctctttcataaagcggcgggtaatgcgacgaatcgcttccggcatggttgcagagaacagagcggtctgatgaccttccgggatctgcgccataatggtttcaacgtcttcgatgaagcccatgcgcagcatttcgtcagcttcatccagaaccagaccgctcagtttagagaggtccagagtgccacgtttcaggtggtccagcagacggcccggagtaccgacaacgatctgcggcccctgacgcagggcgcgtaattgcacgtcataacgctggccgccgtacagagcaaccacatttacgccgcgcatgtgtttagagaaatccgtcattgcttcagcaacctgtaccgccagttcgcgggtcggtgccagcaccagaatctgtggtgctttcagctcaggatcaagattctgcaacagaggtaaagagaatgctgcagtttttccgctccccgtctgggccatacccagaacgtcgcggccattcagcagatgtggaatacactctgcctgaattggagatggtttttcgtaacccagatcgttaagggcttcaaggataggagccttcaggcccagatctgcaaaagtggtttcgaattcagccatgtagtacgtgtgcctcaaaattaatggcggccagtctacataactcatcatgaaattgatcagcaattttcattgaaaagtgtgaaccggctcaaagtaggtgtattaacgaacaacaacgccctcacccgttaaggtgatggcaatcaaaaaagattacgggctgatgtgtacgtcagctattgctggtccgattctgccaggtcatcttggtcctggcccaggagcgataattccaacaatgcgtatcggtgctcaacaaagttatgaacgttgttggcaaccgccagtttgaacagtgccgtggcgctgtccaaatcccccagacttaggtagtacttacctaaatagaagttggtttcactgagatgctcagcgagcgaggtgttatccgttgcgtccgccttgagcctttccattaacgtttgttcgctaatgttgcccaggtagaactcgacaatgttccatccccactgttccttatccgatttttcgaagtgctgtttcaacacttctttagcctgcttctcatcgagcttctgctcggcgagataaagccacagactacggaaaggatcattgggatcgtcttgataaaacgccagcagatcatcttgcgctaacttgtcacgaccgccgtaatataatgcgatcccgcgattcaagtgcgcgtagttgtaagttggatcaagctcaagtacagaatcaaacgcttcataggcagcatcaaaattgcctgcctgcgttaaatatatgcctaagtaattgaatacttcaggcatatccggtcggattgccagcgcttgcgaaaaatcgttacgcgctaatgccctcagaccgagactatcatacaacactccgcgctcatataaaagctgtgcgcgttcgtcatcggttaaagcccgactggcaaggatttgttccatacgtgccagaatcacttcctgctgtaaagtcggttgcaatggtaccgcgaggacttcacttttacgccaggaagtattactgcatcctgcaagcgtaagtgctgtcgcaacgaaacaccagcgcaaaaaaggcttcatttcccactcccgaagaccacggttgaatgaacgtcctgttcccggttgctaacaaggcgtcctgcccggttaaaagccccccgccgcagcggagggcaaatggcaaccttactcgccctgttcagcagccggagcttccggtgctgcagcaggttgagactgctcagtcgcttctttaatgctcagacggatacggccctggcgatcaacttccagaactttcaccggtacttcctgacccatctgcaggtaatcggtcactttctcaacgcgtttgtcagcgatttgagagatgtggaccagaccttctttaccgccgccgatggcaacaaatgcgccaaagtcaacgatacgggtcactttaccagtgtagacgcggcccacttcgatttctgcagtgatctcttcgatacgacgaatagcatgtttcgctttctcgccgtcggtcgctgcaatcttcacagtaccgtcatcttcgatttcgatggtggtgccagtttcttcggtcagagcacggattacagaaccgcctttaccgataacatctttgatcttgtccgggttgatcttgatggtatggatacgcggtgcgaactcagagatatcgccacgcggcgcgttgatcgcctgttccattacgcccaggatatgcagacgcgcacctttagcctggttcagcgcaacctgcatgatctctttggtgataccttcaattttgatatccatctgcagtgcagagataccgtcgcgggaacctgcaactttgaagtccatatcgcccaggtgatcttcgtcgcccaaaatgtcagacagtacaacgtagttgtcgccttctttcaccagacccattgcgatacccgcaacggcagctttgatcggcacacctgcgtccatcagcgccagagacgcgccgcacacggaagccatagaagaggaaccgttggattcagtgatttcagacacaacacgtacggtgtacgggaatttgtccatatccggcatgactgccagcacgccgcgcttcgccagacgaccgtgaccaatttcacgacgcttcggagaaccgaccatgccggtttcgcctacggagtacggagggaagttgtagtggaacaggaaggtatcggtacgttcgcccatcagttcatcaagaacctgcgcgtcacgagcagtacccagcgttgcggtaaccagcgcctgcgtttcaccacgggtgaacagcgcagaaccgtgagtacgcggcagcacgccagtacgcacatccagaccacggatcatatctttttcacgaccgtcgatacgcggttcgcctgccagtacgcggctacgaacaacgtttttctcgatcgcgtgcagaatttcacccagttcgttttcgtccagggtttcgtcttcagcaagcagcgtcgcgatggtttcagatttgatgacatcaacctgcgcataacgctcttgtttgtcggtgatgcggtaagcatcgctcaggcgagcttcagccagtgcagcaacgcgcgcgtttagcgcttcgtttaccggctccggctgccagtcccaacgcggtttaccggcttctttcaccagttcattgatgttctgaataacaacctgctgttgttcatgaccgaacactactgcgcccagcatctggtcttcgctcagcagttgagcttcagattcaaccatcagtacagcggcttcagtaccggcaacaaccagatccagtttgctctctttcagctcgtcctgagtcgggttcagtacgtactggtcattgatgtaacctacgcgggcagcaccaatcgggccattgaacggaataccagacagagacagcgctgcggaagcaccaatcatcgcgacgatatccgggttaacttgcgggttaacagaaaccacggtggcgataacctgaacttcgttgacgaagccttccgggaacagcgggcgaatcgggcggtcaatcagacgcgcgatcagggtttcgccttcgcttgggcggccttcacgacggaagaagctacccgggatacgaccagcagcgtaggtacgctcctgatagttaacggtcagtgggaagaagtcctgacctggtttggcttttttctggccaacaacggtaacgaataccgcggtgtcatccatgctaaccataacagcggcagtagcctgacgagccatcatgccggtttccagagtcacggtgtgttggccgtactggaatttacgaacgatcggattaagcaatgtaatatcctttctctttcttagacagtaccttacggcactggtgttaatacccgatcttctgcgcatcctcgcgactaatgacaaccctaacccagctctatgtgggtaaagcctctcattagccgcgcgaacctctgcaacggaagatcattcatagcaacaatacattagtttccagtgaattgctgccgtcagcttgaaaaaaggggccactcaggcccccttttctgaaactcgcaagaattagcgacgcagacccaggcgctcgatgagctgggtgtaacgtgctacgtctttacgtttcaggtagtcgagcagtttacgacgctgagaaaccatgcgcagcagaccacgacggctgtggtgatcttttttgtgctctgcaaagtggccctgcaggtggttgatctgtgcagtcagcagtgctacctgaacttcggtagaaccggtgtcgtttgcgtcacgaccaaactcagaaacgattttagctgttgcttcagtacttagagacattttaaaactccaaagtatatagaatgaaaggacgccgatctctaattcagcgatcccagtgtacgttacgcaaagtgttaaacaatttacgcgacgttaagcggcagtattctactcgtagcgacctgttatcgcaagacggttaacattacgccgggtattcaaccaccaggcgacgaggcgcaacgcggccttcatcgtcaatttcgcccataccgataaatttgccgttctcaccttccgtgacgcgaaccagtccttccagtggcgcaccagatgtacgaaccgggttaccatttttgaagtaaacagaagacgttaacggaagattcaccaccggatagtccgaagctggactgtccattggcatcagtaatggatcaagtaactccgcggctggaatatcctgctgttcagcttgctcaacaagttcacgcaggtgctccagggtcaccatccgttcaaccggatatttacttaccgccagacggcgcaggtaaataacatgcgcgccacagccgagtttttcacccaggtcatcaatgatggtgcggatataagtgccttttgagcagtgaatttccagctccagctcattgccttcatggcgaataaacagcaattcataaacggtaatcggacgcgcttcacgcggaacttcaatgccctgacgcgcatattcgtacagttttttgccctgatatttcagtgctgaatacatcgaagggatctgttcgatatcgccacggaaagtatccagtgccgctgccagctgctctgcgctaaaggttaccggacgttcttcaacgatctgtccgtcggcatcagaagtatcggtacgctgtccaagacgcgcaatgacccgatagcgtttgtcggagtccagcagatactgggaaaacttcgtcgcttccccgaggcaaatcggcaacatgccggtcgccagcgggtccagcgcaccggtatgcccggcacggttggcgttatatatacgtttcactttttgcagcgcatcgttgctggacataccctgaggtttatccagcaacaaaacgccgttaatgtcgcgaccgcgacgacgaggacgactcattagtcctccttgctgtcgtccgggttaacacgacgttcttcgtcatgtttgaccacgctggtcaccaggtttgacatgcgcatcccttcaaccagagagttgtcgtagaagaaggtcagttccggcacgatacgcaggcgcatcgctttccccagcaggctgcggatgaaaccagaagcttcttgcaacgctttgatgcccgctttaaccgcgtcttcatctttgtcgttgaggaacgtcacatatactttggcatacgccaggtcgcgagacatttcgacaccggaaacggtggtcatcatgcccaggcgaggatctttaatttcacgctgcaggatgagagcgatctctttttgcatttcctgcgctacgcgctgcgggcgaccaaattctttcgccataataaattctcctgacaaaaaaggggctgttagcccctttttaaaattaatttcaggtggaagggctgttcacgttgacctgataagacgcgccagcgtcacatcaggcaatccatgccggatgcagcgtaaacgccttatcccgcatggaaccctaaaaaccttaagcaatggtacgttggatctcgatgatttcgaatacttcgatcacatcgccagtgcggacgtcgttgtagttcttaacgccgataccacattccataccgttacggacttcgttaacgtcatctttgaagcggcgcagggactccagctcgccttcgtagataaccacgttgtcacgcagaacgcggatcgggttgtgacgtttaaccacaccttcggtaaccatacagcctgcgatggcaccaaatttcggcgatttgaacacgtcacgaacttccgccagaccgataatctgctgtttcagttccggagacagcataccgctcatcgccgctttcacttcgtcaatcaggttatagatgacggagtagtaacgcagatccaggctttccgcttcaatcactttacgtgcagaggcatcagcacgtacgttaaagccaaccaggatggcgttggacgccgcagccagggtggcgtcggtttcggtgataccacctacgccagaaccgatgatcttcactttaacttcgtcagtagacagtttcagcaaggagtcggagatcgcttcgacagaaccctgtacgtctgccttcaggacgatattcacttcgtgaacttcgccttcggtcatgttggcgaacatgttctcgagtttagatttctgctgacgcgccagtttaacttcgcggaatttaccctgacgatagagtgcaacttcacgcgctttcttctcgtcacgtacaacggtaacttcatcacccgcagccggtacgccggacaggccgaggatttccaccggaatggacggacccgcttccagcacttcctgacccagttcgttacgcatcgcacgaacacgaccgtattcgaagccacacagaacgatatcgcccttgtgcagagtaccttcacgtaccagaacggtagcaaccggaccacgacctttatcgaggaaggattcgataaccgcaccgctcgccatacctttacgtaccgctttcagctccagaacttccgcctgcagcaggatagcgtccagcagttcatcgataccggtacccgctttcgcagatacgtgtacgaactggctttcaccgccccactcttccggcaggatgccgtactgggagagttcgttcttaacgcgatccggatcagcttctggtttatcgatcttgttcactgcaaccaccaccggtacctgcgccgctttcgcgtgctggattgcttcgatggtctgcggcatcacaccgtcgtcggcagcaacaaccaggactacgatgtccgttgcctgcgcaccacgagcacgcattgaagtaaacgcggcgtgccccggggtgtccaggaaggtgatcatgccgttttcagtttcaacgtggtatgcaccaatgtgctgggtaatgccgcccgcttcgccagaggccactttcgttgaacgaatgtagtccagcagagaggttttaccgtggtcaacgtgacccatgatggtcacaaccggcgcgcgcggttcagccgcagcacccgtgtcacggtcgctcattaccgcctcttccagctcgttttcacgacgcaggataactttatggcccatctcttcagcaaccagctgtgcggtttcctgatcgataacctggttgatggttgccattgcgcccagtttcatcatcgctttgatgacctgagagcctttaaccgccatcttgttcgccagttcgccaacggtgatagtttcgccgatcacaacgtcacggttaacggcctgagcaggcttctggaagccttgctgcagcgaagaacctttacgttttccgcctttaccgccacgtactgctgcgcgtgcttcttcacgatcagcttttgattcagcgtgtttgttgcctttcttcggacgcgctgctttcgcgttacgaccacggccacggccgccttcgacttcacgatcgctttcgtcttctgcctggcgagcatgttgagaagtagtgacgtgataatcgctggaatcttcagtcggttccgcgttatcagtccatttgttttcttccgccatacgacgtgcttcttcagcaacgcgacgtgcttcttcttcgagtttacgacgcgcttcttcttcagctttacgcttgagctctgcagcttcctgctcacggcgggctttttcagcctgggcgtttttagtcatatcgtcttgttgattgctcactttgtctttttccgcagcttcacgtttcgcttgttcagcagcttcacgcttagcttgttctgcggcctcacgttcagctttttgttgcgcctcgcgtttagccgattcttctgcctcacgacgggcttgctcttccgcttcacgctgcgcttgctcttccgctgcaaggcgttcagcctcttgcggatcgcgtttcacaaaggtgcgtttcttgcggacttcgatttgtaccgatttgctttttccaccggtaccaggaatgttaagggtgctgcgtgttttacgttgcagcgtcaatttgtccgggcctgaatttttctgattcaggtggtcaatcaaagtctgtttctcttgtgcagacacagagtcgtcagcagacttccggatacctgcatcagcaaattgctgtaccaggcgttccacggaggtctgtcgctctgcggccagcgttttaatcgttacatctgtcatgctgttccttcctgctacagtttattacgcttcgtcaccgaaccagcaaatattacgggcagccataatcagtgctccggctttttcgtcggtcaacccttcgatatcagccagatcatcaatgccctgttcggcgagatcttccagcgtacaaacgccacgggcggccagtttgaatgccaaatcacgatctaccccttcaaggttcagcagatcgtcagccggtttgttatcaccgaggctttcttcctgggcctgtgcaatggtggccagtgcatttttagcacgctcgcgcagtgcttcaacggtcggctcatcaaggccttcgatttccaacagctctttcatcggcacataggccaattcttccagcgtcgagaagccttcttctaccagaacagtcgcgaagtcttcgtcgatgtcgagatatttggtgaaggtgtcgatcgctgcgtgcgcttccgcctgatgcttagcctgcaggtcgtcaacggtcatcacgttgagttcccaaccgctcagctgcgaagccagacgcacgttctgaccgttacggccaatcgcctgcgccaggttaccggcttcaacggcgatatccatggtgtgtttatcttcatccaccacgatagaagcaacgtctgccggtgccattgcgttaatcacgaactgcgccgggttatcatcccacaggacgatatcgatacgctcgccacccagttcagtagacaccgcctgaacacgcgcgccacgcatacctacgcaagcacctaccggatcgatacgtttatcgttggttttcaccgcgattttcgcacgagaacccggatcgcgagccgctgctttaatttcaatcacttcttcgccgatttctggcacttcaatacggaacagttcgatcagcatttccggcttggaacgagtgacgaacagttgcgcgccacgcgcttccgggcgaacggaatagagcacgccacgaacgcggtcgccagggcggaagttttcacgcggcagcatatcttcgcgcaggatcacggcttcagcgttgttgcccagatccagagagatgttgtcgcggtttacttttttcaccacgccggtgatgatttcaccttcgtgttcacggaactgatcaaccaccatcgcacgttcggcttcacgcactttctgcacgataacctgttttgccgtctgggtagtgatacggtcaaaggtaacagactcaatctgatcttcaacgtaatcgcccaggttcaggctttcatcttcataacgtgcggcttcaagggtgatttccttggtcggctgggtgacttcatcaacaactaaccagcgacggaaagtgtcaaaatcaccgcttttgcgatcgatctgtacgcggacgtcgatctcttgttcatattttttctttgttgctgtcgccagcgcgctttccaatgcttcgaaaatcttctcgcgaggtagcgccttttcattggatacggcttcaactacagccaaaatttctttgttcatcgcgggcttttcacctcatccagactattaaaagtggggaaccaggttcgccttctggatattactcagcgcgaacacttcatctttaccttcgacggtaactgtgatcatttcaccgtctaccgctttgataacgccctgccatttacgacggttttgtaccgccatacggagaaccagagtcacctcttctccgacaaaacgggcgtagtgttcagccgtgaacagtgggcgatcgagacccggtgaggagacttccaggttataagcaacggtgatgggatcttcaacatccagcacagcacttacctggtggctcacatcagcacaatcatcaacattgatgccatcttcactatcaatatagatgcgcagtgtggatgtgcgaccgcgaataaattcgatgccaaccagttcaaaacccagggcctcaactggcgcagtaatcatctctgttaatttttgctctaatgtggacaagcccacccccaagacataaaaaaagggcctaaagcccagttattctgtagtcagataacaaaaaaccccgataaatcggggctttatataactgaaccctataaccgcaactgcggtctggagcactttccagaaggattttttcaaatcccactacgaaggccgaagtcttcacagtatatttgaaaaaggactctaagggaaagtggttgcgggggccggatttgaaccgacgatcttcgggttatgagcccgacgagctaccaggctgctccaccccgcgcctgaaacgtggcaaattctactcgttttgggtaaaaaatgcaaatactgctgggatttggtgtaccgagacgggacgtaaaatctgcaggcattatagtgatccacgccacattttgtcaacgtttattgctaatcatgtgaatgaatatccagttcactttcatttgttgaatacttttgccttctcctgctctcccttaagcgcattattttacaaaaaacacactaaactcttcctgtctccgataaaagatgattaaatgaaaactcatttattttgcataaaaattcagtgagagcggaaatccaggctcatcatcagttaattaagcagggtgttattttatgacgacgattctcaagcatctcccggtaggtcaacgtattggtatcgctttttctggcggtctggacaccagtgccgcactgctgtggatgcgacaaaagggagcggttccttatgcatatactgcaaacctgggccagccagacgaagaggattatgatgcgatccctcgtcgtgccatggaatacggcgcggagaacgcacgtctgatcgactgccgcaaacaactggtggccgaaggtattgccgctattcagtgtggcgcatttcataacaccaccggcggcctgacctatttcaacacgacgccgctgggccgcgccgtgactggtaccatgctggttgctgcgatgaaagaagatggcgtgaatatctggggtgacggtagcacctacaaaggaaacgatatcgaacgtttctatcgttatggtctgctgaccaatgctgaactgcagatttacaaaccgtggcttgatactgactttattgatgaactgggcggccgtcatgagatgtctgaatttatgattgcctgcggtttcgactacaaaatgtctgtcgaaaaagcctactccacagactccaacatgcttggtgcaacgcatgaagcgaaggatctggaatacctcaactccagcgtcaaaatcgtcaacccgattatgggcgtgaaattctgggatgagagcgtgaagatcccggcagaagaagtcacagtacgctttgaacaaggtcatccggtggcgctgaacggtaaaacctttagcgacgacgtagaaatgatgctggaagctaaccgcatcggcggtcgtcacggcctgggcatgagcgaccagattgaaaaccgtatcatcgaagcgaaaagccgtggtatttacgaagctccggggatggcactgctgcacattgcgtatgaacgcctgttgaccggtattcacaacgaagacaccattgagcagtatcacgcgcatggtcgtcagttgggccgtctgctgtaccaggggcgttggtttgactcccaggcgctgatgctgcgtgactctctgcaacgctgggttgccagccagatcactggtgaagttaccctggagctgcgccgtgggaacgattattcaatcctgaataccgtctcagagaacctgacctacaagccagagcgtctgacgatggaaaaaggcgactcggtgttctcgccagatgatcgtattggtcaattgaccatgcgtaacctggatatcactgatacccgcgagaaacttttcggttatgccaaaactggcctgctttcctcctctgccgcttcaggcgtgccgcaggtggagaatctggaaaacaaaggccagtaattcgacatcaaccctgcccttcaggggtggggttaccttgcttatcctctgtaaactcctttctgagcatcacataatcgaaaacatcatggtttgcatccacaacccgtgagtctcctttatagtgtgcaatcacttcctcaagcgtttgcggctgttccggctttgttacccccatccacgcattaataaggtaattattgtaagctgtcgaaaagatgttgttttccgttgtgcgatccacgccatccccaagaacggggctataccagataaacatcgggacatgatatgcctgctggctagcctccctgcctccatgaaaatagacgttcttcttcgtagggtcacgttccaggccgtggtcggcaaaatacatgaccgaggcgcggcgatcttttaataattcaaaaacctgacctagcaaactatctgtgtaatgaatggagttgtcatagcaggcatcctgatcgtcctgcggttgaaacacggcgctggattgcggataggcgctacaagccggttcatggcttccatttaaatgaagaacaatcagtttcttttgctgcgtattttgctgtaatgcttgcgataaatgcggcaacaacaattcatcaaatcctctgacataaactgtttccatggcgcgcatggcgatactggtaactgctgtaccattctgccgaaaagcggattgcgagcttagccagaaagtctgaaatcctgcttgattagccatattaataatgttgtcggggtaattatgaatgtcatgactcaaaacagaatcagcagttaaagaaaggggaaccgacagcgcagtgtaaggtgcgccgcttattgcttgattaaacagtttgatctgttttctttgtgcttcaacttgcggtgtcgtagagcgtgtatatccatacaaagacatattgtcgacacgtacagactcccccacaatcaacacgtaggtatcaatacctgtatccctgactgataattgaaaatacggcaccgtgtttgcaattgagagtaatctttgatgctctttcgctgctaaagcaaaatagttgagattgaaaaacggcgtataggtagcaaatcgcgacgctagtatatatggactgaacgcttttttattttttgcatctttataagcaaattgacaagcggaaaataaactgcccgaaatgacaatcagcaataatattcctgtcactttttttgtcggcaaggaaacatcatattttattattactgccaaaaaaagaagggataaaaaagcaaaggcacatagataagggatatacatccccagcattttgacaacttcatccggatcactctggagcacactaatcgcaaatccatcattgaaagttgtaccaaaggtacaccatgaatagaggctaatactcatgtctgccgcagtcagtaacacaaatggtgcggcaacaagcaggcgaagcggaagggatgatatacgttttacaaccaggatggtcagaacgaagaacagcaagcgctgaaccatatgcgctccggaagaagcgactaagttcgtaataccaaaaacaataacacaaagatacaacaaccaatgagatttaaaagttctagcaaatttgttgaatactgtcatccagaaatccaagttcacaaccaatataaacaattatcaacaatgtttaattttatatcagacatgtttttcaactctgatccatatcagaacgaaacactgttagttttttctttttaaatgatgcggccattgcgttctcagtaattaaataacattatcaatgcgtctctaaacattacgcagaacgtagccatcagtcgttatactgacaggagcaggatggtttatcgagaagtaaacatatccgtattcgtaccggaactggagttgacacaataaagtgccaattatgtcagtagaagggaaaaatttataactaaggcgtaccggcaccatcgtttcaaggtaccagctacgagtaaagcaactggacgagatacagatacctgacaaccattcctcagaccaggaccaaaacgaaaaaagacgcttttcagcgtctcttttctggaatttggtaccgaggacgggacttgaacccgtaagccctattgggcactaccacctcaaggtagcgtgtctaccaattccaccacctcggcacggatactactttttagttcgggatatcgctggtcggcttagccggagcagctggctgagtttgttcggttttcgccggtgcactcagattttcccattcgctacctttattggttttgttgctattgatgttacccagcaccagactgatgatgaagaataacgttgccagcagcgccgtcatgcgggtcatgaagttaccagaaccacttgaaccaaacagcgtagcggaagcgcctgctccgaaggaggctcccatatcagcgcctttaccttgctgcagcatgatcagaccaacaaggccaattgccacaataaggaaaactactaaaagagcttcatacataatcaacctgttccttgcggagttgccgcgtaccaatgcttcaaccaataaagcgggagtttttaatctttcccactgaagcgggtgtgaatactaaccaaagcgaatgaccttcgcaagggcaattttatcgcattgtatcaactgcggaaaaaaacagcaaaaccgatgtgttcgctgagaaaaaaggcgacaatcgccgcctttttagccagttatctaacgctttaaacggcttttactgcatcggcgatgcggtgtgcaaattcagtcacctgcgcttcgtcttcgccttccaccatcacgcgaattaacggttcggtgccggatttacgcagcaacacgcgtccacggttgcccagcgcagcttcaacctctgcggtcacggctttaactgactcatgctcaagtggatcgccgctacctgcggtgtaacgtacgttaaccagaatctgcgggaacattttcatgccgctgcaaaggtcgtgcaggctcatatggttacgtgccatcgccgccagcacctgcaagccagcaacgatgccgtcaccggtagtagttttatccagcaggatcacatgaccggaattctctgcaccgatacgccagcctttctcctgcattttttccagtacgtagcggtcacccactttcgcgcgcgcaaatggaattcctaactgtttcagcgccagttcaagccccatgttgctcatcaatgtacccacagcgccaccacgcagctggccctgacgaagaccttcacgcgcgatgatatacatgatctgatcgccatcgactttattgccttcatggtcaaccataatcacgcgatcgccatcgccgtcgaaggcaataccgagatccgctttttcagccagcacacgagcctggagcgcgcgaacgtcggtagcccccacttcggcattgatgtttacaccgtttggctcacaaccgatagcgataacgttcgcccccagttcgcgcagcacgttcggcgcgatgtgataagtcgcaccgtttgcacaatccaccacaatcttcagttcactgaggctaagttcgttcgggaacgtggctttgcaaaactcgatatagcgacccgcggcatcaacgatacggctggctttacccagttctgccgaatcaacgcagctgatctccttttccatttccgcttcgatggcctcttctaccgcatccggcagtttggtgccgtcgatagagaagaatttaatgccattatcgtagaacgggttatgcgatgcagatatcacaattccggcctctgcgcggaaggtacgcgtcagataagccacggccggtgttggcatcgggccagtgaagagtgcggaaaggcccgctgccgccagacccgcttccagtgctgactccagcatatagccagaaatacgcgtgtctttaccaataataatcttacgggagccgtggcgcgccagcactttacccgcggcccaacccagcttaagcacaaaatcaggtgtgatcggcgcatcccctacacgaccacgaatcccatcggtaccgaaatatttacgattactcatagcgtttgttttcctttgcagacagagtggcttccaccacccgcatcgcttctacggtttctttgacgtcatgaacacgaatgatgtgcgcgccttgcattgcggcaatgaccgcacaggccagactaccgctcaggcgctcggacggccccacgttcagcagctgcccaatcatcgattttcgtgacatacccaccaacagcggcaggttgaaatggtgaaattcagccaggcgcgccagtaatgaatagttatgggagagatttttaccgaaaccgaatccggggtcgagcaacaatttctcttttgcgatacccgcctgctcgcaacgtgctatttgctcaataaagtagcgattcacttctgcaaagacatcgtcatacttcggagcttcctgcatggtttttggatttccctgcatatgcatcagacaaaccggtaaaccggtttctgcagccgcctccagagcgccaggttcggaaagggagcggatatcattaataatgtgagcgccaactttcgctgactcacggatgacttctggtttggatgtatcgactgagatccagacttcgaagcgttgagcaattgcctcaaccacaggaataacacgttgcaactcttcttcaacgctaacttccgccgcccctgggcgcgtggactcgccaccaacgtcaatgatcgtcgcgccagcgttgatcatcagattcgcatgtttcaccgcatctatcagcgagttatgcgtgccaccatccgaaaaggaatcaggcgtgacgttgaggatccccattacgtgaggatggctaaggtccagtgaagtaccctgggcaaagagtttcatgatgttatccctggtatgaattgataagaaaaaaccccggagcacgccccggggttttcggtacaaatacagtcatctgatgcgggaacttacttgtcgcctaactgctctgacatggtgttacccgggttcggcgtacgcggttcatcaaccggacgaggagcctttggactaccattgtcgccagaattgttagaagcgcctggttcttcccagcccgctggcggacgtacatcgcgacgtgccatcaggtcatcaatctgcggtgcgtcgatagtctcatatttcatgagagcatctttcatcgcatgcagaatatccatattgtcggtcagaagctgacgcgcacgattatagttacgctcaatcagtgctttcacttcctggtcgatgatacgtgcagtttcatcggacatatgtttcgctttcgctacgctacggccgaggaacacttcaccttcttcttccgcgtacagcagtggacccaatttctcagagaagccccactgagtcaccatgttacgtgccaggttggtcgcaactttaatatcgttggacgcaccggtagatacatgttccggcccgtagatgatctcttctgccagacgaccaccgtacagcgtagaaatctggctttccagtttctgacggctggcgctgattgcgtcgccctcaggcaagaagaaagtcacacccagcgcacgaccgcgtgggataatcgtcactttgtgcaccggatcgtgttccggcaccaggcgaccgataatcgcatgacccgcttcgtggtaagccgtcgattctttctgcgcttccgtcatcaccatggagcgacgttccgcacccatcatgattttgtctttcgctttctcgaactcaaccatcgacacaacgcgtttgttgccacgagcagcgaacagtgccgcttcgttcaccaggttcgccaggtcagcaccggagaaaccaggagtaccacgggcaatgattgccgcgtcgatatcgggtgccaatggtacgcgacgcatgtgaactttcaggatctgctcacgaccgcgaacatctggcaagccgaccacaacctgacggtcgaaacggccaggacgcagcagggccgggtcgagaacgtccggacggttagtcgcggcgataacgatgataccttcgttaccttcgaagccatccatctcaaccagcatctggttcagagtctgttcacgttcatcgtgaccaccgcccagaccagcgccacgctggcggcctacggcgtcgatttcatcgataaagatgatgcacggtgccgctttcttcgcctgttcgaacatgtcacgaacacgggatgcacccacaccgacgaacatttctacgaagtcagaaccggagatagtaaagaacggaactttcgcttcgcctgcaatcgctttcgccagcagcgttttaccggtacccggaggaccgaccatcaagacgcctttcgggatcttaccgccgagtttctggaagcggctcggctcgcgcagatactcaaccagttcagcaacttcttcttttgcttcgtcgcagcccgcaacgtcagcaaaggtcgttttgatctgatcttccgtcagcatgcgcgctttgctcttaccaaacgacatggcacctttgccaccgccgccctgcatttgacgcatgaagaagatccagacaccaatcagcaacagcatcgggaaccaggagatgaagatagaagccagcaggcttggttcttcaggcggttcaccgacaaccttgacgttcttggtcaacaggttatccagtaatttcggatcctgaaccggaatgtaagtggtataacggttactatctttcttggtaacgttgatttcacgtccgttgatacgcgcttcacgaacctggtcgttattgacctcttgtaggaaggtagagtaatccaccttacggccattagactcgctgggcccaaagctctggaatactgacatcagcacaacggcaatgaccagccagagtattaggtttttcgccatgtcactcaagggattaacctcttattacaactgtgttaaaaacagcgtcaggatactctatatccagcatctttcaaactttcgtctgaaatctcccggttagggtttacgcccggtcgctacaatatacacttcccgcgaacgtgcacgagaagagtccggcttacgaactttgaccttcgtaaacagggagcgaatttcccttagatactcatcgaaaccttcgccctggaacaccttcactacaaaactgccacctggcgctaatacatcacgacacatttctagcgccagttccaccagatacatggcacgggggatatccaccgccggtgttccgctcatgtttggtgccatatcggacatgacaacctggactttgctgtcgccaacgcgctccagcagtgctttcatcaccagttcatcacgaaaatcgccctgaagaaagtccacaccaacgataggatccataggtaaaagatcgcaagcgatgatgcggcctttgccgccaatttgggtgaccacatattgtgaccaaccacccggagcagcaccaaggtcgacaaccgtcattcccggtttaaagagtttgtcactttgctgtatttcatcaagtttaaaccaggcacgggaacgtaacccctttttctgtgcctgttgaacatatttatcgctaaagtgttcctgaagccagcggctggagctggcagaacgcttcttacctgtcatttaactttcccatggggataactcatcgtaaccaattgcgtaaatttttacgcgcctatttggtgatatatgggagatggcggtagaatgacccgttttcaatcccaacgtaagcaaaaaatacgatgaatctgagtactaaacaaaaacagcacctgaaaggtctggcacatccgctcaagccagttgttctgcttggcagtaatggtttgaccgaaggggtgctggccgagattgaacaagcgttagagcaccatgaactcatcaaggtgaaaatcgccaccgaagatcgcgaaactaaaaccttgatcgtggaagctatcgtgcgcgaaaccggcgcctgtaatgtacaggtcatcggtaaaacgctggtgctttatcgcccaactaaagaacgtaaaatctcgctgccacgctaagattatcctaaagttacacacatttgctgtgtaaaacgaggggttttccgcaggcaggagagcaaaatgccacgctctgttcgttgataaaaggccgcatagcggcctttttcctttctttacaatacatcaacatcttgagtattgggtaattcttacaggtattccaccttaattacttcaaattctacttcgccgcccggcgttttgatgaccacaacatcatcttcttctttgccgatcaggccacgagcaataggcgagtttacagaaatcaggttttgtttaaagtcagcttcgtcatcgccaacgatgcgataagtctgttcttcgtcagaatccagattcagcaccgttacggtagcaccaaaaataacgcgcccattgttgggcattttggtgacatcaatcacctgcgcgttcgacagcttggcttcgatgtctttaatacggccttcgcagaaaccctgctgttcacgagctgcgtggtattcggcgttttctttcaggtcgccatgctcacgcgcttccgcgatagcagcaatgatttcaggacggcgcacagatttcagaaaatccagctcttcgcgtaatttttcagcgccgcgtaaggtcatcggaatagcttgcatttgttatacctcttgaatattcctgatagggcaagtcttcacccaccccggctgttcggcctgcccggcataactccttaccgggaccagaagcaaaaaaataccgacccgggtacaagtcccaggtcagctacaattcacattttgatagtcattttaccctgaagttcccgaagggtcatcgtttactttatagggcgttgcgccgtagtatgacggctcgattccaggttgttagcgcgagattatgcgattttccagatttatcatcggattgaccagctgtatagcgttcagtgttcaggccgcaaatgttgatgagtacattactcaactccccgctggtgccaaccttgccctgatggtgcaaaaagtcggcgcgtcggcccccgctattgattaccacagtcagcagatggcgctgcctgccagtacccagaaagtgattactgcgctggcggcgttgattcaactcggccccgattttcgttttaccacgacgcttgaaaccaaaggcaatgtggaaaacggcgtacttaagggtgacttagtggcgcgatttggtgccgatccgacgttaaaacgtcaggatattcgcaatatggtcgcgactttgaaaaaatctggcgtcaaccaaatcgatggcaatgtgttgatagatacctccattttcgccagccacgataaagcccccggctggccatggaatgacatgacacaatgctttagcgctccgcctgccgccgccatagttgaccgcaactgtttctccgtctcgctctacagtgccccaaagcctggtgatatggcttttatacgcgtggcatcttattaccccgttacgatgttcagccaggtacgcaccctcccccgtggttctgccgaagcgcaatactgcgaactggatgtggtgccaggcgacctgaaccgctttacgctgacgggatgcctgccacaacgttctgagccgctcccgttggcttttgccgtgcaggatggagccagctatgccggtgcaattctgaaagatgagttaaaacaggcgggtatcacctggagcggaacactgctgcgccagactcaggttaacgaacctggaacggtagttgccagtaaacagtcggccccgctgcacgatctgcttaagattatgctgaaaaagtcggacaacatgatcgccgatacggttttccgcatgataggccatgcgcgcttcaatgtgcctggaacatggcgggccgggtcggacgccgtgcgtcagatcctgcgccagcaagccggtgtcgatattggaaacaccattattgccgatggttcagggctttcgcggcataacctgattgcccccgccaccatgatgcaggtgctgcaatacattgcccaacacgacaatgaacttaactttatctccatgctgccgctggcgggctatgacggctctttgcagtaccgtgcaggtctgcatcaggcgggcgtggatggaaaagtctcagcgaaaaccggttcgttgcagggggtatataacctggcgggattcattaccacagcgagcgggcaacgaatggcgtttgtgcaatatctttctggctatgcagtagaacctgcggatcagcgtaatcgccgtattccgttagtgcgttttgaaagccgtttgtataaagatatttatcagaacaattagtcaaaaagaaaccccggcacatggccggggcttcagattattgacaaagtgcgctttgtttatgccggatgcggcgtaaacgccttatccggcctacaaaatcgtgcaaattcaacatattgcaattctcttgtaggcctgataagcgtagcgcatcaggctgatttggcgtttatcatcagtgattaacgcttgtaaatgaactcaacgccttcttcgtcgtcttcgtcccagtcgtcatcccagtcttcatcatcctcttcagcaatctcttcaagctgctggcgatgataatcatcccacatgaattcgactttctctggctgtttcgcttcttcagcctgcacgaccgggttttcaatgataaaggtcatcacatcccagcagagatctttcacgcccagtccactcgccgcagagatcagataatatttatcttcccagcccagcgcctcagcgatcgctttcgctttctcttcggcttctaccttatccagcagatcgatcttgttgaacactaaccaacgcggtttcgtcgccagatcctggctgtatttttccagctcgctgataataatacgcgcgttttcaaccggatcggtgccgtcaatcggatcgatatcgatgaggtgcaacaggacgcggcaacgttccaggtgcttcaggaagcgaatgcccagacctgcgccttccgcagcgccttcaatcagtcctggaatatcggcaacaacgaagctcttttcgttgtccattcgtaccacacccagacttggcaccagagtggtaaacggataatccgccactttcggtttagccgccgataccgcacgaataaaggtcgatttacccgcgtttggcatccccaacataccgacgtcagccagcagcatcagctccagcagcagctcgcgcttatcgcccggcgtgccgttggttttctgccgcggtgtacggttaacggacgatttgaaacgggtattgcccagaccgtgccagccgcccttagcaaccagcagacgctgaccgtgtttggtcatatcgcccatggtttcaccagtaccctggtcgattacacgcgtacctaccggcactttaatcgtcacgtctttaccgcgcttaccggtacagtcgcggcttgcgccattctgaccgcgctctgcacggaaagatttttcaaaacgataatcgataagcgtgttcaggttctcgtcggcttccatccatacgtcaccaccatcaccgccgtcgccgccatccgggccgcctttcggaatatacttttcgcggcggaagctcacgcaaccattaccgccatcacctgcaacgaccagaatcgatgcttcatcaacaaacttcattttattctccgtaaatcattcgcctgcgcggggttgcgataccaccgttgtatgcttacgtaatccgccccaaatacgatgaccaatggcggaatacatcgcgcccgcaaccacgacaaacgcaccgagataacctaaaaggtttaacatcggtctggcgaagaaatcgggccaggccagtgataaaagatctgaaaaaaacagcgtaaacagtggggtgagcgtgatgatcgcgctcacctgcgctgcctgccagcgagccatcgcttccgccagggcgccatatcctaccaaggtattcagtccgcaaaaaattaaacatgcgagctgccagtggctaagctgcgctatcactccaggctttgccagagggaagagcgcaattgtacataaagtgtacagtaaaaacaggatctgcggtgaggccagccgacgcaataaaaccttttgcgccacgccataactcacccaaaccgtcgccgcaccgaccccaaagataactccccaggtgtaatcggtgagctttgtaaatatctcgaccagactggtgttaaaaaacatcaccaggccgctcaggagcatcaatgcccctacaacctgagtgctgcgcattttctctttgaggataaatacgctggcaaccatcatgccaactggcgagagttgcccaatcacctgcgaagcggtcggactcaggtattgcaaggatgagctgaacaggatgaagttcccaaacagcccggcggtcgccactgccaacaaaatcaaccagcgtggcttacgaaacacgcgtaatggcggcaacctcttcttcaccgcaagaatggcacccaggccaatactcgccatcaagaaacggtaaaacacgattgtcggaggttccatcacctccagcacctgcttcattgcgattggcaacgccccccagcaaattgctgtggtgagcgccaaaagaatgccaatgcctgcctgctgcttcataccgtattccctgcaaagcgcatttgcggattaacgtcgcaccatgcgcatttttaccggttatcgaatgtaaaaagccccgcaacgtgttgcggggctttcatccgttaccgggacgcgaaaaacttattcagcttcgatgctgataaatttacggtttttcgggcctttaacttcgaatttcactttaccgtctgctttagcaaacagagtgtggtcacgaccgcaacctacgttagcgccagcgtggaatttggtaccacgttgacgaacgatgatgctacccgccagaacggattcgccaccgaaacgcttaacgcccaggcgtttagcttctgaatcgcgaccgttacgtgtggagccgccagcctttttatgtgccatttgaaatctctcctcaggtcttaggcgctgatgccagtaattttcacatcagtgaaccactgacgatggccctgctgcttacgatagtgtttacgacgacgaaacttaacgattttaactttctcgccacgaccgtgagcaacaacttcagctttgattacgccgccatcaacgaaaggaacgccgattttgacttcttcaccgtttgcgatcatcagcacttcagcgaactcaacagtttcgccagttgcgatgtccagcttttccaggcgaacggtctgaccttcgcttactcggtgttgtttaccaccactttggaaaaccgcgtacatataaaactccgcttccgcgcacaccttttcaatgattcagagtgcgctataaatattcacaatagggcgcgaatattacgcaaaacgcacgcctttgacaagtgctacagtcaatacacgaagaaaaaaaacacaacttgtacggtaacgtttatctgtgccattttttcagtacaatcaccctatattcctaaccataaaccctaagttgcctttgttcacagtaaggtaatcggggcgaaaagcccggcttttgcgatgaatttagaaaaaatcaatgagttaaccgcgcaagatatggcgggtgttaatgcggcaatccttgagcagcttaattccgacgtccaactgatcaatcagttaggctattacatcgtcagcggcggcggtaaacgtattcgtccgatgattgctgtactggctgcacgagctgttggctatgagggaaatgcgcatgtcaccattgctgccctgatcgagtttatccacacggcgactctgctacacgacgacgttgtggatgaatcagatatgcgcaggggtaaagctaccgccaacgccgcatttggcaatgccgccagcgtgctggtaggcgattttatttatacccgcgctttccagatgatgaccagcctcggttcgctcaaagtgctggaagtcatgtcagaagccgtaaacgtcatcgcagaaggtgaagttctgcaactgatgaacgttaacgatccggacatcactgaagaaaactacatgcgcgttatctatagcaaaaccgcgcgtctgtttgaggctgccgcgcagtgttccgggattctggctggctgtacgccggaggaggagaaaggcctgcaggattatgggcgctatctcggcactgctttccagttgatcgacgatttactcgattacaatgccgatggcgaacagttaggtaaaaatgtcggcgacgatctgaacgaaggtaaaccgacgctgccgctgctgcatgcgatgcatcatggcacaccagaacaggcacagatgatccgtaccgccatcgaacagggtaacggtcgccatcttctggaaccggttctggaagcaatgaacgcttgtggatctcttgaatggacgcgtcagcgtgccgaggaagaagcagacaaagccatcgcagcgttacaggtgctcccggacaccccttggcgagaagcactcatcggcctcgcgcacatcgctgttcaacgcgatcgttaatcccctcccctcatcccgcgcagcgcgcgggatggttccagtaagttccataaaaacacttattcagctctataacacctgaaaaatagggatgtgcatctttatatattctgaatattcacactctttacaggaactttttagagcaataggccatcaggagtatagtgatgctcgacagaagaagtgttctgaatgaaagcgactaacttaaggagtgaggaaaaatggaaagtaatttcattgactggcatcccgctgacatcattgcgggtttgcgcaagaagggaacgtcaatggcggcggaatctcgcagaaatggtttgagttcctcaacgctggcgaatgcattatcgcgcccatggccgaaaggagagatgattattgcgaaagccctgggaactgacccctgggttatctggccatcacgctaccatgatccgcagacccatgagtttatcgacagaacgcagttgatgcgtagctacactaaaccgaaaaaatgagtggtctggcggtagccccgcgaacggggctgccagctctcagacgattattcgcctttcacacgctcaatatttgcacctaaagcgcgcagtttgtcttcaatgcgttcgtagccacgatcgatgtgataaatacgatcaaccaccgtcgtcccttccgcaatacagccagccagcaccaggcttgctgatgcacgcagatcggttgccataacctgtgcgccagaaagtttttcaacaccgtgacaaataacggtattgctttcgatttcggcgtgcgcgcccatacggctcagctctggcacatgcataaagcggttttcaaagaccgtttcggtgataaacccggtcccttctgccaccaggttcaacagcgtgaactgggcctgcatatcggtcgggaatgccggatgcggcgcggtacgtacgttaacagccttcggacgtttgccatgcatatccaggctaatccagtcttcgccgacttcgatgtccgctccagcgtcacgcagtttcgccagcacggcgtcgagagtatctggctgcgcgttacggcagataattttgccgcgagaaatcgccgccgccaccaggaaagtaccggtttcgatacgatccggcagaacgcgatagacaccgccgcctaaacgttccacaccttcgatgacgatacgatcggtgccctgaccgctaattttcgcacccagcgtaatcaggaagttcgcggtatcgacgatttccggttcacgcgctgcgttttcaataatcgtggtgccttccgccagggttgcagcacacatgatggtcaccgttgcgccaacgctgactttatccatcacgatatgtgcacctttcaaacgaccatcgacggaagctttaacgtaaccttcttccagtttgatggtcgcgcctaattgttcgaggccagaaatgtgtagatcaaccggacgcgcaccgatcgtacaaccgccaggtagtgaaacttgcccctgaccaaagcgcgctaccagcggccccagcgcccagatagaagcacgcatggttttaaccagatcgtaaggtgcgcagaatacattaacgtcgcgggcatcaatatgcacagaaccattacgttctactttcgcacccagctggcttagcagcttcattgatgtatcgacgtctttcagtttcgggacgttctggatctctaccggttcttccgccagtagtgcggcaaaaaggataggcagagcagcatttttagcgccggaaattgtgacttcgccctggagcttcgttggcccctgaacacgaaatttatccatttagtttgttctcagttaacaattcatatccgctaccggcgaatcgcccatagctcaaaagccgttcagtttgcgatcgcgcgcccactccgcaggggtatacgctttgatcgacacagcatgaatgcggttatccgcaatatattccatcagcggaccatagaccgtctgctgttttttaacccgactcatgccgtcaaacaactcacccacggcaataacctgaaagtggctgccatcgccggaaacgtggacttcctggagggagagagcgttcatcaacacgctctgaatttcattattttccatgggatcttcaatcatcagttaataaaccagcgaaacatcttagagcaaagttgcgctggcataaataagcaaaaagcctcgctgataaatcagacaaggctcgacttgcaggcaggtttgccggacaggcggttaacgccatatccggcctgaaaaaatttaacgaggcagaacatcagcaggcaaattatacaatttcgccagggtatacactttgtcgtttaccccctgaagcgtcacattgttgccctgctttttcgccagatcgataagatggagcagcagtgccagtccccccgtatccacgcgggagacacggctaagatcgatgcaggtaatccccttcaccgcttcctcacgcatttcccaaagcggtagcaaaacgtcctgatccagctctccggataacgccagcgtgtcacccgtctgcatccagctcagtgactcgctcattattttttctcttccagagtgattttctgttgagaaatcgatttcagttgcgcagtcaggccgtcgatacctttggtacgcagcagcgttccccactcgttttgtttggtggtgatcatactgacgccttcagcaatcatgtcgtaagcctgccaattgcccgtctgggagtttttacgccactggaagtccagacgcaccggcggacggccattcgggtcaataatggtaacgcgaataggcacaatggttttatcgcccagcggctgttctggcgcaatctgataggtttgaccgtgatacatcgccagcgcctgaccgtaagcctgcttcaggtactcacggaaagcggcaaagtaggcttcacgttgagcaggggtcgcactcttgtaatactggcccagcaccagcgcaccggcgtatttcacctgtacgtatggcagcagttcctgatcaacaatggtacgcagataatccgggttggcccgaatttgcggttgctcattcttcaggcgatcgaacgttttctgcgccgcctcgtccatcagcttatacggattggtctggtctgccgcggttgccgcactcagaggtgcaatcaccagcaaagcgaccatcattaaacgtttaaacatgcgtcggttctcctgaaattatttcgttgtacccacaggttcagtggtttcattattacctggcgcagcagctggcgcatcgccactattcttattgtcatcgcctttactaccgtaaaggaactgaccaatgagatcttccagcaccatcgcagacttagtgtcctgaattgtatcgccatccttcaggatagcagtccccagttccgggtcttcaaaaccgacgtttaatgccagatattgttcccccagcaggccggaagtacgaatgctcagcgaactggtatctggaatgtggttataacgttgttcaatttccagcgttacgcgcggcagataggttttcgggtccagcgtaatatccgccacccgacccacaacaacgccaccaatactgaccggagagcgcgctttcaggccgccaatgttatcgaacgtcgcataaagcgtgtaggtcggttcagtacgtatggacgtcacgttcgccgccttcaggcaaacaaacagcgccgccagcagtgctgctaataaaaagatacccacccaaatttcattttttttcgtttgcatgaactcaattcccaaacatcaatgcggtcagcacaaaatccagccccagaacagccagagacgagtggacaacggtgcgagtggttgcccggctaatcccggcagacgtcgggatggcgtcgtagccgttaaacaacgaaatccacgtcaccgtgatggcgaacaccacgctcttaatcagacagttgaccagatccatacgccagtcgacggcattttgcattgccgaccagaagaacccgctatcaatgcctttccaactgacgccgaccagagatccgccccagatccccacggcgacgaaaataaccgtcaacagtggtaatgaaataaccccagcccagaaacggggagaaataacccgacgcagcggatccaccgccatcatctccatactggagagttgctctgtagcgcgcatcaggccgatttctgcggttagcgccgaaccagcacgcccggcaaacaacaacgcggcaaccaccggccccagttcacgcagtagcgataacgccaccagcatacccagactggtttccgcactataagtggtcagaaccagataaccttgcagccccaacaccattccgatgaacacgccagaaaccacaataatcagcatcgacaggacgccgacattatagagctggcgcaccagcagcggcgcatgtttgcgaaattccggtttgccgaccagcgcattgaataacattaacccggcccgcccgaacgttctcagggttttaatccctttatgtccgagcgacgccagcgcatttaacagcatgagtggcttaactccctggtaaaagatcagcgtgataatcgccggcaggatagcggaacggaacaggcccgtcagctatcccgtccagaaactgacgtacgcgcggatcaggattcgcctgcaacgcctgggcactgccatgagcgacaatttttttgtccgccaggatccaggcgtgatccgcaatacttaacacttccggcacatcgtgagaaaccaccacacaagtcacgcccagcgcgctgttcagctcagaaatcagcttcaccagtacgcccatggtgatgggatcttgcccaacaaaaggttcatcaaacatgatgagatccggctccagcgcaatcgcacgcgccagcgctgcacgccgcgccatcccaccggaaagttcagaaggcattagtttagccgctccacgcagccccacggcctccagcttcatcatcaccgtactatgcaacaatggcgcgggaagttgggtatgttcgcgcagtggataggcgacgttgtcaaatacgttcatatcagtgaacaacgccccggactgaaataacatgctcatccgtttgcgcactgtatacaggcgcgaacgagacatcgccggaatattctcaccatcgaaaaggatctcaccatgatctggtgcgatttgcccgccaatcagacggagtagcgtcgttttaccgatgcccgatggccccatgatcgccgtgatcttccctcgcggcacggtcagggaaatattatcgaagatgcagcgattgccacgcgtaaaactgacatcgcgcatatcgactaaattcgccacagactgctccataattcacccttcgtcttgcgttgattttctaagcatggcgctcaatttaaccttgaacccaacatatttacagaatattacccgccgtggttagcgaaagctggcatttgttttactttttagccgcataaagtcaaaattaagcatccgttacggctttctgaaaatcttcagcggaccggcgagtatacctgaagaaaggacgttagatgcttttagctacggcactgttaattgttggtttacttttggtcgtttacagtgccgaccgcctggtttttgccgcgtctattctttgccgaacctttggcatcccgccgctgatcatcggcatgacggtggtcagtattggtacatcgttaccagaagtcatcgtctcgcttgccgcgtctctgcacgaacaacgcgatttagccgttggtacagccctcggctcaaacattatcaatatattgctgatcctcggtctggctgcgctggttcgtccttttaccgtccattctgatgttctacgccgtgaattacccttaatgttgttggtcagcgtggtggccggttccgtactctatgacggacaacttagtcgcagcgatggtatctttctcctctttctggctgtgctatggctgctgttcattgttaaacttgcacgtcaggctgaacgtcaggggactgacagcctgaccagagagcagcttgcagagctgccgcgtgacggcggattgcccgtcgcgtttttatggctcggcattgcgcttatcatcatgccagtggccacgcggatggtggttgataacgccacggtgctggcgaattactttgccatcagcgagttgacgatgggtctgacggcaattgctatcggaaccagcctgccggaactggcaaccgcaatagcgggggttcgcaaaggtgaaaacgacattgctgtcggaaatatcattggcgcaaacatttttaatattgtcatcgtgttgggtttacccgcgctgataacgccaggagagattgatccactggcgtacagtcgtgactacagcgtgatgttgctggtgagcattatttttgcgttgctgtgctggcggcgctccccgcaaccgggccgtggtgtaggggtattattaactggcggatttatcgtatggctggcgatgttgtactggttatcgccaatactcgttgaataactggaaacgcattatgtcgcacgtagagttacaaccgggttttgactttcagcaagcaggtaaagaagtcctggcgattgaacgtgaatgcctggcggagcttgatcaatacatcaatcagaatttcacgcttgcctgtgaaaagatgttctggtgtaaagggaaagttgtcgtcatggggatgggaaaatcggggcatattgggcgaaaaatggcggcaacgtttgccagcaccggtacaccttcatttttcgtccatcctggtgaagccgcgcatggtgatttaggcatggttaccccacaggatgtggtgattgctatctctaactctggtgaatccagcgaaatcacggccttaattccagtgcttaagcgtcttcacgtaccgttaatctgcatcaccggtcgcccggagagcagcatggcgcgcgccgcagatgtgcatctgtgtgttaaagtagcgaaagaagcctgtccgttagggctggcaccgaccagcagcaccaccgccacgctggttatgggcgatgccctcgctgtcgcgctgttaaaagcacgcggctttactgctgaagattttgcgctctcacacccaggcggcgcactgggtcgtaaacttctgctgcgcgtaaacgatattatgcatacgggcgatgagatcccgcatgttaagaaaacggccagtctgcgtgacgcgttgctggaagttacccgcaaaaatcttggtatgactgtcatttgcgatgacaatatgatgattgaaggcatctttaccgacggtgatttacgccgtgtcttcgatatgggcgtggatgttcgtcagttaagtattgccgatgtgatgacgccggggggaatacgtgtgcgccctggcattctggccgttgaggcactgaacttaatgcagtcccgccatatcacctccgtgatggttgccgatggcgaccatttactcggtgtgttacatatgcatgatttactgcgtgcaggcgtagtgtaaagattcaaggataaacaacaatgagcaaagcaggtgcgtcgcttgcgacctgttacggccctgtcagcgccgacgttatagcaaaagcagagaacattcgtctgctgatcctcgatgtcgatggcgtactgtcagatggcctgatttatatgggcaataatggcgaagagctgaaagcgttcaatgttcgtgacggttatggcattcgttgtgcgctcacctctgatattgaagtcgctatcattaccgggcgaaaggctaaactggtagaagatcgttgtgccacattggggatcactcacttgtatcaggggcagtcaaacaaactgatcgcctttagcgatctgctggaaaaactggcgattgccccggaaaatgtggcttatgtcggcgatgatctcatcgactggccggtaatggaaaaagtgggtttaagcgtcgccgtggccgatgcgcatccactgttgatcccgcgcgccgattacgtgacgcgcattgctggcggtcgtggcgcagtgcgcgaagtttgcgacttattactcctggcgcagggcaaactggatgaagccaaagggcaatcgatatgagtaaagccagacgttgggttatcattgtgctatcactggcggttctggtgatgatcggcattaatatggccgaaaaagacgataccgcccaggtggtcgtcaacaacaatgatcccacctataaaagcgagcatacggacacgctcgtctataacccagaaggggcactaagctatcgattgattgctcaacacgttgaatattattccgatcaggccgtttcgtggtttacgcagccggtacttaccacgtttgataaggataaaatcccgacatggtccgtaaaagcagataaagccaagctgaccaatgaccggatgctctatttatatggacacgttgaagtcaacgcacttgtgccagactctcaacttcgcagaatcacgacggataacgcgcagatcaatctggtgacgcaggatgttacctctgaagacctcgtcacgttatacggaacaacatttaactccagcggtctgaaaatgcgcggcaacttacgcagcaagaacgccgagctgattgaaaaggttagaacatcctatgaaattcaaaacaaacaaactcagccttaatcttgtgcttgccagctcacttctggccgccagcattccggcatttgccgtaaccggagacactgatcagccgatccacattgaatcggaccagcaatctcttgatatgcaaggcaacgtggttacctttaccggtaatgtcatcgtcacccagggcaccatcaaaattaatgccgacaaagtggtcgttacccgtccgggcggcgaacaaggtaaagaagtgattgacggctacggtaaaccggcaacgttctaccagatgcaggacaacggtaaacccgttgaaggtcacgcttcccagatgcactacgaactggcaaaagattttgtcgttctgacgggtaatgcttatctgcagcaggtcgatagcaacattaagggcgataagatcacttacctggtgaaagagcagaaaatgcaggctttcagcgacaaaggcaagcgcgtaacaaccgttctggtgccgtcgcagctgcaggacaaaaacaacaaaggccagaccccggcacagaagaagggtaattaattcgttatggcaacattaactgcaaagaaccttgcaaaagcctataaaggccgtcgcgtggtagaagacgtcagcctgaccgtcaactccggggaaattgtcggtctgctggggccaaacggtgccggtaagaccaccactttctacatggttgtaggcattgtgccgcgcgatgcgggcaacatcattattgatgatgacgatatcagtctgctgcctctgcatgcacgcgcgcgccgcggtatcggctatctgccacaggaagcctccattttccgtcgcctcagcgtttacgataacctgatggcggtactgcaaattcgtgacgacttgtctgctgaacaacgtgaagaccgcgcgaacgagctgatggaagagtttcacattgagcacctgcgtgacagcatggggcagtcactctccgggggtgaacgtcgccgtgtagaaattgcccgcgcactggctgcgaatccgaaatttattctgctcgacgaaccgtttgccggggttgacccgatctcggttatcgacattaaacgcatcattgagcacctgcgcgacagcggcctgggcgtgctgatcactgaccacaacgtgcgtgaaacactggcggtttgtgaacgcgcttatatcgtcagtcaggggcatttgatcgcccacggcacgcctacagaaatcttacaagacgaacacgttaagcgtgtataccttggggaagacttcagactctgatagggtagaagtttgcgacgttttagcaggagagtacgattctgaacatgaagcaaggtttgcaactcaggcttagccaacaactggcgatgacgccacagctccaacaggcaattcgtctgttgcagttgtcgacgctggaacttcagcaggagctacagcaggcgctggagagtaatccgctgcttgagcaaatcgacactcatgaagaaatcgacacccgcgaaacgcaagacagtgaaacgctggacaccgccgacgcgctcgaacaaaaagagatgccggaagagctgccgctcgatgccagttgggacaccatttacaccgctggtacaccatccggcaccagcggtgactacattgacgacgagctgccggtctaccagggcgaaacgacgcagaccttgcaggattacctgatgtggcaggttgagctgacaccgttttccgacactgaccgcgctattgctacctctatcgtcgatgccgttgatgaaaccggttatctgactgtcccgctggaagatattctcgaaagtataggcgatgaagagatcgacatcgacgaagttgaagccgtccttaagcggatccaacggtttgatccggtcggtgtggcggcaaaagatctgcgtgactgtctgctgatccaactctcccaattcgataagaccacgccgtggctggaagaggccagactgatcattagcgatcatctcgatctgttagccaatcacgacttccgcactttaatgcgcgtcacgcgtctgaaagaagatgtgctgaaagaagccgtcaatctgatccagtcgctcgatccgcgccccgggcagtcgatccagactggcgaacctgagtatgtcattccagatgtgctggtgcgtaagcataacggtcactggacggtagaactcaacagtgacagcattccgcgtctgcaaatcaaccagcactacgcctcgatgtgcaataacgcgcgcaacgatggtgacagccagtttatccgcagcaatctgcaggatgccaaatggttgatcaagagtctggaaagccgtaacgatacgctactgcgcgtgagtcgctgtatcgttgaacagcagcaagccttctttgagcaaggtgaagaatatatgaaaccgatggtactggccgatatcgcccaggctgtcgaaatgcatgaatcgacgatatctcgcgtgaccacgcaaaaatacctgcatagtccacgaggcatttttgaactgaagtatttcttttccagtcacgtcaataccgagggcggcggcgaagcttcctccacggcgattcgtgcgctggtgaagaaattaatcgcggcggaaaacccagcgaaaccgttgagcgacagcaagttaacctctttgctgtcggaacaaggtatcatggtggcacgccgcactgttgcgaagtaccgagagtctttatccattccgccgtcaaaccagcgtaaacaactcgtttgacccaaccgataaggaagacactatgcagctcaacattaccggaaataacgtcgagatcaccgaggcactgcgcgaatttgttacagccaaatttgccaaacttgagcaatattttgaccgaatcaaccaggtctatgttgttctgaaagtggagaaagtcacccacacctcagatgcaacactgcatgtaaacggtggtgaaattcatgccagcgcggaaggtcaggacatgtacgctgccattgatggcttaattgataagctggcacgccagttgaccaaacataaagataaactgaaacaacactaattgtccgggcaattagcatgtgcatggcggtctgttgtgcggcacaacgggccatttgtacggttaatgctccgagcctgttccactgtttgagtgggcaggttcttaggtgaaattatgacaaataatgatacaactctacagcttagcagtgttcttaacagggaatgtacgcgaagccgcgtccactgtcagagcaaaaaacgcgccctggaaatcatcagcgagctggcggcgaaacaacttagcctgccgcctcaggtggtttttgaagctatcctgacgcgggaaaaaatgggcagtaccggtatcggcaatggtattgccattccgcatggcaaactggaagaagatactctgcgcgccgttggcgttttcgttcagctcgaaacgcctatagctttcgatgccatcgacaaccaaccggtggacttactttttgccctgctggtgccggcagaccaaactaaaacgcacctgcatactctgtcgctggtggcgaaacgtctggcggacaaaaccatctgccgccgtttacgcgcagcccagagcgatgaagagctgtatcaaatcattacggataccgaaggtactccggatgaagcgtagttattcggtaatgtctcttttagacgttgtgaggagaaacagtacatggtactgatgatcgtcagcggacgttcaggttcaggtaaatctgtcgccctgcgtgcgctggaagatatgggtttttactgcgtggataaccttcccgtagtgttgttacccgatctggctcgaaccctggccgatcgcgagatttctgccgccgtcagcattgatgttcgtaatatgccggagtcaccagaaatattcgaacaggcgatgagtaacctgcctgacgctttctcaccgcaactcctgttcctggatgccgaccgtaataccttaattcgtcgttacagtgacacgcgccgactgcatccgctttccagcaaaaacctgtcgctggaaagtgctatcgacaaagaaagcgatttgctggagcctctgcgttcgcgagcggatctgattgtcgatacctcagaaatgtccgttcacgagctggctgaaatgctgcgtacccgtctgctgggtaaacgtgaacgcgaactgaccatggtctttgagtctttcggcttcaaacacggtatccctatcgatgcagattacgtctttgacgtgcgcttcttgccgaacccgcactgggatccgaaactgcgtccaatgacaggtcttgataaacctgtcgccgcgttcctcgaccgccacacagaagtacacaattttatctaccagacgcgaagctatcttgagctatggttacctatgctggaaaccaacaaccgtagctacttgacggtcgccattggttgtaccggcgggaagcaccgttcggtgtatattgcagagcaactggcagactacttccgctcgcgcggtaaaaacgtccagtcacgccatcgtacgctggaaaaacgtaaaccatgaccgtcaagcaaactgttgaaatcacaaacaagctgggcatgcatgcccggcctgcaatgaagctgtttgaattaatgcagggttttgacgctgaagtgctcttacgtaatgacgaaggcaccgaggctgaagccaacagcgttattgcgctgctgatgttggattctgccaaaggacggcagattgaagttgaagcgaccggtccacaggaagaggaagcactggccgccgttatcgccctctttaattctggttttgatgaagattaatcttcatcactttgacatacaactcccttcaaactccccccgacaataagaaaatcacgtactgaaatcgttctcaatcaacgtcatttgtacattttgtgcgcttttcactttcagaagaaccttaagaaaaccttaagaggcattgtttaggttttgtttaagttaatcgaccatactggagatcgtcagaaaatatttccaggagatggcatgattcgcttatctgaacaaagtcccctgggcaccggaagacatcggaaatgttatgcgcatccggaagatgcccaacgctgtatcaagattgtctaccatcgtggcgatggtggcgataaagagatccgccgtgagttaaagtactacgcgcatcttggtcgccggttaaaagactggagtggaataccgcgctatcacggtaccgttgagacggattgcggaaccggttatgtctacgatgtgattgcagattttgacggcaagccttccattacgctgaccgaatttgctgaacaatgccgttacgaagaagacattgcacaactgcgccagctactgaaacagctgaagcgttatttgcaggataaccgtatcgtgacgatgtcgctgaagccgcagaatatcctctgtcaccgcatcagtgagtcagaggttatcccggtcgtctgcgacaacattggtgaaagcacattgattccactggcgacctggtcgaagtggtgttgtctgcgtaagcaagagcggttatggaaacgatttatcgcccaaccggcgctggctattgccctgcagaaagatctgcaacctcgtgagagcaaaacgctggccctcacttcgcgcgaagcttaatccagctggtgttgttgcataaacggctcaccgcctaactgatacatctgccgtaaaatccacgcctgacggctacgcacgtagcccgatggcgaggagactttgaaacgaagtggattaggtaatacagctgccagtaatgcagcttccgaccgggtaagtttgctcgcgggtttgtggaaataacgttgtgccgcagcttcgacgccaaacacaccgtcgccaaattcggcgatattcaggtaaaccgtcaggatacgctttttgctccagaccgtttctatccccagcgttaatccggcttccagcccttttcgaacccagctacgcccatcccataaaaagagatttttggctgtctgttgagaaatcgttgaagcaccgcgaatacggttttcattgcgctcgttgtgcgccagggctttctcaatggaagcgacatcaaagccccagtgctcaggaaatttctgatcttctgcggcaatcaccgccagtcccatccacggcgagatttgatccatactgacccagtcagaatgtgccacgtaacgaaaattgccatgcagccaggcgctgacctgtcgctcgaccattaccgctgagaagggaacaggcgcaacgctaaacaacgcgatgcccccgccccagaaaacggcgaggacaaccattaaccgcaaaagaaaacggcgaacgaaactaaacaccgttaagcggcttttactcattcagccagaaccagcacgcgggaaaccagcttatcaatgccgctcgccgcttctgcaatgttctgcgccagcatatatgctggggtggtgacaatcttattgtcttcatcaaccacgatatcatcgacaggacacggcacatgctccgcgcccatctcttccagcacttctgcggtatcgatatcagtaccgatggtcaaacgcagcgggaaatcgaaaattttcggcagcatcgccggggcaatacacataaaaccaagcggttttccggcctgatgcatcgcttgtgccagcgcctttaattcacggtcaacggtgcattcgctaccaagactggcaaaattgcttaaattcttcgccgcgccaaacccccccggcacaatcaacgcatccagttcagcggcatcggcctgggccagaggacggatttcaccgcgcgttattcgtgccgcttcaatcagcacattgcgcgtttccgtcatcgcttcgccagttaaatggttgataacatcaacctgctgcttatccggtgcaaagcagaccgcctgcgcaccgctgcgtgaaatagctaacaacgtcaacaccgcttcatgaatttcagaaccgtcatagacgccgcatccgctcagaattacgccaattttcttcattgtgatcatcctttcgcaattgactgaaacacattaatttttttaataaaaatggtacgcatcacacatttaactgattcatgtaacaaatcatttaagttttgctatcttaactgcgtgcggcctgaaaaacagtgctgtgcccttgtaactcatcataataatttacggcgcagccaagatttccctggtgttggcgcagtattcgcgcaccccggtctagccggggtcattttttagtggcttttgccacccacgctttcagcacttctacgtcgtgacgccactcttctttcatctcttcaatccattcaccgacgttatcttcccaggccggaaggtcaggagactgaatttgctgacccagctgttgcagatggcgtaaccccactgaccccgccgcacctttaattttatgtccttcctcaacaatgccttttttatcctgcgccgtcagattcgactccagcacgctgacatagcccggcatcatcttctcaaacaccgctaacccgtcggtgatcagcttcggtcctacaagttcgagatactgttccagcatgggaatatcgagcaatgcttctgatttactgttctcttctgtcgtcaccgtactctcctcatcatcctgggtatcccagaatttcttgatcatcgcggttagcgccggaacagaaagcggcttactcagcacatcatccattccagcattgaggtactcttgtttgtctttcagcacgttagcggttaaggccaccagcggcggtaaatcctcgcgcggataacgtttcgtcagttcacgagagatatccagcccggtcatatctggcaactgaatatccagcaacaccaggtcgtattcgcccggtttaaacatctccagcgccgccttgccggtcatggcgacatcaacgctgttacctaatttttccagcacagaacgcgcaacaatcacgttcagttcaatgtcttccaccagcagcacattcagcgccggtaaaggcatatcgtcttcatcaaacgcatcatcgacctcttctgctaccgacggtgcgtggatcgtcaacgtaaaggttgaacctttgccctgttcgctggtaaccgtaatatcgccgcccatatttttcgccagacgacgagaaacggccagaccaataccggtgccggtggcaggtttaccgccatgactgtctttcacctggtaatacatggcgaaaattttatccagctcatcctgcggaatgccgataccagagtcttccacttcaaaatgcagcatatcgccttcatcgtagcgcacgcgcacggtaacctggccttgctgggtgaatttgacggcgttactgatgaggttccacaggatctgccgtaaacgcgtcccgtcggtaatgacctgatgcggtaatggcagcgtcggctccaggttaaagcgcaatcctttttgttgcgcctgcaatgcggagagattttccagatcggcaaggaagctggtgaaatcaaccggttgattatcaagctggaccttgcgccgttccatcttatccatgtcgataatatcgttaaagatattccccagcgtgacggccgaaacatggatggtcttgagatatttttcctgctcggcggtgagttcggtatccagcagaatgcggctcagaccgacgataccgttcagcggtgtacgcaattcgtgactgatggtggagataaacgtcgttttgtcgcggctggcccgttcaagcgcatcctgataccgcttacgctcggtaatgtcgcgaccaaagcccatcaaaccgtgacgtttacccacgcggtcgtagtacggcactttacggatttcaaagcaggctttgcgcccgtccgggtaatccagccactgttcataggtcagtgacacattatgacggaacactttttcatcggtttcaatgacttttgcggcggcttccggtgagtaaacatcagcaggtttcaggtgaaccagttgtttttcgctttttccggtcagcagctccatcgcgcggttacagccggaaaactctttatcttcgttacgataaaaaaccaggtcgggtgaagcatcaaggaaggaacgtaagaatgaggattgctgctcgagctgaatttgtgtctcttcgcgctctttgatttcaattttcagttggccgaaggtttcctgcagttctgcttccgctttttcacgaacggcaatttcctgatttagctgggcaatattatcttttaactgaacgttgaggctcaaatcgcgctcgcgcatctcctccagtttttgcaccagccgtgacagacgttgtcgtgactcctccagttgctcgacgaccaccgatagaaagtagaccgcccacggcgtaatcagcaaaccaaagaagatagaacgaataacatcaatgctttcgacctgaccatgcagcaccatggttaccgccatttgtaccacaatggcaagaacgacgagggccagcgccagcaacattgagaagcgcaccagacctaacttcatcatcaggtcaacataatactgcgccagcagacgaatttgcttcattagggaattccttcacgacaacctgccccaataatacccaattctgacagttacgttataaattgtgtgagaaatgcggaattcccctcaacgacctactccgttggaggtagccacggacgtcccagcgccgatccctgtacgccatgttcattcagatagcgatccagctcgaccattcccgtccatcgattttcgcaccacagcggagcaagcagcgtcgggcgacgggcgctggcggaaatgcggtggtagatcacttccggtggcgtatggcgaatcatttctccggcagtgagcgtgtaatcctccagttcaataccgttcaaacgccccgcttcccaggctttcgccataatgctgcctttcacaatatgcagcggatgcagctttatgccgtccacgccggtttcaaccactcgctccagcgtttgcaaacattcagcctgcccttcgccaggcaggccgacaattaagtgggaacacaccttcagcccgcgctgacgtgccagctgggttgtacgctgataacaggcaaaatcatggccgcggttgatgcgatgcagtgttttgtcgtgggcggtttgtagccccagctccagccacacttcgtaaccctggtccttatattcgcaaagcagatccagcaccgcatccggcacgcagtccgggcgggtacccacacacaaaccgacaatattggcctggctcaccgcctgctgatacatagaacgcagcacctgaacttccgcaaaggtgctggtatacgcctgaaagtaggccagatagcgtttagcgcggttaactaaattcgcctggtgcgccagttgctcggcaatggaacgatgctgctgcgcttcatcggcaaacgaggcaacattacagaatgtgcagccaccacgcccgatggtaccgtcacggttagggcagctaaaaccgccgtgcagcgtcagcttatgcaccttttgcccataacgacgggtgagatcaccaccaaacatattgactaatttctgtaactgcataatctgatagaccgcgccttgaaaagaggccaaagcctgccatttttagctcaattcggcgatgacctggatcaatcgtcccggcctgcttttatcaactgcataatcaatcaaaattaccgaaatttcatgcataatcacataaatcacttttgcttatcttgtgtcagatttttttatctcctgatggattttaggcaaaaacagtagcatgaaacgtcattaccaattaaggcagtataaaatgctggttttgtcgtcagttcaaggcaggataagggttaacacacctttatgacagtcaggaattgactgtttctctaacgacttcccttttagccttaaagataaaatccattttaatttcagtcatttaataaagaattttgcgctaaagcacatttctgtaccaataagcttgccatttgacctgtatcagctttcccgataagttggaaatccgctggaagctttctggatgagcagcctgctcatcatatttatgcagtaattgagatcccctcttcaccgtattaaccgatgcgaaaaggacaacaagggggcgaatgcgaggcgcgcgtatgacacgcaaaccccgtcgccacgctctttctgtgcccgtgcgcagcggttcggaagtggggttcccgcagagcctgggggaggttcacgatatgttgtacgataaatcccttgagagggataactgtggtttcggcctgatcgcccacatagaaggcgaacctagccacaaggtagtgcgtactgcaatacacgcactggcccgcatgcagcaccgtggcgcgattctcgccgatggtaaaaccggcgacggttgcggcttgctgttacaaaaaccggatcgcttttttcgcatcgttgcgcaggagcgcggctggcgtttagcaaaaaactacgctgtcgggatgctcttcctgaataaagatcctgaactcgccgctgccgcacgccgcatcgttgaagaagaactgcaacgcgaaaccttgtcgattgtgggctggcgtgatgtccccactaacgaaggcgtgctgggtgaaatcgccctctcctctctgccacgcattgagcaaatttttgtgaacgccccggcaggctggcgtccacgcgatatggagcgccgtctgtttatcgcccgccgccgcattgaaaagcgtctcgaagccgacaaagacttctacgtctgtagcctgtcgaatctggtgaacatctataaaggtctgtgtatgccgacggatctgccgcgcttttatctggatcttgcggacctgcgtctggaatcggccatttgcctgttccaccagcgcttctccactaacaccgtaccgcgctggccgctggcgcaaccgttccgctatctggcgcataacggtgaaatcaacaccatcaccggtaaccgccaatgggcgcgtgcgcgtacttataaattccagacaccgcttatccctgacctgcacgacgccgcaccgttcgtcaacgaaaccggctctgactccagttcgatggataacatgctggaactgctgctggcaggcgggatggatatcatccgcgccatgcgtctattagtaccacccgcctggcagaacaacccggatatggacccggaactgcgtgccttctttgactttaactccatgcatatggagccgtgggatggcccggcgggcatcgtgatgtccgacggtcgttttgccgcctgtaacctcgaccgtaacggtctgcgtccggcgcgctacgtcatcaccaaagataagctcatcacctgcgcctctgaagtcggtatctgggattaccagcctgacgaagtggtcgaaaaaggccgcgtcgggccaggcgaactgatggttatcgacacccgcagtgggcgtattctgcactcggcagaaaccgatgacgatctgaaaagccgccatccatataaagagtggatggagaaaaacgtccgccgactggtaccgtttgaagatctgcccgatgaagaagtgggtagccgcgaactggacgacgacacgcttgccagctaccagaaacagtttaactacagcgcggaagagctggactccgtaattcgcgtactgggcgaaaacggtcaggaagcggtcggttcgatgggcgatgataccccattcgccgtgctctccagtcagccgcgcattatttacgactacttccgccagcagtttgcccaggtgactaacccgccaatcgacccgctgcgtgaagcgcatgttatgtcgctcgccaccagtatcggtcgtgaaatgaacgtcttttgcgaagcagagggccaggcgcaccgtttaagctttaaatcgccgattctgctctactccgatttcaaacagctcacgacgatgaaagaggagcactaccgcgcagatacgctggatatcacctttgacgtcactaaaaccacgctcgaagcgacagtcaaagagctgtgcgacaaagccgaaaaaatggtacgtagcggcaccgtgctgctggtgctctccgaccggaatatcgctaaagatcgcctgccggttccagccccgatggcggttggcgcgatccagacccgtctggtcgatcaaagcctgcgttgcgatgccaacatcatcgtcgaaaccgccagcgcccgcgatccgcaccacttcgccgtgttgctgggcttcggcgcgacggctatttatccataccttgcctatgaaacgctgggccgcctggtagacacccatgcgattgccaaagattatcgtaccgtgatgctcaactaccgtaacggcatcaacaaaggcttgtacaaaatcatgtccaaaatgggcatctccaccatcgcctcttaccgctgctcgaaactgtttgaagcggtcggtctacacgatgatgtagtgggcctgtgcttccagggggcggtcagccgcattggtggagcaagctttgaagacttccagcaggatctgctgaatctgtcgaaacgtgcctggctggcgcgtaagcccatcagccagggcggtctgctgaaatacgtccacggcggcgaataccacgcctacaacccggacgtggtgcgcacgctgcaacaagcggtacaaagcggcgagtacagcgactatcaggaatacgcgaagctggttaatgagcgtccggcaaccacgctgcgcgatctgctggcaattacgccgggtgaaaacgcggtcaacattgctgatgttgaaccggcaagcgaactgtttaaacgctttgataccgccgcgatgtctatcggcgcgttaagcccggaagcccacgaggcgctggcggaagcgatgaacagcatcggcggtaattcgaactccggtgaaggcggcgaagacccggcgcgctacggcaccaacaaagtgtcgcgcatcaagcaggtggcttccggtcgctttggggttactccggcgtatctggtcaatgccgacgtcattcagattaaagtcgcccagggcgcgaagccaggcgaaggcggtcagttgccgggtgataaagtcacgccttacatcgccaaactgcgctattcggtgcccggagtgacgctgatctccccgccgccgcaccacgatatctactctatcgaggacttagcgcagctcattttcgacctcaagcaggttaacccgaaagcgatgatctccgtgaagctggtttccgaaccgggagtaggcaccatcgcgactggcgtggcaaaagcttatgcggacttgatcaccatcgcaggctatgacggcggcaccggcgcaagtccgctttcatcggtgaaatacgcaggctgtccgtgggagctggggcttgttgaaacccagcaggcgctggttgctaacggcttgcgtcacaagatccgtttgcaggtcgatggcggcctgaaaacgggtgtcgatatcatcaaggcggcgattctcggcgcagaaagcttcggcttcggcactggcccgatggtggcgctcggctgtaaatatctacgtatttgccatctgaacaactgcgcaacgggtgtagcaactcaggatgacaaactgcgtaagaaccactatcacggcctgccattcaaggtgacgaattactttgagtttatcgcccgtgaaacccgcgagctgatggcacagcttggcgtaacacgtctggtggatctgattggtcgcaccgacctgctgaaagagctggacggtttcaccgccaaacagcagaagctggcgctgtcgaagctgctggagactgccgaaccgcatccaggtaaggcactctactgcaccgaaaacaacccgccgtttgataacggcctgctgaacgcgcagttgctgcaacaggcgaaaccgtttgtcgatgagcgccagagcaaaaccttctggttcgatattcgcaacaccgaccgttctgtcggcgcgtcgctttcaggctatatcgcccagacgcacggcgatcaggggctggcagccgatcctatcaaagcgtacttcaacggcaccgcaggccagagcttcggcgtgtggaacgcgggcggcgtggaactgtacctgaccggtgatgccaacgactatgtcggtaaaggcatggcgggcggcttaatcgccattcgtcctccggttggttccgccttccgcagccatgaagcaagcattatcggcaacacctgcctgtatggcgcgaccggtggtcgtctgtatgccgcaggccgcgcgggtgaacgtttcggcgtgcgtaactccggtgctatcaccgtggtagaaggcattggcgacaacggttgtgaatatatgacgggtggtatcgtctgcattctgggtaaaaccggcgttaacttcggtgcgggcatgaccggcggtttcgcttacgttctcgatgaaagcggcgatttccgcaaacgcgttaacccggaactggtcgaggtcttaagcgttgacgctctggcgatccatgaagagcatctgcgtggtcttatcaccgagcatgtgcagcataccggctctcagcgcggtgaagagattctggcgaactggtcaaccttcgccactaaatttgcgctggttaaaccgaagtccagtgatgtaaaagcactgctgggtcaccgtagtcgtagcgcagctgagttgcgcgtgcaggcgcagtaaggggtagcaacaatgagtcagaatgtttatcaatttatcgacctgcagcgcgttgatccgccaaagaaaccgctgaagatccgcaaaattgagtttgttgaaatttacgagccgttttccgaaggccaggccaaagcgcaggctgaccgctgcctgtcgtgcggcaacccatactgcgagtggaaatgcccggtacacaactacatcccgaactggctgaagctcgccaacgaggggcgtatttttgaagcggcggaactgtcgcaccagaccaacaccctgccggaagtttgcggacgagtctgcccgcaagaccgtctgtgcgaaggttcctgcactctgaacgatgagtttggcgcggtgaccatcggcaacattgagcgctatatcaacgataaagcgttcgagatgggctggcgtccggatatgtctggtgtgaaacagaccggtaaaaaagtggcgattatcggcgcaggcccggcaggtctggcgtgtgcggatgtcctgacgcgtaacggcgtaaaagccgttgtcttcgaccgtcatccagaaattggcgggctgctgaccttcggtattccggccttcaagctggaaaaagaggtaatgacgcgtcgccgtgaaatcttcaccggcatgggtattgaattcaaactcaataccgaagtgggccgcgacgtacagctggacgatctgctgagtgattacgatgccgtgttccttggcgtcgggacttatcagtcaatgcgcggcgggctggaaaacgaagacgccgatggcgtgtacgcagcgctgccgttcctcatcgccaacaccaaacagttaatgggctttggtgaaacccgcgacgaaccgttcgtcagcatggaaggcaaacgcgtggtggtccttggcggtggcgacactgcgatggactgcgtgcgtacgtccgtgcgccagggagcgaagcacgttacctgtgcctatcgtcgtgatgaagagaacatgccgggttcccgccgcgaagtgaaaaacgcgcgggaagaaggcgtagagttcaaattcaacgtccagccgctgggtattgaagtgaacggtaacggcaaagtcagcggcgtaaaaatggtgcgtaccgaaatgggcgaaccggacgccaaaggccgtcgccgcgcggagatcgttgcaggttccgaacatatcgttccggcagatgcggtgatcatggcgtttggtttccgtccacacaacatggaatggctggcaaaacacagcgtcgagctggattcacaaggccgcatcatcgccccggaaggcagcgacaacgccttccagaccagcaacccgaaaatctttgctggcggcgatatcgtccgtggttccgatctggtggtgaccgctattgccgaaggtcgtaaggcggcagacggtattatgaactggctggaagtttaagcgaggtaacaatgaattcgccagactgtgtctggcgaatcaaattactgacgaagtgcgcgttgttttctggcaaatgcggcatgagcgtttgacctttcctataatagggataattttcaataaattgtgctttgttcaccaagtctgatgagtgaagcacatcaagcaatttctcatttacaatccgtctcaattacttgttaacacctctgacaataccgattctgcaagctattcagtcttttcattccatgtaaattgtctcgatattaatatacaaaatatgaatataaaaaaccaatatattatccttaattatctatatattttcctatttttcagcgcaaacattcatgtaatgaataattatcaccacaaaccacctcaccagcaccttattattcacatgatcgtaactataaaattcattaaataaatacatcccagcaagttggctatttctgaacgagttatttatttacattcacaaacagatatatatactgcttcagctttttattttaaaaaataaatttgttattaaggatatgttcatatgtttttcaaaaagaacctcacaacagctgctatttgtgcagcactttctgttgcagcattcagtgccatggcaacagattcaactgatacagaattaactatcatcggcgagtatacccctggtgcatgtaccccagttgttacgggcggcggcattgttgactatgggaaacatcataacagtgcgctgaatccgaccggtaaaagtaataaactggttcaactgggccgcaaaaacagcacattaaatataacctgcacagcaccaacgctaattgctgtaacctccaaggataaccgtcagtcgaccattgtagcgttaaacgacacatcctatattgaaaaagcttatgatactctcgtagatatgaagggaacgaaaaacgcctttggtttaggttctgcgcctaatggacaaaaaattggcgctgcatccattggtattgacaggtctaatggtgggattcacgcggcggacgatacaggtgaaattcctgtcgacctgattcaaactgaccactggtcagcagcgacccccacatggaaagcctcatctaatggcgcattctgctcgctgacaagttgctcagcaatcgagcgcggttattctgttgcaaaaacaggggaactgacacctgttgctattacagcggtcaccttcccgttactgattgatgctgcggtaaatgacaatactattcttggttctgatgaaacgatcaaactggatggtaacgtcactatcagcgttcagtatttataagaacttgtaatacagtttttatttttacgcattaaccagttagctataactcggacagattatgccctatgacatggtctgtcttaatcaatctcatcgcaaacagtgcataacatatattaacaatatgtttctgcgttatttatcattattacaggagttttaatttaaatgctcagacacattacattcactgtatttataacaacatcaatgaataccttagccacagggatggttcctgaaacatcagtattgctggttgatgaaaagcgtggtgaagctagtattaatattaagaatacagatgatcatccttcattgctttacaccaccattgttgatttgcctgaaagcaataaatcaattcgtttaatcccgactcagcccgttattcgtgttgaagccggtcaagtacaacaggttcgatttttacttcaggcgactgttcctctgcaatcagaagagctgaaacgcgtaacgttcgaaggtattccaccaaaagatgacaagagcagcagagttactgtttcaattcgtcaggatctacctgtactgatccacccggcttccctgccggaagagcgagagacctggaaattcctggaatggcgtaaaaatggcgaccaaattgagattagcaaccccagtaattatgtcgttcgtatgaccttacaatttaaaacgctcccttcaggaaaaacgggggctataaataagacctattttctaccacacaccagtacaactactgcattaacaaacgctacggatacaaaagtcgagttttacccagccagccgatatggttatcgcggtaataaatatgtcactgacttaaaataactttgcctggagcgacaaggatgttaaaaaaaacgttactggcctacaccattggttttgccttttctcccccagccaatgcagatggtatagagattgccgctgttgattttgatcgggaaacattaaaatcactaggtgtagatcctaatatatcgcattatttttcccgttcagcccgttttttgccaggtgaatattcactgatagtatcagtaaatggcgaaaaaaaaggcaacattgctacgcgctttgatgaaaatggcgacatttgtcttgatcaggcatttctgcaacaagccggtttaaaaattccttctgaagaaaaaaatggctgttacgactatatattgtcctacccgggtaccacaatcacaccattacctaaccaggaagcgttagatattatcgtttcaccacaggcgatcattcccatagggttggatctcacaaacgcagcaactggtggaacagctgcgctgctaaactactctctgatgagcagccgtgcagaattttctaatgggagttcggactactcccaggctgcacttgaaggcgggattaatattaatgactggatgttacgcagccatcagttccttacacaaacaaatggcacattcagtaaccagaactcgtcaacctaccttcaacgtacctttacagatcttaaaacactcatgcgagcaggtgaagttaacctcaataatagcgtgttggaaggagccagtatttacggtatcgaaatcgcaccggacaacgcattgcaaaccagcggcagtggtgtgcaagttactggtatagccaacacctctcaggctcgtgtcgagattcgtcaacaaggagttttaattcattccattctggttcctgcgggcgcattcactatccctgatgtacctgttcgcaatggtaatagtgatcttaatgtcaccgttgtcgaaacagacggtagttcgcacaactatattgttccctccaccctgtttaatcagcatgtagaaagcttccagggttatcgcttcgcgatagggcgggtagacgatgactatgacgaatcaccttgggtaattagtgcatcgagcggatggaatctgacacgctggagtgcaatgaacggcggcgttatcgtagcagaaaattatcaggcggcatcaatccggtcgagtctggttcccctgcccgatttaacagtgagcagccaaattagtacatcgcaggatacgaaagactcactgcaaggacagaaatatcgtcttgacgcgaactacaatctcccattttcacttgggctaacaaccagcctcactcgatctgatcgccattatcgcgaactgtctgaagcgattgatgatgattataccgatccgactaaaagcacttatgcgcttggtttaaactggtctaactccattctgggtggtttcaacatcagtggctataaaacatatagttacgacggtgacaatgactcaagcaaccttaatattaactggaacaaagcgttcaaacacgccacggtttccgtcaactggcagcatcaacttagtgcttcagaaaataatgaagacgatggtgatctgttctacgtcaacatcagtattccatttggcagatcaaacaccgccacactgtatactcgccatgacgatcataaaacccactatggtactggtgtcatgggagtcgtctcagatgagatgtcctactatgtgaatgctgaacgagatcacgacgaacgtgaaacgagcttgaacggcagtatcagttccaatctccattacacccaagtcagccttgccgcaggagcaagcggcagtgatagccgtacttacaacggtacgatgtcaggtggtattgccgtacatgatcagggagtgaccttttcaccgtggactatcaatgacactttcgccatcgcaaaaatggataacaatattgcaggtgtcagaattacatctcaggcaggcccagtatggacagattttcggggtaatgccgtcattccatcaatccagccgtggcgaacatcaggagttgagatcgataccgccagcttgccaaaaaatgtcgatatcggtaacggcacaaaaatgatcaaacaaggccgtggtgcagtagggaaagtcggattcagtgcgataacacaacgccgtgcattactcaatatcacactttccgacggcaaaaaactgcccagaggcgttgcgattgaagatagtgaaggcaactatctgacaacatcagtggatgacggtgttgtattcctcaataacatcaaaccggacatggtgctagatataaaagatgagcagcaatcatgccgtattcaccttacattcccagaagatgcaccaaaagatgtgttctatgagacagcaacaggagagtgccaatgaaacggataataacaggatgcctgctgctgaacttcgccatggccgctcaggcagagtgtaatatctccagtagcatacaaaatatcgactatggcaaacgaagtgctgccatgcgccaagttgaccggggtaaaacaacacaattagcagacagaacaatcacgctggtaatgcaatgcgatcaggacgctcatattcgtgttcagttgaataccgctaatatttccaacaacggatttggatttggcccgaatggttcattaaatctgatcgccagcgatgcattttcaggtagtaacaatctcgacctggcgttagccagtggcaaaaatgacaatccgggcagcacaggaacagcatcaattagggaaggtgcgaataagcggggaaattcttctcggctgactcagtcatttcatttcttcatgtttgagccgattttttctcccgtaaatgccttgaatcagcctatttagaccgtttcttcgccatttaaggcgttatccccagtttttagtgagatctctcccactgacgtatcatttggtccgcccgaaacaggttggccagcgtgaataacatcgccagttggttatcgtttttcagcaaccccttgtatctggctttcacgaagccgaactgtcgcttgatgatgcgaaatgggtgctccaccctggcccggatgctggctttcatgtattcgatgttgatggccgttttgttcttgcgtggatgctgtttcaaggttcttaccttgccggggcgctcggcgatcagccagtccacatccacctcggccagctcctcgcgctgtggcgccccttggtagccggcatcggctgagacaaattgctcctctccatgcagcagattacccagctgattgaggtcatgctcgttggccgcggtggtgaccaggctgtgggtcaggccactcttggcatcgacaccaatgtgggccttcatgccaaagtgccactgattgcctttcttggtctgatgcatctccggatcgcgttgctgctctttgttcttggtcgagctgggtgcctcaatgatggtggcatcgaccaaggtgccttgagtcatcatgacgcctgcttcggccagccagcgattgatggtcttgaacaattggcgggccagttgatgctgctccagcaggtggcggaaattcatgatggtggtgcggtccggcaaggcgctatccagggataaccgggcaaacagacgcatggaggcgatttcgtacagagcatcttccatcgcgccatcgctcaggttgtaccaatgctgcatgcagtgaatgcgtagcatggtttccagcggataaggtcgccggccattaccagccttggggtaaaacggctcgatgacttccaccatgttttgccatggcagaatctgctccatgcgggacaagaaaatctcttttctggtctgacggcgcttactgctgaattcactgtcggcgaaggtaagttgatgactcatgatgaaccctgttctatggctccagatgacaaacatgatctcatatcagggacttgttcgcaccttccttagtacttcccccaataattggctggtgtttatgcaaaatggtcaagaagtggtaattgatagcggtaaaagcgttagcctcacactgacaatggctccagcttttaaggatgaaggggaactaaccgacatgacagatattacaggcaatctgacggtcctggtggaggcaaaatgaacaatgtaaaattactgattgccggaagtgccttttttgccatgtcagcgcaagccgctgatagagtatcaattgacgttaaggtgactctggaagctgcagcttgtactccaatactaagcaacggcggagttgttaacttcggtagtcattcagtcaatagactttcaacgcagcactacacacagattggaacacgtaatattaatatgactataacttgcgaatccgctaccggcattgcgattaccgctcgtgatacacgaatggatagtatgaccaccggaaaagatagtgggggtcagagtggtgtaaaatataccttaaatggcggaggttatattagccagacaacgcgcttattcggcttagggaaaacaaaagataataaaaatatcggtagttatgccgtgttaattgatagcaacaacattagtgccagcaatggtagccagacgttagctgtatcaatagcaggtgcagatgccgtcataacagggcaaaaaagagcatggcaaacgctcaccgcttatccgcttgcagtcgatcaaagctattattacacctttgtaaaaccaggtgaaacaaccccaactcctgtaacgaacgccattataccgcttcaggtgagcgcatctatcgcgaatgatttaggcggttcagaaaaaatcgaacttgatgggaaagctgtgataagcgtagtctacttgtgataacaatgccggacaggagtactatcaggcattcgttttatacgatcggttaatgtttcaggaaagctcttcgcatatcttggggaaagtaaatgtaatacgctgttcttaattgttcagtgctcaccccccagagtatagctcattccattattcaacttagctccatataaagggacagataatggaatcgctctcagaaggaaccacagcaggctaccagcaaatccacgacggtattattcatctggtcgatagcgcccggacggaaacggtacgtagcgttaacgcgttaatgaccgcgacgtaccaggaaattggccgacgaattgtcgaatttgaacaaggtggcgaggccagggctgcgtatggtgcgcagctaatcaagcgactatcaaaggatttatgtctaaggtataagcgtgggttctctgcaaaaaacttacgccaaatgaggcttttttacctcttttttcaacatgttgaaattcaccagacaatgtctggcgaattaacaccattgggaattccgcagacaccgtctgcagaattcccatcggcaaagatttggcagacgctgtctgccaaatctttccccttgcccaggtccacctacgtccgtttactttccgttaaaaacgctgacgcccgcagcttttatgaaaaagagacgctccgctgtggctggtctgttcgccagctagagcggcaaattgcgacccagttttatgagcggacactactgtcacatgacaaatcagccatgctgcaacaacacgctcctgccgagacgcatattcttccgcaacaggcgatacgcgatccctttgtgctcgaatttctggaattgaaagatgaatattcagaatccgattttgaggaggcgctgatcaaccacctgatggatttcatgctggaacttggggatgattttgcctttgttggtcggcagcgaaggttacgcattgatgacaactggtttcgtgtcgatctgctgtttttccaccgccgtttacgctgcctgctaatcgtcgatctaaaagtgggcaaattcagctatagcgatgccggacagatgaatatgtatctcaactacgccaaagagcactggacgctaccggatgaaaatccgcccatcggtctggttctctgtgcagagaaaggagccggagaagcgcattatgctctggcaggtttgcctaacaccgttctggcaagcgaatataagatgcaactacctgatgagaaacgactcgcagatgaactcgttcgaacacaggcggtgctagaggaaggctatagacgccgttaatttcagcggtttcgaattctgcagacagtgtctgcagaatctttaaaacgaactaagttttaagccattaaatcagccttaaccttcaccacaacctttttaatctctccaggctcgccgacaacgcatcctggtttatgcggttcacctggcataaacacggcgaacattcccggttttaagatgatggcttgctcgttatcaatggtgctgcaaagctgataatcatcctcatggtggaactcttcacactgacgcgcagtgcctgccatgccaaacagaatccgttcctcaccgtttaataacagctggatatcaatgtattgctcgtgcaattccgcttttttctcgacgggcgattgagtgttaaacgtcatgacattcataaagatattgtcgccctgtaattcgtaacgacccggcgctttttcttgcggtctggcagctaatgccagcgttaacgcgtcctgtaacgcaggatgtaacccagcagacggtaatgactgtacttcacccatcatcataatttttctccctgggccaacagcgcagccccaagtaaacctgcatcatggcggtaatgcgccgccagtaaatcaacatgaaatgccgctggctcctgcgccagatacgtttccaccagcgccagatacccttctgccagaccaacgctgccaccgaccaccacgcactggcaatcagttgtggctttaatatcagcgatcagccttgcaagcgtacgtgcggagcggtgaatcagctgctgcgcctgctcgtcaccctgcccggcgcgcgtgaaaatagttttcgcatccgcgccagccaactccccctgcgctgccgctgcaatgccgcgaccagaagcaatcgcttccacgcaacctgtgcgtccacagccgcagactgggccgtgtggatcggcaagcgtatgcccgatatgccccgccagaccgccagggccggtaagcagtttgcagccgctcactacaccgccgccaacgccggtggaaacggtgataaagaccatatcggttatatcgccatccagcgcctgaaactccgcccatgctgcggcctgcgcgtcgttaatggcaatggtcggcaaattggtaagttgttccagcgttttgactaacggaaagtgtagcaatccaccaagattatgcggattaagcgccagcaagctgccgtcacggattatcccggtcgaagcgatggcaacccgctgcgcatgagcttgcaacggagagactaatgcggataaggcatcacgcaaggcttctggtgtctggctggctggcgtaggaagttcacgacgatcgcggatctgcccgtcagcgccaatcagcgcggcggcaagtttagtaccgccgatatcaatcgccagtgtggtcatagcaccgcctttttcatcgctgtgttgtaccactgacaaatgtgctcaagacgcgtgattgcagaaccgaccgtcaccgcccacgcgccgtggcgcatcgcatccgccgcctgagcaggcgtgttgtaacgcccttcggcaatcacccgacatccggcgtcgctcaacgttttcaccagcgccagatccggctcttctggcgtttcaggcgtggtatagccagaaagcgtagtgccaataatttcggctcccagcttttggcatgccaggccgtcttccggcgttgagcagtcggtcatcgccagtaaaccgtgatggtgaatacgtgccagcagcgtttcaacaggcaccggacgcgggcggtcggtgccgtcaatggcgataatgtccgcgcccgcctgcgccagcgcatcaacatcttcaatataggccgtgatgcgtaccggagaatcctccagatcgcgtttcacaattccaataatcggcacgctcaccaccgcacgcgtggcttgcagatttgccacaccttcaatgcgaatggcaaccgcgcccgcctgttctgccgctaatgccatggcggcgacgatttcgggtttatcgagcgggctgtccggaaccggctggcaggagacaatcaggccaccgttagcagcgattttttgatccagttgtgcaagtaacgacatacatcttcccttagcgaaaggcccggtacatagaccgggcaacaggattaacttttggttttgactaaatcgtttttggcgctgccaaacggcacggcaccgctgaatggtttaccgtcgatagcgtcatgagtacgcaacgcttccgggcgcaaccaacgctgaacgcgagaaggcatatccagcccaatcagcaggatcaccacgaacgtcagactgaacgagagcgatgccagcgcagtacccagatccagacgttgagcgatcaacgcgccgatgattggggccagtgcaccgcccaatgcgccaacgttgtaggtaaagcccaggcccgctgcacgctggtcggtatcgaaataaccgccaatcagttttggtaagatcccggcgatcccttgtccaagcatttgctggaagaacagtaacagaccgagcacccagacgtttgcgccgccaatcgcaaataccggaataatcagcagctgcgaggccagcaggctacaaacgtacgctttgcgggttcccagccagtcaccgaggaagccacctacgcagcatcccaccgccgcgccaaagccactaaagaacagcacattggctacagtatgcgggttataagccagatcggttttcagatacgttggcagcagcgcctgaatcggccatgagtagaggaaagcaaacaacacgaccaccatcagcattacgcccgttggccagcgtttgcctgcactctgcaccataaagctgataaagattgcggcgcataacagcccaagaacagcgacgatcgcggcattttgcaggttaccggcgaagcagaaccacagcgcagtagccgccgccagtgtcattacgatattggcaatgcgatgttcaccacggtagagaatatccaccattgtgcgtactggtgctttacctgcgtgtttctctttccagtcttccgcttccgggatgtttttacgcagccagagagcaaagatgattggcaaaatgccgataaagaacagcgcacgccagccccagaccggaaccaccaggctatagacctgagcggcaacgacggcccccacagagaagcctgaaatcaaaaaaccactggctttgttacgcagatgttttggccagctttcaatgacataggtggcgctggaaccgtattcacccgccatccccatgccgatgaccagacgagcgataaacatggtgatgtagcctggcgcaaagccgcaggccagcgtcccggccgagaagagaacgatgctggtgaccattgccagacgacgcccgtagcggtcacccatagcgccgagcatcaggccgccgaaccagcgagagataaaggctgcagagatcagacttgccgcctgcaccgtcgtcagcccgaattcaccttgtacttcggtgagtaccagggcgattaaaacgaaatcaaaaccgtcaagcagatatcccaaccaggcagcggaaaatgcgcgccattgtgcacggttgagatggcgataccacgggatattctgggttgtagtactcattgtgagtctcccgcggtgggcgatgcccacacgctttggtatgaaaattgtagggtacagatgcgtttatttcccctcacccggtaggggcgagcgaggggaaacaactcacccgcgctcttgcatcaactgctgggccagcgccttcagttctggcagatatttttcatctaccggtccaaacggtttgcggcacagcggcacagaaacgacatccatataatggaggacagttttcaggccgcggaatacgcccgttttgatcagtaaatcaatgactttattgcattcagtttgcagtttctgcgcggtctggatatcgccttctttcagcgccttaacgatcccctgatagcgccagcccatgatgttgtaggtactgccgataccaccatcagcgcccgccagcagaccagaggcgaagatttcgtcgtaaccgttatagagcacaagatcaggatgttcacgacggatctgctccatctgatagagatcgccagaggtctgtttcagcgcacctacgccaggcaatgtaacaagtgtgttgatctgatccagggtcagttttaccccactcagggctggaatgttgtacaccaccatcggcaaaccatccgccgaatcaataattgcccgatagtgatcgcagtgttcttcaaagctgaaaggatagtagaacggcgtgacggcggagacggcatcgaagccataacgtttagccgatgccgcaagttgttggctttcggcggtgctgacgcaaccgacgtgggcgatgagtttaatcttacctttcgcctcttcggcgacgatttccagtacctgttcacgctcggaaaggctttgtacaaaggcctcgccggtcgaaccacccacgtataaaccgtcgatgccctgctgaatattgaactgaaccaggcgacgcagactcgctttatccagtgcttgttgttggtcaaaaggagtcaggagtgcagccattacgccacgtaaattcgttgccataaatacctctgaagtgatgcttgtctgataaacgatatacctttatacctgttataccagatcaattaagcaacaccccatacagaaagcttataatgcgatctgcttcactaaagtggcattatttctttttgttggtggtctgaccgaaagcgtgccaggtagcagagacgctgttgagatgcgattgcaacgcacgatcggcttcgtcaggatcatgacggcggatcgcatcaacgatcgcaatatgctgttgataactaacgttgttatgttcgtgcagtgcctgatcggtaaccgttgggcgtgcggcaataagccagtcgagcagggcaacgtggatcgccatgaagattgggttaccggggatctccgccagcacgcggtggaaatcaacgtctgaacgaatgaatgccgcgttgttatccagcgactgactgttgatttccagtgcttttgccagcaaatcgatttgctcatcggtggcatgttcagccgcatagcgcaccagactggattcaaagaacagacgtaattgttcgaaatgggcaatcccaccgggatgagaaaggaaatctttcgccatgccggaaagctcaccgatgatagtgtccgcagaaggacgcgagacgcgagcgcgttcgccgttgtttatttgcaccagacctttgcgttttaacgctgccagcgcttcacgcaccgaaggacgcccgacgttaaagaacgccatcagttcgcgttcagacggtaattgttcaccttcgccaaattcacgacggcggatcatctgttccagctcttcttccaccatttcggagagttttttacgcgccagcgggcggctacgcaagttgcgaccaattgcaggtgaagaatcttcggtttgcgaatcaaatgcgttcataaggcccattctgtaaggtcagtgtgattaacatcatcagtgacatcctatcacaggattgaaagtaggggaaaatggcagggttttctctttgtgcctcatcattaccataattaacggaataattaactattgcgaaaaattaatgtaacgcagataaaaacatcccgtttgaattatttataagactattcacgagcattatgaatattatgaatgtgttcttacaaaataatcataagcgcatattttttaatgaaaaatcacctcacctacaattaaaaacacgacatccgcaccataaatagccttgcaaaaaatataacatcgttgttttcaatctgccgtttatgggattgaccgttttcttttgacacggagttcaacaatgttcggcataattatatctgtcatcgtattaattacgatgggctatttgatcctgaaaaactacaaacctcaggtggtgctggctgccgcaggtatcttcctgatgatgtgcggtgtctggttagggttcggtggtgtactcgatcccaccaaaagcagcggctacttgatcgtcgatatttataatgaaatcctgcgcatgctgtccaaccgcattgccggattggggctgtcgattatggcggtgggcggttatgcccgctacatggagcgcataggggccagtcgcgcgatggtgagcttgttaagccgcccgttaaaactcattcgctcgccgtatattattctgtcggcaacttacgtcatcggccaaatcatggcgcagtttattaccagcgcctccggtctgggtatgttgctgatggtcaccttatttccgacgctggtgagtctgggagtaagtcgtctctctgcggtggcagttatcgcaaccacgatgtccattgagtgggggattctggaaacgaactccatttttgctgcccaggtagcgggaatgaaaattgccacatacttcttccactaccagcttccggtcgcctcttgcgtcattatctcggtggcgatctcccactttttcgtgcaacgcgcttttgacaaaaaagataaaaatatcaatcacgaacaggcagagcaaaaagctctcgataatgtcccgccgctctattacgccattttacctgtgatgccgttaatcctgatgctcggctcgctgttcctcgcccacgtcgggctgatgcagtcagaactgcatctggtggtggtgatgttactgagtttgactgtgacgatgtttgttgagttcttccgcaagcataacttgcgcgaaacaatggacgatgtgcaggcgttttttgacggcatgggtacgcagtttgccaacgtggtaacgctggtggtcgcgggtgaaatatttgcgaaaggcttaacgacgattggcactgtcgatgcggttatcaggggggcggagcattctggtctgggcggtattggcgtgatgattattatggcgctggtcattgccatttgtgccattgtgatgggctctggcaatgcgccgtttatgtcatttgccagtcttattccgaatatcgcagccggactacatgtaccagcggttgtaatgattatgccgatgcattttgccacgacgctagcgcgcgcggtttcgccgattactgcggtggtggtcgttacgtcaggaattgcaggcgtttcgccttttgcggtggtgaagcggacagcgatccccatggcagtcggtttcgtggtgaatatgattgccacaatcacgctattttattaagtcattaaaaagacaaaacaggccgcctgggcctgttttgtattacttcacaacgcgtaatgccggtcgaccaccgcgtggtggctgcggaggttcatcgtcaggatgagtgtcatcatcgtgatctggcttgtcgccatcaataaccgacataacggtttcgttgtctgccgatgcctcttcatcattcatgatgctggtatcttcatcgtaggcagcttcaggctcaaacatcgtgcctgcgccattttcacgggcgtagatagccagcacggcagccagcggcacagaaacctgacgcggaatgccaccaaagcgcgcgttaaagcgcacctcatcattcgccagttccagattgccgacagcacgcggcgcaatgttgagtacgatttgcccgtcacgcgcatattccataggaacctgcacgccagggagcgtcacatccaccaccaggtgcggcgtgagctggttatccagcaaccactcatagaatgcacgcagcagatagggacgacgtggtgttagctgtgacaaatccatacagattaactccggcccagacgcatttcacgttctgcttcagttaaagaagcaaggaaagagtcacgctcaaagacgcgggtcatatagcctttcagctctttcgcacccgggccgctgaactcgatgcccagttgcggcagacgccacagcagcggagcaagatagcaatcgaccaggctgaactcatcgctcaggaagtacggcttctgaccgaagaccggcgcaatcgccagcagttcttcgcgcagttgcttacgtgcggcatctgcttcagaagctgaaccgttgatgatggtgttcatcagcgtgtaccagtctttttcgatgcgatgcatgtacagacggctttcaccgcgagctaccgggtaaacaggcatcagtggcggatgcgggaaacgctcatccagatattccataatgatgcgagattcccacagggtcagctcacgatccaccagggtcggaacgctctgattcgggttgaggtcaatcagatcctgaggcggattgtccttttccacgtgttcgatctcgaaacttacacctttctcagccagcacaatgcggacctgatggctatagatgtcagtaggaccggaaaacagcgtcattaccgaacgtttgttggcagcgacagccatgaaaacctccaggtatagtcagaatttttactgctaccagccaccaggtggccagtcagaagttgtgttacccaataaggaacgactctctttgttcgaaaatcaaacaaaaaatgagcaatacccgacatttgggcagaaaattggatgatagtttaccagattttgcgaccattgtggtgagtcgatgccggaaatggggaaaaagagatgcgctttagtctgaaatagttgacttagtcccttattggcgatgtggtttttgttttacctgtctgtcaggtggcagcaaaaagcaactttccagtttttacgctgattcagattttagctataaaaaaacccgccgaagcgggttttttcgaaaattgttttctgccggagcagaagccaattaacgtttggagaactgcggacgacgacgtgctttacgcagaccgactttcttacgttcaacctgacgagcgtcacgagtaacgaagccagctttacgcagttcagaacgcagggactcgtcgtattccatcagagcgcgggtgataccgtgacggatcgcaccagcctgaccagagataccaccacctttaacggtgatgtacaggtccagtttctcaaccatgtcgaccagttccagcggctgacgaactaccatgcgggcagtttcacgaccgaagtactgttccagagaacgttggttgattacgattttaccgttgcccggtttgatgaaaacgcgagctgcggaacttttgcggcgaccagtgccgtagtattgattttcagccattgcctataatcccgattagatgtcaagaacttgcggttgctgtgccgcgtggttgtgctcgttacccgcgtaaactttcagtttacggaacatagcacgacccagcgggccttttggcaacatgcctttaaccgcgatttcaatcacacgctcaggacggcgagcaatcatctcttcaaaggtcgcttgtttgataccaccgatgtggccggtgtggtgatagtacactttgtcagtacgcttgttgccggttacagcaactttgtcagcgttcagaacgatgatgtaatcaccggtatctacgtgcggagtgtattccgctttgtgcttaccgcgcaggcgacgagccagttcagtagccagacggcccagagttttaccggtcgcgtcaacaacataccagtcgcgttttacggtttctggtttagctgtaaaagttttcattaaaagcttacccaataaatagttacacgttggtgaacacccaaacgtcttcaattgttgaggttcacacgacaaagtccggcaaacctaccccttcgaatagcctatgccagcacacaaaaagttttgggaaaaaaactttcttgtaacgtggggtcgcaggattatagagaagtcggggtcaaagatcgacccctttttgtgatttgtgacaggttttaacccgccaaatgctcgcgcttcagatactcttcgctttgcatctcttgcagacgtgacaggcaacgctggaactcaaacttcagccgatcgccctgataaatttcatacagcggcacttctgcactcaccactaatttgacatggcgctcgtaaaactcatccaccagcgcaataaagcgccgcgcttcgctctccatcaaccgcgtcataactggtacatcaaacaacatgaccgtatgaaagagacgtgagagcgcaatatagtcatgctgactgcgggcgtcgacgcacagcgtagtaaaagagaccgccagcgtctggttctcgacgcccattgttgctaatggccgatggttgatttctaacgtcggtgaattttctcgtttcccccccgccagcgccaaccatagtttatccatttgcgcccgggtttcatcgtgaagtggcgaaagccacagatgcgcctgagtgagtgtacgcagacgataatcaacaccagcgtccacgttcattacatcacaatgctgtttaatggcatcgattgcaggcagaaaacgcgcacgttgcaggccatttcgataaagttcatccggcggaatatttgacgtcgctaccagggtaataccgcgagcgaacagggctttcatcagaccgccaagtagcatggcatcggtaatatcagaaacaaaaaattcgtcaaaacagagcacgtcagtttcggctttaaagcgatcggcaataatttccagcggatcggtctgcccctgtaaggcagttagctcttcatgcacccgcagcataaaacggtgaaagtgcaggcgctgtttccgctctcccggcaggctttgatagaaaaggtccatcagccaggttttcccgcgtcctacaccgccccacatatataagccacgcactggcgtatgctttgtgtcttcgcgtttaccccacagcttaccgacccgcgccattagcccactcgtcctgggggctggtggcgtgctattgatgagttcctgataaataatttccaggcggctgacggcctctttttgaacgtcgtcgggttgatggctgccttcattaagcgccttcaggtattgcgatgttggggtaacgctttgcatgatcttattgttattccttgaataatcggtgcgccgttgttcacggttgacgaaaaaaaggccgttctacactacgcgatatgcagtcgggattccacttctgtggaattaacggttatagtggcataatcagccgcaggcatggagcctgaagccaacaccctacggaaacaaaagacaacgggagatgttcatgacctgggaatatgcgctaattgggttagtcgtcggcatcattattggtgctgtggccatgcgttttggtaatcgtaaactacgccagcaacaggcgttgcagtacgaactggaaaagaataaagctgaactggacgagtatcgcgaagagctggttagccactttgcccgcagcgcggaattactggataccatggcgcacgactatcgccagctgtatcagcacatggcaaaaagctccagcagcctgctgccggaactgtctgctgaagcaaacccgttccgtaatcgtctggcagagtctgaagccagcaacgatcaggcaccggtgcagatgcctcgcgactattctgaaggcgcatccggcctgctgcgtactggcgcgaagcgcgactaatttatttttcgggcgcagccattgcgccctcctcttctctccctccccgactatcatttaatctggtgtctcattgttagccgtctgaaaattcaataacatcaaactgttttgaatctcttttcttatcattcaggtacgagagcaggaataatgaaaaaacaaacccagctgttgagtgcattagcgttaagtgtcgggttaactctctcggcgtcatttcaggccgtcgcgtcgattccaggccaggttgccgatcaggcccctctccccagtctggctccaatgctggaaaaagtgcttccggcagtggtgagcgtacgggtggaaggaacggccagtcagggacagaaaatcccggaagaattcaaaaagttttttggtgatgatttaccggatcaacctgcacaacccttcgaaggtttaggctccggtgtcatcatcaacgccagtaaaggctatgtgctgaccaacaaccatgtgattaatcaggcacagaaaatcagtattcagctcaatgatgggcgcgagtttgatgcaaaactgattggtagcgatgaccagagcgatatcgccctgttacaaattcaaaacccgagcaaattaacgcaaatcgctattgccgactccgataaattgcgcgtcggtgattttgccgtagcggtcggtaacccatttggccttgggcaaaccgccacctctggcattgtttccgcattaggccgcagcgggttgaatcttgaaggtctggaaaactttatccagacagatgcttccattaaccgcggtaactccggcggtgcactattaaaccttaacggtgagttaattggcatcaacactgcaatccttgcgcctggcggcgggagcgtcgggattggatttgccatccccagtaatatggcgcgaacactggcgcagcagcttatcgactttggtgaaatcaaacgcggtttgttaggcatcaaaggcaccgagatgagtgccgatatcgccaaagccttcaaccttgacgtgcagcgtggcgcgtttgtcagcgaagtgttgccaggttctggctcggcaaaagcgggcgtcaaagcgggcgatattattaccagcctcaacggcaaaccgctgaatagctttgctgagttgcgctctcgtatcgcgaccaccgagccgggcacgaaagtgaagcttggcctgctgcgtaacggcaaaccactggaagtagaagtgacgctcgataccagcacctcttcgtcggccagcgctgaaatgatcacgccagcgctggaaggtgcaacgttgagcgatggtcagctaaaagatggcggcaaaggtattaaaatcgatgaagttgtcaaaggaagcccagctgctcaggctggcttgcaaaaagacgatgtgatcattggcgtcaaccgcgatcgggtgaactcgattgctgaaatgcgtaaagtgctggcggcaaaaccggccatcatcgccctgcaaattgtacgcggcaatgaaagcatctatctgctgatgcgttaatgtcgtaaaccgggcatcaggcttacgtgtgatgtccggttaactcgtggtatgctgctgccgttcccttttttaatgacgcctccatcatgtttgtgaagctcttacgttccgttgcgattggattaattgtcggcgctattctgctggttgccatgccttcgctgcgcagccttaacccgctttccactccgcaatttgacagtaccgatgagacgcctgccagctataatctggcggttcgccgcgccgcgccagcggtggttaacgtttacaaccgtggtttgaacaccaactctcacaaccagcttgagatccgcaccctgggatccggtgtaatcatggatcaacgcggttatatcatcaccaataaacacgtcatcaacgacgccgatcagatcatcgtcgccttacaggatggacgtgtatttgaagcattgctggtgggatctgactctctaaccgatctggcggtacttaaaattaatgccactggcggtttacctaccattccaattaatgcacgtcgcgtaccgcacattggcgacgtagtactggcgatcggtaacccgtacaacctcgggcagaccattacccaggggattattagtgccacgggtcgaatcggtctgaacccgaccgggcggcaaaacttcctccaaaccgatgcttccattaaccacggtaactctggcggcgcgctggtgaactcgctgggcgaactgatgggcattaatacgctgtcgtttgataagagtaacgatggcgaaacgccggaaggtatcggctttgcgattcctttccagttagcaaccaaaattatggataagctgatccgcgatggtcgcgtgatccgcggctacattggtatcggcggacgtgagatcgcaccactgcacgcgcagggcggtggtatagatcaactgcaagggatcgtggttaatgaagtgtcacctgacggcccggcggcgaatgcgggtattcaggtcaacgatctgattatttcggtggataacaaaccggccatctctgctctggagacgatggatcaggtggcggaaattcgccctggttcggtgatccctgtagtagtgatgcgtgatgataagcagttaacgctgcaggtcaccattcaggaatatccggcaaccaattaagtcgtgcgctcaaaacaaaaaaccggagtctgtgctccggttttttattatccgctaatcaattacttattaacgaactcttcgcccagggcgatatctttcttcagcgtatccagcataccttccagcgcgttctgttcaaatgcgctcagggtaccgatagatttacgctcttccacgccgtttttacccagcagcagcggttgagagaagaaacgggcgtactgaccgtcgccttcaacgtaggcacattcgacaacgccttgttcgccctgcagtgcacgaaccagagacagaccaaaacgtgcagctgcctggcccatagacagggttgcagacccgccaccggccttcgcttcaaccacttcagtacccgcgttctggatgcgtttggtcagatcagccacttcctgctcggtaaaactaacgccaggaacctgtgacagcagcggcagaatggtaacaccagagtgaccgccaataaccggcacttcaacttcgcctggctgtttgcctttcagttccgcaacaaaggtgttggaacgaatgatatccagcgtggtaacgccgaacagtttgtttttgtcataaacaccggcttttttcagcacttcagcagcaattgcaactgtggtgttaaccgggttagtgataataccaatgcacgctttcgggcaggttttcgcaacttgctgtaccaggtttttcacgatgccggcgttaacgttaaacaggtcggaacgatccatacccggtttacgcgctacgcctgcagagataagaacgacatctgcgccttccagcgccggagtcgcatcttcaccagaaaaacctttgattttcacagcagtagggatatggctcagatcgacagccacaccgggagtcactggagcgatatcatacagagagagttctgaacctgaaggcagttgggtttttaacagtagtgcaagcgcctggccaataccgccagcagcgccgaggactgcgactttcatcctaaactccttattatattgataaactaagatatgttgctccgctgccgcgaccttaatccacaaaattgccgtttacaatgaccacatctcaagaatgtgtagtcacgcaagtttagcgtttatgcatttaattgccgtaatcaggaacctaacttacgtaattaacagtcgcttatgcattagcgcaacattccaacaggtggtgacaatataccctaccgttcagccaaaacaacatcaatttgataacaattaatttacttttaagcagaatttgcatgccgtgacgcaggcatgtttctcaataacgaaatttgataaaatcccgctctttcataacattatttcagccttcttcagggctgactgtttgcataaaaattcatctgtatgcacaataatgttgtatcaaccaccatatcgggtgacttatgcgaagctcggctaagcaagaagaactagttaaagcatttaaagcattacttaaagaagagaaatttagctcccagggcgaaatcgtcgccgcgttgcaggagcaaggctttgacaatattaatcagtctaaagtctcgcggatgttgaccaagtttggtgctgtacgtacacgcaatgccaaaatggaaatggtttactgcctgccagctgaactgggtgtaccaaccacctccagtccattgaagaatctggtgctggatatcgactacaacgatgcagttgtcgtgattcataccagccctggcgcggcgcagttaattgctcgcctgctggactcactgggcaaagcagaaggtattctgggcaccatcgctggcgatgacaccatctttaccacccctgctaacggtttcacagtcaaagacctgtacgaagcgattttagagctgttcgaccaggagctttaatctctgccccgtcgtttctgacggcggggaaaatgttgcttatccctctcaaccccctgctttcccctgcgattaatttaacgaatagtgcgttttactgcgacatgtcattcacacaatgaatacataaggtaaaaaaagcacattatgcaaaattcattatctaattgaaaaaactagaattaacgataaataaccgtatttttaattcttttttgttattaaaattcacatttttaacacttagtatcaactgaaacagttagcgcggtattaattagctcaataattagtgtatacttgattttgtgatatgggtcacgaaacaaaggcccagctaaaagattatgtcgaggtaaaaatcatgaaaatcaaaaccactgttgctgcattaagcgtactttctgttctctctttcggtgcattcgctgccgactccattgatgctgcacaagcacaaaatcgtgaagcaatcgggaccgtatccgtaagtggtgtggcgtcttcgccaatggatatgcgtgaaatgctgaacaaaaaagcggaagagaaaggcgcaacggcctaccagattactgaagctcgtagcggtgacacctggcacgctacggctgaactgtacaaataaaccctcatcgtcttgtccgacgatattgcccccggttcgggggcttttttttgcgctaatgacgaacattaaaacgcaaatgcccttccagctcttcctctgcctcatcaaacagcaatattaacgcgccaaaacggcgacgcgttttctctcccagatgaacaaattcaatctcaagtggtagcggcaggacatcgttcattaacacatcccatagtgagtcgagatcgcgtaccttatctttcgccagaccaaaggtttggctaaagtcacgataaaaatcctcctgactctcaatctcatcaaaatcaaaggtataaatattcatctgttgccaccgtcacgtttcgcggcgagttctgccgtgcatcgctaagtatagccatgaaaaaaccgacgcttttggcgtcggttttgacttaactatcggtcaacgcatgttgatacttatggagcatccccgccagccgatttaccggttccgtcacctgcggtggcgcttgccagatgcgtagcttttcctggtagatttccagttcttccagcaactggccaaagtaccgacgacgtttatcatcgctacgggcagatatcacatggtctgctgtgcggcgcatttgtcggtgaaacgccgataaatcctcgttaaccgggatcggtgcatcacgcaggcgctggtgcgcgataatcatcgtcagcgccaggcgaaatttcggcaaatcccctgggaacttattcatcagcaaaaacagctgctgataaagtgccgggaggtggttctctttacgacgtgccacattggtagtcatcgcggaaacagcggcagaaacaaactgattaagcagtacacgtccggtcctgtcgcgcgatttatcccgcaccagcaaaataacggtgaacgcgagcacacagccgacgatttgccctaatgcgctgtcgagaaactgactgaaatggaaagtcatcgggttatccagcacgataatatttatggtgctggccagtgcccccatcgagcccagtcgccgtttctgtacttctataccgaggaagaatcccagcactgccaggctaatgcacagcagcaacatgctctgttgggtattagggataatcaccaaaaagtagagcagccctaacggcagcgcggccagcgtcccgtagataaagtcgatcgccaccatgcgtggattcggcaaacgcattgccagtgacgtcactaccgcaatcatcaccattgcaccactgccggaagtccagcccgtccacagccagaaaagcgtgcccagaatgcaggaaagtgtggttcgccagaagttaaccattgcatgatgacgttcggctgactctacttttacttccggttcgccttgcaggatctcttcttcggtggcgttgatttttgtgttactgataacgccgcgcttgagaagctgataacgcgttgccgccgcgacccagctataaatggtgacaggcgtttcccgttccccggtccaggcgataactctccgcaggcgtttgagctgcttgtggacgtcctgcgcggtttctaccggcgtgtcaaaaaattcgcggaaagtatcagtgatcaattccgggcgcgtattctgaataagataagtttcgcaggattgggtaatcagcgtcagcgatagcgtattgatcgcttttaaacgtcgattggcccgcgcccagcgggaagattccatattcaggttgctgcgcatgccttgtagcgccgtggtgcgtcgcaccaggtcgccccaggctttatcgacaacttcaccatcgccatgcttgatacagagttgcattaattgatattgcgcgaccagcaaactttccagctctcgatccacttcttgtttgatcgatcgcggagaaaagagcaaatccgccataatcgcacacacaataccgataacgatctcgctacaacgttcgacggcaaactgcggcgtaagcaatggttccggctgaatggtgatcacaatgatcagcgcggtataaccggccagcccccacgcatacgagttttctattcgtaccagcgaggatatccaggtacaaaaaccggcccagatacagcacaccagaatcatcaataatggtgcgcggatcatcgcaatgatgatcaccagtccggcaatacagccaataaatgtgccgatgatgcgcaaaaagccacgatagcgaatagcgccagaatacggttcacctcccgcagcaaaggccgtaccggcggcaacaatcgccgctgtcagtaccgcccagcgtggcgtttccagctggaagtgaaagccaacaaacagcgccagtacaatggcggtcgccagttttaccgcaaagcgaatatgttggttagcaatggagaaaatacccatcgtgattaaccaaactcacgcaggcgatgggccattttacggaagaacgaatcctggctttcgtcgcgatcttgtttgccagtgaccaccactgtagcagtggtgcccgcaggccagatgttctcttgctggttgtcgagacgaatacgaaccggaacacgttgcgcaagacgcacccattcaaggttagagtctatagtcgccatccctttgtcgtcacgcgtgctgctggcgttggtgacccctgcggcaacactatcaacagtccctttcagcactttgttactgccaagcggcgtgatctctgcacgataccccggacgcaccccttccagcttagtttcttccatataggccagtacatagaaggagttctgtttcaccagcgcaaccgccgttgatcctcgagtaataaactcaccggtatagacgttgaggttggtcacccagccatctgctggcgcgcggatcaccgtgcgttcaagatccagttttgccagatcgcgggtcgcctgcgctttcgctaactgatgcagaaccgtttgtagtacgttgttggcctggtcgatctcttcgcgagacatcgcctgcacaccgagacggttacgacgtccggcctcctggcgtttctcctgtgccagtacctgataataagcaacatcggcttgcgcttcctcaagcgccttttgatagcgcggctggtcgatggtgaacagtatctgtccttttttcaccagctggttatcatgaacattcacctgggtaatgagtccagaaacgtccggcgcgatcgcaacgacgtcagcgctaaagcgcgcgtcacgcgtccagggggattcggtgtaatagacccaggcattaaaaattgcgatgaaggccagaatgactaatacgaccgtgatggccgtacgggagaattttcttattagtgttttcacttcaacctcaaacgaacagtcgcgatatcaaataaaacaagcagcaatagagcgcggtgttgaacaacgccggatgccagacaaagtcgtagatacctgttggcacaagtacccggcgcaccagccagaaaatcgccagtgataaaagcaattcaaaaaatatcggtgggaaggacagcccaaacaccacgataacgggaaacagactcatgttgaccttggttgtaaagagagagcaggcgttattattttcagcatctgtcgccgcagagaagggcatggaaagccgggcgagagcaacattgctgtagattgatatttaatatattagcgtaactgttatgctgttatctatattatgtgatctaaatcacttttaagtcagagtgaataatggaacgactaaaacgcatgtcggtgtttgccaaagtagttgaatttggctcttttaccgccgccgccagacagctacagatgagcgtttcgtccatcagtcagacggtatcaaaactggaagatgagttgcaggtaaagctgttaaaccgtagcacacgcagcattggcctgaccgaagccggtagaatttactaccagggctgccgtcgtatgcttcatgaagtgcaggatgttcatgagcaactgtatgccttcaataacacccccatcgggacgctacgcattggctgttcttcaactatggcacaaaatgttctcgccgggctgacagccaaaatgctgaaagaatacccaggtttgagcgtcaatctggttaccggaattccagcccccgacctgattgccgacggtctggatgtggtgatccgcgtcggcgcgttgcaggattccagcctgttttcccgccgtctgggcgcgatgccaatggtggtgtgcgccgcgaaaagctatctcacacaatacggcataccggaaaaacccgccgatttgagtagtcattcatggcttgaatacagcgtgcggcccgacaatgaatttgaactgatcgcaccggaagggatctcgactcgcctgatcccacaaggaagatttgtgactaatgatccgatgacgctggtgcgctggctgacggcgggtgccgggatcgcctacgtgccgctgatgtgggtgatcaacgagatcaatcgtggggagctggagatcctgctgccgcgttaccagtcagatccacgcccggtttatgcgttatataccgaaaaagataagctgccgctgaaggtacaggtcgtgatcaactcgctgacggattattttgttgaggtcggtaaattgtttcaggagatgcacgggcgcgggaaagagaagtaattcatattgtactgttacgttgtacaaacctgtgccaacgggttcccctcaccctaaccctcaccccaaaggggcgaggggaccgttcgtgcacgtagaaagattaattatccttctgaaaatagtgaaattattacgcagtaccgccaacagtcaggttatcgactttcaacgttggctggcccacgccaaccggcaaactttgcccttctttaccgcagacacccacgccgttatccagtttcaggtcgttgccaaccatcgaaatctgctgcatggtttcgataccggaaccaatcaacgttgcgcctttcaccggcttcgttactttaccgttttcaatcagatatgcttctgaagtggagaaaacgaatttgccggaggtgatatccacctgaccgccaccaaagttcggtgcatagataccgtactcaacggattcaataatttcctgcggggtcgatttacccggcagcatataggtgttggtcatacgcggcatgggcagatgggcgtaggattcacggcgaccgttgccagtcggcgtcatccccatcaaacgcgcgttgagtttatcctgcatgtagcctttcagaatgccgttctcaatcagcacgttgtactggcctggcgtaccttcgtcatcaatcgccaccgaacctcggcgatcgaccatcgtgccatcatcaaccacggtacacagttctgaagccaccagctccccgacctgtccactaaatactgaagtgccacggcggttgaagtcgccttccagaccgtgaccaaccgcttcatgcaacagcacgcccggccaacctgcgccaagtactaccggcatggtgcccgctggtgcagcaacggcagaaagattgaccagcgccatacgcactgcttcttttgcccatgcatccgcacggacttcgccgtcgagatcggcaaggaagaattcataaccaaaacgaccgccgccgccactggcaccgcgttcgcgtttgccatcttcttcgacgagaacgctcacggaaagacgcaccagcggacggacatccgccgctagcgtgccgtcggtggccgcaaccaaaattaattcatagacaccactgaggctggcagtcacttcctgtacgcgcttgtccgcttcgcgggcaaccttatcgacgcgacgcaggatatccagcttctcttcacggctcatgctttgcagcggatctaccgaggtatacaacgggctatgctctaccgcgcccagcgtctgtactttaccatcaccactatcacggacgatggtgcgcgccgcttgcgcactctgttccagcgccagcaggctgatttggtcagcgtaagcaaatccggttttttcaccgctgattgcacgcacaccaacgccctgatcgatgttgtaagaaccatctttaataatgcggtcttctaaaacccaggattcgtgatagctcgactgaaaatagagatcgccataatcaaggcgacgttcggccagttgaccgaggatcgcgaacaagtcctgatgtttcaggccgttcgccgctagcaattgttcacttaccaggttaagactcatcgtttttgctactcgttagttactgcagtagaggattttttacggctgccggatgcggcgtgaacgccctatccagcctacggttatgttccggtttgtaggcctgataagacgcacagcgtcgcatcaggcaacggctgtcggatgcggcgtaaacgccttatccgacctacggttatgttccgtttgtaggcctgataagacgcacagcgtcgcatcaggcaacggctgccggatgcggcgtaaacgccttatccgacctacggttatgttccgtttgtaggcctgataagacgcacagcgtcgcatcaggcaacggctgccggatgcggcgtgaacgccctatccgacctacggttatgttctggctcgttggcctttggcaacgattatcctatgagattggggcaattacgcgccctcgtcaaatcattgcgctttttctttacgcggttggcgcaacacttcgttgatttgcggatcgtccagcggacccgaaatgtgatagcgcaaaatggagactttgctccacagcggccccagcactttactggcggcaaacactgccgcgccaacaatggggttaaccgcaaaagccgcagccacgcccaccgtcgcagaaatctctggtgcgacaaccgcttccatattcaggtcgcgacgtaccagatttaccgaccctttcatggcgatatccgcctccaggccatccaccagcgtgtcgtcggtgtgcataacgccgtctttaatccacgcggtgctgcgaatggagtcaaaatagaacccttcgccaaaagtgtctctgaaatcaaaacgcagcttacgcatcagggcatctacgctcaataagcgcagcaattgcccggcatgtccggtattgatttcggtaatttcgcctttacccagttgagtatgaatgatgccattcaacgtcgcttcatctggctgccagggtgctttgcgccagtgtaaatcgtaatccacattaaatgacgactggcgtatgggcgtcgtgacaccaaaaaattctgcggcggcatcaattttctgcccgcgcagttttcctttcagcgaggtacgttcattccccggattattaacccattcaccatcggcagtaagccgcgagaaaccagtatcaatcagtccattggtcagcgttaacgtatcgccagaaatggtgatatcactgtcaatgcgaccgaatttttgcccccagaaccagcactctgtgcatcgtatttgggcgtccggccagccacggaagttaatgcgctccgttgtcgggaaaggtgatgacggcgttgaatcaccacgagttttcgccacgctcgggttgtaataaagatatttgatattcgccagccacggcgcgttattacgcatcgctagcgtggcgttgatttcacgcccttgcgcttcaaccagggtgccatttgccgtcggttgcgaaacaatactcaggttattccattgctgatttcccagtgacaacataggcgtacgtaacgttatgtgttgtgggaaactcgctgcaccaccgacactctccgcagcgcctttctggaacagggccagccactcggcaccattcatcggcggcatattgagttcaacgccactttgttccggcaacggcgggagcgttttactgtctgccgcccaaatagcacgatcgagcgtcagcttttgaccgagcaaccagcggctattgaaatgattatccgcaccagcctgtccggttaattcaaagctgttgagattgccatcaaccttaacgtttaccgctagtggttcacccgcaggtttggctaacggtgaaggtaagtgactgctcacattctttagatcgccgttcagctctatgttataggtcgcaccagcatgataaggcagatcaatgcccactttaccatcccacgccacgctgccactcaatgcttcgttcaccgcttcaggcagaacgccggttttcgccggttgccagttaccgttgaggtttaccgctacctggtaggcttttgccccttctttggtggaaaaatccacgttcaacggctgattaaaccagcttgctgtcagtggttcactttgcagatcgctattgataaagctgaatttaccgctcaaatttttcagggtgctgtcgagtggtttgataaacagactgttattacgcagcgtcacttcacctttcgcggttaccagttcgccgttcagcgggatatcaagatgtaagcgagcattcacatcgccgtcgagctggagttcttgcagggtcgcacccagagaatctttcagcggtgtctcatcaaagtaagggccaacggctttacccggacctttaatgtcagcgtcaatcagcagtttttcttttgagtagtcagggatcactgcggtaagattactcgcgcgcacgccgcccagattaacgccatcggttttcatccataaaccgtcgttaataaagtccagttcaatatcaaggttagttaatgcaggccagtccggctggaaggcaaacttcgcgttgcgcagcggcaccagcacttcaaactgaccttcgttgtgtttataggggaagagttgcggattgccaccataaaccagcgtcgcgttatccgcttcaccgccctgaatcgcgccacttaagtaatcaaccaggtctttacccatcaagttttccgggaaatagcgccaggcttgtgaaccatcatcggtactgatgccagccagaatacccagccagggttcatcgttagcaggttgcaggtaacgaaaaccgccgcgcgcatggacggctttggctttaacgtcaatattacgcccatccagctggaaacctttgttattgttcagccagcttatagttgcctggccgtcggcgatttctagtggcgcacggaataccgtttcgtaaggcatctttgcctgcttcatcgacgcggtaagcaaaccattttcaacgctgccggaaagcgtcccggagaagtgttccgcacccggtaataatttccattgcttccaggccagatcgctccacgatgcctgaaaacgggtcttgtctgccgcctgaagcgggatatccagcgccagagtgttaatcttgccgctcggttgtgtggagcgccaaacatcacccagtgcaggtgaaagtttcgcggccagcgggcgtatgccctccaggcctgccagctccagattactggcgcgaatccggagttcgtcactgcgtttattgtctttgccgccaacgtcctgttccggtatccaggccagcgtcaatgctccgctcggccagggtttgccgtccatcgtgatccgtgtatcgggaatagagaactgccagcccggattttcacgcgtaatatgcgcggtcagattatccaccgacagcgtatgcgtttgcttctcgcccaaccagctggcaccgccctgtttcagccagacgtcaccgccggttacatcgcctttgtcgatcgtcatccagccttcaagggagaactgtgccgtttccagcgcaatattgtcctgcatccatttaccgagccacggcttcaggtcgatgtcatccgcctggagccagacgcgaccattgcttaacaacccctcatcatcgcgcaaatccatgcgcacctgcatcacgccgtgctgtccggtaaggctggagaggcttaccaggccttccgcacggtgtcgacgtggatcgttcagccaggtgagttgtgggatcgccagctcggcgcgctgaccggatggcgtcaggaaactgacttcactgtcgcgaagatcgaaatggtcaaattgacgaagaaacagatcgctgatgtgactggcttccagactgtcatcactaccaccgctggtgataggagtgttggtgcgaaagcgcagctgccagaaagtgaggtcgcgaaactgccagcgcatatgtaacaggctctgccagacatccagcgccagagtaacgcgtttaaccgaaaattcgccgccatcttttagttctgcacggatgtcgtgtgcttcaagcgtcgggccaaaattctgccagctggctgagagctgactggcttctaccggcatgccagtcgcggattctattttgttgaggatttccggacgccaggcgtcaagatgcggtaaagcaatacgcaggccgctaaccagcagggcagcgatcacaacgagcgcggctccagtaagcagtaaaatccccggcaatcgcctcacccgtcactccttgtctgctaaaaatgtgactcaaaaaccctttgccggatggcggcccagcatctgtttacatcattacgacgtcaaactgctcctggttatagagcggttcaatttgtactttaacctgtttgccaacgaaaatttccacttccgccagcgagtgtgactcttcgcctttcaaggcttcagctactgccggagaagcatagaccaggaaacggtcggagtcgtaagcatggtggacacgaacaatctcgcgcatgatttcatagcataccgtttccacggttttcaccgttccgcgaccgtggcaggttgggcattcgttacacagtacgtgctcaatgctttcgcgggtgcgtttacgcgtcatctccaccagccccagcgccgaaaaaccattaacgctggttttcacccggtctttgctcaacgcctgctccagcgagtgcagcactcggcggcggtgatcttcattattcatatcgatgaaatcaataatgataatcccgcccagattacgcaaccgtaactggcgagcgatagcctgcgtcgcttcaatattggtattgaaaatggtgtcgtccagattgcgatgaccgacaaacgctccggtattgatgtccacggtggtcatcgcttcggtctggtcgataatgagataaccaccggatttcagttctactttgcgttccagcgctcgctggatttcgttttcgacatcaaagagatcgaaaatcggctggcgtcctgtgtaatgctccagcttgcttgtcatctcgggaatgtactccgaggtgaactcaagtaacgcttcgtaagtcaggcgtgagtcaacgcgaatgcggtccagttcggcatcggcgaaatcacgcagaacacgctgcgccagcgccagttcgccgtacagctgataacgggtctgcgggcgttttttacgctccataactttggtccagacgcgtttcagataagcggcatcggaggccagttcagcctcgccaaccccttccgctgcggtacggatgataaacccgccctgctcgtcgcaatactctgcgaccacttttttcaggcgttcacgttctgattcgctttcaatacgttgggaaaccccaacgtgagaagcccctggcataaacaccagatagcgagaagggagcgtgatatcggtggtcaggcgcgcacctttagtgccaagcggatctttcaccacctgcaccatcagatcttgcccctgacgaaccagttccgagatgtcgcgcaccgtgaattgcttttgttcttcacccgccacacattcggtgtgcggcatgatgtcggatgcatgaagaaacgcggctttatccagcccaatatctacaaaagccgcctgcatacccggaagtacacgacttacacgacccttgtagatattgcctactattccgcgtcgcgcctcacgttcaatatgaatttcctgcagaataccgccatcaatatacgccactcgcgtttccgaaggcgttacgtttactaacaattcagccgtcatgtttatcccttttctcacgcagtgcgttaaaattacttaataattcatacgtttcaaccagcggtaagccgactacggcgtgatagctgccatttatcttcctgacaaaacagccacccagcccctgaataccgtatgcacctgctttatctaacggttcatcgctggcgacatagcccgcgatgtcttcgtctgttaacgttctgaaagtcacatcggtgaccaccaggcaatcgagaatgtgctggctgtcggccaacgccactgctgtcatcacctgatgggtctgacccgataatttgcgcaacatctgcgccgcatgctctgcgtcgcgcggtttctccagcacttctccgttcaggataacgatagtatccgcacccagcaccgggagatccttcgccgtttgcgcgacacctgcccgtgctttctcgcgcgccagacgcacaacatactgctgcgcgctctcctgcggctgacgctgctcctcaatgcccgtaacaatacgttcaaaggtcacgccaagttgcgcaagtaactcctgacgacgcggagaaccggaagctaaatacagagaagtcatagaaacctttattgcactgcaaactgctgacggactttgcgcatcagcaagaaaatccacggccagagcaccccattgactacactactccagaacacttccggtctgaaagagacgttaatcactaaaaactctgcccagaaaacaataatatccaccaccagcgaaagcaacatgacgaccagcgcctgctgccataatgcgaggttgcggaaaagctggtatttcagcgccaccaggtaagcaatgatgctcatcgccaatacgcgtacgccaagcgtcgagccgctgatcagatccagtatggcacccatcacaaaacctgtgcccacatttacgcgatgaggcaaggccaggatccaatacaacaagatgagtaacacccagtttggccggaaaacaatcaggttatccggccagggcatgatttgcagcaacagcgcaatgaggaaagagagccagattacccagcgtccctggctacgatagctcgccactattgccctcccggcgcacgcgcaggcggttgagcaccactttgcggcggcgtagccctttgtggagagcgattagcagcaggctgtgtcggcgcagcaggcgcagtagctgcatttcctgtcgccggttgctgcggagtcggctgagcgatccccgttgccggttcaggtaactttggccccatcgcgtctggcgaaggcaatacctgcggcatcatctgcatcagacgttcattagcaacacgatgcacctcttccggcgtcatcgggttagcgccgttacgatctgccccccacagcagcagcagataacgcaaacgttgcagccctgcagtcggacgcgcctgaatcacagtataagcgcgctgggtatcgagttttacggaagagacaaccgcgaccggatagccttccgggaaacgaccgcccagaccggaagtcaccagcacatcaccaacacgaatatccgtattcgccggcagatgctcaagctgcaaatcatccgtacaaccgttaccggctgcaattacgcggatatcgttgcgcagcacctggattggcagcgcgtgggtcgcatcacaaatcagcagcacgcgactggtcagtttagcgacggccaccacctgaccaacaacacctttgtcgctgatgaccggctggccttcataaacgccattaacgctacctttatcgataacaacttgatcgctataaggatcgttaaccgtggagataacctgagtcaccattttctgctcatcctgacgcagcggggaacccagcagctcgcgcagacgcgcgttctcctgtttgtattgtccaagcatcagcagttcactgtttttcagcaacagttcctgacgtaacgcccggttttcaagttctaattggtcacgcgaggccagcgtctgcgatacgccatccagcaattcacgaggagcattggaaacaaagtagaaaggactgacggcggtatccatataagtacggatttgactgaacgtccccaggcggctgtcggcaataataatgccgagcgccaccagcaccgccagaataaggcgaatctgtagcgacgggccacggctaaaaattggcttcataagttatgcgtattctcgtatcagaccaggcagggtaaacagacacttcccctgcctgcatccgattactcttcgctgaacaggtcgccgccgtgcatgtcgatcatttccagcgctttgccgccaccgcgcgccacacaggtcagcgggtcttcagcaacaacgactggaatgccggtttcttccattaacaaacggtcaaggttacgcagcagtgcgccaccaccggtgagcaccatgccgcgctcggagatgtcggaagccagttccggcgggcactgttccagtgcaaccattaccgcgctcacaataccggtcagcggttcctgcagtgcttcgaggatttcattggagttcagggtaaaaccgcgtggaacaccttctgccaggttacggccacgaacttcgatttcacggacttcatcgcccggataagccgaaccgatttcgtgcttgatacgttctgcggtggcttcaccgatcagagaaccgtaattacgacgcacatagttgatgatagcttcgtcgaaacggtcaccaccaatgcgcacagaagaggagtaaaccacaccgttcaaggagataacagcaacttcagtggtaccaccaccgatatcaaccaccatagaaccggtcgcttcagaaaccggcaggccagcaccaattgcggcagccatcggttcttcaatcaggaagacttcacgggcaccagcgccctgcgcggattcacgaattgcgcggcgttcaacctgggtcgcgccaaccggcacacaaaccagaacgcgcgggcttggacgcataaagctgttgctgtgcacttgtttgatgaagtgctggagcattttttcagtcacgaagaagtcggcgataacgccgtctttcattgggcgaatggcagcaatattgcccggcgtacggcccagcatctgcttcgcgtcatgacctactgcagctacgcttttcggtgaaccggcacgatcctgacgaatggccaccacggaaggctcattcaatacgatgccttgtccttttacataaatgagggtattcgcagtacccaggtcaatggacaagtcattggaaaacatgccacgaaattttttcaacatactaagggataatcctgaaagctggggcggaaaagaaaatccgcttactttaccaaccacacgcagcagcgacaaggcgcaaaaatcatctgctacggtgaaaattagtgcagttcgtttcctttgttacaaatctctgcctgagtccagaaaggcttaatgcatcagcagcattcctcgcctgtttgcaaccgcgtaaggtcattcatctgcatatgtgctgcaacaatctggcgagcagacaagcacactcccatgagacgcagcgcgcattattctacgtgaaaacggattaaacggcaggttaaaccgagtatctttgtgaatattttttcacgttagtatcaagtggctgtgaggacgcgaaaaaatccccttgcccgcctgtaacaccgcgctgaatcagggtctgccactcgcttcgcgaacgcacgccggtggcgtaaacctgggtgctggtcccggagcaggcttccaccaggctttgaaccagcagctggttctccgttcgcttctcaatgtttctgaccagccccggatggagcttgagtaactcaacattaagttctttgatccaactggtacttaccagcgtcaaaccagcctggttgacggctacccgtacccctaaagcattcactaaacgaataacaggttgtaaacgactgatatgttgacctacatcggcctctgcaagttcaataattatgcgttttcgttgtgatttttcacattgcattaacgtatcgcgcagccaacgctgaaaacgcgggcgaatcagcgactcaacggtaacctgaatcgccagattttcctctggccagtaacgcaatagtggaataagacggctgatttgcagacggtcatactcttccgataagccaaactgcaagaccatcggcatatactccgccgagctaacctcttcattaccatcgaagatgcggcacatgagttcgcgatgatgaacctgaccttcgcgagtaaccgccggtttttgataaaggcgcgggccgccgcgactgagcatttgctcgataagcgtacgccagcgaacattaccgcgtcctttttcaggcaacgagtcatcgtaaatagcccagctattgccgccctgcaatcccgcattacgcgtggcagactctgcatgttccattacctgctcggtatcctgaccactacgccaggcgcagataccaatgtggatcatatcgtcgcgatcgagcattttattgttcggcaaggtatcaacggctttgattaactgaccggcgatgctctctgcctcttttaacgtccggtgcggtaacagcgcagcaaaatcactgcggtggtaacgcgccagcagtgcgccagggtagcgcatcataaatgtcgacagcagattcgtcagagtgaagaactgttcttcaacctggctgtgcccccaggtatcgctcaacatattgaaatccggcagacgaatcatcatcacgatcccgtgggtacctactttctcctgatcttccagtaacgttgctaactgattatcgaaaaagagtcggttattgaggccggttttcacgtcctgggcggcataagagcggatcagcgtatcaagacggctgtgttgttcgcgtgcgttctgaatttcacgaagcagcgtatccagcgcactgctggttctgggcggccattcatagatggttcccaacacattagagccacgctcaccgtttaagatacgagtagcccgggtttccagcaattcttgcccggcaagttgccgttgtaaccagcgtaccgccaggaagagcataacaatgataaagccaatcgcccccgtgagcggcgcggtggtcatcaacgaatggaaatagttgcccatcggatcctgataaaccagacgcaacgacatccccggatgctttatcaacggaacgctcagttcgcgaaacagatcgctggagccaactggacgataactaccatttctggccagggtataaacctgtttatcaccatggagcaggtctacacgaacgatatctgccgacatcattaattcggtaatttgtggccttaatacgctgaagtcattcgacacaaggtgggtatcaatcgccgtcgccaccgcctgaacgcgatgactaaacttatactgaatggcgttgtagaaacttagcgaacagcccagcaaagtcacaaaaattgttaacccggtgagcagcgtaacaaaggccgaaaatttcgtcgttaatctcatccttgtgttaactccgatagtgaggaagcgggcatactagcaaatcagatttatctcgcaatttattgcgcttcatcggctttgcttttccattagcgagtatagtcttcagaaattattttccaatccatcatgcacatgaggaccacttatgcaggcgttacttttagaacagcaggacggcaaaactctcgcatcagtacagactctggacgaaagtcgcctgccggagggcgatgtcacggtcgatgttcactggtcgagcctgaactataaagatgcgctggcgattaccggtaagggaaaaatcatccgtaattttccgatgattcctgggatcgattttgccggaactgtacgcaccagcgaagatccgcgttttcatgccggtcaggaggtgttactcactggctggggcgttggtgaaaaccactggggtgggctggcggagcaggcgcgagtgaaaggtgactggctggttgccatgccgcaagggctggacgcgcgtaaagcaatgattatcggtactgccggttttaccgccatgctgtgtgtgatggcgctggaagatgccggtgttcgcccgcaggacggggagattgtcgtgacgggtgccagtggtggcgtcggcagtaccgccgtggcgctgctgcataagttgggttatcaggtcgttgccgtttccggtcgcgaaagtacccatgaatatctgaaaagtttaggtgctagccgtgttctccctcgtgatgagtttgccgaatcccgtcctctggaaaaacaagtctgggctggggcaattgacaccgttggcgacaaagtgctggcaaaagtgctggcgcaaatgaattacggcggctgcgtggcggcctgtggtctggcgggtggttttactctgccaaccacggtcatgccatttattctgcgtaatgtccgtttgcaaggggtggattcagtaatgacgccaccagaacgccgcgcacaagcctggcagcgactggtcgccgatttaccggaatcattctatacccaggcggcaaaagagatatctctgtcagaggcaccgaactttgccgaggccatcattaataaccagatccagggtcgcacgctggtgaaggttaactaaccatttagcagggaataataagagagggaactcattttgaaatcattattcaatcggttaacgggaaaagcggttagccggacagctttcgtcgaacaccttggtcaggaagttatacaacatcatccaaactggaaagtcatgatttcgactgaccacaaattgatgcgcattgatactccactaaacagctattattgatacgcctccgtcgcctgttaggtttatgttgctttgcctgggcgacgctacgcttagccccttacttatttctggtaccatggggtgaataatctgattttgtttgactacaaattaatcactcgaacctatttaatgctgagcattgtcaatcggttaattttgcgtgctttagcattcacatctatccagacgatgcagtgaaaattgggtaatccccagcaaccgctgcgtaatgtcgtctatcttgtcgcgatcctggcatccctacattatttgtggtctgtgaagattatctcattgcagcccctcatcttcgcagggctggcttttcagcttttcaccttacgttataagaagttccgtcgatgatggcgctaatttcgtgaattgtgcggcttgttgcaaattacacggtgttgaaggttatttacatgttagctgttgattatcttccctgataagaccagtatttagctgccaattgctacgaaatcgttataatgtgcgacctcgtcctccctgacgcagtttttgcgctgcggaaaaggtgacattggcgcaacgaaggtatattttgttttttgccggaggatagcagcagatcgctgcacaatgtccgtcaagtctaacattgacactctggggcaaaatagaccggcgtcccggcctgctggaatttatcgctatgcatacagctgtcggggcatacgctttacagacggcggtgaaacgcctgtcacaatcacactaaacaaagagtacggaacccactcatggatattcgtaagattaaaaaactgatcgagctggttgaagaatcaggcatctccgaactggaaatttctgaaggcgaagagtcagtacgcattagccgtgcagctcctgccgcaagtttccctgtgatgcaacaagcttacgctgcaccaatgatgcagcagccagctcaatctaacgcagccgctccggcgaccgttccttccatggaagcgccagcagcagcggaaatcagtggtcacatcgtacgttccccgatggttggtactttctaccgcaccccaagcccggacgcaaaagcgttcatcgaagtgggtcagaaagtcaacgtgggcgataccctgtgcatcgttgaagccatgaaaatgatgaaccagatcgaagcggacaaatccggtaccgtgaaagcaattctggtcgaaagtggacaaccggtagaatttgacgagccgctggtcgtcatcgagtaacgaggcgaacatgctggataaaattgttattgccaaccgcggcgagattgcattgcgtattcttcgtgcctgtaaagaactgggcatcaagactgtcgctgtgcactccagcgcggatcgcgatctaaaacacgtattactggcagatgaaacggtctgtattggccctgctccgtcagtaaaaagttatctgaacatcccggcaatcatcagcgccgctgaaatcaccggcgcagtagcaatccatccgggttacggcttcctctccgagaacgccaactttgccgagcaggttgaacgctccggctttatcttcattggcccgaaagcagaaaccattcgcctgatgggcgacaaagtatccgcaatcgcggcgatgaaaaaagcgggcgtcccttgcgtaccgggttctgacggcccgctgggcgacgatatggataaaaaccgtgccattgctaaacgcattggttatccggtgattatcaaagcctccggcggcggcggcggtcgcggtatgcgcgtagtgcgcggcgacgctgaactggcacaatccatctccatgacccgtgcggaagcgaaagctgctttcagcaacgatatggtttacatggagaaatacctggaaaatcctcgccacgtcgagattcaggtactggctgacggtcagggcaacgctatctatctggcggaacgtgactgctccatgcaacgccgccaccagaaagtggtcgaagaagcgccagcaccgggcattaccccggaactgcgtcgctacatcggcgaacgttgcgctaaagcgtgtgttgatatcggctatcgcggtgcaggtactttcgagttcctgttcgaaaacggcgagttctatttcatcgaaatgaacacccgtattcaggtagaacacccggttacagaaatgatcaccggcgttgacctgatcaaagaacagctgcgtatcgctgccggtcaaccgctgtcgatcaagcaagaagaagttcacgttcgcggccatgcggtggaatgtcgtatcaacgccgaagatccgaacaccttcctgccaagtccgggcaaaatcacccgtttccacgcacctggcggttttggcgtacgttgggagtctcatatctacgcgggctacaccgtaccgccgtactatgactcaatgatcggtaagctgatttgctacggtgaaaaccgtgacgtggcgattgcccgcatgaagaatgcgctgcaggagctgatcatcgacggtatcaaaaccaacgttgatctgcagatccgcatcatgaatgacgagaacttccagcatggtggcactaacatccactatctggagaaaaaactcggtcttcaggaaaaataagactgctaaagcgtcaaaaggccggattttccggccttttttattactggggatcgacaacccccataaggtacaatccccgctttcttcacccatcagggacaaaaaatggacactcgttttgttcaggcccataaagaggcgcgctgggcgctggggctgacccttttgtatctggcagtttggttagtagccgcttacttatctggcgttgcccccggttttaccggctttccgcgctggtttgagatggcctgcatcctgacgccgctgctgtttattggactgtgctgggcgatggtgaaatttatctatcgcgatatcccactggaggatgacgatgcagcttgaagtaattctaccgctggtcgcctatctggtggtggtgttcggtatctcggtttatgcgatgcgtaaacggagcaccggcaccttccttaatgagtatttcctcggcagccgctctatgggcggtattgtgctggcgatgacgctcaccgcgacctatatcagtgccagttcgtttatcggcgggccaggagctgcttataaatacgggctgggctgggtattgctggcgatgattcagcttcctgcagtctggctttcactcggtattctcggcaagaagtttgcgattcttgcgcgccgctacaatgcagtgacgctgaacgatatgctgtttgcccgctaccagagtcgtcttctggtgtggctggcgagtttgagtttgctggttgcgttcgttggtgcgatgaccgtgcagtttatcggcggtgcgcgcctgctggaaaccgcggcgggtattccttatgaaaccgggctgctgatttttggtatcagcattgcgttatataccgcctttggtggctttcgcgccagcgtgctgaacgacaccatgcaagggcttgtgatgctgattggcaccgttgtgctgcttattggcgtagtacatgccgctggcggcttaagtaacgcagtacagaccttgcaaaccatcgatccgcaactggttacgccacaaggcgctgacgatattctgtcgcctgcctttatgacgtcgttctgggtactggtgtgttttggcgtgattggcctgccgcatactgcggtgcgctgtatctcttataaagacagcaaagccgtacatcgggggatcatcatcggtacgattgtggtcgcaattctgatgttcggtatgcacctggccggagcgttaggtcgggcggtgatccccgatctcaccgtaccggacctggtgatcccaacgttaatggtaaaagtgctgccaccgtttgctgccgggatcttcctggctgcaccgatggctgcgatcatgtcgacaattaacgcccaactgctgcaaagttccgctacgatcattaaagatctctatctgaatatccgtccggatcaaatgcaaaacgagacgcgtctgaagcggatgtcggcggtaattacgttagttctcggcgcgttgctgctgcttgccgcctggaagccgccagaaatgatcatctggctgaatttgttggccttcggtgggctggaagccgttttcctgtggccgctggtgctgggtctttactgggaacgcgccaacgccaaaggcgcgctaagtgcgatgatcgttggcggcgtgctgtatgccgtactcgcgacgctgaatattcagtacctgggcttccaccctatcgtgccctcgttactactaagtttgctggctttcctggtcggaaaccgtttcggtacatccgtcccgcaagctaccgttttgactactgataaataaagagttttgccatgccttggatccaactgaaactgaacaccaccggcgcgaacgcggaagatcttagcgatgcgctgatggaagcgggtgccgtttctatcacttttcaggatacccacgatacgccagtatttgaaccgctgccgggcgaaacgcgcctgtggggcgacaccgatgtgattggtctgttcgacgctgaaaccgatatgaacgacgtggtggcgattctggaaaaccatccgctgctcggcgcaggcttcgcgcataaaatcgaacaactagaagataaagactgggagcgcgaatggatggataatttccacccgatgcgctttggtgaacgactgtggatctgccctagctggcgtgatgtgccggacgaaaacgccgtcaacgtgatgttagatccagggctggcgtttggtacgggtacccatccaaccacctctctgtgcctgcaatggctcgacagcctcgatttaaccggtaaaacagtcatcgactttggctgtggttccggcattctggcgatcgcggcgctgaaactgggtgcagcaaaagccattggtattgatatcgatccgcaggcgattcaggccagccgcgataacgccgaacgtaatggcgtttctgaccgtctggaactctacttaccgaaagatcagccagaagaaatgaaagccgacgtggtggtcgctaacatccttgcaggcccattacgtgaactggcaccgttaatcagcgtcctgccggtttcaggcggtttgctgggcctttccggtattctggcaagccaggcagagagcgtttgtgaagcttatgccgatagcttcgcactggacccggtcgtggaaaaagaagagtggtgccgtattaccggtcgtaagaattaaccttcgcatcgccgtagggtgacgcggggcgaagtgcgagcaagctcacaaaaggcacgtaaatttgccgattatttacgcaaatttgcgtgccaaaattttcattcataaagaaaaattgagaacttactcaaatttctttgagtgtaaattttagtcactattttctaatatgatgatttttatgagtaattatcgcaccacgctcattttaaatgcaattctttgatccatctcagaggattggtcaaagtttggcctttcatctcgtgcaaaaaatgcgtaatatacgccgccttgcagtcacagtatggtcatttcttaactcatgcgcatcggacaatatcagctcagaaatcgcctgatcgcagcgcccatggctggcattacagacagaccttttcggacgttgtgctacgagatgggagccggattgacagtatccgagatgatgtcttctaacccacaggtttgggaaagcgacaaatctcgtttacggatggtgcacattgatgaacccggtattcgcaccgtgcaaattgctggtagcgatccgaaagaaatggcagatgcagcacgtattaacgtggaaagcggtgcccagattattgatatcaatatgggttgcccggctaaaaaagtgaatcgcaagctcgcaggttcagccctcttgcagtacccggatgtcgttaaatcgatccttaccgaggtcgtcaatgcagtggacgttcctgttaccctgaagattcgcaccggctgggcaccggaacaccgtaactgcgaagagattgcccaactggctgaagactgtggcattcaggctctgaccattcatggccgtacacgcgcctgtttgttcaatggagaagctgagtacgacagtattcgggcagttaagcagaaagtttccattccggttatcgcgaatggcgacattactgacccgcttaaagccagagctgtgctcgactatacaggggcggatgccctgatgataggccgcgcagctcagggaagaccctggatctttcgggaaatccagcattatctggacactggggagttgctgcccccgctgcctttggcagaggttaagcgcttgctttgcgcgcacgttcgggaactgcatgacttttatggtccggcaaaagggtaccgaattgcacgtaaacacgtttcctggtatctccaggaacacgctccaaatgaccagtttcggcgcacattcaacgccattgaggatgccagcgaacagctggaggcgttggaggcatacttcgaaaattttgcgtaaacagaaataaagagctgacagaactatgttcgaacaacgcgtaaattctgacgtactgaccgtttctaccgttaactctcaggatcaggtaacccaaaaacccctgcgtgactcggttaaacaggcactgaagaactattttgctcaactgaatggtcaggatgtgaatgacctctatgagctggtactggctgaagtagaacagcccctgttggacatggtgatgcaatacacccgtggtaaccagacccgtgctgcgctgatgatgggcatcaaccgtggtacgctgcgtaaaaaattgaaaaaatacggcatgaactaattcaggttagctaaatgcttgattaaaaaggcgctactcggcatggggaagcgccttttttataggtgtcacaaagggagtgaccatgagaacaggatgtgaaccgacccggtttggtaatgaagctaagaccattattcacggtgatgcgcttgccgaacttaaaaagatccccgccgaaagtgtcgatctgatctttgccgacccaccatataacatcggtaaaaattttgatggtctgatcgaagcctggaaagaagatctgtttatcgactggctgtttgaagtgattgcagagtgccaccgcgttctgaaaaagcagggcagcatgtacatcatgaacagtacggaaaacatgccctttatcgatctccagtgccgcaagctttttaccatcaaaagtcgcatcgtctggtcatatgacagttctggagtgcaggcgaaaaaacactacggctccatgtacgaacccatcctgatgatggtgaaagacgcaaagaactacacattcaacggtgatgctattctggtagaagccaaaaccggatcgcagcgcgcgttgatcgattatcgcaaaaatcctccacagccttacaatcatcaaaaagtaccgggtaacgtttgggattttccgcgcgtgcgttatttgatggatgaatatgaaaaccacccgacgcaaaaaccggaagccttactgaaacgcattattctcgcctcttccaacccaggcgatatcgttctcgacccgtttgctggtagctttactaccggtgccgtagccatcgccagcggacgaaaattcattggtattgagatcaacagcgagtacatcaaaatggggcttcgacggctggatgtcgcgtcgcattactctgcggaagaactggcgaaagtgaaaaaaagaaagaccggcaacctgtcaaaacgaagccggttaagcgaagttgaccccgatctcattacaaagtaaaggatgtgtaagcctggttttcagattattcatttcgtgtatatttcctgccagacttggttaaacatgcacaggctcaggtaatgattcgcaagtattggtggctcgtcgttttcgctgtcttcgtttttctgtttgatactttactgatgcagtggattgaactgctggcaacagaaacagacaaatgccgcaatatgaactcagttaatccactaaaactggttaactgtgacgaactgaattttcaggacagaatgtgaatttacatgacacttaattcattcgtttgatgaattaatttcgttatgttttcatctggcatgaacattcttaatacgttatcgaccagagcgggggcttgtttataaagatcataacccgccatattcattaaccagttttgaacaattccgctgaaggcaccatcaataataatcatcacaacatctaaatcgaggttatttgctacacaaccttgttgctgacacgcctgcaatacttcgcggagagtctgcggattaaagcccatcttttcgcgtatcactccctcggccagcatctcatcattaaattcacatttgtgatataagattttcagcaacgcctgctggcggggaattttggcaatatattgcaagccgacaatcaatttttcacgcaattgttgaaacgggtcatgctctaatccagccgtcaagtgttcctggattaactcccgcaatgaaggctgttgcaaccacatctcattaaacagttgagtcttgttttcgaagtgccagtagatagcgccacgcgtaacgttagcggcgtcggcaatgtcgttgagcgtcgtcttgcttacgccatgctgcgcaaactgggcgatggcagtttcaatcagttcttgccgggtcttcagagcttcggctttggttctttttgccatgattaattattcaggaaataaatatattcgacacagagtgagaaaatagcgaaggttaatctatcacctaatgtgtatttatacgagaggctaatattgagttgctataaatcgttaaataaataatatatattatttacctaagatacattcactacatcaatatatatttcaatttacgaggttttaattctgcctctttcaacccgcgtcaaaataaaacagtagaatattaatctttttttgtgtttatgtgccttgagatgcctgtattcataactattccttacatcgacgaatgataatttgtaggatagcgaactgtatttttctttctgcgagttaacgcgttgcctttttgggtaaataacgcgcttttggttttttgaggaatagtaatgacgaaacatgccaggtttttcctcctgccctcctttattctgatctccgcggctttaatcgccggttgtaacgataagggagaagagaaagctcacgtcggtgaaccgcaggttaccgttcatattgtaaaaacggccccgttagaagttaagactgaattaccaggccgcaccaatgcttatcgtatagccgaagttcgcccacaggttagcgggatcgtactgaatcgcaatttcactgaaggcagcgatgtgcaagcaggccagtccctgtaccagatcgatcccgcgacctatcaggcaaattatgacagcgcgaaaggcgaactggcgaaaagtgaagccgccgccgccatcgcgcatttgacggtaaaacgttacgttccgctcgtgggtacgaaatacatcagccagcaggagtacgaccaggccattgctgatgctcgtcaggccgatgccgccgtgattgccgcaaaagccacagtcgaaagcgctcgcatcaatcttgcttataccaaagtcactgcgccaattagcggacgtatcggcaaatcgactgtgaccgaaggcgctcttgtcactaatgggcaaacgactgaactggcgactgtccagcagctcgatcctatctacgttgatgtgacccaatccagcaacgattttatgaggctgaagcaatccgtagagcaaggaaatttgcataaggaaaacgccaccagcaacgtagagttggtcatggaaaacggtcaaacctatcccctgaaaggtacgctgcaattctccgatgtgaccgttgatgaaagcaccggctccataaccctacgtgctgtcttccctaacccgcaacatacgcttttgccgggtatgtttgtgcgtgcacggattgatgaaggcgtccaacctgacgccattcttatcccgcaacaaggcgttagccgcacaccgcgtggtgatgcaaccgtgctgattgttaacgataaaagtcaggttgaagcgcgccctgtcgttgccagtcaggcgattggcgataaatggttgattagtgaaggactgaaatctggcgatcaagtcattgtcagcggcctgcaaaaagcgcgtccgggagagcaggttaaagccactaccgatacccccgcagatactgcatcgaagtaaggtaatctgacatggcaaacttttttattcgacgaccgatatttgcatgggtgctggccattattctgatgatggcgggcgcactggcgatcctacaattgcccgtcgctcagtatccaacaattgcaccgcctgcggtttctgtttcagcaaactatccgggcgctgatgcgcagaccgtgcaggatacggtgacgcaggttatcgaacagaatatgaacggtatcgataacctgatgtatatgtcctccaccagcgattccgccggtagcgtgacaattacccttaccttccagtccgggaccgatcctgatatcgcgcaagtgcaggtgcagaacaaactccagctcgccacgccgttgctgccgcaggaggttcagcagcaggggatcagtgttgaaaagtccagtagcagctatttgatggtggcgggctttgtctctgataacccaggcaccacacaggacgatatctcggactatgtggcctctaacgttaaagatacgcttagccgtctgaatggcgtcggtgacgtacagcttttcggcgcacagtatgcgatgcgtatctggctggatgccgatctgctaaacaaatataaactgacaccggttgatgtgattaaccagttgaaggtacagaacgatcagatcgctgccggacagttgggcggaacgccagcgttaccagggcaacaattgaacgcctcgattattgctcagacgcggtttaaaaatccggaagaattcggcaaagtgaccctgcgcgtaaacagtgacggctcggtggtacgcctgaaagatgtcgcacgggttgaacttggcggtgaaaactataacgttatcgctcgtatcaacggaaaaccggcggcgggcctggggattaagctggcaaccggcgcgaatgctctcgataccgcgaaagccattaaggcaaaactggcggaattacagccattcttcccgcagggaatgaaggttctctacccttatgacaccacgccattcgtccagctttctattcacgaagtggtaaaaacgctgttcgaagccattatgctggtgttcctggtgatgtatctgttcttgcagaatatgcgagcaacgctgatccccaccattgcggtacccgtggtgttgttagggacgtttgccatcctcgccgcttttggttactccatcaacacactaacgatgttcgggatggtgcttgccatcgggctgctcgtcgatgatgcgatagtggtggtggagaacgtcgagcgcgtgatgatggaggataagctcccgccaaaagaagcgacggaaaaatcgatgtcgcaaattcagggcgcactggtgggtatcgcgatggtgctgtcagcggtatttattccgatggcattcttcggcggttctactggggcaatttatcgccagttctctatcaccatcgtttcggcaatggcgctttctgttctggtggcattgattcttacccctgcgttatgtgcaacgctgcttaaacccgtctctgctgagcatcacgaaaataagggcggtttcttcggttggtttaataccaccttcgatcatagcgttaaccactacaccaacagcgtcggcaaaatcctcggatccacaggacgatatttactgatctatgcgctgattgttgcaggaatggtggtgttgtttttacgtcttccgtcttccttcttacctgaagaggatcagggtgtctttctgaccatgattcagttacccgctggcgcgacgcaagagcggacgcaaaaagtgttggatcaagttacggattactatctgaagaacgagaaagcgaacgttgaaagtgtctttacggttaacggctttagcttcagcggccaggcacaaaacgccggtatggccttcgtcagtctgaaaccgtgggaagagcgtaatggtgacgaaaacagtgcggaagcggtaatccatcgtgccaaaatggaattgggcaagatccgcgacggttttgtcattccattcaatatgccagccattgttgaactgggcacggcaacgggtttcgactttgagttaattgatcaggctgggctgggtcacgatgccctaacccaggcccgtaaccagttgcttggtatggcggcgcaacatcctgccagcttagtcagcgtgcgccctaatggcctggaagacaccgcgcagtttaaactggaagttgaccaggaaaaggcgcaggcattaggtgtttcactttctgacatcaatcagaccatttcaacggcgctgggtgggacttacgttaacgacttcatcgaccgtggccgcgtgaaaaagttgtatgttcaggcggatgccaaattccgtatgctgccagaagatgtcgataaactttatgtccgcagcgccaacggcgaaatggtgccattctcggcctttaccacttcacattgggtgtatggctctccgcgactggaacgctacaacggtctgccgtcaatggagattcagggggaagccgcgccaggaaccagttccggcgatgccatggcgttgatggaaaaccttgcgtcaaaattacctgcgggcattggttatgactggacgggtatgtcgtatcaggaacgcttatcgggaaaccaggctcccgctctggtagcaatttcctttgtggttgttttcctgtgccttgctgcactctatgaaagctggtcaattcctgtctcggttatgttggtagtgccgttagggattgtcggcgtgctgctggcggcgacactctttaatcaaaaaaatgacgtctactttatggtgggcttgctaacgacaattggcttgtcggccaaaaacgctattttgatcgttgagttcgctaaagatctcatggagaaagagggtaaaggtgttgttgaagcgacactgatggcagtacgtatgcgtctgcgtcctatcctgatgacctctctcgcctttattctcggcgtattaccgctagctatcagtaacggtgccggcagtggcgcgcagaacgctgtgggtatcggggtaatgggaggaatggtctctgcaacgttgctggcaatcttcttcgtaccggtgttctttgtggtgatccgccgttgctttaaaggataaatcagaaacataaaggcgctttcgggtgcctttattatttccagtgaaacccataaaaattaataagatattcttctgctcactctttaaaagctttctatagttcccgctcccttcactatttttacaattcacataatttgtcattattcattccgcaagatttataacctccggtgataaaatggcattcagctcgttaataagagagttaacttattaagcgttagcgtttattactgaggtaacaccatgaaaagattaattcctgtggcattgctcaccgcattgctggcgggctgtgctcacgattcgccctgcgttccggtttatgacgatcagggtcgtctggttcacaccaatacctgtatgaaaggcacgactcaggataactgggaaacggctggggctattgccggcggggcagctgctgttgctggcctgacgatggggatcatcgctctatcgaaataactgaacagggcgcggagttccgcgctctttttaacgatacagtatctctccataagataaaatattgctatattctgctgggtaattccctgctgatttagcatgttacatcgcgttatttcgctgctttcgaaataacgcatcaatttaattttcacacttcccaccagaaatatactcacgctaacaatcattattctgcttagtaaaacacgcgtaaatattttgcgccaaaatgtggcgcatgtttcattttcgcaccattgcggggcgctgtttttattatttcctgtctacactcagcttattgcgacgcgaaatcgtgcgcaaaagctggcactacttttgcttataagaggatggccacagacaggtaaaagacgtttcccaaacgtcctataacgataattttcgcctcacaggaagcattatgaaaaagatgatgatagccacactggctgccgccagcgtgctgcttgccgttgcaaatcaggcgctgctggcgcgacgcttgatgccgttcagaaaaaaggttttgtgcaatgcgggatcagtgatggattacctgggttctcttatgccgatgctgacggtaagttttcaggtattgatgttgatatttgtcgtggtgttgccgctgctgtatttggtgacgacacgaaagtgaaatataccccgctcactgcaaaagaacgcttcaccgctttacagtcaggggaggtggatttgctctcccgtaatacgacctggacttcatctcgcgatgccgggatgggaatggcatttaccggcgtcacttattacgacggcattggcttcctgacgcacgataaagcggggctaaaaagcgcgaaagaactggatggcgctaccgtctgtattcaggcgggtactgataccgaactcaacgtcgccgactacttcaaggcaaacaatatgaagtacacaccggtgactttcgatcgctctgacgaatcagcgaaggcactggaatctggtcgctgcgatacgctggcctcggatcaatcacaactgtatgccctgcgcatcaaattaagcaacccagctgaatggattgtcttaccggaagttatctcaaaagaaccgcttggtccggtagttcgtcgtggcgatgatgaatggttctcgattgtacgctggacgcttttcgccatgctgaatgctgaagagatgggcatcaattcccagaacgtcgatgaaaaagcggctaatccagcaacgcctgatatggcacatctgctgggtaaagaaggcgattacggcaaggatctgaagctggataataaatgggcctataacatcatcaaacaggtgggtaactactcggaaatttttgagcgtaacgtaggttcagaaagcccgctgaaaattaaacgtgggcaaaataatctctggaataacggcggtattcagtacgcaccgcccgtgcgttaagtcggtgtgaggtaacgagcgtcgctacggcggcgctctcttcagcgttatgctttccgaggtttctatgtctcatcgccgctcaaccgttaaaggctcactctcttttgccaaccctacggttcgcgcctggttattccagatccttgccgttgttgctgttgtcggcattgttggttggttatttcacaacactgtaacgaatctcaataatcgtggcattacttcaggttttgcctttctggatcgcggcgctggcttcggtattgtccagcatttgatcgattaccagcagggcgacacctacggacgcgtttttattgtcggcttactcaatacgctactggtttctgcattgtgtattgtgttcgcttctgttttgggcttctttatcggtctggcgagactttcggataactggctgctacgaaagctttccacaatttatattgagatcttccgtaatattcccccgctgctgcaaatcttcttctggtactttgccgtgttgcgcaatttgcccggaccacgccaggctgtgagcgcgtttgatctggcctttttgagcaatcgtgggctttatattccgtcaccgcagctgggagacggatttattgcgtttatcctggctgttgttatggctatagtcctttctgttgggctattccgctttaataaaacataccagataaagaccggacaactgcgccgcacctggccgatcgccgcagtgttgatcattggtttgcctttactggcgcaatggctttttggcgcagcactacactgggatgtcccagccctacgaggctttaacttccgcggcgggatggttttaattcctgaactggcagccttaacgctggcactttcggtttatacatctgcatttatcgccgagattatccgcgctgggatccaggcagtgccttatggtcaacatgaagcggctcggtcactgggattacccaacccggttacgctacgccaggtcattattccccaggcattgcgggtgattattccaccgttaaccagccagtatctcaacatcgtcaaaaactcctctcttgccgccgctattggctatcccgatatggtttcgctgtttgccggcaccgtgctgaatcagacggggcaagccatcgagacgatagccatgaccatgtcggtctatctgattatcagcctgactatctcgctgctgatgaatatctataaccgccgcatcgcgatcgttgaacgctaaggagtcatgatgacaaaagtattgctgtctcatcccccgcgcccggcgagccataactcaagccgcgcgatggtgtgggtgcgaaaaaatctgttctccagctggagcaatagcctgctgactattggctgcatatggttgatgtgggaactgatcccaccgttgctgaactgggcatttttgcaggctaactgggttggctcaacgcgtgccgactgcacaaaagccggtgcctgttgggtcttcatccacgaacgatttggtcagtttatgtatgggctttacccacacgaccaacgctggcgaattaacctcgcattactgattgggcttgtgtcgatcgcaccaatgttctggaaaatactcccgcatcgcggtcgctatattgcggcctgggcggtgatttacccactgattgtctggtggctgatgtatggcggtttttttgctcttgagcgggttgaaacccggcaatggggcgggctgacgctaactttaattattgcatcagttgggattgcgggggcgctaccgtgggggatcttactggcgttaggtcgccgctcccatatgccgattgtgcgtatcttatcggtcatttttatcgaattctggcgcggcgtgccgctgattaccgttctgtttatgtcttcggtcatgctgccgttgtttatggcagaaggcaccagtatcgacaaattgatccgcgcgctggttggcgtgatcctgtttcagtcagcatatgttgcggaagtcgtgcgaggtggattacaggcgctgcctaaagggcaatatgaagcggcagagtcgctggcgttgggttactggaaaactcaggggctggttattctgccacaggcgttgaagctggtaattcctgggctggtaaataccatcatcgcactcttcaaagataccagcctggtgatcattatcgggttgttcgatcttttcagtagcgttcagcaggcaaccgttgatcccgcctggttgggtatgtcgacggaagggtatgttttcgccgcgctgatctactggatcttctgtttcagcatgtcgcgctatagccagtatctggaaaaacgttttaacaccgggcgtacaccgcattgaggacactatgagccaaattttactgcaacctgctaacgcgatgattacgctggaaaacgtcaataaatggtatggacaattccatgttttgaaaaatataaatttaaccgtgcaaccgggagaacggatcgttctgtgtggcccttcaggttccggtaaatcgacaaccattcgttgtattaatcatctggaagaacatcaacagggacggatcgtggtagatggcatcgaacttaatgaagatatccgcaatattgagcgcgtcaggcaggaagtgggaatggtctttcagcatttcaatctcttccctcatctgaccgttttacagaactgtaccctggcaccgatttgggtacgcaagatgcctaagaaagaggctgaagatctggcggtgcattacctagagcgggtgagaattgccgaacatgcgcataagtttcccggacagatttcaggtggtcagcagcaacgcgttgccattgcgcgttcgctgtgtatgaagccgaaaattatgttgtttgatgagccaacgtcggcgctcgatcctgagatggtgaaagaggtgctggatacgatgattgggctggcgcagtcgggtatgacaatgttgtgtgtaacacatgagatggggtttgcacgaaccgtcgctgaccgggtaatttttatggatcgtggggaaatagtggagcaagctgcacctgatgaattttttgcgcatcctaaatcagagcgtacgagggcatttttatcgcaggtaatccattaattgaatgttagttcgaaaagcaaaaaggccatcctttcggatggcctttcgcttgatttgatgtctggcagtttatggcgggcgtcctgcccgccaccctccgggccgttgcttcgcaacgttcaaatccgctcccggcggatttgtcctactcgggagagtgttcaccgacaaacaacagataaaacaaaaggcccagtcttccgactgagccttttgttttatttgatgtctggcagttccctactctcgcatggggagaccccacactaccatcggcgctacggcgtttcacttctgagttcggcatggggtcaggtgggaccaccgcgctactgccgccagacaaattcttttctaatctgccgaactttaacctaaaaagtggtgctgatacccagagtcgaactggggacctcacccttaccaagggtgcgctctaccaactgagccatatcagcacgctaaatttgatgcctggcagttccctactctcgcatggggagaccccacactaccatcggcgctacggcgtttcacttctgagttcggcatggggtcaggtgggaccaccgcgctacggccgccaggcaaattctgttttatcagaccgcttctgcgttctgatttaatctgtatcaggctgaaaatcttctctcatccgccaaaacagcttcggcgttgtaaggttaagcctcacggttcattagtaccggttagctcaacgcatcgctgcgcttacacacccggcctatcaacgtcgtcgtcttcaacgttccttcaggacccttaaagggtcagggagaactcatctcggggcaagtttcgtgcttagatgctttcagcacttatctcttccgcatttagctaccgggcagtgccattggcatgacaacccgaacaccagtgatgcgtccactccggtcctctcgtactaggagcagcccccctcagttctccagcgcccacggcagatagggaccgaactgtctcacgacgttctaaacccagctcgcgtaccactttaaatggcgaacagcatcacccttgggacctacttcagccccaggatgtgatgagccgacatcgaggtgccaaacaccgccgtcgatatgaactcttgggcggtatcagcctgttatccccggagtaccttttatccgttgagcgatggcccttccattcagaaccaccggatcactatgacctgctttcgcacctgctcgcgccgtcacgctcgcagtcaagctggcttatgccattgcactaacctcctgatgtccgaccaggattagccaaccttcgtgctcctccgttactctttaggaggagaccgccccagtcaaactacccaccagacactgtccgcaacccggattacgggtcaacgttagaacatcaaacattaaagggtggtatttcaaggtcggctccatgcagactggcgtccacacttctaagcctcccacctatcctacacatcaaggctcaatgttcagtgtcaagctatagtaaaggttcacggggtctttccgtcttgccgcgggtacactgcatcttcacagcgagttcaatttcactgagtctcgggtggagacagcctggccatcattacgccattcgtgcaggtcggaacttacccgacaaggaatttcgctaccttaggaccgttatagttacggccgccgtttaccggggcttcgatcaagagcttcgcttgcgctaaccccatcaattaaccttccggcaccgggcaggcgtcacaccgtatacgtccactttcgtgtttgcacagtgctgtgtttttaataaacagttgcagccagctggtatcttcgactgatttcagctccacgagcaagtcgcttcacctacatatcagcgtgccttctcccgaagttacggcaccattttgcctagttccttcacccgagttctctcaagcgccttggtattctctacctgaccacctgtgtcggtttggggtacgatttgatgttacctgatgcttagaggcttttcctggaagcagggcatttgttgcttcagcaccgtagtgcctcgtcatcacgcctcagccttgattttccggatttgcctggaaaaccagcctacacgcttaaaccgggacaaccgtcgcccggccaacatagccttctccgtccccccttcgcagtaacaccaagtacaggaatattaacctgtttcccatcgactacgcctttcggcctcgccttaggggtcgactcaccctgccccgattaacgttggacaggaacccttggtcttccggcgagcgggcttttcacccgctttatcgttacttatgtcagcattcgcacttctgatacctccagcatgcctcacagcacaccttcgcaggcttacagaacgctcccctacccaacaacgcataagcgtcgctgccgcagcttcggtgcatggtttagccccgttacatcttccgcgcaggccgactcgaccagtgagctattacgctttctttaaatgatggctgcttctaagccaacatcctggctgtctgggccttcccacatcgtttcccacttaaccatgactttgggaccttagctggcggtctgggttgtttccctcttcacgacggacgttagcacccgccgtgtgtctcccgtgataacattctccggtattcgcagtttgcatcgggttggtaagtcgggatgacccccttgccgaaacagtgctctacccccggagatgaattcacgaggcgctacctaaatagctttcggggagaaccagctatctcccggtttgattggcctttcacccccagccacaagtcatccgctaatttttcaacattagtcggttcggtcctccagttagtgttacccaaccttcaacctgcccatggctagatcaccgggtttcgggtctataccctgcaacttaacgcccagttaagactcggtttcccttcggctcccctattcggttaaccttgctacagaatataagtcgctgacccattatacaaaaggtacgcagtcacacgcctaagcgtgctcccactgcttgtacgtacacggtttcaggttctttttcactcccctcgccggggttcttttcgcctttccctcacggtactggttcactatcggtcagtcaggagtatttagccttggaggatggtccccccatattcagacaggataccacgtgtcccgccctactcatcgagctcacagcatgtgcatttttgtgtacggggctgtcaccctgtatcgcgcgcctttccagacgcttccactaacacacacactgattcaggctctgggctgctccccgttcgctcgccgctactgggggaatctcggttgatttcttttcctcggggtacttagatgtttcagttcccccggttcgcctcattaacctatggattcagttaatgatagtgtgtcgaaacacactgggtttccccattcggaaatcgccggttataacggttcatatcaccttaccgacgcttatcgcagattagcacgtccttcatcgcctctgactgccagggcatccaccgtgtacgcttagtcgcttaacctcacaacccgaagatgtttcacttcagagttgcgaaaatttgagagactcacgaacaactttcgttgttcagtgtttcaattttcagcttgatccagatttttaaagagcaaaacttcgcagtgaacctttgcaggtacactctgaagtattttttatttaatcactacagagatggtggagctatgcgggatcgaaccgcagacctcctgcgtgcaaagcaggcgctctcccagctgagctatagccccataacatgtagttaaaacctcttcaaatttgccgtgcaaatttggtaggcctgagtggacttgaaccaccgacctcacccttatcaggggtgcgctctaaccacctgagctacaagcctgtagaggttttactgctcattttcatcagacaatctgtgtgagcactgcaaagtacgcttctttaaggtaaggaggtgatccaaccgcaggttcccctacggttaccttgttacgacttcaccccagtcatgaatcacaaagtggtaagcgccctcccgaaggttaagctacctacttcttttgcaacccactcccatggtgtgacgggcggtgtgtacaaggcccgggaacgtattcaccgtggcattctgatccacgattactagcgattccgacttcatggagtcgagttgcagactccaatccggactacgacgcactttatgaggtccgcttgctctcgcgaggtcgcttctctttgtatgcgccattgtagcacgtgtgtagccctggtcgtaagggccatgatgacttgacgtcatccccaccttcctccagtttatcactggcagtctcctttgagttcccggccggaccgctggcaacaaaggataagggttgcgctcgttgcgggacttaacccaacatttcacaacacgagctgacgacagccatgcagcacctgtctcacggttcccgaaggcacattctcatctctgaaaacttccgtggatgtcaagaccaggtaaggttcttcgcgttgcatcgaattaaaccacatgctccaccgcttgtgcgggcccccgtcaattcatttgagttttaaccttgcggccgtactccccaggcggtcgacttaacgcgttagctccggaagccacgcctcaagggcacaacctccaagtcgacatcgtttacggcgtggactaccagggtatctaatcctgtttgctccccacgctttcgcacctgagcgtcagtcttcgtccagggggccgccttcgccaccggtattcctccagatctctacgcatttcaccgctacacctggaattctacccccctctacgagactcaagcttgccagtatcagatgcagttcccaggttgagcccggggatttcacatctgacttaacaaaccgcctgcgtgcgctttacgcccagtaattccgattaacgcttgcaccctccgtattaccgcggctgctggcacggagttagccggtgcttcttctgcgggtaacgtcaatgagcaaaggtattaactttactcccttcctccccgctgaaagtactttacaacccgaaggccttcttcatacacgcggcatggctgcatcaggcttgcgcccattgtgcaatattccccactgctgcctcccgtaggagtctggaccgtgtctcagttccagtgtggctggtcatcctctcagaccagctagggatcgtcgccttggtgagccgttaccccaccaacaagctaatcccatctgggcacatccgatggcaagaggcccgagggtccccctctttggtcttgcgacgttatgcggtattagctaccgtttccagtagttatccccctccatcaggcagtttcccagacattactcacccgtccgccactcgtcagcgaaacagcaagctgtttcctgttaccgttcgacttgcatgtgttaggcctgccgccagcgttcaatctgagccatgatcaaactcttcaatttaaaagtttgatgctcaaagaattaaacttcgtaatgaattacgtgttcactcttgagacttggtattcatttttcgtcttgcgacgttaagaatccgtatcttcgagtgcccacacagattgtctgataaattgttaaagagcagttgcgacgcggctttcagctcactgtcgcgaggtggcgtatattacgctttcctctttcagagtcaaccctgaatttcaggatttttttctcttcgttgttccgaccatcctgtgaagtgtttcacgttgtcgtctcaacggaggcgcattatagggatcccaattttttgcacaagtatttttttgatctttttttctgtttgttgttttttcaccctttttgctgcaatcgcacacaaaacggtgcttttttgcatactaaaagacttgcacaaggccaataatgcccccaaagtcattagtaaatcatttattgctgaggtaagtatgtctgatgttttacgcccataccgcgatctttttccacaaatcggtcagcgcgtaatgatcgacgatagcagtgtcgtgattggtgacgttcgtctggctgatgatgtggggatctggccgctcgttgtgattcgtggagatgtacattatgtacagatcggagcacgcaccaatatccaggatggcagtatgttgcatgtcactcataaatcctcgtacaacccagatggcaacccattaaccattggcgaagatgtcactgttggtcacaaggtgatgctccacggctgcaccattggcaatcgagttttggttgggatgggctcaattttacttgatggcgcaatagtagaagatgatgtgatgattggtgcgggtagtctggtcccacaaaataaacggctggagagcggatatctgtatctcggtagccccgtcaaacagatccgcccgttaagtgatgaagagaaggctgggttacgctattccgcgaataattacgtgaaatggaaggacgaatatctggatcagggtaaccagacccagccttgatcatcttcactttgttcctgaattaagttttccgcttcttcttccaggtcccagcgatgctgacgaaaactcgctaaccactgttctggcgtatctccagtaaagcgatacgccagactctcgccagagatcgcgcatgtcagttgcataccattcacgagagcgggaaaacatacacattttttattctcgtcccactcttccctgtccggaaactggatggcctgattcacgcggacaattcctcctgcaattgctttataactggttctacgtcaggcagaacaccgtgccagagaagaaaggcatgagccgcctgtgccaccagcattcctaaaccatcagcattacgctttgagcctcgctgctcacaccatgccagaaaaggagtttttcctttctgatagaacatgtcatagcaataaatgcctggatgaatgagcgatgacgggatcgccggaatatcaccactgatgccactggatgttgcattaataatgagatcaaactcatgaccttccagttcgtccatactcaacgcctgaatactgccagtgtgcgcaaacaatttagccaactcttccgcgcgggataccgtccgattagttattgtcaccgcacagtccagggaaaggagtggcagtagtacgccgcgagatgctccaccagcgccgataagcagaatacgtaaaccagggcggataaaagacagacgttccagatcgcttaacaagcctacaccatcggtattgtcacccagcaggcgtccatcttctaaccgcatgagggtattaacagcaccagccaacgctgcccgttcagtaagctcatccgctctggcaaaagcctcttctttaaaaggcaccgtcacattcgcacctttaccaccagcactaaagaaagcgttcagtgtgttgatgaaatcattgatgggtgccaacacgcgcccatagggatgttcaatattcagttgctgagcaaattgctgatgaatgaatggcgatttgctgtgggctatcggattaccaaaaacagcataggtttccattatgttacccctgtcgaaacagttcacccgtcagggcatcgcggatttctgaaggatttaaacgcccccccgtttcaccaggcacaaccgggaacgccgcgccaaattgtgcgcgaacttcgtctactgttcgacaaggtggcaatccactcaagttggcactggtagaaaccagcggtttaccataagcctggcacaaagcaaccaccaacggatggtcggtgactcgtacagcaagcgaatcaaagcggcccgtcaaccagcgcggtgttgtcgcaggcgcgggaaagacaaaggtgacaggacctggccagcgggaaaaaatggtttcacgctgcacgtcagtcaacatggtgtcatcaatatagggtttaagctgctcgtaatttgctgcgattaaaatcagccccttatcaaccggacgctgttttaactccaacagtcgcatcactgctgtttcgctatcaggatcgcacccaacaccgaaaacggcttccgttggataggcgatgacacgttcttcattgagaacatctatcgcagctgcgatagcgtctctttgcaggttattattcacgttattattccgccgaaaccggctttccacattgtttactggcacaaaagtgttttacaccctgcgcggttttcttttcgatgagtagcggataatgacactcagggcattctccagctatgggtttgaagttaatggcaaattgacactccgggtagcgatcacaagagtgaaatgttttgccataacgggagcggcgctggaccagatggcccgtccgacattgggggcatgtaattgctgtttcgtccggtttatcgataagttcggtatgttcgcattcagggtagttaatgcaaccaataaacataccaaagcgtccctggcgtaataccagatttgcgccacatgcagggcaaacctgcccctccagaactttgacgatatgtccatccgctgaagatttcagaggacggacgtagtcacacgccggatactgtgagcatccaagaaacggaccgtgtttcccggatcgaataaccagttcagccccgcactttgggcaggactcattattacgcaccgtgaacagtgctgatttcgccataacaacttatgctgaattaaagaaatgattaatgcagcataccttcattcacttcaaagagtaattcttccatttgctggtacgcattttcgcagcccggaatattgaacaacaccatcaggatcacccatttcagatcatccagttcgaactctgcgttatccagcgcgagcactcgctctatcaccatttcacgagtttcaaggttgagcacctgaatctgctcaaggaaaagcagaaacccacggcagctggcatccagtcgttcacactcttccggtgtataaatacgcatggagagaggatccgaggccagttgcatcggttctgccaacccttcctgataatcagcaagtttttccagccatagcagggcattgtagatatcttctcgctcaaaacctgcgtcggtaagatcctgttcaagtttgtcttgatccacacgcaactcagcttctgtgtgaatataggtttcaaacaaatacattagtacgtcgaacatggcatgccctcctcaatcggacatagccgccgggtacagctgcgatccatcctgctaactccagttcgagtagttgagtaactacctctggcacaggttggccggcacgttcagcgacgacgtcaacaggtgttacctcatctcctacgttagccaggagctcaggaaatggcaatgccacgtcttgctgatctggtgaataaaatgaattttcaggggcgtctggcaaccagtgcaatccaaattgcaagttttccagaatttcttccggttccgtcacaagaatcgcaccttgttttattaaccagtgaggcccttcgcttcccggattccctattggacctggcaaggcaaaaacttctcgcccctgctcaagcgcacaacgtgctgtcaccagcgaaccactacgcaaagccgcttccaccaccagtacacctttacttagaccactgataatgcgatttcttcgtgggaaattgtaagcaaggggtggaacatcgaggggaaattccgagacgagagcgcccccctgttcaagcagactggcagccagtcgggcatgacggcggggatgaatggtattaagtccattccccaatacagcaatgctgacgccatttacctgtaaggctgctttatgcgctacaccatcgattccacgcgccagtccactcgtaattgtcactccacgcgtcgccagagtttcgcaaaataatcgtccccatcgctcgccataccatgaatgcgcccgactccccactacggcaagctgaaatgaatgcagcgcgtgcagttctccttcaacaaacagtgcgccggggtaatctgtcgtcgccagaagttgaggaggataaaattcgctgtccgcaggaattaaatgatggttgggttgctccaaccaacaaagtgagctttcgatactctttcgtggaaatgaaagaaagcgttgtgcctgccgcaatgtaagccctgtttgctgcaatacaaccgcatcaatatgcgactgttttgccacccagtgagcgatacggaccatatcatcgccgtacaagctgctgatactcattaaacgcagccaaatttctgtatcgaccatccttatctccctgccataagcagccttagcaatctttgcgattggtcagtgatgctgtcaatcagagggggatttgtctagaatagaagaaataatctttctaactcctgaacacatctctggagatttatgtcagttttgcaagtgttacatattccggacgagcggcttcgcaaagttgctaaaccggtagaagaagtgaatgcagaaattcagcgtatcgtcgatgatatgttcgagacgatgtacgcagaagaaggtattggcctggcggcaacccaggttgatatccatcaacgtatcattgttattgatgtttcggaaaaccgtgacgaacggctagtgttaatcaatccagagcttttagaaaaaagcggcgaaacaggcattgaagaaggttgcctgtcgatccctgaacaacgtgctttagtgccgcgcgcagagaaagttaaaattcgcgcccttgaccgcgacggtaaaccatttgaactggaagcagacggtctgttagccatctgtattcagcatgagatggatcacctggtcggcaaactgtttatggattatctgtcaccgctgaaacaacaacgtattcgtcagaaagttgaaaaactggatcgtctgaaagcccgggcttaaggataagaactaacgtgtcagaatcactacgtattatttttgcgggtacacctgactttgcagcgcgtcatctcgacgcgctgttgtcttctggtcataacgtcgttggcgtgttcacccagccagaccgaccggcaggacgcggtaaaaaactgatgcccagcccggttaaagttctggctgaggaaaaaggtctgcccgtttttcaacctgtttccctgcgtccacaagaaaaccagcaactggtcgccgaactgcaggctgatgttatggtcgtcgtcgcctatggtttaattctgccgaaagcagtgctggagatgccgcgtcttggctgtatcaacgttcatggttcactgctgccacgctggcgcggtgctgcaccaatccaacgctcactatgggcgggtgatgcagaaactggtgtgaccattatgcaaatggatgtcggtttagacaccggtgatatgctctataagctctcctgcccgattactgcagaagataccagtggtacgctgtacgacaagctggcagagcttggcccacaagggcttatcaccacgttgaaacaactggcagacggcacggcgaaaccagaagttcaggacgaaactcttgtcacttacgccgagaagttgagtaaagaagaagcgcgtattgactggtcactttcggcagcacagcttgaacgctgcattcgcgctttcaatccatggccaatgagctggctggaaattgaaggacagccggttaaagtctggaaagcatcggtcattgatacggcaaccaacgctgcaccaggaacgatccttgaagccaacaaacaaggcattcaggttgcgactggtgatggcatcctgaacctgctctcgttacaacctgcgggtaagaaagcgatgagcgcgcaagacctcctgaactctcgtcgggaatggtttgttccgggcaaccgtctggtctgatagtccactcttctaagcccggtcttgccgggcgtttttatacttatgaaaaaacaacgtaatttacgtagcatggcggcccaggccgttgaacaagtcgtcgagcaagggcaatcattaagcaacattctgccaccgctccagcaaaaagtttccgataaagacaaagcacttcttcaagagttgtgctttggcgtactgcgtacgctttcgcagttagactggctgattaataagttaatggcccgtccgatgaccggcaaacagcggaccgtgcattacctgattatggttggtttgtatcaactgctttatacccgcattccacctcatgctgcgctggctgaaacggttgaaggcgctatcgcaattaagcgtccgcaacttaaagggttgataaacggtgtattacgccagttccagcgtcagcaagaagagttattagccgagtttaatgccagtgatgcacgttatctgcatccttcctggttgctgaagcgtctgcaaaaagcgtatccagagcagtggcaatccatcgtcgaagccaataaccagcgtccgccaatgtggctgcgtattaatcgtacgcatcattcccgcgacagctggcttgcattgctggatgaagcaggaatgaaaggtttcccgcatgcggattaccctgatgctgtacgtctggaaacacctgcacctgttcatgcgctacctggttttgaagacggatgggttaccgttcaggatgcatcagcacaaggttgcatgacctggcttgcgccacaaaacggtgaacacattttggatctttgtgccgcccccggcggtaaaacaacgcatatccttgaggtggcaccagaagcgcaggttgttgcggttgatatcgacgaacagcgcctctctcgggtttacgacaatttaaaacgccttggtatgaaggcgaccgtgaaacaaggtgatggccgttacccttctcaatggtgtggcgagcaacagtttgatcgcattttattagatgcgccttgttcagcaaccggtgtgattcgtcgccatccagatattaaatggttacgtcgcgatcgcgatatcccggaactcgcgcaattgcagtctgaaattctcgacgccatttggccgcatttaaaaaccggtggaactctggtctatgccacctgttcggtgttaccggaagagaatagcctgcagattaaagcctttttgcaacgtaccgctgatgccgaactttgcgaaacaggaacaccagagcaaccgggtaaacaaaatctacctggtgccgaagagggcgacggcttcttttacgctaagctaatcaaaaagtgatgagataacgggtcgcgactgatgaaaattatcattctgggtgccggccaggttggcggcacactggcggaaaacctggttggcgagaacaacgatattactgttgtcgataccaacggtgagcgtctgcggaccttacaggataaatttgacctgcgggtcgtgcaggggcatggctctcatccacgcgtattgcgggaggcaggtgccgacgacgccgatatgctggttgctgtaaccagttcagatgaaaccaatatggttgcctgccaggtagcctactcacttttcaacacccctaatcgcatcgctcgtatccgctcaccagactacgtgcgcgatgccgataagctatttcattcagatgctgtgccgattgatcatctgatcgcaccagagcagttggttatcgataatatttaccgactgattgagtatcccggcgcattgcaggtggtgaacttcgctgagggtaaagtcagcctggctgtggttaaagcctattatggcggcccgctgattggtaatgcactttcgaccatgcgcgaacatatgccacatatcgatactcgtgtggcagcaattttccgccacgatcgccccattcgtccgcaaggttcgaccattgttgaagctggtgatgaagtgttctttattgccgcttcacagcatatccgcgcggtgatgagtgaattacagcgactggaaaaaccgtataagcggatcatgctggttggtggcggtaatatcggtgcagggctggcgcgtcgtctggaaaaagattacagcgttaaactcatcgaacgtaatcagcagcgcgctgccgaactggcggaaaagttacagaatacgatcgtcttttttggtgatgcgtcggatcaagaactactggccgaagaacatatcgatcaagttgatctgtttattgccgtcaccaacgatgacgaggccaatatcatgtccgccatgcttgccaaacgtatgggtgcgaaaaaggtgatggtattgatccagcgtcgcgcttatgtggatctggttcaggggagcgttatcgatattgcgatttcaccacaacaagcaactatttctgcgttgcttagccatgtgcgaaaagcagatattgttggtgtttcctcattgcgccgcggcgtagcagaagctattgaagccgttgctcacggtgatgaaagcacctcacgcgttgtcggcagagtcattgacgaaatcaagctaccgccaggaacgattattggagcggtggtacgtggaaacgacgtgatgattgccaatgacaatctgcgcattgagcaaggcgatcacgtaattatgttcctcacagataaaaagtttattaccgacgtcgaaagactcttccagccaagccctttcttcttgtaattaataaggcgtctaatgacgccttattatttccctttgattatcaaggattaattaaattcattcctggcaggaaaatggcttaacatttgttagacttatggttgtcggcttcatagggagaataacatgagcattattaaagaatttcgcgaatttgcgatgcgcgggaacgtggtggatttggcggtgggtgtcattatcggtgcggcattcgggaagattgtctcttcactggttgccgatatcatcatgcctcctctgggcttattaattggcgggatcgattttaaacagtttgctgtcacgctacgcgatgcgcagggggatatccctgctgttgtgatgcattacggtgtcttcattcaaaacgtctttgattttctgattgtggcctttgccatctttatggcgattaagctaatcaacaaactgaatcggaaaaaagaagaaccagcagccgcacctgcaccaactaaagaagaagtattactgacagaaattcgtgatttgctgaaagagcagaataaccgctcttaacaagcgcctgaaagcagaagaccagtggtaaaaaagtgatttactttcttgccactggcctcccagttcccccgattgccatgttttccttttcgcatgtaactgcctttccccttcttatttttctctacgcgctgtcggaataagggatcatgtagtaatgcttctatcgcattatcctttatctgccctttagtatgctgatatcgactcataaaaactccagttggttatttaacggcgcgagtgtaatcctgccagtgcaaaaaatcaacaaccactcttaacgccactcgccccttgttcaagagcttcaagaatcgaacaataaacactgctatgagcagtcccacaacaggcatcgttaaggcgttgcaaggaacgctgcatactctgcaactcggctatccgtgcttcgacttcctgcaatctttcctgcacaatgccttttgactcctgacaggtatggtgttcaggatcgatgcggatcgacagcaactcgcggatcgactccagactgaaacctagttgtctggcatggcggataaatttcaatcgctggagatcgctttcggtatataggcgaaacccaccttcagtacgcacttcatgctccatcatctgctgtttttcgtaataacgaatcgtgtcgggtgttacttccgccatttttgccagctcaccaatgcgatacatacatactccactagttatcgttgattttgtccaacaacttgtcagcataatcgccgcgtaaaaaatcggtactcaatccagcttgtcgcagcttcaattccagtaatgacaatcgacggctaacctcttgatattgcggatcatcgtgacggatacctttgagaatatccagaagctgaattgcttctctccgttgctcaagttctggcggtaagcaaccggcattcttcagcaagcgataccccgcacgtaattccggtggcacgtgagaatcatcatccagtatcaatggttcgccgctacctgccaggttatcaaactcacctttcgcttgcgcttctgctatatggcgctctgcccactggtcaagtaaccacataaatactccaggggatgaacaaaaagagtacagctattgtagataagtggggatactacgggtataaaaaaacccgccggggcgggtttttttacgttgcttcagattactctgcagcagcttctgctttctctgaacgatcaaccagctcgatgtaagccatcggcgcgttgtcgcctgcacggaagccacacttcagaatacgagtgtaaccaccggcacggctcgcgaaacgcgggcccagttcgttaaacagttttgccacgatctcgttatcacgagtacgggcgaatgccagacgacgattagcaacgctatcagtcttggcaagagtaatcagcggctcaactacgcggcgcagctctttcgctttaggcagagtcgtcttgatgatttcatgacgaaccagtgaacctgccatattgcggaacatagcctggcgatggctgctgttgcggttcagttgacgaccactcttacgatggcgcatgaccttatccttctcagtaaaaccttaacctgtgatccggttactcgtcagcgatgcttgccggtggccagttttccaggcgcatgcccagagacagtccacgggaagccagcacgtctttaatctcagtaagagattttttaccaaggttaggcgttttaaggagctcaacctcggtacgctgtaccagatcaccgatatagtggatagcttctgctttaaggcagttagcagagcggacagtcaattccagatcgtcaacagggcgcagcaggatcggatcgaactctggtttctcttctttcacttcaggctgacgtacatcacgtaagtcaacgaaagcttccagttgttcagccagaatggttgccgcacgacgaatcgcctcttcaggatcgattgtgccgttggtttccatttcgatgaccagcttgtccaggtcggtacgctgttctacacgcgctgcttcaacattgtaggcaatacgctccacagggctgtagcatgcgtcgaccagcagacggccgattgggcgctcatcttcttccgaatgaattcgggtagaagccggcacataaccacgaccgcgctgaactttgatacgcatgctaatagacgcgttctcatcggtcaggtggcagatcacgtgctgcggcttgacgatttcgacatcaccgtcgtgggtgatatcggctgcagtcacagggccaatgccagatttattcaaggtaagaataacttcatctttgccctgaactctcaccgccagccctttcaggttgagcaggatttccaggatatcttcctgaacgccttctttggtgctgtactcatgtagtacaccatcaatctcaacctcggtcaccgcgcaacccggcatcgatgagagcagaatacggcgcagtgcgttacccagagtatggccaaagccacgctctaaaggctcaagggtcaccttggcgtgcgtcgaactcacttgctcgatatcaaccaggcgcggttttagaaactctgtcacagaaccctgcattgtgtcctctctttggtactaagctttacttggagtaaagctcgacgatcaggtgttcgttaatgtccgcagacagatcagaacgctccggcttacgcttaaacgtaccttccatcttgccagcatcaacttccagccaggttggcttttcacgctgctcagccagctccagagcggctttcacgcgagactgcttcttcgctttctcacgaatgcttacaacgtcattcggactaacctgataagaagcgatgttaacaacacgaccgtttaccataattgctttatggctaaccagctgacgtgcttctgcacgagtggcaccgaagcccatacggtatacaacgttgtccagacgaccttccagcagagccaacaggttttcaccggtgttgcctttcagacgtgctgcttctttgtagtagttacggaactgacgctccagcacaccatagatacggcgaactttttgcttttcacgcaactgcacaccatagtcagacagacgcggtttacgcgcaccgtgctggccaggagcttgttcaattttacacttggtatcgatcgcgcgaacgccagacttaaggaataagtcggtgccctcacgacggctcagcttgagcttaggacccaaatatcttgccattttctttctccaacaaacctggaaaacgaggcgttatacgcgacgttttttcggcggacgacaaccgttatgagggatcggagtcacatcagtaatgttagtgatgcggaaacctgcggcgttcagagcacgaatagtagattcgcggcctggacccggacctttaaccataacttccagattcttgatgccgtattctttcacggcgtcagcgcaacgctctgctgcaacctgagctgcaaacggagtggatttgcgagaaccacggaaaccggaaccaccggctgttgcccaacccaacgcgttaccctgacgatcagtgatagtcacgatggtgttgttgaaagaagcatggatatgagccacgccgtcagagacttgttttcttacacgtttacgtgcacgaattggtgcctttgccattattcaatcaccccgattatttcttgatcggtttgcgcggacccttacgggtacgtgcgttggtcttggtacgctgaccgcgaaccgggagaccacgacgatgacgcaaaccgcgatagcaaccaagatccatcaggcgcttgatgctcatgctgatttcacggcgcagatcaccttcaacgacaaatttggcaacttcgtcacgcagcgtgtcgatttgtccttcagacagctcactgatcttaacatcttcagcgatacccgctgcagccaggatggctttagaacgggtcttgccgacgccataaatcgaagttaatgcgattacggcatgcttatgatcaggaatgttaatgcctgctatacgggccactatgcactcctactatttaatatgtacgttccatgctgaaaagcccgttttcaggatactcaaatggaaacgcacagacatacaaaagattggctggctaatctagccagctcaacccaactttgcaagaaaaatatgcgaaaaaatcagccttggcgctgtttatgcttcggctcggcactgcaaatcacacggatgacaccatcacgcttaacgattttgcagttacggcataatttcttgacggaagcacgaactttcatttttactctccgtaacttctcgggcgaccaattatcggccgtagcctttcaggttcgccttcttcaatgcagactcatactgactggacatcatcagagtttgcacttgagccataaagtccataatcacgacaacaacgataagcagtgaggtcccaccgaagtagaacggtactttcattgcatcacgcatgaactccgggatcaggcagataaaggtaatatacagcgcaccaaccagggtcaggcgggtcattactttatcgatatacttcgccgtttgctctcccggacgaattcctggtacaaatgcaccggacttcttcaggttatctgctgtttcacgcgggttgaaaaccaacgccgtgtagaagaaacagaagaagatgattgcagacgcatagagtaacacataaagcggttgcccaggctgcaaatacagcgaaattgttgtcagccagttccaaccagtaccgcccccgaaccatgacgcgatggtcgccgggaacagaataatactggaagcgaagattgccgggattacccccgccatattcactttcagcggtaaatgtgtgctctgtgcagcatagacacgacgaccttgctgacgtttcgcgtagtttaccacaatgcggcgttgaccacgctcaacaaatacaacaaagaacgtcactgcaaatactaatactgcaaccaacagcaacacgaggaagtgcaggtcgccttgacgcgcttgctcgatagtatgggcaatggctggcgggagtcccgcgacaataccggcgaagataatgattgaaataccgttgccgatacctcgttcagtaatctgttcgcccaaccacatcaggaacatggttcctgtgaccagacttacaacagcggtgaagtagaatgcaaagcccgggttaatcaccaggccttgcataccaggcatattcggcagaccggtagcaataccgatcgactggaatattgccagcaccagagtaccgtagcgggtgtactggctgatcttacgacgaccagactccccttctttcttaatttctgccaacgttgggtgaaccaccgtcagcagctggataatgatcgacgccgaaatatacggcatgatccccagagcaaagatagaagcacggctgagagcaccaccagagaacatgttaaacatctcaatgatggtgcctcgctgttgctcaagcagtttggcaagtacagcggcatcaataccagggatcggaataaaagagccaatacggaacacaatcagcgcaccgataacaaacagcagtctgcgtttcagctcgcctaagccacctttggcactttgaaaatctaatcccggttgtttagccatctgctacttattcctcgattttaccgccagcagcttcgatagcagcacgagcgcctttagtaacacgcaggccacgaacagttaccggagtcgttacttcgccagccaggatcactttcgcgaactcgatctggataccgataatgttagccgctttcagcgtgttcaggtctactacaccgccttctactttagccaggtcagacagacgaatttcggctgtaatcgctgctttacgagaagtgaagccgaatttcggcagacgacggtacagaggcatctgaccaccctcgaaaccgcgacgtacgccaccgccagaacgagacttctgacctttgtgaccacgaccaccggttttaccgaggccagaaccgataccacgacccaggcgtttacccgcctttttggagccttcggccggagacagagtatttaaacgcatctcttactcctcaactttaaccatgaaggaaaccgcgttgatcataccgcgaatagcaggagtatcctcgcgctctacggtgtgaccaatacgacgcagacccaggccaagcagcgttgccttgtgtttcggcagacgaccgattgcactgcgggtttgagtaattttaatagtctttgccatggtttatttccccagaatttcttcaacggatttaccacgcttggcagcgaccatttctggagaattcatattttccaggccatcaatagttgcacgaaccacgttgatcgggttggtggaaccataggctttagccagaacgttatgaaccccagcgacttccagaacggcgcgcattgcaccaccggcgatgataccggtaccttcggaagccggctgcatgaatacgcgagaacccgtgtgaacacctttaacagggtgttgcagagtgccgttattcagcgcgacgttaatcatattgcgacgggctttttccatcgctttctggatcgctgctggaacttcacgcgctttaccgtaaccaaaaccaacgcgaccgttaccatcgccaactacagtcagagctgtgaaggagaaaatacgaccacctttaacggttttagatacgcggtttaccgcgatcagcttttcctgcagttcgccagcttgtttttcgatgtgagccatcttacacctctaccttagaactgaaggccagcttcacgggcagcatctgccagtgcctggacacgaccatgatattggaacccggaacggtcaaaggatacatctttgatgcctttttccagagcgcgttcagcgacagctttacccacagctgcagccgcgtctttgttaccggtgtacttcagttgttcagcgatagctttttctacagtagaagcagctaccagaacttcagaaccgttcggtgcaattacctgtgcgtaaatgtgacgcggggtacgatgtaccaccaggcgagttgcgcccagctcctggagcttgcggcgtgcgcgggtcgcacgacggatacgagcagatttcttatccatagtgttaccttacttcttcttagcctctttggtacgcacgacttcgtcggcgtaacgaacacccttgcctttataaggctcaggacgacggtaggcgcgcagatccgctgcaacctggccgatcacctgcttatcagcgcctttcagcacgatttcagtctgagtcggacattcagcagtgatacccgcaggcagctgatggtcaacaggatgagagaaacccagagacaggttaatcacattgcctttaaccgctgcacggtaacctacaccaaccagctgcagcttcttagtgaagccttcggtaacaccgataaccattgagttcagcagggcacgcgcggtaccagcctgtgcccaaccgtctgcgtaaccatcacgcggaccgaaggtcagggtattatctgcatgtttaacttcaacagcatcgttgagagtacgagtcagctcgccgtttttacctttgatcgtaataacctgaccgttgatttttacgtcaacgccggcaggaacaacgaccggtgctttagcaacacgagacattttttcctccgattaggctacgtagcagataatttcgccaccaagaccagcctggcgcgctgcacgatcagtcataacacctttagaggtagaaacaactgcgatacccagacccgccataactttcggcagctcatctttacgtttatagatgcgcagacctgggcggctgacacgctgaatgctttctacaacagctttgccctggaaatacttcagagtaagttccagttcaggcttggtgtcgccttcaactttaaaatcttcaataaaaccttcttccttcagcacgttggcgattgccactttcagcttggaggaaggcatggtgaccgcagctttgttcgcggcctgaccgttacggatacgggtcagcatatccgcgatcggatcttgcatgctcatctgtctttactcccgtgattcaattggtgacaattaccagctagcctttttcagacccgggatttcaccgcgcatagcggcttcacggaccttaatacggctcaacccgaacttccgcaggaaaccatgcggacgacctgtttgacggcagcggttacgctgacgagacgggctggaatcacgcggcagagtctgcagcttgagaacagcgttccaacgatcttcgtcggaagcgttcacatcagagatgatcgctttcagttcagcgcgtttcgcgaagtatttatcagctaaagctacgcgttttacttcgcgtgctttcattgattgcttagccatttagtaaccctaccttacttgcggaacgggaagtcaaaggcagccagcagagcgcggccttcttcgtcagatttcgcagtagtggtaatggtaatatccaaaccacgaacgcggtcgactttatcgtagtcgatttctgggaagatgatctgctcacggacacccatgctgtagttaccacgaccgtcgaaagacttagcggacaggccacggaagtcacggatacgaggtacagcaatagtgatcaggcgctcaaagaactcccacatgcgttcgccacgcagagttactttacagccgatcggatagccctgacggattttgaagcctgcaacagatttgcgtgctttggtgatcagcggtttttgaccggagattgctgccaggtctgctgctgcgttatccagcagttttttgtcagcgatcgcttcaccaacacccatgttcagggtgatcttctcgacccgagggacttgcatgacagaattgtagttaaactcagtcatgagttttttaactacttcgtctttgtagtaatcatgcagtttcgccatcgtactactccaaattacttgatagtttcgctgttagacttgaagaaacggacttttttaccgtcttcgaatctaaagcctacacggtcagccttgccggttgccgcattgaagattgctacgttggaaacctgaatagcggcttctttttcaacgatgccacccggttggttcagggccggaaccggcttctgatgtttcttaaccaggttgataccttcaacaatgaccttgccggaagacaggacattcttaactttaccgcgtttacctttatctttaccggttaacacgataacttcgtcatcacgacggattttcgctgccatgattcgctccttagagtacttctggtgccagagagataattttcatgaacttctcactacgaagctcacgagttaccggcccaaaaatacgcgtaccgataggctgctcgctgttgttgttcagaagaacacaagcattaccatcgaagcgaatgacagaaccgtccgggcgacgaacacccttcttggtgcgcaccactaccgccttcagcacatcaccttttttgaccttaccacgcggaattgcttctttgatggtgatcttgatgatgtcgcctacgcctgcgtagcgacggtgcgagccacccagaaccttgatacacattacgcgacgtgcaccggagttgtcggcgacgttcagcatagtctgttcttggatcattttagtgctccgctaatgtcaactactactgagacccgaaaatcaggtcgttaaaaatccccatatcgagggcgcggcattataacaccgcttcaaggatatgggtagaaaaaataaacggctcatttctgagccgtttattcgtattgagagagtgtactgtattacagaaccgctttctctacaacgcgaaccagcgtccaggatttagtcttggacagcggacggcattcgcggatttcaaccacgtcaccgataccgcattcgttgttctcgtcatgtacgtgcagtttggtcgtacgcttgatgaatttaccgtagatcgggtgtttcacaaaacgttcgatagcaacaacaatggatttctccattttgtcgctaacaacgcgaccttgcagagtacggattttatcggtcattacgcacccgccttctcgttcagtaaagtcttaacgcgtgcgacatcgcgacgcacttgcttcaacaggtgagactgttgcagctggccacttgcagcctgcatacgcaggttgaactgctcacgcagcaggttcagcagctcggtgttcagctcttcaacgctcttctcacgcagctcttttgctttcattacatcaccgtcttagttacaaaggtggttttaatcggcagtttcgctgctgccagcttgaatgcttcacgggccagctcttccggaacaccgtccatttcatacaggactttacccggctgaatcaaggcaacccaatactccacgttacctttacctttacccatacgcactgccagcggcttttcagtgatcggtttgtccgggaacacacggatccagatcttaccttgacgcttaactgcacgggtcatagcacgacgtgctgcttcgatctgacgggcagtcagacgaccacggccaacagctttcagaccgaagctgccgaagctaacatccgtaccctgcgccagaccgcggttacggcctttgtgcattttacggaattttgtacgctttggttgtaacatcagcgacgctccttatttacggcctttacgctgctgctttttaggctgagcagccggtttttccggttgttcaacagcagccataccacccaggatctcgcctttgaagatccacactttaacgccgattacaccgtaagtggtgtgcgcttcagaggtgttgtagtcgatgtcagcacgcagagtgtgcagcggtacgcgaccttcgcggtaccattcggtacgtgcgatttccgcgccgcccagacggccgctaacttcaactttaatacctttagcgcccagacgcattgcgttctgtacagcacgcttcatagcacgacggaacataacgcgacgttccagctgagaagtgatgctgtcagcaaccagttttgcgtccagttcaggcttacgaacttcggcgatgttgatctgtgcaggaacgccagcgatgtccgctacgaccttacgcagtttttctacgtcttcaccttttttaccgataacgatacccgggcgagcagtgtgaatggttacacggatgctcttagccggacgctcgataacgatacgagatacggacgctttagccagttccttagtcaggtactgacgtactttaaaatcgctgtccaggttgtcagcgaattctttggtgttcgcaaaccaggtagagttccatggttttacaatacccaggcgaataccattaggatgtactttctgacccattgctagtctccagagtctcagcgatcggacacaaccacagtgatgtggctggtgcgcttcaggatgcgatctgcacgaccttttgcacgcggcataatgcgcttcatgctcgggccttcgtctacgaaaattttcgtaactttcagatcgtcaatgtcagcgccatcgttgtgttcagcgttagcaatggcagattccagaactttcttgaccagtacagccgctttcttgttggtgtaggtcaaaatatccagagcctgcgacactttcttaccgcgaatcaggtcagcaacaaggcgaaccttctgagcagaagaacgagcatggcgatgtttagcgatagtttccatctcttcctcctaccttatttcttcttcgcttttttatcagcagcgtggccgcgataagtacgagtcggtgcgaattcacccagtttgtgaccaaccatttcgtcggttacaaataccggaacgtgctgacgaccattatggacagcgatggtcaaaccgatcatgttaggaaagatcgttgaacgacgggaccaagtgcgcaggggcttcttgtctccgctttccaccgctttctctaccttcttcagcaagtgcaggtcaataaaaggacctttcttgagagaacgtggcatggcttatcctctaaaattatttgctacggcgacgtacgatgaatttatcagtacgcttgttgctgcgggtcttcttacctttggtctgaacgccccacggagttaccgggtgcttaccaaagttacgaccttcaccaccaccatgtgggtggtctaccgggttcatcgcggtaccgcgaacggtcggacgaacaccacgccagcgtgcagcacctgctttacccagaacgcgcagcatatgctcagcattgccaacttcgcccagagttgcacggcagtctgcttctactttacgcatttcaccagaacgcagacgcagggtgacataagcaccatcacgagcaacgatctgaacgtaagtaccagcggaacgtgccagctgaccgcctttacctggtttcatttctacgttatgaacagtagaaccaaccgggatgttgcgcatcggcagggtgttacctggtttgattgcagcatcaacgccagactgaatctggtcgccagctttcaggcctttaggggccaggatgtaacggcgttcaccgtctttgtacagaaccagcgcgatgttcgcggaacggttcggatcgtactcaagacgttcaacaactgccgggataccgtctttgttgcgtttgaagtcaacaatacggtaagcctgcttgtggccaccaccgatatgacgagtggtgatacggccattgttgttacgaccaccggatttgctgtttttttccagcaacggagcaaaaggtttgcccttgtgcagctcagggttaaccactttaactacgtggcgacgacccggagatgtcggtttacatttaacaactgccattgtattactcctccgacttactcagcgccgccaacgaagtccagattctggccttctttcagggtgacgtaagcttttttccagtcgctacgacgaccgatacgctgtccgtgacgtttaactttccctttaactaccagggtgttaacgacttcgacttcgacttcaaacagtttctgcacagcagctttgatttctgctttggtcgcgtctttagcaactttgagtacgatggtgttggatttttccatcgcagtagacgctttttcagaaacgtgcggtgcacgcagcaccttcagcagacgttcttcacgaatcatgccagcatctcctcaacttgcttaacagcatcagcagtcattacgactttgtcgaaggcgatcaggctaaccgggtcgataccagttgcatcgcgtacgtcaaccttgtgcaggttgcgcgcagccaggaacaggttttcgtccagctcaccggtgatgatcagcacatcttccagagccatgtctttcagtttctgtgccagcagcttagttttcggcgcttctacagagaacttctcgacaacgatcagacgatcctgacgtaccagttcggacaggatgcttttcagcgcgccgcggtacatcttcttgttaactttttgactgtggtcctgcggacgagcagcaaaggtcacgccaccagaacgccagatcgggctcttgatagaaccagaacgcgcacggccggtgcctttctggcgccacggttttttaccggaaccagttacttcagcacgagtcttctgagcacgagtaccctgacgagcaccagctgcataagcaacaacaacctggtgaaccagcgcttcgttgaaatcacgaccgaaggtagtttcggaaacagtcagcgcgctctgcgcgtctttcaatactaattccattgctatctccttacgccttcacagctggtttaacgatcaggtcgctaccggttgcacccgggacagcacctttaaccagcagcaggttgcgctcagcgtcaacgcgtactacgtcaaggctctgaacggttacacgttcgttacccatctgacctgccattttcttgcctttgaacactttgcccggagtctggttctgaccgatagaacccggaacgcggtgagacaaggagttaccgtgagtagcgtcctgggtacggaagttccagcgcttaacggtacctgcgaaacctttacctttagaggtgccagttacgtcaacttttttaacgtcagcaaacagttcaacgctaatgctctgacctacagtgaactcttcgccttcagccaggcggaattcccacagaccacggccagcttctacgccagctttagcgaagtggccagcttcaggcttggtcacacggttagcttttttagcaccggtggtcacctgaatagcacggtagccatcgttagccaggtctttaacctgagtaacgcggtttgcttcaacttcgattacggttactgggatagaaacgccgtcttctgtgaagatacgggtcatacccacttttttaccgactaaaccaatcattgtttcaacctctcaatcgctcaatgacctgattaacccaggctgatctgcacgtctacaccggcagccagatccagacgcatcagagcatcaacggttttctcggttggctcaacgatgtcaaccagacgcaagtgagtacggatttcgtactgatcgcgcgcgtctttgttgacgtgcggggagatcagaacagtgaagcgctctttgcgtgtcggcagcgggatcggaccacggacctgcgcaccagtgcgcttggcagtctcgacgatttccgcggttgcttgatcgatcagacgatgatcaaacgctttcaggcggatacggattctttggttctgcatgagaccagagctccaattattttataaacgaaaatgattactcctcagacccattacgattgatgggagagtgtaaccgttcttacgtagctccccgattgggagcattgttaggtagccaaattcggctaactgaggttcagattgaacctgctgtcaactacgacaagcccgcgcattatacatacttaaccaccgaacgcaagcgtattgctagtaaagtaaacagccttcgggttatctctcaagttcgttcagtgcatttttgacacgctctcttaaaccggctttctcttcgctttcttccacagtattttcttcgtcttcagaagaagagggggcattctcaaccgcgacgcctgggtcatcttcctcctcgacggattcgacgacggggagtggctgttttttgaagaaatagtgttgtgttgattgtttaaaagcgggcgtttcagcctctacagtgacttcggcttttactatccaaagcacccatagctgcctggcatacccaccaaccagcaccattcctgcaaaccacaggcaaatcagtaataaacaaattacatatattatggtgctgtgtttttgtcgggagaagataccagggtgacctgtttctttctgctcacgcgcggcgatatagaattcaaacatgtcatttccccttcactgttgtttccggggaaatatttgcttcatcccgatataagtaggcactctcccctgccacctgccagagatgtactaacgttgaaaagccaacaacaccgtcagttttcaagtggtggcttttttgaaattgctttattttttctaccaacaagggacgccactccgccgaaggttctgtcgaaatatgcaatgcgcggtttaacatcgtttccagccagagaatctcttcctcgctgctatcacgcgtaatggtactctccccttccggcgacattttccacaacagaagataatcacccgtccataccgactcaaaccatttatgtgtcagcgtccacgtttgctgacctacgaggacatcaacgctagcctcaccgacgcgaacgaccacaacaggcaattttttgtccccgactttaagcgatgcgatccagggcaaattctgatctaccaatgtttgtaaagaagcattcccacttttacatgccagccccgctcttactgcctgatcgcaccaggccgaatcagctgggacctcgtacccccatacgccgtataacacgcttagcgcctcactatcgcgcatcaccacatgagcaatatccttagtcatatcttgtttaactactggcgttacgggtatcagccacgcaggaacgggtaacgtagctgtaaaagaggacagcagtagccaaccacaggtaagagcgataatggttccactcatcaccacggcaagctgcattttccgggggcggttatcacccaatatgcggtaaatcattcgccattgttttgctgtgaaaacgctggtctgctcggcttgctgtaataagcgaattgtttcgccggcaagcgccagctttctgcgatcgccccgacataataaagctatccgtttcagaactctggcggttaaaaggagatcgggttggtcaatattctgaccttcaaggatgcttgccttaagttcgtgctccgtcagacgtcctatcgagacaagttcaatgccctgttttttaaaatcacgttcgacttttcgatcgggtctgccgatcagcaaaaattgaccgtcaggaataagagatattgcgcgttggagatcatcaagtatgcggcggtgattcaggtgagcattttcaataataataagagggcagcgactatcagttcgatgaagcgcatgcagtaattgccccgccatctcatctcgcgtccaggcgctgtcacggcagccctgttcagccgcgttatcgtcggtaacgatccatgcggccttaccttgccaggaaacaacgaggcttaaagtaatcacacggcgatgtttatctttttgcagttgctgcgccagccaggtttttccacttccagcctcacccaacaaatagcatagacgccaggtttgacgtttctcacacaaccaggaaagaataacttctcttctcgtagacatagaacttcctgttttaattattgattatccttaatcataaaaataatgtatgtatttattaattaaatacatattactaatataaataaattttgcttgattcatgcaagcggcattaatactatttatactaacgtcaatatacaacccacccaatctattttattagaacatacatcgtgcccacactacgtttccccttccatctggcgaatcataataaagatgctgccatcaatatattgattatatttataagcatagggtcgattatttttaatgtgaattatttccatacaactatagttaaaaatggacagatcattaatcaaccaacaaacgcatttcagtctgatttcagccttgccgctttatggcgtaacgaaaatcatgctggggtaaaagatgcaaatcccgtggcagttaatcaggaaacacctaagctctctatagcgcttaatggcattgtactcacatcgaatgatgagacttcttttgtcttaattaatgaggggagcgaacaaaagcgatactccctcaacgaagcccttgagtcagcgccgggaacgtttattagaaaaataaataaaaccagcgttgtgtttgaaactcacgggcattacgaaaaagtaactctccatccagggctacctgacatcatcaagcagcctgattcagaaagtcaaaatgtactcgctgattatattatcgccacgcctatacgtgatggagaacagatatacgggcttcgattgaaccctcgtaagggcctcaatgcatttaccaccagcttgctacaaccaggggatatcgccctcaggatcaataatctttcgctgacccaccctgatgaggtttcacaggcattaagtttactgctaactcaacaaagtgctcagtttacaattcgtcgcaacggcgtaccccgcttgataaatgtttccgtcggggaacttacaggaatgaatggactgcgtcatgaaaggactcaataaaatcacctgctgcttgctggcagcactactcatgccttgtgcaggacacgctgagaacgaacaatacggcgcgaacttcaataacgccgatatccgccagttcgtggaaatagtgggtcagcatcttggcaaaacgatcctgatcgacccttcggtacagggaaccatttccgtacgcagtaatgatacgtttagccaacaggagtactaccagttctttttaagtattcttgatctttacggttattccgtgatcacgctggacaatggttttctgaaagtggttcgctcagctaatgtaaaaacatcgccagggatgattgctgacagttctcgtccaggcgtaggtgatgagttggtcacccgaattgtaccgcttgagaacgttcctgctcgtgacctggcccccctgctccgccagatgatggatgcgggtagcgtcggtaatgttgtgcattatgaaccctccaacgttcttattctgaccggtcgtgcctccaccattaataaactgattgaagtcataaagcgcgttgatgtcatcggcacagagaagcagcaaattattcatctggaatatgcgtcagcggaagatctcgccgagattcttaatcaattaatcagcgaaagccacggtaaaagccagatgccagccctcctctccgcgaagattgtggcggataagcgaaccaactctcttatcatcagtggaccggaaaaagcacgccagcgcatcacttcattactgaaaagccttgatgtcgaagagagcgaggaaggaaatacccgggtttattacctgaaatatgctaaagccacgaatctggtggaagtgctaaccggtgtttccgaaaagctgaaagatgaaaaagggaatgcgcgtaagccctcctcttctggcgcgatggataacgtcgccattaccgccgatgaacagactaactctctggtcattaccgctgaccagtccgtccaggaaaaactcgccacggtaattgcgcgtctggacattcgccgtgcacaggtgctggttgaggcaatcatcgttgaagttcaggatggaaatggactaaacctcggcgtgcaatgggcgaataaaaacgttggcgcacagcaatttaccaataccggattaccgatttttaacgctgcgcaaggtgtggctgattataaaaagaatggtgggatcaccagcgcgaatcctgcctgggatatgtttagcgcctacaatggcatggccgcaggcttcttcaatggcgactggggagtactgcttaccgcgctggccagtaacaataaaaatgacatcctcgccaccccaagcatcgtaacgctggataataaactcgcgtccttcaacgtggggcaggatgtgccggtgctatccgggtcacagaccacttcaggggataacgtctttaataccgtcgaacgcaaaacggtggggacaaaactcaaagttactccgcaggtcaatgaaggcgacgcggtgttgctcgaaatagagcaggaagtctccagcgttgactcttcctctaactcgacgctcggcccgacgtttaatacccgtactattcaaaacgccgtgctggtcaaaaccggtgaaacggtggtcctgggcggattgctggatgatttttctaaagagcaagtgtcaaaggttcctctgcttggcgatattcctttagtggggcaactcttccgctatacctccaccgagcgcgctaaacgcaacctgatggtatttatccgtccgacgattatccgtgacgatgatgtttatcgctcactgtcaaaagagaaatacacccgttaccgtcaggagcaacaacagcggatcgacgggaaatcaaaagcgctggttggctcggaagatttgccggtgctggatgaaaacacgttcaacagtcacgcccctgcgccatcgtcacggtgaggcattcatatgagaattcactcaccgtaccccgccagttgggcgctggcacaacgaattggttatctctattcagagggcgagattatttatctcgccgatacgccattcgagcggttactcgatattcaacgtcaggttggccagtgccagaccatgaccagcttgtcacaggctgattttgaagctcggctggaagcggtattccatcagaataccggtgagtcgcaacagattgcgcaggatatcgatcaatccgtcgatcttctctcgctttcggaagagatgcccgcaaatgaagatctcctgaatgaagattcagcggcaccggttatccgcttgatcaatgcgattttgagtgaggccatcaaagaaaccgcctctgatatccacattgaaacctatgaaaaaacaatgtcgatccgttttcgcatcgacggcgttttgcggacaattttacagccaaacaaaaaactggcggcactgcttatctcccgaattaaggtcatggctcgtcttgatatcgccgaaaaacgtattccacaggatggaagaattagtttgcgtatcgggcgacgtaacatagatgtccgcgtatccacactgccgtccatctatggtgaacgcgccgtactccgcctgctggataaaaacagcctccagctttcattgaacaacctggggatgacggcagcggataagcaggatttagaaaatctcattcagcttccgcacggtattatcctggtgacagggccgacaggctccggtaaaagcaccacgctctacgccatcctttcggcgctgaatactcccggccgcaatattctgacggtagaagatcccgtggaatatgagctggaaggcattgggcaaacgcaggtgaatacccgtgtggatatgtctttcgctcgcggcctgcgcgccatacttcgccaggacccggatgtcgtcatggtgggggaaattcgtgatacagaaaccgcgcagattgcggttcaggcctcgctcaccggccatctggtactctcaacactccacactaacagtgcatcaggcgcagtgacccggctccgcgacatgggcgtcgaatcattcctgctttcgtcttccctggcagggattatcgcgcaacgtctggttcgtcgcctgtgtccgcaatgccgacaattcacgcccgtatcaccccaacaagcgcagatgtttaaatatcatcagctcgcggtgacaacaattggcactcccgtaggctgccctcattgccatcaatccggctatcaggggcgcatggcgatccacgaaatgatggtggtgacgccggaattacgggccgctattcatgaaaatgtggatgaacaagcactggagcgactagtccggcaacaacacaaggccttaatcaaaaatggcctgcaaaaagtgataagcggtgacacctcctgggatgaggttatgcgcgtcgccagtgccacgctggagagcgaagcatgaattatcgctatcgcgccatgacccaggatggtcaaaaattgcaagggatcattgatgctaacgatgaacgtcaggcacgactgcggctgcgtgaagaagggcttttcctgctggatattcgcccccaaaaaagttcgggagtaaaaacacgtcgcccgaggatcagccatagtgaactgacgcttttcacccggcagttggcaaccttaagcgcagcggcattacccctggaagagagccttgccgtaatcggtcaacaaagcagtaataaacgactgggtgacgtgttaaatcaggtacgcagcgccatccttgaagggcatcccctttccgatgcattacagcattttcccacgcttttcgattcgctctatcgtaccctggtaaaagcgggcgaaaagagcgggctgctggccccggtgttggaaaagctggctgattacaatgaaaaccggcagaaaatccgcagcaagctcattcagtcactgatctacccctgtatgctcactacggtggcgattggggtcgtgattattctcctcactgctgtcgtgcccaaaattaccgaacagttcgtgcatatgaagcagcaactgccgctgagtacacgcattcttttaggtctgagcgacacgttgcaacgtaccggcccgacattattagcgacagtgtttattgtcgctgtaggtttctggctctggttaaaacgcggcaataaccgccaccgttttcatgccatgttgctgcgcgttgcgctcatcggcccgctgatttgcgccattaacagcgcacgctatctccgcactttaagtattttgcaatccagcggcgtccctctgctggatgggatgaatttgtccaccgaaagcctcaacaacctcgaaattcgccagcgtctggcaaatgcggcagagaacgttcgccagggtaacagcattcatctttcgctggaacaaaccgcaattttcccgccgatgatgctctacatggtggcctctggcgaaaaaagcgggcagctcggcacattaatggtcagagccgcagataaccaggagacactccaacaaaatcggatcgccttaacgctctccatcttcgagccagcactcattattacgatggcactgatcgtcctgtttattgtcgtgtcggtactccaacctcttcttcaacttaactcaatgattaattaaggaaagcatatgcgcgcaacggataagcaacgcggttttacattactggaaattatggtggtgatcgtcattatcggcgtacttgccagcctggtggttcctaacctaatgggcaataaagaaaaggcggataagcaaaaagccgtcagcgatattgtggcgctggaaaacgcccttgatatgtacaaactcgacaatcatcactatccaaccacaaatcaggggcttgaatccttagtagaagcgccgacactgccaccgctggccgcaaactataacaaggaaggttatatcaagcgtctgcctgccgatccctggggcaatgattatgtcctcgttaatcctggtgaacatggtgcatacgatctgctttcagcagggcccgatggtgaaatgggaaccgaggacgacatcaccaactggggtttgagcaagaagaaaaagtaagtcagcgatgaatcagcaacgcgggtttaccctgctggagatgatgctggtgctggcgctggtcgctatcacggcaagcgtggtgctcttcacatatggccgggaggatgtcgccagcactcgtgcgcgcgaaacagcggcgcggtttaccgctgcacttgaattagccatcgaccgcgccacgctcagtggtcagcctgtcggtatccatttctctgattcagcatggcgcattatggtaccgggcaaaacaccatcagcctggcgctgggttccattacaagaagatgccgcagacgagagccaaaatgactgggatgaagaactctcaattcatcttcagccatttaaacctgatgacagcaaccagccacaggttgtgattctggccgacggacaaatcacgcccttctctttgttgatggctaacgccgggaccggtgagccgctcctgacgttagtctgttcaggctcatggcccctggatcaaacgctcgccagagatacccgcccatgaacaaacaatcagggatgacactgcttgaagtcttactggcgatgagtattttcaccgctgttgctctgactttaatgagcagtatgcaagggcaacgaaatgccatcgagcgaatgcgtaacgagacgctggcattgtggatagcggataaccagcttcagtcacaagattcattcggcgaggaaaacacgtccagttctggcaaagagttaataaatggcgaagagtggaactggcgcagcgatatccactcaagcaaagacggcacgcttctggaacgcaccataacggtgacattacccagcggtcagacaacctcgcttacgcgttatcaaagcatcgataataaatccgggcaggcacaagatgattaatcgccagcagggtttcacattgctggaggtcatggcggcgctggcgattttctcaatgcttagcgtgctggcgtttatgattttttcgcaagcttccgagttgcatcaacgctcacagaaagaaatccagcagttcaatcagctacagcgcaccatcaccattcttgataacgatctcctgcaactggtcgcccggaggaatcggagtacggacaaaatcatggtgttgggtgaagaagctatttttaccacgcaaagtcgcgatccgctggctcctctcagtgaagcacaaaccttactcactgttcactggtatctgcgaaatcatacgctctaccgtgctgttcgtacttctgtggatggcaggaaggatcaacccgcccaggcgatgctggaacatgtcgagagctttcttctggaaagtaacagcggggaaagccaggaacttcctctctcagtcacgttacatctgcagactcagcaatatggggggttacagcgccgttttgcattacctgagcagttagcgagagaagagtcgccagctcagacgcaggccgggaataataaccatgaataatgaacaacgcggcgtcgcgctgctcattgtactcatgttactggcgctcatggctgctctggcagcagacatgacgctcagttttcacagccagcttcagcgaacccgccaggtaaaccatcatctgcaacggcaatatgatattgaactggcggagaaacttgcgcttgccagcctcacccaggacgttaaagataacgacagacagaccacgttgcagcagtactgggcacagccacaacagttgcagctggaagatggcaatacagtgaagtggcagttacgcgatgcccagcactgttttaatctcaatgcgttagcaaaaatctctgacgacccgctggcttcccctgatttccccgcccaggtattcagtgcgctgctgattaacgccggtatcgatcgcggaaacaccgatgagatcgtgcaatcaatcgctgactatattgatgtcgatgactcaccacgctttcacggcgcagaagatagcttttaccaaagccagacgccgccccggcatagtgccaatcagatgctttttctgactggcgaattacgtcagataaaaggcataaccgaaaacatctatcagcggcttatcccgtatgtctgcgttctcccgaccacggaacttagcatcaatcttaatatgctaacggagaacgatattccgctcttcagagcgttattcctcaataacatcacggatgctgacgctcgggtcttattgcaaaaaaggccgagggaaggctggctaaccacggatgcatttctttactgggcgcagcaggatttctccggtgtgaagccactggttgctcaggtgaaaaggcatctctttccctatagccgctattttacgctgagtacggaaagtatcagcgacgaacaatcccagggatggcaaagccatatttttttcaaccgtaaacagcagagcgcccaaatctatcggcgtacgctgcaactctactaatcataaggatcgtgatgcctgaatcgttgatggtcatacgttcttcctcgacgctgcgtaagcattgggaatggatgacgttctccgcagatagcgtatcttcggtacatacgctcacggacgatcttccgctggagtcgctggccgatcagcccggtgccggaaatgttcatcttttgatcccaccagagggccttttatatcgttccctcacgctgcccaacgccaaatacaaactcaccgcacaaacattacaatggctggcagaggagacgttacccgacaacacccaggactggcactggacggttgtcgataaacaaaacgaaagtgtcgaggtgataggcattcagtcggagaaactcagtcgctatcttgagcgtttacatactgccggactcaacgtgacgcgggttttgccagatggctgctatcttccctgggaagtagatagctggactctggttaaccagcaaacaagctggctcattcgcagtgccgcacatgccttcaacgaactggatgaacactggttacagcatcttgctgcccagtttccgcctgagaatatgctttgttatggtgtagtacctcacggcgttgcagcggccaatccacttatccagcatcctgaaataccatcactgagtttgtattctgccgatattgcattccagcgctatgacatgctgcatggtatttttcgtaaacagaaaactgtaagcaaatcgggaaaatggctcgcccgcctggcagtaagctgtctcgttctcgccattctttcttttgttggcagccggagcatcgcgctctggcatacgcttaagattgaagatcaacttcagcaacaacagcaagaaacctggcaacgttatttcccgcagatcaaacgcacccacaattttcgtttttactttaagcagcaactcgctcagcaatatcctgaagctgtgccgttgctctatcatttacaaacacttctgctggaacaccctgaactgcagttaatggaggcgaactatagccagaagcaaaagtcgctgaccttaaaaatgagtgctaagagtgaagctaatatcgatcgtttctgtgagttaacacagtcctggcttccgatggaaaaaacagaaaaagatccggtcagtggtgtatggacagtaaggaactcagggaaatgattaaatcatggtgggcagaaaaatccacatcggaaaaacagatcgttgcggcactggcggttctctcgctcggcgttttttgttggcttggggtgataaaaccgatagatacctacattgcagagcatcagtcccacgcgcaaaaaattaagaaggacatcaaatggatgcaggatcaagcgagcacccatggtttactcggtcatcctgcgcttacgcagcccatcaaaaatatccttctcgaggaagcaaaacgtgagaatttggctatcacgctggaaaacggcccggacaatactctgacaattcatcctgtcacagctcccctcgaaaacgtctcccgctggctcactacggcacaggtaacatacggtattgttattgaagaccttcagtttactcttgccggaaacgaagagatcaccctcaggcatttgtccttcagggagcaacaataatgacaatgctactgccgctcttcattctggttggttttattgcagattattttgttaatgccatcgcctatcacctctcgccgttggaggataaaacggcgttaacgtttcgccaggtattggttcatttcaggcaaaaaaaatatgcctggcatgatacagtgcccctgatactttgtgttgctgctgctatcgcctgcgccctggcacctttcacgcccatcgtgactggcgcactctttctctatttctgtttcgtactcacgctcagtgttattgattttcgcactcagctcctgcccgacaaactcaccttaccgctgctctggcttggcttggtatttaatgcgcagtatggattaattgatttacatgatgcggtttacggcgcggtagcgggctatggggtgctgtggtgtgtttactggggcgtctggttagtttgtcacaaagagggattgggctacggtgatttcaagctactggccgctgcaggcgcatggtgtggctggcaaacgttgccaatgatactgctgattgcctcgctgggtggcattggttacgccatcgtttcacaacttctgcaacgccggactataaccactatcgcattcggcccgtggcttgcgctcggcagcatgataaacctggggtatctggcctggatctcttattaaccgggagggttctccctcccgacacggctcaaccttcttcgcggatctgtgcttgcagataattttgcaggcccatcttctgaatcagatcaagttccgtttccagccagtcgatatggccttcttcatcacgcaaaatttctatcatcatatcgcggctgacgtaatcatgaacgctatcggcataaccaattgcctcacgcaaattcttcgcgccatccagctcaagtgccagatcagaacgcagcatttcctcaacatcttcaccaatgttcagtttgcccaggtcctgtaagtttggaagaccttccagaaaaagaatgcgctcaatataacgatcggcgtgtttcatctcatcaatggattcatgatactccacatcattgagacgtttgagaccccagtttttaaacattcgggcatggagaaagtactgattgattgcgacaagctcatttcccaacagtttgttgagataatttataactttagtatcacctttcattttttgactccttcgcttccactctttgaagagtagaacggcttacgagtaagtcaaaaaacacactccgtttatgcggactccttaaactccggcagctgcattaattcatcctccatcacttcacgcgcggcccggacacatttaccgcactgattgccgaccggaataaatttttttaattgctggaacgagtgaggggaaaactggcgcacagcctgacgaatttttttatcgctgataccattacaaagacaaacgtacatagagactcccgtatactttcttcaaaaataaatgaaaatagttcttatttcaattacggaaagactcttttttaagcaaagaatagaaatatgaataaaaataatgggctaccaaaagtagcccattgacaaaaaatgcggcgatactggaaggtatcgccaacacatttattgcttagtaaacggcgcgaagatttcgctaaatgcgtacttcggtgcctgttctttagtcaggccgtggaattccggagacaggttagtgccgcccggcaggtcgcgcgcgattgaccagataccaaccataccgagattacgcttctgcgcatcctgcatgaccagacgagcatcagagagatagaacacctcgccctgaacgtcgttcacgccaaccatcggcgtggtacccatcatagcgtcaatttctgcatcgctcttattgggatggaggcctttcaattgtgaatgcaggttggcaatcgcagacgttgcacacttaccgtgaatgttctggccttcggtatttgcagactgacaaatcgcgttaccgtagtccattgtcatcacgttcacacccgccagctcaacacctttcgctttggcatcgctcaggacattcatcccttccggcgtcaggccagtcggcagaattggcaaggtgtaccagatagcaatatctttgccttctgacttccatttatcctgcactttcttcacagcaaggttacgacgttcaatagatgcctgatccgcaacccaggtgccttcgatatcgaagtccaggactttgaggttcaggttatcaacgatgtcataataatgctgcatcagatcgtctacgttcttacaggaagcagccagcggagcgttgttagcaccaccgatagacagcatcacatcgccgccagcctcacgcagagctttgattttgctgtactgagcgtaattctgcataccgtaagcggtaccccatgtcggcagacaggtgttcgcatctttactcaccacaaacgccagcgtgaagtggttgacgttatgattcttagccagcgcagccagatccgggatcgtattcagcgtaaagtcgacatacggtgcataaacgtgtttcggccacgctttcttcggcgtacctacgcgctctttggttccggtccagtcaacaaaaacacgccacgggttgctgtcagaaggagaaactttctgcactttactctgagaaatgtagttcacaccgttaaagcgaatcagcgtatcgctggcataaagcgtttctggattaaactgcggcgcattattcagctcttcgttgctatagctctgagccttacctaacggcttccacgggcggctattgctaccggtggcgttttggttcgccaccagagcagggttgtcactttgcgtccagaacagcgcttcataagcctgcccatcaacaacaacgcgatcacctttcacgtacacagtggatgcggaccatgctttcgccggttcgtatttcttccacgggttatcgccgcccgggacaaagccccatgcgtcttgatcgacagaagttttataatgtgcatcgttataatctacgatgctgtccgcgctgtacgctttgctggcctggaaaccatccgcaacaatgacgccgccgttatcaatttcacaggtagtcgggttaccgtactgactcaattccgcagcggtagctgtacgctcgagacgccatgggttattggagttttcagcgctggtaccccgtgggcaatctttagacccaacccaccaggcgttcttgtaaacattaccattgaaaataacatggtaaatttcgctaccttcctggccgctccacgcttgcaatgagtaatcgttaacgctatccgctggtgttgatggctcgctgttatccggagttggggtcaccggtgtttccggagttggatcaaccggagtcacagcaccgccattattatccggcttaacggaacaggagccagggttaccatactggctgatttctgttgccgttgccgcgcgaacataacgccatgggttactggcatcgttttctttcgcatcgcctgggcaatttgccgcgcctacccaccaggcgttcttataaatgccgccgttatagataacgtaccatgtagaagaaccttcctgacctttccaggctactacagcatagttgtcgtttgacttatcagctggggctggctgaacatcaggagccggtttaacgtccggtgccggtttcacatccggtgaaggctgtggtgctgaagtacaggactgtggattactggtttctgagatttccgttgccgtagcggcacgaacataacgccatgggttgctggcatcattgcttttcgcatcacccggacagttagaagaggctacccaccaggcatttttatataccgcaccattaaagacgacataccaggtctgaccgccctgctgtttattccaggcaactacagaagaattagacggaacagtgccctgtgctggtgtagccgaaccgccattagccggcgtattggatgcaggcgtatttgaatttgaagaagatgagctgccgctcttttcgcaggaaagtgtattgccaaactgactaatttcagcagctgttgcggtacgctttaaacgccacgggttagttgcatcatttgctttcgcttttcccgggcaatttgtagaagaaacccaccaggcattttcataaattttgccatcgaaaataacctgatatttattaccaccttgttggttattccatgcttccattgccaatgctggcagagcggaacacaccagccccataccaatcatagatttagtaaatatatttaatttcattataatcccttgtgacgtaaaaactgcaaaacaaaagtcctacgcaggaattatttacgttttacgagaacccttcaatatgaattaaattacggcattaaaaataagaaaaaagcctgacaaatgaagcattttaaaaacagaaacattcatatttaaaatgttaaattgaattgatattttaaatatgaataatttattcgttctgacagtacgaataagatatgccgtcaacaaatgcaaaaagggcgccgaagcgcccttttcaattcaaaactaattaacgtgtaattagcccagaactttagcaacaacgcccgcgccaacggtacggccgccttcacggattgcgaaacgcagaccgtcgtccatcgcgatcgggtggatcagggtaacaaccattttgatgttgtcgcccggcattaccatctctacgccttccggcagttcgatggtaccagtcacgtcagtagtacggaagtagaactgcggacggtagcctttgaagaacggagtatgacggccgccttcatctttggacagaatgtacacttcagattcgaacttggtgtgcggcttgatggtgcccggcttagccagtacctgaccacgttcgatttcttcacgtttgataccacgcagcagaacacctacgttctcaccagcacggccttcgtccagcagtttgcggaacatttcaacgccagtacaggtagacttctgagtctctttgataccaacgatttcaacttcttcaccaactttgatgataccgcgttctacacgaccggtaacaacggtaccacgaccggagatggagaatacgtcttcgatcggcagcaggaacggcttgtcaatcgcacgctctggttccggaatataagaatccaggaagccagccagttccaggattttcgcttcccactctgcgtcgccttccagcgctttcagagcagaaccacgaacgatcggagtgtcgtcgcccgggaagtcgtactgagacagaagttcacgaacttccatttcaaccagttccagcagctcttcgtcatcaaccatgtcgcatttgttcaggaacacgatgatgtacggaacgcctacctgacgacccagcaggatgtgctcacgagtctgcggcatcgggccgtcagtcgcagcaactaccaggatcgcgccgtccatctgagcagcaccggtgatcatgtttttaacatagtcggcgtgccccgggcagtctacgtgtgcgtagtgacgggtcggggtgtcgtattcaacgtgagaagtgttgatggtgataccacgagctttttcttccggcgcgttatcgatctggtcgaatgcacgagcagcaccgccgtaggttttagccagtacggtggtgattgcagcggtcagagtagttttaccgtggtcaacgtggccgatagtaccaacgttaacgtgcggttttgtacgttcaaatttttctttagacacggctatattccttactatagtgctctccccttcaggagagagcacgggactttggtattaacccttaggcttatttaccacgggcttcaattacggcctgagcaacgttactcggcgcttcatcatacttcaggaattccatagtgtatgatgcacgacctttggtcagagaacgcagctgagttgcgtatccgaacatttcagacagcggtacttcagcgtggatcttaacgccagtaacttcagattcctgacctttgagcataccacgacgacggctcaagtcaccgataacgtcaccggtgttctcttccggagtttctacttcaaccttcatgatcggctcaagcagaactggtttcgctttcttaaagccttctttaaaggcgatagaagcagccagtttaaacgccagttcagaggagtcaacgtcatggtaagaaccgaagtgcagacgaatacccatgtctactaccgggtagcctgccagcggacctgctttcagctgttcctggatacctttatcaacggccgggatgtattcgccagggattacaccacctttaatgtcgttgatgaactcgtagcctttcgggtttgaacccggctccagcgggtacatgtcgataacaacatgaccatactgaccacgaccaccagactgtttcgcgtgtttaccttcaacatcggtaactttctggcggatagtttcacggtaagcaacctgcggtttacctacgttcgcttcaacgttgaattcacgcttcatacggtcaacgatgatgtcgaggtgcagttcgcccatacccgcgatgatggtctggttagattcttcgtcagtccatacacggaaagacgggtcttctttagccagacggcccagagccagacccattttttcctggtcagctttggttttcggttcaactgcgatggagattaccggctcagggaattccatacgttccagaatgatcggcgcatccgggtcacacagggtgtcaccagtggttacgtctttcagaccgatagcagcagcgatgtcgcccgcgcgaacttctttgatctcttcacgtttgttagcgtgcatctgaacgatacgaccgaaacgctcacgtgcagctttcacggagttcagtacggtatcaccagagttaaccacaccggagtaaacacggaagaaggtcaggttaccaacaaacgggtcggtagcgattttgaacgccagtgcagagaacggctcgtcatcacttgcgtgacgttcagccggagtgtctttaccgtcgtccaggataccgttgatcgcaggtacgtcaaccggggatggcaggtaatcaattaccgcatccagcatcgcctgaacacctttgttcttgaacgcagaaccacaggttaccaggatgatttcgttgttcagaacgcgctgacgcagagcacctttgatttctgcttcagtcagttcttcaccacccaggtatttttccatcagctcttcagaagcttcagctgcggattcgatcaggttctggtgccattcgttagccagttcaaccatgtctgccgggatatcttcgtattcgaaggttacgccctggtcagcgtcgttccagttgatagctttcattttcaccaggtcaacaacaccggtgaaatgttcttcagcaccaatcgccagctgcagcggaaccgggttcgcgcccagacgggttttgatctggttaacaactttcaggaagttcgcacccatgcggtccattttgttaacgaacgcaatgcgcggaactttatatttgtttgcctgacgccatacggtttcagactgcggctgaacaccaccaactgcgcagtaaaccattaccgcaccatcgagaacacgcatggaacgttctacttcgattgtgaagtcaacgtgccccggggtgtcgatgatgttgatgcgatgcggctcatactgcttagccataccagaccagaatgcagtagtcgcagcggaagtgatggtaataccacgttcctgctcctgctccatccagtccatggttgcagcgccgtcatgaacttcaccgattttatggtttacaccggtgtagaacagaatacgttcggtagtagtggttttaccggcgtcgatgtgcgcactgataccgatgttacggtagcgtgcgatgggtgttgtacgagccatttgtttcctcgtttatcttttaggcgttcaatttaagtagcccaaagcgggctgcttactggaagcgcccgcctggtgactaaaactccgaagggataaccaacggtagtgtgcgaacgccttgttggcttcggccatacggtgaacgtcttcacgtttcttaactgcagtacctttgttttctgcagcatcagaaagttcgttcgccaggcgcagagccatggatttatcaccgcgtttacgagcagcttcaacgatccaacgcattgccagagcattacgacgaaccggacggacttcaactggtacctgataagtagaaccaccaacgcggcgagacttaacttctacagtcgggcgcacgttttcgagagctacttcgaatgcttccagttcagatttaccagagcgctgagccagggtctccagcgcgctgtatacgatagattcagcagtagattttttaccatctaccatcaggatatttacaaatttagccagcagttctgatccgaacttcggatccggcagaattttacgctgaccaatgacgcgacgacgtggcatggaaatactccgttgttaattcaggattgtccaaaactctacgagtttagtttgacatttaagttaaaacgtttggccttacttaacggagaaccattaagccttaggacgcttcacgccatacttggaacgagcctgcttacggtctttaacgccggagcagtcaagcgcaccacgtacggtgtggtaacgaacacccgggaggtctttaacacgaccgccacggatcaggatcacggagtgctcctgcaggttgtgaccttcaccaccgatgtaggaagtcacttcgaaaccgttagtcagacgaacacggcatactttacgcagcgcggagttcggttttttaggagtggtagtatatacacgagtacatacgccacgtttttgcgggcatgcttccagcgcaggcacgttgcttttcgcaactttgcgagcacgtggtttgcgtaccagctggttaactgttgccattaaatagctcctggttttagcttttgcttcgtaaacacgtaataaaacgtcctcacacaatatgaggacgccgaattttagggcgatgccgaaaaggtgtcaagaaatatacaacgatcccgccatcaccaggccatctggctggggtgcttaaccgtaagtctgacgaaatcagtatagtcaatgagaatgatgtcgttcgaaatttgaccagtcaaaccgcgggcaataaggtcttcgttcagggcatagaccttaatgggggcattacgcagactttcaaggtagcggttaccgtcaactgcggcagttacgccatcttgcaataatagcagttcgtctccttcactgagcagacgcagcagcgcagcaaaatccgtcagccagggtgagcgatgtaatgtgtgcagcataaacgcctcaaaacctcaaaataacatcgtagttggcgagttcgcggcgtaaggcatctgcttcgagcggcgtggcttcgacaacaaagggtgtctgcggatctaacccgcgttcgcgcagtgaagccgcacaaacccagcactgttcaatgtcgtacagacccaacaatttaaaagtggcaatgtaatcacgcgccagcactgcatcgggcttttgtcctggcagcagctgaaaaacgccatcagctataaagaagacagccagatcgtcagttaatgcggaagttgccagtaaagcatctaaaccttcccggcctgcggctgtaccatgaggtgcagtagaaaaaacaaacgcaattcgtttcatcagaactgtaccaccctgtcacaggtcagcgaggcttccgccagcgccccaagtccgcttaaggtaaatccctgctgaaggtttgacgaagccagccccagtcttccggcctccgtttcatcaacaacgccacggcgtaatgctgccgctacgcagatattcagcgccacaccatgttgcgcattcagttgttgccaggcccgtacgaggtcaaattcgtcacttgccggagaggtcaattggttagcgttatagaccccttcccgatagaaaaagacgctgcttaactcatggccatctgctatcagcgcctgcgcaaactgaaaagcactactcgcctgttgcgtaccgtatgctggcccggtcaccacgatggcaaaacgcattacttatcttgcccctggaaatcaccgctcttgaactggcggatgtagagatagacagtgtgtttggagatgttcaggcggtcagcaacctggttgatcgcatctttaatatcgaagatccctttctcgtagagattcagcacgatctgacgatttttggcgttattagaaacattgcgatcggcattcacttcttcgatggtgaactccagcgtttgggtaaccagatcttcaacagaagaggcaaagttgacgcttgaaccgacatccggggtttctggcggcacaaaggtgctcataatctgcgagaagggaacatcaagattcatattgatgcacagcagaccaattacacgctgttcgcggttacgaatcgcgatagtcagggacttcattaatacgccgcttttggcgcgagtaaagtagcatttagaaacgctgctatccgctcccgtcatatcgtgcagcatacgtagcgccaggtcagtaattggcgaaccaatcttccggcctgtatgttcaccgttagcaatgcgaatggctgaacattttagatcctgcaaagagtgcaaaacgatttcacagtgggagccaataagcatcgctaacccgtccaccaccgcttcgtaggatttcagaatatcaaaatcggtctggtcgaaaggacgttgatccagtaaatccaactcactggtttcgttggttaaaagcgacctggacatgaaaaaaaacactccttttcaggagcctgtcgttaacttttcagggcaggctcattaatgatgcgggtaactaaattaatacagcggaggttccgctttccagcactaattatatccggcctgtaataaaaaaaccgccgcctggtcaggcggcggttcttaatgcttattttttagcagaatctgcggctttcgcatcagcttccggctttgcatcagccttcggcgctggtttcacatccagcagctctacgtcaaacaccagggtagaattcggtgggatccccggaacacccgctttgccgtaagccagttctggtggaataaccagtttgatcttaccgcctttcttgatgttcttcagaccttctgtccaacccgggataacaccgtccagacggaaagaaagcggttcaccacgggtgtaagagttgtcgaactctttaccgtcgatcagcgtacctttgtagttcactacaacagtatcgctgtctttcggtgcttcgcctttaccggcttctactacctgataaaccagaccagttgaagaggttttcacacctttctctttggcaaatttctcgcggtactctttaccttttgcttcgttatcagccgcgtctttttccatcttcgcctgagcagaagacttcacgcgagcttcgaatgcttgtagagtctgttcgatctcttggtcggagagtttgctcttatcagcaaatgcatcctgaacaccagcgatcagctgatctttatccagtttgatgcccagtttttcttgttcttttagagagttttccatgtaacgacccagcgaggcacccagtgcataagctgatttctgatcgtcatttttgaacgctgctttgctgtcagcagctgtagcaggttttgcagcttcagcagcaaaagtgattggtgcatgcagggcaacggccattgtggtcgccagcagcgttactttaaacagtgatttcatccatatctccaggatcggggcatctcaccccagggttaactattatcagaagggtactataaagcgttgtcgaacaaatctacatacagacacgccctattatcatctattttcagactctttttgtttaaattagtttcgatgaccgcgaaatgagtgctgtctcgggcagcaaagttaagtagaatccgcggcgaccattcgacaaaagaggtgaatcatgcaggatttatcattggaagcacgcctggcagagctggagagccgactggcttttcaggaaatcaccattgaagaactgaacgtcacggtgaccgctcatgaaatggagatggcgaaactgcgcgatcatctgcgtctgctgaccgagaagttaaaagccagccagccgtcgaacatcgcgtcgcaggctgaagaaacgccaccgccacattattgaggcgtaaaaaaagcggggattccccgcttttttgtcactttttcggtattagtggcaaccgcaaccgccgttgcctttaccgccacagcagccttcgccaccgtgttcatgaccgtgatcgtggccatgaccgccgcagcaaccgtcgtggtcgtgatcgtggtggtgatcgtgcgcgccgtgaacgtgaccatgagccagttcttcttcagtcgcttcgcgaatcgccacaacttcaacgttgaatttcaggttctgaccggccagcatgtggttaccatcaaccacgacgtgatcgtcttcaaccgcagtgatttcaaccggtaccggaccctggtcggtttcagccaggaaacgcatacctacctgcagttcatcaacgcccataaatacgtctttaggaacacgttgcaccaggttttcgtcgtactgaccgtaagcgtcgttcgcgccaacagcgacatcaaatttgtcgccaacttcatgaccttccagcgccgtttccaggccagagatcagggaaccgtgaccatgcaggtagtccagcggcgcactcaccggagactcatcaaccaacacaccgtcttctgtacgtacctgataggccaggctgaccaccaggtcttttgctactttcatgatatctcctgagcatgggaagaatagtggcgcagattgtagcggaattctgcagccgtgtactcactagcttaaaaaaactcggcgcatatcgctagtccggatgaaaaatcccgatcacttgctcatctttgcgaacgtgatcgcgggcttctttgtctgcttctcgcatctgatgtccgcacttaacacattcaacaatatcaatattattttcgcgccacatcgccattgaatcctgcgcctgacaggccgggcattttgcgcccgcaataaaacgttttcggattgccatctttaccctctactcaaattcatcccagccgtccagctggcgtcgttcttgttgcatttcacgctggaaaatctcttccagttcgcgtcgggcttccctggcgcgagaaatttgtacggtatcggcatgcattgggatgagctctcgcagcatccgcatatccaggcggcgaaaatgcagttgcgctcgctgtgcctgatgcggatgcatgccaagcgtgaccagcgtcttgcgccccagctctaacgcactggagaatgtttcacgggaaaactgcgtcacccctgcctgtaataactcatgcgcttccacacgtccgcgcgctcgcgcaagaatatgcaaatgcggaaagtgctgttggcatatttccaccagcttcatggtgtcttccggctcgttacaggtaatgacgatagactcagcggcctctgcacccgcagaacgtaaaagatcgacctgcgtggcgtcgccgtaataaactttgtagccgtatttacgcatcaggttaacggcgctgatatcccgctccagcacggtaatgcgcattttatttgccatcagcaaacgaccaatcacctgaccaaaacgcccgaagcccacgacaatgacctggggtttatcatcgttgacccacggtttttcgtcttcttcttccggtccgttaaactggcgggatagccatttatccaccagcttcatcagcaacggcgtggtcatcatggaaagcgtcaccgtcaccagcaacaacgccatctggtcgccctggaataagcgttgtgaagaagcggtagaaaagaggacaaaggcaaactcaccaccctgactcaacacgccagcaaactgcatccgctctgagctacgcacgccatacaatcgcgccagcagatacagcacgagaattttcaccgccaccagcacaaccacgcttatcactacccacaacagatgggtataaagcaccccgaggttgagtgacatgccgacagagataaagaacaaaccgagcagcaagcctttgaagggatcgatagccgtttccagttcatggcgatattcactttccgccagcagcacgcccgcaataaatgtaccgagcgccatcgacagccccagcgcatccataaacaatgcggaacccaacaccagcagcagcgtcgcggcggtgaacacttcccgcacgccagaagctgcaataaagcggaataccggacgcagtaaatagcgcccaccaatcagcatgccgacaaacgccagcaccttcatgccgaccttcatccagtcgaaatgttcgtctgccgaccccgccaacaacggcactaacgccagtgctgggattactgccagatcctgaaacagcagaaccgaaaacccgagctggccggattcgctgcgattcatccctttctcacgcatcaattgcaacgccattgcagttgaagacatcgcaaggccaatgccaccgaccaccgccgcctgccaggcgaaatccgtcagcatcaataatcccgccagcaacgccgcgcttaacagcacctgtgccgcgcctacgccaaaaatcgaacgccgcagttgccaaagtttggagggattcaactcaaggccgatgataaacatcaggaataccacgccgagttccgaaaagtggaggatctcatcgacgtcgctaataaaccccagcccccacgggccaattgcaatccctgccagcaaatatcccaacacagcgccaatacccagccgcgatgccagcggcaccgcagccaccgccgcgaagagaaacagcactcctgcgagtaaaaaatcggaaccttccatcagcggcctcctggagacagcggatttgccagccagtcaccgtaggctctggcgtggctcgccagctcctgtgcgctttgccgtctcgcccagtaaataatgatgggacttaaccaatgcatccggcacatgcccgccgccagttcaaaggggcgcagcacatcgctcatcgggtagcgattcagcgcgtcataacggtaagcactttccggctcgccggtggtaatcacgctacgccagtactttcccgccagttggtttcctcccggcccgctggcaaaaccacgacttaatacccggtccagccactctttcagtagcgccgggcagctataggtataaagaggatgctgaaagacaatcacctcgtgctcgcgcagtaatgcctgctcacgggggatatcaataaaaaaatcgggatagtgcgcgtaaaggtcgtgcacggtaacattgctgagctgcgtggccggtttaagcagtacccggtttgccaccgagtcctgagattccggatgggcatacagcagcaaaactttcgctggctgagacatcatccccctcccggtatggtttttgtgtatagtcgctgttttgggctaccattgcgcccggtgcggcagctcgcccatacattacattatcataatgataagttaacatagtctgaacatacggcaccttatgattgttttctcctcgttacaaattcgtcgcggcgtgcgcgtcctgctggataatgccaccgccaccatcaaccctgggcagaaagtcggcctggtgggtaaaaacggctgtggtaaatctaccctgctggcattgctgaaaaatgaaatcagcgccgacggcggcagctacacctttccgggaagctggcaactggcgtgggtgaatcaggaaacgccggcgttaccgcaagcggcgctggaatatgtcattgacggcgaccgtgaatatcgtcaactagaagcgcagctacacgacgccaacgaacgtaacgacgggcacgccattgcgaccattcatggcaagctggatgctattgacgcatggagtattcgctcccgtgctgccagcctgctgcacggcctcggtttcagcaatgaacaactggagcgcccggtaagtgatttttccgggggctggcgtatgcgtcttaaccttgcccaggcgctgatttgccgttcagacttgctgctgctcgacgaaccgactaaccacctcgatctcgatgccgttatctggctggaaaaatggctgaagagctatcagggcacgctgatcctgatctctcacgaccgcgacttcctcgatccgatcgtcgataaaattattcatatcgaacaacaaagcatgttcgagtacaccggcaactacagttcgtttgaagtacagcgcgccacccgtctggcgcagcaacaagcgatgtacgaaagccagcaggaacgcgtagcgcatctgcaaagttatatcgaccgtttccgtgccaaagccaccaaagcgaagcaggcccagagccgcattaagatgctcgagcgtatggagctaattgcccccgcgcacgtcgacaacccgttccgctttagcttccgcgcgccggaaagcctgccaaatccgttactgaagatggaaaaagtcagcgcgggctatggcgatcgcattattctcgactcgattaaactgaacctggtgcccggctcgcgtattggtctgttaggccgcaatggcgcgggtaaatcgacattaatcaaactgttagccggtgaacttgcgccagtcagcggtgaaattggtctggcgaaagggatcaaactcggctacttcgcccagcatcaacttgaatacctgcgcgccgacgaatcacctattcaacatctggcacgtttagcgccgcaggagctggaacaaaaactgcgtgactacctcggcggctttggtttccagggcgataaagtaaccgaagaaacgcgccgcttctccggtggggaaaaagcccgcctggtgctggcattaattgtctggcagcggccgaatctgctgctgctcgacgaaccgactaaccaccttgacctcgacatgcgtcaggcactcaccgaagcattaatcgagtttgaaggcgcgctggttgtcgtttcgcacgaccgtcatttgctgcgttccaccactgacgatctctacctggttcacgatcgtaaagtcgaaccgttcgacggcgatctggaagattatcaacagtggttgagcgacgtacaaaagcaggaaaaccagaccgacgaagcgccaaaagagaatgcgaacagcgcccaggcacgtaaagatcagaagcgtcgggaagctgagctgcgtgcgcaaacccagccactgcgtaaagagattgcccgtctggaaaaagagatggagaagctgaacgcgcaactggcgcaggcggaagagaaactcggcgacagcgaactgtatgaccagagccgtaaagcggagttgaccgcctgcctgcaacagcaagccagcgccaaatccggcctggaagagtgcgaaatggcatggctggaagcccaggagcagcttgagcagatgctgctggaaggccaaagcaactgatggcgcagataacgacgaccgatgccaatgaattcagcagcagtgctgaattcatccccatgcgcggctttagcaattgtcatctgcaaaccatgctgccgcgtctgtttcgtcgtcaggtgaaattcaccccgtactggcagcggctggagttgcccgacggcgattttgtcgatcttgcgtggagtgaaaaccctgcacaggcgcaacataaacctcgtctggtggtgtttcacgggctggaaggcagtctcaacagcccttacgcccacggtctggttgaggcggcgcaaaagcgcggctggctgggcgtggtgatgcattttcgcggatgcagcggtgaaccaaaccgtatgcaccgcatttaccattcgggcgaaaccgaagacgccagttggtttttacgctggctgcaacgcgaatttggtcatgcgccaacggctgccgtcggctattcgctcggcggtaatatgctggcctgtttgctggcaaaggaaggcaatgatctcccggttgatgcggcggtgattgtctctgcgccgtttatgctggaagcctgtagctatcatatggaaaagggcttttcccgcgtttatcagcgttacttgctgaacctgttaaaagccaatgccgcgcgcaagctggcagcctaccccggaacgctgccgattaatctcgcgcagttaaaatcggtacgtcgcatccgtgaatttgacgatctcatcaccgccagaattcacggctacgccgacgctatcgactattatcgtcagtgtagcgccatgccgatgctgaaccggatcgccaaaccgacgctgattattcacgccaaagacgatccgtttatggatcatcaggtgatcccgaaaccggaaagtctccccccgcaggtggagtatcaactgactgaacatggcggtcatgttggctttattggcggtacattacttcatccgcaaatgtggctggagtcacgcattcctgactggttaacaacgtatctggaggcgaaatcatgttgattccgtggcaagacctctcccccgaaacgctggaaaatttaattgaaagctttgtgttacgtgaaggcaccgattatggtgaacatgagcgtacacttgaacagaaagtcgccgacgtcaaacgccagctacagtgcggagaagcggtgctggtatggtcggagctgcacgaaacggtcaatattatgccgcgcagtcagtttcgcgaataacctgcaaccgtcggcggacgagataataatgatagctaagtcatggagttactatgtctgccaaacatccggtcattgcggtaacaggatccagcggcgcggggaccaccaccaccagcctcgcgtttcgtaaaatattcgcgcagttaaatctgcatgcagctgaggtggaaggcgacagttttcaccgttacacccgcccggaaatggacatggcgatccgcaaagcgcgcgacgccgggcggcatatcagctacttcggccccgaggctaacgacttcggcctgctggaacaaaccttcattgaatacggtcagagcggcaaagggaaatctcgcaaatatctgcatacctacgacgaagccgtaccgtggaatcaggtaccggggacattcaccccctggcaacctttaccggaacccactgatgtactgttttatgaaggtttacacggcggcgtagtcacgccacagcataacgttgcgcagcatgtggacttactggtcggcgtggtgcctatcgttaaccttgagtggattcaaaaactgatccgcgacaccagcgagcgcgggcactcacgagaagcagtgatggactcagtagtgcgttcaatggaagactatatcaactacatcacaccgcagttttcccgcacccatcttaacttccagcgcgttcccaccgtcgacacttcaaacccgttcgcggcaaaaggtatcccgtcgctcgatgaaagctttgtggtgatccattttcgtaatctggaagggatcgatttcccctggctgctggcgatgttgcaaggctcattcatttcccacatcaatacgttagtggtaccgggcggcaaaatgggtctggcaatggaattaattatgctgccgctggtgcaacgattgatggaaggaaagaaaatcgagtaactctgctattacgccggataaaatactatccggcttcacaacgggatagttaagtcacgcggcaaccacttcatacgagtgagtaatattcaccgctttttccagcatcaacgccactgaacaatatttctcggcagagagatcaaccgcacgcgcaaccgctgcgtctttcaggtcgcgaccggtgacgataaaatgcagattaatgtgcgtaaacaggcgtggtgcctcttcgcggcgttcagaggtcaattttacttcacaatcgaccacatcctgacgccctttttgcaggatcgaaaccacatcgatggcactgcaaccacccgccgccatcaacaccatttccatcggacttggtgctttatcgcctgagttgccgtccattaaaatctgatgaccagaggcggattcgcccagaaaagttaacccttcgacccacttcactcgcgcttgcatttttgctactccactgcgtcaattttcctgacagagtacgcgtactaaccaaatcgcgcaacggaaggcgacctgggtcatgctgaagcgagacaccaggagacacaaagcgaaagctatgctaaaacagtcaggatgctacagtaatacattgatgtactgcatgtatgcaaaggacgtcacattaccgtgcagtacagttgatagccccttcccaggtagcgggaagcatatttcggcaatccagagacagcggcgttatctggctctggagaaagcttataacagaggataaccgcgcatggtgcttggcaaaccgcaaacagacccgactctcgaatggttcttgtctcattgccacattcataagtacccatccaagagcacgcttattcaccagggtgaaaaagcggaaacgctgtactacatcgttaaaggctctgtggcagtgctgatcaaagacgaagagggtaaagaaatgatcctctcctatctgaatcagggtgattttattggcgaactgggcctgtttgaagagggccaggaacgtagcgcatgggtacgtgcgaaaaccgcctgtgaagtggctgaaatttcgtacaaaaaatttcgccaattgattcaggtaaacccggacattctgatgcgtttgtctgcacagatggcgcgtcgtctgcaagtcacttcagagaaagtgggcaacctggcgttcctcgacgtgacgggccgcattgcacagactctgctgaatctggcaaaacaaccagacgctatgactcacccggacggtatgcaaatcaaaattacccgtcaggaaattggtcagattgtcggctgttctcgtgaaaccgtgggacgcattctgaagatgctggaagatcagaacctgatctccgcacacggtaaaaccatcgtcgtttacggcactcgttaatcccgtcggagtggcgcgttacctggtagcgcgccattttgtttcccccgatgtggcgcagactgatttatcaccccgatatcaactatgcacttcgacaaacgctggtgctatgtttgcccgtggccgttgggttaatgcttggcgaattacgattcggtctgctcttctccctcgttcctgcctgttgcaatattgcgggccttgatacgcctcataaacgttttttcaaacgcttaatcattggtgcgtcgctgtttgccacctgtagcttgctgacacagctactactggcaaaagatgttcccctgccctttttgctgaccggattaacgctggtacttggcgtcactgctgagctggggccattgcacgcaaaattgcttcctgcatcgctgctcgccgccatttttaccctcagtttggcgggatacatgccggtctgggaaccgttgctcatctatgcgttgggcactctctggtacggattgtttaactggttttggttctggatctggcgcgaacaaccgctgcgcgagtcactaagtctgctgtaccgtgaactggcagattattgtgaagccaaatacagcctgcttacccagcacaccgaccctgaaaaagcgctgccgccgctgctggtgcgccagcaaaaagcggtcgatctaattacccagtgctatcagcaaatgcatatgctttccgcgcaaaataatactgactacaagcggatgctgcgtattttccaggaggcgctggatttacaggaacatatttcggtcagtttgcatcagccggaagaggtgcaaaagctggtcgagcgtagccatgcggaagaagttatccgctggaatgcgcaaaccgtcgccgctcgcctgcgcgtgctggctgatgacattctttaccatcgcctgccaacgcgttttacgatggaaaagcaaattggcgcactggaaaaaatcgcccgccagcatccggataatccggttgggcaattctgctactggcatttcagccgcatcgcccgcgtgctgcgcacccaaaaaccgctctatgcccgtgacttactggccgataaacagcggcgaatgccattacttccggcgctgaaaagttatctgtcactaaagtctccggcgctacgcaatgccggacgactcagtgtgatgttaagcgttgccagcctgatgggcaccgcgctgcatctgccgaagtcgtactggatcctgatgacggtattgctggtgacacaaaatggctatggcgcaacccgtctgaggattgtgaatcgctccgtgggaaccgtggtcgggttaatcattgcgggcgtggcgctgcactttaaaattcccgaaggttacaccctgacgttgatgctgattaccaccctcgccagctacctgatattgcgcaaaaactacggctgggcgacggtcggttttactattaccgcagtgtataccctgcaactattgtggttgaacggcgagcaatacatccttccgcgtcttatcgataccattattggttgtttaattgctttcggcggtactgtctggctgtggccgcagtggcagagcgggttattgcgtaaaaacgcccatgatgctttagaagcctatcaggaagcgattcgcttgattcttagcgaggatccgcaacctacgccactggcctggcagcgaatgcgggtaaatcaggcacataacactctgtataactcattgaatcaggcgatgcaggaaccggcgtttaacagccattatctggcagatatgaaactgtgggtaacgcacagccagtttattgttgagcatattaatgccatgaccacgctggcgcgggaacaccgggcattgccacctgaactggcacaagagtatttacagtcttgtgaaatcgccattcagcgttgtcagcagcgactggagtatgacgaaccgggtagttctggcgatgccaatatcatggatgcgccggagatgcagccgcacgaaggcgcggcaggtacgctggagcagcatttacagcgggttattggtcatctgaacaccatgcacaccatttcgtcgatggcatggcgtcagcgaccgcatcacgggatttggctgagtcgcaagttgcgggattcgaaggcgtaatgcaggctaaaccatcggataaggcattcacgccgcatccgacatcttttgcctgatgcttcgtatttacgccccaaccaccttcgccaccgcgtgggcgaaacgttgcatcccttcatcgatatccgcatcttccaccaccagcgacggtgcaaaacgcatcacatccggtccggcattcagcaccattacgccagcctctgcgcccgcatacaggaaatcacgcgcccgacctttgtactgtggtttcagctctgcgccaatcaacagccccataccgcgaatatcgctaaatacatcgtactgctgatcgatcttctgcagatggtcaacaaaacgctggcgtttcgcctgaatgccttccagcacttcaggggtattgatgatatcaaacgccgcccccgctactgcacaggccagaggattaccgccgtaggtggaaccgtgagaaccaggatgaaacgcagaagcaatttccgccgtggtcagcatggcgctaatcgggaagccgccgcctaacgctttcgcagaggtcagaatatccggcgtaacgccgtagtgcatgtaagcaaacaaatcgccggtccgccccatcccgcactgcacttcatcaaacaccaataatgcctgatgttgatcgcacagctcgcgcaagccctgcaaaaactctggcgtcgctgccgtcacaccgccctcgccctggatcggctcaaccaccaccgcacaggtgtgatcatccatcaccgctttcactgcatggagatcgttaaagggaacgtggatgatgtctgccggtttcggcccaaagccgtcggaatattttggctgcccacccaccgaaacggtaaacagcgagcgaccatgaaaagcgttatggaaggcaataattttggttttgaacgggctatgacgcacacaggcgtaatggcgtgccagtttaaaggcggtttcgttagcttccgtgccggagttcataaacaccacgcgttcggcaaacgttgcctcaatcagtttacgcccaagacgcagcgccggttcattggtgaaaacgttactgatatgccacagagtttcgccctgggtttttaacgcgttcaccagcgcaggatggcaatggcccaacgccgtaactgcaatgccacccgcgaaatcgacatactccttgccttgctgatcccagattcggctgccctgaccttttaccggaataaactctgccggagcataaatcggcaggatcacttcatcgaaagtcgcgcgtgtaattgctgtttgttcaattgccatctcatgatcaccctgttacgcataaacaaatgtgaaattataaccacaaaatatgcataaaaaatcactaaatggcaatcagaaatcagcgatgcaggaaattagccagcagttgatgtccttgttcgctaagaatactttctggatggaactgcacaccttccagatcccactggcgatggcgaatccccataatctctcgggtttcgctccaggccgtcacgtcaaagcacgctggtaatgagtcaggttccaccaccagcgaatggtagcgtgtcacggtaagtggatttgccagcccccgaaatacgccctcaccgttatgtgtaatcggcgaggttttgccgtgcatgacctttgcggcgcgcacaactttaccgccaaatgcctgcgccattgcctgatgaccgaggcagacgccaagaatcggcaagcgcccggcatagtggcgaataacgtcaagggagatcccggcttcatctggcgtacaggggccaggtgagatgacaattttttgtggtttaagggcgtcgatatccgccagcgtcaacgcatcgttgcgcttaaccagcacatccgcccccagttcacaaaagtactggtagaggttccaggtaaaagaatcgtagttatctataagcaggatcatggcggctccggtacaaaagaaccgcgctattttactcagattccccggcttcgcttaccactttgctaaatatcatctgcagtgcggtgagatcccccattgccccactctgatttgcctgattccaggcctctttttcgataccctgccagctcagttgatatccggcatgaatcgccagttgctcgaagaagatccgctgtgccagaccacttcccacccggaagggatgcagcacgttgatttcacaatagtaatgcgccagccgctcgacgaacttcgctttctccaggccaaccagataaccttcttcctccagatcctgcatcagggcattgccctctttttcgatataagcaaagtggcagaacggcgtatcaccctgataaatatcaacttcacgcagttgccctgcccagtcgaaaatatcctgatacagctggcgatggatagttcgcaaatgcggtaaaccgcgcaccagcggaccaagctcaatggtcgcagcacgcagcgccgtcatttcgtaagcggcctgttccagccgctgctgctggcggatgttcagccggttacgcatgatatcaaggcctggataaagatacggatcgcgcccttcgccgaatttatcgctcatagtgactcctcagctcttcaaggcgcgctaaagcctctgcggcagtaagagtgactaaaggcatctcgacgccttcaagacggcgactggcctgaaaattacgattacgctgaagctcccagagacgggacttttgcttatcggtgagtttcttcacttgatgcctccctgaacgtgtccatttgccacaagtataagcggcaaatccgggttacgccgggagagcagaagcgcgggcaagattgcccgcgcgagaaatcattacggcaggactttagcggaaaggataactaccggttttgacggcacattctggtacggaccaacgtcatgagtcggcacctgggaaatcttatcggcaacgtccatgcctttcaccactttaccaaataccgcgtaaccgaaatcacgctgaccatggtcaaggaaggcgttatcggcaacgttgataaagaactggctggtggcgctgtctttgtcagcggtacgtgccatcgcgatggtgccacgcgtgttgcgcaggccgttatcggcttcatttttgattggcgggtttggttttttctgctgcatctgctcggtgaaaccgccgccctgaatcataaagccaggaatgacgcggtgaaaggtagtgttgttataaaaaccgctgttcacataatcgacaaagttttgcacagacactggcgctttttgtttatccagctccagttcgatgttaccagctgaggttgtcaacaatacgtgcgggtcccctttcgctgccattgctgcgggagaaagagcagaaagagcgaaaacagcagccatcgccgccagggtcgatttgaacatgagatttccttaacaaacagagcagaaaaaaagcaagtgaagagattctaaatagccttcaagaacaaggccatccctttacctaattttacgtatctgaaatatatgtaacctgacgatcactttttattccgtgatcaaaatcacctcttaaaatgcaatttagcaaccgattgcaataaaacatttaaacagatcacaaaatcacctaaaatcgcccgctcgcggcatatcccgctatgccattttatttttgaacgcaggccaatcatgactaacagcaatcgcatcaagctcacatggattagctttctctcctacgcactgactggtgcgttggttattgtcaccgggatggtgatgggaaatatcgccgattatttcaatctgcctgtttccagtatgagtaataccttcaccttcctcaacgccggcattttaatctctatcttcctcaacgcctggctgatggaaatcgtcccgttgaaaacgcagttacgttttggctttctcctgatggtgctggcggttgccggtttgatgttcagccacagcctggcgctgttctcggcggcgatgttcattctcggggtggtcagcggcatcaccatgtcgattggtacattcctggtaacacaaatgtatgaagggcgtcagcgcggttcccgcctgttatttaccgactccttcttcagtatggctgggatgattttcccaatgatcgccgcgtttctactggcgcgcagcattgagtggtactgggtttatgcctgcatcgggctggtgtatgtcgctatttttattctgaccttcggctgtgagttcccggcgctgggcaaacatgcgccaaaaacggatgctccggtagagaaagaaaagtgggggatcggcgtactgtttctctctgttgcggcgttgtgctacatcctcggtcagttaggttttatctcctgggtgcctgagtatgccaaaggcctgggcatgagcctgaacgacgcgggcacgctggtgagtaacttctggatgtcatacatggtcggcatgtgggcgttcagctttattcttcgcttctttgatttgcaacgcattctgaccgtactggctggtctggctgcgattctgatgtacgtctttaacaccggaacaccagcacatatggcgtggtcaattctcgctctgggcttcttctccagcgcgatctataccaccatcatcaccctgggttcacagcagaccaaagtaccgtcgccaaaactggttaactttgtcctgacctgcggaaccatcggtactatgttgacctttgtggttaccggcccgatcgttgaacatagcggtccgcaggcggcactgcttacagcaaacggtctgtacgctgtcgtctttgtgatgtgcttcctgttaggtttcgtcagccgtcaccgtcagcataacaccctgacctctcattaattgctcatgccggacggcactatcgtcgtccggccttttcctctcttcccccgctacgtgcatctatttctataaacccgctcattttgtctattttttgcacaaacatgaaatatcagacaattccgtgacttaagaaaatttatacaaatcagcaatatacccattaaggagtatataaaggtgaatttgatttacatcaataagcggggttgctgaatcgttaaggtaggcggtaatagaaaagaaatcgaggcaaaaatgagcaaagtcagactcgcaattatcggtaacggtatggtcggccatcgctttatcgaagatcttcttgataaatctgatgcggccaactttgatattaccgttttctgtgaagaaccgcgcatcgcttatgaccgcgtacacctctcgtcttacttctctcaccacaccgccgaagagctgtcgctggtgcgcgaaggcttctacgagaaacacggcatcaaagttctggtcggcgaacgcgctatcaccatcaaccgtcaggagaaggtgattcactccagcgccggacgtaccgttttttatgacaagctgatcatggcaaccggttcctacccgtggatcccgccaatcaaaggttctgatactcaggactgctttgtctatcgcactattgaagacctcaacgccattgaatcctgcgcccgtcgcagcaaacgcggtgccgttgttggtggcggcctgttaggtctggaagccgcaggcgcgctgaaaaacttaggtattgaaacccacgttatcgaatttgcccctatgctgatggcagaacagcttgatcagatgggcggcgagcagctgcgtcgcaaaatcgaaagtatgggcgtgcgcgttcacaccagcaaaaacacccttgagattgtgcaggaaggtgttgaagcgcgtaaaaccatgcgttttgccgacggcagcgaactggaagtcgactttatcgtcttctctaccggtatccgtccgcgcgataagctggcaacccagtgtggtctggacgttgctccgcgtgggggtattgtcattaatgattcctgccagacttccgatccggatatctacgccatcggtgaatgcgcaagctggaacaaccgtgtatttggtctggtagcacctggctacaaaatggcgcaggtcgccgttgaccatattctcggtagcgaaaacgcctttgaaggtgctgaccttagcgccaagctgaaactgctgggcgtagacgtaggcggtattggtgatgcgcacggtcgcacgcctggcgcacgtagctacgtttacctcgacgaaagtaaagagatctacaaacgcctgattgtcagcgaagacaacaaaaccctgctcggtgcggtactggtgggcgataccagcgactacggtaacctgctgcaactggtgctgaacgctatcgaactgccggaaaacccggattccctgatcctgccagcacactcgggtagcggcaagccgtctatcggtgttgataaactgccggacagcgcgcaaatctgctcctgcttcgacgtcaccaaaggtgatctgattgctgccatcaacaaaggctgccacacagttgcggcgctgaaagctgaaaccaaagcgggtactggctgcggtggctgtatcccgctggtcactcaggtactgaacgcggaactggcgaaacagggcatcgaagttaacaacaacctgtgcgaacactttgcttattcgcgtcaggaactgttccatttgatccgcgttgaaggcattaaaaccttcgaagaactgctggcgaaacacggcaaaggctacggttgtgaagtttgtaaaccaaccgtcggttcgctgctggcctcctgctggaacgaatacattctgaagccggaacatactccgctgcaggattctaacgacaacttcctcgctaacatccagaaagacggcacctactcggtgatcccgcgttctccgggcggtgaaatcaccccggaagggctgatggcggtaggtcgtatcgcgcgtgaatttaatctctacaccaagatcactggctcccagcgtctggcgatgtttggcgcacagaaagacgatctgccggagatctggcgtcagctgattgaagccggcttcgaaaccggtcatgcctatgcgaaagcactgcgtatggcgaaaacctgcgtgggtagcacctggtgccgctacggcgttggcgacagcgtcggcctcggcgtggaactggaaaaccgctacaaaggcatccgtacgccgcacaaaatgaagttcggtgtctccggctgtacccgtgaatgttcagaagctcagggtaaagacgtgggtattatcgccactgaaaaaggctggaacctgtatgtttgcggtaacggcggcatgaaaccgcgtcatgcggatctgctggcggcggatatcgatcgcgaaacgctgatcaaatatctcgaccgcttcatgatgttctacatccgtactgccgacaaactgacgcgtaccgcaccgtggttagaaaacctcgaaggcggcatcgattacctgaaagcagtgatcattgacgacaaactggggctgaacgcacatctggaagaagagatggcgcgcctgcgtgaagcggtactgtgtgagtggactgaaacggtcaatacgccgtctgcgcagactcgcttcaaacacttcatcaacagcgacaagcgtgacccgaacgtgcagatggtgccagagcgcgaacagcaccgtccggcaacgccgtatgaacgtatcccagtaactctggtggaggacaacgcatgagccagtggaaagacatctgcaaaatcgatgacatcctgcctgaaaccggcgtctgcgcgctgttaggtgacgagcaggtcgcgattttccgcccgtatcacagcgatcaggtgtttgcgatcagcaacatcgacccgttcttcgagtccagcgtgctgtcacgcggactgattgcggaacaccagggcgagctgtgggtcgccagcccgctgaaaaaacagcgttttcgcttaagcgacggcttgtgcatggaagacgaacagttttccgtcaaacattacgaagcgcgagtgaaagacggcgtggtgcagctgcgcggttaatgttttaacgggaggcgcaatgcctcccctttttgcatggtcctgtaataatcttcggtatattgcaggacattttttaaactttttgttttattttttgtttttattttttaaaggataatcaaatgtttacagacactattaataagtgtgcggctaacgctgcgcgcattgcacgcctgtcggcaaataacccgctcggcttttgggtcagctccgccatggcgggcgcgtatgtgggtcttgggatcatcctgattttcacgctcggtaatttgctcgatccatccgtacgccctttggtgatgggcgcgacctttggtatcgccttaacgctggtgattatcgccggttctgaactgttcaccggacacaccatgttcctcacctttggggtaaaagcgggcagcatcagccacgggcaaatgtgggcaatcctgccgcaaacctggctgggtaacctggtcggttccgtcttcgttgccatgctctatagctggggcggcggtagcctgctgccggtagataccagcatcgttcactccgtcgcgctggctaaaaccactgcaccggcaatggtactcttcttcaaaggtgcattgtgtaactggctggtttgcctggcaatctggatggcgctgcgcactgaaggggcggcgaaatttatcgctatctggtggtgtctgctggcatttatcgcgtccggctacgagcactctatcgctaacatgacgctgttcgcgctctcctggttcggcaaccacagcgaagcctacacgctggcgggtattggtcataacctgctgtgggtgacgctgggtaatactttatcaggtgccgtattcatgggattgggttattggtatgctacgccgaaagcgaatcgtccggttgcggacaaatttaatcaaactgaaacggctgccggttaattactaaggggtttttacgtggatcatttgcctatattttgccaattacgcgatcgcgactgtctgattgtcggcggtggtgatgtcgcggaacgcaaagcaaggttgctgttagacgcaggcgctcgcttaacggtgaatgcattagcgtttattccacagttcaccgcatgggcagatgcaggcatgttaaccctcgtcgaagggccatttgatgaaagccttctcgacacctgctggctggcgattgcagcgacggatgatgacgcgcttaaccagcgcgtcagcgaagccgctgaagctcgtcgcatcttctgtaacgtggtcgatgcgccgaaagccgccagctttattatgccgtcgattattgaccgctcaccgctcatggtagcggtctcctctggcggcacctctccggttctggcacgcctgttgcgcgaaaaacttgaatcactgctgccgttacatctgggccaggtagcgaaatacgccgggcaattacgcgggcgagtgaaacaacagttcgccacgatgggtgagcgtcgccgtttctgggagaaattgttcgttaacgaccgcctggcgcagtcgctggcaaacaacgatcagaaagccattactgaaacgaccgaacagttaatcaacgaaccgctcgaccatcgcggtgaagtggtgctggttggtgcaggtccgggcgatgccgggctgctgacactgaaaggactgcaacaaattcagcaggcagatgtggtggtctacgaccgtctggtttctgacgatattatgaatctggtacgccgcgatgcggaccgtgttttcgtcggcaaacgcgcgggataccactgcgtaccccaggaagagattaaccagatcctgctgcgggaagcgcaaaaaggcaaacgcgtggtgcggctgaaaggtggcgatccgtttatttttggccgtggtggcgaagagctggaaacactgtgcaacgcgggtattccgttctcggtggttccgggtattaccgcagcttctggttgctctgcctattcgggtattccactcacgcatcgcgattatgcccagagcgtacgcttaattaccggacacttaaaaaccggtggcgagctggactgggaaaacctggcggcagaaaaacagacgctggtgttctatatggggttgaatcaggccgcgactattcagcaaaagctgattgaacacggaatgccaggcgaaatgccggtggcaattgtcgaaaacggtacggcagtcacgcagcgcgtgattgacggtacgctcacacagctgggagaactggcgcagcaaatgaacagtccatcgctaattattattggtcgggttgttggcctgcgcgataaactgaactggttctccaaccattaatttaacccgggccagagaattctggccttcttaatgactctttttatatattcagcaaataaaacatagccccttaataaatattatctgctaatgggttatattcaccgttacagcgacttacaaaattaagtcattcgctcactgacgccaattaaatattcctgtatcgttcttaacgagcagtctgcttatattcatataatcaatgaatattaattaatatataatacatagggaatgtaaatgaacaaatttattaaagttgcactggtaggtgcagtactggctacgttaactgcatgtactggtcatattgaaaaccgtgataagaactgctcttacgactacctgctgcacccggcaatttctatttctaaaatcattggcggttgcggtcctactgcacagtaagtctctgacagaaatcggctaacaccggtttaattgcccgacgccctctggattttccgagggcgtatttgtttctatgtccttcttgcccccgcccgtaaaaatattttcactttaaattcaatttgataactacatccattagccacagcgcgatcctgtgcgaaattttgtgatcttcctccacattacataacatcatatgttgttatattcatcatgcattgtcatgttaccttttaaatgactgcaaactctcccctacaacgtattggacaagaaaaaggtatcgctatgggaagccaggaactccaacgcaagctcggattttgggccgttcttgcaatcgccgtcgggacaaccgtcggctccggtatttttgtatctgtgggtgaagtggcaaaagcagcgggcacgccgtggcttacggtgctcgcgtttgtcattggcgggttaattgtgatcccgcaaatgtgcgtctatgcggaactatccaccgcttatccggaaaatggcgcagattatgtttatctgaaaaatgccggaagccgaccgctggctttcctctccggctgggccagcttctgggccaacgatgcgccgtcattgtcgattatggcgctggcgattgtcagcaatcttggctttttaacgcctatcgatccgttgctcggtaaatttatcgccgccggattaattatcgcctttatgttgctacacctgcgctccgttgaaggcggcgcagcgtttcagacgctaattaccatcgccaaaattatcccgttcactatcgtcattggccttgggatcttctggtttaaagcggagaattttgccgcccctaccaccactgcgattggcgcaacgggcagctttatggcgctgctggcggggatctctgccaccagttggtcgtataccggcatggcctctatctgttatatgaccggcgaaattaaaaaccccggaaaaaccatgccacgagcgctgattggttcctgtctgctggttctggtgctctacaccctgctggcgctggtgatttccggcctgatgcccttcgacaaactcgccaattctgaaacgccgatttccgacgccctgacctggatccccgcactcggcagcaccgctgggatctttgttgccatcacggcgatgatcgtcattcttggttcgctttccagctgcgtgatgtaccagccgcggctggaatacgcgatggcgaaagacaacctgttctttaaatgcttcggccatgtgcatccgaaatacaacacgccggatgtctccatcatcctgcaaggggcgctggggatcttcttcatcttcgtttccgatctcaccagcctgctgggttatttcaccctggtgatgtgtttcaaaaataccctcaccttcggctccatcatctggtgtcgtaaacgcgacgattacaaaccgctgtggcgtactccggctttcgggctgatgaccaccctcgccattgcgtcaagcctcattctggtcgcctcaacctttgtctgggcaccgattcccggccttatctgcgccgtcatcgttattgctactggtctgcctgcttacgccttctgggcgaagcgtagccgccagctcaacgctttgtcgtaatgttatctggagaaaataaaatgttggatattgataaaagcaccgtggactttctggtcaccgaaaatatggttcaggaagtggaaaaagttctcagccatgacgttccgctggtgcacgccatcgtggaagagatggtgaagcgcgacattgatcgtatttatttcgttgcctgcggatcgccactcaacgcggcgcaaacggcgaaacatctggcggatcgcttttccgatcttcaggtctacgccatttccggctgggagttctgcgataacaccccgtatcgcctcgacgatcgttgcgcagtaattggcgtttctgactacggtaaaaccgaagaggtaatcaaagcgctggagctgggccgggcctgcggcgcactcactgcggcgttcaccaaacgcgcggatagcccgattacctcggcggcggaatttagcattgattatcaggccgactgtatctgggaaattcacctgctgctctgctacagcgtggtgctggagatgatcacccgcctcgcgccgaacgcggaaatcggcaagatcaaaaacgatctcaagcagttgccgaatgcgctcggtcatctggtacgcacctgggaagaaaaaggccgccagcttggtgaactggccagccagtggccgatgatttataccgttgctgcgggtccgctgcgtccgctgggttacaaagaaggcattgtaacgctgatggaatttacctggacgcacggctgcgtgattgagagcggagagttccgccatggcccgctggagattgtcgaaccgggcgttccgttcctgttcctgctcggcaatgatgaaagtcgccacaccaccgaacgcgccattaactttgttaaacagcgtactgacaacgtgatcgtcatcgattacgccgaaatttcgcaagggctgcacccgtggctggcaccgttcctgatgttcgtgccaatggagtggctctgctactacctgtctatttacaaagatcacaacccggatgaacgccgctattacggtggtctggtggaatattaatccctctcccggcccggcaacgggccggatttacgcaaggagttacccgatgaaaacaggtatgtttacctgcggccaccagcggctgcctattgaacacgcatttcgtgatgcaagcgagctgggttacgacggcatcgaaatttggggcggtcgcccgcacgcgttcgcgccggacttaaaagcgggcggcatcaaacaaatcaaggcgctggcgcagacgtatcagatgccgattatcggctatacgccagaaaccaacggctatccgtataacatgatgctgggcgatgaacatatgcgtcgcgaaagcctcgacatgatcaagctggcgatggatatggcaaaagagatgaacgcgggttatacgctgatttccgcggcccacgcgggctatctcacgccacctaatgttatctggggacggctggcagagaacctaagcgaactgtgtgagtacgcggaaaacatcggcatggatctaatcctcgaaccgttaacgccgtatgaatcgaacgtcgtgtgtaatgctaatgatgtgcttcatgcgctggcgctggtgccttcgccgcgcctgttcagcatggtcgacatttgcgcgccgtatgtccaggcggaaccggtgatgagttatttcgacaaactgggcgataaattacgtcatctgcatattgtcgacagcgacggggccagcgacacgcattacattcctggagaaggcaaaatgccgctgcgggaactgatgcgcgatattattgagcggggctatgagggttactgtacggtggagctggtgacgatgtatatgaacgagcccagactctatgcccgccaggcgctggaacgctttcgcgcgctgctgccggaggatgagagatgaaaaccctggcgacaatcggcgataactgcgtcgatatctacccgcaactgaataaagcgttttctggcggtaatgcggtcaatgtggcggtgtactgcactcgctacggcatacagccgggatgcattacctgggtgggtgacgatgactacggcacaaagctgaagcaggatctcgcccgcatgggcgtcgatatcagccatgtccatacgaaacacggcgttaccgcacaaactcaggtggaactgcacgacaatgatcgcgtttttggcgactacaccgaaggcgtgatggccgactttgccctgagtgaagaggattacgcctggctggcgcagtatgacattgtgcacgcggcaatctggggacatgcggaagacgcattcccacagctgcacgctgcgggcaaacttaccgctttcgacttctccgacaagtgggacagcccgctctggcagacactggtgccgcatctcgattttgcctttgcctccgcaccgcaagaagacgaaacgctgcgtctgaagatgaaagcgattgttgcccgtggcgcaggaacagtgattgtcacgctgggtgaaaacggcagcattgcctgggatggcgcgcagttctggcgtcaggctcctgaaccggtgacggttatcgacaccatgggtgccggagattcgttcattgccggattcctttgcggctggtctgcggggatgacattaccgcaggcgatagcgcagggaacggcgtgcgcggcgaaaaccattcagtaccacggtgcctggtaggtataacgttggcgtgagcatcttcacgccaacgtgctgttacttgccggaaaacgaccctataatccgagtaattcattctttatttcagggtcgattatgtcagctacggaccgctactctcatcaactcctctacgctaccgtccgccagcgactgctggatgatatcgcgcagggggtttaccaggccgggcaacagatccctaccgaaaacgagctttgtacacaatataacgtcagccgcattaccattcgcaaagccatcagcgacttagtggcagacggcgtactgatccgctggcagggaaaaggcacctttgtacaaagccagaaagttgaaaacgccctgcttactgtcagtggttttaccgattttggcgtctcacaaggcaaggcgacgaaagagaaagtgatcgaacaggaacgggtcagcgccgcgccgttttgcgaaaagctgaacatccccggaaacagcgaagtgttccatctctgccgggtgatgtatctcgataaagagccgctgtttattgatagttcatggatcccgctgtcgcgttatcctgactttgatgagatttacgtcgaaggaagctccacctatcagttatttcaggagcgttttgacacgcgagtggtcagcgacaaaaagaccatcgatatctttgccgccacccgcccgcaggcaaaatggctgaaatgcgaactgggcgaaccgttgtttcgcatcagcaaaatcgcctttgatcagaatgacaaaccggtgcacgtctccgaactcttctgccgcgccaatcgcatcaccttaactattgataataaaagacattaaccgtaggccggataagatgcgccagcatcgcatccggcgatgctggcgcgttgaattttacatcccgtacgttcccctcaccctaaccctctccccaaaggggcgaggggaccgttcagtacggaatttagcttgacggtgctatccagcattaaatactggcaatactctcacgcaaaatccgcagcaccgtctcttcaccgctgcgattcgggttaatgcgaatcgcacaatgttctgattgtggattcgcctggcgaaacgttccggaaaggcgataaaagagcggcgggatttcatatttcgactctgcacccaccgggtaaggcaaggcaccgcgcttttgcgcctcttccagcactctggcggcaatcggctgatgaaactcgacaatcaacaccttcgactgcgcattagcaatcaccgcgcttttcacttccggcaccgcaccaccgttaagcaaagccagcaaccgttcagatacccctgcctgcaccgcgtgcatcactggcgcaaacaccagaccacgcaatacttccagcgcctgtgcgccctggatctggctaccgccggagtaaagcgtggcgcgaatacggttgataacatcagcatcgccgaccactgcaccaacaccctctggcccaaatagcttgaagcaggaaaatgtcgagacattcgcgccgcattcacagccgattcgagccaccttcatcaccgcatagttgtcatcggttaacgctggaacacctgccgcgcgcaacgttgccagcacatctgccagcacgtagctgtcctgcggctgctggcgcgtatgctgcaccagcgccgcatccggttgttgctcgtcgacgacctgcttcagtgccgacaggtcattgaaatcaacagtaataagcgtcagccccatctgctcaataataacccgtgtcgtcgggtaaacaggcgcgtcatgcaccagaagacgctgccccggtttgagcaaagccgccagcccggcgcgaatcgcgccagtccccgcgccctgcaccagcgccgcagcctgtgcgtgaaatgcatcagccagcacctgttccacacgctgggtaacgcgcggttgattcagtcctggcgttaagcctaaatcaccgccagtaagaaactcgctgccggggaaatggcgacaaatgctatccaccagcgcaaactgcttttgctgcgcctcaataatcgtcaggctttgcagaggaaacgtcttcataggtgccttccttaagccggaacgaacaggccaagccagtaaagaacattcagcagaataccggtgatcattactgccacgaccggtgccgccattttctgtaccggacggcccagggattcgttgaggaagtaaatggcaaccgcgatagagaatccggtataacccgccatcttaattgctgcgaaaatcgaaccgaccagcagcgccacttccatcagcatattcatggcgttacggatgttatccgacgcattacgcaccgacgggtagcgtcccagccatttgccgatcgaacgaagcagcaagacttccgccgaaataaccactgcgcctaataccgctgcaaccatcggattcggcgagagatagtccaccgcataaacaaaggtaaagcccgcaactgcatacacacccgttgctaacgcggtggtggcaatcaacggcacaaaccccagtccgcgcataaattctgccagagccgcctgattaatcagcgtttgcgattgttccggcgttacgcctgcggaatatgctttctccagtgtgaagatcgacacttcactgccagcaaaaatcttcatgctggcaacggcggcaatcaatgctcccacgatggcgatatagggtaagtttttgataatccgtgacgtgcgttcttcaaacaccgaaagcccgctggcatcaatgtcattttcatcacgatgacgcaggtcgtgagttatcgcgatccccagcagcatcaccatgccaataaagatttcgatggattcagggttaagatgtgggaaatagcgcacgactaccacacgggtcatcagtaccaccacggcggcgatcagactttgcttccagccaaactggtagaaaatcgccaccagcgggaacagtgcaaaagctgaaaccaccggcgagcttaattcccccaggctacctaatacatccaccggcagcgcggtcagcagctggtttactggcaacaggcaagtaaggatcaacacgccccagatagcgccaagaccaaacgccatcaggctgtttatcgccaggacgccgaggatatcggtaggaagaaagagtaaccatgcgttgagcagcccggttttcagggtaaaagagatccccaccgaggccacaaaaccaatgctcagaccaaaagcgatactccccgcctcgcgacggttcatatagccttcaatcagttgcggcaggatcgggcggatgccgtcatgaaaaacagccgccgagcgatgcgccagaagcgatgtcatacccgtcaggcacgccaccacgataatctgaatatacagatccatagtcgtgccttttatttcagatggttaatcagcatcggaatcgcgtgttcgacgtgctcaacggaaaggccaaacgccacttttccttcagcgatcattttggcgatatgctcgtctttcgctttaatgcctggtttggcaatggtgcaacttttgttatagcctatcaccgcgatggcaatcgacaatgccgcgcccgcaccggtattacacgcgccgatgtaataatccagttgcccggatttcaccttcattgccgcttccatgtcgttgtgaatgaaaacttcaaaacagccaggagccgtcgcttcaatagtttttttaatctgctcacgctgtaagcctgcaacgccaatctttttcatgagtctgtccttattggaaaaattgagagggattttcacgtaacatcacatccacatcggcctgactgaatcctgactggcgcaattgcggaataaaggtggttagtaaatagtcatagccataaccaccgttggcttttaaatgggagcggcgcgtaatatccatcgacagcatgacgcggttcagcaacccacggtcgcgtagcgcatgaagcatcgcaatacgcttttcgtccgggtagtaactgttcttgccgatggtgtcgaactgcacgtacgcgccgagatcgatcatcttcaaaatgttgtcgaggttgtctttcagatcgcagtgaccaacggtgacgcgcgaaagatcaaccccgtgggcttgtagcaacgccagttgctccagccccatcgtgctgaacgacgtatgcgtggagatcgggcgtccggtctggttatgcgccagcgcagcggcaataaataccttctcttccagcggcgtaatctttccttcgctggtgccgatctccgcgatgatcccggctttcagctccgtgccatcgataccctgttcaatttcatcgaccatctcctgcgccagttcctgcacgctgcgggtcgccacatgttccgggaaaaacgcgtcctggtaataaccggtacaggccaccacgttgatccccgtctcgcgcattacatcaagcataaattgcgcattgcgccccatgtaacggttggtcatctcaatcacattacgcacgccccgggtcatcaggtcgttcatctcctggcaaatgaacgcatactgatcaaggcggcagtccacgttgtttttaaagccggagagatcaatatgcagatgctcatgggcgagggtgtaacccgtcggatcaaaactcatagggtgtctcctgcaaaccggagggaggaaagaaaagagcgaccattttgtggcggtggcgcgcggaaaaattcacacacggtagcccccacatcagaaagcgtggtgcgcacaccgagctgcgtagcgatcatcccttgctgataaaccagcactggcaccacttcgcgggtatggtggctgtgaccaatggtcggatcgttgccgtgatccgccatcacgaccaggcaatcatctggctgcatcgcctcaacaagccgggcaaggttacggtcaacgacctgcaaacgttcggcataacgtgcgacgtcttctgcatgaccagcgaggtcggtttcctgaatgttggtgcaaataaacgccgtcggatgggtgttaaattcgttgagggtgatatccataatccgctggctatccaccagattttgccagctcacgccataaggattgttgacgatatctgccaccttacccaccagcacggttggcacgcctgcttcatacagtttttgtggcacctgcactttttcatcgacgccatagcccatatgcacgacctggaaaccgttgtcataagcgccagaacgcggcgcattgataccaataaagcgcccttctttgctttctgcggcatcgagaatgcgttgactgtcggttaacaggccaccaaatgtaatgacccgaccgacctgtacctgctcacgcacgatacgaccaattttgattgcgtcgtcaaaagagatcacagagagattggcggtaatgttatagacctggcctaaatccgcctcgagattatcgccaatcgcaaccgcctgattgacccacagaaattgcagatcatcgccacggcgctccacctgccagccagcggaaactaatgcctgctcaacacggtcaatcacatcgcgaaaaggcatccgcagcggcggtaacgggcgcgtgcctaaaatttcctgatgccccataaaggtatcgccaccttcatgttgcagctctgccacgccccaggttgcggaatctgacggctgcatatcgcctggcgcataacccaatgcgttgattagccccagcgtctccagcgttggtagctgcaaatgcggcaactggctcaggatgtgaccacatgtattcgctcccgcatcttgcggacgcaccagcgtgacatctttcattgcccctacgccaaagctatcaatcactaacaccacaaatcgcgccattacgcccccagagagtttccaagactgtcataacgaccgacgatttccggttcgccacgatgaataccggacaccagcaccacatcgctacgggtgacaaaaatctgcgtgcgaaaacagagcaccactgcactgcttaccggaaactcgcctgccagcggcagggtgtagtcgatactgctgtcatccacagttttgagattggtttcagtaatcttttgattttctggcgtaaacaccaacgcatgttgcgcatgaccacgacgatagtaaccgccgccgtagcagtagctgtcgccacggaaatgatgggagatttcacttaaccagagcatcgcgatacgttcaggctgatcgccctgctggtttgccggaatagtgcccgtcagcgcatgaccgggttcggcatgagtcacaccgtattgcgccagtaatggcagcgaagtgcagctggtcgctgaaggcgcgttcagttgctcaagtgcaataccagatttcgccagttgatcccgtgcctgtatcagcgtgtgaagattcggtgtcggcaaaacttttccgacagcctcatcccaaagcaggcaagggaaatgggtaagtccggctaaatgcagccctggcagattctggatttcggcgacaatctccggcaacaccttgagggcaaaaccgctctcctggcccggataaagaaaatcatcgtcgctataaactttaagcagcacagactggattcgcccggccttcaccgccgccgcagaaacttcccgcgctttgtcgagagtaaacacggtgatgacgtcggtgccctgttcaacggcgtcagcaacctgatgacaagggatttgtaccagatgcccctgatgcgccacaggcaaaccagcgcggcgcatgactcgcgcctctttgtaatccaccgccacaatgccgctgtagcctaatgccagcaatttttccgccagccacggattacgaccaaactgcttggtcatcagatacagttcaatgccgtaaagccgcgccgtctcaatcagccgcttaccgttttccagtatctgatccacgtcgatcacccagctgtccggggcgatcttgccctgctgccacaggcttagtgcggcggaaatcagcgccgggttctggcgtttcaatgcttctacaaacatcttgttgcctcgtttctgttccttgaattaaatattcatttttttgaatatttaggttgtgcgacgtggatttgtcgggagcttcaaacctcttcgttagcagccatccataatccataaaggttggccagcaaatagccttcttcacacgggttaacttccagtgcgaattccttcaacaacacctgatgcaattgcacaacggcttgccagtggctggattgcgccagttctgccagcaactcgttatccagcggctctatttcttcaccacggcgactgcgcatcagtgcactcgccatatgtgtcatcgccatcgttccttgctcactgcgcaccggcagatggcactctgtttccagtacgttgacgacctgcatcatgcctttgcagatgtccttatcaataacgcctgcctcgcaaagcaggttgagtctggtttccatatcagatgcctttcgtttaataactcggttcctgttccccactcactacccgttgttgatgggcgagcagggcgtgtttatctacaacggcacgcagcagttgttgcattgggtaatcatcgactcgcgtcaggaccacggcttcggtggcctgtaaaaatcgcggatcgtctgtgagcggcgtcgcctctaatcccagcatggtcagttcgttttccgccaccacgttccagatcaccgcatcgacatcgcctttaacaatgcgttgtaaactctcgtgataagagagatcgactcgttccacatcactaccgccaaaaaaaacatcggtcatgattttctgatccgccgaacggttatccagccccacgcgcttcacgtttgcggactcgcctttacggcaaatcaactggtgctcgccaacgtaggtgtgcggccccaactccagcgcgaggcataagcctttttgcgtgagataactttccgccgctagtcgcgaaaccaccgccatgtcatacacgccattaagcagacactccacgcgaatatccgcgccacgcatgtgcgcatagtaaaaaggaatgccatcaaactgggctttcaatccgctcgccaggccttcgtacaaacgggtatagggcaagggcattgcacataccacgttgttgatatccacatgagtcagcaatgctttgttatccatctcgaccagataactgccattgcgcccacggcgttcaatccgtatcgctccgcttgattccagcgttttcaacgcggcctgcgtcaggccaacggatgaacggcattcatttgccagctcatctatggttttcaatcgattaccgcacttttcacccaacaaataacgggccagcgtcgtgatgacgacgccttcttttttgataaacgttcgacgcataataaattttcagtaaattgaatatttatatcttcaggaatttgaagataaggcgcaacagcgagatgtggaaacggcgaggcacttcacattttttcggattattgcaaatgaggataaaaaaaccgggtttccccggtttcagagtgatgataaaagcaaaattgcctgatgcgctacgcttatcaggcctacatttccttgcaatatgtgcattactttgtaggccggataaggcgttcacgccgcatccggcatgaacaaagcgcaatttgccagcaatagtgaattacggcttcgccacaaaaccaatcgcttcgtacaccgcttttagcgtacgggaagcgtgcgcgctggctttttccgcgccatctttcatcacctgttgcaggaaggcttcatcgttgcggaaacggtgatagcgttcctgcaattcagtcagcataccggaaacggcatcagccacttcacctttcagatgaccatacatcttgccttcgaactgtttttccagttctgggatgctctggcccgttaccgctgaaaggatatccaacaggttggaaacgcccgctttgttctgcacatcgtagcgaactaccggcggctcgtcggagtcagtgaccgcacgtttgattttcttcactaccgatttcggatcttccagcaggccgataacgttattgcgattatcgtcagacttggacatcttcttggtcggctccagcagcgacattacgcgcgcgccagatttcggaataaacggctccggcaccttaaagatctcgccatacagcgcgttgaaacgctgggcaatatcgcggctcagttcgaggtgctgtttctggtcttcacccaccggtaccagattagtttgatacagcaggatgtccgctgccatcagcaccggatagtcaaacagaccagcgttgatgttctcggcataacgcgcagatttatctttaaactgcgtcatgcgactcagttcgccgaagtaggtatagcagttcagtgcccagcctaactgtgcatgttccggcacgtgggactgaacaaaaatggtgcttttctcaggatcgataccacaagccagatacaaggccagcgtatccagcgtcgctttacgcagcttctgtgcatcctggcgcacggtgatcgcgtgttggtcaacgatacagtaaatgcaatggtagtcatcctgcatgtttacccactgacgcagcgcacccatgtagttaccaatggtcaattcacctgagggctgtgcgccactaaaaacgatgggcttagtcatttttcgattcctgattttcgctatgcggaagccctaatgcgggcagaaggtcatttatagactgataaattacatcaggctggctgagatcgatagcctcgccgtagttatatccgtaggttaagccaactgatgggcaacctgccgcttttgccgcctgaatatcattgcgtgagtcgccgacaaacagcatctgttgtggggcaattcccatccgctcagccaccagtaacagcgggtccggatgcggttttttgttttgcacatcatcaccaccaatcaccacgctgaagtatttggcgatatctaaggcttcgagcagcggcgcgacgaacggcgtcggtttgttggtgaccaggcctagcggcaggcctttagcctgcaacgcgcccaacgtatcggcaacgtgcgggaacaaaaacgtcccctcttcggcaacctcgccatagtagcgatcgaacagtttacgcagaatacgtacctgttcttctgccggaatgtcgtcatcaacgggcggtttacccattgttttacgctgagtcgcacgttcctgacgcgcccaggtcaatgcgcgctccatcagaacatctgcgccgttaccaatccaggtaataacgcgttcttcacctgcgacgggcaactccagcgcatacagcgccatatctaccgcagcagcaagaccaggagcactgtcgaccagcgtaccatcaagatcaaaagcgacgccgcgaatatcttcaaacttattcatgacttacctttgccagttcactgcgcatttcatcaatgacttttttgtagtctggctggtcgaagattgccgaaccggcgacgaacatatccgcgcccgccgcagcgatttcgccaatgttgttcaccttcacgccaccgtccacttctagtcgaatgtcaaagccagactcgtcgatacggcgacgtacttcgcgcagtttatccagtgtttgaggaatgaaagactgaccgccgaaaccagggttgacggacatcagcaggatcacatccagcttatccatcacgtaatccagatagctcagaggtgtcgccgggttaaataccagacccgctttacagccattttctttaatcagttgcagcgtgcggtcaacatgctcggaggcttctggatgaaaggtaatgatgctggcaccagcggcagcgaaatcaggcacaatgcgatcgacgggtttcaccatcaggtgtacgtcgataggggcggtaatgccatagttacgcaaggatttcagcaccattggcccaatcgtcagattgggaacatagtggttatccatgacgtcaaaatgcacgacatcagcgccagctgccagggcttttgcggtatcttcacccaggcgggcaaaatcagccgacagaattgagggggcaatcaaatactgtttcatccgcttctccttgagaattattttttcgcgggtgaaacgactcctggtttgtacaaagccagcagttcgtccacctttttacgtgtgccgccgttgctgcttatactgcgtcgaactttgacgacatgcaattttgcgcgctgataccactcacgcgttaacatcgtatcgtgattggagatcagcactggaatatggcgctcaaccagaccttcggcgatctccgccagatgcgcttgttgttcaagcgtaaaactgtttgtgtgatacgccgtaaagttggcggtcgcagacagcggtgcataaggcggatcgcaatagacgacggatgcatcatctgcgcgcgccatgctatcggcgtaagactcacaatagaaaaaggcattctgcgctttttcagcgaagtgatacaactctgcttccgggaaatagggttttttgtagcggccgaacggcacgttaaactcaccgcgcagattgtaacgacacaggccgttgtaaccgtagcggttcaaatataaaaacagtaccgcccgacggaacggatcctggcttttgttgaactcttcgcggaactgatagtaaacctcggcgcaatttgtttcgggaacaaacagctcgcgtgcggcctgtacgtactcatcagtacgcatcttcacaatgttatagagactgatcaggtcgctattgatatcggcaaggatataacgagaaaagtcggtgttgagaaacaccgacccggcacctacaaaaggctcaaccagacattcgcccttgggcaaatgccgtttaatatcatcaagcaggggatacttgccccctgcccacttcaaaaaagcgcgatttttcttcatgctgactaactaattacaccttctccggctgtggagaaagctccgacagcatccagcgcttcaggcaactcccgcaacgataaaccattgcgggagataaccttgattacttcagatcggcctgtacctgacgcagcggtttcgcccacgggtttttggcctggacatctgctggcaatgtagataccgcttttttcgcctcttctttcgaagcgtacacgccagaaaccaggacataccacggctgaccattacgcgtcgtttcatagacaacgtagtttttcagattctctttcttcgcccaaccgttcaggttgtcgtagttagaggaactgctcagctgcagagtgtaatggctggacggtgccgatttcaacgaaccaacattacctgcggtcttcgccccagcagcgggtgttgctgtggtttgcgccggggatgccgtctgtactggagccgtagtcgccgtctcttttggtgctggcgtagaagtcgcagccggtgccttcgtgctcgccacaggggcagctggttcagtacgcttcggcgtctgtgctaccggcttcggctccgttttcacggttgcttgcggttttttcggttcaatcaccgcctgctgacgagctgggcgcgtagtggacggacgttcagcggtttgcgttttcgccgtgtcacgcgatgcattgccattgcgaacaggcgcaaccgttgcgggttcagtcggcaacgtggaattgaccgccacattgttcagctgttgctgattttgtggctgggtcagcgcattgttcaggtcaccctgcacttcaacacgttgttgaccatccgttgccaccggggtttgcccttgagtcggcgtagaagagatcggtggcagagaaacatcctgctgagtattttccgcagacgtggttcccggcgctggctgcacgccattcgcctgatcggtcgcattgccagcaagatcaatactcttctcgccagacgcggtttgatcgctggaagtggtcgagggggcttttagcgcagaaccgataccgatgatcaacagcagtagaaccagaatgccgacgcccatcatcatatactgacgagaagcgggtttactggctgcttttttgcgcttacgcggacgacgctctacgcgctcttcatccacggtttcatcttcggattcgtcaatttcttcttcgatttccggttcctcattgcgctctttttgcgcacgagtcggacggcgatcgtcagtgtcatcaagttcaatatcatcaaaattgatctgcggttcgccacgttcagtacgctcagaacgttcagaagattgacgagaacgaccagtacgacgatcgctgggatcgggtttcagctcgtcttctggtttgaattcatccatttaacaccccactaaaaggttaatgcttaccacgttgcaattaacctgaagctaatagaccgcttgataagcggcctgacctttcttgttgttacgctgattgacaatcggcaatggcgttaagaacaagctcgtgcgaaacgccgctgcgaacttcactcttaccaattgccaacggaagaattaagcgcatctctcccgcaaggactttcttgtcacgcagcatatgcggtaaatacgcctgcgcggacatttcgcgcggcccattgaccggtaacccagcccgcttgagcagggttataatacgctgcgtttcggcagaactaaactgcccgagacgttccgacgtccgcgccgccatcaccatacccgcagcgaccgcttcaccatgtaaccaattgccataccccatttcagcttcaatggcatgaccaaaggtgtgtcccagattcagtaaagcacgtaacccggtttcgcgctcgtcggcggcgacaacttctgccttcagttcacaacaacggcgaatacagtacgccattgccggaccgtccagacgcaacaacgcatccagattctcttccagccagttaaaaaacgcaccgtcaagaataatgccgtatttgatgacttctgccagccccgacgctaactcacgcgggggaagcgttttcagacagtcgagatccaccaccactgaagcaggttggtagaacgcgccaatcatgtttttaccgaggggatggttgaccgcagttttgccgccaacggaggaatcgacctgcgacagtaacgtcgtcgggacttgaatgaaacggacaccgcgctgataactcgccgccgcgaagccggtcagatcgcccactacgccgccgccaagcgccaccagcgtagtatcgcgaccatgcggtttttgtaacaacgccgtaaagacggtatcgagtacagccaggcttttatactgctcgccgtcagggaggataacgctatcgacgttaacacccgcctgttcaagtacgccgcggaccttatcgagatacagaggagccagggtttcgttggtgaccaacatgacctgctcgcccgatttcagcggtaagaatgaagctggttcattaaacaaaccagatgcgatggtaattgggtaactacgttccccgagagtaacgacaatcctctccataacgcgacatccaccttaattactgtacccgcagacgagtgtatataaagccagaattagttgctttccagcatgtgaataatctggtttgcaaccactttagcgctttgatcatcagtacgaatggtcacgtcggcaatctcttcatacagcggattgcgttcattggccaacgcttccagaacttcacgcggcggtgtttcaacgtgcagcaacgggcgttttttatcacgctgcgtgcgtgcaagttgcttttcgatggtcgtttcaagataaacgacaacgccacgagcggaaagacggttacgcgtttcacgggatttcacagagccgccgccagtagccagcacaataccctgtttctcggtcaactcattgatgaccttttcttcgcgatcgcggaagccttcttcgccttctaaatcgaaaacccagcccacatcagctccggttcgtttctcaatctcttgatcggaatcgtaaaattccatattgagttgttgagctaactggcgcccaatagtgctttttccggcacccataggcccaaccagaaagatattgcgtttctctgccattttttcggtactactaagactattcgttaatgataaacccgcttcgctcagagagcgccgcaggacatgaactgaaacctcataagatattgcgagagtcagactgaaaattatctcaatactccagcgggtttggcaactgaataaatcacccatccctctgcatatctggtcgctgcaagcgcgctgccttgctaccaccgctctggcgataaatcaccgggtaagattagcgtaaaaaagacagcaaaatgccgcctgaatgataaatcatcatcatggaacgcaggcagcgaagagcaccaactctcaaatcggtactccttgtatgctaaatacctgcgcgcgtcaaatagatgaaacacgttcagcgtaaaaacattaccgcttttacggctgtttactcactggaaaccagtcgtggcgtgataaacaccactaactcgcgtcgttcatcttcttttccgtcatgacgaaataattgcccgaaccagggaatgtcgccaagcaacggtacgctatcctgacccgatttatttttacgggtaaaaatgccgcccagcgccaacgtttctccgcttttgacctcgacctgcgtttcgatctcctgcttatcaatcgccagcacttcgccatcggcctgctgtagcacctgccccggaacgttctggctgatgtgtaatttcagccggatgcgacctttttgtaacaccgtgggcgtgacctccatccccaggacggcctctttaaattccaccgacgtcgcgccactttccccgctggaaacctgatatggaatttcgctcccctgtttaatgctggcaggctgaagatgtgaggccagcagacgcggactggcgataatatccagctgctgtttttgttcgagcgcggaaagctcaagatccagcaagcgtccgttgatgcgcccaatgttaaaaccgacatgcgttgtcgccgtcgctacggagaggtcgctaccaagcgtggtgacttgcccaacgccaccagcgtgttgcgcatcggccagcgtccatttcacgcctaactcacgcaaacttttttcattaatggtgacaatatgcgccgacagctcaacctgcccgaccggcagatccatttgcgctacccactgttcaagcgcgcttaacgccgttttgttatctcgtagcaaaaggcgattggtgcgtttatcgacggtcatactccctttggcactcagtagcttctcccccgctttcgccagttctcccgcgtcggcgtattgcagggttatactgcgattttccagcggcagatttgcctgcgcccgcgcctgctccgcctcctggcgggcgatattgttattctgccaggcaatggaatgcactgagagaatgttgccttcctgccgcgttatcagtccggcgcttttcactacagtttgtagtgcctgcttccagggaacatctgttagatgtaacgacaccgtaccgctgacgtctggcgacacgaccaggttcaacttctcctgttcagccagcgcctgcaacacctgagctaccggaacgtcatccaccatcagcgtcactttttgcggctttgccgcctgtacgccgggtatcagcatcaacagtagtgcggctatccattgcttcatttgtatctccttgccgttgccacaaccattgtggcggttcgcagtttgtcccggtacccagcgttagtacgtctggcgtcagctgtaaaattgtccagccgttttccagcacatcgttttgctgcacccgtcgccatttcttttgcccgtcttttattacaccgatgatgcgctcgcctcgccctaccatcccctgatagcgccactggctaagttcgctaatccggcatagatcttccggcggtttaaaagggtcacgcataccggttaaaaggcacaatgcaatacctgccaacaaccagcgtttaaccctcatgcggcgtctccagttgtagcgtgaacaaaagatcatcaccttccacgcttaacgaaaaacggctcacgctgacgttgcgctctgccagccgtgtaaatgccgacggcactgcttcccacagcgttttcaacgccaactcgcctccctgcgcggatggatgccaggaaaccagttgcgcgccggataactgaaaatccagtggcgaaaagggcagcgttttttcctcgctgaagggagcggtgtctaccaggcgatacagtgcggcccactgctggtgatgacttgcccgtagtcgaattaatgcgtcgcgctcttcatggtgtgtcgatgacagaaaaatgagcgtaactaacatcagcaaccagaatgcccagcaaagctggcggaggcggggtgatgtggcgaaccaccagtcaaagaacatgttcatcgctaaccttccttgttaactgatactcaaattgccagcgtccctgcgcatcctgctgcgtggctccccgctgattgagatgaaaagatgcatcctggcggagtgacgtttctagtgcgtttaacgcggtaatgcttgttgtcagccccttgatctccagcgttccctgctgccagcttatcgttgtcagccaggcgtgctcgggtaaaagcgccgccagtgcttccagcgcagattgccagtcgcgggtaaattgtcgctggcgctgccgttgcgaacgctgttcgcgtaactgctgttgctccagcaaacgtggcttcgttatctgtaagctgcgggcgagttgttgttccgcctgaagcaaaactgcgtctatgcgcgcttcggcgctgcctgtcagacgcagtattagcgttatcccgacggccagcagcagaggcgcaacgaacatcagcaaccagaaacgcagaaaagcggtccggcgttgctgtcgccagggcaaaaaattaattggcgggttcatcagtacgccttcccaagcgccagccccagcgcgatggcaaagtctccacctggcggcggtagcggcggctgacgaacagaaacggcctcccagggatcaaatccgccttcgccacatatcgcgacgctttcgggatcaacggataacgctgccgccagctccttcgcgctagtcatccccaccgccagtttgcgcccccagctatagcgcgtcgcccacagccactgttcgttatcacgccaggccagacattgctgatgagaaggtaaaaaaggcaggaatcgctgtaatgcactggcatccggggtgatcgcgctcacatgaacacgcaacctttctgccagagtaagcagcgttgccagctctttgctttgcgcggcagtcacgttataggcgggactgagtgagtcttcgctgtaatcgaagcgcagggagtccggatccatatccagctcgcgggccatcgtccctgacagccaggccgtttgctcccgctcaccaagggacatcgacgggcgcggaaatgaccgctgtaatgtgcgactggcgggaaacgccaacataatgtgatgacgctgcggcagttcgcgactccacggtaacaacgttttagccagctgctgcgcatcaacaatccgcccatctttgataatgtcgttctccagcggcaaccgccaccagcgttgcaaaaagcattcttttgcgccccgcacgatcgcaaccgctaccgcttcttgctgttgtaaatgcaaaccaatttgccagatcttaaatgccattgtgatgatctccttatcacccgtcactctgacgggtatatcaatgcgtctggcttgcctttatactaccgcgcgtttgtttataaactgcccaaatgaaactaaatgggaaatttccagtgaagttcgtaaagtattttttgatccttgcagtctgttgcattctgctgggagcaggctcgatttatggcctataccgctacatcgagccacaactgccggatgtggcgacattaaaagatgttcgcctgcaaattccgatgcagatttacagcgccgatggcgagctgattgctcaatacggtgagaaacgtcgtattccggttacgttggatcaaatcccaccggagatggtgaaagcctttatcgcgacagaagacagccgcttctacgagcatcacggcgttgacccggtggggatcttccgtgcagcaagcgtggcgctgttctccggtcacgcgtcacaaggggcaagtaccattacccagcagctggcgagaaacttcttcctcagtccagaacgcacgctgatgcgtaagattaaggaagtcttcctcgcgattcgcattgaacagctgctgacgaaagacgagatcctcgagctttatctgaacaagatttaccttggttaccgcgcctatggtgtcggtgctgcggcacaagtctatttcggaaaaacggtcgaccaactgacgctgaacgaaatggcggtgatagccgggctgccgaaagcgccttccaccttcaacccgctctactcgatggatcgtgccgtcgcgcggcgtaacgtcgtgctgtcgcggatgctggatgaagggtatatcacccaacaacagttcgatcagacacgcactgaggcgattaacgctaactatcacgcgccggagattgctttctctgcgccgtacctgagcgaaatggtgcgccaggagatgtataaccgttatggcgaaagtgcctatgaagacggttatcgcatttacaccaccatcacccgcaaagtgcagcaggccgcgcagcaggcggtacgtaataacgtgctggactacgacatgcgccacggctatcgcggcccggcaaatgtgctgtggaaagtgggcgagtcggcgtgggataacaacaagattaccgatacgctgaaggcgctgccaacctatggtccgctgctgcctgccgcagtcaccagcgccaatcctcagcaagcgacggcgatgctggcggacgggtcgaccgtcgcattgagtatggaaggcgttcgctgggcgcgtccttaccgttcggatactcagcaaggaccgacgccgcgtaaagtgaccgatgttctgcaaacgggtcagcaaatctgggttcgtcaggttggcgatgcatggtggctggcacaagtgccggaagtgaactcggcgctggtgtcgatcaatccgcaaaacggtgccgttatggcgctggtcggtggctttgatttcaatcagagcaagtttaaccgcgccacccaggcactgcgtcaggtgggttccaacatcaaaccgttcctctacaccgcggcgatggataaaggtctgacgctggcaagtatgttgaacgatgtgccaatttctcgctgggatgcaagtgccggttctgactggcagccgaagaactcaccaccgcagtatgctggtccaattcgcttacgtcaggggctgggtcagtcgaaaaacgtggtgatggtacgcgcaatgcgggcgatgggcgtcgactacgctgcagaatatctgcaacgcttcggcttcccggcacaaaacattgtccacaccgaatcgctggcgctgggttcagcgtccttcaccccaatgcaggtggcgcgcggctacgcggtcatggcgaacggcggcttcctggtggacccgtggtttatcagcaaaattgaaaacgatcagggcggcgtgattttcgaagcgaaaccgaaagtagcctgcccggaatgcgatattccggtgatttacggtgatacgcagaaatcgaacgtgctggaaaataacgatgttgaagatgtcgctatctcccgcgagcagcagaatgtttctgtaccaatgccgcagctggagcaggcaaatcaggcgttagtggcgaagactggcgcgcaggagtacgcaccgcacgtcatcaacactccgctggcattcctgattaagagtgctttgaacaccaatatctttggtgagccaggctggcagggtactggctggcgtgcaggtcgtgatttgcagcgtcgcgatatcggcgggaaaaccgggaccactaacagttcgaaagatgcgtggttctcgggttacggtccgggcgttgtgacctcggtctggattggctttgatgatcaccgtcgtaatctcggtcatacaacggcttccggagcgattaaagatcagatctcaggttacgaaggcggtgccaagagtgcccagcctgcatgggacgcttatatgaaagccgttcttgaaggtgtgccggagcagccgctgacgccgccaccgggtattgtgacggtgaatatcgatcgcagcaccgggcagttagctaatggtggcaacagccgcgaagagtatttcatcgaaggtacgcagccgacacaacaggcagtgcacgaggtgggaacgaccattatcgataatggcgaggcacaggaattgttctgattaaaaaggcgcttcggcgccttttcagtttgctgacaaagtgcacttgtttatgccggatacggcgtgaacgcgttatccggctaacaaaatcgtgaaaactcaataaattgcagaaaccccataagcctgataaacattgtgcatcaggcaaacttcacgcatttacactcgcccctgccctttcaaccattcgcgcacgaggaacagcgcactgacattgcgcgcttcattgaagtcagggtcttccagcaaatccatcatatgcgccagcggccagcgcacctgtggtagcggctctggctcatcgccttccagtgattccgggtagagatcttgcgctaccacgatattcattttgctggaaaagtaagacggtgccatgctgagcttcttcaaaaaagtcagatcgttcgctccaaatccaacctcttcttttagctcgcggttagcggcttcgtagacgctttcacccggatcaattaatcctttcgaaaaacctaattcgtaggattcagttcccactgcgtattcgcggatcaggatcaggtgatcgtccacaatcggcacaatcatcactgcttcccggttggttggacgcattcgttcataaacacgccgcacgccattgctgaactccagatccacgctctcgacggtaaacagtcgggaacgggctacagtttcaacattcagaatggtgggtttttgtaatgatttgctcatcgtgggatctatgctgtgaaatcagcggttattgtgcgatatcggacacgctttcggcaatgtgaattgcatgttatttacatttatgtaacttaataaataatcgtcctcaaatcaaattaaaagtcaataggttgaaataactccaggaatttgctgatattccgccttcagagggtttgctatgatcagcggttactgtgatgtgcttaatgatgctcaagttaaactccacgcttgccgatagccaaccgcagaatcatgtattgtgtccggtgcgactgaccacgcctgacagactaagtaagatggggaaagcatgagcaccattgtgatttttttagctgctttgctggcctgctcactacttgcgggatggctgataaaagtgcgatccagacggcgtcagctgccctggaccaacgccttcgcggatgcgcaaacgcgtaaactcacacctgaagaacgtagcgccgttgaaaattatcttgagagcctgacgcaggtattacaggtgcctggcccaacgggagccagcgcggcaccgatctctctggcgctgaatgccgaaagcaacaacgtcatgatgctgacacacgctatcacgcgttacggcatctctaccgacgatccgaataaatggcgttactacctcgattcggtagaagtccacctgccccctttctgggaacagtacatcaacgatgagaataccgttgaactgattcataccgattcgctgccgctggttatttcactcaacggtcatacgctgcaggagtacatgcaggaaactcgcagctatgccttgcaacctgttccgtcaacgcaggcgtcgattcgcggggaagagagtgagcaaatcgagctactcaatattcgcaaagaaacgcatgaagaatatgcgctgagtcgtccgcgcgggctgcgtgaagcgttgctgatcgtcgcctccttcctgatgttctttttctgcctgattaccccggatgtatttgttccgtggctggcaggcggcgcgttactgctgctgggcgcaggtctgtgggggctattcgcgcccccggcaaaatcctccctgcgggaaattcattgtctgcgcggtacaccccgtcgttggggattgtttggcgaaaacgatcaggaacagatcaacaatatttcactcggtattatcgacctggtctatcccgcacactggcagccatacattgctcaggatctcggtcaacaaaccgatatcgatatctatctcgaccgccatgtagtgcgtcagggacgatatctttcgctgcatgatgaagtaaaaaactttccgttacagcactggctgcgcagtacgattatcgctgcgggctcgctgctggtgctgtttatgctgttattctggatcccgctggatatgccgctgaaattcactctctcatggatgaaaggcgcgcagaccattgaagccaccagcgtaaaacaactggctgacgctggcgtgcgggtaggcgatacattgcgtattagcggtacgggaatgtgtaatattcgaacttccggaacctggagcgcgaaaaccaattcaccttttttaccgtttgactgctcgcagatcatctggaacgacgcccgctcattgccattaccagaatctgaactggtcaacaaagcgacggcattgactgaagcagttaatcgccagctgcaccctaaaccggaagatgaatctcgcgtcagtgcctcattacgttcagcaattcaaaaatccggcatggtattgcttgatgattttggcgacattgtactgaagacagcggatttatgttctgccaaagatgactgtgtgcgactgaaaaatgcgctggtcaatctcggcaacagtaaagactgggacgcgctggtaaaacgcgccaacgccgggaagctcgatggcgtgaatgtgttattacgcccggtgagtgcggaatcgctggataacctggtggcaacctccaccgcgccgtttatcacgcatgaaacggcgcgagcggcacaatcactaaacagtccggcccccggcggattcctgattgtcagcgacgaaggcagcgattttgttgatcagccctggccttcggcatcactttacgactacccgccgcaagaacagtggaacgctttccagaaactggcacaaatgctgatgcatacgccgtttaacgccgagggtatcgtcacaaaaatcttcactgacgccaatggtacgcagcatattggccttcatccgatcccggatcgttccggcctgtggcgctatctcagcaccacattgctgctactgacgatgctgggtagcgccatttacaatggcgtacaggcctggcgtcgttaccagcgtcatcgcactcgcatgatggagattcaggcctattatgaaagctgcctgaacccgcaactgatcaccccttcagaaagccttatcgaataacacgtttgcgcggcaggttatgctaccctgtcgcgcaaattgcttcactctggagatttccctcatgcatatcaacattgcctggcaggacgtagataccgttctgctggatatggacggcacgttgctcgacctcgccttcgataactatttctggcaaaagctggtgcctgaaacatggggcgcgaaaaacggggttacgccacaggaagcgatggaatatatgcgccagcaatatcacgacgtacagcatacgctaaactggtactgtcttgattactggagtgagcaactgggtctggatatctgtgcgatgaccaccgagatgggaccgcgtgccgtactgcgtgaagataccattccgtttcttgaggcactgaaagccagcggtaagcagcgaattttgctcaccaatgcgcatccgcacaacctggcggtaaaacttgagcataccggtctggacgcacaccttgatttattactttccacccacacatttggttatccgaaagaggatcagcggttatggcatgcggtggccgaagctacgggtctgaaagctgaaagaacgctgtttattgatgacagcgaagcgattctcgatgctgccgcgcaatttggtattcgttactgcctcggcgtgactaatcctgattccgggattgccgagaaacagtatcaacgccatccgtcactgaatgactaccgccgcctgatcccctcgctaatgtgaaggagacgccatgaaagagaaacctgctgttgaggttcgactggataaatggctatgggctgcccgtttttataaaacccgcgcgctggcccgtgaaatgattgaaggcggtaaggtgcattacaacgggcagcgcagcaagccgagcaaaatcgtcgagctgaatgccacgctcactctgcgccagggaaatgacgaacgcacggtgattgtaaaggcgattactgaacagcgtcgccccgccagcgaggcagccttgctgtatgaagagactgcggaaagtgtagagaaacgcgaaaaaatggcgctggcacgtaaacttaatgccttaaccatgccgcacccggaccgacgcccggacaaaaaagagcgccgcgacctgttacgatttaaacacggcgacagtgaataactgtcacctgcaagagagatgattatgccgcaacatgaccaattacatcgctatctgtttgaaaactttgccgtgcgcggcgaactggtaaccgtttcggaaaccctgcaacagatccttgagaaccacgattatccgcagcccgttaaaaacgtgctggcagaactgctggttgcgaccagcctgttaaccgctacgctgaagtttgatggtgatatcaccgtacagctgcagggcgacggtccgatgaatctggcggttattaacggtaacaataaccagcagatgcgcggtgtggcgcgcgtgcagggcgaaattccagaaaatgccgacctgaaaacgctggtcggcaatggttacgtggtgatcaccattaccccgagcgaaggcgaacgctatcagggcgtagttggtctggaaggtgataccctggcggcctgcctggaagattactttatgcgttctgaacagctgccgacgcgcctgtttattcgcaccggcgacgtagacggcaaaccggctgcaggcggtatgttgttgcaggtaatgcctgcgcaaaatgcccagcaggacgactttgaccacctggcgacgctaaccgaaaccatcaaaaccgaagaactgctgaccttaccggcaaacgaagtgttgtggcgtttgtatcacgaagaagaggtgacggtttacgatccgcaggatgtggagttcaaatgcacctgctcgcgtgaacgttgcgccgatgcgctgaaaacgctgcctgatgaagaagttgatagcatcctggcggaagatggcgaaattgacatgcattgtgattactgcggtaaccactatctgttcaatgcgatggatattgctgaaatccgcaacaacgcgtctccggcagatccgcaagttcattaatgagtatgtccggcagagagggctctgccggattttacgactaatacacctgatgcgctttgtcactcattcagattcacattcagcctttcaccatccactacaagatcgcgccacgctttaggcttcgtccccagttttccatccttcgcagctgtgagtaatttttctttcgttatttcgttcggaagtaaactcatatcaagcgcgtcccattcttttctgtctgagtcaaagccatagacaatgactctgtcatcattaaaagcaaacaggatccgctccgcctgaccatcactattcagatcttgctcgaccaggacgcaggcgtctttttcaatacaggtcatcacgttatagcgatcctggattaaggccgaccagaatgtcgcatcaggtttaacagaaccaggggcaattaacacattatcggctaatactttttccgatacctgttgctgaagatgttgctctccatctaacgccatcagcagatcccgcgcgcgtttcgggtctttcataaacccggcatcgcttttcagcgactcaagcgcagcacgtccatagcgaccgctctgctcgagcatgtagatagttacctggtctgacgtgtttttgccgctctgataacgcgccatatggctgttcacgctaatgcgcatactgtccagcaccggcgaattaagaagcaccagtatcaccaacaccaataacgaaaccgcaaggttcactttgccctgaagaacaacgggattttgccctttacgccagacgatgctgacaaaataccccagcgaccacaccagtaacaccagcaccgccagcacgccctgcaagcggtcgacagtccagccgtactgagcgacccgcagccataacgcccaggcggcgacgaacacatacagcggagcaaccagcaaagcggttttaatcaggcaacgcaacggccctgtccagggaagtgacgctttttgcggatcgcggacaatagccattaagatcaattgcaaaaaggccagcgtcaacagcaacccggcggcggagatgtggcgagaaatcgcgctcaggcccgtaaacggcagggtgatgataaacatcagggttagcaatgatactaacggcagcaaccccgtggcgattaacgtgaacaacttttgaatagagtcgattaaacgtgactgtgttcgcgcgaggatcaccgccagcgcggtaaccagacctaacgtgagataaataaaccagtcggttgcaaaaaagagcgtattgaaaaacgtgatgccaacaagtttaaacaactcactccacagtaaaagcaccagccacgtcaagccattggcgagaaaaatcaccagtaatataagtacgttatgccatactgactggtaaaaatagcgatagcggctactgtcattgcggatgcgaaggctttgttgtatccacggtagcaacaacattgccatcaacagcagatagcaaccaaaatcccaaagcgccttttcagctctccaggggttcatgccatcagtttgccacttcagccagccgctcatccccagcgtggcaataaacactagcgccagccatccccaaaggcgcttctgtttaaaagagatcacggagaagagtaaaacggatgaaaacgcgacggtcgcaggcacgccataaacaatccaactgtgattttttccggaaagccaggcgatcagcaggtagcaaaccagaccctgaagtaatccggtagcaatcatcccccagcgtgttgcgggtgaaagttcaacgttatccatgttggttatccagaatcaaaaggtgggttaattatcgcatccgggcagtagtattttgcttttttcagaaaataatcaaaaaaagttagcgtggtgaatcgatactttaccggttgaatttgcatcaatttcattcaggaatgcgattccactcacaatattcccgccatataaaccaagatttaaccttttgagaacattttccacacctaaaatgctatttctgcgataatagcaaccgtttcgtgacaggaatcacggagttttttgtcaaatatgaatttctccagatacgtaaatctatgagccttgtcgcggttaacacccccaaaaagactttactattcaggcaatacatattggctaaggagcagtgaaatgcgcgttaacaatggtttgaccccgcaagaactcgaggcttatggtatcagtgacgtacatgatatcgtttacaacccaagctacgacctgctgtatcaggaagagctcgatccgagcctgacaggttatgagcgcggggtgttaactaatctgggtgccgttgccgtcgataccgggatcttcaccggtcgttcaccaaaagataagtatatcgtccgtgacgataccactcgcgatactttctggtgggcagacaaaggcaaaggtaagaacgacaacaaacctctctctccggaaacctggcagcatctgaaaggcctggtgaccaggcagctttccggcaaacgtctgttcgttgtcgacgctttctgtggtgcgaacccggatactcgtctttccgtccgtttcatcaccgaagtggcctggcaggcgcattttgtcaaaaacatgtttattcgcccgagcgatgaagaactggcaggtttcaaaccagactttatcgttatgaacggcgcgaagtgcactaacccgcagtggaaagaacagggtctcaactccgaaaacttcgtggcgtttaacctgaccgagcgcatgcagctgattggcggcacctggtacggcggcgaaatgaagaaagggatgttctcgatgatgaactacctgctgccgctgaaaggtatcgcttctatgcactgctccgccaacgttggtgagaaaggcgatgttgcggtgttcttcggcctttccggcaccggtaaaaccaccctttccaccgacccgaaacgtcgcctgattggcgatgacgaacacggctgggacgatgacggcgtgtttaacttcgaaggcggctgctacgcaaaaactatcaagctgtcgaaagaagcggaacctgaaatctacaacgctatccgtcgtgatgcgttgctggaaaacgtcaccgtgcgtgaagatggcactatcgactttgatgatggttcaaaaaccgagaacacccgcgtttcttatccgatctatcacatcgataacattgttaagccggtttccaaagcgggccacgcgactaaggttatcttcctgactgctgatgctttcggcgtgttgccgccggtttctcgcctgactgccgatcaaacccagtatcacttcctctctggcttcaccgccaaactggccggtactgagcgtggcatcaccgaaccgacgccaaccttctccgcttgcttcggcgcggcattcctgtcgctgcacccgactcagtacgcagaagtgctggtgaaacgtatgcaggcggcgggcgcgcaggcttatctggttaacactggctggaacggcactggcaaacgtatctcgattaaagatacccgcgccattatcgacgccatcctcaacggttcgctggataatgcagaaaccttcactctgccgatgtttaacctggcgatcccaaccgaactgccgggcgtagacacgaagattctcgatccgcgtaacacctacgcttctccggaacagtggcaggaaaaagccgaaaccctggcgaaactgtttatcgacaacttcgataaatacaccgacacccctgcgggtgccgcgctggtagcggctggtccgaaactgtaatgatttgaagctggagaatatctatccagtatcttatagaaagcaaaacgggaggcaccttcgcctcccgtttatttacccttcttttgtcgtgccctgcgcccgcgttaccggcactggcagccaggcgcgaatggaaagcccgccccgctcgctggtgccaagctccagcatcccgttatggttatccacgatacgctgcacaattgccagccctaatcccgtgccgctaatggtgcgcgcactgtcgccgcggacaaacggctggaacaggtgcttacgttgttccggcgcaattcccggaccgtcatcttccacctggaaccaggcgcgattcggctccgttccgctgctgactttgatccagccattgccataacgggcggcgttgaccaccatattcgccaccgcgcgtttgatcgacagcgggtgcattttcacttcaatgctgccggggtaaagcgcggtttcaatttcccgctcatagccactttcggcagcaatcacctcaccgagtactgcattaagatccgccatttccatcggcatctcctgcccggtgcgcaggtagtcgataaactgctcaatgatggcgttgcactcttcgatatctttattgatcgattctgccagatagccatcctgctcgctcatcatctcagtcgccaggcgaatacgcgtcagcggcgtgcgcaagtcgtgacttacccccgccatcagcagcgtgcggtcatccgccagttgcttaacaccagccgccatatggttaaaggcacgggtaacggaacgcacctccgaagcgccatactcacgcagcggcggcggaataatccctttaccaacctgcaaggctgcgtgttcgagatcgaccaacggtcggttctggatacgaataaacagccacgccccgcctatcgccaatagcataatcgccagcgtatagcggaacagcggagagaaatcgccctgatgaatttcggtcagcggcacgcgtacccagatattgggcgacagccaggttttcagccagacgacaggcgaacttttgttgacctcaacgcgcacttccgtcgggccgcccagttgctgcgccatctgatggcttaagaattcatagtgttgcgcccaacgcagacctgcctcttcggcagcctcgttggagtagagagagatccccagctcacggtagatctcccgacggaaagcgggaggcacaaccaactgcgtgccgtcctccagttgcagtttgtcggtcatcaacatacgcacttcgtacgcgaggactttattaaactgctggaggctcggcaaaatcgcgaagttcagcaccaccagataagtcgtcaccaggctggcgaacagcaaggtgacgatgagcaataacgtacgggcaaatgaacttcgtggcgagaagcgcaatcgcctcatgctttagagccgtccggtacaaagacgtagcccagaccccagacggtctgaatgtaacgcggatgcgctggatcttcttccaccatgcggcgcagacgcgaaatctgcacgtcgatggagcgttccattgcggaatattcacgaccacgggcaaggttcatcagcttatcgcgggagagcggctcacgcggatggctgaccagtgccttcagtaccgcaaactcaccgctggtgagcggcatcggctcgtcttcgcggaacatttcgcgcgtaccgaggttaagtttgaacttaccgaaagcaattaccgcctcttcctgtgacggtgcgcctggcagttcgttcgcctgacgacgcagcaccgcacggatacgggccagcagttcacgcgggttaaacggttttggaatgtagtcgtcagcgccaatctccaggcctacgatacggtccacttcttcccctttcgccgtcaccataatgatcggcatcgggttgctctgactacgaagacgtcggcaaatcgacaagccatcttcaccaggtaacattaaatccagtaccataagatggaaagattcacgagtcagcaggcgatccatctgttctgcattagcgacgcttcgaacctggaagccttgttcggtgagataacgttccagcagcgcacgcaggcgcatgtcgtcatcgaccaccagaatcttgtagttctcttgcattgtttgtactcccaaaggttcgcaacaatttgtaagcgtgtattcttaaaaaagctcacgttcgtcaccagctaaatctggtatgaatttcagcctaaattgttacaaagcatattaaacagcagcttaagtatacaatttattcggcgaaacattattgattctgttgatatgatcacgttatacccaatgtgcgcattatcaaacagacaaagggaatcaacgagatgaaaacgcccctggttacccgggaagggtatgaaaaactcaaacaagagcttaattatctctggcgtgaagaacgcccggaggtcacaaaaaaggtgacctgggccgcaagtctgggcgaccgcagcgaaaatgctgactatcagtataataaaaagcgtctgcgtgaaatcgaccgtcgcgtgcgctatctcactaaatgcctggaaaatctcaaaatcgtcgattactcccctcagcaggaaggcaaagtcttttttggcgcgtgggtggagattgaaaacgacgatggcgtgactcaccgtttccgtattgtcggctacgatgaaatttttggccgtaaagattacatctctatcgattccccgatggcccgcgcattgctgaaaaaagaagtcggcgatctggcggtggtgaatacccctgccggggaagcgagctggtatgttaatgctatcgagtacgtgaaaccgtaaggaagagtcttaacctcctgccgatggctggcatttttgccagccagtccgtataactatcccctgatttttgatccgaaaagatgaactcaaaccatgatgaatgattcgttctgccgcattattgcgggtgaaattcaggcgcgcccggaacaggttgacgctgccgttcgcctgcttgacgaagggaataccgtgccgtttatcgcacgttatcgtaaggaaatcaccggcggtctggatgacacgcagctgcgtaatctggaaacgcgtctgagctatctgcgcgagctggaagagagacgtcaggcgatcctcaagtccatttccgagcaaggcaaactcaccgatgatctggcgaaggccatcaacgccaccctaagcaaaaccgaactcgaagacctctacctgccctacaaacctaaacgccgcacccgcgggcaaatcgccattgaagcagggcttgagccgttggctgacctgctgtggagcgatccgtcacacacgccagaagtcgccgctgcacaatatgtttatgccgataaaggcgtggcagataccaaagccgcgctggatggcgcgcgctatatcctgatggaacggtttgccgaagatgccgcgctgctggcgaaagtgcgtgattatctgtggaagaacgcgcatttggtttctacggtggtgagcggtaaagaagaggaaggggcgaaattccgcgactatttcgatcatcacgaaccgttgtccacggtgccttctcaccgcgcgctggcgatgttccgtgggcgtaacgaaggcgtacttcagctttcgctgaatgccgatccacagttcgatgagccgcccaaagagagctattgcgagcaaatcatcatggatcaccttggcctgcgcctgaacaatgccccggcggatagctggcgcaaaggcgtggtgagctggacgtggcgcatcaaggtgctgatgcatctggaaaccgaactgatgggcaccgtgcgcgaacgtgcggaagatgaagcaatcaacgtctttgcccgtaacctgcacgatctgctgatggcggcccctgccggactgcgtgcaacgatgggcctcgatccgggtctgcgtactggggtaaaagtggcggtggtcgatgccactggcaaactggtggcgaccgacaccatttacccgcacaccggacaggccgcaaaagcagcgatgaccgttgctgcgctgtgtgaaaaacataacgttgaactggtagcgatcggtaacggtacagcttcccgcgaaactgagcgtttctatctcgatgtgcagaagcagttcccgaaagtgaccgcgcagaaagtaatcgtcagcgaagcaggcgcgtcggtttactcggcttccgagctggctgcacaggagttcccggatctcgacgtttcgctgcgtggcgcggtgtctatcgcccgccgtttgcaggatccgctggcggagctggtgaaaatcgatccgaaatctatcggcgtaggtcagtatcagcatgacgtcagccagacgcaactggcccgcaaactggacgcagtagtagaagactgcgtaaacgccgttggcgtcgatctcaacactgcttctgttccgctgttaacccgcgtggcgggcctgacgcgcatgatggcgcaaaacatcgttgcctggcgcgatgagaacggtcagttccagaaccgtcagcaactgttaaaagtgagccgtctggggccgaaagccttcgagcagtgcgcgggcttcttgcgcattaaccacggtgataacccgctggacgcgtctaccgttcacccggaagcctatccggtggtggaacgcattctggcagcaacacagcaggcactgaaagatctgatgggtaacagcagcgaactgcgtaacctgaaagcgtctgactttactgatgagaaattcggtgtgccgacggtaaccgacatcatcaaagagctggaaaaaccgggtcgcgatccgcgtccggaatttaaaaccgctcagtttgccgatggcgtcgagacaatgaacgacctgcaaccgggtatgatcctcgaaggcgcagtgaccaacgtcaccaactttggcgcgtttgtcgatattggcgtgcatcaggacggcctggttcacatctcttcattgtcgaacaagtttgtggaagatccgcataccgtggtgaaagcgggcgacattgtgaaggtgaaagtgctggaagtggatcttcagcgtaaacgtatcgccctgactatgcgcctggatgagcagcctggcgaaaccaacgctcgtcgcggcggcggtaatgaacgcccgcaaaacaaccgcccggcagccaaaccacgcggtcgtgaagcgcagcctgccggtaatagcgcgatgatggatgcgctggcggcggcaatgggcaaaaaacgttaaacgcccgtactggcctacggttcgaatttgcacgaaatcgtagggcagataaggcgttcacgccgcatctggcaacgaacgccttgcctgacataaaagtgccggagaatatctccggcatttttattccacagccaaactcataatatattccggcaatatttatcatttcattaacaactgaaaccttaattaaacattagccagtccgggtaattcactattcgaattatattttcgctgcgatataaccttgagccacatcaacattgagtcagattattattcaaaccaacattcgcacacattttaagtattgctgatagaaaccattctcattatcattgtgttgttgattatttaatctctcctttgttggcaaatcatctggtctcatgtcgctgtcaaacgccccatgaggtagttatccagttaatgagaaacaagtaggcacctatgcaatacactccagatactgcgtggaaaatcactggcttttcccgtgaaatcagcccggcatatcgccaaaaactgctttctcttggcatgttacctggctcctcttttaatgtggtgcgcgtcgctccactcggcgaccccattcatatcgaaacccgtcgtgtgagcctggtattacgcaaaaaagatctggccttattagaagtggaagcggtttcctgttaatacggtgataacaacaatgaaaaaattaaccattggcttaattggtaatccaaattctggcaagacaacgttatttaaccagctcactggctcacgtcagcgtgtaggtaactgggctggcgttaccgtcgaacgtaaagaagggcaattctccaccaccgatcatcaggtcacgctggtggacctgcccggcacctattctctgaccaccatctcatcgcagacctcgctcgatgagcaaatcgcctgtcactacattttgagtggcgacgccgacctgctgattaacgtggtggatgcgtctaaccttgagcgtaacctgtacctgacgctacaactgctggaactcggcattccctgcattgtggcactgaacatgctcgacattgccgagaagcaaaatattcgtattgaaattgatgctctgtcggcgcgtctgggctgtccggtgatcccgctggtttcaacccgtggtcgcggtattgaagcgctcaagctggcgattgatcgctataaagctaacgagaatgtggaactggtgcattacgcacagccgctgctcaacgaagcagattcactggcaaaagtgatgccttccgacatcccgctgaaacaacgtcgctggctgggcctgcaaatgctggaaggcgatatctacagccgcgcctacgccggtgaagcgtcgcagcatctggatgccgccctcgcccgtctgcgtaatgagatggacgatccggcgctgcacattgccgatgcgcgttaccagtgcattgctgccatctgtgatgtggtaagcaacaccctgacggcagaacccagccgtttcaccactgcggtagataaaatcgtgctcaaccgtttcctcggtctgccgattttcctctttgtgatgtacctgatgttcctgctggctatcaacatcggcggggcgttacagccgctgtttgacgtcggctccgtggcgctatttgtgcatggtattcaatggattggctacacgctccacttcccggactggctgactatcttcctcgcccagggcctgggtggcggcattaacaccgtgctgccactggtgccgcagattggcatgatgtacctgttcctctccttccttgaggactccgggtatatggcgcgtgcggcgtttgtgatggaccgtctgatgcaggcgctgggcttgccggggaaatcctttgtgccgctgatcgtcggtttcggttgtaacgtaccgtcggtaatgggtgcacgtacgcttgatgcaccgcgtgaacgtctgatgaccatcatgatggcaccgtttatgtcctgcggcgcgcgtctggctatcttcgcagtattcgcggctgccttcttcgggcagaacggtgcgctggcggtcttctcgctgtatatgctgggtattgtgatggcggtgctgactggcctgatgctcaagtacaccatcatgcgcggtgaagcgacgccgtttgtcatggagttgccggtctatcatgtaccacacgttaaaagcctgattatccagacctggcagcgtctgaaaggcttcgttctgcgtgctggtaaagtgatcatcatcgtcagcattttcctgagcgctttcaacagcttctcgctgagcgggaaaatcgtcgataacatcaacgactcggcgctggcgtccgtcagccgggtgatcaccccggtcttcaagccaattggcgtgcatgaagataactggcaggcaacggttggcctgtttacaggtgccatggcgaaagaagtggtagtgggtacgctcaacaccctctacaccgcagaaaatattcaggacgaagagttcaatccggcagaatttaacctcggtgaagagctgttcagtgcgatagatgaaacctggcagagcctgaaagacaccttcagccttagcgtactgatgaaccccattgaagccagcaaaggcgacggcgaaatgggtaccggggcgatgggcgtgatggatcagaaattcggtagcgcagcagcagcttacagctacctgattttcgtcctgctgtatgtaccatgtatctcggtgatgggggctatcgcccgtgaatcaagccgtggctggatgggcttctccatcctgtgggggctgaatatcgcttactcactggcaacattgttctatcaggtcgccagctacagtcagcatccaacttacagcctggtgtgcattctggcggttatcctgtttaacatcgtggttatcggtctgctgcgccgcgcgcgtagccgggtggatatcgaactgctggcaacccgcaagtcggtaagcagttgctgcgcagccagcaccaccggtgattgccattaatggcttcacttattcaggtgcgcgatttgctggcgttacggggccgtatggaagcggcccagataagccagacattgaacactccacagccaatgattaacgccatgctgcaacaactggaaagtatgggcaaagccgtgcggattcaggaagaacctgacggctgcctctctggcagttgtaaaagctgcccggaaggaaaagcctgtctgcgcgagtggtgggcgctgcgttaaccttactccatcgcctgttttggaaagcccggtatgcgtctgcatccgggcttttttgcgtgcggctttccataaaaatgcaactcttgcagcacggcgtaagttcctttgaaagcatctcgcagggatgaaaactcgctaatacacaggtgtggagtggcgcgtagagtcgcggcattcaaacaacaggtgaaggaacgccatgagcaaaaagcagagttccaccccacacgatgcgctgttcaaactctttttacgccaaccggacacggctcgtgattttcttgcgtttcatttaccggcacccattcacgcgctttgtgatatgaaaaccctcaagctggagtcgagcagctttattgatgacgatctgcgtgaaagctattccgatgtgctgtggtcggtgaaaacggaacaaggaccaggatacatctattgtctgattgaacatcaaagcacctcaaacaaactgatcgcatttcgcatgatgcgttacgctattgccgcaatgcaaaatcaccttgatgctggatacaaaacgttgccgatggtggtgccattgttgttttaccacggtattgaaagcccctatccctattcgctgtgttggctggattgtttcgccgatcccaaactggcaaggcagctttatgcctccgcatttccgctgattgatgtcaccgtcatgcctgatgatgaaatcatgcagcaccgacgtatggcgctgctggagttaattcaaaaacatattcgtcaacgcgacctgatggggctggtagagcaaatggcctgcttattaagtagtggatacgctaatgacagacaaatcaaagggctgtttaattacatactgcaaactggcgacgctgtacgttttaacgattttatcgacggcgttgccgaacgttcaccgaaacacaaggagagtttaatgactattgcggaaagattgcggcaggagggggaacaatccaaagccctgcatatagccaaaataatgcttgaatccggagttcctcttgcagacatcatgcgctttaccgggctgtcagaagaagagttggctgcggcgagtcagtaaagttctgtctcgccatttcaaaagccacctacaccctctgcttcaacgccaccagcaggtgacaaaactcggccggatgcgaaataaatggcgcatgggccgctttggcgaagatatatgattcgctgtgaggccaaagtttatccagcatcggcaccactttgcgcggcaccagaccgtcgagatagccatacaatcgcaaaaacggcatggacacgttttgcagcggctgacggagatcgaccgttttcaggatttccagcccgccattaagcacgtcaacctccggcatcggtaacgccagaacggttttcttcaacgcccgcgcatcctggcgcgccgtttcagtccccatggtttgtaacgccaggaaccgctccactgtacgctgaaaatcatcactgagttgctgctgaaatcccgccagcacgtccggttttatccccggccactcgtcacgagcactaaaacaaggtgacgacgccacggtgaccagcgcctgaacacgctcgggatgggttaacgcaatctggcttgccaccagcccgcccagactccagcctaaccaaatggctttatcaggtgcctgttgcagcacggcttcggccatatcagcaagtgacagcgcaccaaatccccggctacgcccgaagccgggcaggtcaacaaggtgcagcgtaaaatgcgagctaagttcctcgtcaatgcaacgccacacttcggcattcagtccccatccgtgcagcagcacaagatgaacattcccctgacctttggtctgccaccagatgttattcatccgctattgttctcttttgacttacaaggatgaacatatgctaacagtaccgggattatgctggctatgccgaatgccactggcgttaggtcattgggggatttgttcggtctgttcacgcgccacccgcacagataaaacgttatgcccacaatgtggattacccgccacacactcccatcttccctgcggtcgctgcctgcaaaaaccgccgccctggcaaagactggtcacggttgccgactatgcgccgccgttaagtccgcttatccaccagcttaaattttcccggcgcagtgaaatcgccagcgccctgtcacgtctgttactattggaagtcttacacgctcgtcgcaccaccgggttgcaattgccggatcgcatcgtcagcgttccgttatggcagcggcgtcactggcgtcggggatttaatcagagcgatttgctgtgtcagccgttatcacgctggttgcactgccaatgggatagcgaagccgtcacacgtacacgggccactgcgacccagcattttctcagtgcccggctgcgcaagcgcaacctgaaaaatgcctttcgtcttgaattgcccgtgcaaggtcgccatatggtgattgtggatgatgtcgttaccaccggaagtaccgtcgcagagattgcgcagttgcttttacgcaatggtgcggcggctgtccaggtctggtgcctttgtcgaaccttgtagagcctcgatgatgggcgtattataaccaactaaaatagtcaactattaggccattactatgatccgtatttccgatgctgcacaagcgcactttgccaaactgctggcaaatcaggaagaagggacacaaatccgcgtatttgtgattaaccctggcacgcctaacgctgaatgtggcgtttcttattgtccgccggacgctgtggaagccaccgacacagccctgaaatttgacctgctgaccgcgtatgttgatgagttaagcgcaccatacctggaagatgcagagatcgattttgttaccgaccagttgggttcccagttaacgctgaaagccccgaacgccaaaatgcgtaaagtggcagacgatgcaccgctgatggagcgcgtggagtatatgctgcagtcgcagatcaacccacagcttgctggtcacggtggtcgcgtttcgctgatggaaatcaccgaagacggttacgccattctgcaatttggcggcggctgtaacggttgttccatggtcgatgtgacgctgaaagaagggatcgagaagcagctgctgaacgaattcccggagctgaaaggtgtgcgcgatctcaccgaacaccagcgcggcgaacactcctactactaagttatcccctcttttgtagattgcccgatgcgacgctaaagcgtcatttcgggcctacgttgaacatgtgccagacgttggcgcagcattgctttgtcaaatcctcggttcgtttccccgcgataatatgaccaacctctcataatttaaatttaccccgctctggtgattctcaaacgccagatgttacccgtatcattcacatgggtaccaaacatactcctgacatctgactacaataattagttttagtgggtatcagtcgtggtgccgcaatatctctgttcccgattgggataattagagtttgtcgtcagaaaattgacgttacccataacaaatgaaaggccaggtaaatcatgccattagtcattgttgctatcggtgtaatcttgttgttgctcctgatgatccgcttcaaaatgaacggcttcatcgctctcgtcctcgtggcgcttgctgttggattaatgcaaggaatgccgctggataaagttattggctccatcaaagccggtgtcggcgggacgctcggtagccttgccctgatcatgggttttggcgcaatgctgggcaaaatgctggcagactgcggtggcgcacaacgtatcgccaccacgctgattgccaaatttggtaaaaaacacatccagtgggcggtggtactgaccggttttaccgttggttttgccctgttctatgaagtgggctttgtgctgatgctgccgctggtgtttaccatcgcggcttctgcgaatattccactgctgtatgttggtgtaccaatggcggctgcactgtctgtgacccacggcttcctgccaccgcatccgggtccgactgcgattgccaccattttcaatgccgatatgggtaaaaccctgctgtacggtactattctggcaatcccgaccgtgattctcgccggtccggtttacgctcgcgtgttgaaaggtatcgataagccaattccggaaggtctctacagcgcgaaaaccttcagcgaagaagagatgccgagctttggcgtcagcgtctggacctctctggtgccggtagtactgatggcgatgcgtgcgattgccgaaatgatcctgccgaaaggtcacgctttcctgccggtagcggagttcctcggtgacccggtaatggcaacgctgattgccgtgctgattgcgatgttcacctttggtctaaaccgtggtcgttcaatggatcagattaacgacacgctggtttcttccatcaaaatcattgcgatgatgctgttgatcatcggtggtggcggtgcgttcaagcaggtgctggtagacagcggcgtggacaaatacattgcttccatgatgcacgaaaccaacatttctccgctgctgatggcctggtcgattgctgccgtactgcgtatcgcgctgggttccgcaaccgttgcggcaatcactgcgggtggtatcgcggcaccgctgattgcaacgacgggtgttagcccggagctgatggttattgcggttggttccggtagtgtgattttctctcatgtgaacgatccgggcttctggctgttcaaagagtactttaacctgactatcggcgagaccatcaaatcctggtcgatgctggaaaccattatctcggtgtgcggtctggtaggctgtctgctgctgaatatggtgatttgataacactgactgccggatgcggcgtgaccgccttatccggcctacgattcgggatgaattagtaggccggataagacgcgtcaagcatcgcatccggcatcaaccgcactctacttcttcttcgctgcagctctgcgccgtctgtccaaatccttcagcaacttgttcacgccatcatcggcaaacatcgactcaagcgttgcggaaagcttgcgtcgccagtttttatactggtaactggtgccaggaatattcaccggttcggccatatccagccagtcttccggctgtagtcctaacagagcactgttactgtcggcaatgtagcgctgcaaaccacggttcagcgtcggcgtcatcgacatcaacgatgccttatgcccggcacgtttcggcagacaaccatatttatgcagtgcatccagcagcccttgcttcgccagttcgcgatcctgatacagaccgcgcagtaccacttcatccggatacagccccagggttttgcccagcgttagatccccgcactcccagtaaccgcgcagcgttggcaggtcatgtgtcgccgcaaccgccatcgactgctccggatacgctttcggtgcacggaacgtcttctcgtggtcgttttcgaaatagagcactttgtaagagtacacaccgctgctgcgcagcttaccgacaatctctaccggtacggtaccgagatcttcaccaatcaccatacagcgatgacgtttactttcgagtgccagaatcgagagcagatcatccaccggatagtgaacatacgcgccctgatctgccgtctcgccatacggtatccaccacaaacgcagcatcgacatcacatggtcaattcgtaatgcgccgcagttttgcatattggcacgcaacagctcgataaacggttcataggcacgcgcggtgatgatatgcgggtccattggcggtaatccccagttctgccccaacgggccgaggatatccggcggcgcgccaaccgatgctttcaggcaatatagttcacggtcacaccaggtttccgccccaccttccgctacgccaaccgccagatcacgatacaagccaatcggcatttcatagccctggcttatctcccagcaggcggcaaactggctgtaagccagccactgcaaccagagataaaaatcgacgtcatcacgatgttcttcgcagaactgacgcacttctggtgaatccacgttctgatacatctctggccatgcaggccagccccagcgcatttcgtcctctttcacttgctgggcatgtagcgcatcaaaggctgcctgccagaacaggctgtcgccctgctctgcaacaaactggcgaaacgcggccatctgctcatcatcacgttgcgcgaaacctttccacgccattcgtaatgctgtcatttttagggcggtaaccgtggagtaatcgacccagtcggcatcgcgcgcctgttgcagcgtctgttgcgtggtcggcaactgccaccaggcctgagcctcttcgctaagatggaaatcttcaacggcgttaacgtcgatataaatcacattcagccaacggcgagaagacgggctgtatgggctggcgctctccggatttgccggatagagcgcatgaatcgggttcaggccaatgaacgacccgccacgttttgccacatccaccagcatcgctttgagatcgccaaaatccccaataccccagtttttttccgatcgcagcgtataaagctgaacgcaggcaccccacagcttttgtttattcagcaacgcctgcggttcgtaacagcgtttcggggcgacaatcacccggcaatgcgcgcgctggtcgtcctgggtgagtgtcagcgtgtgataaccttccggcagcttcgtcggtagattgaacgctttgccccccgttacatggcctttgtactgcgttccttcttcggtggtcagcagccagctatattcgccgctgccctccaccaccatcggcatttttttgccgctggtataaaccatgacattcgggactggcgttaccgccactttcgtggcggtacgttgatgcatcgcgtcaagcaaacgccgtttggtttcggcgctaatcgactgcggtttaccgtgggcattgatgtaattggggctaatccccgccgccagcgcggcattatccagacgtttgctttccatcgagcttccttagcgttttgcctgccagatacgagcctgataatcgcgaatagagcgatccgagctaaacataccgcagcgggcggtattgaggatcgccgcgcgagtccaggcctcctggtcgcggtacagcacatccacctgcttttgtgcctctacataggctgcgaaatccgccatcaccagatacggatcgccgccctgtttgccgatactgtgcagcatctggtcgaaggcatgcttatcgccgtcgctgtatttaccgctttccagctctttcaatactgcgtccagcaccttatctttcttccgccatttcaccgggtcgtagcctttggccagaattgccttcacttgttccacggtatgaccaaaaataaagatattttcttcaccgactttctcggcgatttcaacgttcgccccatccagcgtaccgacagtaagcgcaccattgagcgccagtttcatattgccggtaccggaagcttctttacctgcagtcgaaatttgttcggagatatccgccgccgggatcagtttttccgccgccgaaacgcaataatccggcaggaacaccaccttcaacttatcgccaaccagcggatcgttgttgatcacgtcagccactttgttgatcgcaaagataatattcttcgccaggtagtagcccggtgccgctttcgcgccgaagaggaagacgcgcggtacgcgatcagcctgcgggttttcacgaatttctttgtacaacgccagaatatgcagcagattcaggtgctggcgtttgtactcatgcaaacgtttgatctgaatatcgaaaatcgcctgtggattgatctcaataccggtacgaactttcacaaactccgccagacggactttattcgcctgcttgatctcgcgatattgctgacggaatttcgcatcatcagcgaatttttccagattgatcagctgatcgagatcgttagcccactctttttgcagtgatttatccaacagagccgccagtgccgggttgcactgtttgatccagcgacgtggggtaataccgttggtgacgttatggaatttgttcggccatagctggtgatattccgggaacagatctttcaccaccagatccgagtgcagcgccgcaacaccgttcaccgcgaaaccgccaaccacacacaggttcgccatatgcacttgtttgtcgtgcaccaccgccagtttggcccacactttttcatcgcccggccaggttttctctaccagcgttttaaagcgagtattaatttcgttaataatctgcatgtggcgcggcagtaagcctttcaccagtttcacatcccagcgttccagcgcttctggcatcagggtatggttggtgtaagcgaaagttttgctggtaatggcccaggcgtcatcccagctcatctggtgctcatcgatcagcacgcgcagcagttctggaatcgcgatagttgggtgggtatcgttcagctgaataacttcgtaatccgccagttcgtgcagtttacgccccgccagatgatggcgacgcaaaatatccgctaccgaacaggcacactggaagtattgctgcatcaggcgcagctttttaccggcagtatggttgtcgtttggatagagaactttggtcagtttttccgcattgatgccctgctgttcggcacgcaagaaatcaccgtcgttaaatttagtcagatcaaacggatgcgcgtgcgtcgcctgccacagacgcagcggctgcgccacgccattacgatagccgacaacggggagatcccacgcttgaccggtaatggtaaactccggctcccagcgtccgtctttcgtcactttaccgccaatccctacctgcacatccagtgcttcgttgtggcggaaccacgggtagttactgcgatgccagtcatccggcgcttcaacctgtttgccatcgacaaaagactggcggaacaaaccatattgatagttcagaccgtaacccgtcgcagactgaccgacagttgccattgagtcgaggaagcacgccgccagacgtcccagaccaccgttacccagcgccgggtcgatctcttcttccagcaggtccgtcagattgatgtcataagccttcaacgaatcctgtacatcctgataccagccgagattcaacaggttgttgcccgtcaggcgaccaatcaaaaactccattgagatgtagttaacatgtcgctgattcgccaccggcttggcgaatggctgagcacgcagcatttcggccagtgcttcactcactgctagccaccactggcgaggagtcatttcagccgcagaatttaagccataacgctgccactgacgtgaaagcgcttcctgaaattgcttatcgttaaaaataggttgtgacataggagttccacttttcttagattttcaacacaacgttatcgctagtttgccaggctcgatgttgaccttcctcatcctgcgggggattaggcagggaggagttgcggggatgagcaaggaaatgtgatctcaaccacttaaagctagtgcaaaccacaggattagcatcaaatcaatgcaatacagcgcagaaaatctgtatctaagtgcaaaaaatggccgttgcgtattttcaaaaagcggaaggtaactctataaattaagtaaaggagtgaaacagtttcataagtaaaatatccagtgtgctccatctcattcttaatagatttattaagatcatctttttagatggcactttcatcaggaatgaagaagaaacccttgcttaaatgaatctgatgaacataagggaaaccagtattcacgctggatcagcgtcgttttaggtgagttgttaataaagatttggaattgtgacacagtgcaaattcagacacataaaaaaacgtcatcgcttgcattagaaaggtttctggccgaccttataaccattaattacgaagcgcaaaaaaaataatatttcctcattttccacagtgaagtgattaactatgctgattccgtcaaaactaagtcgtccggttcgactcgaccataccgtggttcgtgagcgcctgctggctaaactttccggcgcgaacaacttccggctggcgctgatcacgagtcctgcgggctacggaaagaccaccctcatttcccagtgggcggcaggcaaaaacgatatcggctggtactcgctggatgaaggtgataaccagcaagagcgtttcgccagctatctcattgccgccgtgcagcaggcaaccaacggtcactgtgcgatatgtgagacgatggcgcaaaaacggcaatatgccagcctgacgtcactcttcgcccagcttttcattgagctggcggaatggcatagcccactttatctggtcatcgatgactatcatctgatcactaatccagtgatccacgagtcaatgcgcttctttattcgccatcaaccagaaaatctcaccctggtggtgttgtcacgcaaccttccgcaactgggcattgccaatctgcgtgttcgtgatcaactgctggaaattggcagtcagcaactggcatttacccatcaggaagcgaagcagttttttgattgccgtctgtcatcgccgattgaagccgcagaaagcagtcggatttgcgatgacgtttccggttgggcgacggcactacagctaatcgccctctccgcccggcagaatacccactcagcccataagtcggcacgccgcctggcgggaatcaatgccagccatctttcggattatctggtcgatgaggttttggataacgtcgatctcgcaacgcgccattttctgttgaaaagcgccattttgcgctcaatgaacgatgccctcatcacccgtgtgaccggcgaagaaaacgggcaaatgcgcctcgaagagattgagcgtcaggggctgtttttacagcggatggatgataccggcgagtggttctgctatcacccgctgtttggtaacttcctgcgccagcgctgccagtgggaactggcggcggagctgccggaaatccaccgtgccgccgcagaaagctggatggcccagggatttcccagcgaagcaattcatcatgcgctggcggcaggcgatgcgctgatgctgcgcgatattctgcttaatcacgcctggagtctgttcaaccatagcgaactgtcgctgctggaagagtcgcttaaggccctgccgtgggacagcttgctggaaaatccgcagttggtgttattgcaggcgtggctgatgcaaagccaacatcgctacggcgaagttaacaccctgctagcccgtgctgaacatgaaatcaaggacatcagagaagacaccatgcacgcagaatttaacgctctgcgcgcccaggtggcgattaacgatggtaatccggatgaagcggaacggctggcaaaactggcactggaagagctgccgccgggctggttctatagccgcattgtggcaacctcggtgctgggtgaagtgctgcactgcaaaggcgaattgacccgctcactggcgctaatgcagcaaaccgaacagatggcacgccagcacgatgtctggcactacgctttgtggagtttaatccagcaaagtgaaattctgtttgcccaagggttcctgcaaaccgcgtgggaaacgcaggaaaaagcattccagctgatcaacgagcagcatctggaacagctgccaatgcatgagtttctggtgcgcattcgtgcgcagctgttatgggcctgggcgcggctggatgaagccgaagcgtcggcgcgtagcgggattgaagtcttgtcgtcttatcagccacagcaacagcttcagtgcctggcaatgttgattcaatgctcgctggcccgtggtgatttagataacgcccgtagccagctgaaccgtctggaaaacctgctggggaatggcaaatatcacagcgactggatctctaacgccaacaaagtccgggtgatttactggcaaatgaccggcgataaagccgccgctgccaactggttgcgtcatacggctaaaccagagtttgcgaacaaccacttcctgcaaggtcaatggcgcaacattgcccgtgcacaaatcttgctgggcgagtttgaaccggcagaaattgttctcgaagaactcaatgaaaatgcccggagtctgcggttgatgagcgatctcaaccgtaacctgttgctgcttaatcaactgtactggcaggccggacgtaaaagtgacgcccagcgcgtgttgctggacgcattaaaactggcgaatcgcaccggatttatcagccattttgtcatcgaaggcgaagcgatggcgcaacaactgcgtcagctgattcagcttaatacgctgccggaactggaacagcatcgcgcgcagcgtattctgcgagaaatcaatcaacatcatcggcataaattcgcccatttcgatgagaatttcgttgaacgtctgctaaatcatcctgaagtacctgaactgatccgcaccagcccgctgacgcaacgtgaatggcaggtactggggctgatctactctggttacagcaatgagcaaattgccggagaactggaagtcgcggcaaccaccatcaaaacgcatatccgcaatctgtatcagaaactcggcgtggcccatcgccaggatgcggtacaacacgcccagcaattgctgaagatgatggggtacggcgtgtaagtttagccggataacgcgccagatccggcttacatctctgcatcattcaatgctcacccgcgttacgccatctgtttctatcaaactaaaccgcaccggcaagaaacgctccaccaccgcgatattggtcagcagatggcatgagggatgggcgaccgtaaattcccccgcgcccgccagcgccatcggtagcaccagttggtcagcaagatattcccccaccgccgccgtgcttgccaggtagcgtttcacctctttcaccaactgtgccgcaaccacctcggcactgacgcgcttttcaccgacgacaaaaaagcgttcggtgatattttcactttcgacttcaagcgagacggtattacccggcccctggtcgcgcggcaggttatgaatattctgttcatgcagggaaaaactccccgccagtgtagcgatttcacgctcagcaacatggcgcggcacaccagctaatagaacttctccacgcatctgcacaatgttcccgcgctcgccaagttgcaaggtgttaaacgatgccacgggcgagacttccgttgccaccacaccgcctccggcagggtaaaaaccgtggcgtaacagcgtggtttgctgatgaattcctattttcgccagcagcggctccagcacccggcggataaaatccgcaggcggcgccgacgggttatcggtgccgccgctcacttcaacacgcgaaggtccatcggcaaaccacagcgcgggcagcaccgtttgcagcaccagcgtacaacttccggcgctaccgatagcaaagcggtaatcgccgccgcgcacggtgccgggccggaagagcagacgctgcgaccccagctccgcgccttccacggttgctccgcaaatttccgtcgccgcctttaccgcggtcagatgctggcgcaacagccccggtttcgcccgcccggcacgaatgctggtgatggtaaatggctggccggttatcatcgacaggctcagcgccgagcgcaggatctgcccgccaccttcgccctgtgcgccatccagcgcaatcatccttttcatcatttatccttttacgcacaccacctgacgcagggtatagataacttccaccagatcgctttgtgccgccatcaccgcatcaatatctttatacgccatcgggatttcgtcgatcacttcggcatctttacggcattccacatgcgcggtggcacgaatttgatcttccacgctgaacagttttttcgctttagttcggctcattacccgcccggcaccgtggctgcacgaacagaacgactcttcatttcccagcccacggacgataaagctttttgctcccatcgaaccgggaataattccatattgaccagcacgcgcagacaccgcgcctttacgcgtcacgtagatctcttcaccaaagtgctgttctttttgcacatagttgtggtgacagttgatctcttccatcgccagcgtttgtggctgtctgaccgttttctgcgtaatgctctgcaatgccgttaccacgttttccatcatcgcatcgcggttaaggctggcaaaaagctgcgcccaggccacggctttcaggtaatcatcaaagtattccgtaccttccataaagtacgccagatcacgcgacggcaacgtctcaagcgtttcctgcatctctttttgtgccagatcgataaagtaagtcccgatggcgttaccaattccgcgtgaaccggagtgcagcataatccacacctggtccgactcatcaaggcagatttcaataaagtggttaccggttcccagcgttcccaggtgtttatagttattggtattcaggaaacggggatatttttgcgttaaccactgataaccggcttcaagctcagcccatttagcatcgacgttaacaggtggattttcccaggcacctttatcacgtttacaacggccagtggtacgcccgtgcggcacggccgtttcaatcgcctgacgcagctctgccaggttttcaggcaggtcttccgccgttaacgcggtacgcagcgcgttcattccacagccaatatccacgcccaccgccgccggaataatcgcccctttggtcgggatcacgctaccaatggtggaacctttacccaggtgtacatcaggcattaccgcaatatgtttgaaaataaacggcatcttcgccgtattaataagttgctgacgcgcatcggcctctaccggcacgcctttggtccacatttttaccggggcattttcagtggtcagtaattcgtaattcattttgtttttctcttttcgttgtttgctgtcctgataattgcaaccgtcgtgccagaaaattaaataagcagcttaattttttaattcattgttttaaaaaagattatatctttacgtccgtaaccggagatttcccgcaaagccaatttaccgataatgaaatatcgtcttttataaggatatctaagatgcgtaaaacagtggcttttggctttgtcggtaccgtactggattatgccgggcgcggcagtcagcgctggtcaaaatggcgtccgacactctgtttatgccagcaagaatcgttggtcatcgatcgactggaattgttgcacgacgcccgctcgcgctcgctatttgaaacgcttaaacgcgatatcgccagcgtttcgccagaaacagaagtggtgagcgttgagattgaactgcataacccgtgggatttcgaagaggtctacgcctgcctgcatgatttcgcccgtggttacgagtttcagccagaaaaagaagactatttaattcacatcaccaccggtacccacgtcgcgcagatttgctggtttctgctggcagaagcgcgttacctgcccgcccggctgatacaatcttcacctccgcgcaaaaaagaacagccgcgcggcccaggtgaagtaacgattatcgatctcgatttaagccgttataacgccatcgccagccgctttgccgaggaacgccagcaaacgcttgattttcttaagtccggcattgccacgcgtaacccccacttcaaccgcatgattgagcagatcgaaaaagtggcgatcaaatcccgcgcgccgattctgcttaacggtccaaccggcgcgggcaagtcatttctggcgcgacgcatcttagagttaaaacaggcgcggcatcagtttagcggcgcgtttgtggaagtgaactgcgccaccctgcgcggcgataccgccatgtcgacgctgtttggtcatgtaaaaggcgcgtttaccggggcgcgggaatctcgtgaaggtttattacgcagcgccaacggcggaatgttgtttcttgatgagattggcgaactgggcgcagacgaacaggcaatgctgctgaaagccattgaagagaaaaccttttacccgtttggcagcgatcgccaggtgagcagtgattttcagcttatcgccggaacggtgcgcgatttgcgccagctggttgccgaaggcaaatttcgcgaagatctgtacgcgcggatcaatctctggaccttcaccctgccgggtctacgccagcgccaggaagatattgaaccgaacctggattatgaagtggagcgccacgcctcactcactggcgacagcgtgcgttttaacaccgaagcgcggcgcgcctggttggcttttgcgacctctccccaggcaacatggcgcggtaactttcgcgaactttctgccagcgtcacgcggatggccacctttgccactagcggacgcatcactctggacgtggttgaagatgagataaaccgtctgcgctataactggcaggagagccgcccctccgcgcttacggcgttgctgggcgcagaggcagaaaacatcgatctcttcgaccgtatgcaactggaacacgttatcgctatctgccgccaggcaaagtcgctttccgcagccggacgccagctttttgacgtttcgcgccagggcaaagccagcgtcaatgacgcggatcggctacgcaaatacctggcgcgttttggtctgacgtgggaagccgtgcaggatcagcacagctccagttgaatatggtggtccgtcagcacctgcatcacgcttactggcggcggggcgtcggtgtagacggcatctaccatgctgatgctgcccatattgaccatcgcgttacggccaaatttcgagtgatcgacaaccagcataacgtggcgcgagttctcaataatggcgcgtttggtgcgaacttcgtggtaatcgaactccagcagcgagccgtcgctatcgatgccgcttatccccagaatgccgaaatcaaggcggaactgggagataaaatcgagcgtcgcttcgccaatgatcccgccatcgcggctgcgtaattcgccaccggcgagaatgatgcgaaaatcttcttttaccatcaacgtgttagcaacgttgagattgttggtgacaatgcgcaaattgctgtgattgagcagtgcgtgcgctaccgcttccggcgtggtgccgatatcgataaacagcgtcgagccattggggatttgctccgccactttgcgggcgatgcgctctttttcttcggtctgggtggccttgcgatcgtgccacggcgtgttaaccgaactggaaggcagcgccgcaccgccatgatggccaggatcaggttttgctccgccagctcattgaggtcgcggcgaatagtctgcgggctgacggagaaatgctctaccagctcttcggtactgacataaccctgctgtttaaccagttcgataataccgttgtgacgttgtgtttgtttcatttataaatccctggaattattttcgttttcgcgcattgagcgaatcaacaaaagccatcgctaaacccacggctaacccggcgatgtgtgctccgttcgccatcgacatcccaaacaaatcaaaccatccggcgacaatccagatcagcgcaaagataattaacccacgttgcaggtaaatgccactttgcggatcgcgttcgccacgtagccagacgtagcccatcagcgcatacaccacgccagaaagcccgccaaaccacggcccgctgaatttttgctgcacatagccgcttaacagggcgctgataagcgtaatgacaattagcttaccgctaccgaggcgtttttccaccgcaccgccgagataccaccaccagagcaggttaaagaggatatgcatcagcgagaagtgcattaacgcgtgggtgaagtaacgccagaactcaaatttcagtgttggatcgaatggccaggccagccataacatcacttcctgatcgccgagaatttgcatggcaataaacaccaccacgcaggcgatcatcatcacccaggttaccggacctgcgcgttcacgcaaggcggcaaagaaaggataacggcgataatgcaggccactgccggtatggcctgcctgccagctcgccgccagataacgcggatctgccgggttttcgagaaaacgcgccagctccgcccgtacgcgctcggcctgggactcatccgccagccagacatcgctttggttatgttgttgaatcgtgaggataacaccctgcgtcgccatgtaatcaacaaacgcctgcgccacgcgggggttagcaaaagaggtaatcatcaacatcgttgctgtcgcttattccacacaaaaggggacagtataaagcgttacgcgccgtacgccacctctgcgggaaactgacgttgccaggcttcaaagccgccgtcaatgctatagaccacatcgtagccctgttgcagcagatactgcgccgcgcctttgctgctattgccgtgataacacatcaccatcaccggagtgtcaaagtcgttatcacgcataaaagcgcccagcgtgtcgttggttaaatggaaagcctgcaccgcatgtcccattgcgaaactctgtggatcgcgaatatcgaccagcaccgcctctttttcctgcaacttctggtgcgcgtcggcaacgttaatacattcgaactgatccatgcgtctctctttctttacaaacaagtgggcaaatttaccgcacagtttacgtcgaagcggcagataaacgccataatgttatacatatcactctaaaatgttttttcaatgttacctaaagcgcgattctttgctaatatgttcgataacgaacatttatgagctttaacgaaagtgaatgagggcagcatggaaaccaaagatctgattgtgatagggggcggcatcaatggtgctggtatcgcggcagacgccgctggacgcggtttatccgtgctgatgctggaggcgcaggatctcgcttgcgcgacctcttccgccagttcaaaactcattcacggtggcctgcgctaccttgagcactatgaattccgcctggtcagcgaggcgctggctgaacgtgaagtgctgctgaaaatggccccgcatatcgccttcccgatgcgttttcgcctgccacatcgtccgcatctgcgcccggcgtggatgattcgcattggtctgtttatgtacgatcatctgggtaaacgcaccagcttgccgggatcaactggtttgcgttttggcgcaaattcagtgttaaaaccggaaattaagcgcggattcgaatattctgactgttgggtagacgacgcccgtctggtactcgccaacgcccagatggtggtgcgtaaaggcggcgaagtgcttactcggactcgcgccacctctgctcgccgcgaaaacggcctgtggattgtggaagcggaagatatcgataccggcaaaaaatatagctggcaagcgcgcggcttggttaacgccaccggcccgtgggtgaaacagttcttcgacgacgggatgcatctgccttcgccttatggcattcgcctgatcaaaggcagccatattgtggtgccgcgcgtgcatacccagaagcaagcctacattctgcaaaacgaagataaacgtattgtgttcgtgatcccgtggatggacgagttttccatcatcggcactaccgatgtcgagtacaaaggcgatccgaaagcggtgaagattgaagagagtgaaatcaattacctgctgaatgtgtataacacgcactttaaaaagcagttaagccgtgacgatatcgtctggacctactccggtgtgcgtccgctgtgtgatgatgagtccgactcgccgcaggctattacccgtgattacacccttgatattcatgatgaaaatggcaaagcaccgctgctgtcggtattcggcggtaagctgaccacctaccgaaaactggcggaacatgcgctggaaaaactaacgccgtattatcagggtattggcccggcatggacgaaagagagtgtgctaccgggtggcgccattgaaggcgaccgcgacgattatgccgctcgcctgcgccgccgctatccgttcctgactgaatcgctggcgcgtcattacgctcgcacttacggcagcaacagcgagctgctgctcggcaatgcgggaacggtaagcgatctcggggaagatttcggtcatgagttctacgaagcggagctgaaatacctggtggatcacgaatgggtccgccgcgccgacgacgccctgtggcgtcgcacaaaacaaggcatgtggctaaatgcggatcaacaatctcgtgtgagtcagtggctggtggagtatacgcagcagaggttatcgctggcgtcgtaaattaacgtaaggtgatcaggtcagatttcaatctggcctgagactgatgacaaacacaaaactgcctgatgcgctacgcttatcaggcctacgtggtttatgcaatatattgaatttgcatggtcttgtaggccagataagacgttcacgtcgcatccggcatgaacaaagcgcactttgtcaaaaatctaacctactttttaattcagggaattaccgcaaagcccacgccatcatacccaacgtaacaaaactcaggcacgttccccactcgccccgagaaaaatagcattaatgcgcccagcgccagcataaaaattttgagcagaaggtaaattgttggcgtgataaggatattacaaacttcaataataccggcaagtccgacacccagcatggcaataaccaccgccaaaaattgcgccagtatggggatgccgaaaaaagtcattaccagcgaggtcaaaatccattttctgttttgcattattctttccattctttttgaatggtgaaattatactccccgagtccccttgccccttctggacacttttccgaaatgatggcggaaaaaaacgggaccctttggccccgttctatttattggtgaacttacaatctcaccggatcgatatgccagatatgatcggcgtactctttgatagtacggtcagaagagaagtagcccatattggcaatgttcagcatcgcttttgcggtccactcttcctgaagctcgtagagttcatcgactttatcctgacaatcgacatagctgcgataatccgccagtacctggtagtgatcgccgaagttgatcagcgaatcaaccagatcgcgatagcgacccggatcttccggactgaatacaccgctgccgatttgcgtcagcacctgatgcagctcctcatctttctcgtagtattcacgcggtttgtagccctgacgacgcagttcttccacttcttccgctgtgttaccaaaaataaagatattgtcagcaccgacatgatccagcatctcgacattcgcaccgtccaacgtaccgatagtcagcgcaccgttaagcgcaaacttcatgttactggtgccggaagcttccgtccctgccagcgaaatctgttcagacagatctgccgccggaatgatcaactgcgccaggctaacgctgtagttcgggatgaacacgactttcagcttatcgccaatctgcggatcgttgttgatcactttcgctacgtcattgatcaaatgaataatgtgcttcgccatgtaataggccgaagccgccttaccgccaaaaatattcacgcgcggtacccacttcgcatccgggtcggccttgatgcggttatagcgggtaatcacatgcaacacattcatcaattgacgtttgtattcgtgaatacgtttgatttgtacatcgaacaacgcctttggattcaccaccacattcagctgctgggcgatatactctgccagacgctttttgttctccagcttcgcctgatgcacagcgtgattaaccattgggaaatcacagtgttgttgcagctcattaagcaggctaaggtcggtgcgccagttacggcccaggtgttcgtccagcacggctgaaagcgatgggttcgctaccgccagccagcgacgcggcgtcacaccgttggtgacgttggtgaaacgacccgggaagattttcgcaaagtcggcaaacaacgattgcaccatcagattagagtgcagttccgatacaccgttaactttgtggctcacaacaaccgccagccaggccatacgcacacgacgaccgttggattcatcaatgatcgacgcccgtcccagcagatcggtatcgttcggatactgttcctgcaaggttttcaggaaatagtcgttgatttcaaagatgatctgcaggtgacgcggcagaattttacccagcatatcaaccggccaggtttccagcgcctcgctcatcagcgtgtggttagtgtaggagaagacctgacaacacacctcaaacgcgtcgtcccagctaaattggtgctcatcgatcagcagacgcatcatctcaggaatcgacagtaccggatgggtatcattgagatgaatcgcgattttatccgccaggttatcgtaggttttatgcaactgataatggcggcttaaaatgtcctgaatggtcgaggaaaccaggaagtattcctgacgcaggcgcagctcacgcccggagtaggtggagtcatccggatacagtacgcgagatacgttctcggagtggtttttatcttccactgccgcgaagtagtcaccctggttgaatttaccgaggttaatttcgctactggcttgcgcactccacaaacgcagcgtgttggtcgcgtcggtgtcgtaaccagggattatctgatcgtaagcgactcccagaatctcttcggtttcaatccagcgcgtttttttaccttcctgctgaatgcgaccgccaaaacggactttatagcgcgtgttgtggcgtttgaattcccacgggttaccgtattccagccagtagtctggcgactctttctggctaccgttaacgatgttctgcttgaacataccgtagtcatagcggatgccgtaaccgcgccccggcaaccctaacgtcgccagagaatcaaggaagcaagccgccagacgtcccaggccaccgttaccgaggcctgggtcattttcttcatcaatcagctcttcgagatttaaccccatcgcttccagtgcgccctgtacatcttcgtaaattcctagcgacaacatggcgttggagagcgtacggccaatcaaaaactccatcgacaggtagtaaacctgacgagtttcttgcgacaactgggcacggtttgaacgtaaccagcgctccacgagacgatcgcgcacagcaaataacgttgcgttcagccattcatgtttattggcgacgaccgggtcctttccaatcgtaaacatcagcttgtaagcgatagagtgcttaagagcttctacgctaagcgtgggcgatgaatatgtaaacggagcattcatataggcgtttcctgaaaactatttcaagcgatagtaaagctcacggtacgacttcgccgcgacctgccagctaaaatccattgccatagcctgacgttgcacaaaccgccacagtgaaggacgggaccacagtacaaaagcacgtcgaatagcccgtaacagcgaccaggcattactatcttcaaagacaaacccactggcgacgccatctgcaaggttctcaagagaacagtcagaaaccgtatcagcaagcccaccggtgcgccgcactaacggcagcgtaccgtacttcaatccataaagttgcgttaagccgcacggttcaaaacggctgggcaccagaatgacgtccgcgccgcccataatgcgatgcgaaaatgcttcgtgatagccaatctgaacgcccacctgaccggggtattccgctgccgccgcaaggaaaccttcctgcagcaccggatcgcccgcgccgagtagcgccagctgcccgccctgctccagaagacccggtaaggcttccagcaccaggtcgagacctttctggctggtcagacggctcaccactgcaaaaagcggcactttatcgtcaaccttaagccccattgcgatttgtaactggcgcttattttccgctttatcttccaacgtatcgcgggtgtaacgcgaggccaacagtaagtccgtctctggactccagattttctcgtccacgccgttcagtacgccggaaagacgcccttcacggtgacgctgttgcaacagaccttccataccgtaggcaaactgcggttcggtgatctcgcgagcgtaggttggactgaccgccgtaatgtgatcggcatagtacagaccggccttcaggaaagagatttgtccgttgaattccagcccatgaatattaaagaatgaccatggcaattggatgtcattcatgtgatgtgcataaaacatgccttgataggccaggttgtgcacagtaaacaccgacttcgccggacgcccgcgcgccgccagatacgcaggcgcaaggcctgcatgccagtcgtgcgcatgcaccacatcaggacgccagaatgggtcaagcccgctggccatttctgccccaacccaccccagcagcgcaaaacgcaatacgttgtcggtataggcaaataagttggtatcgtgatacgggcttcccggacgatcatagagatgcggcgcgtcaatcaggtaaatgccaaccccgttgtaatgaccgaacaacagcgtgatatgtccggcgaaggtatcacgacgggatactacctgcgcatcggtcacgccacggcgaatatcgggaaatgcaggcaacagtacgcgagcgtcaacgccgtctgcgatttgtgctgcgggtaatgccccaataacatcagccagaccgccggttttaagcagcgggaacatctctgaacatacatgtaaaacctgcattatcgctcctgtttatgccctaacttccgtagcatttcgcgcgttaccagcacgatgccttcttctgaacgatagaaacgacgtgcatcttcctctgcgttttcaccaatcaccatgccttccggaataacacaagcacgatcgatgacgcagcggcgcagacggcacgagcgacctacccatacttccggtaacaatacggcggaatcaatgttgcagaatgaattcacgcgaacgcgcgagaacagaacggactgcaccaccaccgaaccggagatcacacaaccgccggaaaccagtgagttaagggtcatcccgtggctaccggagcgatcctgcacgaatttcgctggcggtaatgattcattgtaggtgcgaattggccaattgcgatcgtacatatccagttccggcaccacagaggccagatcgaggttcgctttccagtaagcttccagcgtacccacatcgcgccagtacggctcggcatccgggtcggattgtacgcaagagagcgggaacgggtgcgcataggccagaccggcttcggtgatcttgggaatcaaatctttgccaaagtcgtggctggagttctcatcgcgatcgtcttcttccagcagttcatacagatagtcggcgtcaaagacgtagatacccatactcgccagagatttgctcggatcgttcggcattgacggcgggttagcaggtttttcaacgaattcgataattttatcgttctcatcaaccgccataacgccaaatgcggaggcttcttcaatcggtactggcatacaagcaacggtgcaacgtgcgcctttttcgacgtgatcgataagcatacgcgagtagtcttgcttgtagatatggtcgcccgccaggatcaccacgtattccgctttataacggcggataatgtcgaggttttgggtgaccgcatctgcggtgccgcgataccagttttcccctttcattctctgctgtgctggcagcagatcgacaaactcgttcatttcttcattgaagaatgaccagccgcgctgaatgtgctgcaccagagtgtgggactggtactgggtgatcacgcccatacgacggatcccggagttgatgcagttagacagcgcaaagtcgataatgcggaacttaccgccgaagtgtacggccggttttgctcgcttattggttaaatccttcaggcgggtaccacgtcctcccgccagtatcagggcaacagatttcaatggcagctggcgcgccaacattaagtgatcgttcttctctaaactaaccatgactaactccttttttatcatctctggaacacacacaatccgtgtgcaggtccctgccagacagccgtaatcactgggttatcctctccagcgaatgggggaatggcgtgccactccccagcaggtaaaacaatctctgttacctcaagcgtggcgttaattgcgatcaaaaagcgatccgagagcagaatttgcagctgtttcggcccgttttgccactcatccgtgcttaaaggttgagcatatcgatttagccaacggacattgccgtcgccttcttcccaccagcgattctccaccaaagcgggaatgcgcttgcgcagatggattaacgcggcggtaaatgcggttaaaccactgcttgcctgcgaccagtccaaccaggttaattggttatcctgacagtaggcattgttattgccatgctggctgtgaccatgttcgtcaccggccagtaacatcggcgtaccctgggagagcaacaacgttgttaacagggcgtgaatgctgtcgcgccgccgttcaaccaggtcaagagaaccgcctaacccttctttaccatgattgttactgtaattgttgttggtcccgtcgcgattttcttctccgtttgcttcattgtgtttatggttgaagcaaacgcagtcgcgaagcgtaaaaccgtcatgcgcggtgacgagattaatcgcggcactcggcagacgaccattacgtttaaaaacatcgctggaggcagcaaaacgcccggcaaacgcccccagaggcaaatcataatgtagccagaaacgacgggcagcatcgcggaaatgatcgttccactcggcaaacagcggcgggaaatttcccacctgataaccaccaggagcgatatcccacggttcagcaattaacttcacctgcgagagcaccgggcagttctggatagcggtaaacaacggcgcatcctgacggaactctggcgtacggcccatgactgccgccagatcaaagcggaaaccatcgacgtggcaggtttctacccaataacgcaggcaggcgctggcataatccaccaccgccggatgactcaaattgagcgtgttgccgcaaccggtccagttgtgataatcgccgtcttctcttatccaataatagctacggttatcgatcccacgcagcgagaataacgggccgtcgaggtccagttccgcactatggttgagcacgatatcaagaatgacttcgatacccgctttatgcagtgctttgattgcatcgcgaaactcatccagcgccgtttctggcgagcaggcatacgccggatgcagcgcaaacatcgccaccgggttgtaaccccagtagttacttagccccatgcgttgcagacgtggttcactggcaaactgcgccactggcagcagttccagcgcggtaatgcccaattgtttcaaatagttgatcatcaccggatgcccgagggctttataagtgccacggatctcgaccgggatctccgggtgcaagtacgttaatcctttgacatgggcttcataaatgatggtgctgccccacggcgtgcgcggcggggcatcatcttcccagtcatagtgatcaaccaccactacgcatttcggcgcaatggcggcgttgtcgcgatagtcaggttcattatgaccggcgtgcagcagcgggttatctttaaactccccgtcaatttgccgcgcgcaaggatcaatcaacaacttcgccgggttaaagcgatgcccctcggcgggttgccaggggccatgaacgcgataaccataacgcaaacccgggcgcgcatccggcagataaccgtgccaaatgtcgccactgtgccctggcaagtcatagcgatgttcctggccattggcgtcaaagacacacagttctacccgctcggcatgagcggagaaaagtgtgaagttgacgccctgaccgtcgtaatgcgcgccgaggggagcgggtttgccaatggcgagttgtgtcattctgcctcccgaaccagccagatagtggccagcggtggtagcgtcaggcttagtgaatgctgacgaccgtggctggcaatctcatcgctgtgtaccgtgccgccattgcctgcattactgccgtgatagtgcatggaatcggtattgaggatttcacgccatttgcccggctggtttatgccgaagcgataatcatgacgcggtaccggcgtaaagttactggcaacgatgatttcgttaccctctttatcgcgacgcacaaagatcagcaccgagcgttctttgtcatccaccaccagccattcaaagccgtacgggtcaaaatccagttcatgcattgctttatggtggcggtaggtgaggttcagatcgcgcaccagacgctggacaccgtggtgccagttatcgccgccttccaacagatgccagtcgaggctggcgtcatggttccactcgcggccctgggcaaattcgttacccatgaacagtagtttcttgcccgggaatgcccacatccagccatagtaggcgcgcaggttcgcgaatttctgccatgcgtcgcccggcatgcggtcgagaatcgattttttaccgtggaccacttcatcatgcgacaacggcaggacgaagttttcagtgtagttgtagagaatcccgaaggtcagtttatcgtgatgatactgacgataaaccgggtcgagcttcatgtagtccagggtgtcatgcatccagccgaggttccacttgtaccagaagcccagaccgcccatatcctgcggacgagaaacgccagggaaatcggtagactcctcagccattgtcaccgcaccggaaacctgctcaccaagaatacggttggtattacgcaagaattcaatcgcttcaagattctcgcgcccgccaaattcgttcgggatccactccccctctttacggctgtagtcgcgataaatcattgacgccaccgcatcgacgcgcagcgcatcaataccaaaacgttcaatccagtaaagcgcgttaccgacgaggaagttactgacttcacggcgaccatagttgtagatcagcgtgttccagtcctgatgatagccttcacgcggatcgctgtgttcatacaagttcgtgccatcaaattcggcaagcgcaaagtcatcagtcgggaagtggcctggcacccagtcgagaatcacgttcagaccagctgcgtgtgcggcatcaatgaaataacggaagtcgtcgcgagtaccaaaacggcgggttggcgcatacaggccggttggctgataaccccaactgccatcgaagggatgctcgttaatgggcagtagttcgaggtgggtaaagcccatccatttagcataaggcaccagttgatcggccagctcgcggtagctcaaccagaaattgttgtcggtgtggcgacgccaggaacccaggtgaacttcataaatagagattggcgcatcaaactgattcgcttttttgcgctcttcagtctgtacaaccttttccggcagcccgcaaataagagacgcggtttccgggcgcatttgcgcttcaaaggcataagggtcggacttcagacgcaagttgccattggcatcaatcatctcgtatttatagagctgaccgttatgcgccccagggataaacagttcccagatgccgctctctttacgcaggcgcatcgggtgacggcgaccgtcccagtagttgaattgcccaaccaccgagacccgacgggcgtttggagcccagacagagaaacgcgtacctgtgacgccatccatagtatctgcatgcgcgcctaaggtttcatacgggcgcaggtgagtaccttcagataatagccaggcatccatttcctggattagcggaccaaaacggtaaggatcatcaatcaggttttgctgaccatgccagacaacagccaactgatagcggaaaaaattcttacgtcgcggaatgacgccgctaaagaatccccgtgagtcgagacactccagttttgcgagtttgcgcccggttttcggttcaatcacccacacatcggtagcgtcgggtaaaagggcacggacttccagtcccgcggtggttttatgcattcccagtacggaaaaaggatccgcaaaatggcctgcaattagcgcgttaatcacgtctctatcgatacgatcggacatgcttgtcttcctgttttattgtgtcaccccatccaattggatttttgacttctggttgtgacatttttttgacctgaacggcgcagcactctgtgcatcctctctgcgtcgtcctcacttcaggtaaggctgtgaatactcatgtattcagccacccttaaagaatagccaatgctctatttaactcccggtaaatcatgaaacatctgcgcttactcctgtattacgcactaacaggggcggcatcgcgccccagatttaatgaataaagattacgccagttgacgaagcatccgacgcagcggctccgcggccccccacagcagctggtcgcccacggtaaaggctgacaggaactctggtcccatattcagcttacgcaggcggcctaccggcgtggtcagcgtgccggtaacggcagctggggttagctcacgcatagtgatttcccgatcgttcggaacgactttcgcccacggattgtgcgcagccagcagttcttccacggtcggaatagacacatcttttttcaatttaatagtgaatgcctggctgtggcagcgcaatgccccgacacgcacacataaaccatctaccggaattacggaagatgtgttgaggatcttgttggtttccgcctgccctttccactcttcgcggctctgaccgttatcgagctgtttgtcgatccacggaatcaggctacccgccagcggcacgccaaagttatccaccggcagctcaccgctacgggttaaggttgtgactttgcgttcgatatcgagaatagcagaggacggggtcgcgagttcatctgccacatggccatacagatggcccatctgggttaataactcacgcatatgtcgcgcaccaccgccggaagcggcctggtaggttgcaacggacacccaatcaacaagatcattggcgaataaaccacccaacgacatcaacatcaggcttacggtacagttaccgccaacaaaagtcctgatgccattatttaatccgtcggtaatgacgtcctgattgacggggtcaagaatgatgatggcgtcatctttcatgcgcagagacgatgctgcgtcaatccagtaaccttgccatccgctttcacgaagctttggatagatttcgttggtataatcgccgccctgacaggtcacaatgatatcgagggcctttagcgcctccagatcaaaggcatcctgaagtgtgccagtggttccgccaaaagacggcgcagcctggccaagctgagaagtagaaaagaagacagggcgaatggcgtcgaagtcgcgctcttcaaccatgcgttgcatgagaacggagccgaccataccgcgccagccgataaaaccaacatttttcataagcgtttttttcctgcaaagatgtgtgctgtataaatgtgccggtctcctcttggcacatctttcaccatacaaaaagcagccaaagtcgcaagtgaaattaatcaatgatagcgaagccatcagtaatgcgacttatcctgctttgttagcacgcagaaagtccgcggcaattatcagggaatttgagttatgaatgaaatcatttctgcagcagttttattgatcctgattatggatccgctcggaaacctacctattttcatgtccgtactgaaacatactgaaccgaaaagacggcgggcaatcatggtgcgagagttgcttattgctctcctggtgatgctggtgttcctgtttgcgggtgagaaaattctggcatttcttagcctacgagcagaaaccgtctccatttctggcggcatcattctgtttctgatcgccattaaaatgattttccccagcgcttcaggaaatagcagcgggcttccggcaggtgaagagccatttatcgtgccgttggcaattccgttagtcgccgggccgactattctcgccacgctgatgttgttgtctcatcagtacccgaatcagatggggcatctggtgattgctctgctgctggcctggggcggcacctttgtcatcctgctacagtcttcgctatttttacgtctgctgggcgagaaaggggtgaacgcacttgaacgcctgatgggattgattctggtgatgatggcaacccagatgttcctcgacggcattcgaatgtggatgaaggggtaacgaggagagtttttcgaaaagaacccggtagcgtcacaactaccgggcgaacaaacttaactcaacagctggaacgcaatcatcccaacgatggcaccgacagtgccgaggatggtttccatcatggtccaggttttcagcgtttcggcttcggtcgcgccggtaaatttaccgaacaaccagaaaccggcgtcgttaacgtggctgacaacaatcgaaccaccagcgatacaaatcgacagcgccgccatttgcgcaccggagtagttcagttgttcaataaccggcatcaccagtcctaccgccgttaaacaggctacggtggcagaaccctgaatgatgcgcactgcagctgccagcacgaagcaggtgatagcaatcggcaggcccatgccggttaacgcttcgcccagtgccggacctacgccagagtcaaccagcacctgtttgaacacgccgcccgcaccaatcaccagcagaatgatccccgccggttgcagcgcgtgaccgcaaatctccatcactttgtcttttggcatgccctgacgcattgccagaccgtaaatcgccaccagacaagcaaccagaatcgcggtaaacggatgaccgataaactcaaaccattcgtaagcagttgatccttccggcacaaaacgcgcggcaatggttttcagccctaccagcaccagcggcagcaggatcagcgacaggctgaatccgaaagatggcattttgccttcgccgagatgcggttcgctgatgtcgtcaggaatatgcagctcaacgtaacggctgatgaagttaccccacagcggcccggcaataatcattcccggaattgccgcacacaggccaatcaggatcatccagccaaagtcggcattcatctgcgatgccagcagcatcggcgctggtccaggcaccagaaatgccgccgctgccgccacgcctgcaaataatgggattaccagcttcaccaggttcgtaccggtgtggcgcgccattgagaaagcaacgctaatcagcagaactatcgccacttcaaagaacagcggtagcgcacagaccagccccgcaaggccgatggcataatgcgcgcggctgtgaccgaaggatttgagcattttgacggcaatctgatcgactgcgccggtttcatgtaagatcttgccaaacatagctcccagggcgacaaccaccgccaggaagccgagggtgcctcccatccctttttccatcgtcgctgcgattttatcgagcggcataccagaaaaaaggccagcccccatggacaccaccattaaagccaggaaagcgtgcatacgcgccttcatgactaaaaacagcagcagtaaaacagaccctactgctgttaaaacaagcgttaatgtagtcactacttatttgccttttttaataacctcaatggtgcttgccacaacaccttccagcggttgatcgatatccaccaccagtacatcggtttcgtccgcacccggctcctgcagcgtttcaaactgcgtcaccaacatttgggttttaaagaaatggcctttgcgcgctttcaggcggctttcaatcacatcaaaatcgcctttcaaatagatgaaagagagattcggattaccttcacgcagcaagtcgcgatagtgttttttcaatgcagaacagacgatcagcgacactttattagtgcgctgcatagcaaacgcggcgtcgttcagcgcctgcaaccacggtttgcgatcgtcgtcattcagtggttcgccagacgccattttttcgatattgcgccgtggatggaggaaatcgccatcaagaaacgcggcatgaagttgatgcgccacttcactggcgaccgcagatttgccgctgcccgatacgcccatcaagacgtaaatgtggtgatcatggttagtcgtgctcaaagtggtgcccccacaatacaagaattaaaaatgttacgggtaactgttatcggtaacattgtccagccggacaatatcagaagcaatatccatccatgccttaagtgtataagtgtgagctacttcaaatttgtgggcttaaatagatccgcccggtgacaaggtgaaacctaaatctaacattttcggtgtcacagattcgccacgaatacgcgccagcaggcgttcagcgccaatactgcccatccgctcacgcggcgtcagcacgctcgcaagtcgtggctccatcacctgaccaatgtcatgaccgtggaaaccggcaatcgccatatcgtcaggaacttttaaccccagacgctgacattcaaacgccgcgccgaccgccaggtcatcattcgtacagaacacgccatccagctgcggatattcccgccgcgcctggcgaatcagttcaataccggaagagtaagaagaagattgctcaaccatcacgctatatggcaccaggcctgcatccagcatcgcctgttcgtatcccttctgtttgatgatagtacgttcgtcgagacgtgcgccgagataggcaatgtggcgatgcccgcgagcaataatggcagtggtcatctggcgtgctgcttcaaagttatcaaaaccgacggcgatatcaaggcatggcgacttgctgtccatcagttccaccacgggaatacccgccacttcaatcatctttaaggtgcgcggcgtgtgggtacgttcggtgaggatcaggccgtcgatattccaggagagcatggattcgaggcgttcttgctccatttccggtttataaccgtagtgcgccagcatggtctgataaccgtgcgcgtcggtgacgctttcgattccgcgtaatacttccgcgaaaacctggttggtgagagaaggtaacaggacgccaatcgcccggctggtggcgttagagaggatatcgggcgcacgattgggaatatagcccagttcatcaagagccgcggcaatcttgccgcgtagagcgacggaaacctgctccgggttgcgtaaaaaacggctgaccgtcattttggtcacgcctacacggtcagccacatcctgaagtacgggtcttttctttttcatcgtcctgaaggtacaaaagagatagattctcttagtttaacacggacacatcagaaccttcccggggaaaacagtgcttgtttacaattattagatatacactaaatcaattgcatcgcattgtgctaacgacgcggcaaaaccccggaagcgtacatcagcacgcgaccggagcgagcgaggaagcctgcaaaaaggcaggcttcaaagatgccgttgagttttaaaccggcggcagatcgaacagtaacacttcgctgtcgctatccgcatggatggagattgcctgctcatcccagattgccagaccatcgctggtcgaggctttcacgccgttaatggtgacattgcctttcaccacctggatccagacgcggcgttcagcggcaatctgatgcaccgactgctcatctttcagcaacgcccagcggtacagttccatatcctgatgcactttcaatgaaccatctcgcgcatccggcgagagcaccagctgtttgccctgtacggcatcgaagcgacgctgttcataacgcggcgtaataccgttttcttcaggcatgatccagatctgatacagatgcagacgctcggtgctgcttgggttgtactctgagtgacgaatacccgtaccagcactcataatctggaactcacccgccggaacctgctctttattgcccatgctgtcctgatgctcaacagtaccttccagcacgtaggtcaaaatttccatatctttatgcgggtgagtgccgaagccctgccctgcttcaatcacgtcgtcgttaatcacgcgcagcgcggagaagcccataaagttcggatcgtaatagttggcaaaagagaaagtatgccaggagtccagccagccatgatttgcatgaccacgttcatttgctttgcgtaagtagatcatttgtattcgccccctgaatgatttcgatgggcttagtgtggacccgatctgcctgggatgatagagggtgaaaattgacccctctgttcaaaaaaattgaactattcgaggggccatcaaacttacttagcgagagttactgtggagggagaggcttgctcaaatccgcgttcaaggatttccagattggtaagaacttcagattccttgacgtaatttggcgcaccgtgggtgatggtttgatacaacgcatcataaacgcgcccgtaatcgcccatctccggcttcatctcttctctgaccgtcacgccctcgtcattgacatactccagcacaccgaccgaatcatccgctgcgaatcccggttcgcccggcataatattagccttcaggctggtttcctgctggtcgataccgtatttaataaacgaacctttcttaccgtgaacgataaatttcggataatcgattttcaccagatggctggttttgacgatggctttcaggtcgccataaaacagttgcgcttcaaaggtgtcgtcaggattggctttattacgcaggctgcggatgtcataagcgacgtgatccgggcgaccgaacagagaaataatctggtccatcgtatgcacaccaaggccataaaacgcgccatcctgcggcagcccaggtttggtttctgccaccgggcggtaatagtcaaaatggctttccacttcaacaatctctcccaacttgccactttcaatcgcttttttcgctgtcaggaagcaggagtcaaagcgacgattctgatacggcgtgacggtcagccctttgcttttcgccaacgcaaacagctctttcgcctgcgcaagtgtcggagtgaacggtttttcgaccagcacatttttcccggcttccagcgcgcgtttcgcgtactcgaaatggctgtccgcgtgggtgcagacaacaaccagcttaacatcgggatcgtttagtacttcgtcgagatcgctggtgaaatggatatgggaataaatgggagcctgttcttccggcttcgcatggcgacgaaaaatatgcgcgacatgccagctatccttgcggttaagtacatacggcagatggtaacgggtggtgcttttgccgaagccaataaaggcgcagttgatgaccatgatttcgtcctttttaaggtggttatttacaccttagcgcaaagcggacgtggttcctactggagtgcgcataacgaacacaagcactcccgtggataaattgagaacgaaagatcaaaaaaaaagccagcacccggctggctaagtaatactggaagcaatgtgagcaatgtcgtgctttcaggttctccgcgagggtcttcctgatcgcgagacaataataatcattctcattcgcacttgtccaacactttttgcaaaaaaatgcatttgactcgcatttgaaagtcaatgatgttgaaagggacatttaccccaaagaggacaaaggaatgagtgagatagtaatacgccacgcagaaacacgggattacgaggccatcaggcagattcacgcccagccggaggtgtattgcaacacactacaggtgcctcatccttccgatcatatgtggcaggagcgactcgccgatcgtcccggcatcaagcaactcgtcgcctgtattgatggagacgtcgtgggccatctcaccattgacgtgcaacagcgcccacgccgcagtcatgttgccgattttggtatctgtgtcgactctcgttggaagaaccgcggcgtcgccagcgccctgatgcgagagatgattgaaatgtgcgacaactggttgcgggtagatcgcattgaactaaccgtgtttgtcgataacgccccggcaattaaggtctataaaaaatacggctttgaaattgaagggactggtaagaagtacgcattgcgtaatggtgaatatgtcgatgcatattatatggcgcgggtgaagtaagatagtgccctttttctgagatggaaaaagggtgtcattcaaaatcgacataccttcctttaaggtatttatttgcccaatacatatattgagatttaactcataattacttcctaaagtgtaatattttattttttaatatatacgcctacaatttcctggagtaaataaataacaattaacaagcataatattgccattgataaaatagcatgccataaaaggacttttcagggatgagtaatattgtttacctgacagtaacgggagaacaacaaggaagcatctccgcaggttgtgggacttctgagtctacaggtaatcgttggcagagcgggcatgaggatgaaatatttacattctcactcttaaataatattaataatacggggcttggttcacagttccatggtataacattttgtaaattaattgataaaagcactccattatttattaattccattaacaataatgaacaattatttatgggatttgacttctatcgaataaatagatttggtagattggaaaagtattattatatacaactaagaggcgcttttttatcggctattcatcaccagatcattgaaaaccaactggatacagaaacaataactattagttatgaatttatcctctgtcaacatcttatcgcaaataccgagttcagctatttggcactccctgaaaattataaccgtttgtttttaccaaattcaaaaaaccaaacaaataatcgtttcaaaacgttaaacagcaaagctattggcaggctacttgctgctggtggcgtatacaatgggaacattgaaggattcagagatactgcggaaaaactgggtggagatgcaataaaaggctatgatcaaatactaaatgaaaaaacagcgggcatagcgatagcaacagcatctattcttttaacaaagcgttctaatgttgatacatatacagaaataaatagttacttaggcaaacttagaggtcaacaaaaacttcttgatggtatagacataatagaaataatatacattaagagaccttcaaaagacttagctaacttacgaaaggagtttaataaaactgtaagaaaaaattttcttatcaaacttgcaaaaacctccgaagcatctggaagattcaacgccgaagaccttttaagaatgagaaagggcaatgttcctctaaattataatgttcaccataaactatctctagatgatggtggtactaatgatttcgaaaatttagtattaatcgaaaacgaaccatatcataaagtttttactaacatgcaatcacgaatagctaagggaatattagtaggtgaaagcaaaatcactccctgggccattccatctggctcaatttatcctcccatgaaaaatattatggaccacacaaaatgatgactaaaacccaaataaataaattaataaaaatgatgaatgatttagactatccatttgaagcaccgctcaaggaatcatttattgaaagtataatccaaatagaatttaattctaattcaactaattgcctggagaagttatgtaatgaagttagtattctttttaagaatcaacctgattatcttacttttttaagagcaatggatggattcgaagttaatggattacgattatttagcctctcgattccagaaccttcagttaaaaacctttttgccgtaaatgaattttatagaaataatgatgatttcataaaccctgatctacaagaacggttagtgatcggggattatagcatttcaatatttacttatgacattaaaggtgatgctgccaacttactgatttagtgtatgatggtgtttttgaggtgctccagtggcttctgtttctatcagctgtccctcctgttcagctactgacggggtggtgcgtaacggcaaaagcaccgccggacatcagcgctatctctgctctcactgccgtaaaacatggcaactgcagttcacttacaccgcttctcaacccggtacgcaccagaaaatcattgatatggccatgaatggcgttggatgccgggcaacagcccgcattatgggcgttggcctcaacacgattttacgtcacttaaaaaactcaggccgcagtcggtaacctcgcgcatacagccgggcagtgacgtcatcgtctgcgcggaaatggacgaacagtggggctatgtcggggctaaatcgcgccagcgctggctgttttacgcgtatgacagtctccggaagacggttgttgcgcacgtattcggtgaacgcactatggcgacgctggggcgtcttatgagcctgctgtcaccctttgacgtggtgatatggatgacggatggctggccgctgtatgaatcccgcctgaagggaaagctgcacgtaatcagcaagcgatatacgcagcgaattgagcggcataacctgaatctgaggcagcacctggcacggctgggacggaagtcgctgtcgttctcaaaatcggtggagctgcatgacaaagtcatcgggcattatctgaacataaaacactatcaataagttggagtcattaccgacattaaaagtaacttttttgaaattagagataatattggcacagaaaatatattcagttcgtttagtgatttctcttcattcttaaacgaaatcatggacagttgttcataataatcaaaaggaaacaaaaatcattgtaaaccatgccatctttttagagattaccagcagaaaattccttgttcgaaatttagcagtgcaagctatggaaaaacttacaacggaactacactccttaagtgagatggaccgaagacatgtagtctctattttagccgaaatagctaatggctatgatgattttaatgacatgttgatttatttagaattttacccgaatcataagattctgatatcttaaataagaaaatcccgttcgacgttctgaaaaagaaatcataaaatattagcagatacttatttcgtgactatatcttatccgatgaacttttttcaaaaccagcatttaataatatctttgacgaagatgaacgcgtctttgctcaatgtatcacacaggaataataatataacactcaacaataatatttattataattatgattacttatcacgacgcattcgcgaaagcgaaccattaccttgatgatgcagatctcccggtcgtcattactctacatggacgctttagccagggctggtatttctgtttcgaagcacgagaatttctcgaaactggagatgaggccgcgcgcttagctggtaacgcaccttttattattgataaagacagtggtgaaattcattctctgggaacggcaaaaccgctggaagaatatctacaggattacgaaataaaaaaggctaccttcggcttgccctgacaaaatagccctcttcccacgaagagggccgctaaccttagtaccccgccgttaaatcatccaccgagcgcgggtcggatgcgccgtacaactcaccgtccggcccaaccataatgctttgtgtactgcccatcgcctctttcagcgccactttctgaccttttgcttccagcagcttgagcgtatccgggctaaaccctttttcgacacgcagctcgtccggcaaccactgatggtggaaacgcggcgcattggtcgcttcggcgacgttcaagccataatcgatgctattcaccaccatttgcagcactgtagtgatgatccggctaccgcctgggctaccggtaaccagccaggttttaccgtctttcaccacaatggtcggcgacatcgacgacagcgggcgtttgttcggcccgacggcgttggcatcaccgcccaccagcccgtaaacgttcggtacgcccggtttggcggagaaatcatccatctggttattaagcagaataccgctctcgcccgcgacaatgcccgtaccgaaggtggtgttcagcgtataggtcaccgccaccgcgttaccatctttatccaccactgagtaatgggtagtttgattactctcataaggcgcaagcttgccggggcgaatttcgctggatggcttcgctttattgatatcaatttgatcggcaatagatttggcataggctttattggtcagcgcctgccacggtactttgacaaaatccgggtcgccaagatattccgagcggtcggcgtaggcgtatttctccgcttctgccatgatttgcatcgcatcggcgctgccaaagccgtatttcttcatatcgaagttttccagaatattgaggatttgtacgatatggatcccgccggaggatggcggtggcatggagtaaacctgatacccgcgataatcgccgcttatcggagtgcgttcgaccgctttataggctgctaaatcttctttagtgatcaagccaccgtttttctgcatctcctgggcgatctgttccgcaatcgtgcctttatagaattcgtccgggccgttttcagcaatcatctccaggctctttgccaggttcgcctgcaccagcgtgtcgccctttttcagcggctcgccctctttccagaagatagctttactgttttcgtgattcggcaacacttcgctaccgtaggttttgagatcgtcagccagcgcgtcgttaacgataaaaccatcgcgtgccagtttaaacgcgggctgcacgactttgttcagcggcatggtgccgtatttatccagcgccagcgagaaacctgctaccgtacccggtgtgccggaagccagatgcgaagtgagtgattttttgctgtccgggttgccctgatcatcgaggaacatatcgcgggtcgctttggcgggtgccatttcgcggaaatcgatagccgtggtattgccatttttcgagcggattaacataaaaccaccaccgcccagattccctgcctgcggatgcgttaccgccagcgcgtagcccaccgccacggcggcatcaacggcattcccgccctccttgagaatatccacccccacctgagtggcagtggcgtccacagacgctaccattccctgtttcgcgcgtaccgggtggaagacatcttcctccacaccatacgagacgggcggcgcaggaggcgcggcggcggcgctaaaacaacttcctgagagcagagcagcaatggccacccggcgtaaaaacgtcggttttatcatcgttattctccagagattaaggggcaaccccagctaagcctggtatataactctgaattaatcatcgttttgtcgggaagcgagtaaacttaaaggatatcttcagaggaggatacgcgatgaaacgacttctgattcttacggcactcctgccgtttgtcggctttgcacagcccattaatactctgaacaaccctaaccagccggggtatcagatacccagccagcagcggatgcaaacccagatgcagactcagcaaatccagcaaaaagggatgctgaatcagcaactgaaaacgcaaactcagttgcaacagcagcatttagaaaaccagataaacaataattctcagcgggtgttgcagtcacagccgggggagcgaaatcccgcccggcagcaaatgctgcccaacaccaacggcgggatgttaaacagcaaccgtaatccggatagttcgttgaatcagcagcatatgctgccggagaggagaaacggcgacatgctgaatcagcccagcacgccgcagcctgacattccgttgaaaactattgggccgtaaagttcggaccaatcacgtcaatcgcatcggtacagatgcaatccacaccccagcgcagcaactctgctgcgcgctggggtttattgacggtataaaccagaatccgcagtccggcgtctttcaactgcatcactcgcgctttattgagtaacttatgattgagatgaatagagacgcagcccagccgcgcggtcagttcgcgccagtcgtcgcgccactcatccagcaacaaaccgcgcggcagttccggtgccgcctgttgtgcagcttctaaagcatcaatctcaaacgatgacagcagcggcggcgtcataccggcccacagctcgcgtgccgccagcgccaccattttgcccgttaatggcccggtgccggtggtgggtttgatttcgatattcgccatcatcccgtgttcgcggcaacgttccgccacctgcgaaagcaacggtagcggctcacctttaaacattttgctgtaccaactgcccgcatccacgcgcagtaaatcctgccagttcagttcacccgcgacgccccagccgttgctggtacgttcgagattgtcgtcatggagcaggaagatctcgccatctttcgataacttcgcgtcaaattcgatcatcttatgaccgtattttgccccgacgtcgattgacgccagggtgttttccggggccagcttaccgccgccacgatgagcgacgatgcggggataaggccagttactcatactcgttgtcctgtttcaccatcaaaaagatgcagctgattttccgccagatgcagccacagcgtgctgcctgccgtcgggcgctcctgatgcgccagtcgcaccaccagcttctgctcgccccagcgtccgtgcgccaggttatctgcgccgaggatctccagcgtgtccatcaccatcggtacgccgccttctgcctgcgagcttagcgcaatatgttccgggcgaatgccgagagtcattttacgcccggcatactgacggtagccaccgtttagcggcagctcaataccgccgtccagttcgaaatgcgtgccttcgttattcacgcggcctgtcagcaggttcatcgccggactgccgataaaactcgctacaaacaggctggcgggcttttcgtagacttcaactggtgtgccaatctgttcggcaacaccgccgttcatcaccattactcgctgggcgagcgtcatcgcttcaacctgatcgtgagtaacgtagagtgaagtcgttttcaggcgacggtgcaactgttgcagttcaagacgcatctgcacgcgcagcttggcatcgaggttagagagcggctcatcaaacaggaacaccgccggatcgcgcacaatcgcgcggcccatcgccacacgctggcgctgaccgccggaaagctcgcgcgggcgacgtttgagcagaccgtccagctccagaatgcgcgccgcttctttaacgcgctcggcaatttgctgcttgcccatgccgcgaattttcagcccccacgccatgttttcttcgacactcatatgcggataaagcgcgtagttctggaacaccatcgcaatcccgcgatcttttggctccatttcagtcacgcgctggtcgttgatccagatatcgccttctgtcacccgctccagcccggcaaccatgcgcagcagcgtcgatttcccgcagccagacggcccgaccatcacgataaattcgccatccgccacatcaagggtcagcggtttaatgacctgggttttaccatcccagcttttggttactgcctgtaatttcagtcctgccatcttatttctcactatcgaccaggccgcgcacgaaggcacgctgcatcactaaaacaatcaccaccggagggataagcgttaacaacatcgccaccatcactgagttccattccgtggtgccttcgcctgtagcgatcatccctttgatccctgccacggtggtgccgagatccacatcggtaataatcaacaacggccacaaatactgattccagccgtagataaaggtgatcacaaacagcgccgccagattagttttggagagcggaaaaacgatgtcgcaaaagaagcgcattggcgatgcgccgtcgatccgcgcggcttccaccagctcatccggcagcgtcataaagaactggcggaacaggaaagtagcggtcgccgaggccatcagcggcagcgttaaaccggcgtagctgtcgagcatctgcaggttggcgatgacttccaccgtcgggaagatacgtacttcaaccggcagcatcagggtgataaaaatcatccagaagaagaggttacgtagcggaaaacgaaaccagacaatggcaaatgccgagagcatcgagacggtaattttgccgagcgtaatgctgaacgccatcacaaagctgttaagcaacatccgccagaacggcgcgctattcgtgcctaccccgttcacccagatgttgtggatgttttccagcagatgtgtgccggggatgagcgtcatcggcgcggcatagacggcctgtttatccagcgtcgccgcgacaaacgccacgtacagcgggaagaggatcaccgcgatcccgaggatcagcatggtatggctgaatatcgtcagccacggacggttctcaatcattggtaacgcaccttgctttcaacatagcggaactgcaccaccgtcagcacgatgacgaggaacatcaacaccaccgactgtgcggcagacgaagccagatccagtccggtaaaaccttcgcggtagatcttataaatcagcgtcgtggtggcctgaaccggcccgccggacgtggcggcgtcgatcaccgggaaggtgtcgaagaaggcatacaccaggttcactaccagcaggaagaaactcaccggggcgataagcggcagcgcaatcttaaagaagcggcgaatcggccctgcaccgtcgatggctgcggcttcgatcaacgaacggggaatggattgcagcgcggcatagaagaacaggaagttgtagctgatttgcttccatactgaggcaaacaccaccagaaacattgcctgaccgctgttttgcgcgtggttccagtcgtagccgaactccgcgagaaaatgggtgatcagcccgcgaccggggttaaacaggaagatccacaatacggcggcaacggcgggagccacggcgtaaggcagcaacattaaggtttgatagaaacggctgccgcgcacgatgtactccaccagcgccgcaaagaacagcgataccagcaaaccgctgacggtgacaaaggtgctgaattttatcgtcgtccagaaggagtcgagatagtagctgtcatggaacagcgtgacgaagttatccaggccgacaaactggctggagaaaccaaacggatcgacgctttgtagcgagtaccacaacgcttcgcccgcaggccagataaaaaagataacggtgatgatgagctgcggcgcgaccagcagataaggcagccagcgcgagcggaacaccggacgggatgatgacattacggttaattcctgaactgtgccggatgcgcttcgcttatccggcctacacgcgatgccaggtcagataagcgaaacgcatccgacattacactgattaagacttcgtcgatttctcaaagcggcgcagcaactgatttccacgctcaacggcggtatccagtgcctgctgtggtgtcttcttaccggtccacacgctctccagctcttcatccacaatcacgcggatctgcggcatgttgcccagacgcagccctttggtgaacggcaacggcggcttattcagcatctgacgcgtcgcggtatccgcccctgggtttttctcataaaagccctgctcacgggtcaggtcatacgctgctttggtgattggcagataaccggttttctgatgccactcggcagcgttttctggcttcgcgaggaaatcgaggaacttcgccacaccggtatacgtttctttatctttaccctgcatcacccacaggctggctccgccgataatggcgttttgtggcgcatctttcgcatcggcgtcgtaaggcatcatgcctacgccgtagttaaatttggcgtactcgcgaatgttggcaagagaaccggaagaggcggtggtcatcgcgcaatcaccgttatagaacttctcggtggattcatccttacgaccgacgtagctgaagtcgcccttcttgttcatctcctcgagcatggcgatgtgtttcacctgctccggcttattgaactccagcaccgcgtccgtgccgtcaaagccgttgtttttgctggcaaacggcagaccgttccaggcgctaaagttttccagttggatccagccctgccagccgctggcgtagccgcacttcatgccggaggctttcagtttcgcggcatagtccgccagatcctgccaggttttcggcggctgttccgggtctaatcctgctttcttgaaggcgtctttgttgtaatagagaacgggggtcgagctgttgaatggctgggagagtaagtggcccgttttgctgtcggagtagtaacctgaaaccgtcggcacaaactgcgactcatcgaactgaatccctgcctctttaaacacgtcatacaccggtttaatggctttcgacgccatcatggtggcggtgccaacttcataaacctgcaaaatagccggcgcgttgccggtacgaaatgcggcaatccccgcgcttaaattctgttcgtagttgcctttataggtcggtacaattttgtaatccgggttttcggcgttaaaacgttgggccagagaatccacctctttacccagttccccttccatagaatgccagaacggaatggtcgtcactgcctgtgcattccccattaacgccagtccgagcgccagtgctgaagctgtataatgtaacggtttcatcgtttatctctcttgttgtaccgaatgcgcgaattcacgcgttttatgctcgcggggtaacatgacatgctcgaattacagaaaaataacttttttgttacatttgtaagatagtaaggtgtcagaaagatgacaaggcggtgacggcgtgggtgagggaaaatgggagatggggcacggataagcgggaaaatatagaaggtctgaatcaaactctacagattgctcatcgtttcatgccggatgcggcgtaaacgccttatcaggcctacaagatcgtgcaaattcaacatattgccactcacccagtaggcctgataagcgcagcgcatcaggcaattttacatttgtcacctgtctcaaaggagtcttttgactccctatcaatcaacgtgttattacccgcctaaatacgcacttctcaccgcttcattcgccagcagcgcatcaccagtatcggaaagcactacatggccgttttccagcacgtagccgcgatccgccagctttagcgcctggttggcgttctgctcgacgagaaagatagtcatcccctgctcgcgcagctgctcgatggtgtcgaaaatttgctggatgataatcggcgcaagaccgagcgatggctcatcaagcagtagcaaacgcgggttgctcatcagcgcacgaccaatcgccagcatctgctgttcaccgccggacatggtgcccgcccgctgaatacggcgctcatgcagacgtggaaacagctcatacacccactttatgcgctcctggaactggtcgcgttcagcaaaaaaaccgcccatcgccaggttctcttccaccgtcatccgcgagaagacgcgacgcccttccgggacaatcgccaccgcttcgcgcatgattttcgctgtctgccagtcggtaatgtctttatcatcaaacacaattcgcccgctggtggcacgcggatcgccgcataacgtgccgagcaaggtggttttccccgccccgttcgcgccaatcagcgtgacaatctcgccctgattgatatgcaggctcacctcatgcagcgcctggattttgccgtagtgggcgctgactttgtcaaaggacaacatgactttttccatcttatgcctcacctaaataggcacggatcacgtccgggttattacggatctgctccggcgtaccgtttgccagcggcgtcccctgattgaccacgtaaattcggtccgaaattcccatcaccagcttcatatcgtgttcaatcaacaagatagtggtgttgtgatgattgcgcagttcggcaatcagctcatccagctctttcgtctctttcgggttaagacctgccgcaggttcgtcgagcattaaaatctccggctgcgtcaccatgcagcgggcaatctcaagacggcgctggtcaccataggccaggttactcgcctgacggttggcgtgttccagcaaaccaatgcgctcaagccaggtcgcggcgcggtcgagcgcttcgctctgggcgcgacggaaggatggcgttttcaacaggccagagaacagcccggttttcagttgctgatgctgcgccaccagcaggttttcaattaccgtcatttcacggaacagacgcacatgctggaaggtgcgcaccacgcccatgcgggcaatttgctgccccggtaaaccttccaggtgctgatcgcgcagtaaaatggtgccgccggtgggtttgtagaatccggtcagacagttaaaaaccgtggtttttccggcaccgttagggccgattaacgagacgatctcctgcgggtacagttcaagattgacgttgttcaccgccagcaggccgccgaagcgcatcatcaggccgttaacagataataatggctgactcatgcctgctctcctttcgctgcgccgtttttcagcttcagttgcgggcgcgtcatgggcagcaagccctgcggacgccagatcatcatcagcaccatcaaaccaccgagcattaacatgctgtattcgttgaaatcacgcatcaactcgcgcgacaccaccagcaaaattgccgccagaatcaccgcaaattgcgagcccataccgccgagcaccactatcgccagcacaaacgccgattcggcaaaggtgaaggattccgggctgacaaagccctgacgcgccgcaaacagcgttccggcaaaaccggcaaacgcggcacttatggtaaaggcagtcagcttgatacgacgcgggcttaagcccagcgaacggcaggcgatttcatcttcacgcaacgcttcccacgcacgccccagcggcatccgcagcaggcggttaatgacaaacaggcttagcaccaccagcagcaacgccaccaggtagaggaagatgacacgatcggagggatcgtatttcaggccaaagaaattactgaacgtgtcccagccgccttcacgagcggtacggctgaactcgagtccgaagagtgtcggtttcgggatctgactgattccgttcgggccgccggtaatttcggtgttattgagcagcaatatgcgcacaatttcgccgaaaccgagggtaacgatcgccagatagtcaccgcgcaaacgcagcaccggaaaaccgagcaggaagcccgccgccgctgccattaatccagcaatcggcaggcaggtccagaagcccaagccgtaatagtgattgagcagcgcaaaagtgtaagcgccgatggcgtaaaaaccgccgtaccccagcaccagcagaccagaaagaccaacaaccacgttcagcccgagaccgaggataatgtagatcatggtcagggtggcaatatccaccgtcccgcgtgaaaccataaacggccacgccaccgcaagcaccaacagcgccacgaggaacagtttctgcttcaccgtggagccatcaatggcgggcagaataaacttcggtccggaaacgcttttcaaccctttctggaaagccggtcgcaaaagctggaagaaaaagaccaccgccgtgccgataaacacccactgccaacggacatccgaagccgtgtcgaccaccagtttggtgccatccagctccagttgcacgcccataaagacgcccgccagcacaaagaacatcgcggcagagagcagcgccattgcaatatgcatcggtttcatactttctctacctccgggcgacccagaataccggtcggcatcaccagcagcaccagaatcagcagggcgaatgagaccacatctttatattccgtactcagataggcagaagagagcgcctccgcaatccccagaatcaggccgccaatcatcgctcccggaatgctgccaatcccaccgagcaccgccgcggtaaaggctttcatcccggccataaagccgatgtaggggttaatgacgccgtagaactgaccgagcagcacacccgccaccgccgccatcgccgcgccaatcacaaaggtcagcgcaatcacccggtcggtgttaatgccaagcagactcgccattttcagatcttccgcgcaggcacgacacgcgcgacccatgcgggaatagcgaatgaaaatcgtcagcgccagcatggcgaggaaggtaacaatccagatcaccgcctgcatggtggtaatagaggcagagaagttttcgctatgccccaccacccactgaccgttaaacaggctcggcagcgccacgtcgcgcgaaccttcggtcaggctgacgtagttttgcaggaagatggacataccgattgcagagatgagtgcaatcaggcgcttagagttacgcaccgggcggtaagccacccgttcgatactccagccgtaggcgctggcaatgacgattgcgccgacgaatcccgcagctaccagcagccagccggtatcaatgcccatcatcatcagcgcggcgatgatcataaatgagacgtagctgccaatcatataaacctcgccgtgggcgaagttgatcatgccgataatgccgtaaaccatggtgtagccgatggctatcagcgcgtaggtactgcccagcgtgacgccgttaaacatctgctgcaagaaatacaaaaactgctcagacataaggtaacctttctaaacccgcccgcattttacgggcggtgggatgatcacttggctgccgtggatgaaccgtcggcgtgccactggaagacaccaaaatcaaatcccttaagatcgcctttttcatcccagttcagcggcccaatcacggtgtttgcaccgttagcttttaaatctttcaccagcgccagcggctcatcgctgccggtacgctcaagggcagtcgccagagattgcaccgccgcgtaggtgatccagacataaggcccggacggatctttcttgtctgctttcagcgcatcaacgatgccctggtttgccggatcctggtcatagcgttttggcatagtgaccaacatgccttcggcggcatcaccggcaatgttcgacaacgacgcattacccacaccttccggccccataaactgggttttcaggccaacggaacgggcctggcgcagcatctgccccatttccgggtagtaaccgccgtagtaaacgaagtcgatgttttcttttttcaggcgggcgatcagcgcggagaaatctttctccccggcggtaataccgtcgaagaagacgacgttggcgttagccgctttcagcccgtcctgcaccgaacgcgccagcccttcgccatactgttgtttgtcgtgaatgatggcgatgcgctggggcttcaccgtctcaagaatgtattttgccgccgttggcccctgggaagagtccagcccggcagtacgcataatgtgttgataaccgcgttgggtcagctccgggttggtcgctcccggcgagatcatcagaataccttcgtcttcatagatatctgacgcaggctgggtagaagaagaacacagatgaccaataacgtatttaatgccgtcattaacgattttgttggcgaccgcaacggcttgtttcgggtcgcatgcgtcgtcatattccacgccaaccagtttatcgcccttaattccccctttggcattaatgtctttaattgcctgacgcgcgccgttaaattccatatcgccccactgggcaatcgggccggacatcgcgccgacaacggcgactttaatatcgtcagccatagcggtgtgtgaaattgccagtgcaatcatccctgcgatgatagttttcgcattccgtttcatagtcaaaaatccccattcgtgatgttgtgttgctttgtttttatgtgttaacaaatcagactgttctttttttatactgcactgtttttgcctgtctgattaaggggttagcgcagtattttgtgataatagcgattaaaatccctatttttcagtcgattaagaacagataatattctgaatttattgatagataaacagaaaaaagtgcctttgtcagcataaaataacggcacaaagggcggaataattcactatcattcaggggattatgctggacatttttcattctctaatgttttaattttgtaattattgctgttaaaaaattaatcacctgccaaaagaaataaaaaagagaaagcctccgattaaattatttcgctacactggttccacttttgtgatttacacgggttacccatgaagctgaccatcattcgattagaaaaatttagcgaccaagaccggattgacctgcaaaagatctggccggagtattccccttcctcgttacaggttgacgataaccaccgtatctacgccgcgcgttttaacgagcgcctgctcgctgccgtgcgggtaaccttaagcggcaccgagggagcactggattccctgcgcgtgcgggaagtcacccgccgtcgcggtgtggggcaatatctgctggaagaggttttgcgtaacaatcctggcgtttcatgctggtggatggcggatgcaggcgtggaagatcgcggtgtgatgacggcgtttatgcaggcgctggggtttacggcacaacagggcggctgggagaagtgttaatcgtcaagtttgatttcaaaagtgatattgcctgatgcgctacgcttatcaggcctacaatgtgtgttgcaatttactgatttctttggatcttgtaggccggataaggcgtttacgccgcatccggcatgaagcaacgtactcgatattagcaatttggcggcaacccaaagttgccgattaatgattacttcgcatcggtcgccgtgccgttggcgtgccagtcaaatacgccgaactcaaagcctttcagatcgcctttctcatcccaggtcagcggtcccattacggtatccacggagttcgctttcaggtatttggcgatttcagccggatcgtcagactgattcaggcccgcctgcaaagattgcagcgcggcgtaggtggtccaaacgaatgcgccacttgggtcctgttttttcgctttgatcgcgtcaacaatgggtttgttcgccggaacctgatcgtagttcttcggcttggtcaccagcagcccttccgctgattcgcccgcaatgttagacagcgaaacgttagccacaccttccggccccataaactgagttttcagccctgccgcgcgtgcctgacgcaggatttgccccatttccgggtgataaccgccgtagtaaacgaagtcgatattctcttttttcagacgcgccaccagcgttgagaaatctttttccccggcggtgatgccatcaaagaacaccacgtttgcattgcctttcttcaggccgtcctgcaccgctcgcgccagaccttcgccgtattgctgtttgtcgtgaacgatagcaatacgctgcggtttcactttctcaagaatatatttcgccgccgtcggcccctggtcggagtccaggccggtggtgcgcaggatcagctgatagccacgggcggtcagctccggcgcggttgccgctggggtgatcattaaaatgccttcgtcttcgtagatgtcagacgcaggctgcgttgatgaagaacagaggtgaccaatcacatatttaatgccgtcgttaacgactttgttcgccaccgcaaccgcctgtttcgggtcacaggcatcgtcatattttacgatttgcagtttgttgcctttaatgccgcctttagcgttgatatccgcaaccgcctgctctgcgccggtaaactcctggtcaccgtactgcgcaaccggaccggacattgcgcccacgaccgcgactttaatatcttctgccagagccatattgctgaatgccagcgcgatacatcctgccagtaacgctttaccctttatgttcatcctgagaatccccattcttctggttattacgtgtgttgtgatgttgtttttcagcactttatttcgttttatgcatgactacccgtgctttagcagcatactctgctaaaacatacccgatttttatgatattggaatagctattttgacagtttattaacaatctgcgtggggattggcgttttgccggaggggaaattgattattacagaggcccaaaaaacaaaaaccccggactctcatccagggttctctgcttaatagcggaaattacgcttcaatggcagcacgcaattttttcatcgcgttcttttccagctggcgtacacgctcagcggaaacgccgtaacggtcagccagttcctgcaacgtggacttgttgtcttcgtccagccagcgcgcacggatgatgtcctggctgcgttcgtccagaccctgcatcgcgtcggtcagacggtttgccgcctgctcttcccagttatcatcttcaatgccgtcggcaaagttagatgatttatcctgcagatagagcaccggagccatcggctggctgtcggaatcgtcgtcggaagacaggtcaaaggtcatgtcctgtgccgccatacgtgattccatctcacgtacgtctttgctggttacgcccagttcacgggccaccatttcgacttcatcctggttaaaccagcccagacgctgcttggttttacgcaggttgaagaacagtttgcgctgcgctttggtggtcgcaactttgacgatacgccagttacgcagaacgtattcgtggatctctgctttgatccagtgaacggcgaaggagaccaggcgcacacccacttccgggttgaaacggcgcactgctttcatcaggccgatgttaccttcctgaatcaaatccgcctgtggcaggccatagcccgcataattacgagcaatatgaacaacaaaccgcaggtgagacaggatcagcgttttagctgcttccagatcgccatggtaatgcagcttttcagccagcgcccgctcctcgtcagccgacaacatcggccacgcgttagctgcccggatgtaggaatccaggttgccaactggggctaaagctaaactttgcattttgtcagtcattcaaatcctctcaatcgatatcttctggcgcttcagtggtagcaacaactgtgccagagcttaagagcaacgaggttatcattcactgttttatcagaccgtgattttatccacaagttcaatgcaagcttgtgaataaattacgcacaaaatgtgacatagagatgaaataccgggaagagacaacggggtctctttccctgctacggaacccattgcagggaaagagtataacacgcttttattattcaggcgtaaagtggcgtaaatgttgtaccgtggcaagccacgctgccacccagccaatcatcgagcataccagcagcaatagcaggcattcatcgaatgataagccattgatatcaaacttcgttccgaaaacctgtgccacttccgcaaccgccgatgacaatcgcagcaccagaatttctgacaaaattaatgacaacaatgcgccagaaaatcccagcagtgcgccaccatacaggaacgggcgcaggatgaatccatctgtcgcaccaatcagtttctgtacgttaatggagtcacggcgagcaaagatactcagacgcacactgttaccgatgacgaggaacacggccgccaccatcaacacgccgatcatcgccgaaacgcgcccgaccagcccggtcaacgccgccagacgggcaaaccagctgtcatccatccgcacttcgtcaatgccgttaatctgcgtgatacgatcacgcagcgtattcagtgattccgtcccctggaaatcgagtttcgggatcaccaccgccactgccggaagcgggttttcttccagcatatccagcgcaccaccaaaaccagaccagttacggaactcacccagtgcgtcttcacgagaaagatagttcactttctccacgccttgctcggcctgcaactgtgccaccacgcccgcagcagcgtcatcgtccagcgttttttgcagataaacagtgatttgcggtgacggataatactgcgtcgccgcctggttaacgtttttgtacaccatataacagacgctgggcagcgtcagagaaatggcgataaccatcaccgttaaaaacgtggcgaacggtttgcttttcagatcctgcaatgcgccgtggaaggcatagcgcacctgttcgttgaaaacgttggttttgcgatttaccggttttggcgaggatttcgcgcgttttggtgcgttacgaccgccgtcgcctgagccgccgaccgatttacggaagcgatcaagacgcccgccaaactgccgaatatgattgattgcatcgcgcttattcatggcccacgcctccatgcaagtgaccatcgctcagggtgagcatgcgataggaacgccgcgagatcaggttgatgtcgtgcgttgccatcaatacggttaccccaacgcggttaaactcttcaaacagacgtaaaatgccttccgacagcgcgtcgtccaggttaccagtcggttcgtccgccagcagtaccgcgggcttgttcaccaccgcgcgggcaatgccaacacgctgttgttcaccgcccgaaagctgaatagggaagttcttcgctttgtccagtagcccgactttatccagcgccgccgacacccggcgacgaatatcgtcaccgctggcaccggcgataatcagcgggatcgccacgttatcgtagacagtacggtccatcagtagatggtgatcctggaaaatcatgccaatctggcggcgcagaaacggaacttcacggtttttcagacgcgtgatgtcatggccgctaaaccagattttcccggcgctgggccgctcaatcccacagatcagcttcaggagggtacttttccctgcgccggaatgaccggtcagaaacgccatctcacccggctgcatatggaacgtaacgccctgcagcgcctgtctcccaccgagataagccttgctgacatgttcaaagcgaatcattgttaatcctctcgggcaaaaagtgcctctataaagtcgtccgccttaaacggacgcaaatcctcaatacgttcgccgacaccaatgtagcggatagggataccaaactggtcagccaccgagaaaattaccccgcctttcgccgtgccgtccagtttcgttagcgtgatgccggttaagccaacggcttcatggaacagtttggcctggcttaccgcgttctgcccggtgctggcatcaatagtcagcataacttcatgcggcgcttcaacgtcgagtttcttcatcacgcggacgattttcttcaactcttccatcaggtgcgatttgttctgcaggcgtccggctgtatcggcaatcaggacgtcgatattacgcgctttagctgcctgaatggcgtcgaagataacagaggcggaatccgccccggtatgctgggcaatcaccggaatattgttgcgctgaccccagacctgaagctgttcaaccgcagctgcacggaaagtatcacccgccgccagcatcaccgatttaccctgctgctcaaactgacgcgccagcttaccaatcgtcgtggttttacccacaccgttgacgcccaccatcaggatcacaaacggcgctttgccttcaacattcagcggctcatcgactttcgccagaatctcgcccatctcttctttcagcaggccatagagcgcctcggcgtcacgaagctgcttgcgggatgcgccttccgtcagattggtgataattttacgtgtggtttccacacccacatcggcgatcaaaagctgctcttccagctcctcaaacagatcatcgtcgatttttttaccgcggaacaggctgataaatccggaaccgagattttctttggtttttaacaggctgcgtttcaggcgcgcgaaaaaaccttctttggtcggtttttcctgctcctgagcgatttcttccaccggctgctcttcttctgccggaggaaccaccatcaccgcctcttctgccgcttcggcagccagcgccgtttccagctcttcgtcggtaatttcttctttagccgcttcttcttccgccgcttcgacaatctctacggtttccgcttcagcctgccactcttctggcgaaaccgcttcggcgttgacgtcttccggcaacggcagctcttcacgttcgatagccactggctccggcgtttcttctacgaccggttccggctgtgcaacgacttccgcttcaggctgcgctttttcactttcagcaacctgttcagtgacttccacaacgtcggcagcaaaagtttccgcctcggcttcagtatgcgcttgcggctgctcttcaacggcttgttcagaggccttcacaggctcttgcgcctgaacgatttcttctacaaccggttgttcattctgaacttctgtctctttttccggggtctgctctttttgaccaaagcccagccaggaaaaaaagccacgttttttttctttcgccatttgcgactacactcctcgctgttgcttcatggcacagcgttaacgctatgtacatagcagctaaaaaaatgatgaaatagtctatcacttaacttaattcacatcaccgcctgcaagtatgtgttatctggcggattgagcaatttatcatgaaaaaaccgaatcattccggcagcggccaaatccgcattattggcgggcagtggcgaggccgtaaactcccggttcctgatagcccaggtctgcgccccaccaccgaccgcgtacgcgaaacgttgtttaactggctggctccggtcattgttgacgcccaatgtctggattgcttcgccgggagcggcgcgctggggctggaagcgttatcgcgctacgctgcgggggcaacgttgattgagatggatcgcgcggtttctcagcagttaattaagaatctggcgacactaaaagcaggcaatgcacgcgtggtgaacagcaacgcgatgtcattcctggcgcaaaaaggtacaccgcataatatcgtgtttgtcgatccaccgttccgccgtggcttgttagaagagacgataaatttactggaagataacggctggctggctgacgaagccctgatttatgtcgaaagcgaagtcgaaaacggtctgcccactgttccagcaaactggtcattacatcgggaaaaagtggcgggtcaggtggcttatcggctgtatcaacgcgaagcacaaggagaaagtgatgctgattaatattggtcgtttgttaatgctctgcgtttggggatttttaatcctcaacctggtgcatcccttcccacgcccgctgaatatcttcgttaacgtggcgctgatttttaccgtgctgatgcatggtatgcagctggcgctattgaaatccactttaccgaaagatggcccgcagatgaccaccgccgaaaaggtacggattttccttttcggcgtgtttgaactgctggcctggcagaagaaatttaaagttaaaaaataaccttattgttcgcctacaaagctgacaaagcgcgttcctttatagctcagcgtacctttatcgcccactgtcagggcgtggtactgctgggcgtcgaggcgaaacgtctgctccattcctccgctttgcggtttgaagcttgcctcatagcgtatactggtgcctgccggagtcacttcctgctggcgcgaacggcgatcgttaatcggtttttcccgcttgttgctcaccaccaccagcttttgctggagcggagccatatcattatcagctttttcccgtcgctgttgcataaaacgaaacgatgcggcgacgacaattaagccaatgataacaataaagaaaagaggtggtttgctcatctttatccctcatcggaaaatgcggaaataagcataccctgccagttatggtgttgtcatccgtccaccctcgccactaaactggaagcaagaccgtaggcattccgcttacgaaaaaataacgaattcaaggaactaagatgctttggtcgtttatcgctgtctgtctttccgcatggctatctgtggatgcatcgtatcgtgggccaacctggcaacgctgggtgtttaaaccgttaacccttcttctcctgctgttactggcctggcaagcgccgatgttcgacgccattagctatctggtgctggcagggctgtgcgcctcactgctgggcgatgcgctaaccctgttgccacgtcaacgtctgatgtacgccatcggcgcgtttttcctctcgcacctgctgtacaccatctatttcgccagtcagatgacgctctctttcttctggcctctaccactggtgctgctggttctgggtgcgctgttactggcgattatctggacgcgcctggaagagtaccgttggcctatctgcacgtttatcggcatgacgctggtgatggtgtggctggcaggtgaactgtggttcttccgtccgaccgctccggcgctctctgcgtttgttggcgcttcgttgctgtttatcagtaactttgtctggctggggagccactatcgccgacgcttccgtgcggataacgcgattgctgcggcctgctactttgccggtcacttcctgatcgtccgctcgctgtatctctgataaaacttgactctggagtcgactccagagtgtatccttcggttaatgagaaaaaacttaaccggaggatgccatgtcgactcctgacaatcacggcaagaaagcccctcaatttgctgcgttcaaaccgctaaccacggtacagaacgccaacgactgttgctgcgacggcgcatgttccagcacgccaactctctctgaaaacgtctccggcacccgctatagctggaaagtcagcggcatggactgcgccgcctgtgcgcgcaaggtagaaaatgccgtgcgccagcttgcaggcgtgaatcaggtgcaggtgttgttcgccaccgaaaaactggtggtcgatgccgacaatgacattcgtgcacaagttgaatctgcgctgcaaaaagcaggctattccctgcgcgatgaacaggccgccgaagaaccgcaagcatcacgcctgaaagagaatctgccgctgattacgctaatcgtgatgatggcaatcagctggggtctggagcagttcaatcatccgttcgggcaactggcgtttatcgcgaccacgctggttgggctgtacccgattgctcgtcaggcattacggttgatcaaatccggcagctacttcgccattgaaaccttaatgagcgtagccgctattggtgcactgtttattggcgcaacggctgaagctgcgatggtgttgctgctgtttttgattggtgaacgactggaaggctgggccgccagccgcgcgcgtcagggcgttagcgcgttaatggcgctgaaaccagaaaccgccacgcgcctgcgtaagggtgagcgggaagaggtggcgattaacagcctgcgccctggcgatgtgattgaagtcgccgcaggtgggcgtttgcctgccgacggtaaactgctctcaccgtttgccagttttgatgaaagcgccctgaccggcgaatccattccggtggagcgcgcaacgggcgataaagtccctgctggtgccaccagcgtagaccgtctggtgacgttggaagtgctgtcagaaccgggagccagcgccattgaccggattctgaaactgatcgaagaagccgaagagcgtcgcgctcccattgagcggtttatcgaccgtttcagccgtatctatacgcccgcgattatggccgtcgctctgctggtgacgctggtgccaccgctgctgtttgccgccagctggcaggagtggatttataaagggctgacgctgctgctgattggctgcccgtgtgcgttagttatctcaacgcctgcggcgattacctccgggctggcggcggcagcgcgtcgtggggcgttgattaaaggcggagcggcgctggaacagctgggtcgtgttactcaggtggcgtttgataaaaccggtacgctgaccgtcggtaaaccgcgcgttaccgcgattcatccggcaacgggtattagtgaatctgaactgctgacactggcggcggcggtcgagcaaggcgcgacgcatccactggcgcaagccatcgtacgcgaagcacaggttgctgaactcgccattcccaccgccgaatcacagcgggcgctggtcgggtctggcattgaagcgcaggttaacggtgagcgcgtattgatttgcgctgccgggaaacatcccgctgatgcatttactggtttaattaacgaactggaaagcgccgggcaaacggtagtgctggtagtacgtaacgatgacgtgcttggtgtcattgcgttacaggataccctgcgcgccgatgctgcaactgccatcagtgaactgaacgcgctgggcgtcaaaggggtgatcctcaccggcgataatccacgcgcagcggcggcaattgccggggagctggggctggagtttaaagcgggcctgttgccggaagataaagtcaaagcggtgaccgagctgaatcaacatgcgccgctggcgatggtcggtgacggtattaacgacgcgccagcgatgaaagctgccgccatcgggattgcaatgggtagcggcacagacgtggcgctggaaaccgccgacgcagcattaacccataaccacctgcgcggcctggtgcaaatgattgaactggcacgcgccactcacgccaatatccgccagaacatcactattgcgctggggctgaaagggatcttcctcgtcaccacgctgttagggatgaccgggttgtggctggcagtgctggcagatacgggggcgacggtgctggtgacagcgaatgcgttaagattgttgcgcaggagataaggcaaaccgatcgcaacattgagcgcgatcggtcccctcgcccctctggggagagggttagggtgaggggaaaaggcggcatcgaagccaatcagcccctatcaaccgcctttacgaatcaaataacgataaggcagtccatccgtctctttagcaaccagttcgtgttccataaaggtacaaaacccaggaatatcgcgggtagtggccggatcgtcggcgataatcagcaacgtttcgccaggctgcatattgcgcacggttttgcgcaccatcatcaccggttccgggcagcgcaggccaagcgcgtcgagtgtgtggtcagggctggaaaagagatcggtcattttcttctcatcacttaaaaaaacggcgctagtttacgccctgtgagtccgtaagcaaactaggttaacgattgcgtgaaaattaaccattgcattgtcaacgtaaagcagtatcatgcggcggctcgaaaaaagggtaagcacgttattatgttaaggtaacagacgtgtcgtacgtattgggttccctcaccccaatggttaatcaaaaaggtacaatatgaacgttttctcgcaaactcaacgctataaggcgttgttctggttatcgttatttcatctgctggtgatcacctccagtaactatctggttcagcttcccgtctccattttgggtttccataccacctggggcgcgtttagctttccgtttatttttcttgctaccgacctgaccgtgcgtatttttggcgcaccgctggcccgacgcattatcttcgcggtaatgatccctgcgttattaatctcctacgtcatctcgtcgctattctatatgggttcctggcagggattcggcgcactcgcccacttcaacctgtttgtcgcccgtatcgccaccgccagtttcatggcctacgcgctggggcaaatcctcgacgtgcacgtttttaaccgcctgcgtcagagtcgccgctggtggctggcaccgacagcgtccacactgttcggtaacgtcagcgacacgctggcctttttcttcattgccttctggcgtagcccggatgcctttatggctgaacactggatggaaatcgcgctggtcgattactgtttcaaagtgttaatcagtatcgttttcttcctgccaatgtatggcgtattactcaatatgctgttgaaaagactggcagataaatccgaaatcaacgctttgcaggcgagttaaaggttcgttatcagagttgtgataagatggatgaatgagccgttatggccgtttatcgaaaggaagaagtcaatgcgcaatctggttaaatatgtcggaattggcctgctggttatggggcttgcggcctgtgatgataaagacactaacgctacggcgcagggttcggtcgcggaaagtaacgctaccgggaatcccgtcaacctgcttgatggcaagttaagtttctcgctgccagcggatatgaccgaccagagcggtaagctgggaacgcaggccaataacatgcatgtctggtccgacgccaccgggcagaaagcagtcatcgtcatcatgggcgatgatccgaaagaagatctggcggtgctggcgaagcgtctggaagatcagcaacgtagccgcgatccgcagctgcaagtggtaaccaataaagccattgagctgaaaggtcacaaaatgcagcagttagacagtattatctccgcgaaaggccagacggcgtactcttccgttattctgggtaacgtgggtaatcaactgctgaccatgcaaattacgctgcccgctgacgatcagcaaaaagcgcagaccaccgcagaaaacatcattaatacgctggttattcagtaagttttaagatgatgaggcggcctcagggacgtgttccggaggccgtttttttaatcgccacgtcagtaataacgcgattgcgaccagtcccgccgccgccagataaatcaccggtacgcccgcccagctcatcaccagcccagccagtggtccagtcacgccaagcgataaatccataaatacggtgtaagttgccagcgccgccccctgattttgctgcggaaccgcttttaccgccactacacccaatgccgggaacaccagcgaaaacccggcccccgccagtaagacgccgattttcgccatccacggcatagtcgccacgccaaccagtagcaggccgattatctcaacgctaaagcaaatcatcgctacgtttaagccaccgatacggttaatgccgttagggaataacaaacgcgtaccgacaaacgcacagctaaacagcgtcagcgcgaaagccgcaccgtcccaacctttagcgtcataaaacagcgtgataaaggtggcgatgacgccaaatccggcggaagccagtgccagcgccataccgtacagccagacgcgcccaagcaccgcgcgaaacggcagcggtttgcctttactggcttttaccgtcggacgcgggatcgccaacaaaatggccaccagcgccacgcccataatgattaacgctaacgcctgcaagccgccccagtgataaaacacgacgcctaacggcgcacccatcgccatcgccccgtaagtgacaatgccgttccacgaaatcacccgcccgatatgcagcgagccaaccacgccaacgccccatagggtcgatcccgttccggcaaaactttgcccaatcccaaggatgacgcgccccaggcaaagtaataacaggctgatgacaggcagactggcggttaatcctgccgtcagataccccagaccgctcaaaaagcagccgcataaaccgaagacgacaatctttttgggtcccagcgaatcggcgtaacgtccggcatgagggcggctcagcaaggtggcgaaatattgcaggctgataaccaatcctgcccagaaggcgctaaagcccatcacatcatggacatagcccggtaatacagcgagcggcaacccgatggtgaggtagctggcgaagttaaacatgactatagagacaatgcgcaaattcaggcgcaatccgtttagcgcgggttcggctacgggttcgggcatgaggatcaccacatttttacaacagtgtttcatttttaccacgtgctgacgtgaaaatcagcagtaagaatcagaatattgctggcgtgactcccgctacacttaatacaaaaagtcacaaggaagccccaatggaaacccctcaacccgataaaacgggcatgcacattctgctcaagctggcctcgctggtagtgatcctcgcgggcattcacgcagcggcagatatcattgtgcagctgttactggcgctgttttttgccatcgtcctcaacccgctcgtcacctggtttattcgtcggggagtacaacgccccgttgccattacgattgtagtggtggtgatgctgatcgcactaaccgcgctggtcggcgtactggcggcatcgtttaacgaatttatctctatgctgccgaagtttaataaggagctgacgcgcaaactttttaaattgcaggagatgttgccttttcttaatttgcatatgtcgccggagcgaatgctgcagcggatggactcggaaaaagtggttaccttcaccacagcgctaatgaccgggctttccggggcaatggcgagcgtgcttttgctggtgatgaccgtagtttttatgctgtttgaagtgcgccacgtcccttacaaaatgcgttttgcgctgaataatccacagattcacatcgcgggattacaccgcgcacttaaaggcgtttcgcactatcttgcattgaagacgctactcagtttatggacaggtgtcatcgtctggctggggctggagctgatgggggtgcagtttgcgctgatgtgggcagtactggcgtttttgctcaactacgtgcccaatatcggcgcggtaatttccgccgtaccgccaatgattcaggtgctgctgtttaatggtgtttacgaatgtattctggtcggcgcattgtttttagtggtccatatggtcatcggcaatattttagaaccacggatgatgggccatcgcctggggatgtccaccatggtggtatttctttcattgttaatttggggatggctgctcggcccggtagggatgctactttcggtgccattaaccagcgtgtgtaaaatctggatggaaaccaccaaaggcggtagcaaactggcgattttactggggccgggcagaccgaaaagtcggttaccgggatgaggcgacaagtgatacgatacgcactttcattttccattaaacgttggccctgatatgtatcggatagttctggggaaagtttcgaccttaagcgcagctccactgccaccgggtttacgcgagcaagcaccgcaaggtccacgacgcgaacgctggctggcggggcgtgcattgctttcgcacacgctttccccgctaccggagatcatctatggcgaacaaggcaaacctgcatttgcgccggaaatgccgctatggttcaacttaagccatagcggtgacgatatcgccctgctgttgagtgatgaaggcgaagtcggctgcgatatcgaagtgattcgcccgcgcgccaactggcgctggctggcgaacgccgtattcagcctcggggaacacgctgagatggacgccgtgcatcctgatcagcaactggaaatgttctggcgcatctggacgcgcaaagaagccatcgttaaacagcgtggcggcagcgcctggcaaatcgtcagcgtagacagcacctatcactcctcgctgtcagtcagccattgtcagcttgaaaatttaagccttgcgatctgcacccctactccctttacgctcaccgccgacagtgtgcaatggatcgattcagttaactgatccgcccacccgactgcccatctattgatccagaacaggtaatcagtatgacgaatacttaaaatcgtcatacttatttccgccatctattttaatccattggggttaccatgctctccacactccgccgcactctatttgcgctgctggcttgtgcgtcttttatcgtccatgccgctgcaccagatgaaatcaccaccgcctggccggtgaatgtcgggccactaaacccgcacctttacacgcctaaccagatgttcgcccagagcatggtttatgaaccattggtgaaatatcaggcagacggttcggtgatcccgtggctggcaaaaagctggactcattcagaagatggtaaaacctggaccttcaccctgcgtgatgacgtgaaattctccaacggtgaaccgttcgatgccgaggcggcggcagaaaacttccgcgcagtgctcgataaccgtcaacgtcacgcctggctggagctggcaaaccagattgttgatgttaaagcactcagtaaaacagagctgcaaattaccctgaaaagcgcctactatcctttcctgcaagaactggccctgccccgtcctttccgttttatcgctccctcgcagtttaaaaaccatgaaaccatgaacggaattaaagcgccgattggcaccggaccgtggattttgcaggaatcgaaactgaatcagtacgatgtcttcgtccgtaacgaaaactactggggcgaaaagccagcgattaaaaagatcacctttaacgtcatcccggacccgactacccgcgcggtggcgtttgaaactggcgatatcgacctgctgtacggaaacgaagggttattaccgctcgataccttcgcccgctttagccagaatccggcttaccacacccaactgtcacagccgatcgaaaccgtgatgctggcgctcaataccgccaaagcccccaccaacgagctggcagtacgtgaagctcttaattacgcggtaaacaaaaaatcgctgattgataacgcgttgtatggcacccagcaggtcgccgacaccctgtttgccccttctgtgccctacgccaacctcggcctgaaaccgagccagtacgatccgcaaaaagcgaaagcgttgctggaaaaagccggttggacgctgcctgcgggcaaagacatccgcgagaaaaatggtcagccgctgcgcattgaactttcgttcatcggcaccgatgcgttaagcaaatcgatggcggaaatcattcaggctgatatgcgccagattggcgcagatgtctcgctgattggcgaagaagagagcagtatctatgctcgtcagcgcgacggtcgttttggcatgattttccaccgcacctggggcgcgccatatgatccacacgccttcctcagttcaatgcgcgtaccgtcacacgctgacttccaggcacagcaaggattagccgacaaaccgctgattgataaagagatcggcgaagtgctggcgacccatgacgaaacgcaacgtcaggcgctgtatcgcgacattctgacccgtctgcatgacgaggcggtttatctgcctatcagttacatctcaatgatggtggtatcaaaaccggagctgggtaacatcccctacgcgccgatcgccaccgaaattccgttcgaacagattaaaccggtgaaaccttaatgttgcgttacgtattacgccgctttctgctgctgatcccgatggtgctcgccgcctcggtgatcatttttctgatgctgcgcctcggtaccggcgacccggcgctcgattatttgcgtctgtctaacctgccgccgacgccggagatgctggcctctacccgcaccatgctgggactggatcagccgctgtacgtccagtacggcacctggttgtggaaggcgctgcatcttgactttggtatctcattcgccagccaacgcccggtactggacgatatgctgaacttcctgcccgccacgctggaacttgcaggtgcggcgctggtattaattctgctcacttccgtaccgctcggtatctgggcggcgcgccatcgcgaccgtctgccggatttcgccgtacgtttcatcgcgtttcttggcgtgtcgatgcctaacttctggctggcgtttttactggtgatggcgttttcggtgtatctgcaatggctacccgcgatgggttacggcggctggcagcacatcattttgcctgcggtttccattgcctttatgtcgctggcgattaacgcgcgtttactgcgcgccagtatgctggacgtcgccggtcagcgtcacgtcacctgggcgcgtctgcgcggcctgaacgacaaacagaccgaacgtcgccacatcctgcgcaatgcctcgctgccgatgatcaccgccgtggggatgcatatcggcgaactgattggcgggacgatgattatcgaaaacatctttgcctggccgggcgtcgggcgctatgcggtgtcggcgatttttaaccgtgactatccggtgatccagtgctttacgctgatgatggtggtggtttttgtggtctgtaatttgattgtcgatttgctcaacgccgcgctggacccgcgcattcgtcgtcatgaaggagcgcacgcgtgaactttttcctctcttcccgctggtcggtacgcctggcgctgatcattatcgccctgctggcgctgattgcgctcaccagccagtggtggctgccgtatgacccacaggcgattgatttgccgtcgcgcctgctttcgccggatgcgcagcactggctgggcaccgatcacttaggtcgcgatattttctcgcggctgatggcagcgacccgcgtgtcgctcggttcggtaatggcctgcctgctgctggtgctgacattagggctggttattggcggcagcgccgggttgattggcgggcgcgttgatcaggccaccatgcgcgtcgccgatatgtttatgaccttcccgacctcgattctgtcgttctttatggttggcgtgctcggcaccgggctgaccaacgtaattatcgccatcgccctgtcgcactgggcgtggtatgcacgcatggtgcgcagcctggtgatttcactacgccaacgcgagtttgtgctggcgtcacggctttccggtgcgggccatgtgcgggtgtttgtcgatcatctggcaggcgcggtgatcccttcgctgctggtgctggcaacgctggatatcggccatatgatgctgcacgtcgcggggatgtctttccttggcctcggtgtgaccgcgccgaccgccgaatggggcgtgatgattaacgacgcgcgccagtatatctggacccagccgctgcaaatgttctggccggggctggcgctgtttatcagcgtgatggcctttaacctggtgggtgacgcactgcgcgatcatctggaccctcatctggtgacggagcacgcacactaatgccgcaacagattgaactacgtaatatcgcgctacaggccgcgcagccgctggtacacggtgtatcgttaaccctgcaacgcgggcgcgtgctggcgttagtcggcggtagcggcagcgggaaatcattaacctgcgccgcaacgctgggcattttgcccgctggcgttcgccagacggcgggggaaattttagccgatggcaaaccggtttcgccttgcgccctgcgcggcatcaaaattgccaccatcatgcagaacccgcgcagcgcctttaatccactgcacaccatgcacacccacgcgcgggaaacctgcctggcgttagggaaacccgccgatgacgctacgcttaccgctgccatagaagcggtggggctggaaaacgccgcgcgcgtgctgaagctgtacccgttcgagatgagcggcggcatgttgcagcgcatgatgattgcgatggcggtgctgtgtgaatcaccgtttatcatcgccgatgaaccgaccaccgaccttgacgtggtagcacaggcgcgcatcctcgatctgctggaaagcattatgcaaaaacaagcgccgggaatgctgctggtgacccatgatatgggcgttgtggcgcgtctggcggatgacgtggcggtgatgtctgacggtaagattgtcgaacagggcgatgtagaaacgctgtttaacgcccccaaacatacagtgacgcgcagcctggtttccgctcatctcgccctctacggtatggagctggcatcatgactttacttaacatctccggcctttcccatcactatgcgcacggtggatttaacggaaaacatcaacatcaggcggtgctgaataacgtttccctgaccctgaaaagcggcgaaaccgtcgccctgctggggcgcagcggctgcgggaaaagtaccctcgcgcggttgctggtgggtttagaatcgcccgcgcaggggaatattagctggcgtggcgaaccgctggcgaaactcaatcgcgcccagcgtaaagcgttccgccgcgatattcagatggtatttcaggactccatcagcgccgtgaatccgcgcaaaaccgtgcgcgagatcctgcgtgaaccgatgcgccacctgctatcactgaaaaaatccgaacaactggcgcgcgccagcgaaatgctgaaggcggtcgatctcgatgacagcgttctcgacaaacgcccaccgcagttaagcggcggccagctccagcgcgtctgcctggctcgcgcgctggcggtcgaaccgaaactactgattctggatgaagccgtttctaaccttgatctcgtgttacaggcgggtgtcattcgcctgctgaaaaagctacaacaacagtttggcaccgcctgcctgttcatcacccacgacttacgcctggtagaacgcttttgccagcgggtaatggttatggacaacggacaaatcgtcgaaacccaggtggtgggagagaaattaaccttttcctctgacgccggacgtgtgctacaaaacgcggtattacccgcattccccgtgcgccgtcgcaccacagaaaaggtttaacgcaaatgcaacgagtcaccatcacgcttgatgacgatttactggagacgctggacagcctgagccagcgtcgtggttataacaaccgttccgaagctatccgcgacattctgcgtagcgccctggcgcaagaggccacccagcagcacggcacgcaaggtttcgcggtgctgtcgtatgtgtatgaacacgaaaaacgcgacttagccagccgcattgtctccacccagcatcatcaccacgacctctccgtcgccacgctgcatgtgcacatcaaccacgacgactgtctggaaatcgccgtgttgaaaggtgacatgggtgacgtgcagcattttgccgatgacgttatcgcccagcgcggcgtgcggcacgggcatttgcagtgcttgccgaaggaagattgagtctattattgggtcctttggtgaacgatcaacaaagggccactagcacacctgattcctctctaaataccctatccgaaccttctcttttgtaacgttctaaatatattcctaaaaatcttcaattcattgtgaccacaagtttttcttcgctttttcgtatgaagatactgtcattaaaataatagaaaaggattttacgatgagcggaaaaccggcggcgcgtcagggtgacatgacgcagtatggcggtagcattgttcagggttcagccggggtacgtattggtgcccccaccggcgtggcctgttcggtgtgccccggcggagtgacgtccggccatccggtcaatcccctgctcggtgcaaaggtccttcccggtgaaaccgacatcgccctgcccggcccgctgccgttcatcctctcccgcacctacagcagttaccggacaaaaacgcccgcgccggtggggagcctcggccccggctggaaaatgcctgcggatatccgcttacagctgcgcgataacacactgatactcagtgataacggcggcagaagcctgtattttgagcacctgtttcccggtgaggacggttacagccgcagcgagtcactgtggctggtgcgcggcggcgtggcgaaactggatgaaggtcaccggctggccgcactctggcaggcgctgccggaagaactccgcttaagtccgcatcgttatctggcgacaaacagtccgcaggggccgtggtggctgctcggttggtgtgagcgggtgccggaagcggatgaggtgctgcctgcgccgctgccgccgtaccgggtactgaccgggctggtggaccgcttcgggcgcacacagacgttccaccgcgaagccgccggtgaattcagcggcgaaatcaccggcgtgacggatggtgcctggcgtcacttccggctggtactgaccacgcaggcgcagcgggcagaagaagcccggcagcaggccatttccggcgggacggaaccgtccgcttttcctgataccctgccgggttacaccgaatatggccgggacaacggcatccgtctgtctgccgtgtggctgacgcacgacccggaatacccggagaatttacctgccgcgccgctggtgcgctatggctggacgccacgcggcgaactggcggtggtgtatgaccgtagtggcaaacaggtgcgcagctttacttacgatgataaataccggggccggatggtggcgcaccgtcacacgggccggccggaaatccgttaccgttacgacagcgacgggcgggtgacagaacagctaaacccggcaggcttaagctacacgtatcagtatgagaaagaccgcatcaccatcaccgacagcctggaccgccgtgaagtgctgcacacgcagggcgaagccgggctgaagcgggtggtgaaaaaggaacacgcggacggcagcgtcacgcagagtcagtttgacgccgtgggcaggctcagggcacagacggatgccgcaggcaggacaacagagtacagcccggatgtggtgacgggcctcatcacgcgcataaccacgccggatggcagggcatcggcgttttactataaccaccacaaccagttaacgtcagccaccgggcctgacgggctggaattgcgccgggaatatgatgaattgggccgtctgattcaggaaactgcccctgacggcgatatcacccgctaccgttatgataatccacacagtgacttaccctgcgcaacggaagatgccaccggcagccggaaaaccatgacgtggagccgttacggtcagttgctgagcttcaccgactgttccggttatgtaacccgttatgaccatgaccgcttcgggcagatgacggcggtgcaccgcgaggaagggctgagtcagtaccgcgcatacgacagccgtggacagttaattgccgtgaaagacacgcagggccatgaaacgcggtatgaatacaacatcgccggtgacctgaccgccgtcattgccccggacggcagcagaaacgggacacagtacgatgcgtggggaaaggccgtccgtaccacgcagggcgggctgacgcgcagtatggaatacgatgctgccggacgggtcatccgcctgaccagtgaaaacggcagccacaccaccttccgttacgatgtacttgaccggctgatacaggaaaccggctttgacggccgcacacagcgttatcaccacgacctgaccggcaaacttatccgcagcgaggatgagggtctggtcacccactggcactatgacgaagcagaccgcctcacgcaccgcaccgtgaagggtgaaaccgcagagcggtggcagtatgacgaacgtggctggctgacagacatcagccatatcagcgaagggcaccgggtggcggtgcattacaggtatgatgagaaaggccggctgaccggtgagcgtcagacggtgcatcacccgcagacggaagcactgctctggcagcatgagaccagacatgcgtacaacgcgcaggggctggcgaaccgctgtataccggacagcctgcccgccgtggaatggctgacctacggcagcggttacctggcaggcatgaaactcggcgacacaccgctggtggagtacacccgcgaccgcctgcaccgggaaacgctgcgcagcttcggccgttatgaactcaccaccgcttatacccctgccgggcagttacagagccagcacctgaacagcctgctgtctgaccgcgattacacctggaacgacaacggcgaactcatccgcatcagcagcccgcgccagacccggagttacagctacagcaccaccggcaggctgaccggcgttcacaccaccgcagcgaatctggatatccgcatcccgtatgccacagacccggcaggtaaccgcctgcccgacccggagctgcacccggacagcaccctcagcatgtggccggataaccgtatcgcccgtgacgcgcactatctttaccggtatgaccgtcacggcaggctgacagagaaaaccgacctcatcccggaaggggttatccgcacggatgatgagcggactcaccggtaccattacgacagtcagcaccggctggtgcactacacgcggacacaatatgaagagccgctggtcgaaagtcgctatctttacgacccgctgggccgcagggtggcaaaacgggtgtggcggcgtgaacgggacctgacgggctggatgtcgctgtcacggaaaccgcaagtgacctggtacggctgggacggcgaccggctgaccacgatacagaacgacaggagccgcatccagacgatttatcagccggggagcttcacgccactcatcagggtcgaaactgccaccggtgagctggcgaaaacgcagcgccgcagcctggcggatgcccttcagcagtccggcggcgaagacggtggcagtgtggtgttcccgccggtgctggtgcagatgctcgaccggctggaaagtgaaatcctggctgaccgggtgagtgaggaaagccgccgctggctggcatcgtgcggcctgaccgtggagcagatgcaaaaccagatggacccggtgtacacgccggcgcgaaaaatccacctgtaccactgcgaccatcgcggcctgccgctggcgctcatcagcacggaaggggcaacagcgtggtgcgcagaatatgatgaatggggcaacctgctgaatgaagagaacccgcatcagctgcagcagcttatccggctgccggggcagcagtatgatgaggagtccggcctgtattacaaccgccaccgctattatgacccgctgcaggggcgatatatcactcaggatccgattggactgaaggggggatggaacctgtatggatatcaattgaatccgatatcagacatcgaccccctgggtttatctatgtgggaggatgcaaaatcgggggcatgtactaatggtctttgcggcacactatccgctatgataggtccagataaatttgattctatagatagcaccgcatatgacgccttaaataaaataaatagccaatctatttgcgaagataaagagttcgctggtttaatatgtaaggataatagtggcagatatttctcaacagcacctaaccgaggagaaagaaaaggatcatatccattcaatagcccttgccctaatggtactgagaaagtatcagcttatcatactcatggtgcagatagtcatggagaatattgggacgaaatattttcaggtaaagatgagaaaatagttaaaagtaaagataacaatatcaagtcattttatttaggtacgcccagtggtaattttaaagcaatagataaccacgggaaggaaataacaaacagaaaaggattacctaatgtctgcagagttcatggtaatatgtaaaaaaatattgtttaggaactgtgtcattgtatctttgtttgtttttacatacaacacatgggcgcagtgtaataataatattaaaataatgcgcaagtatgaaagtgaaggtaaatataccgttagaaatttggttaaaaataaagctatagcattggaattagctgagatatatgttaagaatcgttatggacaggatgccgcagaagaagaaaaaccatacgaaatcactgagttaacaacaagttgggttgttgaaggtaccattcactcagaccaaattgctggtggggtttttattatagaaataggcaaaaatgatgggagaattctgaattttggccacggaaaataagtatgtaaggataatcaaacatcgtgtgcgctgatggcagagtaggtggaggactccagacagtcaaacgatagaaaaagatagcctttatggaggttcctgcaatgtcaaatacataccagaaaagaaaggcaagtaaagagtatggtttatataataaatgtaagaaactaaatgatgatgaattatttcgcttacttgatgatcgcaattccttgaaaaggatttcatctgccagagtattacagttaagaggggggcaagacgctgttagattggcaattgaattctgcactgacaaaaattatatccgtagagatatcggagcatttatactcgggcaaatataaatttgcaaaaaatgcgaagataatgtttttaatattttgaacaatatggcattgaatgataagagtgcttgcgttcgagctacggcaatcgagtcaacggccagggaaagatcatcaaaagttcactttttgcactaaataattcgcattttatgtttaaaaattgagatattccttattacctgaagctgttttttattgcttatacatgatcaaatactccttacctaattaaggagaacaaaatggaacttaaaaaattgatggaacatatttctattatccccgattacagacaaacctggaaagtggaacataaattatcggatattctactgttgactatttgtgccgttatttctggtgcagaaggttgggaagatatagaggattttggggaaacacatctcgattttttgaagcaatatggtgattttgaaaatggtattcctgttcacgataccattgccagagttgtatcctgtatcagtcctgcaaaatttcacgagtgctttattaactggatgcgtgactgccattcttcagatgataaagacgtcattgcaattgatggaaaaacgctccggcactcttatgacaagagtcgccgcaggggagcgattcatgtcattagtgcgttctcaacaatgcacagtctggtcatcggacagatcaagacggatgagaaatctaatgagattacagctatcccagaacttcttaacatgctggatattaaaggaaaaatcatcacaactgatgcgatgggttgccagaaagatattgcagagaagatacaaaaacagggaggtgattatttattcgcggtaaaaggaacccaggggcggctaaataaagcctttgaggaaaaatttccgctgaaagaattaaataatccagagcatgacagttacgcaatcagtgaaaagagtcacggcagagaagaaatccgtcttcatattgtttgcgatgtccctgatgaacttattgatttcacgtttgaatggaaagggctgaagaaattatgcgtggcagtctcctttcggtccataatagcagaacaaaagaaagagccagaaatgacggtcagatattatatcagttctgctgatttaaccgctgagaaattcgccacagcgatccgaaatcactggcacgtggagaataagctgcactggcgtctggacgtggtaatgaatgaagacgactgcaaaataagaagaggaaatgcagcagaattattttcagggatacggcacattgctattaatattttgacgaatgataaggtattcaaggcagggttaagacgtaagatgcgaaaagcagccatggacagaaactatctggcgtcagtccttgcggggagcgggctttcgtaatcttgccctgaatacaggactgagtatcaaaaagccggttaactgaaactgtccaggttttgggggtcagttcataaacgccttatccggcctaaaaacaactaaaattcaataaattgcaccgatgcgtagtccctataagcttacgcatcgggcaattgtatttacgccattgtcccaatcgtcttcctgaatcgcagcagcgcaatggtgaaaaatgcgccgccaattgccatcagcgtcagaaactgcggccagacgatttcgaatccggcaccccggtagaggatggcctgcgcgaggctaacaaagtgtgtcgtcggcatggtcagcataatgtcctgcaccatctgcggcatactttcgcgcggcgtggaaccaccggaaagcatttgcagcggcagcagcaccagaatcaccagcagccccagttgcggcattgaacgcgctatcgtccccataaaaatgccgattgacgtggtggcaaacagactgagcgccacgcccagcataaacagcgggatcgagccttcaatcggtacgcccagtacacctttcaccatcagcaccagcgataatcccgataccaccagcaccaccagccccatcgaccagatcttcgccatcatgatctcaaacggcgttatcggcatcaccagtaagtgttccaccgtgccgtgttcacgctcgcggatcagcgccgatccggtcaatacaatcgccagcatggtaatgttgttgatgatcgccatcaccccgccaaaccacgcgggatcgaggttcgggttaaagcgcatccgggtttccagcgataccaacggttcgctgttatcacggtagcgcgcgacaaagctgttcacttcaccgttgataatattctggatatacccattgccggtaaatgcctggctcatgcgcgtggcatcgacgttcacctgaatatccggctggcgtccggcgaggacatcacgctgaaaattaggcggaatatttatcgcgaaggtatagcgtccggcgtccagtccggcatccatctcatcggcggtgatcatctccggtggcaaaaaccacggacgatagaagctgttaacgatccggttcgataactgcgattgatccatatcggcaatggcgatcggcgcgaggttcaacgatcctggcgtaacggtcgctgacgaatacaccgacaccgtaaacgagaagacaatcagcgtcagcatcgctttatcaccgagcagactgcgcaactctttgatacccagattaaaaatattgcgtaaatggcgcatcatccctcctgttttttcagcagcaggatacttaagcccatcaccagcgggatggctatcagtaacgggataaaaagttgccacaaatcagtcagatccagcgctttcgagaacgtcccgcgggcgatagtcagaaaatgactggtcgggtaaacctcgccgatccaacgtccaggcccttccagcgaagctaccggatcgatcatcccggaaaactgtgtcgccgggatcaacgtgataatcgccgttccgaaaatggcggcaatctggcttttcataaaggtggagatcagcagccccattccggtggcaatgatgatatacagcagcgccgccagggtgagcgtcaggaaactgcctttatgcggtacgccaaacacaaacaccgacaggccgcagagcaggaaaaagttcagcatccccagcgcgatgtatggcaactgtttaccaagcaaaaattcactacgcgtggtgggggtcacgtaaaggttgataatcgacccaagctctttttcccgcaccacgctaagggcgcttagcattgacgggatcatcatcagcagaagcgggatcaccgccggaacaatcgctggcaggctttttacgtccgggttatagcgatagcgcgtctcaatattcatcagcccgctttggctggcgggtgtcgattgtcggctcgccacatcctgtaaccagctctggtgcatggcctgcacgtaaccttttaccgtttcagcacggctcggcatcgctccgtcgatccagacgccgagttccacaggcgtaccacgcgcgatatcgcgcccgaaattgggcgggatctcaatcgccaccgtgatatcgcccgcacgcatccgacgatcaagctcgtcataactggtgagcggcggctgttcgataaagtaacgggaaccggagaggttgagtgtccacgcctggctactgacggtctggtcgcggtcgagcaccgcaaagcgcaggttttccacatccatactgatgccgtaacccattatcagcatcaggatcaccgttcccatcagcgccagcgtcgaacgtactggatcgcgtcgcagttccagcgcttcgcggcggctgtagctaaacagacggcgcaggctaaatccctgacgcggcgcgtgggtggtgtcgtgtaccacgggcggcgcttcggcttcgttgctctgccctgccgcttcctgcaaataggcgataaatgcctcttccagactggcggctccgcgtttctcaaccagttcctgcggtgtaccgctggcaagcacttttccggcgtgcatcagtgagatgcggtcgcaacgttccgcttcgttcataaagtgggtggagatgaagatagtcactttgtcctggcgcgagagatcgaccatcaactgccagaacatatccctcgccaccggatcgacaccagaagtaggctcatcgaggattaacatctccgggcgatgaatcaccgccaccgccagcgaaagccgctggcgaatgccgagcggcaatgactccggcagaatatcttcaacgtcgttgagcttaaaacgctcgctcatttcagccactcttgcgggaatttccgcttccgggatgtgaaacaaacgggcatgtaactcaaggttttgccgcacggtgagttcgttatagagcgaaaacgcctgcgacatatagcccacccgacggcgggtatcgatatcttttggatcaaccggttgcccgaacagccacgcctcaccttcgctggcgggcagcagtccggtgagcattttcatggtggtggatttaccgcagccgttcgaaccaagaaaaccaaaaatctccccgcgtggaatgcggaaattaacgtgatcaacggcaacgaaggaaccaaaacgcatggtcagatcgcgcgcttcgatggcaatctctgcgttttcaggttgatacggtgggatcactaccgcctgatgcgcctggcgttgcgcttgcggtaacagatttataaatgcttcttccagcgtagcgctttgcgtttgctgccgtagctcttcggcgctgccagttgccagcacttctccggcattcatcgctaccagccagtcgaagcgttcggcctcttccatataggcggtggcgaccagcacgctcatattgctctgccgctggcgaatactgtcgatcagatcccagaactgggagcgggagagcgggtcaacccccgttgttggctcatcaaggatcaacagttccgggtcgtggattaacgcgcagcacagcccaagtttttgcttcatcccgccggagagtttccctgccggacgatcgcgaaacggtgctaacccggtgctggtcagcagctcattgattcgcacttcccgctccgctttgtcgtgaccgaacaggcgagcgaaaaaatcgacgttttcatacaccgacaaggtgtggtagaggtttttgcccagcccctgcggcatccaggcgatgcgcgggcagacgtcgcggcgatgcttcgggtcgcgcatatcgccgcccagcaccatcacattgccctgttcaatgacgcgggcaccggaaatcaacgacaacaagctcgacttcccgacgccgtccgggccaatcagcccgaccatacagcgggccggaatatcgagagtgatattgttcagcgcaacggtttttccataatgctggctcacgcccgccagttgcgcgacaggcgggacgggaaccagttccagatgcgtcattgcggcaacctcaccacgaggtcgtcaggccacggaagttcttcattcacccgcacccacgctacgcccggcaaaccggttttgacatattccagatgctgctggagtaattccggtgggatacgcgctttgacgcggaacatcagtttcagccgttcatcgctggtttcgacggtttttggcgtgaactgggcgacactggcgacaaaactgatggttgcaggaatacgcagatctggcgcggcatcgaggatcagccgggcttcaccgcccagtttcagcgtgcccgcctgttcggttggcaggaagaaagtcatatagacgtcgctgagatcgaccatattcagcacccgaccgcctgccgccagcacttcgcctggctcggcaacccgatactgcacgcgtccgtcacgcggggctttcagttcgctgtcatcgatatctgcggcaatgcgccgttcagtggcttgtgccgcttcgacgcgggtttgcgcctgaatgatattggtgcgtgccgcttctatagccgctttagaagccgatacctgagctttcgccgattccagcgcagctcgggcgctctcagcggcggcgcgatcgtcatccagctgttgcgcagaaatagcccctcgttgggccagtgaacgggaacgcgtatgacgttttgctacggagtccagttctgcctggcgttgattaaccagcgactgtgcggcacgagtttcgctttgtcgttgctccagcaaagcctgcgcggcagcaacggcgctttgtgcctctttgatttgcgcgatggcttccagtcgctgttcctgcaacacgcgagtatccatcttcgccagcacttcaccttcgcgaacaaacttgccttctttcaccagaatggtgtcgatacgcccggcaattttgctggcaatatccacttccgtcgcttcaatgcgcccattactgacagcaaagccttccggcacacctgccgggcgcaacagccaccacgccacgatagccgccaccgccagtaacccgacaacccaccacgccagatggcgcttactcttatccataatcgacccgccataatccctgtaagcaaacgacgcgtgttacaactgccgccgaacgacgttcagcggattcttccatccgggataagaaggaaacggcaaatacgaccagcgcgcagagcattgagcgccaacggggaaggcttagtgaaaacgggtagtaatgttgtcatcatcagcattcctggccgtaaatgaaacacgcatactcataagtgtgatctataaaactggctgacaaaacggtatccatcctgttggatagcgtttcacgcctgttcagttgcaggaacagagcattcctttttacgttttatcaacagtctcaaccagatagtaacattaatattcatgttgtctatggttcagagctgtaacattgtgcgccttctaatcaaaggcataagtccatttctgtttttttcatgctggtaagacttccagggagtggttatctcaggccctgcaccagggttaatttggcaattatgcatgctgaacattcttccagcatgtttactgtcacgggcgttaagacctaaaactgtccccgtttcgcctatgcgttctcttccaccatttccgttatgtgcaacaacttgatttatacctaacatttgtgaacatgctaatagtgcttcaagtttaggtctgtaatctgtcgaaacagaaaaataacgattaaaggatcgacaagagatagcccggctagttttaaactttttgccattaattatagcatgatgctttttattgataattgccgctaattcgaccggatcgagagcattggtcatttcatcaatagagactgttatcggtcctataatgtaacgttttcgctgatcatcaaaagttatcccatgatgatttgccattattttgtatttggggtcatagaaacatacaggataatcttttatcccagagtaggtatcctcatcgagtggtttcatacgcgtgaagttctgcatatagttaccattgcaattcgtttcatgatttccagctaatacatgaacattttcattgatactcattatgcgttttaacaaatcgatgataaattgatcaccacagatattgctaaatcgatcgccggtttggtcgcccagaaacgtacatggcgtcacagcgtctttattaataactaaataaggctgaagactttctaaaataatgtctcttctgttcaggatactgattattgtattaacattagtgttaagttgctcattaaagttctcccttagcaatacgttgagaacttcatcttctatattaagcaactggctaaggaaattttctccttcagccatgattcccaaatgtcccgttgcgaaaagcgcgaacaaaactgcaccgactgagccatcggtatcaccaaaataggttggtctggtacttgtgggatcaacgggtaaacaattggagaaatagattctgtcagcgaactggggttttatcattgtttcgaatttaatatcagatacattatattgcgatattttccagttccagatgggtttgtacgactcagtaactgcaacatcattagcattatcatttactgtcatattattaagtaaataaacaatactgcaccaattaatatcggtattatcaagagagcaaccgtaatttttgctattaattgtcacaataaactgataattattattcctacgtagaatatgagcacgcatgcccgatagcatactatatttttctgaatgatccgtttgtatggtaaatgaaattttgtcatcttgaatagattgttggaaccgttctatttgccaatcatctattttttccacaacctcaccgagcattgtcctggcaatacttgatatatcatcacctataccatttgcaatatacccaaacagttctttagtgaagttggtaacatgctcttgcaccatatcatttgttgcgattgtcgttgtactgtcgttagtgcctgccacagttccaattttcatattttacctcatattatttaccgcgaggaatacatagttaacattttatcttatgacatacacctcatgttcgatgggaaaataattatattttgcacaaatcattcagcctcaaagcataatatgaaatttcttatctcatagcagagaaagtccctaaagattgtagaggcgtcatcagaacatgcctctacaatcgattaagaaaacctatgaaatactggcaggattaaaaagacataccaccgtattcatggagttttaatgtagttgaaaacaactaagccctgaggaataaattattttattatttttatcacgtgcttccttcagggaatttagccccataataccattatcaaattgttgattatgatctaccccgggcccatgatgcccatatttttgtctaatgtatttgctggggtcttcacctttgagtgtctccccacatatgaagatacgttcacgtgctggtctgaaatcagtagtgttatcaaaataattagcatatacaggtgtgggtttcaaagtattgcttcggattagatggaatagaggatcatccatgtgttctttatgttttttattaaaaatattggctaattcctcaggatcagtaggatttttcatctgattaaatggaacctgcaaagcaccgagacaataacatttttttcttcatctcttattattccgtgatgactggttaaaacttgcctttctgagtcataattacaaacatcgagcgttttaattaagttatacgtatcaccggcagagagtttatgatttgctagtcgtgcagtatagttaccattaaaattgatttcatgatttccagccagaacgacgacatttttattaatacggctatctttattaccctccatatttcgcatagaatttagcaaagtaaggatatatttatcaccaaaaatagtactaaatctatcgcctgtatgatccccaaggaagatacaaggggttatcgcatcgtcctttaaaaaaacatgttgatgcaactcattcaagatcatgtctctcgtatttaataaatcgtagagcactttattatttttatgtttgtatgcagatgaagccatctcttcgtgttttaataattcacataataaactccaacccttttccctgatgcctatatgccctgaaacgagcaatgcataaagtacagcgcctactcttccatctgtatcgccaaaataagccgtgttggcattttgtgggttaatcacaccacactgtttatagaagtctatttttgaaaacacagatttaacatagctatcaaacttttccttagtaaacgtctctttagagacatcccaacgccagtcaggtttgaaattaccactaagaagagtaaagaaatttctcgctatgatagaaagcccatcaactttataaattatatctgatttatctccagaggaattaataaaataataaccgcccttacactcaacagtaacggtaatgggagacgataattttaacacatggttattgtctggtataattgtaaagataaacgtatcagtagtattgtcggcgaatctattatattcttgaatatctatagaaggttcactattataaaaccatactttctccatctggtgactacgatcatttaccttccagtgaccatgttgcaggaaatagatgatatgcaggccaaaatcgttatctatttgcgaatcattatccagtttatcaaattcaactatctttgcacgatgtgttttatcaaccttgccatggtgttgatgactgttaactttatctgaatgcttatcttgatggcttgaagagatgtttctaatctgattgtcaattgctttcataaataacctgtgatatttttgaattgtttgtaacaaaataaatgatacttgtctgaaaaacagatttacgacgatataaaataataatacttatatgttcgctgattttaagcaccgagactatccggtcttttaccaaataatgaagaataatccctccctggaagataattgtaaaaaacaacagcataagaattaatcttaggataaatttttatttatcatggccttttgaacgctgaaaagtagcgctctgcaaagtaaaccccgctatagttatgctatgcatttgtctttaatgatatctcgtcattatattaacaggatgaaattatcattaatgcatatttcaatattagcagggatacctgaggagtttaaagtgaacatatatatcgggtggcttttcaaattaatccctttgattatgggcttaatttgtatcgcgttaggtggctttgtgctggaaagttcagggcaaagcgagtatttcgtcgcgggtcatgtgctgatttctctggcggccatatgcctggcattattcactaccgcatttattatcatttcgcagctcacgcgcggcgttaatacgttttacaatacattgttccccattattggctatgcggggtcaattatcaccatgatatggggttgggcactgttagcaggcaatgatgtgatggcagacgagtttgtcgccggccatgttattttcggcgttggtatgattgccgcctgtgtatcgacggtggcagcgtcatccggtcactttctgctcattcccaaaaatgcagcggggagcaagagcgacggaacaccggtacaggcttattcttcattaatcggtaactgcctcattgccgttcccgttttactcaccctgctcggtttcatttggtctattacgctgttacgtagtgctgacataactccgcattatgtcgcgggtcacgtattgcttgggttaaccgcaatctgtgcctgtctaattggccttgttgccacaattgtccatcaaacacgtaatacgttttcaactaaagaacactggctgtggtgttattgggttatttttctcggctcaatcacggtactgcaggggatatacgtcttagtcagttccgatgcaagcgcccgactggctcccggcattattcttatttgcctcggaatgatctgttacagcatattctcaaaagtctggctactggcactggtatggagacgtacctgttcgttagccaacagaataccgatgattcccgtcttcacctgcctgttttgccttttcctggcatcgtttcttgcggaaatggcgcagaccgacatgggatattttattccttcgcgagttctggtcggtttgggagcggtatgctttacgttgttctcaatcgtttcaatattagaagcgggttctgctaaaaaataattgcaacgtaccggataaaaccagcgttgaccatttgcgtaacgctggtttttcttaggcatcatgaaataacgcagcattaatgcatagtggttaagtataaaaaacagcaaagttactgtttttttcaacctgttcatatttcataaagatctggccactgagtgagttttcaatcacctttccatccaccttatattaagcatggagggtttcagttcacgggctcattagaaaataatcacaagataaccactatcaaaattagctcatttttaatgcgactctaataattttcatctttaggaaataggtcaggacgactttgctgcaatcaaatcctgcgcacaagcccacgcactcgaccacgcccactggaagttatagccccccagccagccggtgacgtccatcacttcgccgatgaagtacagcccaggcactttgcgcgcttccatcgtccgtgaagagagttcgttggtgtccacgccgccgagcgtcacttcggcagtgcgatagccttcagtgccgttgggttgtacgcgccagtcggtcaatgtgctaatcagtgcctgttggtcacgcacgttgagctgttttagcgaaacatccgggatttgcccgagttgctgtaagcgttcaaccaaccgcttcggtagatgaaccgccagtgtgtttttcaggctttgattcggatgtgcgttacgctgctcattcaggaaggtttcgaggtccacatccggtagcagattgatgctgacaaattcccccggttgccagtagcttgaaatctgcaacaccgccggtccagacaagccgcggtgggtgaagagtaagttctcacggaaaacggtgccgttttcagcggtaatcacggaaggcaccgccacgcccgccagcacctgtaactcttcgagcaacggtttatgcagagtgaatggcaccagacccgcgcgggtcggcagcacgttgaggccaaattgttcggcaatcttataaccaaacggcgacgcgcccagccccggcattgacagcccaccagtcgcgatgaccagcttttcgcaaccgacagtcatgccgttcagatcaagcgtgaagcctgtttcatccttcgccacactcagcacttcgctacgcaatctgaaggtcacattgcccttctcgcactcatccaccagcatgtcgacaatctgctgcgcggagtcatcgcagaagagttgccctaacgttttctcgtgccaggcgatgccgtgtttattgaccagatcaatgaaatcccactgggtaaaacgtgcgagtgcagacttacaaaaatgcggattctggctcagataagcgcctggttcgacataaaggttggtaaagttgcagcgcccaccgccagacataaggattttgcgccctggttttttaccattatcgatcagcagaacccggcgtcctgcctgacctgccagcgcagaacagaacatacccgccgcaccagcgcctataataatggcatcaaacctttccacgttgcgctcctcttagaaaaaacgggcgtgaattgtaaagattcctcagtggtcgcaccagcatcaatattactaaaaggaagtatttgcctgaattatataagataattattttttgagtgaaatccatacagggggcaaatcaaaaaaagtctatatttcactttgcccgcgccgcgaaagtcactgataatgcgccgcgttcatgtcctcaaaatggcgtaacgtcctatgctacatttgtttgctggcctggatttgcataccgggctgttattattgcttgcactggcttttgtgctgttctacgaagccatcaatggtttccatgacacagccaacgccgtggcaaccgttatctatacccgcgcgatgcgttctcagctcgccgtggttatggcggcggtattcaactttttgggtgttttgctgggtggtctgagtgttgcctatgccattgtgcatatgctgccgacggatctgctgcttaatatgggatcgtctcatggccttgccatggtgttctctatgttgctggcggcgattatctggaacctgggtacctggtactttggtttacctgcatccagctctcatacgctgattggcgcgatcatcgggattggtttaaccaatgcgttgatgaccgggacgtcagtggtggatgcactcaatatcccgaaagtattaagtattttcggttctctgatcgtttcccctattgtcggcctggtgtttgctggcggtctgattttcttgctgcgtcgctactggagcggcaccaagaaacgcgcccgtatccacctgaccccagcggagcgtgaaaagaaagacggcaagaaaaagccgccgttctggacgcgtattgcgctgatcctttccgctatcggcgtggcgttttcgcacggcgcgaacgatggtcagaaaggcattggtctggttatgttggtattgattggcgtcgcgccagcaggcttcgtggtgaacatgaatgccactggctacgaaatcacccgtacccgtgatgccatcaacaacgtcgaagcttactttgagcagcatcctgcgctgctcaaacaggctaccggtgctgatcagttagtaccggctccggaagctggcgcaacgcaacctgcggagttccactgccatccgtcgaataccattaacgcgctcaaccgcctgaaaggtatgttgaccaccgatgtggaaagctacgacaagctgtcgcttgatcaacgtagccagatgcgccgcattatgctgtgcgtttctgacactatcgacaaagtggtgaagatgcctggcgtgagtgctgacgatcagcgcctgttgaagaaactgaagtccgacatgcttagcaccatcgagtatgcaccggtgtggatcatcatggcggtcgcgctggcgttaggtatcggtacgatgattggctggcgccgtgtggcaacgactatcggtgagaaaatcggtaagaaaggcatgacctacgctcaggggatgtctgcccagatgacggcggcagtgtctatcggcctggcgagttataccgggatgccggtttccactactcacgtactctcctcttctgtcgcggggacgatggtggtagatggtggcggcttacagcgtaaaaccgtgaccagcattctgatggcctgggtgtttacccttccggctgcggtactgctttccggcgggctgtactggctctccttgcagttcctgtaatcgtacgcaccaaaacgagcgggtcagctggcccgcttcagattgtgacatagtgcgctttgttcatgccggatgcggcgtgaacgccttatccggcctacaaaaacatgcaaattcaatagattgcagagattatgtaggcctgataagcgtagcgcatcaggcaattttgcgtttgtaatcagtctcgagcgggtcagtttactggcccgctttttttatgcgttattattgctgaagtgcttaatgccaaatcatcaatgcaatcaggctgaccaccaccagaccacacaatgcgctggtcagaataaactgccgacgcacccgctcacagcggcgaataaattcatcatcgtgatgatcgcgataacgttgggcatagatataccaaacgagacgcacctgtttgttgggttggccatgtgaggtaaaaaagccccctccatcaacatattgatagagcaatggatcgcagttacgcagtaccactaacaacgcgcgtagtgatgagaaatagcgcgccatgttaacaatgcaaacgacacataaagcccaaaataatgcgacggtgcttatcatacctcctccccggcgacctgcccgcggagttccaccccggggctaccgctcccgatacgctgccaatcagttaacaccaggtcctggagaaaccgcttttgtggtgaccaacatacgagcggctctatagatagtgtaggagatcaggttgttttttttccagaaggttaaccactatcaatatattcatgtcgaaaatttgtttatctaacgagtaagcaaggcggattgacggatcatccgggtcgctataaggtaaggatggtcttaacactgaatctttacggctgggttagccccgcgcacgtagttcgcaggacgcgggtgacgtaacggcacaagaaacgctagctggccagtcatcgacaactttatggaaggagtaacactatggcttataaacacattctcatcgcggtcgacctctccccggaaagcaaagttctggtagagaaagcagtctctatggctcgcccctacaatgcgaaagtttctctgatccacgtagatgtaaactactctgacctatacaccgggcttattgatgtgaatctgggtgatatgcagaaacgcatctctgaagagacacatcatgcactgaccgagctttccactaatgcaggctacccaatcactgaaaccctgagcggcagcggcgacctgggccaggttctggtcgatgcaatcaagaaatacgatatggatttggtggtttgtggtcaccaccaggacttctggagcaaactgatgtcttccgcacgtcagctgatcaacaccgttcacgttgatatgctgattgttccgctgcgcgacgaagaagaataatcttccctctacgacgtgttcctgaacgcccgcatatgcgggcgttttgctttttggcgcgccttgttacctgatcagcgtaaacaccttatctggcctacggtctgcgtacgcaatcaaaatccccagccaatacaacatttaacaccatcatattttccatcattagtgtgatcatctggttattttctgttgtaatagtgtattaatctattcaccgcatcaatattaagaatctctgacagatgtaaactttttcgcgcgttatcccttacgcgttcatacttttcaggatggtattggaaggttaataaatatgaatacaacaacacccatggggatgctgcagcaacctcgcccatttttcatgatcttttttgtcgagttatgggagcgattcggctactacggcgtgcagggcgtactggcggttttcttcgttaaacagcttggattctcgcaagagcaggcttttgtcacttttggtgcttttgctgcgctggtctatggcctcatttccattggcggctatgtcggcgaccacctgctggggaccaaacgcaccattgttcttggagcacttgtgctggcgattggctacttcatgaccggcatgtcgctacttaagcctgacctgattttcatcgccctggggactatcgctgtcggtaacggcctgtttaaagctaacccagccagcttgctttcgaagtgctatccgccgaaagatccgcggcttgatggcgcattcaccctgttctatatgtcgatcaacatcggctcgttgatagcgttatcgctggcccctgtgatcgctgatagattcggttattcagtcacctacaacctgtgcggggcggggttaattatcgcattactggtttacatcgcctgtcgtggaatggtgaaagacattggttctgaacccgacttccggccaatgagcttcagcaaactgttgtacgtgttacttggcagcgtggtgatgatcttcgtatgcgcatggctgatgcacaacgtagaagtcgccaatctggtgctgattgttctctccatcgtcgtcaccatcatcttctttcgtcaggcattcaagctggataaaaccgggcgcaataaaatgtttgtcgcctttgtcctgatgctcgaagcggtggtgttttacattctctacgcccagatgccaacatcgctgaacttctttgccatcaacaacgtgcatcatgaaattctcggtttttccatcaacccggtcagcttccaggcgcttaacccgttctgggtggtactcgccagcccaatactggcaggcatttacacgcatctgggtaacaaaggcaaagacctctcgatgccgatgaaatttactctcggcatgtttatgtgctcactgggctttttgacggcggcagctgcgggaatgtggtttgcggatgcacaagggctgacatcgccatggtttatcgtgctggtgtacttattccagagcttaggtgaactgtttattagcgcccttggcctggcgatgattgctgccctggtgccgcagcatttgatgggctttattctcgggatgtggttcctgacgcaggctgccgcgttcttgctgggcggctatgtggcaacatttaccgcggtgccggacaacattaccgatccgcttgagacgttgcccgtctataccaacgtgtttggtaagattggtctggtcacgctgggcgttgcagtagtgatgctgttgatggtgccgtggctgaaacgcatgattgcgacgccggaaagccattaattattcttgcagaaagcagggtagcgttatcgctaccctgttttagttttacactggcgtacctgcatagatatcaaagcgatgccctttagtgactaccgcgtttggcgtggcgacattcgccagcggtggcgcgtagtccgggcgctttaccaccacgcgtttggtcgccagcaagcgtgcaggctccagtaatccatcggcatcaagatccggtcccaccagcgactgaaagacacgcatctcttttttcactagcgcgcttttctgcttatgcgggaacatcgggtcgagataaaccacctgcgggcgcggggtaatatcagtcagcgccgtcaggctggaggcgtgaattaactgcaaccgctcctgcaaccagccgccgatttccgcatccgcataaccacgcgccaggccgtcgtcgagtagcgcggcaaccactggattacgctccagcatccgcacgcggcagccgactgaagccagtacaaaggcatcgcgcccaagtcctgcagtggcatccaccacatccggcaaataatcgcctttaatgcccaccgctttcgccaccgcctcaccgcgaccaccgccgaatttgcgtcggtgcgccatcgctccgccaacaaaatcaacaaagatgccgccaagttttggctcatcacgcttgcgcaattccagatgttccggcgttaacaccagcgccatcaggttgtcttcatcgtgctccagcccccagcgggccgccagaacagataaggcaccgtctccggtgcctgtttcatcaattaagcagattttcactgaatgatcagcccttaatgccgtaatgctccagcatcgcatccagctgcggttcacgaccacggaagcgtttgaacagatccatcggctcttctgaaccgccacggctcagaatgttgtcgaggaacgactgcccggtttcacggttgaaaatgccctcttcctcaaagcgcgagaaagcatctgccgccagtacgtcagcccacaggtagctgtagtaacctgcggcataaccaccggcgaaaatatggctgaaagcgtgcgggaaacggccccaggacggagatggcaccacggcaaccagtttcttgatttctgccagagtttcgaggatttttgccccctgatccgggcggaactcggcatgaaggcggaaatcaaacaggccgaactccagctgacgcagaataaacagcgccgcctggtagttcttcgccgccagcattttatccagcaactctttcggcagcggttcgccggtttcatagtgaccagagataaacgccagcgcctccggctcccagcaccagttttccataaactgactcggcagttcgaccgcatcccacggcacaccgctgataccggaaacaccagcggtttcgatgcgggtcagcatatggtgcaggccgtgaccgaactcgtggaagagggtgatcacttcgtcgtgagtgaacagcgccggtttaccatttaccgggcggttgaagttacaagtcaaatacgcgaccggtttttgcaaagaaccatcagctttacgcatctggcctacgcagtcatccatccacgccccgccgcgcttgttttcacgggcatacagatcgaggtagaagctaccgcgcagttcgttattttcgtcatacagttcgaagaaacgtacatccggatgccagacatcaacatctttacgctctttagcggtgatgccgtaaatacgcttaaccacttcaaacaggccgttaaccgctttgttttccgggaagtacggacgcagctgttcgtcactgatgctgtagaggtgctgtttttgtttttcgctgtagtaagcgatatcccacggctgcaactcatcgacgccaaattcggctttggcaaaggcacgcaattgcgccagctctttttcgccttgtggacgcgcgcgttttgccagatcggttaagaaatccagcacctgctgcgggttttctgccattttagtggcaagggatttaaaggcgtagttttcaaagcccagcagttgcgccagttcgtgacgcagcgcgaggatctcttccatcaccttgctgttatcccatttaccggcgtttgggccttgatcggaggcgcgggtgctgtaagcgcgatacatctcttcacgcagagcctggttgtcgcagtaggtcattaccggcaagtagcttgggatatccagcgtcagcaaataaccttccagctctttcgcttcggcctgggcttttgccgcagccagcgcgctttctggcatccccgccagctccgcttcgtcggtaacgagtttggtccagcccattgtcgcatcgaggacgttgttgctgtactggttgcccagttcagaaagacgggtcgcaatttcgccgtaacgctgctgtttctctttcggcagacctatgccagagagttcaaagtcgcgcagtgcgttatcaaccgctttcttctgcgccgtgttcagcgtggcgtaatgatcgccatcgcgcaggtcgcgatacgctttatacagcccttcatgttgccctacccaggtgctgtattccgacagcagcggcagggtttgttcgtaggcttcacgcagttccgggctatttttcaccgagttcaggtggctgaccggggagaagatacgccccaacacatcgtccacttccgccagcggctggcagagattttcccaggtgtacggtgccccttgcgctactacgcgctccacgttttcgcggcagtcgttcaatgccttagtcacggctggaacgacatgttccgggagaattttagaaaacggaggcaattcaaagggagtcagtaacggattcgtcattcgcgcagtcctggttaaagaggttaaggaagcgctcaacaggcgctttacataatgtgtgtagcatggggttaagtgtagtgaatttcaatgagaaacgttacgctttcgcggcggcggcctcttttcggtatactgtcctgatacgcttttgtgcgccccgaatacgggccgatttttacttaccggaacacctttacccatgctcagttatcgccacagctttcacgctggcaaccacgccgacgtccttaaacataccgttcagagcctgatcatcgagtcgctgaaagagaaagataaaccgtttctctatctcgacacccacgcaggggccgggcgttatcagttaggcagcgaacatgccgagcgtaccggcgaatatctcgaaggcatcgcccgtatctggcagcaggacgatttgcccgcagaactggaggcgtacatcaatgtggtaaaacacttcaaccgtagcggtcagttgcgttactaccccggttcgccgttgattgctcgcctgctactgcgtgaacaggacagcctgcaactgaccgaactgcacccgagcgattacccgttgttgcgttctgaatttcagaaagatagccgtgcgcgtgtcgaaaaagccgacggtttccagcagcttaaggccaaactgccgccggtttcccgccgtggtttaatccttatcgacccgccgtatgaaatgaaaactgactatcaagcggtggtcagcgggatagcagaaggttacaaacgtttcgccactggtatttacgcactgtggtatccggtggtgctgcgtcagcaaattaagcgcatgatccacgatctggaagcgaccggtattcgcaaaattctgcaaattgaactggcggtactgccagacagcgatcgccgtggcatgaccgcttccggcatgattgtgattaacccgccgtggaaactggaacaacagatgaataacgtgctgccgtggctgcacagcaaactggttccggcaggcaccgggcacgccaccgtaagctggatcgtgccggagtaattgcagccattgctggcacctattacgtctcgcgctacaatcgcggtaatcaacgataaggacactttgtcatgactaaacactatgattacatcgccatcggcggcggcagcggcggtatcgcctccatcaaccgcgcggctatgtacggccagaaatgtgcgctgattgaagccaaagagctgggcggcacctgcgtaaatgttggctgtgtgccgaaaaaagtgatgtggcacgcggcgcaaatccgtgaagcgatccatatgtacggcccggattatggttttgataccactatcaataaattcaactgggaaacgttgatcgccagccgtaccgcctatatcgaccgtattcatacttcctatgaaaacgtgctcggtaaaaataacgttgatgtaatcaaaggctttgcccgcttcgttgatgccaaaacgctggaggtaaacggcgaaaccatcacggccgatcatattctgatcgccacaggcggtcgtccgagccacccggatattccgggcgtggaatacggtattgattctgatggcttcttcgcccttcctgctttgccagagcgcgtggcggttgttggcgcgggttacatcgccgttgagctggcgggcgtgattaacggcctcggcgcgaaaacgcatctgtttgtgcgtaaacatgcgccgctgcgcagcttcgacccgatgatttccgaaacgctggtcgaagtgatgaacgccgaaggcccgcagctgcacaccaacgccatcccgaaagcggtagtgaaaaataccgatggtagcctgacgctggagctggaagatggtcgcagtgaaacggtggattgcctgatttgggcgattggtcgcgagcctgccaatgacaacatcaacctggaagccgctggcgttaaaactaacgaaaaaggctatatcgtcgtcgataaatatcaaaacaccaatattgaaggtatttacgcggtgggcgataacacgggtgcagtggagctgacaccggtggcagttgcagcgggtcgccgtctctctgaacgcctgtttaataacaagccggatgagcatctggattacagcaacattccgaccgtggtcttcagccatccgccgattggtactgttggtttaacggaaccgcaggcgcgcgagcagtatggcgacgatcaggtgaaagtgtataaatcctctttcaccgcgatgtataccgccgtcaccactcaccgccagccgtgccgcatgaagctggtgtgcgttggatcggaagagaagattgtcggtattcacggcattggctttggtatggacgaaatgttgcagggcttcgcggtggcgctgaagatgggggcaaccaaaaaagacttcgacaataccgtcgccattcacccaacggcggcagaagagttcgtgacaatgcgttaaatgttaaagggctaagagtagtgtgctcttagcccttaattacgtttccgctatcagttcagaagctgaagcagaaagcggatcagttccagcagcgcaattaacgcccctagaacgatgattgctttatcaatcacccgttttctccatgcgatggagtgagaatgcatccgcttactcatccactgcctgtcacggcgcatgtctcattgttagataagaactctctcactccggccagagcatcagttaacggcaccacccgtacttctgaccaggactttgaaagcgtttatgcgcattgccagagtgaaaatgcctcagagctaactggataatcatacagtacatgcaggttataaaaccagcacgtccttgcaatagtttcagtatggtattagcattgatgcgttagatgatggctatctcactccagtcagagccaccaactcagggctggaaagtaaaaaaccgacgcaaagtcggtttttttacatccggattcggacaaggcttaatatgacgatgacccagtgaaagtatataaatcgtcactgcgatatataccgaagtgctccctccgccagctgaagaaatcgctaattcttgcaatgttagccactggctaatagtattgagctgttagataagaactctctcactccagccagagccaccaactcagggctggaaagtaaaaaaccgacgcaaagtcggtttttttacgtcctgattcagacctcctttcaaatgaatagccaactcaaaattcacacctattaccttcctctgcacttacacattcgttaagtcatatatgtttttgacttatccgcttcgaagagagacactacctgcaacaatcaggagcgcaatatgtcatttctgttacccatccaattgttcaaaattcttgctgatgaaacccgtctgggcatcgttttactgctcagcgaactgggagagttatgcgtctgcgatctctgcactgctctcgaccagtcgcagcccaagatctcccgccacctggcattgctgcgtgaaagcgggctattgctggaccgcaagcaaggtaagtgggttcattaccgcttatcaccgcatattccagcatgggcggcgaaaattattgatgaggcctggcgatgtgaacaggaaaaggttcaggcgattgtccgcaacctggctcgacaaaactgttccggggacagtaagaacatttgcagttaaaaatttagctaaacacatatgaattttcagatgtgttttatccgggaggcattatgttactggcaggcgctatctttgtcctgaccatcgtattggttatctggcagccgaaaggtttaggcatcggctggagtgcaacgctcggcgcagtactggcgttagttacgggcgtggtccatccgggtgatattccggtggtgtggaatatcgtctggaacgcgacggctgcgtttatcgccgtcattatcatcagcctgctgctggatgagtccggcttttttgaatgggcggcgctgcacgtctcacgctggggtaatggtcgtggtcgcttgctgtttacctggattgtcctgctcggtgctgccgttgccgccctgtttgccaatgatggcgcggcgcttattttgacaccgattgtcatcgccatgctgctggctttagggttcagtaaaggcactacgctggcgttcgtgatggcggccggattcattgccgataccgccagcctgccgcttattgtctccaacctggtgaatatcgtttccgctgatttctttggcctcggctttcgcgaatacgcctcggtgatggtgccggtggatatcgccgcgattgttgccacgctggtgatgttacatctctattttcgcaaagatattccgcagaactacgatatggcgctgctgaaatctcccgcagaagcgatcaaagatcctgctacgttcaaaactggctgggttgttttactgcttctgctggtgggatttttcgtcctggaaccgctcggcattccggtgagcgccattgcagctgtgggcgcgctgatattatttgtcgtcgctaaacgcggtcatgcgattaatacgggtaaagtcctgcgcggtgccccctggcagattgtcatcttctcgctcggcatgtatctggtggtttatggcctgcgcaatgccggattaacggaatatctttctggcgtactcaacgtgctggcggataacggcctgtgggccgcgacgctcggcaccggattcctcaccgccttcctctcttctattatgaacaatatgccgacggtactggttggcgcgttgtccattgatggcagcacggcatctggcgttatcaaagaagcgatggtttatgccaatgtgattggctgcgatttgggaccgaaaattaccccaattggtagcctggctacgctactctggctgcacgtactttcgcagaagaatatgactatcagctggggatattacttccgtacagggattatcatgaccctgcctgtgctgtttgtgacgctggctgcgctggcgctacgtctctctttcactttgtaatgagatactgatatgagcaacattaccatttatcacaacccggcctgcggcacgtcgcgtaatacgctggagatgatccgcaacagcggcacagaaccgactattatccattatctggaaactccgccaacgcgcgatgaactggtcaaactcattgccgatatggggatttccgtacgcgcgctgctgcgtaaaaacgtcgaaccgtatgaggagctgggccttgcggaagataaatttactgacgatcggttaatcgactttatgcttcagcacccgattctgattaatcgcccgattgtggtgacgccgctgggaactcgcctgtgccgcccttcagaagtggtgctggaaattctgccagatgcgcaaaaaggcgcattctccaaggaagatggcgagaaagtggttgatgaagcgggtaagcgcctgaaataaagcggcgatatcccccccacaggttgttagaaaagtgcgctttatttatgtcggatgcgacgctggcgcgtcttatccgacctacaaagttatgaaaattcgatgaatagtatgttatttgtaggcctgacaggcgtagcgcatcaggcgattttgctatttacacagtactccctgcgtgagattccaattatcgcgtccagcatggtgtatcagtgagctgcttagttatcagcgatacagcgcagtagtttaaagacgtactggattatgatttatcagtggtttacacaacaaattattaaataattataagataccttaacccattttattattacacatctaaaacatcacaaaaaaaatcacttcacacactatcagagaacataataactttttaaaatgagcgcattttgatagttgttaacgatttcctttacgatactatcactaccctttttttacacacaaatattaccgggtggagataaaagggaaatcaaaggtaattatatcaggaagatataacgcattacatttattgtgtgtagaagaaaatccattcctgttctaattatccaatttaaacatcttagcataaaacaaatgatgaataaggaattttatgtcaattgactttaccccaggtataataaatacatatcacggcgatatttataactgcacaacaaataccgataatgctaaaacgccagacacaccgaagtggccttgcgataattgggaagaacaacaacccattaattccacattctctggagaaggatatatctctgatcaatatgatttagcgcaacaccaacttcaacaaattaatgcgtgccacacgaacactacatatacaaatgcagactactcaaaagttgtggctcaacttgtaagtcttattactaacattgaaacgataagttcgacacaacttacgcaacagacacaatcaatacttaatcagattaataacattagatatgaaaaaaacaaaagtgctgaatgtcgaatcattgttatcgctaatcctaaacccgacaaggcaatcataactaaaattagcgtagaagagggaatacccataacattcagtgtccaaaccatgttttcagatactaattttattgctgaacaacgagctgacttaccaactaatataaaagatattcaaagcctgtatcaaaaaatgacgaagttatatattgagcacagtgaaaataaaaacaggatgaaagtctttgccggaaccaactttattgatttcaatatgacaggacagaacctgtccgggttcgttctaaccttgtcaaggttttatttcgaagatctacttaatataaatttcactgacgcaaatttagggaaggtgcgaataagcggggaaattcttctcggctgactcagtcatttcatttcttcatgtttgagccgattttttctcccgtaaatgccttgaatcagcctatttagaccgtttcttcgccatttaaggcgttatccccagtttttagtgagatctctcccactgacgtatcatttggtccgcccgaaacaggttggccagcgtgaataacatcgccagttggttatcgtttttcagcaaccccttgtatctggctttcacgaagccgaactgtcgcttgatgatgcgaaatgggtgctccaccctggcccggatgctggctttcatgtattcgatgttgatggccgttttgttcttgcgtggatgctgtttcaaggttcttaccttgccggggcgctcggcgatcagccagtccacatccacctcggccagctcctcgcgctgtggcgccccttggtagccggcatcggctgagacaaattgctcctctccatgcagcagattacccagctgattgaggtcatgctcgttggccgcggtggtgaccaggctgtgggtcaggccactcttggcatcgacaccaatgtgggccttcatgccaaagtgccactgattgcctttcttggtctgatgcatctccggatcgcgttgctgctctttgttcttggtcgagctgggtgcctcaatgatggtggcatcgaccaaggtgccttgagtcatcatgacgcctgcttcggccagccagcgattgatggtcttgaacaattggcgggccagttgatgctgctccagcaggtggcggaaattcatgatggtggtgcggtccggcaaggcgctatccagggataaccgggcaaacagacgcatggaggcgatttcgtacagagcatcttccatcgcgccatcgctcaggttgtaccaatgctgcatgcagtgaatgcgtagcatggtttccagcggataaggtcgccggccattaccagccttggggtaaaacggctcgatgacttccaccatgttttgccatggcagaatctgctccatgcgggacaagaaaatctcttttctggtctgacggcgcttactgctgaattcactgtcggcgaaggtaagttgatgactcatgatgaaccctgttctatggctccagatgacaaacatgatctcatatcagggacttgttcgcaccttccttaggtgacactatttttttacataaagaacaccctacccccaaattatataaagatggacaatatcttgacaaacaaatcgaaggtttattttcaacattattaaccattaatgacaaccttttacgagcaaaagcggaaattgcttcgacaataattaaatttttagaggccaggataaccaatctttcatacaatgacatattaaaatatcagcaagaattccaaagacaatgttataagcaagttaaagcctttacgacactctcccgatacaataaaattcaaacatgggcagaaatgtctgaatatcaattcgaagtatttcaatacgagacgcttaacccaaaaaaaatgtcacacacgccttatttaaagaggccactgcctaatgaaaaagatataaattatggggtggaaatagaaataccatctggtaaaagaattcgcttatcaaatcattaccagaatataataccataatattgattattagcactttataatcattgaataaaaatagattttatgtacttttaaaacaatgcactatattatggggtgatggatattcatgtcacgccccaaaattaactgagttcacctaaacagaaaggatataaacatcagacaggtttacgttactatcaggcatatcacctcagaatcagatgaaaactataaagaaatatctattatggttttaatatttgttgataaggatagtaacatgaacatgacaaaaggtgcactcatcctcagcctttcatttttgcttgccgcatgtagttcaattccgcaaaatatcaaaggcaataaccaacctgatattcaaaaaagttttgttgctgttcataaccagccggggttatatgttggtcaacaagcgcgctttggtgggaaggttatcaacgttatcaatggcaaaacggatacgttgttagaaatctctgtattaccgttggatagctatgcgaagcctgatattgaagccaactatcagggccgactgctcgccagacaaagcggcttccttgatccagtgaactatcgtaatcactttgttaccatcctcggcaccattcagggtgaacaacctggctttatcaataaagtcccgtataacttcctggaagtgaatatgcagggcatccaggtgtggcatttgagagaagtggttaataccacctataacctgtgggattacggctatggtgcattctggccggaaccgggctggggtgcgccttactacaccaatgcggtgagtcaggtaacacctgagctggtcaaataacaccaccgaaagatgcagatgctttctcagcatctgcatcatgcattacatcaaattaatacacagtaagctaactattattattataagccctgtcctgttaattacctttggcaaactgattataaagttaatgtccgcaccaggagtcggttatgtttcttataattaccagggatacgatgttcttcaccgcgatgaaaaacattctgagtaaaggtaatgtcgttcatatacagaacgaagaagagatcgacgtaatgttgcatcagaatgccttcgtcattattgatacattaatgaataatgtatttcattctaattttctcactcaaattgaacgattaaaacctgtccatgtcattattttctccccctttaatattaaacgctgcctggggaaagtgccggtgacctttgttccgcggactatcactatcattgattttgtcgcactcatcaatggcagttactgctctgtgcctgaagcggctgtgtcactttcgcgcaagcaacatcaggttctgagctgcattgcgaatcaaatgacaacggaagatattctggagaaactgaaaatatcgctaaaaacgttctactgccataaacacaatatcatgatgatcctcaatcttaagcggatcaatgagctggtacgccatcagcatattgattatctggtgtgaatttcaggcttacggtgagtctggctacgctgccacacagattagctaattgaaacgcctttcacccctgccataccttttaataatcgcaacaggtcttctatcgacgttgtggcatgaagctggatatcaatggcgaccacttcatgatcttcattttcctgcaacgaaactaaatcagtttttattttttgctgcttaaaccagtcgagcattgataccgtattaccgttcactaatgtcagctgtaaatggtaatttttgttcatcaggcggaaggttaattgatggaagacttccagcaccaacaaggtcatcactgaaccataaatacccagttcgtacataccgctgccaataaccatacctatggcggcggtcacccagatatccgctgccgtcgtcagacctacaatattttggttacgaacgagaatgttacctgcaccgataaacccgacgcccgtcaccacctgagcagcaatacggctggggtcgagtccgacgtgatctaaagacagcacgtcagcaaaaccatatttcgaaacaatcataaacagggcgcttcccatgccaattaatacatgtgtgcgtaaccctgctcctttgccgcgcatttgcctttccatgccaatagcgccacaggcaattgccgcgagtataagacgtataataaattctgctgtcatataaaaatgcaaaaaggagcagcaagatggctcaacttgctactcctttttacttgcacctcattaattcggcaagtcattagatgcttgatttttgaaggtatacaaatttttctgcgggtttttcttacagtattcgatcactttaggaatttgagtgagatcggtttcatttaaagtaacggtatcgccacctttatatactgtttcttcatgcagcatccaccatgcaaccggggtcattgcttttggattcagatcaataaattcctggcaggtcatatctttagcggattcattggctgccaacgcagattgtgcgttcaccagtgacaaagccgctacagcgcccataaaaataaacgctttacggagagatgaaatattcattttgtaacccattcaatatagagattatatatgaacaggaggaatagctgcttttaaagaagatattccggcctgttcaatatgcaaggaagtacgatgtaacgcattcccggaattacatatctttcttaattttgtcccattcgcctttaactttatctttaaagttggcttgtttatcctgagtacaagcctgaacgatagctggggttacggttgcaataccctgaacatctaaaaccgcatcttctggtttatctttgttgttcagcgcttcagcaaaaccaactgcagttggctggaaggattcgtccacagccaggaaatcttcacaggtccaggagttgaccggttttttgttatcagctgctttttgcgcatccgctgcattgctcacaactggcagaagaagcagaccaccaagaataacgcctaatacttttttcatcgtaatatcctcaactataaagtgaaagagccgtcacgaatcaatttcgacactgaggttataacctggttttctgtatatgtcatgttgatggaaaatatcaaaatcagatatttttatttcaatacaatgagttacagatgcatcagatactgcaattaggaaatttttattaaatcgactgcattcttagacgcgtttttggcatagattgatagcaggggattttcttcttaattttatagggtggttctatgttatatatagataaggcaacaattttgaagtttgatctggagatgcttaaaaaacatcgcagagcaatccagtttattgccgtgctgctgtttatcgtcgggttgctgtgtatcagtttcccgttcgtctctggcgatattttaagcacagtagtgggtgcattattaatctgctcgggtattgcgcttattgtcgggttattcagcaaccgcagtcataatttctggccggtattatccggtttcctcgtcgcagtcgcctatttattgatcggctatttcttcatccgcgcaccggagctgggcatttttgccattgcggcatttattgccggtttgttctgtgttgcaggggttattcgcctgatgagttggtatcgtcagcgttcaatgaaaggcagctggctacagctcgttattggtgtgctggatatcgtcattgcctggatattccttggtgcaacgccgatggtgtctgtaacgctggtttccacactggtgggaattgaactgatatttagcgccgccagcctgttcagcttcgccagtttgttcgttaagcagcaataattaccccggttgtcacccggatcatagtcacttgatgtgactatgatccgattaatactctctccgctacgcagtgttgtagatcaattgcgcactatcattgaaataattacctgctagtgattatttcaacctactgaatttcatctaatttttttcactctatggcaaattagccatttcaaacattatcatggctgatattttccgtagtcaggtttaatgttttaaaagtgctgtgggaaagtgaacaaagagttccgtaagcgttgatgctatgggcggttaaataagtaatccgggttcatttttttgcaactggcgttgattacattgcataaatatccgtgtctccagacgctatataaaaacctgaagacatgaatgcgttatttactcaggtaatttcaatgcgttaaaagaaagctggcaatccaattgccagcttaagtcgaaacaaggagactcgatatttaaatcggattacattttaactttagtaatattcttcagagatcacaaactggttattgataacttattcttgggcagtaatccgcaaacgttaactttttgtttgctatttacaagctgataacaaccaggaatcttacttaggatcaatatatggagtgcgtgatggataaatctgaagtattgattagtgttaatagacgtattagttcacgaagggtaaagttcttataggcgtttactatattgaacaacgattcggacaaggatgtaaataatgaaaaggatgacatattcgaaacgataacggctaaggagcaagttatgatttttctcatgacgaaagattcttttcttttacagggcttttggcagttgaaagataatcacgaaatgataaaaatcaattccctgtcagagatcaaaaaagtaggcaataaacccttcaaggttatcattgatacctatcacaatcatatccttgatgaagaagcgattaaatttctggagaaattagatgccgagagaattattgttttggcaccttatcacatcagtaaactaaaagctaaagcgcctatttattttgttagccgcaaagaaagtatcaaaaatcttcttgagattacttatggtaaacacttgccccataagaattcacaattatgtttttcacataatcagttcaaaattatgcaactgattctgaaaaataaaaatgaaagcaatatcacgtcgacgctcaatatttcgcaacaaacattaaagattcagaaattcaacattatgtacaagctgaaactaagacgtatgagcgacatcgtcaccctgggtatcacatcttatttttagtcaggacataagcaactgaaattgatggctggcatgacgagggatgcagatgctgatttcattacccccggtgattactaaaggagaggctaaaacgactttattcccctggtatgtgtatccaccagtagaacccttcgttgcccgaatgctggcaggaactgttggcagaacggcaacattttttttgtcgttgacctcaccatgtcgatcactgtgcctgtatcccaccttactggctgacaaccccactatgccgctggtctgtaaatccctcatatctctcctcgcgcgcaatttaaagaaccgttatttctcaagaattttcagggactaaaatgaacagaagaagaaagctgttaataccgttgttattctgcggcgcgatgctcaccgcctgcgatgacaaatcggcggaaaacgccgccgccatgacgcctgaggtcggtgtcgtcacactctcccccggttcggtcaatgtgttgagcgaattgcccggtagaaccgttccttatgaagttgccgagatacgtccccaggtgggcggtattatcattaaacgcaactttatcgaaggcgataaagtgaaccagggcgattcgctgtatcagattgatcctgcacctttacaggccgagctaaactccgccaaaggctcgctggcgaaagcgctctctaccgccagcaatgcccgcatcacctttaaccgccaggcatcgttgctgaagaccaactacgttagccgtcaggattacgacaccgcgcgcacccagttgaatgaagcagaagccaatgtcaccgtcgccaaagcggctgttgaacaggcgacgatcaatctgcaatacgcgaatgtcacctcgccgattacgggcgtcagcgggaaatcgtcggtgaccgtcggcgcactcgttaccgctaatcaggcagattcgctggttaccgtacaacgtctggacccgatttatgtcgatctcacgcagtcggtgcaagatttcttacgcatgaaagaagaggtcgccagtgggcaaatcaaacaggttcagggcagtacgccagtacagctcaatctggaaaatggtaaacgctacagccagaccggcacgctgaaattctccgacccgacagtggatgaaaccacgggctccgtgacgttacgggcgattttccccaacccaaatggtgacttgctgcctggcatgtacgtcacggcattagtggatgaaggtagccgccagaatgtattactggtgccgcaggaaggcgtcacccacaacgcccagggtaaagcaacggcgctcattctggataaagacgatgtcgtgcagctacgcgaaattgaagccagcaaagccatcggcgaccagtgggtcgtcacctctggcttgcaggctggcgatcgggtgatcgtttccggtttgcaacgcattcgtccgggtatcaaagcacgagcaatttcctccagccaggaaaacgccagcaccgaatcgaaacaataacgttgcaggcttaaggggactttcatggctaactattttattgatcgcccggtttttgcctgggtacttgccattattatgatgcttgcaggtggtctggcgatcatgaacttaccggttgcgcagtatccgcagattgcgccaccgaccattaccgtcagcgctacctatccaggtgccgatgcgcaaacggtagaagactcggtcactcaggtgattgagcaaaatatgaatgggcttgatggcctgatgtacatgtcttcaaccagtgatgcggcgggcaatgcctctatcactctgaccttcgagactgggacatctcctgatatcgcacaggttcaagtgcaaaataaactgcaactcgctatgccttcattacctgaagcagtgcagcagcaggggattagcgtcgataagtcgagcagtaatatcctgatggtagcggcgtttatttctgataacggcagcctcaaccagtacgatatcgcggactatgtagcgtctaatatcaaagacccgctaagccgtaccgcgggcgttggtagcgtacaactctttggttccgagtatgccatgcgtatctggctggacccgcaaaaactcaataaatataacctggtaccttccgatgttatttcccagattaaggtgcaaaacaaccagatttccggtggtcaactgggtggcatgccacaggcggcagaccagcagctaaacgcctcgatcattgtgcagacgcgtctgcaaacgccggaagaatttggcaaaatcctgttgaaagttcagcaagatggttcgcaagtgctgctgcgtgatgtcgctcgcgtcgaacttggggcggaagattattccaccgtggcacgctataacggcaaacctgctgccgggatcgccatcaaactggctgccggagcaaacgccctggatacctcgcgggcagtcaaagaggaactgaaccgcttatcagcctatttcccggcaagtctgaagacggtttatccttacgacaccacgccgtttatcgaaatttctattcaggaagttttcaaaacactggttgaggctatcatcctagtcttcctggtcatgtatctgtttttgcagaatttccgtgccacaatcatcccgacgattgccgtaccggtggttattctcgggacgtttgcgatcttgtcggcggtcggtttcaccatcaacacgttgactatgttcgggatggtgctggcgatagggttactggtggatgacgccatcgtggtggtggagaacgtcgagcgtgtcattgcggaagataagctaccgccgaaggaagcgacgcataaatcgatggggcagatccaacgtgcgctggtcggtattgccgttgttctttccgcagtgtttatgccgatggcctttatgagcggtgcaaccggggagatctaccgccagttctccatcacgctgatctcctccatgctgctttcagtatttgtggcaatgagcctgacccctgccctgtgcgccaccattctgaaagccgcgccggaaggcggtcacaaacctaacgccctgttcgcacgcttcaacacgctgtttgaaaaatcaactcaacactataccgatagcacccgctcgctgttgcgttgtaccggtcgctacatggtggtctacctgctgatttgcgccgggatggcggtgctgttcctgcgcacgccgacctctttcttaccagaagaggatcagggggtatttatgaccaccgcgcagttaccttccggtgccaccatggttaacaccacgaaagtgctgcaacaggtgacggattattatctgactaaagagaaagataatgtccagtcggtgtttaccgttggcggctttggcttcagcggtcaggggcaaaacaacggcctggcgtttatcagtctcaagccgtggtctgaacgtgtcggtgaggaaaactcggttaccgcgatcattcagcgggcaatgattgcgttaagcagtatcaataaagccgtcgtcttcccgttcaacttacccgcggtggctgaactgggtaccgcgtcaggttttgatatggaactgctggacaacggtaacctggggcacgaaaaactaacccaggcgcgaaacgagctgttatcactggcagcgcaatcaccgaatcaggtcaccggggtacgcccgaacggcctggaagatacgccgatgttcaaagtgaacgtcaacgctgcgaaagctgaagcgatgggcgtggcgctgtctgatatcaaccagacaatttccaccgccttcggcagcagctacgtgaacgacttcctcaaccaggggcgggtgaaaaaagtgtatgtccaggcaggcacgccgttccgtatgttgccggataacatcaaccaatggtatgtacgcaacgcctctggcacgatggcaccgctttctgcctactcgtctaccgaatggacctatggttcaccgcgactggaacgctacaacggcatcccgtcaatggagattttaggtgaagcggcggccgggaaaagtaccggtgacgccatgaaatttatggcagacctggtcgctaaacttccggcaggcgtcggctactcatggaccggactatcgtatcaggaagcgttatcctcaaatcaggctcctgcgctgtatgcgatttcactggtcgtggtgttcctcgccctcgccgcactctatgagagctggtcaattccgttctcggtgatgttggttgttccgttaggcgtcgttggcgcattactggccaccgatctgcgcggcttaagtaatgacgtctacttccaggttggtttgctgaccaccatcgggctttccgccaaaaacgccatcctgattgtcgaatttgccgttgagatgatgcagaaagaagggaaaacgccgatagaggcaatcatcgaagcggcgcggatgcgtttacgcccaatcctgatgacctctctggcctttattctcggcgtgctgccgctggttatcagtcatggtgccggttctggcgcgcaaaacgcggtaggtaccggcgtgatgggcgggatgtttgccgcaacagtgctggcaatttacttcgttccggtctttttcgttgtagtggaacatctctttgcccgctttaaaaaagcgtaacgtgtaaatgagagtaaggttgaacatgaaggttcagccttactctttcctgctaaccattcaccactcaacaaccagctaaccgtcaggaataccaggcttagtacacagcactgaaagtagaaaccactccagccattcgtcatcaatttgaacaacacaatactgacccacattcccgtaatcgtatgaattgtcagcttaataatcccaaacatgccgagtcttttcctcctgaaaataccgataccgcctggcaaactgcgaaagagaactagccggtagcccggcagaaatcatcagggaagagtttcacatgaagcaggtgtgagatcctgaccaatattcaaatgcgaaatatgtcaggaaaaggtacctggcgaatgttgcgcaaactgatgtggcgttacaccataatattgtcgaaatgtgtttataaagtacgatgtactgctatagccacatttttccgcaatagtatgcagaggaatttgacgtaactcgagtaatcgtctggccatcgacatcctggaggcgagtaatattttactgaaacaggtattttcatcctgcaacttttttttgattagactctcgctggtatacattctttccgcgatatcgcgcagataccaacgtttggcgatatcaaagctaataaggcgttcaacttttcctgaaacagtgctgatgctattgaaaagtaaggggatcagttctttcttatgagaaaacatcgataaacaggaaaggtagagcatattgctcagtatcggtgaatttaccccggattcattgaagctatcaaaaatcgccgtcaccagcggcatggggggtgactggttaattaacaaacggtctttgctgtgtaaccctaaattgcgtggtagctgacgaatattttgtaagtaatggcaaactgtcagctcatcgatatccagtcgtcgcgtatccggtgaacaaaacgcaaaatcgtctgccaaatttttctccagcagcagaatactctcgttatgcagcgatattttttgctgttcatgataaatatcgaatgaacgacgaatgaggatcaccgagcagacatgagtcatgattatcccttatatttcatactgcgattatttcaatttcagtatactaatgaaatgatgccagactgtttcttagcgcaaaaactgccagatttggtaggaccaaaatttatccacaaagtagttttgcataacagttaattgataataagtaaatgcagcacgaatatattttcgcacagcgtatagcttatgtttataaaaaaatggctgatcttatttccagtaaaagttatatttaacttactgagagcacaaagtttcccgtgccaacagggagtgttataacggtttattagtctggagacggcagactatcctcttcccggtcccctatgccgggttttttttatgtctgagtaaaactctataatcttattccttccgcagaacggtcagtgccgtaaaaattcccttgcgcaacaatacttgccgccgagtcacggttcgacaatctctgcgccgatcgctcctgatactctgtgggcgtcatcccataataatttcgaaagacgtaaatgaaatacgacacgctgtgatatccacaggatactgcaactcgcttaattgaaaaaccatgtataacaataagttgcaaagcacgttgcattctacactcagtaagcaactgtgaatatgatgtctcttcttcgcgcaattttttctttaacagacttggactcatcaacagctcgctggcgattcgggctagtgtccactcatgggcgatattattattgataaccgtacaaactcgtgttcgcatgttcggttgtaaaacgttcagaagcagcggtataaagtgctcatcctcaagaaaaacagataacaacgcaaagattaatgctcttttacgtagcatttctgcatagcgaagattcttattctgcgatagttgcgcaacttcctgaaaaacaggaatatctctactacagtgatgaacgagtaatgaagaaacttttttatgtgcatgaagatttaatgcctcctccttgagcatcgggagaaataatgaaagcgtgtcccttgacacgaatacaaaattttcaacacacttatctactcgaatttggcttgcatccgcaaaaaccaggtcaccgccattaaaatagcgatattcaccattaaccatggtgagaatatatttatgtcttgcatacgcaattagacaattcccatgtagtgattgcatagttgacttaatattacataaacatattactgtttattaatgtagcacgccgccctcttaagtcaaattgattgataaataaatttaaacgaagcgggagaacaggatgataatgtgtgatgttctacgggcaggatgactggatttataatacaaaaacgtgtttaagaacacagggaaattaatagtaagcaaataatcccttttcgtgacattaaaggtaatcgctacatttaataaacattcatataacatatatcttatcaacacgatgaatagacagccaatatattattgcgattaataagcaaccgaatgcccagctgtttttttaaaggctgggcattcggtttttacaacgttatgttatcaggtgtgtttaaagctgttctgctgggcaataccctgcagtttcgggtgatcgctgagatatttcagggaggctttgtagtcttccagcaacagttcagcaaagtccatttcgaagccgcgacgacacataatgcgcatcaccacgatgtcggtggcttcaccgccgagagtgaaggccggaacctgccagccgcgcagacgcagacgttcagagaggtcgtacagggtgtatcccggatcttcaccatctttcagtttgaagcaaaccgccgggatgccttcgtccgggcgacccgtacagatgaactcatacggccccagtttggcgatttcatccgccagataagcggcaacctggtaagaggcgttctgtactttggtatagccttcacgaccgaggcgcaggaattcatagtactgtgcaattacctgacccgccgggcgggagaagttgatggcaaaagtaccaatttgaccacccaggtagtcaacgttgaacaccagttcctgcggcagcgcttcttcgtcacgccagataacccagccgcagcccagcggagccagaccgaatttatggcctgaagcactgatcgatttcacacgcggcaggcggaagtcccagacgatatccggggcgacgaacggtgccaggaagccaccgctggcagcgtcgatgtgcatgtcgatgtcgataccggtgtcggcctggaatttatccagcgcatcgtgcagcggttgtgggaactcatagttaccggtgtaggtcacgccgaaagtcggcaccacgccgatggtgttttcgtcacaggcttcaatcatgcgtttcgggtccataaacaactgaccggggcgcatagggatctcacgcagctccacatcccagtagcgggcgaatttatgccagcagatttgtaccggaccgcacaccaggtttggtttatccgttggtttgcctgcagcttccatacgcttgcgccaacgccatttcatcgccatcccgccgagcatacaggcctcggaagaaccaatggtgttggtgccaacggcctgaccatttttcggcgcaggcgcatgccacagatcggcaaccatatttacgcaacgcaggtcgatggctgcggattgcggatattcttctttgtcgatccagtttttattgatcgacaaatccatcaatttatggacgttttcgtcgtcccaggtctggcagaaagtggccaggttctgacgagcgttgccatcaagatataattcatcattgataatctgaaatgcgacatcatcgcgcatttcgtgcagcggaaatcgttttgactccgcgatagtagaaatggcctttgcgccaaaacgtgaatcgagtagttctgagcggaaatccgttaacagcttctggtccatttcgaactccttaaatttatttgaaggcaataaaaaagtaggatttatccgcaatggaagcaaggcattacaggcttaatttaaataacaaaatcctaagcagaaaaacgactttttataatataaacatttaacatgataatattaaaaacagactttattatcgtaataaaaatcgcccaaacattgctgttcgggcgatcaaattaattattgtttatcctgcatatacggcgtgtacaccccgttcagactgtgcaggaaagctacgatatcatccacatcctcctgcggcagctctttgcctacctgatagcgcagcatcagtttcaccgccccgtccagcgtcggcacgtcaccgcgatggaagtacggtgccgttaaagcaacgttacgtaaaccgggtactttctgacgcaatttatcacgctcttctttagtcacattcatacgaccaatatccgccgccgtaatttccccaaagttaaagtcttttttcagccccaacggttcaaaggaacgtccgccgagaataataccaccatgacaagttgcacatttattatctttaaataattgatagccttttttctgttgcgccgtcagcgcattttcatctccgcgcaaccatttatcaaatggggaatccggcgtaattaatgttttctcaaattcagcaatggcatcagtaatattttcgccactgaaaccttgcggatagacttcgaggaactgcgttttaagctgcggatctttttccagcttagcaataatttcgtcccaggatttcgacgccatttcaatcgggttcaacggcggtccaccagcctgatcctgcaatgttgccgcacgaccatcccagaactgctcaacgttaaatactgagttaaataccgtcggcgcgttaatcggcccaactgcgccaccaacaccaatcgatgtttttctgccatcgacgccccccgcattcaacgcatggcaatgagcgcatgaaatggtgctatcagccgataaacggggatcgtgatacagcgcaaaacccaacgccactttttgcgcatcggtaggcagtttttgcgggatgggctgcaccggttcattgcgatgttccggagcagtatcattgctggcgtaatattccgcgcgctgttttgcaatccaggccagtatttccgcccgctcttcatcactcaccttacccgcccagtgtagcgcggtataacgcgttggtggcatagtttcatactgcatcacccattcaatcttattcaaatcgctttgcgaaacgggtttatcagccagcagtgccgcacgcacggcctcaaggttaaaagatttatatccaagcttaatgtcgtaatccatcaactgtttcgcgccaggaatataataataggcgggtaattctgccgaaggcgtgtggcaatagtcgcatcctttttcgcggagaaagcctaaaaccttattattttcactgacagcagatgcctgaacatcggcctgtttactgcgtttattatcgtggtaccacacataaccagataaccctaaatagcaaatcgcgacgccagccaggccgatcgcggtaatacgtgagaccattttcattattcttccctcacggtggtgagttattgtgacccagaaaattttccagaatgctgcaaacgtctctgcgagacaaagccatcataaaaaacagggagatacgctttttgataggaatcaatcaattacatgaatataaactatcaataagatagcctgtgcctattacccagatcaggaatggcatatcatgattgcggcgagagcaggattgaatgttctgaaaatgaaaaacaacaccaaatcggtatttttataaattccattgatattagtgcgttatattttttgacaggttaataaacgtgatccaccgcacgctttgtcgcccaccaggcggagcgaatgactacccttaaagaaaagccgataattagcgacgaatttcggaggttggatccttatgctcaatcagaaaattcaaaaccctaatccagacgaactgatgatcgaagtcgatctctgctatgagctggacccgtatgaattaaaactggatgagatgatcgaggcagaaccggaacccgagatgattgaagggctgcctgcctctgatgcgctgacgcctgccgatcgctatctcgaactgttcgagcatgttcagtcggcgaaaattttccccgacagtaaaacctttcccgactgcgcacctaaaatggacccgctggatatcttaatccgctaccgtaaagtgcgccgtcatcgtgattttgacttgcgcaagtttgttgaaaaccacttctggctgccggaggtctactccagcgagtatgtatcggacccgcaaaattccctgaaagagcatatcgaccagctgtggccggtgctaacccgcgaaccacaggatcacattccgtggtcttctctgctggcgctgccgcagtcatatattgtcccgggcggccgttttagcgaaacctactattgggattcctatttcaccatgctggggctggcggaaagtggtcgggaagatttgctgaaatgcatggccgataacttcgcctggatgatcgaaaactacggtcacatccccaacggcaaccgcacctattatttgagccgctcgcaaccaccggtttttgcgctgatggtggagttgtttgaagaagatggtgtacgcggtgcgcgccgctatctcgaccaccttaaaatggaatatgccttctggatggacggtgcagaatcgttaatccctaatcaggcctatcgccatgttgtgcggatgccggacggatcgctgctcaaccgttactgggacgatcgcgacacgccgcgtgacgaatcctggcttgaggacgttgaaaccgcgaaacattctggtcgcccgcccaacgaggtgtaccgcgatttacgcgcgggggcggcctccggttgggattactcttcccgttggctgcgtgatactggtcgtctggcgagcattcgtaccacccagttcatccccatcgatctgaatgccttcctgtttaaactggagagcgccatcgccaacatctcggcgctgaaaggcgagaaagagacagaagcactgttccgccagaaagccagtgcccgtcgcgatgcggtaaaccgttacctctgggatgatgaaaacggcatctaccgcgattacgactggcgacgcgaacaactggcgctgttttccgctgccgccattgtgccactctatgtcggtatggcgaaccatgaacaggccgatcgtctggcaaacgccgtgcgcagtcggttactgacacctggcgggattctggcaagcgagtacgaaaccggtgaacagtgggataaacccaacggctgggcaccgttacaatggatggcgattcagggatttaaaatgtacggcgatgaccttctgggtgatgaaatcgcgcgaagctggctgaagacggtgaatcagttctatctggaacagcacaaactgatcgaaaaataccatattgccgatggtgttccccgcgaaggcggcggtggcgagtatccgttgcaggatgggtttggctggactaacggtgtggtacgccgtttaattggtttgtacggcgaaccataatatttttacagccagccgctaacttcctgctggctgtaaaattatcctcttcaggaggagatatttaacatcattgccgcctgggtgcgatttttcacttccagacggcgatacagggattccagatgcgcttttaccgttccggtactgatattcagcgctctgccgatctccttatttgattcgcccgccgctaacatggttaaaatctcccgctggcgggcgcttaacgatttgagatctttaatgtccttttccggcgtcgtccgccagtctccaggcagaaacatcatccccatcgccgcactatttaccgccaacgcaaatgtctcgacggttgaatcacgaggcacaatggccagcacattaaaatggataacttcctgtaaccaccgtttattgcaatccgtcgccgtaattaacaccttaacctcaggaaattgcaccacggttttttgcagcaaccagtagcaaaactcaccatcctgatcgccatcgagcataactaaggcttcagggtaactttccagcttttgccataactcgtctgcctgactggccccctgaatactcactcctggaatacgctgctgtaaactgattttcattccatgaataaatattgactgcctgtcaaacatgactatttgcataactgaatctccacctgaatacgttaaaaagacttaagtagtggaagggtattacccgcgagaaaaaataagaattcgccatttggcggtggccattctacagagatgacgtgtagaaaatagttaccgatataaatagttacagctaaacgcctgaaattacatgtcgagggcactatttaaaacaattttgaggatttccttatattggtggttagtacgcatgcaattaaaaatgaaattccgcgaccacaagccaaaataacaaacggcaaggagacaaaaataagcacaaatagccaacacgtcctctgttcactttaaagggaatcgctgaaaaatacgctctgtttaaggggattcacctttctcagaaagctattccgcccttttcctgctgagaaatcgccacattcggcatgacaacattgtgaaacccggcattagatgttagaaaaaacaataaacaatgcgatatgcgcgttactgtttcgctgtgaacaacaatcggtcaaagaaatggataaaattcacgcaatgcagttgttcatcaaagtcgcggagctggaaagtttttcccgcgcagcggatttctttgctttgccaaagggaagtgtttcgcgccagatacaggcactggaacatcaacttggcacccagcttctccagcgcaccacgcgacgggtcaaactcacgccagaaggcatgacctattatcaacgagcaaaagatgtgttgagtaatctcagcgaactggacggtctgtttcaacaggatgccaccagtatcagcggtaaattacgcatcgacatcccgccaggaatcgcgaaaagcctgttactgccgcgcctgtcggaatttctctatctgcatccgggaattgagctggaactgagtagccatgaccgtccggtagatattcttcatgatggttttgattgcgtgatacgcactggcgcgttaccggaagatggcgttatcgcccgtcccctcggcaaactgaccatggtcaactgtgccagtccgcactatctgacgcgctttggttatccgcaaagccccgatgatctgacttcacacgcaatagtgcgttatacaccgcacctgggtgtacatccgttaggttttgaggttgccagcgttaatggcgtccagtggtttaagtctggcggcatgttgacggtaaacagtagcgaaaactatctcaccgccggtcttgccggtctggggattattcagatcccgcgcattgccgtgcgcgaagccctgcgtgccgggcggcttattgaagtattacctggctaccgtgccgagccgctctccctttcgctggtttatccgcagcgtcgggagctttcccggcgtgtaaacctgtttatgcagtggctggctggcgtaatgaaagagtacctggactgaccgactatactttttaagaatgaccacgacagaaggacaaaagagcggatgacgcaggaaaacgagatcaaacgtcccatccaggatctggagcacgagccgattaagccgttggataatagcgagaaaggcagcaaagttagccaggcgctggaaaccgtcaccaccactgccgaaaaagtccaacgccaaccggttattgcgcacctgattcgcgcgacagaacgctttaacgatcggctgggtaaccagtttggtgcggctatcacctatttctcatttttgtcgatgataccaattttgatggtgtcgtttgccgcagggggctttgtgctggcctcccatccgatgttgctacaggatatcttcgacaaaattctgcaaaacatcagcgatccgacgctagccgccacgttgaaaaacaccatcaacaccgccgttcagcagcgtacgactgtagggcttgtcggcctggcggtggcactttattccggcatcaactggatgggtaacctgcgtgaagcgattcgtgcccagtcgcgcgatgtctgggaacgctcgccgcaagatcaggagaagttctgggtaaaatatctgcgagattttatttcgctgattggtttgttgattgcgctgattgtgacgctttcgatcacctcggttgccggttcggcgcagcaaatgattattagcgccctgcacctgaacagcattgagtggctgaaaccgacgtggcgattgattggcctggcgatttccatcttcgccaactatctgcttttcttctggatcttctggcggttgccgcgccaccgtccgcgcaaaaaagccctgattcgcggaacatttctggctgctattggttttgaagtgattaaaatcgtgatgacctacaccctgccatcgttgatgaaatccccctctggcgcagcatttggttccgtgctggggctgatggcatttttctacttcttcgcccgtttgacgctgttttgcgcggcgtggattgccaccgccgaatataaagacgacccgcgaatgccggggaaaacgcagccttaaaataggccggatgcggcgtaaacgccttatccggcatacgattttattcggcctggctccccgtaggccggataagatgcgccagcatcgcatccggctataatgcgcacataacctcttgaaactcgtccccagagcctcttcagccatctatttgggagcaaacaatttcattccaactcataaccccagcatataaatccagttggtaacttttatttaacctgaaaccagttttatccactatttataaaattatgtgaagcatttcatagaagaaaaatcactggcctaaacattatcccctttttgcctgatttttgaccatttccgcgatttgttacacattgaaatatcacttttgctgtgcgtaatatggctattcgttagccaaaaaataagaaaagattatgcaagcaacagccacaacactcgaccacgagcaagaatacacgccgatcaactcgcgtaataaagtccttgtcgcctctctcattggcacagccattgagttcttcgacttttacatttacgccactgcggccgttattgtgtttccgcatatcttcttcccgcagggcgatcctacggcagcaacgctacagtcgctcgccaccttcgccatcgccttcgtcgcgcgccccattggctctgccgtttttggtcattttggcgatcgcgttgggcgtaaagcgacgctggtcgcctcgttgctaacgatggggatttcgaccgtggtgattggtctgctgccgggctatgccacgattggtattttcgccccgctgctgctggcgctggctcgatttggtcagggtctgggcttaggcggtgaatggggcggcgcggcgctgctggcgactgaaaacgccccaccgcgcaaacgtgcactgtatggctcctttccgcagctgggcgcaccgattggcttcttctttgccaatggcactttcttgctgctttcctggctactgaccgacgagcagtttatgagctggggctggcgtgtgccatttatcttctcggcggtgctggtcattatcggcctgtatgttcgcgtgtcgctgcatgagtcgccggtgtttgagaaagtcgctaaagcgaaaaaacaggtgaagatcccgctgggtacgctgctgaccaaacatgttcgcgtaaccgtactgggtacgttcattatgctggcaacctatacgctgttttacatcatgacggtctactctatgacctttagtaccgccgccgcgccagttgggcttggcctgccgcgtaacgaagtgttgtggatgttgatgatggcagttattggttttggcgtgatggtgccagtcgctggattactggctgatgcctttggtcgccgtaaaagcatggtaatcatcaccacgctgatcatcctgttcgcgctgttcgcctttaacccactgctcggttctggcaacccgattctggtttttgccttcctgctgctggggttaagtctgatgggtctgaccttcgggccaatgggtgcgctgttaccagagctgtttccgacagaagtgcgttacaccggagcatcgttctcttacaacgtagcgtcgattctcggggcttccgttgcgccatatatcgcagcctggttgcagactaactacgggctaggtgcggtggggttatatctggcggcgatggctggcttgacgttaatcgccctgctgctgacccatgagacgcgacatcagtcgttgtaataagagtgaaaagcctgatgcgctacgcttatcaggcctgaatttccatacaatatattgaattcgcaaggatttgtaggccggataaggcgttcacgccgcatccggcatgaacaaagcacactttgccaacaatctaaatctgtttaattgccggatgtcagacatccggcaattatcatcacttcttcatctgcgacaaaatcgtccgacactgattagcctccccttcggaaggtgagatcagtgccagtaacgccgccgccggtgttaccagcgttgccagtgccgcagcaacagcaccacgggcaatcagcggtccggctttcaccccagcctgcggatttttaaacgtcccccgcacatacagcggcgaacgcagtgtgataatccgaattcctttactctccggatcaatagtcaaatccagctgttccgaagcaaaacttgccgtgccggtaacattaatcaacgcgttctcagtatcgaaagcaaaaatctgcgggcgcgccacgccgttggcaatattcagattcgccgccgcgcagttcacccgcacctcatcatcaccaaatatcgcaccgacaatgtagttgccgacattcagcccaacaatctccatcaggttgcggctcaccagcccgtcattcatcaacagtttcaggttgccgttactgttgcctaaaagtgccgccaccgagttaccgctaccgcgtagttccgcgtcaccgttcatttcccccagcgtcttctgcatcagttccacatcgggcatcagttctttcagtttcagtcgacgagcctgaatatctgcccgcccctgcatcggctttttatcgccttccagatgaatattcgccgcaatgctgccgcccgccatgccaaatttcagcggttgcaggcgcaggtcagcatttttgaggatgatatgagtagaaagatcgctaatcggcaggctactgccatgctcaatgcgccgccctttgaagcgaacatcggcatccataacgtcccatttatcggtttcgaagcggtcataaggcagcactttgcccgcaggctgaacgcttttttcgcccttcttctgttcagaccgtttcgacttttctgcccctttcccggaatcaacgccaatcaacggtcccaggtccgccagccgcaattgccgcgactcgacatcaccttccagttttggtcgtggctttccggtggtgtagaccagagaaccgtggatatcgctatcaccaattcgcccattaaaaccgcgataatcaaagaccgacgatttttcagtgtcgattttcgctaccagccgaccatccgtttcaaacggcggggtatcgggcagcagaacgcccgtcagttcatagagatcacccagtgaatcgccagaaaatttaagccgtaaatcgacaccgcccatcttcattgggtcattcacgacgccatcaaaagcaacacgggtgttaccagagcggaaatcagcctgtaccggaaacggcgtcccttcgccacgcagcgccagcataccgcctatttttcccgtacccgtgagcggttcaccgttatatcgtccctgcgccttcaggccaaaaacgtaatcgcccaccttttctttatccgctttacctttcgatccagtaacttcgctgaacggcagcggcttgcctaagggatcaacaaaaatctccagatccgctttgcttactttgtcatcaatggcgatccgcccttgatcgaaaagaatattatccagccgaaacgaccatgccgacggctttgcattcgcgtctttgttatcatcgttggcaagattaaacgtccagttattgttcttttcagagaggcgaatcaggcgcgcgtcgggcttttcgagcttgatccacggcagccagaccgttttggtcagcagcgccagcggggccagcgttgcctctacgcgtggcaaatgcaccatcgtgacttcgggaatatccggtggattgccaagaatgatgtcttccgcgtgtacatggggccacggcacccagctgcgccagccagtttcttgtttttgccgctcccacaccacgcccagatcgccacggatagcgaacggacgattcaactccgcagagactttctggttgatagtcggtttgagtcgattccagtcaaaagttgcaatcaaaatgatcgccacgacaatcaacaacaagaaagcccctgaaatcgcagcggttattttgcctgccttgctcatcgttcgcttcctcatattcttcctgtgccagtcctaaagatagtccagccaggcggaaaatgaggcagcttatagcgccagaaccgccgtattcagcgtttctatcggtgccgggcgtgaaagaaaccagccttgtgcggcgaatgcgggcgagttctgaacatcacgccactcttccggcgtttctacgccctcgacaatcaccccgcgacaatagcgattcattagatgtaaaagctgagaaaagagtgtgcgtccttccggcgactgacgcagcatcacaaacagttctcgcgcgattttgatgtagtcataacgcacttcacttagcgcagagaaatttgccatcccggtaccaaaatcatccagccacagcgggccaaattcacacatcgaggcaaaggttgaatctttcggcagacggatatgctccaccagttcgaaacgcagccagggaagacgctcaatctggcgcaggatttttggttgctgacgcagggcgatgagcgtagggccatcaatattgaccgatgccagcaggccgtgctctataaagaagtcggctttttgcgccagcaaatcaatctgctctttcacaacctccatccgatggctgacggtgatttcagtaaaatagcgatccggcggcaggcgttgcgaagggttcaagggatgcgtgaccaccgttaatagctccacggccattaaccgcccgcatgtttgatagatcggctgccaggtgtaagcacgctcacactgcaaccaaaaacgccgttcctgcaagctctcgatgcttgcttcagggttgcttattcgctggataacctgccttatcatcaaagatgtcctgtgtttaaaagtgatgctgcccggactcgacaaagattatcggcgcgtaagggcagaactttaccgcctggccggggtaaatttcctcactccacaacggaatctttcaggaatacgttctggctcaaaaaaataatggaacactgttttaatatggttgaccagcaaaccaccacagcgcaaactaacgctaattttttacagatcaggttcacgactatgtccaaaaagattgccgtgattggcgaatgcatgattgagctttccgagaaaggcgcggacgttaagcgcggtttcggcggcgataccctgaacacttccgtctatatcgcccgtcaggtcgatcctgcggcattaaccgttcattacgtaacggcgctgggaacggacagttttagccagcagatgctggacgcctggcacggcgagaacgttgatacttccctgacccaacggatggaaaaccgtctgccgggcctttactacattgaaaccgacagcaccggcgagcgtacgttctactactggcggaacgaagccgccgccaaattctggctggagagtgagcagtctgcggcgatttgcgaagagctggcgaatttcgattatctctacctgagcgggattagcctggcgatcttaagcccgaccagccgcgaaaagctgctttccctgctgcgcgaatgccgcgccaacggcggaaaagtgattttcgacaataactatcgtccgcgcctgtgggccagcaaagaagagacacagcaggtgtaccaacaaatgctggaatgcacggatatcgccttcctgacgctggacgacgaagacgcgctgtggggtcaacagccggtggaagacgtcattgcgcgcacccataacgcgggcgtgaaagaagtggtggtgaaacgcggggcggattcttgcctggtgtccattgctggcgaagggttagtggatgttccggcggtgaaactgccgaaagaaaaagtgatcgataccaccgcagctggcgactctttcagtgccggttatctggcggtacgtctgacaggcggcagcgcggaagacgcggcgaaacgtgggcacctgaccgcaagtaccgttattcagtatcgcggcgcgattatcccgcgtgaggcgatgccagcgtaaacgcagcatatgcaaaaggctggataaagtgttacccctctatccagctcatccataaatacctgatggttgtgctaactcatcaccatcaggcattactgtgcaggtggaatatccgtcacttcaggatgtacgtcatccgtggcgacagaggtggtcgcagcggcggtagatggggccatgatttgatcccagaccgcctgcaacgctttcatgttaaattccggctcgcctttcggctgcagcagtattaacgccatatcattcgacaactgttgacgcagatcctgatttaacatctctaccgtcaggctattaaggaaatcctgccgcagtttctgatattgctccggcgcgatatcgacaacctgattttgcaacgaacgcatccgctgacccatcagaatatcggtatcagctcgtgcataggcggcaaacagtttctgcagctccagtttcttttgcgccactaacgcattgaactcttcttccggcagacctttatcgcgaaccttcgccagttcacgcgccaccagattaaggttgctgttcagcttgtcgtttggtgattcgatgttgatggcacactgcgcacgcagatacagcacacggcagtcaaatccaagaccgatgtctttgctgttactggcacttaacgcttgctgaacatgccagaacagcgcctcgcgggccaggtccgcacgccagtagcgcagcagtgcggctgattcacgaatcggctgccacggcgtatcccacatgatagataaccggtcctgacgcaccgcgtcagtcataatactcaccgcttccgcacgcagcggagaaagcgtcggcaccggagctggcgtttcacgtttgcctttcagttcgccaaacgttttgtttatttggtcgacaaccgagcgcgcatccacgtttcccaccaccagtagcgtcattgcatccggggtgtaccatttctgatagaaatctttaattttttccgcttcaacgggttgtttcagcggatcggcaggatcgtgacctaacaaggttgaccctttcagacgatagcgccaccagccctctttagtatcggcaggccaggttgccaccatgtcctgactttgcagcgcgtggttgatggtttctggtgtgatggtcaatttgccagtggcatttgccagataagagagcgcttctttcagcaaatcgttacggttattgggcaaactcagattaaacagcgtggtgtcataagagacaattaccggcggcatcgggcgtttagggtcgatcccctgctgccacaatgaacgcgcctgtgctgcgtcaaggccaccgctttgcgttagcgcaatacgagggatggcgtgactgtaaccgctctgttgtgtactttcggcgagcgaaccggtattaaccagcaggcgaatttcaacacgatcgctgggacgctggggggtggtcagcacttgccactgtaaaccgttggaaagcgtcccctgttgccatgctggatcaggctggagcgcatctgcctgcacatagccagcagtggccatcatcagcaaaccgcccgctaaaagtcgaatttttgtgccctgcatgtgaacccctgatcaactatcctggtaataaaaaaactgcccgttgtcggtcagtctaaatgacgttaaaaacacttcgtgttagaccgcaagaacatgaaaatgtcacggaagaagtgaaataaacctgaactcacccaggtggtaagttcaggcacaggggtcaattatgcgcaaacacccgcactcggggaagggagtgcgggcataagtgatgagattaagaggataattcgtgcgttttgccatccggcgcacgattattcagcacatcgtccagttttttgtggtccagttctttcacccacttagcaacgacaatggtcgctacgccgttaccgaccaggttagtcagcgcacgagcttctgacataaagcggtcgataccgaggatcagcgccagacccgctaccggcaaatggcccaccgcagagagcgtcgccgccagcacgataaagccactacccgttacccctgccgcccctttagaagaaagcagcaacacgattaacagcgtgatttggtggacgatatccatctgactgttagtggcctgggcgataaacaccgccgccattgtcaggtatatcgatgtgccatcaaggttaaacgagtagcctgtcgggatgaccagccccaccaccgatttacggcagccgagtttctccatcttgtcgagcatacgcggcagcgccgactcggaagatgaagtccccagtacaatcagcagttcttcacggatgtagcggataaatttgaagatactgaaaccagtcgctttagcgattgaacccaataccagcaccacaaacaggatacaggtaatgtagaaacagataatcagctgccccagttgcaccagtgtgccgacgccgtatttaccgatggtaaacgccattgccccgaacgcaccaataggtgccagacgcatgatcatattgatgatgccgaagatgacctgcgagaaactttcgatgacgttaaaaatcagttggcctttgctgcccagacggtggagcgcaaaaccaaacagtacggcaaacagcagcacctgcagaatgttaccgctggcaaatgcgccaatgacgctcgccgggatgacatccataatgaaggcgacaatgccctggtctttcgcctgatcggcgtaaaccgctaccgctttcgcatcaagcgttgccggatcgacgttcattccggcaccaggctgcacgacgttaacgatgataagaccaataatcagcgcgatggtactgacaatttcaaagtaaagcagtgcgactgcgccggtacgaccgaccgccttcatgctttccatgcccgcaatgcccgttacgacggtacaaaagatgacaggagcgatgatcatcttaatgagcttaacgaagccgtcgccaagcggtttcatttgctcgcctatttcaggatagaaatggccaaggagaataccaatggctatcgctgtcaggacctgaaagtaaaggcttttaaacagagaggttttcatagggtgtcctttagtaaaaccacaggtcttgtaaggttatggggtacctgcggccttaaaataacacccagacaacatcacagaaatgtacctggatcataattgaaacaaaaaggttaaaaagtttgagctggctcgcacaaaccagcactttttaaagttttgtaatcagtttggggtagctacttttcttccaggtaactctcttcgaagatttcaatagggagtgggcgagcaaaaaggaagccctgggcaataccaacgcccgcttttgccagccagtcgcgttgtgcttcagtctccacgccttcggcaatcatttgtaagttcaggctctgcgccagcatgataattgcagcaatcatgctgctatctcccggcaagccttcaacaaacattttgtcgattttcagtacgtcgattggcaacgatttcatatgctgcagctgacgcagccctgcgtagcccatgccgaaatcatccagcgccacccgaactccggcattgcgcagcggacggaggattgccaccgcagcatgagggtcgtcaatacgtcggctttctgtcacttccagaatcagtgttcccggctgaatgcgatagcgggttaacagttccagcatatccgccaccatattcgggtgcatcagttgcagcgcagagaggtttaccgacaagggcagcataatgccgcgctcttgccaggctgcaagcaatcgacaggactcttccagcacccagtgaccgacggtaaccatcagcccacagcactcaatgcgatcgattaagccatccggcaggtcccaactgccatccggttgctggatacgcagtaacacttccgcactgaccagtttaccgctggtcatctcgacctgtggctgtaaccaaatagcaaactgatgattttccagtgcattaaggatatcgctctcttccgtcaaccgcttctgggcggcttccatctgctgcggatcaaagaactgaatctgattcttgcctttatggcgagcggtaaatgccgcagaaatagcgcgactgtaaagctgttcggcggtgagatcgccgtagaacatcgccacgccaatgctacagtgcggacggagttgaatacgttcaatcggcaggcgctcgctcatgatagtgagcacttgctgacctaaggtgattgcgtgccacggttcctgtacaccgttggcaatgacagcaaagtcataaccgctaatctgcgcgaggatcatacgtggcgacagtaccgatttgagtttttccaccagcgtcagcagcagaatttctcgttgcgcctctttcagcacgcccgcagtatcacgcagggtttcacaggtgatgatcatcagcgcggtggtttgtttacgcgcgacaacctgctccagcatctccatcagcaaggctttgttcggcaaatccgacaccgggaagcgcatcgcattttcgttctgttcttcataatggcgctgcagcaattgctggttgaggttgtaactgcgcaccaacataccgatttcatcgtcctgatgcagacgcggtaatgccagttggtgaccaacaagctccttggctgggatggcgttaagttcgcgagcaatattgcgtaacggatgcaaaatcaggcggttaatgcaccagctgatggcgacggtcaggataagcgacaaaagtaagtaaatggtcactaacgttgagagggtgctcatcacgaacttatacatacggaaggaatccgcctgtagtaccagataggcaattggctgcgggtttgccggacgttcgagcgagtaaacgcccagcgagatttgaaccggtagctcaaacaggcgagtaaccattaccggcaccgggcgctctggaataaaacttttacgcagcgcctggaactggttaggcagcactacatcggcacggctgaccacgcctgccggtttaatgctggcaagaatagcttccgcttcgggaatatcgcctttcaaaatagctgaagataagggttcgcggacagagcgagcaatgctttccagttgcgtagccgtgttatagcgattctgctggaccagatggaacagcaaaacggtgcaaaaaataaaaacgaacaccaggacaacggctgccaccattgccatctgcttgattgttaacgagcgacttacgcgcaaattgtctccccccggaaatcccagattgccgcccgagtatacccgatcgcagcggcattaagagaggcgctatctgaaaacttaccagtcggcgtaaggtatcagcggctgcggcggtaaatccatgtcaccctgccatccggcggcggaataacgtacgtagagcaggaaatggctgggtgcgtaatctttcgcctgctggatatcaattgccgtgccaacaaaccagttggaagtaacacgtcgttcaagtaatgcccgcgccgtgtagccgaagccctgactgctgccgccatcgttggattgccgcgcagcttcttcctgccagtcggtcgggatcagattcatcagcggataacgcggcatggttttggtgcgtgaatgcgaccacgagccagacgcacccagctcccacgaccagttttccgtgcgctcccgccacatcaccggtatggcaaacgacaggtattcctgcggactgtagtaaccgccctgaccgagtgagtagccactcagatctttgtcgtaatgccagatcatgttgttcaggccgattgtgacgcggcgattgttctggttaatgaccttatagtaatagcccgtcatccagcgcacgcgccagttatcttcgacatttttaccggttaactggtcgccactaagcgatgcccagacgccgtttgcttcacctttatcgtagctcagacttagccccacaccgtcggcacgtacgccaccccattttttcccggtattgctcggggagtctttttgcccaccaaaggccagcaaagaactggagatgggccgacggtgggcgttaacggtgtaacccagcggcccgatatcatcgctgtaactgatgccgccgaccacatccaccacgttgaagcccatcggcgtggtaccgatatcccagctccagacgtcatttcgccagccgaccgccacgctggcaccggaatccgactggctgcggttgccgctacagtcctgtaatgtacaggtgccccagttgtcatcccatttgccatcggcattagtggagaaactgccgacgttcatattgacgaaatcactgcgaaagaacatccgcccgtcagaatacggcgcatccacctgcaacatggtagtgtgcgctttcagatcggagtaaccaccggtgccgctcgaaccccagtaatcgtgctcaagggtgacgttaagatcctgctggcgatagaggtccgccgcatcgctgcgcacgccacgtttcagccagtcatctttctcgtcgttacgggtcagtcgggtaaaggtgtcgttatcctgcggacgcgtcgtagtcacaccggatgcgaccatggcgtctttgtaggtttccagcgcctgcgttggatcgcccgcctgcgcttcaaacttcgcaccatcacgcagcaccatcgcgctttccatcgacggtggctgagattttgcctgcgggatcaacttattaaacgtccgctgcgctgctgcggtatcgccaagctgcgcctgtgccagcgccacgcgccgctgtgtgttcagcgaggcgttatcggtagcgggcagtttcgccagctggctacgtgccgccgctttgtcaccggcagcaatatccacttccgtcagaccaagaatggcgtcggcgttagctggctcccgcgtcaggacattctgatatgcagcgcgggcggcggtgtaatcacgtcgttgttgcgcccagtcagccagcgtgaggtcaatacgcgtggaaggtggttgctggcgcagcatcgcttccgcttctgcctctttgccgctttctcgcaggcggttagcggtttccagcacctgatcgctttgcagtcgattaaccagctcctgaatattgctgttccactgcgcacgcggcaggctattgatatgcgccagcgccgctctgtcctggtcatgaccagagaggtacagcccgtaagcgtaaacctgctccgggtcgttcgacttctgctgcgccagattgcgcattaacgtatcggcctggctgcgttgtccggcctgccagagatcctgcgaaagtcggtaagtaatccatacgctgccggggtccagcgccagtcgttgccgctgaagtgctgccgcctgcgcccatttgccctggttttccagtgcctctgcctgctgtgccagacggtcgttttgcaggctgcgttcgatatcatcaatgctacgccgctgactggcagagagcgaggcgataaacgcttcagctttttctggcgattgctggcggtaaatatttgccagcccgcgcacggcgttagtgttgccgctgtccatacgcaaggtctgctgataataacgttcggcggcgggataatcttttcgcgccatcgccacatcgcccagccccagcactgcataactgtcggtgttatcgacattacgcgcctgctggaacaggcgttctgcccggtcaggattattggctttcagcgcagcatcgccctgctggatcgccagccagtagcggtttactttcagcagactgttccatttgtcgttgttgctgctgtgcgggtccagtgcgagggctttttccagattcgccactgcattggcgcgatcgcctttctgagaatacgcctggcccagcgcccccagagcttcactgtctttcgggttcgcccgcaccgcctgttgtagttcgggaatggctttacccgccataccagagtccaccgccgctaaaccttgcgcacgagcgcggaaagcaggatcggccagctgtttttgctgttctgccagttgcgattgcgcagccgccacgctatcgccatcactaaagatcgagagatattttttcagcgccgacacactggcatcactgacgggcatgtctttaatctgcccgtaccagattttagaggccccttcgcgcccggcgttcgattttgccatctgttccaggacggcaaaaccttcgtcacggcgatcgctactaaacagcaatagcgccagattgttttgcaggcccgtattgcccggtgcatccgcattgatgcgttttaactgattaatcgcttcgccacggcgagccggaattttcgccaccgtactccagtactcgacagcaatgtcaccttccggcggcgcaccgttgaacagtttgttgtaactcgccacagcttcttctgcatgaccggtcgtcgcctgcaatcgtgcctgttgcagtgcctgacgaccatccggcgtggaaagtagcatcgtagtccgcgacgatttatacgcatttgaactcggcgctaactgcgacagccgatcgagctgtttttgcgcgccatcaatatcgccctgacgtaacaaagaacggaaacgggcggcaacgacgtccgggttattcggatcaataagttccagccgatataacgactgttgcaccagatcttcacgatgggtcgcttcgcctaaccgaacttgctccagcaactgttgctgagcggttggtgctgcctcgaccatcggcatgacggccagaccgagggaaagcgtgaatatgtttagtgtgaatttgcgcattcctggccccagtcaggtaataactcaccttttgtcgagaagcggaaacggtgttgatcccagccttgtccaaacagggtcagcacatagttgtaataggcatcgctgccgggaaagttatcggccacgcgctggcgctgaacggcctgcgcatcgcggttttgtaaaaagggcagcatggcggcagaaaaaccgactggtcctttaccctgcgctttccccgtagccacatccactttttccggcggataaccgtttttctcagtgaatgtcgccatcggtttaaaccggttgagcatccgcgctttttgcggatcgctgtcaggcatcatgcctacccacatgtaaacgcggatagcgtcgtagctgctgatcaatgttttttcggcttttagctgccagcctttgtctttctcatagcgcacccagtctggcgaaaaacctttcggggcggtttccagcaataaacgttgattggtttcgcgcagcgtggtccacggcgcgccaaagcgggtgaaatactgcgccagcgtcggcggcaggtagctggggttaaaacgccagctgttatcctcagcaaaacccactttgcccggtaacaacatggaacccagcccaggcaccgtcaccacttcctcccgcgcgatacgttttagcaacgcgctgccgatgtcggtataacgctgctctttccacaaacgccccgcctccagcaacgaccaggccatccagacatcaccatcggaggccgaattgctgtccagcacttcccacttactgttctctttcttgccccacagccaggcgggcaaacgttcttttaaagaaccctgagcgagattgttctgcgtccagtcgagaatattatcgaaagctgcacggtcgttagccgccagggcagagaacatgccgtaactttgcccttcggaggtggtgattttgcgcgcgtcgctggggtcgatgacgcgcccttcctgactgatgtaatcctttttaaactgctcccaggcaggccaggtacaggctgcctgaacactaaaggcagccagcagcagcatcgtcacgattccactacgcaacacattcatcttcaattactcgttatccgggttaagacgacgacgactaataattcgcagcagacgccacagtacccatgccagcaatatcacactgatagccgccagcaccgccagcagaatcggatggtttgccagcgcataccacacgcgctcgaaccacggcagatgacctacgtaataaacgtcgccaacacgtaggctgttgataccggactcgcggatcaccgcgaccgaaccgaacatggtggcgcgtttgccgctatcgttcaccgcatcgttaagcatttcataaccgcgtgggctatctgccaacagcgcaatcacgctgcgctggtcgttatacggcgactggaagccaatcaccgccgccatcgcaccggaagaggtcagcgttgaccgggtttctgccgcgcgatcgctctcgtccggcacaatgccggggaacggggtctggcgcatcggtgttttcacccagctttcggtcgcctgcaccaataggtcgatctgcttatcgtctttcagtttgtccgggataccaccgatgatcatgatgtcggcatctttgccctgaatggtgctgccatcatcggtcaccgtcagattaatcgccgggaagcccgtctgtgcgccgataaaaccaacagtattcagcaacgtttccatctgtgcttcgttaggcgctttcggcatcacggtgatggtttgcgacagatccgccatccggctgaatgggaagcccgcgttagcaaaggcgcgtagatccggcatcgggatgaagtggtaatacttcgagaagtcgatggtggagtcgtcaccaatcaccacatgattctgcaccggctggaaggtaatacagttatccaccgaaccgcccggcatcgggttcatatactcaaagtcgaagcgcagctggttggtcgcgcccagtttcagcgccggaatagagacatctgttttgccatccagcaaaccttgtaataccggaatccgcagcagcaggcggttcgcctcctgtttgctgctcaggttgaaggattgcaggaactggttattcaggctgatatccatccgcgaactgtctttcaccggcggcatggtgtagcggtaattaatatccatatcaatgccggtactgcgcatcaggtagagatccggcggcaggtttagcgaaacgttaatcgctgctggctcaagaccgctggattgtaactgttcttcataggttttcagttcgccaaatgtgaccggacgatcggtacgtacccagttcggcgcatcgtacggcttacgcggtagcagcggtttcacttcattcactaccacgctttcaccacggaacagaatgttaccctgagcgatacctttcgctgcctgcaacaggtctttgtcgtcacgaccaaacaccaccagcagtttgacgtaaggattctgcggatggttaatcatctcaatcaccggggcttttaccgccggatgatcgcgcaggaagtccggccgtttgtcgttggttgcaaagacaatggcattgcgatccggcagttggttatagagtaccgggaagttctgcccacgccagccagaacgcgaaccaaaccacgaggcgacaatggcagaggcttgttgcagcccaacatccggcgcacccgcaaagaccatcggcaaggtgttggtgcggttatcgctcgggtcaaagaatggcaccgggaagtgtgacaggtcattcttcacattcagggtctgataggtcagatccagtccactgctccgcccaacatccagccaaagcgtggtgctggccggtttttcgcacacgtcctgataatggccgacaaactccagccgtacacggttgaagtcgctaataaacagtgggttaatgggcatttgcgccagcgtttttttacccaactgttctttggtcactggcagcacgcccatcagttcatcattgagataaacctttaactgcgactggacaggcagtaacgatggcgatggggtgtattcgaggttgagcatcgccttcgtcaccacttcatcgctgcgcataccaaactcaatgctgccgttcgggttaatgccacgtagcaccatgctgcccggcggcggtgcaatttgcgcaaaggtcagcttcacatcacgcgaaggaccgttctgcgccacgactggcgcatcagcgccctgcacgcccggcatcacttgccccacctgcggattttgttccgtctgggcggctacagctggctcagcattgatcagtggttgcgttgctggcgtcgcctgcgtcatgaaagaggggaacgcactcatccccatagccactgcacaaatccagaatagttttcttttcatcgcgttatcatcattgttgagccaaagcctgatccgatggttgtgccgtttcgctccgctccgggcggcgcggaataaacgatacaacccaggaaaccagagaagtcagcacacggaatatgcccttcaccgaagaaggcgcaaactccgccagatggcggtagccacggaagccgagcttcagaatatccagcagactttccagcggcttatcttccgggtagctgtcctgccagagcgcccatgtatccgcacgggcaaacgtacactgcacaaaatcgatatgttgctgggtggtgagcggcattaatttcagcccaacttcattacccatcacgcgcgccacctgggtcgggaagacgtattcctgctgaccgcgtttaagcaacagattcactttctgcccttccagaatctgcgcctgaccgttgatcttgatccccaaaccaccgtcggagaaatcctgaacggtacacgagaagaggtgaccatcttcgcgggcaattgccgcgggcatcgtcatctccacgcggtgcgatcggcgtacctgtttgctttctaccgataccgcaactgcgccgccaagaacaatcaggttgtagaacacccacaccatactgacgaccacggtgagcatctcggttggcgggccatagaagtagcgccagatgcctaccgcaacgcccaccaggttgagcaggacaaggaagatgtagggccgcgagatcacccagtcgacgtactcttcttccaccagtccacctttggcggtgacgttaaatttgcctttgtgcgggttaatcagcgccaccagcgtcggtggtgcgatataccacgccagcaccgtttcgtagatttcactccagaaagagtggcgatatttgccctggatcttggagttggtcaggctggcatggatcatatgcggcagcacgaatagggcgatcatcaacgctggcgcatagatgatgtaggcatgaagcagcaggaacgccagcggcgcagtcaggaagatcagccgtggaatgcccgacaagaagtggaacatggcgttgacgtaacatagccgctgagcaaacttcagccctttaccggtgagcgggttatcgagacggaagatttgtaccatcccgcgcgcccagcgaatacgctgaccgatatgcgccgacagactttcggtcgccagccccgccgcctgcggaatacgcatatacgcggaggtatagccacgacggtgcaaccgcagagaagtatgcgcatcttcagtcacggtttcgacagcaatgccgccaatttcatccagcggcttacgacgaatcaccgcacaggaaccgcagaagaaagtggcgtcccacatatcgttgccatcctgcaccagaccatagaacagcgtgccttcgttcggcgttttacggaaacgccccaggttgcgttcaaacgggtccggtgagaagaagtggtgcggcgtctgcatcatcgccagctgtttttctttcaggaaccagcccatggtcatttgcaagaacgatcgcgttggtacgtggtcgcagtcgaaaatcgacacgaactcgcctttggcatatttcagcgcattgttgatgttgcctgctttcgcatgttcatgagtggtgcgggcgatatatttcacccccacgttttgcgcaaactggcgaaactcttccctgccgccgtcatcaaggatccagatattcagcttatctttcggccagtcgatacccagcgaggcgtaaatggtatttttcaccacgttgagatcttcgttgtaagtcgggacaaagatatccaccgacggccacagcgacatatctttcggcaatggcaccggctgacgattcagcggccatactacctggaagtagccgagcaccagcacaatccacgcgtacgtttcagcgaagagcagaataagcccgcacaccaggctgaccggatcgtcccagttcagcgtagaggtgtaacgccaccagatataacggcaagaaacggtcagcgacagcacaatcaacattagcgccgagaagcgccccggcatccgccgtacgatcagcgctaccccccacagcagcatcaggaagataaactgcgccagcgggttaaacggctgagtaacgcagattaacgccagaatcagcgagaaggtgacgatgataccgaggatcaaccgccgcgccccggcactcaaatgaccgagctcttttttctcatccagatgctgtgttttatggctaacgcgctcaggcagctcgttcatccattgatggtaacgtccacgaatattttgcagacctgaaaatgcccgcctgcgcggtttcggcgtttctttgcgcgatgcaccgatcaataaccagcatgtttgaatgagataacggaccgggtccagcggacgcggacgcgaggcgttgatatgcggatacaggtttttatgttctgcgcgaatacgctgccagcgcgggtgctccagcggaataaaaatccaggccaggatcatccagaaacagccgagcgtcgcgctgaaagccgacgcaccgtgacgacgataatcgcgataacgcccgataagccgcgcgttgaccggcgggataagcaaccaccgggtcaggatactcatgatgcactcccgactggcgttttcagcccggagtagttcaacaggcaccagttcgccagcgtcagtatctcttcagccgccagcgcatcactgcgatattcacctactggttgcttagccgccaggcattcagccatcgcttcatcacgatgaatgagcatcggcagtaatcggcgctggctttgcaaccaaagctggtaaatatcgtcctgaacctgactgccaatacggaagtcattaatcaaaatatgtgcgccatccggcagcgcttgctgatgcagtcggatatggcagttggcatccacattgacgattgccagcgagtgatcgcacaaactcagcagctggtgggttatctgcgaggcatcacgcggtaagtcgattaaaatccactggtaacgcccgctggcttttagttgctgtaagccggagcaaatatcgctcagccgggtttgccagtgctgtggattttcttgttcttcaatggataactgaccaaaaggcagcaaatcgagctgcgaggtgtagcgcaacccagcgtcacgccagtcctggccatccagcatcgctctggcccagccctgacggtgggtaaaatcaacattaaatgacaggcgcaacaagttgtccgggcaggcatcgaccaccaggacattttctcccaacatttgtaatgaccaggctaatgcggcggtgatggttgttgtccccacgcctccccgcaccccctgctatcccagtacggccattcaccaatcccctacttttgttgcgcaaactctgccagcaacggccagcgttttaatgccgcggccaactgttcgcgttgggaaatatcggcataatcaatatcaggcagtgaaaatgcctgctttaacgccacaatatcattctggaagatatagcctatcgcgggatcaggcagagtatctggttcattgttattcattttgcttgatccctatgaaataaccgtaccgttcatgagacaattctaaccgtgagcatttcgccggtttattgtttacggcgagacgggaatttgctcactttttgactttccgttacgcaacagaaaaagttaaaaacgaaaagactaaaatcacacgtcttgtgaccttctaaattgattcacatgctaaatctgataagttttaatttcaatggtaggtttatttcttagctttcgctagtaaactgataatcagacaaaatggtgacatgagggacattgtggaccctgtattctctatcggtatctcatcattatgggatgagctgcgacatatgccagcaggcggcgtctggtggtttaacgtcgatcgccatgaagatgctatcagtctggcgaatcaaacaattgcatcccaggctgaaaccgcacacgtcgcggtcattagcatggacagcgatccggcgaaaatctttcaattagatgattctcaagggccggaaaaaataaaattattttcaatgctaaatcatgaaaaaggtctatactatttgacccgtgatttgcagtgttctattgatccccataattacctttttattcttgtttgcgcaaataacgcatggcaaaacattcctgccgagcggcttcgctcatggttggataaaatgaataaatggagcaggttaaaccattgttcgcttttggtaattaatcccggaaataataacgataaacaattttcattgttgcttgaggaataccgttcactttttggtcttgccagtttgcgttttcagggtgaccaacatttgctggatattgccttctggtgcaacgaaaaaggggtcagcgcccgtcagcagcttagcgttcagcaacaaaatggtatctggacattagttcaaagcgaagaggcggagatccaaccacgcagcgacgaaaaacgcattctgagtaatgttgctgtactggaaggtgcgccgccgctatcggaacactggcaactgttcaacaataacgaagtcctgttcaatgaagcccgtaccgctcaggcggcgacggtggtcttttctttacagcaaaatgcgcaaatcgagccactggcccgcagcattcataccctgcgtcgccagcgcggtagtgcgatgaaaatcctcgtgcgggaaaataccgctagcctgcgcgccaccgatgaacgtttgttattggcctgcggtgcaaatatggttattccgtggaatgcgccactctcccgttgtctgacgatgatcgaaagcgtgcaagggcagaagtttagtcgctatgtgccggaagatatcactaccttgctgtcaatgacccagccgctcaaactgcgtggtttccagaagtgggatgtgttctgtaatgccgtcaacaacatgatgaataaccctctattacctgcccacggtaaaggcgttctggttgccctacgtccggtaccgggtatccgcgttgaacaagccctgacgctgtgtcgccctaaccgtaccggcgatatcatgaccattggcggtaatcggctggtgctgtttctctcattctgtcggattaacgatctggataccgcgttgaatcatattttcccattgcctactggcgacattttctcaaaccgtatggtctggtttgaagatgatcaaatcagtgccgagctggtgcagatgcgcttgcttgccccagaacaatggggcatgccgctgcctttaacgcaaagttctaaaccggtcatcaatgccgagcacgatggtcgccactggcgacgaataccagaacccatgcgactgttagatgatgctgtggagcgctcatcatgatgaccatcagcgatatcattgaaattattgtcgtttgcgcactgatatttttcccgctgggctatctggcgcggcactctttgcgacgcattcgcgacaccttacgtttgttctttgctaaacctcgttatgttaaaccggccgggacgttacgccgcacggaaaaagccagggcaaccaaaaaatgactcaatttacgcaaaataccgccatgccttcttccctctggcaatactggcgcggcctttccggctggaacttctattttctggttaagttcggcctgttgtgggcgggatatcttaacttccatccgctcctcaatttggtgtttgccgcgtttctgctgatgccccttccgcgctacagcctgcatcgcttgcgccactggattgccctgccgatcggctttgctttgttctggcatgacacctggttgcctggcccggaaagcataatgagccagggttcgcaggtggcggggttcagtaccgattatttaatcgaccttgtcacacgctttattaactggcagatgattggggccatttttgttttattagtggcctggttattcctgtcacaatggattcgcattaccgtttttgtggttgccatactgctatggctgaacgtacttaccctggcgggaccaagtttctccttgtggccagccggacaaccgacgaccactgtaacaacgacgggtggtaacgcagcggcaaccgttgcggcgacgggtggcgcaccggtagtgggtgatatgcccgcacaaactgcaccgccaacaacggcgaaccttaacgcctggctgaataatttctataacgcggaggcgaaacgtaaatcgaccttcccgtcttcgctgcccgctgatgctcagccatttgaactactggtgattaacatctgttcgctttcctggtcggatatagaagccgccgggttgatgtcgcatccactgtggtcgcatttcgatattgagttcaagaactttaactccgccacctcctacagtggcccggcggcgatccgtttactgcgcgccagctgcgggcagacttcgcacactaatctgtatcaaccggcaaataacgactgctatctgtttgataacctttcgaaactgggctttacccagcacctgatgatgggacataacggccagttcggcggttttttgaaagaagttcgcgaaaatggcggcatgcagagcgaattgatggatcaaacaaatctgccggttattttgctgggctttgatggttcgccggtttatgacgataccgctgtgcttaaccgctggctggacgttaccgaaaaagataaaaacagccgtagtgccacgttctacaacacgcttccactgcatgacggcaaccattatccgggggtcagcaaaacagcggattacaaagcgcgggcgcagaaattctttgatgaactggacgccttctttactgaacttgagaaatcgggtcgtaaagtgatggtggtcgtggtgccggaacacggcggcgcgctgaagggcgacagaatgcaggtatctggcctacgtgatatccctagcccgtctatcaccgacgtccccgttggggtgaaattcttcggcatgaaggcaccgcatcagggggcaccgattgtcatcgaacaaccgagcagcttcctggctatctccgatctggtggttcgcgttctcgatggcaagattttcaccgaagacaatgttgactggaaaaaactcaccagtgggttgccacaaacagcaccggtctccgagaactcaaatgcagtagttattcaataccaggataaaccgtacgttcgcctgaacggcggcgactgggtgccttacccgcagtaagaacgaaaaaggccgcagagtttcccccctgcggcctggtccgggcgcaaattgccattacggcagcctgacgcccgcatgacacgttacttccgcttgttcagccagttcacgatcatactggcaagaatgccagcaatgaccggagccgctaaatcatgccagaaggccatgcccagctctgcgaacgtcatatagccgcctgtgttgtaatgacaacgtttcgcggctattcttgagtggtctagagtcaagattagcccccgtggtgttgtcaggtgcatacctgcaacgtgcgggggttttctctctccagcaaccaatgccaccagggataaagcccccgcaacattgcgcctcaccggaacctttccggcttgccgctgattctacgattgctttttactgtcagcacccggcaatcttcctcattgcgcgatgccttccagcttaatttctttatttgcaatagttgcagttcatatccgggctgactccagactggtagtgaaatgcgcaattttgtagaattgcgcctcctcgcgacctccccagtgaatctgttgcctcattttttacatactgcgtattcgacttctccacctgttgcgcaagagaaactgggtttattcatttttgcgaggccgacttctttctggacaggactttatgcagcacaacacactatcgaaacacaatcagaaattgccgtttacacgctacgacttcggctgggttttattatgcataggcatggcgattggtgccggaaccgtgctgatgccagtacaaattggcttgaagggaatttgggtatttattaccgcagcgatcattgcttatcctgccacctgggtagtgcaggacatttatttaaaaaccctttctgaaagcgattcctgtaatgactacaccgatattatcagtcattacctggggaagaactggggaattttcctcggggttatctactttttgatgattatccacgggatttttatctactctctctccgtggttttcgacagcgcctcgtacctgaaaaccttcggtttaaccgatgccgatctttcacaatctctactttataaagtcgctattttcgccgtactggtggcgattgcgtctggtggtgaacgattactgtttaagatttccgggccaatggtggtggtcaaagtagggattattgtcgtgttcggttttgcgatgatcccgcactggaatttcgccaatataaccgccttcccgcaagcctccgtctttttccgcgatgtcttgcttaccattccattttgcttcttttctgcagtatttattcaggtacttaacccaatgaatattgcctatcgtaaacgggaagcggataaagtactggcaacccggctcgcgctgcgtacccaccgaattagttatatcacgctcatcgcggtgatcctgttttttgccttttcgtttaccttctcaattagccacgaagaagccgtttctgcctttgaacaaaatatctcagcactggcgctggccgcgcaggtgatccctgggcatatcattcatatcacctctacggtgcttaatatctttgccgtactgaccgcattctttggcatttatctcggtttccacgaggccattaaaggcattattctcaatctgttaagccgaattattgataccaagaaaattaactcacgcgtgctgactctggcgatctgcgcttttatcgtcattacgttgacgatttgggtttcgtttcgtgtatcggtgctggtgttctttcagttgggaagcccgttatatggtattgtgtcgtgcctcattccgtttttcctgatctataaagtcgcacaactggaaaaacttcgcggatttaaagcctggctgattctgctgtacggcattttgctatgcttgtcgccactgttgaagctgattgagtaaaccggagcgcatggccccggttttgtgagttaacgctgcggattttcatcctgatcaacagcaaaacaagctaccagttgaccgccgtagtcttttagctgcggctgcaactgggtgcaggggccgaagcgccgacgacagcgggcgttgaaggcgcaacccggcggtggattcagtgggcttggtagttcaccgctgagcttgatgcgctcgcggcgatcgtccgggttcaggcgcggcgtcgcggaaagtagcgcctgagtgtacggatggcgcgggttattgaagatttggtctttcgttcccttctccacgcagcggcccaggtacatcaccatcacttcatcagcaatgtgctccaccaccgacaggtcgtgggagataaagacataagacagccccaactcctgctgcaaatccatcatcagattcagcacctgcgcgcgcactgaaacatccagcgcggaaaccggttcatcggcaatcaccacatccgggtcgagcatcagaccacgggcgatggcgatacgctgacgctgaccgccggagaacatatgcggatagcggtcatagtgctcggttttcaggccgactttcgccatcatcgacagggctttttcccgacgctgttctttgcttaagctggtgttgatcagcagcggctcttcaagaatttgcccgacttttttacgcggattcagcgaaccgtaagggttctggaagacgatctggattttctgccgacgcagcttctgcgcctgcggatcgtgcttaagcagatcctgcccctggtaatacagctcgccaccggtgggcatttcaatcatcgtcagcaaccgaccgagggtcgatttaccgcagccagattcgcccactactgccagcgttttgccacgttcaaggttaaacgaaacgccatccagcgctttaaccagacgttccggcgcgaacatgcctttcttcaccggataatgttttttcaggtcgatagcctgcaacagcggttgttgcagggtggcctcttgcgtactcatagtgtcggcctcccggcatcatcaagtgggtaatggcatttggactgacgcccgtcagcgagcatattcagcgccggttcttcagcgcgacatctgtcagtggcataggggcagcgcgggttaagcaggcagccgttcgggcggtcgtacttgccgggaacgacacctggcaacgacgccagacgttctttgtcctgagcaaattctggcagcgcacgcagcaatgcctgagtatacgggtgacgcggcgcatggaagatggcgtgcgcatcaccggtttccaccacctggcctgcatacatcacgatgattttatgtgccgcttccgccaccagcgccaggtcatgggtaattaacaccagcgccatgttctctttctgctgtagctccagcagtagttcgatgatttgcgcctgaatggtcacgtccagcgcggtggtcggttcatcggcaatcagcagttttggccgacaggcaatcgccatggcgatcatcacgcgctggctcatgccgccggaaagctgatgcgggtaaacatccagacgcgatgccggatcgggaataccgacctgattcagcaggtcaatcgctcgctgacggcgggtacttttgttgccgccctgatgcaccttaatcgcttccataatctggaaacccacggtgtagcacgggttaaggctggtcatcgggtcctggaagatcatcgccacttcggcacccaccaggttgcggcgctctttttctgagatacgctgcaaatcctggccgttaaactccagtttttctgccattacgcggcccggataatcaatcagccccataatcgccagtgaactgaccgacttaccggagccggactcacccacaatcccgaccacttcgccctgttttacgctgtagctgatgcggtctacggcgcggaacggcgcgctttcgtcgccgaaatgcaccgataatttatctacatttaataacgccatctcgaacctcttactgcttcagtttgggatcgagcgcgtcacgcagaccgtcacccatcaggttaaatgccagcaccgtcagcaggatcgccagacccgggaaggtcacgacccaccaggcgctttgcgcgaactgcaacacgtcggagagcatggtgccccactcaggcgttggcggctgtgcccccatgccgaggaaaccaagagcagccatatcgagaatggcgttagagaaaccgagcgacgcctgaacaatcagcggcgcaaggcagttcgggaagatgttaataaacatctgacgcatcgccccggcacccgccacgcgagacgcggtgacgtaatcgcggttaacttccaccagcacggcggcgcgggttaagcgcacatagtgcggcaaggcaacgaaggtcagtgccagcgcggcgttaccaatcgacgggccgaaaattgccaccagcaccagcgccagcagcagacttggcagcgccagcatgatatcgaccacgcgcataatgatgttatcgaccaggccgccaaagtaaccggcgatcaggccgagaataacgcccataatcagcgataacacaactaccagacagccaaccagcagcgacaggcgcgcaccgtacatcaggcgcgacagcacatcacggcctacgtcatcggtgcccagcaagtgcgccatgctgccgccttcctgccaggctggcggggcgagcagtgcatcgcggaactgttccgccgggttatagggtgcaatccagttggcaaagatcgcgatgaacagcacgatgacgacgtaaaccagcccgacgaccgcgcctttgttgcgtttaaaatagtgccagaactcctgtaacggggtcatcggcaccggtgcgctaatcactttattttcagtaacctgtgacatgatgtccccttacttcttatgacgaatacgcgggttcaccacgccgtacagcagatcgaccagcaagttgacgaggataatcatcgtcgccaccagcaatacgccgccctgcactaccggatagtcgcggcgttgcagtgcgtcaatcaaccagcgtcccagaccgggccacgagaagatggtttcggtcagaatcgcccccgccagcaatgttcccacctgcaggccgataacggtcaccaccggcagcatcgcgttacgcagcgcatggacgataatcacccgcatgcgggttagccctttggcgcgcgcggtgcggatgtaatcctcgcccagcacttccagcatcgaggagcgtgtcatacgcacaatgaccgccagcggaatagtacccagcacaatggcaggcaagatcatatgggcgacggcatcgataaagttgccgtcttcaccccagatggcggtgtcgattagcataaaaccggttaacggattggagtcatcgaggaacaccatatcgctcacgcgaccggagacgggcgtcaggttccagtgcaccgaaaccagcatgatcagcatcatgccccaccagaagataggcattgaataacctgtcagcgccaggccaaccgctgtgtgatcgaaaatggaaccgcgtttaaccgcagccagcacgccgaccggaataccgactgccgtagcaaaaatcatcgcgcagacgccaagttccagcgtggcctggaagcgcggcacgaactcttcccaaaccgggatgcggcttttcattgaaatgcctagatcgccatgcataacgccccaaatgtaatggagatactgctgccacatcggtttatctaagccgagttcagccagcagctgcgcgtgacgctctggggagatcccacgttcgcccgccatgatcatcaccggatcgcccgggatcatgtggacaaaggcaaatgtgagaagggtaataccgataaacgtggggatgacgagtcccaaacgtcggagaataaactgcaacataacccggattctctatagtgacccgcagcctggaactgcgtgtctgtattgctcacaaatcaattcccgcccttatcggacagggaatgaagtattgctgccggatggcgctgcacgcagaggcacagcgccaccgggtatacagattgttgacaaagtgcgctttgtttatgccggatgcggcgttaacgccttatccggcctacaaaatcgtgcaaattcaatacattgcagaattttcgtaggcctgataagcggagcgcatcaggcatttttgcctttgccatcagtcttgtatggcttttaattattcgatagagacgttttcgaagtgatgtttgcctaatggatcaaccacatagcctttaacttctttacgtaccggttcaaacacggtggagtgagcgatgatcagtgccggagcctgatcgtgcatcaccacctgcgcttgtttgtacagttcaacgcgtttattgtggtcgtcggtagcacgcgccggttgaatcagatcttcaaacggtttgtagcaccattttgagtagttggagccttgttcagaggcggcgcagctgaacagggtggcgaagaagttatccggatccccgttatcgccagtccagcccatcattaccgtctggtgctcgccatctttcgcacgcttgaggtactcaccccattcgtaggtgacaattttggcctgcacgccgactttcgcccagtctgcctgaatcatctccgccatgcggcgagcgttcgggttatacggacgttgtaccggcatcgcccacaggtcgatggagaaacctttttccagacccgcttctttcagcaaggctttcgctttttcaggatcgtaggtgtagtcctgaacgtcgtcgttatagccccacatggttggcgggatcaggtttttcgctgatacgcccgcgccctgataaaccgctttgatgatcgcgtctttgttcaccgcgtaggtcagagcctggcgaactttcacgtcatcgagtggttttttctgcacgttatacgagagataaccgacgttcagccccggcatttccatcagattgatggatttatcctgcttcatgcgagcgatatctgccgggttcgggtacggcatcacctggcattcattcttctgcaatttcgcgtaacgcacggaagcgtcaggggtaatagagaaaaccagcgtatcgatctgcggtttggtgccccagtagccatcaaacgctttgtagcggatacgggaatctttttgatactgctgtaactggaacggaccggttccgattgggttgaggtccagtttttccggtgtaccggctttcatcatcgcatcagcatattcttttgacagaatagaggcgaagtccattgccaggtcagcgaggaacggcgcttccgggcgagtcagcacaaactgaacggtgttgtcgtccacctttttcacttcactgatcagctctggcaagcccatgccttcgaagtattcgtagctgccgccagaaactttatggtacgggttttgcgcgtttttctgacgatcgaacgagaacaccacatcatcggcgttcagttcacgcgtcggtttgaattctttattgtcgtgccacttcacacctttacgcagatggaaggtataggttttaccgtcttcgctgacttcccacttttcagcgaggcccgggatcacttcggtggtgccgattttaaattcaaccagacggttataaagcgggacggaagaggcgtcataggtggtgccggaggtaaacagctgcgggttaaacccttccggagatccttctgagcaataaaccagagttttagcctgaacacttgctgcgacggtcatagccaccaggctgagaccaagcttcagcatccctgactttttcaaggaaatacgcattattctgctccaattgtgatgtttgttgttttaaccctttgcagtgggttgtcgctgcctgaccttttttgttttttgcccggtcgggtcaacgttatgaggtggggatgccgtactaattaacatcagtgtaacagtgcggatcctccataaaatgcccctcgtgacctacaatctgtcaacagaatgtgaaaacgtcaatacagccaaccgggatttacaccaacggtgagaatccacacacaaagattaaaaaaacttcaaacagctatttgcagcagagaaatttgtgctactccaacatgaccagaacaatcagcttaatatttagcaacatttggtgattaagttttatgcatttaatgaaaaaaatctgaggaaaaggtggatatctgagcgattaataccatgaacgctaaaacgcacagcggaaaatgccagggccagccataagtaacgcaaaaaaagatttaagcaaatataaaaaaagacaatggtttctgtcacaaatccgttaatggatagtgagatatggggcgcaaatttggcagggaaatgtgtgtcgtgtaggtcgaataaggcggtcgcgccgcatccgacaatggccggcacatttgcctgatgcgacgctgacgcgtcttatcaggcctacgtcgagtcgaacctccctgcccccggaggttctcatcctcatgagctgcagatgcaaaaaagcctgctcgttgagcaggcttttcgaatttggtcggtgatagaggattactcgccacttcgtggctcgccctgcgggccgttgctggcgcaacgttctctcgcttcgctcgagtcgaacctccctgcccccggaggttctcatcctcatgagctgcagatgcaaaaaagcctgctcgttgagcaggcttttcgaatttggtcggtgatagaggattcgaacctccgaccccttcgtcccgaacgaagtgcgctaccaggctgcgccaatcaccgaatgcggggcgcatcttactgcgcagatacgccctcgtcaatcccttaatagcaaaatgccttttgatcggcgagaaagtcagcaggccgcttagttagccgctgcctcttttgcctgcgggatgtgacaccagttgttgttttcgttaattccaccatccggtgaagtatagccaagacaacccatgatggtatcgtacagctctacgtgacggcgtggcactttcatgtcggcttcttttttcagctgcgcaaacgcctgcgcattggccggattttccagatatttatctgacatccagaccatcatcggtacgcggaactgctccggcggtgccagttcacgcggcgtgccgtgcaggtgctcgcgttcattaattgactcaccgtggtcagctgcgtagaacacaatcgctttcttatcgcgaacctgatcaatcacgctggagataaagtgatccacataggtcaccgagttgtcataggagttgatcatctgcgctttggtacagccgctatcaacaccaatacattccggcttccactgcgcgaagctacgcggataacgctgggtgtagttaaaatgcgaacctttggtatgcagaatgatcagatgcttaccatccgggttgcgccctagcgattgctgcatttcgtctaccagcaacatatcatctaccggcttgccacgattacgtggctccgcaccaatctgctcacgataagcaatgttgtccgccatcgtgttgctgtagaaccacatttcgctctgcatagcgtagaggtcagaactgaatcctaactgcttcagaaccgcgaaaatgttctgttcttttaatgtgcgctgcggattatcttccgcgcccccctgacgtacaaacatgcaacgcagtgagagtttggttgcggtatcacaggagtaaccacggaacgccgccagatttttctcctgggccagtttcggcgtggtattacgctcatagccgaaaatacccatatggtcccaacgcgtggtttcaccgatgataaacacgacataagtgtcatcaacgttttgcggtgcctgataagtgaatttcttcgccggattaagcaatgaattattatcggaagattcatcgacccgcgcccaggcatacagccccaacgcagaaagccagtttgatggcagataagagttcgctacgacaccgccataactcggcaaatcaacgccggtcgccctctccactttcttctgctggatatccagcaaacgaatcggtgcccaaaccataatacccgccagtacgacgaccgccaggctgcgaatacgctgccctggggttcgcagttgtcggagcaaggtgtagcgacagcggttattccagataaggataagaggcaatgcactaacggcgattaaccagagaataaagttcagaccaacaacttcttttgacaggtcgatatcggtggtcatgacggaagcgatgatgccataaccaatgaccacattaaggaaggtcatgtaatagctggcacctgcggaaaagagcaccaccagcgatgccagaatacgccagctgcggcggccaaacagcgaaagaagacgtagtaaaaagaaggtcaccagtacggtggcggccagttcaacaacagcagaaatgcctttccagacggtaaaatcgtgcgcatagctgccgaagcggcggtaaaaaaccgcgccattcataaaaaggccaatatagattgcaagcaaaaagctcagcttctgctgtgtaatcgatttgatgtatctcatgcaaacaaaccctggacaaacaggtgataacaccctgcttagtggcttttcaggcccggcagggaaaaagtgcggaggtagtcagataagtaaaatctacacgcgcgaataagtagaccacagcaaagggaaaaagtgtggggaaagagtgtgcatgaagcacaaatttacaaaaatgcaagtttgaaaagagactttagcgttacaaaaagcagtaaaaagggccagttaattggcccaaattttacgagtcattgtttatacatttcgttgatgcgtttgatgcacacggaagctgaagcccagtagctcgcggctgagcattaaagggagccatgcgcctcacgcaacattttctgctctggctgacgaatcgtcgtagaaagcgccaatgacagaatcagcagggcgaaaatcacgtagaaggtcacatagaagccgccaaacagtgaggcgataatcgaaccacaaatgctaccgataccgaaaccgagataaatcacaccgtagtttttcgccaggttattgaggccaaagaactcactgaccagtgacggaaagacggtaatagtgccgccaaagttaaatgccacgcaggcaatcgctgcaaagaacgtcactgcattcaatggtgcaaacagcagggccgccatacccaccagcgatatcacctgaccaatggtaataacacggatacgggcgattttgtcagacagaatacccagcaccagacgacctgaaaggttggcgatggaaataacagtgactgcattggctgcggaaaccacatcaaggtgtgccagactttgggcgatatctttcgctaccccaatcacgtacaggccgctcatgcaggcggtcaggaacattaccgctaacatccagtactgcggtttacgcatcgactctgccagcgtgtaatctttctccaccacaccattgctggttttcacttcctgttttggtgcgtctttcattaacgttgcgccgaaaacaatcatcaacagcgcaatcgctccccaaatcacaaaggttttttccagaccgaccgtttccagcagctgcgtgtcgataaatttgaaacccaggctacccagaccataagaaccgatagcgaacgcggagatcagacctttacgctccgggaaccacttcacacagttagagagcgtcagcagataacccgcgccatctgccagtcccaccagcacaccggcgcttaaccacagcatcatcaggttgtcagaatgcgctgtcaggaagaagcctaatcccagcaaaatgccggaagccatggtgacgcgtttaacgccaaaacgttcctgtaatttgcccgcaacagaagacgaaattgccagccccagacttaacaagccgaaagagaaagcgacctggcttaccggcgcatccagcttggcggaaagcgcgccattaaacaggctccaggtataaaccgaccccagcgcaaactgggtaatgatagtaccgatgagtgtcagccagcgggtacgctgataatttgaaggtgtcatggcagtattcctgcagtaataaaaaggaaaaatctctgccgacaaccataacgaagtgcactttatgcctggggaaaaacggcatgaaatgccatcagaacggaatgaaatgccttagttcaggaatgaatgacgcgacaattattcaccaaatttattatttggtaagttagcacccactatcgccacaactattgttatttaatggtttcaattgtgactgttacgttaaaatctggcgctaacccccatcgtatacagatagtcgctattattagtggtattttctgcctgagttagcgcggcataggcggcaatattttgattgagcaacatatcagcgcctacggtgacatccagccagttgccgttctggtttgtcgccgtcatccggctcaggcctgattgcgccttccagatattctcgccaaattgctggttatagctgatttgcgcccagggtcggagatcgccaagccgggagtcaacacgccagcctaaggtactcacgctggcatgccataacggatcggtcagcgtggtagtactgtcgccaaactcgttatacatcgaggtggttgtgccatcgtaatgtaatgccgcgaccgggccggttgtaacctgttcatataaaggaaaattccagcccatactcatactgctggtcacatccacaggggtttcttccgccagattgacttccagtcccagcgccctttggctactttgaatacgttgcgacaaaatatcgttgtaatcaggttgatgatcactatcccaggtgtaacgctctgtggaaagtccgggttgcgtatcaacgatatattcttgttgccaggcgtaagctgtgttgagaaaaaaggcactgattaccacgctcgccagcaggcttagctgccagcgaccaccgcttttttttatgatcattaacacgactccagggaagagccgaattcggcaatattattgtcattgtatgaaggatatcgggcatagtagccctgtattaaatattgactttttcaccgatgcgtcaagaaaagcggctgaaatttttacgatcgggtacatagcgagggaaagtatggaacgttgcggctgggtgagtcaggacccgctttatattgcctaccatgataatgagtggggcgtgcctgaaactgacagtaaaaaactgttcgaaatgatctgccttgaagggcagcaggctggattatcgtggatcaccgtcctcaaaaaacgcgaaaactatcgcgcctgctttcatcagttcgatccggtgaaggtcgcagcaatgcaggaagaggatgtcgaaagactggtacaggacgccgggattatccgccatcgagggaaaattcaggcaattattggtaatgcgcgggcgtacctgcaaatggaacagaacggcgaaccgtttgtcgactttgtctggtcgtttgtaaatcatcagccacaggtgacacaagccacaacgttgagcgaaattcccacatctacgtccgcctccgacgccctatctaaggcactgaaaaaacgtggttttaagtttgtcggcaccacaatctgttactcctttatgcaggcatgtgggctggtgaatgatcatgtggttggctgctgttgctatccgggaaataaaccatgattcgggaagcgcaacgttcagaactccccgcgatcctcgaactgtggctggaaagtacaacctgggggcatccctttataaaagcgaattactggcgtgactgcattccgctggtgcgggatgcctatcttgccaacgcgcaaaactgggtctgggaagaagacggtaagcttctcggttttgtcagcattatggaaggccgatttctggcagcgatgtttgtcgcaccgaaggccgtcaggcgcggtattggtaaggcgctgatgcagtatgtgcagcagcgccatccccacctgatgctggaggtttatcaaaaaaatcaaccggcgataaatttttaccaggcacagggttttcacattgtcgattgcgcatggcaggatgaaacccaactacccacatggattatgagctggccggtggttcaaacgctgtaagtgtcagttccggaccgttgtatttttccagccatgccagcgccgtattacccgcacagccattccccagccgcgagctggggagatctttggtcagcacgttcactgcgccgtttttacaaataccgtcagcggttaaatccagatccggccatgccccttcgtgaatgcaaatcacgccaggtttaattccctcgctaatgaccgctccggcaagaatttgcccgcgtgcgttccacaaccgaacagtatcgccatcttgtatgccgcgctcctgggcatcgtcaggatgaatggtgacaggctcacgatttgccaccgcgtacaattcgcgcagagaactgtaattcagctggctgtgcaggcggtgcgccggatgggcagaaagtacctgcaactgttctggttcggcattgccctgccattcgtccggctccagccacattggatgcccagggcaatccgggtaaccgtaatcggcaatacgctgtgagaagatttcaatcttgccgctggcggtttttaacggatgcgccagcggatcgcggcaaaaatcagcgaagcgaataaaccgctcgctgtccgggttttccggcatctcaattaactggttggcttgccagaactcagcaaatggcggcaattcaacctgctggcttgccccgcgctgtcgggcaacgttataaaacgtttccagccattgcagctcactttttccttccgtaaaacgtgcataaccgcccttctcccagcgttcacttaactcggcaaaaacatcaaaatcattacgcgcttcatagcgtggcggcaccacttgcttcatcggcaccagatgctgattactgtaatcaccggtcatggtgagatcattacgctcaaaagaggtagtcgcaggcagaacgatatccgcgtgttttgccgccgccgtccagaagcattcagagatcaccaccagctccggtttttgccaggcacggatcaggcgattggtatcctgatgatgagtaaagttggcaccgcccgcccaccagataaaacgaatatccgggaaatgtcggttcataccgttgtgttgatatgcgccaccagggttttccagtgcttcaacaatgcgggcaacagggattttatccaccgcatcgcagccacccggcaagctgccctgcatggaagagagcaccgcagaacgccgcgtggggttaccaccattggcaaaatggtaagaaagaccaaaaccgccgccgggtgtgccgatttgccccaacattgctgccagcgtgacgatcatccagtgtttttgctcaccaaactgttggcgctgcattccccagcctgccatcagcatggtggtattttggtggaaaatagccgccagctcgcggattttcgctgcgccaacaccacaaatctctgctgcccattcggcggttttcgctattccgtcactctcgcccagcaaataagaggcgaagacggcataacctgtggtgcaacgcgccagaaacgcttcgtcgtgccaaccattttccaccagcgtatgggcgatccccagcatcagcgcaacatcggtgcccatgtgcggtgccacccactccattttatcgccaaagaaatcgacggtttccgatcgcattggatcaatgcagatcagctttttcccgctgtcacgcagtgcagaaaagtaagaaagcccctgctcatcggatgcattccacgcaattttcagcgtattgagtgggttagcactccacagcaccacgacatcgctatgttccagcaccagcggccaactggtctgctgttgataaacttcactaccacccacgacatacggcatgatcgcctgtgccgcgccggtcgaataatcccccagatgcccggtataaccgcctgccagcgccatatagcgttgtaataatgtcgaggccttatgcagcacgccgtttgaacgccagccgtaggaaccagcaaaaatcgatgccggaccataagcctcacgaatgcgtttatgttgttggtgaataagatccagcgcctcatcccaactcacgcgaacaaattcatcctgcccacgaatgccttgcgggttttccggtgacgcaagaaagccttttcgcaccattggaaatcgtacccgcgtattgctgtgaacctggtcgcgaaccgcgctctgcaaggagttttccattcctgtggctaacgcgccacgcgagctaaacacggtttcgccgtcggtttcaaccagcatgggcccccaatgggcggcagtcagaacggaatatcgtgaggatgagttggccaaaccgaagactcctgaaaggttagatgtattgagcagttaaatattacttacaaatttccgagtattcccaggaataatcttcatgttcacgcggcataatctcccgccacggaacccgtggcaaagaataaaaaggttattaaggattaacaatgaagaaacgtgtttatcttattgccgccgtagtgagtggcgctctggcggtatctggctgcacaactaacccttacaccggcgaacgcgaagcaggtaaatctgctatcggcgcaggtctgggctctctcgtgggcgcgggtattggtgcgctctcttcttcgaagaaagatcgcggtaaaggcgcgctgattggcgcagcagcaggcgcagctctgggcggcggcgttggttattacatggatgtgcaggaagcgaagctgcgcgacaaaatgcgcggcactggtgttagcgtaacccgcagcggggataacattatcctcaatatgccgaacaatgtgaccttcgacagcagcagcgcgaccctgaaaccggcgggcgctaacaccctgaccggcgtggcaatggtactgaaagagtatccgaaaacggcggttaacgtgattggttataccgacagcacgggtggtcacgacctgaacatgcgtctctcccagcaacgtgcggattccgttgccagcgcgttgatcacccagggcgtggacgccagccgcatccgtactcagggccttggcccggctaacccaatcgccagcaacagcaccgcagaaggtaaggcgcaaaaccgccgtgtagaaattaccttaagcccgctgtaatccctttcatgccaggtgatgcagaaatcacctggcattcttcagttttccttcatcatatttcaggctaaggtgatcgccttatcagtgaatggagagaagcatgaagccgtccgttatcctctacaaagccttacctgatgatttactgcaacgcctgcaagagcatttcaccgttcaccaggtggcaaacctcagcccacaaaccgtcgaacaaaatgcagcaatttttgccgaagctgaaggtttactgggttcaaacgagaatgtaaatgccgcattgctggaaaaaatgccgaaactgcgtgccacatcaacgatctccgtcggctatgacaattttgatgtcgatgcgcttaccgcccgaaaaattctgctgatgcacacgccaaccgtattaacagaaaccgtcgccgatacgctgatggcgctggtgttgtctaccgctcgtcgggttgtggaggtagcagaacgggtaaaagcaggcgaatggaccgcgagcataggcccggactggtacggcactgacgttcaccataaaacactgggcattgtcgggatgggacggatcggcatggcgctggcacaacgtgcgcactttggcttcaacatgcccatcctctataacgcgcgccgccaccataaagaagcagaagaacgcttcaacgcccgctactgcgatttggatactctgttacaagagtcagatttcgtttgcctgatcctgccgttaactgatgagacgcatcatctgtttggcgcagaacaattcgccaaaatgaaatcctccgccattttcattaatgccggacgtggcccggtggttgacgaaaatgcactgatcgcagcattgcagaaaggcgaaattcacgctgccgggctggatgtcttcgaacaagagccactgtccgtagattcgccgttgctctcaatggccaacgtcgtcgcagtaccgcatattggatctgccacccatgagacgcgttatggcatggccgcctgtgccgtggataatttgattgatgcgttacaaggaaaggttgagaagaactgtgtgaatccgcacgtcgcggactaagccgcgactgcgtagagtaaagcccgataatcgctcgggcttttactctttattgggttgcagtaactgctgtagtccaggcctgattaaacgcctgatgctgtgccggtaatggcgcaatcagtttgttatattcacttgcctgctgtgaagtcgggaactggatgccatttgcgacaaagctcacctgagtaccttgctgagcaatgtagtctccaaccatcaccagttgttgcgtgaaagtttgtgccgccggaatcaacggttgcaatgcatcagctggcgtcgttaccactttggtgaatgcctgatcaaagaccggtttcaaatcatcgctctgttttagcgcagagtgcgcagcatcggcctgcaacttcgcattttgcagttgttgcgccagcacacccagcgaaccgttcatttcacgcagcggaccgctttgcgtaacgtaatcctgcggtacgcgaattgcgttaacgctgtctacaaccgggcgcagaccggaatccatcgcctgattcacctgctgagaataaccatacagaatcgcgtaatcagagacaaaaggaccaaactgttttttctgatcggcagtcagggttggtagacgttcaccgctacgcatcactgtattctgcaggaagtcgataaacgctttacgctgatcgccttctttatcaaaacacccactcaggctaactaccattaataacgccgcaagaggcgcaaaccagcgagagcaggactttcctgtcgccattttcttactcctttcacccaaaaaaagcgcacaacgacacacgcgtgtctgacgtgacaaggatagtccaggacaggcttgcaggataccctttctacgtaatcttcctggtaaaatcatggagaaaatgaaacaaggttaatttgttgtttcattgttaaaaaatgatagtgccgttgccttttttgtagccagagatttacgccttcgcagaaggttagattttcgaaatctttacaaaacaggagtggtaagagatatatcggcatttatcagatcgttaggtggctataagtcacgctaaatgacaggctgaatcgaatcatagccagagcatgccctgacttcaccccgctgtgtctgcttttcccgactattcttaatgagcttcgatgcaattcacgatcccgcagtgtgatttgaggagttttcaatggaatataaagatccaatgcatgagctgttgagcagcctggaacagattgtttttaaagatgaaacgcagaaaattaccctgacgcacagaacaacgtcctgtaccgaaattgagcagttacgaaaagggacaggattaaaaatcgatgatttcgcccgggttttgggcgtatcagtcgccatggtaaaggaatgggaatccagacgcgtgaagccttcaagtgccgaactaaaattgatgcgtttgattcaagccaacccggcattaagtaagcagttgatggaatagacttttatccactttattgctgtttacggtcctgatgacaggaccgttttccaaccgattaatcataaatatgaaaaataattgttgcatcacccgccaatgcgtggcttaatgcacatcaacggtttgacgtacagaccattaaagcagtgtagtaaggcaagtcccttcaagagttatcgttgatacccctcgtagtgcacattcctttaacgcttcaaaatctgtaaagcacgccatatcgccgaaaggcacacttaattattaaaggtaatacactatgtccggtaaaatgactggtatcgtaaaatggttcaacgctgacaaaggcttcggcttcatcactcctgacgatggctctaaagatgtgttcgtacacttctctgctatccagaacgatggttacaaatctctggacgaaggtcagaaagtgtccttcaccatcgaaagcggcgctaaaggcccggcagctggtaacgtaaccagcctgtaatctctgcttaaaagcacagaatctaagatccctgccatttggcggggatttttttatttgttttcaggaaataaataatcgatcgcgtaataaaatctattattatttttgtgaagaataaatttgggtgcaatgagaatgcgcaacgccgtaagtaaggcgggaataatttcccgccgaagactcttactctttcaatttgcaggctaaaaacgccgccagctcataactctcctgtttaatatgcaattcacacagtgaatctcttatcatccaggtgaaaaataaaagcgtgaaacaaatcactattaaagaaagtaatctatatttctgcggcattcccagcctcctgtgttgatttccaacgagtatgtactgcacccattttgttggacgatgaaatggaatagcccctaatatgtcaaagccaaaatacccttttgaaaagcgccttgaagtcgtgaatcactacttcacaactgatgatggttacaggatcatctcggcacgttttggtgtcccccgaacccaggtcaggacatgggttgccctctatgaaaaacatggagaaaaaggtttaattcccaaacctaaaggcgttagtgctgatccagagttgcgtattaaggtcgtgaaagctgtgatcgagcagcacatgtcccttaatcaggctgctgctcactttatgcttgctggtagtggttctgtagccaggtggctgaaggtctatgaagagcgcggagaagctggtttacgcgcgctcaagattggcaccaaaagaaacattgcaatatcagttgatccagaaaaagcggcatcagcattggagctgtcaaaagaccgacgcattgaggatcttgaaaggcaagttcgatttcttgaaacgcggcttatgtatctaaaaaagctgaaagccttagctcatcccacgaaaaagtgaaagtactcaacgagctaaggcagttttatcctcttgatgagcttctcagggctgcggagataccgcgcagtacgttttattatcatctaaaggctctcagcaagcctgacaagtatgcggacgttaaaaagcgtattagtgagatttatcacgagaatagaggccgatacggataccgtagggtaacgctgtctcttcatcgagaagggaaacagattaaccataaagctgttcagcgcctgatgggaaccctctcacttaaagcagcgattaaggtcaagcgataccgctcttacagaggagaggtagggcaaaccgcccctaatgttctccaaagagatttcaaggctacgcggccaaacgagaagtgggttaccgatgttactgaatttgcagtcaatgggcgcaagctgtatttgtctccagtaatagatctcttcaacaacgaagttatttcttacagcctttcggaaagaccagtgatgaacatggttgagaatatgctcgatcaggcattcaaaaagcttaatcctcacgagcatcctgttctgcactctgaccagggatggcagtatcgtatgagaagatatcaaaatatccttaaagaacatggtattaaacaaagcatgtccagaaaaggcaattgtctggataatgctgtggtggagtgtttctttggaaccttaaagtcggagtgtttttatcttgatgagttcagtaatataagcgaactgaaggatgctgttacggaatatattgaatactacaacagcagaagaattagcctgaaattaaaaggtctgactccaattgaatatcggaatcagacctatatgcctcgtgtttaactgtccaactttttggggtcagtacaaactttgatttatagtcaggtggggcttttctctgtctgcctttcggtgaatacctgagacaaacagtctcaagcacccgtggctattctagcttaataagtttgtttcttctccttgatataatcctaaaaaaatctcataaaattaatatatgagataatctttattcagcagaagattattaaaggttgctgtattatttagcgataaaaaaagcctgccagatggcaggctatttaataacggcgttattattgcaacagcgaaatatccgcaacgcgcaggaacagttcgcgcagtttctccagcatggtcagacggttgatacgcaattctttgtcatcaaccatgaccatcactttatcgaagaaagcatcaaccggttcacgcagctcagccagttcgaccagcgcatcctggtaacgaccttccgtaaagtacggctccagcttgtcacgtagcaccacaacctgcatcgccagtttaatttcttccggctctttcagggtagaggcattcacgcggtcgctcagcacttcgtcagatttcgccagaatgttagatacacgtttgttcgccgccgccagtgcagcagctgcatccagggtacggaaatgcgataccgctttcatacgggcatcgaaatcagccggacgagtcggacgacgcgccagtaccgcctggatggtgtcaacggtataaccttcgtcctgataccaggcgcggaagcgaccgagcataaagtcgataacatcatcaactacgttggcattagtcagcttatcgccatacagacgcaccgcttcttcggtcagcgtttgcagatcaaggttgaggttcttctcaacgataattcgcagcacgccaagcgcggcacgacgcagcgcaaacgggtctttgtcgcctttcggatgctgaccgataccgaagatacccgccagggtatccatcttgtcagcaatcgccagcgcacaagctactgggttggacggcaggtcatcaccagcaaaacgcggctgatactgctcattcagcgccaccgcgacatcttccgcttcgccatcgtgacgcgcatagtgcatccccataacgccctgggtgtcggtgaactcgaagaccatgttggtcatcaggtcgcacttagacagcagacccgcacgggtagcgtggttaacgtcagcgccaatctgttcagcaatccagccagccagcgcctggatgcggtcagttttgtcgcgcagcgtccccaactgttgctggaacaacacggtttgcaggcgcggcaggttatcttcaagacgttttttacggtcggtgttgaagaagaactcggcatccgccagacgcggacgaacgactttctcgttaccggagataatctgctgcggatctttcgattcgatgttggcaacgaagataaagttcggcagcagtttgccgtcgttcgcatacaccgggaagtatttctggtcacctttcatggtgtaaaccagcgcttcagccggcaccgcgaggaatttctcttcgaattttgcggtcagaacgaccggccactccaccagcgaagccacttcttccagcaggctttcgcttaagtcagcgttaccgccaatcttacgcgctgcttcttcggcatcggctttaatcttcgccttacgttcttcgtaatcggcgatgactttcccacgctcacgcagaatttccggatactgatcggcgttatcgatggtgaattccggctcgcccataaagcggtggccgcgaatcacgcgatcggactgaatgcccagaatggttgccggaatgactttgtcgcccagcagcagggtcacggtgtgcaccggacgcacgaagtgcacgtcgcttgcgccccaacgcatcagtttcgggatcggcagtttcgccagagaagtcgcaaccatattcggcagcagtgcttcggtgctttcgcccttcacatgggcgcgatacagcagccattcgcctttatcggtagtcagacgctcagcctggtcaacggtaataccgcaaccacgcgcccaaccttctgccgctttgctcggtttgccttcagcgtcgaacgcctgggcaatcgccgggccgcgtttttcgatttcacgatccggttgcgcttccgccaggttagctactttcagcgccagacgacgcggagcagcaaaccattgaacggtgccgtgtgcgaggccagcgttatccagctccgcagtaaagttcgcagcaaaggactcagccaggctgcgcagtgcttttggtggcagctcttcagtgccgatttccaccagaaaagttttctcagacatagccgcctcttacttatctttgttgcacatcgggaagccgagggcttcacgggaagcgtagtatgcttctgccactgctttggtcagggtgcgaatgcgcagaatgtagcgctgacgctcggtgacggagatggctttacgcgcatccagcaggttgaagctgtgggcggctttcagaatacgctcgtaggctggcagcggcagcggattttccagcgccagcagctgctgcgcttctttctcgtactgctcgaagcaggtgaacaggaagtccacatccgcgtattcgaagttgtaagtggactgctccacttcgttctgatggaacacgtcgccgtaggtggttttacccagcgggccgtcgctccagaccaggtcgtaaacgctgtctacgccctgaatgtacatggccagacgttccagaccgtaggtgatctcgccggtaaccggtttacactccagaccaccaacctgctggaagtaagtgaactgcgtcacttccatgccgttcagccacacttcccagcccagtccccaggcacccagcgtcgggttttcccagttatcttccacgaaacggatgtcgtgaatagtcgggtccatgcccagctctttcagagaaccgaggtacagctcctgaatattgtccggcgatggcttaatgaccacctggaactgatagtagtgctgtaaacggttggggttttcgccgtagcgaccatcggtcgggcgacgagaaggctgaacataagcagccgccatcggttctggccccagctcgcgcagacaggtcattgggtgagaggttcccgcgccgacttccatgtccaatggttgaacaatggtgcagccctggcgagcccagtaatcctgtaaggtcaggatcaagccctggaaggtcctggtatcaaacttttgcatattatttcgtgctggatacgtgtggatttaaaggaagggatcagtatacccgctggatggaagatatacagtacgaaacgggaaaaagcagggcttaacgcatggaaagatgcaaaaaatggccatccgcgtcaaaagaacagacaaactgctctttacggaaggtataaccgcgcatttcatagcttccctggaactgttcgaaggcggtgacgtcgattttttgctcgccggtgttataacgttttgccgcctgatccttgcataacgcttccatattcaacgaacgcagaggatcaacctttacccgttgtgctttctgcacgggtgacggtatagaacaacccactagcaccataagcgccattgccggaaagaaagcgttcatcatcattaaattaccgtctggtttgcaggtgagtcttattatttatatcggtatagtggctgatatcttacgaatttccttaagcctctataagctgtagtgataaaactcagattattccagtgcgccaaccaaatgatttatcggtcagactttttttaaccagatacagagacacagatgcagcccaaaatttactggattgataacctgcgagggatagcgtgtttaatggtggtgatgattcacaccactacctggtatgtgaccaatgctcatagtgttagccccgtcacatgggatatcgccaatgttctgaattctgcctctcgtgtcagcgtgccgctatttttcatgatttccggctatctcttttttggcgaacgcagcgcccagccgcgccatttcttgcgtatcggcttatgtctgattttttatagcgcaatcgcactgctctacattgcgctgtttacctccatcaatatggagttagcgctgaaaaacctgctgcaaaagccagtgttttaccacttgtggtttttcttcgcgattgcggtgatttatctggtttcaccgctgattcaggtgaagaacgtcggcggaaaaatgttgctggtgctaatggcggtgattggcattatcgctaacccaaacacagtgccgcagaaaattgacggttttgaatggctgccaattaacttatatatcaatggcgatactttttactacattctgtatggcatgttgggccgcgctatagggatgatggacacacagcataaagcactgtcgtgggtgagcgccgcgctgtttgcgacgggggtttttattatctctcgcgggacattatatgaattgcagtggcgcggaaattttgccgatacctggtatctttactgtgggccgatggtttttatctgcgcaatcgcgctattgactctggttaaaaacacgctggatacgcgtaccattcgcggacttggcttaatctcccgccattcattgggtatatacggattccacgccttgattatccatgcgctgcgcacccggggaattgagcttaaaaattggccaatactggatattatttggatcttttgcgcgacgttggcagcgagtttgttactttctatgctggtacaacgaatcgacagaaacagattagtgagttaagtaaaagcccggtcacattggactgaccgggcttacgtgagttattcgctgtattcttcctgggtaacctgtgtttcttttggtgggtttattccggcatcacgaatatttttctgcaccgctactgcaccaaacaagcttaagaagaaagccagtccataaaaacctttttcgctgagtaataatgtcgcattccacagacctaccatcagtaatgcaacagagataataaagacagtcaggcaggtcatataataaatggaagtggtcggtatgccttcatacttgtcccgaacggtcttttgataagacgccgcagaaaacagtcctaataccagtacggcaaaataatatcctttttcatttaactgcatctctgcattccatagccctaacagataggtaacgataccaccaacgagagctatccatgacacaatactaaaggccggtgaataggttgatattttgttgtccatcacagtattcctttcattcctgaatatgtaagagctttatgttgctcatgccgagcgaaacaaacgcatttgaccaaacaagcagacaaaaaaggcgatgggatagatcaccatttcataagtattgataggtgcgtttaaaacaccgataaacaagagaccgatagtgattaacgcaactaactggcagatatgggtaaaaaaatcatccagttgcccgagtttttctgcgcgaagatatgcatagttgccaaaagttgctgtcattaacacgccaagaaaatagccttttccacttaacaatgggcatgagatccatagcccaaccagataaaccagcgccccgacaacaaataatagttttgccacagtctttgaggttttcataacgatctccatatctaccagcgatacattacgagtaaccaacgaaagacaaaactgaaaaatgccattaacaaatgattttcagaataaattcatactaaatattaattaattactgagatatatagatgtgaattatcccccacccggtcaggcaggggataacgtttacgccattaatggcagaagttgctgatagaggcgacggaacgtttctcgtcgtggctgataagcggcataacgctgcgcatctggtagatgcgactgttctaacggtagttgcggcaacaattcaatgagcgatttctctggattcgccgcgatctgcgccagccttgctgcgcccagtgctggccccacatccccccccgtacggtaatcgagctgctgaccgctgatatccgccagcatctgacgccagtactcactacgcgccccgcccccaatcaacgtaacactttgcggtttaataccgcaggcatgcacgacatccatgccatctgccagcgcataacccacgccttccagcactgctcgcgccagttcattggggccatgttgatgagtcaaaccaaagaaaacccccttcgcctggggattattgtgtggcgtacgctcgccggaaagataaggcagaaaccaaactggctcggcactttcatcagcctgttgagctgcagcgattaaagctgggacattgctcaggccggttaatttcgcggcccaatccagacacgacgctgcactcagcatcacagacattaaatgccaacgttgcggtagcgcatggcaaaagctatgtacggcgctttctggcttgcttaagaacccttcgctgacagcaaaatagacccccgacgtccccagcgataacattgcctgattagcatcaaccattcccacaccaactgcaccagctgcattgtcgccaccgcctgcgacaactggcaccgtcgccataccccacgctttcgcaacttcaggtaacaaagcaccagtaatttcgctgccttcgtataatgcgggcatctggtcacgagataagtcgcaagcctgcagcatgacgtcactccagtcacgctttgcgacatccagccacatggtgccagctgcgtcagacatatcgctggcaaactcccccgtcatacgcagacgcaagtaatctttcggtaataatactttgtcgatttgacggaatatctccggctcatgccgctgaacccatagcaatttaggcgcagtaaatccgggcatcatcaggttgccggtaatcacccgcgattgcggaactcgcgcttccagcaaagtgcactcttgcgcacagcgcccgtcgttccacaaaatggcagggcgtaacacccgttgctgagcatccagcaaggttgctccgtgcatctggccggcaatacccaatgctttaacgtcctgcagagaatgctgatcgcccagagctttcattgcgcgatcagttgcctgccaccactgttccgggtcttgttccgaccagagtggatgcgggcgcgaaacggtcagcttttccgtttgcgcagcaaccacctcaccctgctcgttgagcaaaataacttttacgcccgaggtgccaagatctatcccgatatacatatcgatcgttccttaaaaaaatgcccggtatcgctaccgataaccgggccaacggactgcacagttagccgttatttgtcgaacagataatggtttaccagattttccagttgttcctggcgaccactctgatgcaccggagacaaatgatgttcctgagcatatttggctaaatctgccagtgacatttggcctttcaggatttgctggcccaattcgctattccagccggaataacgctgcgcgatgcgtttatccagctcgccatcttcaatcatgcgcgctgcaattttcagcgccagtgccatcgtatccatcgcgccgatatgaccgtaaaacagatcatatttatcagtactttgacgacgtactttggcatcgaagttcagaccaccggtggtgaaaccgcctgctttgagaatttcatacatcaccagcgcattctcttccacactgttcgggaactggtcggtgtcccagcccagttgcgcatcgccacggttggcgtcgacagaaccgaacaggccaagcgcaatggcggtggctatttcatgatggaaagagtgacctgccagcgtcgcgtggttagcttcaatgttcagtttaatctctttttccagaccaaactgtttcaggaagccatagaccgtcgcggcatcgtaatcatattgatgtttggtcggttcttgcggtttcggttcgataagcaacgtgccctggaaaccgattttatgtttatgctcaaccaccatctgcataaagcggcccagttgttcacgctcctgacgcaagtcggtatttaacagcgtttcgtaaccttcacgaccgccccacaggacatagttttcaccgcccaatttatgggttgcttccatcgctgtaacaacttgcgttgccgcccagctgaagacttcaggatctgggttcgtcgccgcacccgcgccgtagcgagggtttgtaaagcagttggccgttccccacagcagcttcacgccgctctcttcttgcttgcctgccaggacatcaaccatttgcgcaaaattattgatgtactcttttaacgacgcgccctcaggggaaacatccacatcgtggaagcaataaaatggcacatgtaacttgtggaaaaactcaaatgcgacatctgctttacgcttcgccaacgccagtgcctcaccaggctgctgccacggacgattaaacgcccccacaccaaacatatccgccccgttccagcagaaggtgtgccagtagcaggcggcaaaacgcaagtgctcttccatacgcttacccaacaccagttcgtcgggattgtagtgacggaatgctaacgggtttgaggattttgagccttcataacgaacgcgatcgagctggtcaaaataggcttgcatattgaactccataatcaggtaatgccgcgggtgatggatgatgtcgtaatattgggcactccctttcagttgctcaattatgttatttcacactgctattgagataattcacaagtgtgcgctcgctcgcaaaataaaatggaatgatgaaactgggtaattcctcgaagagaaaaatgcaataagtacaattgcgcaacaaaagtaagatctcggtcataaatcaagaaataaaccaaaaatcgtaatcgaaagataaaaatctgtaattgttttcccctgtttagttgctaaaaattggttacgtttatcgcggtgattgttacttattaaaactgtcctctaactacagaaggccctacaccatgaaaataaagaacattctactcaccctttgcacctcactcctgcttaccaacgttgctgcacacgccaaagaagtcaaaataggtatggcgattgatgatctccgtcttgaacgctggcaaaaagatcgagatatctttgtgaaaaaggcagaatctctcggcgcgaaagtatttgtacagtctgcaaatggcaatgaagaaacacaaatgtcgcagattgaaaacatgataaaccggggtgtcgatgttcttgtcattattccgtataacggtcaggtattaagtaacgttgtaaaagaagccaaacaagaaggcattaaagtattagcttacgaccgtatgattaacgatgcggatatcgatttttatatttctttcgataacgaaaaagtcggtgaactgcaggcaaaagccctggtcgatattgttccgcaaggtaattacttcctgatgggcggctcgccggtagataacaacgccaagctgttccgcgccggacaaatgaaagtgttaaaaccttacgttgattccggaaaaattaaagtcgttggtgaccaatgggttgatggctggttaccggaaaacgcattgaaaattatggaaaacgcgctaaccgccaataataacaaaattgatgctgtagttgcctcaaacgatgccaccgcaggtggggcaattcaggcattaagcgcgcaaggtttatcagggaaagtagcaatctccggccaggatgcggatctcgcaggtattaaacgtattgctgccggtacgcaaactatgacggtgtataaacctattacgttgttggcaaatactgccgcagaaattgccgttgagttgggcaatggtcaggaaccaaaagcagataccacactgaataatggcctgaaagatgtcccctcccgcctcctgacaccgatcgatgtgaataaaaacaacatcaaagatacggtaattaaagacggattccacaaagagagcgagctgtaagcgttacgccccagcgcggagcgggggcgtgatttctctccatgccgcgtgaatgaattggcttaggtggagtcgttatgccttatctacttgaaatgaagaacattaccaaaaccttcggcagtgtgaaggcgattgataacgtctgcttgcggttgaatgctggcgaaatcgtctcactttgtggggaaaatgggtctggtaaatcaacgctgatgaaagtgctgtgtggtatttatccccatggctcctacgaaggcgaaattatttttgcgggagaagagattcaggcgagtcacatccgcgataccgaacgcaaaggtatcgccatcattcatcaggaattggccctggtgaaagaattgaccgtgctggaaaatatcttcctgggtaacgaaataacccacaatggcattatggattatgacctgatgacgctacgctgtcagaagctgctcgcacaggtcagtttatccatttcacctgatacccgcgttggcgatttagggcttgggcaacaacaactggttgaaattgccaaggcacttaataaacaggtgcgcttgttaattctcgatgaaccgacagcctcattaactgagcaggaaacgtcgattttactggatattattcgcgatctacaacagcacggtatcgcctgtatttatatttcgcacaaactcaacgaagtcaaagcgatttccgatacgatttgcgttattcgcgacggacagcacattggtacgcgtgatgctgccggaatgagtgaagacgatattatcaccatgatggtcgggcgagagttaaccgcgctttaccctaatgaaccacataccaccggagatgaaatattacgtattgaacatctgacggcatggcatccggttaatcgtcatattaaacgagttaatgatgtctcgttttccctgaaacgtggcgaaatattgggtattgccggactcgttggtgccggacgtaccgagaccattcagtgcctgtttggtgtgtggcccggacaatgggaaggaaaaatttatattgatggcaaacaggtagatattcgtaactgtcagcaagccatcgcccaggggattgcgatggtccccgaagacagaaagcgcgacggcatcgttccggtaatggcggttggtaaaaatattaccctcgccgcactcaataaatttaccggtggcattagccagcttgatgacgcggcagagcaaaaatgtattctggaatcaatccagcaactcaaagttaaaacgtcgtcccccgaccttgctattggacgtttgagcggcggcaatcagcaaaaagcgatcctcgctcgctgtctgttacttaacccgcgcattctcattcttgatgaacccaccaggggtatcgatattggcgcgaaatacgagatctacaaattaattaaccaactcgtccagcagggtattgccgttattgtcatctcttccgaattacctgaagtgctcggccttagcgatcgtgtactggtgatgcatgaagggaaactaaaagccaacctgataaatcataacctgactcaggagcaggtgatggaagccgcattgaggagcgaacatcatgtcgaaaagcaatccgtctgaagtgaaattggccgtaccgacatccggtggcttctccgggctgaaatcactgaatttgcaggtcttcgtgatgattgcagctatcatcgcaatcatgctgttctttacctggaccaccgatggtgcctacttaagcgcccgtaacgtctccaacctgttacgccagaccgcgattaccggcatcctcgcggtaggaatggtgttcgtcataatttctgctgaaatcgacctttccgtcggctcaatgatggggctgttaggtggcgtcgcggcgatttgtgacgtctggttaggctggcctttgccacttaccatcattgtgacgctggttctgggactgcttctcggtgcctggaacggatggtgggtcgcgtaccgtaaagtcccttcatttattgtcaccctcgcgggcatgttggcatttcgcggcatactcattggcatcaccaacggcacgactgtatcccccaccagcgccgcgatgtcacaaattgggcaaagctatctccccgccagtaccggcttcatcattggcgcgcttggcttaatggcttttgttggttggcaatggcgcggaagaatgcgccgtcaggctttgggtttacagtctccggcctctaccgcagtagtcggtcgccaggctttaaccgctatcatcgtattaggcgcaatctggctgttgaatgattaccgtggcgttcccactcctgttctgctgctgacgttgctgttactcggcggaatgtttatggcaacgcggacggcatttggacgacgcatttatgccatcggcggcaatctggaagcagcacgtctctccgggattaacgttgaacgcaccaaacttgccgtgttcgcgattaacggattaatggtagccatcgccggattaatccttagttctcgacttggcgctggttcaccttctgcgggaaatatcgccgaactggacgcaattgcagcatgcgtgattggcggcaccagcctggctggcggtgtgggaagcgttgccggagcagtaatgggggcatttatcatggcttcactggataacggcatgagtatgatggatgtaccgaccttctggcagtatatcgttaaaggtgcgattctgttgctggcagtatggatggactccgcaaccaaacgccgttcttgattttgataaaaattttctcaaagccggttacgtattaccggttttgagtttttgcatgattcagcaggaaaagaaccatgtttactaaacgtcaccgcatcacattactgttcaatgccaataaagcctatgaccggcaggtagtagaaggcgtaggggaatatttacaggcgtcacaatcggaatgggatattttcattgaagaagatttccgcgcccgcattgataaaatcaaggactggttaggagatggcgtcattgccgacttcgacgacaaacagatcgagcaagcgctggctgatgtcgacgtccccattgttggggttggcggctcgtatcaccttgcagaaagttacccacccgttcattacattgccaccgataactatgcgctggttgaaagcgcatttttgcatttaaaagagaaaggcgttaaccgctttgctttttatggtcttccggaatcaagcggcaaacgttgggccactgagcgcgaatatgcatttcgtcagcttgtcgccgaagaaaagtatcgcggagtggtttatcaggggttagaaaccgcgccagagaactggcaacacgcgcaaaatcggctggcagactggctacaaacgctaccaccgcaaaccgggattattgccgttactgacgcccgagcgcggcatattctgcaagtatgtgaacatctacatattcccgtaccggaaaaattatgcgtgattggcatcgataacgaagaactgacccgctatctgtcgcgtgtcgccctttcttcggtcgctcagggcgcgcggcaaatgggctatcaggcggcaaaactgttgcatcgattattagataaagaagaaatgccgctacagcgaattttggtcccaccagttcgcgtcattgaacggcgctcaacagattatcgctcgctgaccgatcccgccgttattcaggccatgcattacattcgtaatcacgcctgtaaagggattaaagtggatcaggtactggatgcggtcgggatctcgcgctccaatcttgagaagcgttttaaagaagaggtgggtgaaaccatccatgccatgattcatgccgagaagctggagaaagcgcgcagtctgctgatttcaaccaccttgtcgatcaatgagatatcgcaaatgtgcggttatccatcgctgcaatatttctactctgtttttaaaaaagcatatgacacgacgccaaaagagtatcgcgatgtaaatagcgaggtcatgttgtagcgatgatgagaattgtcggcgtcacatcaggtaacgctgcgtggttgtcggatgcggcgtgaacgccttatccgacctacccgccaggcatgataaaacgcaccaacaacgcttcaggctcgtagctcaactgcctgagacaaagtaaaaagccttatccgactgacaagtcggataaggctcaaggaaatgcaattacatatgcgccgcgattaaccgttggttatcctggtacattgcgaacaggtagttgttataactcttccctttggtcgagtagcccttcagcttgtgaatcatcgctgtggcagtcacttcctgatccgctttacgcagctgcgcacgcgatttacggaacgaagagtaagccgggtgcgtattcaggttagtgacataggcgctcaccgattctttgacagaactaaactgtgagtaccctttcactttacctggcgcattggtacaacgtcctttcatgcatttcatgccgaacaggttgttgttgttgcgcgccagcttcgacgttccccaaccgctttctgctgcagccatcgtcgccaccatactggtggggataatgtctacgcgttcaagcaaggtattccacgggatttttcgcgtattaccggaccacttcaccttgtagcgtttggcgatgtctttcagacgcgcacgctcagcaggtgaccattggccctgatactgttttgaaatgagccagttacgttccgcagtaatggccgcattttggctggtaatgtaaggcattacggtccggagaaacgcctttttccttggtgttccggaagggtattttcgcaaatcaggaagtgaactactctttgcactattgcgagaatactcttgtttactgcttacctgtttattactagctttagttaagtgggacttttgactcgctgttgttgtgtgcgtcttcgctaacacctcactcgaaaacaccagagtgagtaacataagaatcatcgccccatatcgtcgtatgggagtcaaaatcatcaggtctcctggtcggatttaatcattccaacaccttatatttttcacaaatttgagagttgaatctcaaatcatatcaaaaatagctgtcaagagcaccccaaggaatagtccaaatctgaaactatgtcacgtgttaacgattcagattggcgctaaatcgcagaaaatgtgggggttatcgcaaaattcagccgttttttgcgcgagatcgctcacccttgcttctcatcctgtggacttaccgctcagggatgagttttgtttggcttatcgctggcaaactgtctgaaatcgcagcaataaggactcatccgccatgaaactcgccgcctgttttctgacactccttcctggcttcgccgttgccgccagctggacttctccggggtttcccgcctttagcgaacaggggacaggaacatttgtcagccacgcgcagttgcccaaaggtacgcgtccactaacgctaaattttgaccaacagtgctggcagcctgcggatgcgataaaactcaatcagatgctttccctgcaaccttgtagcaacacgccgcctcaatggcgattgttcagggacggcgaatatacgctgcaaatagacacccgctccggtacgccaacattgatgatttccatccagaacgccgccgaaccggtagcaagcctggtccgtgaatgcccgaaatgggatggattaccgctcacagtggatgtcagcgccactttcccggaaggagccgccgtacgggattattacagccagcaaattgcgatagtgaagaacggtcaaataatgttacaacccgctgccaccagcaacggtttactcctgctggaacgggcagaaactgacacatccgcccctttcgactggcataacgccacggtttactttgtgctgacagatcgtttcgaaaacggcgatcccagtaatgaccagagttacggacgtcataaagacggtatggcggaaattggcacttttcacggcggcgatttacgcggcctgaccaacaaactggattacctccagcagttgggcgttaatgctttatggataagcgccccatttgagcaaattcacggctgggtcggcggcggtacaaaaggcgatttcccgcattatgcctaccacggttattacacacaggactggacgaatcttgatgccaatatgggcaacgaagccgatctacggacgctggttgatagcgcacatcagcgcggtattcgtattctctttgatgtcgtgatgaaccacaccggctatgccacgctggcggatatgcaggagtatcagtttggcgcgttatatctttctggtgacgaagtgaaaaaatcgctgggtgaacgctggagcgactggaaacctgccgccgggcaaacctggcatagctttaacgattacattaatttcagcgacaaaacaggctgggataaatggtggggaaaaaactggatcagaacggatatcggcgattacgacaatcctggattcgacgatctcactatgtcgctagcctttttgccggatatcaaaaccgaatcaactaccgcttctggtctgccggtgttctataaaaacaaaatggatacccacgccaaagccattgacggctatacgccgcgcgattacttaacccactggttaagtcagtgggtccgcgactatgggattgatggttttcgggtcgataccgccaaacatgttgagttgcccgcctggcagcaactgaaaaccgaagccagcgccgcgcttcgcgaatggaaaaaagctaaccccgacaaagcattagatgacaaacctttctggatgaccggtgaagcctggggccacggcgtgatgcaaagtgactactatcgccacggcttcgatgcgatgatcaatttcgattatcaggagcaggcggcgaaagcagtcgactgtctggcgcagatggatacgacctggcagcaaatggcggagaaattgcagggtttcaacgtgttgagctacctctcgtcgcatgatacccgcctgttccgtgaagggggcgacaaagcagcagagttattactattagcgccaggcgcggtacaaatcttttatggtgatgaatcctcgcgtccgttcggtcctacaggttctgatccgctgcaaggtacacgttcggatatgaactggcaggatgttagcggtaaatctgccgccagcgtcgcgcactggcagaaaatcagccagttccgcgcccgccatcccgcaattggcgcgggcaaacaaacgacacttttgctgaagcagggctacggctttgttcgtgagcatggcgacgataaagtgctggtcgtctgggcagggcaacagtaacttttccggcttcccgttcgtcagtacctcgggaagccgccaaccaggataaaatgtcagccctaatcagcgttgcaggataaagcaccgctcactcttcaacagaccgatttgcaccccagcaaatgtagcgttattgttaccttccttgctacagagttcgacagatatcccgctatgacattctccctttttggtgacaaatttacccgccactccggcattacgctgttgatggaagatctgaacgacggtttacgcacgcctggcgcgattatgctcggcggcggtaatccggcgcagatcccggaaatgcaggactacttccagacgctactgaccgacatgctggaaagtggcaaagcgactgatgcactgtgtaactacgacggtccacaggggaaaacggagctactcacactgcttgccggaatgctgcgcgagaagttgggttgggatatcgaaccacagaatattgcactaacaaacggcagccagagcgcgtttttctacttatttaacctgtttgccggacgccgtgccgatggtcgggtcaaaaaagtgctgttcccgcttgcaccggaatacattggctatgctgacgccggactggaagaagatctgtttgtctctgcgcgtccgaatattgaactgctgccggaaggccagtttaaataccacgtcgattttgagcatctgcatattggcgaagaaaccgggatgatttgcgtctcccggccgacgaatccaacaggcaatgtgattactgacgaagagttgctgaagcttgacgcgctggcgaatcaacacggcattccgctggtgattgataacgcttatggcgtcccgttcccgggtatcatcttcagtgaagcgcgcccgctatggaatccgaatatcgtgctgtgcatgagtctttccaagctgggtctacctggctcccgctgcggcattatcatcgccaatgaaaaaatcatcaccgccatcaccaatatgaacggcattatcagcctggcacctggcggtattggtccggcgatgatgtgtgaaatgattaagcgtaacgatctgctgcgcctgtctgaaacagtcatcaaaccgttttactaccagcgtgttcaggaaactatcgccatcattcgccgctatttaccggaaaatcgctgcctgattcataaaccggaaggagccattttcctctggctatggtttaaggatttgcccattacgaccaagcagctctatcagcgcctgaaagcacgcggcgtgctgatggtgccggggcacaacttcttcccagggctggataaaccgtggccgcatacgcatcaatgtatgcgcatgaactacgtaccagagccggagaaaattgaggcgggggtgaagattctggcggaagagatagaaagagcctgggctgaaagtcactaaaaattgcctgatgcgctacgcttatcaggcctacatgatttctgcaatatattgaatttggaagaatttgtaggccggataaggcgtttacgccgcatctggcataaacaaagcgcactgttccggcgttgagaaacgccggaaaacgtttcaaacaggctgctgccgtagccgatgccgctgcactttctcgacatccatgcactgcaacgcctttgtcgggcaggcttcaacacaggccggtcccgtctcccgatgccagcacagatcgcacttaatcgccctcgcctttttgcgcgaagaaacgacctccatcgcaccaaacgggcaagccagcatacagcttttacagccaatgcaacgtgtttgttcaacgaaaatatgcccatgttcgcggcttatcgcgtcaacagggcagacattcgcgcacggtgcatcttcacactgatgacaggctactgccgtggtccagcagtggtctttaatgacacgaatacgggaaataaactcgtctggtgacaacgcagcgcaatcctgattctcatgatgcgacactgcgcaagccacttcacaggtacggcaaccgatacatttcgtcgcatccgcaataataaaccggttcatgatcactcctttgcactaaaacagcagagtgccagagagcgcgtccctactgctttgatccaacgaaggaaatgttaaagttttggcacttgtccaaagcgttatgtgatcgcgcccaggtcatccctgacagtaaatcccagttcattagaaatagcctgcgcggtttcacgcagtggtttcaggagatttttctctcccacctgtttcagacgtgatgtcgaaagcgaaatcgacacggcgtacggcacccgcccatgaatatcaaacaccggaacagcaatacaggagacgccgagttcgttttcttctctgtccatcgccgctccgctttcacgaatgtgcgccagttcgtcgaacatcgcgggcagctcggtaatggtattgcgggttaacggctggatctcatgctgatggctttcccagtatgacttcacgtagtccgggtgaccaaacgccatgtagatcttgcccattgcggaacagtagagcggcatatgctggccaatataggcacgggttcgcagcatcccggttgtgggttccagcttataaatcaaaatagcgtgatcgtcttcgcggctggagaagttaatggtttcaccagtggcgatgttcagtgcctcaagatgcggagcggcgatatgaatgatattcagcgaagacagcgccttctgcccgacggcaataaatttggtggtcaggcgataactccctgcggcaggcgcggtggtcacatagccgcaggactgtaatccctgcaataagcgatggacggtactcttatttaaaccagccagctccgaaagatgcgccaacggacaaccgtttggatagttgctcaaaatctcaatcagcatcaacccgcgaaacagactctggcttccggctggacgctctttttcctgcgccatctcgttctctttttttcccatcacttctttccccattttgtcgcgtcctgatggtagcgcaaagtgtgccgtagttcacgatctcgacagataatttataaccaattgatttttatgtcttttgaaattcatcaatcagattgccttgttaaaaagtgatcgatatatttgaaatcaagtttcgcatattgaaattttaagccaaaaaagcgatcaaaaaaacaaggaagcctgggatgaaagtgacatttgagcagttaaaagcagcctttaatcgggtcttaatttcacgcggcgttgacagcgaaacggctgacgcctgtgcagagatgttcgcccgcaccaccgaatccggcgtttattctcacggcgttaatcgtttccctcgtttcattcaacaactggaaaacggcgatatcattcctgatgcccaacccaaacgtataaccagcctcggcgcaattgaacagtgggacgcccagcgttcgatcggtaacctgacagcgaaaaagatgatggatcgcgccattgaactggctgccgatcacggtattggtctggtggcactacgtaatgccaaccactggatgcgcggcggcagctacggctggcaggcggcggaaaaaggctatattggcatttgctggaccaactccatcgccgtaatgccgccgtggggcgcaaaagagtgtcgcataggcactaacccgctgatcgtcgccattccttccacgccgatcaccatggtcgatatgtcgatgtcgatgttctcttacggcatgttagaagttaaccgtctggcaggtcgtcagctcccggtcgatggtggctttgatgatgagggcaatttgaccaaagaacctggcgttatcgagaagaatcgccgcattttgccgatgggctactggaaaggttctggcatgtcgattgtgctggatatgatcgctactctcctttccgacggcgcatccgttgccgaagtcacccaggacaacagcgacgaatacggcatttcacaaatttttattgccattgaagtggacaagcttatcgacggtcccacccgcgatgccaagctgcaacgcatcatggattacgttactagtgccgagcgtgctgacgaaaatcaggccattcgcttacccggccatgaatttactaccctgctggccgaaaaccgccgtaacggcatcactgttgatgacagcgtgtgggccaaaatccaggcgttatgaggagataagtcatgatttttggacatatcgcgcagcccaatccgtgccgtttgcccgccgccattgaaaaggcgctcgattttctgcgcgctaccgatttcaacgccctggagccgggcgttgtcgaaatcgacggcaaaaatatttatacgcaaattatcgatttaaccacacgcgaagcggtggtaaaccgtccggaagtgcatcgtcggtatatcgatattcagtttctggcgtggggcgaagagaaaatcggcattgctattgatacgggaaataataaagtcagcgaatcactattagagcagcgcaatattattttttatcacgacagtgaacatgaatcatttatagaaatgataccgggcagctacgcaattttctttccgcaggatgttcaccgaccaggttgtattatgcaaacagcctctgagatacgaaaaattgtggttaaagtcgcattaacggcgctgaattaatcgaataatcgtctacgccagaacgcctgggtaatgttattgctctaactatattaataattcaggttgctgcacatgcgacttgaattatgacagacatagcctcaaggaatagctatgaaaaaaatactcgaagcaatactggcgattaatctcgccgtactttcctgtattgtatttataaacattattttaagatatggttttcagacaagcattttatctgttgatgaattgtcacgttatttatttgtctggttaacgtttattggcgcgattgtagcttttatggataacgcccacgttcaggtcacctttctggtggagaaactctcccccgcatggcagcgacgagtcgctctggttacccattccttaatcttatttatttgtggcgcactggcctggggcgcaacgctaaaaacaattcaggactggagcgattattcaccgatcctcggtttacccatcggcctgatgtatgccgcttgtctgcccaccagcctcgttatcgcattctttgaactgcgtcatttatatcaactcatcacgcgtagcaattctctaacgtcgccaccgcaaggagcttaatcatggctgtgctgatttttctgggctgtctgttgggtggtattgctatcggtttgcctattgcctgggcactgttgttgtgcggggcggcgttaatgttctggctggacatgtttgatgtccagatcatggcacaaacgctggtgaacggagccgatagcttctccctgctggcgattccgttctttgtgctggcgggtgaaatcatgaatgcgggcggcttgtcaaaacgcattgttgacctgccgatgaaactggtggggcataaaccaggcgggctgggctacgtcggcgtgctggcagctatgattatggcgagcctttctggttctgccgttgcggataccgccgccgttgccgctctactggtgccgatgatgcgcagcgccaactatccggtcaaccgggcggcggggctgattgcctctggcggcattatcgcgccaattattcccccttccattccgtttattatcttcggcgtttccagcggattatccatcagtaagctgtttatggcgggcattgcccctggcatgatgatgggcgcaacgctgatgcttacctggtggtggcaggccagtcgccttaatttaccccgccagcaaaaagcaacgatgcaggaaatctggcactcttttgtctccggtatctgggcgctgtttcttccagtcatcattattggcgggtttcgctccggcctgtttacccctaccgaagccggggccgttgctgctttctatgcgctgtttgtcgccacagttatttaccgtgaaatgaccttcgccacactttggcatgtactcattggcgcggcgaaaaccacctcagtggttatgtttctggtggcctcggcacaagtttccgcctggctgattaccattgctgaactgccgatgatggtttctgatttactgcaaccgttggtcgattcaccgcgtctgctgtttatcgtcattatggtggctatcctgattgtcggcatggtcatggatttaacgccgacggtattaattcttaccccggtattaatgcctttagttaaagaggcaggaatcgatccgatttatttcggtgtcatgtttatcattaactgctcaatcggcttaattacaccgcctatcggtaatgtacttaacgttatttcaggggtggcaaaactcaaattcgatgatgcagtcagaggcgttttcccttacgtcctggttttatattcattattagtcgtatttgtttttattcccgatctcatcatcctccctttgaaatggattaattaaaaggaaaatattatgaaattacgctctgtaacctacgcattattcattgctggcctggctgcattcagcacatcttctctggcggcacaatctttacgtttcggttatgaaacatcacaaaccgactcgcaacatattgcggcgaaaaaattcaatgatttattgcaggagagaaccaaaggcgagctgaaattaaaactgttcccggacagcactctcggtaacgcgcaggcgatgatcagcggcgtacgtggcggcaccatcgatatggaaatgtccggctcgaataactttgccgggttatcaccagtgatgaacttgcttgatgtccctttcctgttccgcgataccgctcacgcgcataaaacgctcgacggcaaagtcggtgatgatctgaaagcctcacttgaaggtaaaggactgaaagtactggcctactgggaaaacggctggcgcgatgtcaccaactcgcgcgcaccggttaaaacccccgccgacctgaaagggctgaaaatccgcaccaacaatagcccgatgaatatcgccgcattcaaagtctttggcgctaacccgatcccgatgccgtttgccgaagtctataccgggctggaaacccgcactatcgacgctcaggaacacccgatcaacgtcgtctggtcagcaaaatttttcgaagtgcagaagttcctttctctgacgcaccacgcctattccccgcttctggtggtgatcaacaaagcgaagtttgatggcttaagtccggagttccagcaggcgctagtttcatctgcacaagaagcgggtaactatcagcgcaaactggttgctgaagatcagcaaaaaatcatcgacggcatgaaagaagcgggcgtggaagtcatcaccgatctcgaccgcaaagcctttagcgacgcactggggaatcaggttcgcgacatgtttgttaaagatgtgccgcagggagctgatctgctgaaagccgtggatgaggtgcaataaaccatgacgcaatactggctggggttagattgtggcggtagctggctgaaagccgggctgtatgaccgcgaaggccgggaggcaggcgtgcagcgcctgccgctgtgcgcattaagcccgcagccaggctgggcagagcgcgatatggcagaactgtggcaatgctgcatggctgtcattcgcgccctgcttactcattctggtgttagcggggaacaaattgtcggtatcggcatctccgcacagggaaagggcttgtttttgctggataaaaacgacaaaccgctcgggaatgctattttgtcctcggaccgccgggcgatggaaatcgttcgtcgctggcaggaagatggcatcccggaaaaactctacccgctgacccgacaaaccttgtggaccgggcatccggtgtcgctgttacgctggctgaaagagcacgaaccagaacgctacgcgcaaattggctgcgtgatgatgacgcacgactacctgcgctggtgtttaactggcgtcaaaggctgtgaagagagcaatatttccgagtccaacctctacaacatgagtcttggggaatatgacccgtgcctcaccgactggctggggatcgctgaaatcaatcacgccctgccgcctgttgtcggatctgccgaaatctgcggggagatcaccgctcagacagccgccctgaccggtctgaaagcgggtacgcccgttgttggcggcctgtttgatgtggtttccaccgcactctgcgccgggatcgaagacgaatttaccctcaatgcggtgatggggacctgggcggtgaccagcggcataacccgcggtttacgtgacggtgaagcgcatccgtatgtctatggtcgctacgttaacgatggtgaatttatcgttcacgaagccagccctacctcttccggcaacctcgaatggtttaccgcacagtggggagaaatctcgtttgatgagatcaatcaggccgttgccagcttgccgaaggctgggggcgatctctttttcctgccgttcctgtacggcagcaacgccggactcgagatgaccagtggtttctacgggatgcaggccattcacacccgcgcgcacctgttgcaggccatctatgaaggggtggtgttcagccatatgacccacctcaaccgaatgcgcgaacgttttactgatgttcacaccctacgcgtcactggcggcccggcgcactccgatgtctggatgcaaatgctggcggacgtcagcggtctgcgtatcgagctgccgcaggtggaagaaaccggctgctttggtgcggcccttgccgcccgcgtcggcaccggggtttatcacaacttcagcgaagcccaacgtgacttgcgacacccggtgcgcaccctgctgccagatatgaccgcccatcagctttaccaaaaaaaatatcaacgttatcagcatctcattgccgcacttcagggctttcacgcccgcattaaggagcacacattatgagccgaccacttctgcaactggccctcgaccactcatcacttgaagccgcgcagcgcgacgtgacgctgttaaaagacagcgtcgatatcgtcgaagcgggcaccattctctgtttaaacgaagggcttggcgcggtgaaagccttgcgcgaacagtgcccggacaaaatcatcgttgctgactggaaggtcgccgacgctggtgaaacgctcgcgcaacaggcgtttggcgcaggcgctaactggatgaccatcatctgcgccgcgccgctcgcgacggtagaaaaaggccacgcaatggcacaacgctgcgggggtgaaattcagatagagctgttcggtaactggacgctggacgacgcccgcgactggcatcgtattggcgtgcggcaggccatttatcatcgcggtcgtgatgcacaggccagcgggcaacagtggggcgaagccgatctggcacgcatgaaggcgctttcagatatcggccttgagctttccattactggcgggattacccctgctgacctgccgctgtttaaagatatccgcgtgaaagcgtttattgccgggcgggcactggcaggcgcggcaaatccggcgcaagtggctggcgatttccatgcgcaaatcgacgctatctggggaggtgcgcgtgcgtaatcatcagttagggatttatgaaaaagcgctggcgaaagatctctcctggccggagcggctggtgctggcaaaaagctgcggttttgattttgtcgaaatgtcggtggatgaaaccgacgaacggctctcacgtcttgactggagcgccgcacaaaggacttcgctggttgccgcgatgatcgaaacaggtgttgggatcccgtcgatgtgcctgtccgcacatcgtcgctttccctttggtagccgtgacgaggcagtgcgcgaacgggcgcgggaaatcatgagtaaagcgattcgcctggcgcgcgatctcggcattcgcaccatccagctggcaggttatgacgtctattacgaagaccacgacgaaggcacccggcaacgttttgctgaagggctggcgtgggcagtcgaacaggcggcggcatcacaagtaatgctggcggtggagattatggataccgcgtttatgaactccatcagcaaatggaaaaaatgggacgagatgctcgcctcaccgtggttcaccgtctacccggacgtcggcaacctcagcgcctggggcaatgatgttcccgccgaactgaaactgggcattgaccgtatcgccgcgatccacctgaaagacacccagccagtcaccgggcaaagtcccggacagttccgcgacgtgccgtttggcgaaggctgcgtcgatttcgttggcatcttcaaaacgctgcataaactgaactatcgcggttctttcctgattgagatgtggaccgaaaaagccaaagagccggtgctggagattattcaggcgcggcgttggattgaagcgcgtatgcaggaggctggatttatatgttagagcaactgaaagccgacgtgctggcggcgaatctggcgcttcccgctcaccatctggtgacgttcacctggggcaatgtcagcgcggtagacgaaacgcggcaatggatggtaatcaaaccttccggcgtcgagtacgacgtgatgaccgccgacgatatggtggtggttgagatagccagcggtaaggtggtggaaggcagcaaaaaaccctcttccgatacaccaacgcatctggcgctctaccgtcgctatgccgaaattggcggtattgtgcatacccactcgcgccacgccaccatctggtcacaggccgggctggatctccccgcctggggcaccacccacgccgattatttttacggtgccatcccctgcacgcgacagatgaccgcagaggagattaacggcgaatatgaatatcagaccggcgaagtgatcattgaaaccttcgaagaacgtggcaggagtccggcacaaatcccggcggtgctggtgcattctcacggcccgttcgcatggggtaaaaacgccgccgatgccgtgcataacgccgtagtactcgaagaatgcgcctatatgggtctattctcgcgccagcttgcgccgcagctccctgcgatgcaaaacgaactgctggataagcactacctgcgtaagcatggggccaatgcctattacgggcagtaatccctcacgccggggcttcatcgccccggcactacgaattgatatgttccttgctgtaacgccgcttccacgctgctggcgttaaaccagtatgtttctgaaaaatctgccggaaatagccaacgtcattaaaccgtattgcatggagcaggccgacaacgtcgagtcactgcataacctgttgctgcccgccgatgcgccatttacgacatttgaaggcaagggattgttcagccataagatcctgattcagacgccaggttcccggtatgaacagagcaatccagagcaacaacctttgtggcattacgacggagcaccagccgcaccgacatccaccggtgaattaaaaacgccagctcaccccggtgacaaaggtaaaactctcattacgatcaatcatcgggctgtcggtaatctcttccggcagctcgctgtatcctgcgctcgccatcaatacgacgtgctctcctatcgggtattttgccgtcaggctgacatagggcacccaggcatcctgcgcggaataacttgccagaccgctacgacgggactcactctctgaaatgccatagtaatagtcactgaaattctcgtcataatagagaacgcccagcgcaggtgtcagcgacagacgacctatctgcattttgtggaataccgatagctcccccacccagccgttgctgttatccagaacgtccgcagctgcagaggctttcacggttccccaacgctcgtggtgataccaggcaacccccgccatagccgtactatcacgcttatcaagctgttgcatggcataatcgtcattatcggtagggtcaaattccagcggcatccaggatgcggtcaggctaagttcatttttttcactttgcgacagaataaaacctaacgtggtctgacgaacataaaaagtatcaccttcataactaatcagcggaattgccttcgtattttcattataaccgcgataaggcgattcattataagccgcaccagcaccaatggataattcagaagcagttgcgcttgccataaaaggcaacgcaaataacgccacaatattgcgattaattaacatgtccggtattccattttaaaataagataaaaaagagtcggcataataatgcttacaatttctccggtgcaagattcatatttatatagtaatatataaaattatatataattgggctgttgcgatgacaaaattacaacttaagtaccgggagttaaaaattatctcggtaatcgctgccagtgaaaatatcagccatgccgcgactgtacttggcatcgcacaggccaacgtcagcaaatatcttgctgattttgaatcaaaagtgggtttaaaagtctttgaccgaaccacccggcagctgatgctcacaccttttggcaccgcgctgttaccgtacatcaacgacatgctggacagaaacgagcaacttaataattttattgcagattataagcatgagaaacgtggtcgggtcaccatctacgccccaaccggcataattacctatttatccaaacatgtaatcgataaaattaaagatatcggtgatatcaccttatcgctaaaaacctgcaatcttgagcgtaatgccttttatgaaggcgtcgaatttcctgatgattgtgatgttttaatcagctacgctccaccaaaagatgaatcgctggttgccagttttattacccaatatgccgtaaccgcttatgccagccagcgctatcttgagaaacatcccattagccgtcctgacgaactcgaacatcactcctgtattttgatcgactcgatgatgatcgacgacgcgaatatctggcgcttcaacgtcgccgggagtaaagaggtgcgggattatcgcgtgaagggaaattacgtttgcgacaacacgcaatctgcgctggagctggcacgaaatcacctggggattgtgtttgcgccagacaaaagtgtgcagagcgacctgcaagacggcacgctggtgccctgctttcagcaaccctatgaatggtggctggatctggtggctatcttccgtaaacgggaataccagccctggcgggtccagtatgtgctggatgaaatgctgcgtgaaattcgccaccagcttgctcagtcgcagcaactgcggcctgaacaagcggcggaaagcgaagattaatgatcgagataaaggtaatgcacccagctggtcatgcgtaatagcactttgcgcatcaccgagacatggctgaaatgatcagagtaaaccgccacctgggcgtaaataccgtctggtaaagcgctcaaatcagtgtgctcatccagttcaatggtcgcgataacgccatctgaacccggcgctgtgtttaacgtctgtaaggtgccggtcgactgataagctccgccgggaacggctggactaatggctgccagcttaccgctgaataccttacctggcagagcattaaacaccacttccgcatcgtcgccaggagccagtcgcagcaaggagttctgacggaactgcgccacgatttgtcgtttctgatcgggtataaacaccatcaccggacgtagcggcagcgacgcggcataggtacccggacgaatcagtacctgggtcacataaccatcgctcggcgcacgcactatcgtctgctcaaggttatattttgcttccgcgagctgtgctttcaggctggcgatttgagaatgttcacccaacaccaggctatccagctggctctggatctgtttttgttccgccgccgatgacttcacggaggcttcctgcgccagataattttgccgcgccacatcgatatcgcgttctgaaaacgggtttactttcgcctggctgccacgtgcgtaacgctgatactctttagcgaatttatcccgcgtggcctttgcctgctgagtattcgccgccatctcatctaactctgcgcccaacgcccgctgtttatgttctgcggtaacgatatccgccatcagccgatccacccgcgcctgataacgcgtcgggtccagtcgaaatagcacctcaccttttttaatcagcgtatttttcttatccgtcacttcaatcaccacaccagtcacctgtgggacaacaggaatagaaataaccgctttttgcgctttaaaggtatacggatggttatagttcattaacagaattagaccgctgacaataaatattccacccagggccgctgtgggaatggtccatttatttacgggaattttgaagatcttaaacattgcccatgcaaaagccacataggtcaaaataatcagtaaatccataagtattactcggcagaagaggatttgatgtcggcgagctgtttctccagcccggcaatgcgctgttgcagttgcataacggatgaatcatggctttgcattccccatccccgctccgggcggtaaagcgtggcccaaatccacaaaaacggccagataacatgtaacgtaaaaagactcacccaaccagcaacatgaatggcgtcggcatgaggatgattacgttttttggcaatcaggtagggaatatcatgtaaaataatgatcccatagaagatcaccagaaatacaaaaataagcactcccagtgcaaaatagtccaggaacatatttccctcaaagaatataaaaaagaacaattaacgcatattatgaaatgccatgatgcagtgcaatttccttatttatataacgacatattgttttttatatactttcttaaatgtgctgtctggtttttcaacaggacgaggtttatcatattgaaatagtggaactattggccaaactaatgaataactccagtaaaacatccacagtacagattaagcgtattaaaccttcaattatctaccgtttattgctgattggcctcggatcaccaatggtgatttacggcctggttcgcccgctcaccatcgaaacgcgagattaaactcctgacaaaacacgccccagaaacgtacttctgttggcgtagtctgggttattgcgcacgtaggtttaaaacgtaaattgtaacaacgtgcgctttgtttatgccggatgcggcgtgtacgccttatccggcctacggtcaggttcccgtaggcatgataagacgcgtaagcgtcgcatcaggcaatgaatacccaatgcgaccagcttcttatatcagaacagccccaacggtttatccgagtagctcaccagcaggcacttggtttgctggtaatgctccagcatcatcttgtgggtttcgcgaccgatacctgattgtttgtagccaccaaacgccgcatgtgccgggtaagcgtgataacagttggtccacacgcgcccagcctgtatgccgcgccccatcttataggccagattaccgttgcggctccagacgcccgcgcccaggccatattgcgtatcgttcgccagctccagcgcttcttccatcgttttgaaggtggtcaccgccagcaccgggccaaaaatctcctcctggaacacccgcatattgttctgaccaaacagaatcgtcggttcgaggtagtagccgtctttcagttcaccttccagcagcttgcgccgcccgcctgtgagcacgtcagcgccctcttttttaccgatatcaatgtagttgaggatggtttccagttgcccgtgagaaacctgcgcgcccatttgcgtcacgctgtcgagcgggttaccgctacgaatgctttcgacacggcggatggcgcgttccataaagcgttcgtagatagattcctgcactaaagcacgactcggacaggtgcaaacttcgccctggttaaaggcaaacagtgcaaagccttccagcgctttatcgaaaaaggcatcttcttcatccatcacatcagcaaagaagatatttggcgacttaccgcccaactccagcgtcaccggaataatgttttgcgttgcgtattgcataatttgttggcccacttccgttgagccggtaaacgccactttggcgatgcgtttcgaggtcgccagatattcgccaattaccccacctgcgccattgaccacgttcaccacgcccggcggcagtaaatcaccgacaatttccattagcagcagtacagaaagcggggtaagacgtgcgggtttcagcaccacacagttgcccgccgccagcgcgggagccattttccagctcgccatcagcagcgggaagttccacgggataatctgccccaccacgcctaacggttcatggaaatgataggccacggtttcgctatcaacttcactgatcccaccttcctgcgcccgaatacacgaggcgaaatagcggaaatggtcaatcgccagcggtacatccgcagcactggtttcgcgaatgggtttgccgttatcccaggtttcagctgtcgctaacagctcgaggttttgttccattcgatcggcaatcttaaacagaatcgccgcacgatcctgcaccgaggtgtgcgcccatttatctttcactttgtgcgcagcatccagcgccagatcgatgtctcgtttgcccgaagacgccacttcgcacagcagctgcccggtcaccggcgtcagattctggtaatactcgccgtcggcaggggctacccattcgccgccaataaagttgtcatagcgggcttttaacttgagggggaaaccatactcgccgggcttaatctgtgctgaagggggattattggtcatgatcgtctccttgcggtgtgaggtataacaagggtagacgtgactggcgaaatcttcgccagtcggtaacagctttacgacagctatcacgaatttacgggcaagggttacagagatagttgaaaaagcggctaacaatttgccagccgttgtggaaatgatgattacatcgctgcgcgataaatcgccacaatttcttcgtgagttgcctggatcgggttagtaaagccacaggcatctttcagggcattagtcgccaataccgcgaaatcttcttctttcacgttcaggtcgcgtaggcctgccgggatatccactttcttcgccagttcacggatggcgttaatgcaggcttcagcaccttccgcgtcgtttttacctgtcacgttcacgcccattgcagcggcacagtcacgcagacgtgcagcggcgactttgctgttgaatacctgaacgtgcggcagcaaaacggcgttacatacaccgtgtggcaggttgtagaaaccgcccagctggtgcgccatcgcatgaacataacccagagaagcattattgaacgccataccggcgaggaactgggcataagccattgcttcacgcgctttcgcattactgccatcttcaacggctaacggcaggttttcggcaatcatggtcacggctttcagtgcacaagcgtcagtgatcggcgtggcggcaatagaaacatatgcttcgatagcgtgcgttaaggcatccatacccgttgcggcggtcagtgacttcggcataccaatcatcagagaggagtcattgacagaaagcagcggagtgacatgtttatcaacaatcgccattttgatatgacgcgcttcgtcagtgatgatgcagaaacgggtcatttcagaggccgtacccgccgtggtattgatggcgatcatcggcagctgcggttttgcagagcggtcaacgccttcgtaatcgcgaatatcgccgccattggctgccaccagcgcaataccttttgcgcagtcgtgtggagaaccaccgcctaaggagatcacgctatcgcaattattctctttaagtaatttcaaacctgcggcgacgttttccgtggtggggttaggttgggtgccatcataaataacgctaaaaatattgcgttcttccagtgctttttgcacatcgcccgccatacctaatttcgttaacatattgtcagtgacaattaaggtacgggtaaatccataatctgccatcatattcattgcatcagtcaatgaatcagcgccgatgacattcacagaaggaataaagaacgttgaagctgccataacacactcctgaaagtgtaaaaaagggcgggcagcttactgaggattttcattcgaaaatatgatcagtattattgattatcaaaattaatctaataaaaagcacattgtattcattaaacaatgtgctttttttaaattcataagaattttgtattaatttattttaaaacttaattaatcatttccttatttttccggaaataataatgcgtcgcgcaataaatgatcatttccacgacgacgcgtaaagccaatgcggtcaaaatattccagaatctgaattgccagctttcggcctacgcctaagcgatcgcggaaatccgccgcgcaggttgaaccacactcctgatcgagatcgcggatcatattggcaaactcgacaatccgatcgttacggtaataacgatctttaacgatcgcggtaattattccttgctgcgccgcctggcgtagagtcaggcgcattgcctgctcgtcggttcccgtctcttttgccaggtcacgcacccaccacggttcgtcaccaaacagtggctctgctttttgccagatggcctgctgctcttcgctgaagcccgctttgtgatctggcagatgcagccagccgtgatggctgtggatgtcgccgctttcgcgcatcttttcaatcagcaacagtaccagcgcttcatcttccattggcaacgccatacgtcgcagacgttcgcgcccagggccaggttcatcgcgatgttgctcatgataagtcgctaatgtgtcgagaattttccgctgccagcgggcggcaaccggcgcattcaacaagctataaccagcctgaatataaccaggctgttgcagcaattcgcgcatcccttcgccgttgagctggcgcgcccaggcgaaatccgcaaggttaaccgcgccgcgttccagatgaacagataacgcatcggcatcgctctgcgcccgtgcaagagacgccagccattgcagatattccggcttacgtttaccgcgacgcggcgggttaagcatcacgacgcgcgctccggccagcgtgttgcgggcagagatatcgcgcaataccaggcggtcgttatctgccagccataacggggtgtcgaagaccagttcagcaaggttatcttccagcagtgaaacgcgtcccgtgacgtggctggcggcgtggtgaatatgcagcggctgccactgggtcagcggtgtatgggtttgaagctcgacaatcacccgtgtgaacggctctggcggcacatcggcaagcagccagtcgccacggttaatctgctctttttccgcatcacccgcgatgttaagcgcgatacgctgcccggcattggcggtttctgttggctggttttgcgcatgcagcgcacgtacacgcatcggtttatttacaccagtcagccagagtgaatcgcctaccttcacttccccgcttaacgccgtaccggtgacgaccagcccggcaccttttacggtaaatgcgcggtcaatcgcgaggcggaaactatgttggctggcgtgctcgcgttccggcaactgaagcagatgctcgcgcagggcatccattccccgaccttcggttgctgcggtgataaacagttttgcctcagcaaaaccgtattcccgcagaacctcctttacctggcgttcaacctcatcaacacgcgcttcgtccacgcgatcggctttggtcagcgccactgtcagcatcgggttaccggtcagctgcaaaatcgccagatgctcacgggtctgtgccatcacgccgtcatcgcacgccaccaccaacagcgcgtgatcgataccaccaacgcccgccagcatgttggaaagaaacttttcatgaccgggaacgtcgataaaaccaggcacgcgaccatccggctgcggccagtaggcatagccgagatcgatggtcatgccgcgctttttttcttccggcagacggtcagcatttacgccagtaatcgcctgcaataaggttgttttgccgtggtcaacgtgtccggcagtcgcaataatcatttcaacaacatctccaaaaaccgttgctcatcttcaaggcagcgtaaatccagccacaatcgtccgtcataaatacgaccaatcaccggcactggcaattcacgccagcgggcggctaatgactcaaggtggctaccgcgtccatcatggggtgtaaacgttaatgccgcgctcggcaggcgatcaaccggcagcgaaccactgccaatctgcgaaagacatggcataacctgtaccgcaaactccgcgccgtaatgtgcggcaaggggggcctgtaaacgttgtgcctggatttgaatgacctctgcgctgcgggtaagcaggcgcagggtcggtaatttttcactcagagcttcagggtgtaaataaagacgcaacgtggcttccagcgccgcgagggtcattttatccgcgcgtaatgcacgcttcagcgggtggctttgcaggcgggcgatcatctcttttttaccaacaataattcctgcctgcggcccgcctaacaacttgtcgccggagaaactcaccagactgacgcccgccgcaatcaactcctgcggcattggctctttcggcaaaccgtactggctaagatcgaccagcgagccactgcctaaatcagtcactacgggaacatccagctctttgccgagcgccaccagttccgcttcatctatcgctttggtgaacccctgaatgctgtagttactggtatgtactttcatcaacagtgcggtattttcattcaccgcctgacgataatcattcgcgtgcgtgcggttggtggtccctacttcgtgtagggtgcagcctgcctgacgcataacatcgggaatacgaaacgcgccgccaatctccaccagttcgccgcgagataccaccacctcttttccgctggcagtggccgccaacatcaataacaccgccgccgcattgttattgacgatacaggcatcttccgcccccgtaatacggcacagcagctgcgccagcgcccgatcgcgatgtccgcgtccggcgtcgtccagatcatactcgagggtcactggcgaacgcatagcctgcgcaacggcttccaccgcggcttccgcctgtaaagctcgcccaaggttggtatgcagcacggttcccgtcaggttgatcaccggacgcagcgcgctctgcgcttctttcgtcaaccgggcatcgacttcttgcgcccagttttcacaccacgcaggcagcgtctggctgccacgaatcacttctcgcgcttcgtcgagcatctgacgcaacaattccaccacgcgggtgtgaccataagtatcacgcaaagaaaggaaggagctatcgcgcaataagcgatcaatagccggaagttgactatagagggaacgcgtttcggttgtcataggaaacctggctgatcaaggccctctcacacggagaagggcgtttaacataaccacggattgtaacgtgagatgggtcaggaggacatatcgcgcatcaagcctttggcggttcggtgcgagcaaaactttcgcggctaaacaggttttcgaccagtttgactaagtgtgggcggtcgacacaccaacctggcgcaacgcggcggaaattgagatatccgacggcacaggcaatggcgatagtcgccagattgaccgtatcggttttgagtgtgccatcgaccagatatccttccagcacatccagactgcggttgattttctcccgctggcgtaacaattcatcttcagactgctgcgccgctggacgcgcctgttcacgcaccgataccagcccggcatccataatgccatccgccagtgcctcaattttgcgcacccgcaacgactccagcggatcgcgcggcaacatcgccggagcgacattcattaattcaatatattcagcgatgatcggcgaatcaaaccagcattcgccctcttcggtcaccagcaccggcacttttcctaacgggttaaattgcgccacgccgttgtccgcgttatagggcagttcattaataaattcgaaagttatgcccttttctaacaacagaatagaaagtttgcgtacaaacgggctggtgtagctaccgacgagtttcatgccgagtcctttgtgcgaggaaaaatatcagtatggcctggtgatgggaaaaagggcagaaaatgttgatggtttgttacttccaaataaatcacatatttatcatggtgatataaatattttcctaattatttcactctgatggatatctcacttcaggctttcttataaatctgtagggtttcgcctgtcagcagacaaataacccgataaaacaaggatgagaaatgagcggaaaaccggcagcgcgtcagggcgacatgacgcagtatggcggtagcattgttcagggttcagccggggtgcgcattggtgcccccaccggcgtggcctgttcggtgtgccccggcggagtgacgtccggccatccggtcaatcccctgctcggtgcaaaggtccttcccggtgaaaccgacatcgccctgcccggcccgctgccgttcatcctctcccgcacctacagcagttaccggacaaaaacgcccgcgccggtggggagcctcggccccggctggaaaatgcctgcggatatccgcttacagctgcgcgataacacactgatactcagtgataacggcggcagaagcctgtattttgagcacctgtttcccggtgaggacggttacagccgcagcgagtcactgtggctggtgcgcggcggcgtggcgaaactggatgaaggtcaccggctggccgcactctggcaggcgctgccggaagaactccgcttaagtccgcatcgttatctggcgacaaacagtccgcaggggccgtggtggctgctcggttggtgtgagcgggtgccggaagcggatgaggtgctgcctgcgccgctgccgccgtaccgggtactgaccgggctggtggaccgcttcgggcgcacacagacgttccaccgcgaagccgccggtgaattcagcggcgaaatcaccggcgtgacggatggtgcctggcgtcacttccggctggtactgaccacgcaggcgcagcgggcagaagaagcccggcagcaggccatttccggcgggacggaaccgtccgcttttcctgataccctgccgggttacaccgaatatggccgggacaacggcatccgtctgtctgccgtgtggctgacgcacgacccggaatacccggagaatttacctgccgcgccgctggtgcgctatggctggacgccacgcggcgaactggcggtggtgtatgaccgtagtggcaaacaggtgcgcagctttacttacgatgataaataccggggccggatggtggcgcaccgtcacacgggccggccggaaatccgttaccgttacgacagcgacgggcgggtgacagaacagctaaacccggcaggcttaagctacacgtatcagtatgagaaagaccgcatcaccatcaccgacagcctggaccgccgtgaagtgctgcacacgcagggcgaagccgggctgaagcgggtggtgaaaaaggaacacgcggacggcagcgtcacgcagagtcagtttgacgccgtgggcaggctcagggcacagacggatgccgcaggcaggacaacagagtacagcccggatgtggtgacgggcctcatcacgcgcataaccacgccggatggcagggcatcggcgttttactataaccaccacaaccagttaacgtcagccaccgggcctgacgggctggaattgcgccgggaatatgatgaattgggccgtctgattcaggaaactgcccctgacggcgatatcacccgctaccgttatgataatccacacagtgacttaccctgcgcaacggaagatgccaccggcagccggaaaaccatgacgtggagccgttacggtcagttgctgagcttcaccgactgttccggttatgtaacccgttatgaccatgaccgcttcgggcagatgacggcggtgcaccgcgaggaagggctgagtcagtaccgcgcatacgacagccgtggacagttaattgccgtgaaagacacgcagggccatgaaacgcggtatgaatacaacatcgccggtgacctgaccgccgtcattgccccggacggcagcagaaacgggacacagtacgatgcgtggggaaaggccgtccgtaccacgcagggcgggctaacgcgcagtatggaatacgatgctgccggacgggtcatccgcctgaccagtgaaaacggcagccacaccaccttccgttacgatgtacttgaccggctgatacaggaaaccggctttgacggccgcacacagcgttatcaccacgacctgaccggcaaacttatccgcagcgaggatgagggtctggtcacccactggcactatgacgaagcagaccgcctcacgcaccgcaccgtgaagggtgaaaccgcagagcggtggcagtatgacgaacgtggctggctgacagacatcagccatatcagcgaagggcaccgggtggcggtgcattacaggtatgatgagaaaggccggctgaccggtgagcgtcagacggtgcatcacccgcagacggaagcactgctctggcagcatgagaccagacatgcgtacaacgcgcaggggctggcgaaccgctgtataccggacagcctgcccgccgtggaatggctgacctacggcagcggttacctggcaggcatgaaactcggcgacacaccgctggtggagtacacccgcgaccgcctgcaccgggaaacgctgcgcagcttcggccgttatgaactcaccaccgcttatacccctgccgggcagttacagagccagcacctgaacagcctgctgtctgaccgcgattacacctggaacgacaacggcgaactcatccgcatcagcagcccgcgccagacccggagttacagctacagcaccaccggcaggctgaccggcgttcacaccaccgcagcgaatctggatatccgcatcccgtatgccacagacccggcaggtaaccgcctgcccgacccggagctgcacccggacagcaccctcagcatgtggccggataaccgtatcgcccgtgacgcgcactatctttaccggtatgaccgtcacggcaggctgacagagaaaaccgacctcatcccggaaggggttatccgcacggatgatgagcggactcaccggtaccattacgacagtcagcaccggctggtgcactacacgcggacacaatatgaagagccgctggtcgaaagtcgctatctttacgacccgctgggccgcagggtggcaaaacgggtgtggcggcgtgaacgggacctgacgggctggatgtcgctgtcacggaaaccgcaagtgacctggtacggctgggacggcgaccggctgaccacaatacagaacgacagaacccgcatccagacgatttatcagccggggagcttcacgccactcatcagagttgaaaccgccaccggtgagctggcgaaaacgcagcgccgcagcctggcggatgcgcttcagcagtccggcggcgaagacggtggcagtgtggtgttcccgccggtgctggtgcagatgctcgaccggctggaaagtgaaatcctggctgaccgggtgagtgaggaaagccgccgctggctggcatcgtgcggcctgaccgtggagcagatgcaaaaccagatggacccggtgtacacgccggcgcgaaaaatccacctgtaccactgcgaccatcgcggcctgccgctggcccttatcagcaaggaagggacaacagaatggtgcgcagaatacgatgaatggggcaacctgctgaatgaagagaacccgcatcagctgcagcagcttatccgcctgccggggcagcagtatgatgaggagtccggcctgtattacaaccgccaccgctattatgacccgctgcaggggcggtatatcactcaggatccgattgggctgaaggggggatggaatttttatcagtatccgttgaatccagttacgaatacagatcctctggggttagaagtttttcctagaccattccccttgccaattccatggcccaaaagccctgcacagcagcaagcagatgataatgctgcaaaagcattgacaaaatggtggaacgatacagcatcacaaagaatatttgactctctaatattgaataatccgggactagcattagatataacaatgatagcttctcgtggaaatgttgcagacacagggataactgatcgtgtcaatgacataataaatgacagattctggagtgatgggaaaaaacccgacagatgtgacgtacttcaggaactaattgattgtggtgatattagtgctaaagatgcaaaaagcacacagaaagcctggaattgtcgtcactccagacagtcaaacgataaaaaaagatagcccttgtggaggttcctgcaatgtcaaatacataccagaaaagaaaggcaagtaaagagtatggtttatataatcaatgtaagaaactaaatgatgatgaattatttcgcttacttgatgatcacaattccttgaaaaggatttcatctgccagagtattacagttaagaggtgggcaagacgctgttagattggcaattgagttctgctctgataaaaattatatccgtagagatatcggagcatttatactcgggcaaataaaaatttgcaaaaaatgcgaagataatgtttttaatattttgaacaatatggcattgaatgataagagcgcttgcgttcgagctacggcaatcgagtcaacggctcagcgatgcaagaaaaacccaatttattcacctaaaatagtagaacaatctcaaattactgcttttgataaatcgactaatgtcagacgtgctacagcatttgctatttctgttatcaatgataaagcaacaattccactattgattaatctgttaaaagatccaaatggagatgtcagaaactgggccgcatttgcaataaatatcaataaatatgataatagtgatattagggattgttttgtggagatgcttcaggataaaaatgaggaagtccgtattgaagcaataatcggactttcctacagaaaagataaaagggttttatctgttttatgcgatgagttaaaaaaaaatactgtttatgatgatatcattgaagctgcgggtgaattaggtgataaaacgctacttcctgttttagatactatgttgtacaagtttgatgacaatgaaattataacttccgctattgataagctgaagcgttcatagcgtgagttgcctatgcacagtgggggattcccgccggcacggtgcagatgctcgaccggctggaaagtgaaatcctggctgaccgggtgagtgaggaaagccgccgctggctggcatcgtgcggcctgaccgtggagcagatgaaaaaccagatggacccggtgtacacgccggcgcgaaaaatccacctgtaccactgcgaccatcgcggcctgccgctggcgctcatcagcacggaaggggcaacagcgtggtgcgcagaatatgatgaatggggcaacctgctgagtgatgagaacccgcatcatctgcagcagctcattcgcctgccgggtcagcagtatgatgaggagtccggcctgtattacaaccgccaccgctattatgacccgctgctggggcggtatatcactcaggatccgattggactgaaggggggatggaatttttatcagtatccgttgaatccggtcataaatgtagatccgcaaggtttggttgatataaatttataccccgaaagtgatcttatccattctgtagctgatgagattaatatcccaggcgttttcacaatcggggggcatggtacccccacatctattgaatccgcaacgcgcagtatcatgacagctaaagatctagcatatctaattaaatttgatgggaattataaagatgggatgacagtttggttattttcttgtaatacaggtaaaggacaaaattcatttgctagctaattagctaaagagttacatacaaatgtaataggacctgacacgctatggacgtggtgggggcgaggaactaatggtaagttaaaaatggatacagtgctaacagcaccaacgaaccttaattcaaataaggatctaatggctataacaacaaaagaccttggtaattggataacatatgggccatctgggcaccccatttctaatatgcaaggtacgccagaaaaacccagtgatataagataggttgtagatgtatgaaagcatgcttgttactatttttttatttctcttttatttgtcaattgcatggtgctgatgtgaaaataaaacaaaacgaaagtatgatggggtctacagcaatgacctatgatttaagtgaagaaaagttgatgaaactgaagtataaatcacaacatggtgattcagaggcatcatttcgactatatcaatattactgctttactaaaaataacatttacaaacaattgcgattcttggaaagatcagcatctcaggggaatgttacagcgcagtttaattatggggtctttttatcagatacaaatccaacattatcagaatattataatttgaatagagctatttattggatggaattcgctgtaaataacggtaatattgatgcaaagagcaaacttcaagagctcaaaaagctaaagcgaatggatagaaggaagaataaggagaatccgtaaaagcaatagttcatcagactgccgcagcagtagtatgatgatgaatcagggctgtactataactattatcggtaacattaaccgcagcaggggcggtataacactcaggctccgattgggctggaaggtaggtggaatttttatcagtatccgttgaacccgatttctggaatcgatccccttgggattagccacctgtttatacagcataactttaggtatgctttcgtgtgtttcagatataccatgtgatgataatttttatgatgtgcttagtattccagtcgcttctggtaataatatgcaatgtaaaaataatccccgttgtacacatttataaatagatggccaatacctcaaggcctatggagttggaatgttaatgacccgggagcaagcaatagaaaacctgacggcatacgattagtaccgtcagttaatacaggaacttataatcgcaatggattttcaatacatagttgtttaaacgcttttggtccgtctttaggacctcgattctgttccgagggttgtataactggtttatctaatgacatgcaaaaattaaatgagttaatattttcagagccagatagcacattaacagttacggactaaaaaatatggcaaggttattaacaattgtatttttttctctatttctgcgagtgcagttactgcaagacaatttcagagagagttagatttggcagacaaagcaatattatgggcactaatatcagccagtactaaagagggacgaaaagcgtgttcactaagctattttgcctgtaaggccgcagaggctgaactcggactggcatatatggctgcgaatgataacaaggaatttctcacatccttatctaatataatgaggtacaaaatagatgctggactttccgaatcctatacatgctatttattaagtaagggaaagatcataagaccatatctgaaaaatctaaatccactccaacttgccgctgattgcattgaaacagtaaataaaataaaagataagaataaaaaaaatcattgatataaattcagttaatatttgtagtgatgataaaaatataaaattgagagttaatagtactattatggccattgatgattctataaagtgcatcgatgaatgataacttaattttatttaaaaatatattaataactcactctccaggagtttttttaacttagttttataatgaatacgataattaaaagtgaagaagaaaatagttgtatacatatattccatgaccctacattgtgatctatagattaaatattttttaaatgtgactgtcatccttcagataataaagccatcatcgcaatagatggaaaagcactcctgctcttttttgattagagccgtcgcaggaggaacaactcatatcatcattgcgatctcgacgatgtatagtctcatcctgcggcagaacaagacggataaaaaatccaatgagagcacactcatccagaacttattaacataatgaatattaaagaaaaatcatcgaagctaatgaagtaatatgcaaaaataattagtccttacaaggagcaaagttccataatctcccccctccccctcaatgatccaaataaagataatgcatccagctggtcattcttagcagcactttccgcatcaccgaaacatggctgaaatggtcggagtaaaccgccacctgggcgtagatgccgtcgggtaaggcatcgatatcatcgttagggtccagttcaatggttcccagcacaccgtccgtgccgggcacgaccgttaatgattgcaataccccctgcgcctgataagaaccgcctggcacgacaggtaaaatactagtcagtttgccgtgaaacacctgcccaggtagcgcgttaaacaccacttccgcatcatcgccaggtttcagacgtaacagcgagttttgccgaaattgggcgacaatttgccgtttttgctcggggatgaagaccatcaccggacgcagcggcaaggcagctgcgtatgtacctgggcggatcagtacctgagtaacgtagccattgctcggcgcgcgaatgacagtctgctcaaggttatattttgcttcagtaagttgcgctcttaagctcacaatctgcgattgctcgccgttaaccatactgtcgagctggctctggatctgcgcctgctccgccaccgagcctttcaccagcgcatcctgcgcgaggaaattttgccgcgcatcgtcgatgtcacgttccgagaacggattcaccgccgcctggctgcctttcaagtaacgttgataatttttaaacagacggtcgcgctccgctgaaacctgggtggtgttggcctgcgcttcagtgagctgcgcacgcagcgtctttatattatgcgtcgccgtcatcaggtcagcctgaagtctgtcaactcgcgcctggtaacgaaccgggtcgagcttaaaaagcacctcgcccttttgaataagctgattattcttgtcagtgacttcagtaacaattcccgtcacctgtggcgtgatagggatcgctatcactgccttttgcgcggtaaaagtgtaagggtggttgtagttcatcaacaaaatcaaaccactcaccagaaacacgcctcccagcgccgccgtcgccagcgtccactgatttaccggaatgcggaagattttaaagaccgcccacgccagcgccacgtaagttaaaacaatcaatagatccataattagatctccgggaacgtggaatagtcagtctttttctcggcggcgagttgatgctccagccgggaaattcggtcagaaagtgcggcgatttccgggtcagtcgctttctcctgcgacgcaacatgtgactgcataccccagccacgctccggttgatagagcgtcgcccagatccacagaaacggccagataacatgcagagtaaacaggctcacccagcccgccgtatgaatagcgtcggcatggggatggttgcgctttttggcaatcagataagggatgtcatgtatcgcgatgattccataaaaaatcaccagaaagacgaagatcagcactcccaacgcgaaatagtttagaaacatatctgcctcggattcacgtttatcagtgttgtttttgggctggcagccagaagggagtcaggctgatattttgacaataatccgggttcgcgattctcgccataacaccaaagaataatttttagaggtgatgagttgcttagttacataacgattgtatgacgaaggcataacatgctgtagatcacatcaggtgaacgccgtaagaaaatatcttgtgattcagatcacaaagattcaacaaaccatcaaaacaaaaatgtgacactactcacatttaaatgccatttttagcgaaaatcgccgccttgttgcttttttacacaagcgttttgtgatgaacgtcacgtcaattacctctctaccccctatatttatgtgattgatatcacacaaaaggccgtcgactggacagttaaccgattcagtgccagatttcgcagtatctacaaggtccggctacctctgccgccacattaacaaaaaacctcgggcttccagcctgcgcgacagcaaacataagaaggggtgtttttatgtcatccgatattaagatcaaagtgcaaagctttggtcgtttcctcagcaacatggtgatgccaaatatcggcgcgtttatcgcgtggggtatcatcaccgcgttatttattccaacagggtggttaccgaacgagacgctggcgaagctggtcgggccgatgatcacttatctcctgccgctgctgatcggttataccggtggtaagctggtaggcggcgaacgtggcggcgtagtcggtgccatcaccaccatgggcgttatcgtcggcgcagacatgccgatgttcctcggttctatgattgcaggtccgctgggcggctggtgcattaagcacttcgaccgctgggtagacggtaagatcaaatccggttttgagatgctggtgaataacttctccgcaggcatcatcgggatgatcctcgctattctggcattcctcggcattggcccgattgttgaagccctgtccaaaatgctggctgcgggcgttaacttcatggttgtccatgacatgctgccgctggcgtctatctttgttgaaccggcgaaaatcctgttcctcaacaacgccattaaccacggtatcttctcgccgctgggtattcagcagtcccatgaactgggtaaatcaatcttcttcctgattgaagctaacccaggtccaggtatgggcgtgctgctggcgtacatgttctttggtcgtggtagcgctaaacagtctgcgggcggtgcggcaatcatccacttcctggggggtatccacgaaatctacttcccgtatgtgctgatgaatccgcgtctgatcctcgcagtcatcctcggcggtatgactggcgtgttcacgctgactatcctgggcggtggtctggtttctccggcatctccgggttctatccttgctgtactggcgatgacaccaaaaggtgcttacttcgctaacatcgcgggtgtgtgtgcggcgatggctgtctccttcgttgtctctgctattttgctgaaaaccagcaaagtgaaagaagaagatgatattgaagcagcaactcgtcgtatgcaggacatgaaagctgagtctaaaggcgcatctccgctgtctgctggcgatgtgactaacgacctgagccacgtacgtaaaatcatcgttgcctgtgacgccggtatgggttccagtgcgatgggcgcaggcgttctgcgtaagaaaattcaggatgcaggtctgtcgcagatttctgttactaacagcgcgatcaacaacctgccgccagatgtggacctcgtcatcactcaccgtgacctgaccgaacgcgctatgcgccaggttccgcaggcacagcatatttcgctgaccaacttcctcgacagcggcctgtacaccagcctgaccgaacgtctggttgctgcccaacgccacacggcaaacgaagagaaagtaaaagacagcctgaaagacagctttgacgattccagtgctaacctgttcaagctaggcgcggagaacatcttcctcggtcgcaaagcggcaaccaaagaagaagcgattcgttttgctggcgagcagctggtgaaaggcggttacgttgagccggaatacgttcaggcgatgctggatcgtgaaaaactgaccccgacttatctgggtgagtctatcgcggtgccacacggtacggttgaagcgaaagatcgcgtactgaaaacgggcgtcgtgttctgccagtacccggaaggcgtgcgcttcggtgaagaagaagatgacattgcccgtctggtgattggtattgctgcccgtaacaacgagcacattcaggttatcaccagcctgaccaatgcactggatgatgagtccgtcatcgagcgtctggcacacaccaccagcgtggatgaagtgctggaactgctggcaggtcgtaagtaatccaatcccaccctctccacatggagaaggtggggttaattgcctgatgcgctacgcttatcaggcctacaggatgcatcacaatttgttgaatttgcacgttcttgtaggccggataaggcgcttacgccgcatccggcgctgcccctctcctcacggagagggtttgggtgagggaaaagcctcaccccagccctctcgggtaaaaacattgatgaaggttaatactatgaaagcattacattttggcgcaggtaatatcggtcgtggctttatcggtaaactgctggcagacgcgggtatccaactgacgtttgccgatgtcaatcaggtggtacttgatgccctgaatgcccgtcatagctatcaggtacatgtggttggtgaaaccgagcaggtagataccgtttccggcgtcaatgctgtcagcagcattggtgatgatgtcgttgatctgattgctcaggttgatttagtcactaccgccgttggcccggttgtgctggaacgtattgctccggcaatcgccaaagggcaggtgaaacgtaaagaacaaggtaatgaatccccgctgaacatcatcgcctgtgaaaacatggtacgcggtaccacgcagctgaaaggccatgtgatgaacgccctgccggaagacgccaaagcgtgggtagaagaacacgttggctttgtcgattccgccgttgaccgcatcgtaccgccttcggcttcggcaactaacgatccgctggaagtgacggtagaaaccttcagcgaatggattgtcgataaaacgcagttcaaaggcgcactgccgaacatcccaggcatggagttaaccgacaacctgatggcatttgtcgaacgtaaactcttcaccctgaacacgggtcatgctataaccgcgtacctcggaaaactggccggtcatcagaccattcgtgacgcgattctcgacgagaaaatccgcgcggtggtaaaaggtgcgatggaagaaagtggtgcagtattgatcaagcgctacggctttgacgctgacaagcatgcggcgtacatccagaaaattctcggccgttttgagaacccgtatctgaaagatgatgtagagcgcgtaggccgtcagccactgcgtaaactgagtgctggcgaccgtctgatcaagccactgctcggtacgctggaatatggtctgccacataaaaacctgattgaaggtattgccgctgcaatgcacttccgcagtgaagatgatccgcaggctcaggaactggcagcactgatcgctgacaaaggtccgcaggcggcgctggcacagatttccggtcttgatgccaacagcgaggttgtatccgaggcggtaaccgcttataaagcaatgcaataatggtggaccaggcgcaggacaccctgcgcccgaataacagattgtcagatatgcaggcaacaatggaacaaacccaggcctttgaaaaccgtgtgcttgagcgtctgaatgctggcaaaaccgtgcgaagctttctgatcaccgccgtcgagctcctgaccgaggcggtaaatcttctggtgcttcaggtattccgcaaagacgattacgcggtgaagtatgctgtagaaccgttactcgacggcgatggtccgctgggcgatctttctgtgcgtttaaaactcatttacgggttgggcgtcattaaccgccaggaatacgaagatgcggaactgctgatggcattgcgtgaagagctaaatcacgacggcaacgagtacgcctttaccgacgacgaaatccttggaccctttggtgaactgcactgcgtggcggcgttaccaccgccgccacagtttgaaccagcagactccagtttgtatgcaatgcaaattcagcgctatcaacaggctgtgcgatcaacaatggtcctttcactgactgagctgatttccaaaatcagcttaaaaaaagcctttcaaaagtaagcaacgtctgcttactgcccctctacctgcttcggccgataaagccgacgataatactccagacgttgtagatataacggcacgctttcatcgggtattccggacggaatcgcgttacggggaggaagttttttcagatactcccggaacgcctggcttgatgccatgaaatctacggctttatcgataagaagcggaacgttttcacctaatttgcccatgatgatatctccgtattaccccgcgccgggaatgcgcggccgccaattttagtttaggttcccggtaaagatgacattaaggaaaacgtgctgaatcctcaataatcatccgctgctgtttattatcttttttctatagatttcttaattaatcaacgaattgcgcagtttttgagcatgttaatgattacgttacagaactattacaatgtcattagttgtgaacaaagcacctggtcgcgcatactaggggctataaatttatctttatcagaagccatcacatgaaagaagtcgaaaaaaacgaaatcaaacgcctcagcgatcgcctggacgccatccgccaccagcaggccgatctttcgctggttgaagccgcagacaaatatgccgagctggaaaaagagaaagccacgctggaagcagaaattgctcgcctgcgtgaagttcatagccaaaaactgagtaaagaagcacagaagctgatgaagatgccattccagcgcgcaattaccaaaaaagagcaggctgatatgggcaagctgaagaaaagtgttcgcggactggtcgttgtgcacccaatgaccgcactgggccgcgaaatgggcctgcaggagatgactgggttttcaaagaccgcgttttaagaacacagtatctacagggtgattctgcacattcctataggccgagtaaggtgttcacgccgcatccggcaagataaggcgctctggatcaacaacctaagggcaattctctgatgaggattgcccttttctttaccagacatctccccccacaagaattggccctaccaattcttcgcttatctgacctctggttcacaatttcccaattaaaactcacatcaatgttgccaatacataacatttagttaaccattcattgtcattatccctacacaacacaattggcagtgccacttttacacaacgtgtgacaaggagatgagcaacagactcattacacgatgtgcgtggactccaggagacctgcaatgaatctctggcaacaaaactacgatcccgccgggaatatctggctttccagtctgatagcatcgcttcccatcctgtttttcttctttgcgctgattaagctcaaactgaaaggatacgtcgccgcctcgtggacggtggcaatcgcccttgccgtggctttgctgttctataaaatgccggtcgctaacgcgctggcctcggtggtttatggtttcttctacgggttgtggcccatcgcgtggatcattattgcagcggtgttcgtctataagatctcggtgaaaaccgggcagtttgacatcattcgctcgtctattctttcgataacccctgaccagcgtctgcaaatgctgatcgtcggtttctgtttcggcgcgttccttgaaggagccgcaggctttggcgcaccggtagcaattaccgccgcattgctggtcggcctgggttttaaaccgctgtacgccgccgggctgtgcctgattgttaacaccgcgccagtggcatttggtgcgatgggcattccaatcctggttgccggacaggtaacaggtatcgacagctttgagattggtcagatggtggggcggcagctaccgtttatgaccattatcgtgctgttctggatcatggcgattatggacggctggcgcggtatcaaagagacgtggcctgcggtcgtggttgcgggcggctcgtttgccatcgctcagtaccttagctctaacttcattgggccggagctgccggacattatctcttcgctggtatcactgctctgcctgacgctgttcctcaaacgctggcagccagtgcgtgtattccgttttggtgatttgggggcgtcacaggttgatatgacgctggcccacaccggttacactgcgggtcaggtgttacgtgcctggacaccgttcctgttcctgacagctaccgtaacactgtggagtatcccgccgtttaaagccctgttcgcatcgggtggcgcgctgtatgagtgggtgatcaatattccggtgccgtacctcgataaactggttgcccgtatgccgccagtggtcagcgaggctacagcctatgccgccgtgtttaagtttgactggttctctgccaccggcaccgccattctgtttgctgcactgctctcgattgtctggctgaagatgaaaccgtctgacgctatcagcaccttcggcagcacgctgaaagaactggctctgcccatctactccatcggtatggtgctggcattcgcctttatttcgaactattccggactgtcatcaacactggcgctggcactggcgcacaccggtcatgcattcaccttcttctcgccgttcctcggctggctgggggtattcctgaccgggtcggatacctcatctaacgccctgttcgccgcgctgcaagccaccgcagcacaacaaattggcgtctctgatctgttgctggttgccgccaataccaccggtggcgtcaccggtaagatgatctccccgcaatctatcgctatcgcctgtgcggcggtaggcctggtgggcaaagagtctgatttgttccgctttactgtcaaacacagcctgatcttcacctgtatagtgggcgtgatcaccacgcttcaggcttatgtcttaacgtggatgattccttaatgattgttttacccagacgcctgtcagacgaggttgccgatcgtgtgcgggcgctgattgatgaaaaaaacctggaagcgggcatgaagttgcccgctgagcgccaactggcgatgcaactcggcgtatcacgtaattcactgcgcgaggcgctggcaaaactggtgagtgaaggcgtgctgctcagtcgacgcggcggcgggacgtttattcgctggcgtcatgacacatggtcggagcaaaacatcgtccagccgctaaaaacactgatggccgatgatccggattacagtttcgatattctggaagcccgctacgccattgaagccagcaccgcatggcatgcggcaatgcgcgccacacctggcgacaaagaaaagattcagctttgctttgaagcaacgctaagtgaagacccggatatcgcctcacaagcggacgttcgttttcatctggcgattgccgaagcctcacataacatcgtgctgctgcaaaccatgcgcggtttcttcgatgtcctgcaatcctcagtgaagcatagccgtcagcggatgtatctggtgccaccggttttttcacaactgaccgaacaacatcaggctgtcattgacgccatttttgccggtgatgctgacggggcgcgtaaagcaatgatggcgcaccttagttttgttcacaccaccatgaaacgattcgatgaagatcaggctcgccacgcacggattacccgcctgcccggtgagcataatgagcattcgagggagaaaaacgcatgattatttccgcagccagcgattatcgcgccgcagcgcaacgcattctgccgccgttcctgttccactatatggatggtggtgcatattctgaatacacgctgcgccgcaacgtggaagatttgtcagaagtggcgctgcgccagcgtattctgaaaaacatgtccgacttaagcctggaaacgacgctgtttaatgagaaattgtcgatgccggtggcactggctccggtgggtttgtgtggcatgtatgcgcgtcgtggcgaagttcaggcagccaaagcggcggacgcgcatggtattccgtttactctctcgacggtttccgtttgcccgattgaagaagtcgcgccagccatcaagcgcccaatgtggttccagctttatgtactgcgcgatcgcggctttatgcgtaacgcgctggagcgagcaaaagcagcgggttgttcgacgctggttttcaccgtggatatgccgacaccgggcgcacgctaccgtgatgcgcattcaggtatgagcggcccgaacgcggcaatgcgccgctacttgcaagcggtgacacatccgcaatgggcgtgggatgtgggcctgaacggtcgtccacatgatttaggtaatatctcagcttatctcggcaaaccgaccggactggaagattacatcggctggctggggaataacttcgatccgtccatctcatggaaagaccttgaatggatccgcgatttctgggatggcccgatggtgatcaaagggatcctcgatccggaagatgcgcgcgatgcagtacgttttggtgctgatggaattgtggtttctaaccacggtggccgccagctggacggtgtactctcttccgcccgtgcactgcctgctattgcagatgcggtgaaaggtgatatagccattctggcggatagcggaattcgtaacgggcttgatgtcgtgcgtatgattgcgctcggtgccgacaccgtactgctgggtcgtgctttcttgtatgcgctggcaacagcgggccaggcgggtgtagctaacctgctaaatctgatcgaaaaagagatgaaagtggcgatgacgctgactggcgcgaaatcgatcagcgaaattacgcaagattcgctggtgcaggggctgggtaaagagttgcctgcggcactggctcccatggcgaaagggaatgcggcatagtcgtttgcgccccctcaccctaaccctctccctcagggagaggggaccgttcggcgctgtatgtactccctcactctgaaacgacaccgcactctttttttctccctcgcccctccggggagagggccggggtgaggggaaaaggccgcactgctcaccaattttctgctatcctgcccccgcactaagggggcagtatgctaaacatcgtactttacgaaccagaaattccgccaaatactggcaacatcatccgtctttgcgctaataccggctttcgtctgcatatcatcgaaccgatgggatttgcctgggacgataagcgcctgcgccgcgcggggctggactatcacgagtttaccgccgttacgcgtcatcatgactatcgcgcgttcctcgaagcagaaaatccccagcgcctgttcgccctcaccacgaaaggtacacctgctcacagcgccgtaagctatcaggatggcgattatctgatgttcggcccggaaacacgcggcctgccagcgagcattcttgatgccctgcccgctgaacaaaaaattcgcattccgatggtgccggacagccgcagcatgaatctgtccaatgcggtgtcggtagtggtgtatgaagcctggcggcagttggggtatccgggagcggtattgagagattagttactgtaggccggatagatgattacatcgcatccggcacgatcacaggacattagatcccatccccatactcaaatgtatggttaataccgttgaaatgctggtccatatccattgatggcttatcgctgtctggtttaccgacaatacgagccggaacgccagcggcggtggtatgcggcggcaccggttgcagcaccacggaacctgcgccaatcttcgcgccgcgcccaacttcaatattgccgaggattttcgcgcccgcgccaatcatcacaccttcacgaattttcgggtgacggtcaccaccagatttacccgtaccgccaagcgtcacagattgcagaatcgatacgtcgttttcaatcaccgccgtttcaccaacgacgatgcctgtcgcgtggtcaagcatgataccgcgaccaatttttgctgccgggtgaatatcgacctggaacgtcacagaaacctggttttgcagaaagattgccagtgcgcgacgcccctgattccacaaccagtgaccgatgcgataggcctgcaaggcatgaaaacccttcaggtataacaacggggttgagtatttatcgactgccgggtcgcgggtacgcaccgcctgaatatcacaggccgcagaggcgatcatttccgggtcagcggcgtaggcttcttccaccacttcacggatagcaatagcaggcataattggcgatgacagcttgttcgccagcatgtagctcagtgcactgccaaggttttcgtgcttgagtagcgtcgcgtggtaaaaactggccagcattggctcacagtccgccagcgttctggcttcggctttaatattgttccagacaatttccagttcttcacacgacattgcttactccacacgatgagataatgaccggcccgttctgcgcgggccgggtcatagcggtaacaaaggttccctggggttagtggctgctgcgctcgtccttgcgtgcacgacctagtaaagtcaatgctgcctcgcgcgcgttttttccgcaatataatacttgataaatttcctcggttattggcatttcaacgccgaagcgatgcgccagttcgcggacttctttcgtattgcggtagccttccaccacctgaccaatcttctcctgcgcgctttgtacatccatgccctgaccgagcatcatgccaaaacggcggttacgcgactggttgtcggtacaggtaagcaccagatcgccaagccccgccatgcccataaaggtggcagggtcggcacccagcgccgcaccaagacgcgacatttcagccagcccacgggtgatcagcgccgtacgcgcattcgcaccaaaaccgataccgtcggacatccccgcaccaatggcaataacgtttttcaccgcgccgccaagctgcacgccaatgaaatccggattgctgtaaacgcggaaacttttgccgcagtgcagcagctgctggagatcatcggcaaaggtctgatcggtcgaggccagcgaaatagctgtcggtaaacctgccgccagttctttcgcaaacgttgggccagagataaccgccagcggaatttgatcgcctaaggcctcacgcgccacgtcctgtaacagacgtccggtttccgcttccagccctttggtcgcccacaccagacgcgcatcaggacgcatcagtggtttaatctggcgcagcacttcaccaaagacatggctgggtacgacgacgagaatattacggctggctgccagcgcagtggcgagatcgctttcaagatggagcgtatcgggaaaaggcacatcggggagaaacgcggcgttacagcggtcgcgttcaagcgttgcgatatgttcagggtcatggccccagaggacaacctcgtggccatttcttgccagggtgatggcaagagcggtgccgtacgagccggcaccgatcacagtcattgaagcattacgttggttcatcaggcatcctgatgttcttcagtaccttcgccagcctgctgctgcaaatagttcatgaacagcgcatcgaagttaaccggcgcaaggttcagttgcgggaatgtaccgcgggataccatgctggtgatgcactcacgagcatacgggaacagaatgttcgggcagtatgctcccaggcaatgcgccatctgggtgccttcgatacccgcgatggagaaaataccgccctgctgaacttcacacaggaacgcggtttcttcgcccaaagaggccgttacggtaacacgcagtaccacttcgtatacgtcatctgccagttgggaagatgccgtatccagatcaagtttaacttctggttgccaatctttctggaaaacgtgcggcgcgttcggcgcttcgaaagagatatccttggtataaatacgttggatctggaaagtcatttcagtgttgttttgttctgacatgtgtagaaaacccttaagtgttgtccttaaatactgcgcaatgtaatgccaacgttcacacgttatttcagcaggggatccagtccaccacgtgcatccaatgcatacaagtcatcacagccgccaatgtgctgtgcgtcaataaaaatctggggaaccgtggtgcgaccgctgcgtttgatcatctcttcacgcttggcggcgttgccatcgatcggcagctcctggaaactcacgcccttgctgctcagcagtgcttttgcacgatggcaatacgggcaggtttctttggtatagatttcaacattggccataaattagctcctgtttttttaccctgaaatttcatgttgcagggcggcagcaaaatggagtgtccccagaagcttataacaataagtcgctgggggcctaattgcagctaacggcctgcatcatgaaagacgacaggtaaattatttgccgcgcaccaaaggcaagttttcgccagcccagccagcgacgccttctttcagcacgaatacttgcgcaaaaccagctttcgtcagtgcgtttgcaggctcctggcactgcatgccagaaccgtctaccacgataaccggtttgtctttgtgcttctcaagctcaccaacattgttggctttgatttcgctcggcaacagattaatagaacctgcgatatggcctttacggaagtcatcacgctgacgtaaatccacaaccacagcgtcttctttgttgatcagacgcgtagcttcaccacgagtaatcaccttcactttcgaggtcaggctcttaaacgtagtcacaagaaccgccaccagtaacgcgatccaggcgatactcagtatgggatgacggccaacaaattgcataatttcttgcatggggggtaacaactcccgacgtagtgattaaaaaaaccaggaaaggagtatacctgcgcggtgcggcaaatacagccagcgcgttaactggaatgcaattttgcggggcgcgacgaaaaaaaagcgtaaatctggcatcggcttgccgcgagcggtcgtatattttgatcttcagaggctattttatcgattcagctgtagtaaaattacgcaaattttgactcttgagtatgaggttgtcgcaatgttggtttctaaaaaacctatggtactggtgattctggatggctatggctatcgcgaagaacagcaggataacgccatttttagtgctaaaaccccggtaatggatgcactgtgggccaatcgtccgcataccctaatcgacgcttccggtctggaagtcggtctgcctgaccgtcagatgggtaactccgaagtaggccacgttaacctgggtgccggccgcatcgtgtatcaggacctgactcgtctggacgttgaaatcaaagatcgcgctttctttgctaatccggtgctgactggcgcggtagataaagcgaaaaacgcaggcaaagcggtacacattatgggtctgctctccgcaggcggcgtacacagccacgaagatcacatcatggcgatggtagaactggcagctgaacgcggcgcagaaaaaatctacctgcacgcattccttgacggtcgcgacactccgccgcgcagtgctgaatcctcgctgaaaaaattcgaagaaaaatttgccgcgctgggcaaaggccgcgtagcgtccatcattggtcgttactacgcgatggaccgcgataaccgttgggatcgcgtagaaaaagcttatgacctgctgactctggcgcagggcgagttccaggccgataccgccgttgctggtttgcaggctgcttatgctcgcgacgaaaatgatgaattcgtgaaagcgaccgttatccgtgctgaaggtcagccagacgcggcaatggaagacggcgatgcactgattttcatgaacttccgtgctgaccgcgcgcgtgaaatcactcgtgctttcgtgaacgctgatttcgatggcttcgcgcgtaagaaagtggttaacgtcgatttcgtgatgctgaccgaatacgccgctgacatcaaaactgcggttgcttacccacccgcttccctggttaacaccttcggcgagtggatggcgaaaaacgacaaaactcagttgcgtatttccgaaaccgaaaaatatgcccacgttactttcttcttcaacggtggcgtagaagagtcgttcaaaggcgaagatcgcattctgatcaactcaccgaaagtggctacctacgatctgcaaccggaaatgagctccgcagagctgaccgaaaaactggttgcggccatcaagagcggcaaatacgacaccatcatctgtaactatccgaacggcgacatggtaggtcacaccggggtgatggaagcggcggttaaagcggttgaagcgctggatcactgcgtggaagaagtcgcgaaagcggttgagtccgtgggtggacaactgctgatcaccgctgaccacggtaacgctgagcagatgcgcgatccggcaacgggtcaggcacacacggcacacaccaacctgccagttccgctgatttacgttggtgataagaacgtgaaagcggttgaaggcggcaaactttctgacatcgcgccgaccatgttgtcgctgatgggtatggaaatcccgcaagagatgactggtaagccgctgttcatcgtggaataatccctccccatgaggggaaaggcgattaataccatgacacgggccgtgaaaccgcgcaggtttgcaatcaggcccatcatctacgccagcgttcttagcgctggcgtattgttgtgcgccttttccgcccacgcggatgagcgtgaccaactcaaatctattcaggctgacatcgccgcaaaagagcgcgcggtacgccaaaagcaacaacaacgcgcaagcctgctcgcacaattgaaaaagcaggaagaagcgatctctgaagccacccgtaagctgcgcgaaacgcaaaacacgctcaatcaactcaataaacagattgatgagatgaacgcgtcgattgccaaactggagcagcaaaaagccgcccaggagcgcagcctcgccgcacaactggatgccgcattccgtcagggcgagcataccggtattcagctgattctcagcggtgaagaaagccagcgtggacagcgtttacaggcttatttcggctatctcaaccaggcgcgacaagaaaccattgcccagttgaagcaaacgcgtgaagaagtcgccatgcagcgtgctgaactggaagagaaacagagcgagcaacaaacgctgttatatgagcagcgcgcccaacaggcgaaactgactcaggcgctgaacgagcgtaaaaagacgctggcagggctggagtcttccatccagcaaggtcagcaacagttgagcgagctgcgcgccaacgaatcccgtctgcgtaacagcattgcccgtgcggaagccgcggcgaaagcgcgtgcagaacgagaagcacgtgaggcccaggcggttcgcgaccgccagaaagaagcgacgcgcaaaggcaccacctacaaaccgaccgaaagcgaaaaatcgctgatgtcccgtaccggtggtctgggcgcgccgcgtggtcaggcattctggccggttcgcgggccgacgctgcatcgctatggcgaacagctacagggtgaattacgctggaaaggtatggttatcggtgcttctgaaggtactgaagttaaagcgattgccgacggtcgggtgattctggctgactggctgcaaggctacggtctggtggtggtggttgagcatggtaaaggcgacatgagtctttacggctataatcagagcgcactggtgagcgttggttcgcaggttcgcgcgggccagccgattgcactggtgggcagcagtggcggtcagggtcggccttcactctatttcgaaattcgccgccagggtcaggcggtcaatccacagccgtggttgggaagataagttttgtttccatttcgtcgtaacgttcttgcatttgccgctctgttggcgctctcctcccccgtacttgctggcaaacttgccatcgtcattgatgattttgggtatcgcccgcacaacgaaaaccaggtgctggcgatgccttccgctatctccgtcgctgtattacccgattcaccgcacgccagagagatggcgaccaaagcgcataacagcgggcacgaagtgttgattcatctcccgatggcaccgttgagtaaacagccgctggagaaaaatacgctacgcccggagatgagcagcgacgaaattgagcgcattattcgtagtgcggtcaataacgtgccctatgccgtggggatcaacaaccacatgggcagcaagatgacctctaacctgtttggtatgcagaaagtgatgcaggcgctggagcgttacaatctttacttcctcgacagcgtaaccatcggtaatacccaggcgatgcgcgccgcgcaaggcactggcgtgaaggtgatcaaacggaaggtattcctcgacgattcgcaaaatgaagcggacatccgtgtgcaatttaatcgcgcaattgacctggcgcgtcgcaacggttcgaccattgccattgggcatcctcaccctgcaacggtacgcgtgttgcaacagatggtttataacctgccgccagacattacgctggtgaaagccagcagcttgctgaatgaaccgcaggttgatacttctacaccgccgaaaaacgctgtgcctgatgcaccgcgtaatccgttccgtggcgtgaagctgtgcaaaccgaagaaaccgatagaacctgtttatgctaatcgcttctttgaagtattaagcgaaagcatcagccagagcacgctgatcgtttacttccagcatcagtggcaaggctggggcaaacagcccgaagcggcgaagtttaacgctagcgcaaattaaaggcgctacgcgtaatgcgatggtgcgaccgcgttttgtcgcgccattgccataagcggaaagaccacagtaacgcctggtaaccgaccttcacgctgcgcacattggtaatcaggcgcttatacataccggaagtaaatatctcggcaatcatccgttggcgggtaagaatatccggctctttgcgcaccgcatggcaaacacgcaatgcctcgtaagttatttgctgatgaaattccggataaatcataattttgtcggcataatttcgatttaatttctccagcaggcgggtaatcttaatatagtgacgttgataattaaggtttttattcccttgtctatgcaaccgactcactgacgtattatgcagataatatttatataatgattgctcggtatatcgcgcacgcagcgcgttaaacatgaattctgttgtccagacaatatcctgatgatgtaatccggcaataaatttaatgttatttttaacaataacatcacggcgataaacccccatccagacaacgtgagtccaacggcgcgaagaaagccccatccgcagccagtccgggccggttaatacgccggttgagcgaaggcgatcggtggggatggattgccaggtttctcccgtttcacgaaaacaccagtcagcgttgcactgcgccacgtcgaggtcgtcctctaacgccatggtcatcagcgtttcgtacatggtgggatagacttcatcgtcagcatcgacaaaagcgacatatttgcccgttgccacttcaatcccacgattacgcgccaccgatgcgccagcattcgcctgatgcaacaaacgaacgtgcggatagttttctgcgtaatactttgctatttcaacagaattatccgttgaaccatcgttaataataatgatttccagagcagtccaggtttgcgtaattaaagattccatacaagtgcggaaatcatcgcccgcattatataacggaataataacactaagtttattggtgctgttcatcataaattaccgacgacctctgaagttatcctgacgttttacaggctttgtattaagaaactattaagcctgtgagatattatttttacaggtgagagagtcacttcagggtagagagataatgagagcagctatataagagatcagcacaattacgaactctttattacactgacaggattttacatatttaacagattatcctcagataaaagggctggaataccagcccttgttcgtgttaatcccagctcagaataactttcccggactggcccgaacgcatagcgtcaaagcccttctggaaatcatcgatagagaaacgatgggtaatgatcggcgaaagatcgaggccagactgaatcagcgccgccatcttgtaccaggtttcaaacatctcacgaccgtaaatacctttaatgaacaagcctttaaagatcactttggtccagtcgatagacatatcagacggcggaatacccagcatcgcaatacggccgccgtgattcatggtgtcaagcatggtacgaaacgctggcggcgcaccggacatttccagaccgacatcaaaaccttcggtcatgcctaactccgccatcacgtcattgagattttctttggcgacgttaaccgcacgggtgatacccattttacgcgccagctcaaggcggtattcgttaacatcagtgatcaccacattgcgtgcaccaacgtgtttcgccaccgccgctgccataataccaatcgggcctgcaccagaaaccagcacatcttcgcccaccagatcaaacgacagcgcggtatgcacggcgttaccgaagggatcaaaaattgcggctaagtcatcggaaatattgtcggggattttgaaggcgttgaatgccgggatcaccagatattcggcaaagcagcccgggcgattaacaccaacgcctatcgtgttgcggcacaaatgggtacgaccaccacgacagttgcggcaatgaccacaggtgatatggccttcgccagaaacgcgatcgccgatcttgaagcctttcacttcctgaccaatacctaccacttcaccgacatattcatggcccacgaccatcggcaccgggatggttttttgcgaccactcatcccagttatagatgtgaacgtcagtcccgcagatggctgttttacggattttaatcagcagatcgttatgcccgagttccggtacaggaacgtcggtcatccagatgccctcttccgctttcagtttggataacgctttcatctcacatcctcaggcgataacgcccagttgtttaccaatacgcgtaaatgcttctactgcacgcgtaatttgctcaggggtatgcgccgcagacatctgggtacgaatacgcgcctgacctttcggaacgaccggatagaagaaaccggtaacgtaaatgccctctttttgcagctcacgggcaaatttctgcgccactaccgcatcaccaagcatgaccggaataatggcgtgatcggctcccgccagggtaaagcccgccgccgacatttgctcacggaactgacgcgcgttcgcccacagacggtcacgcagttcgctgcccgcttcgaccatctccagtactttgatggacgcggcaacaatggccggtgccagcgagttggagaacaggtacggacgagaacgctggcgcagccactcaaccacttctttgcgcgccgcggtataaccaccagaagccccgcccagcgctttaccaagcgtaccggtgataatatcgacccggcccatcacatcgcagtattcatgggaaccacgaccattttcaccgacaaaaccgaccgcgtgggagtcgtctaccatcaccagggcatcatatttatctgccagatcgcaaacgcccttcaggttggcaatcacgccgtccattgagaacacaccatcggtggcgatcagcacatgacgcgcaccggcttcacgcgcttctttcagacgtgcttccagctcctgcatatcgttgttggcatagcgatagcgtttagctttgcacagacgcacaccatcaataatagacgcgtggttcagtgcgtcggagataatggcgtcttccgcacccagaagcgtttcaaacaggccaccgttagcatcaaagcaggaagagtagagaatcgcatcttccatccccaggaaggccgccagtttttgttcaagctctttatggctgtcctgagtgccgcaaataaaacgcaccgaagccatgccgaaaccgtgagaatccattcccgcctttgccgccgcaatcagatcaggatgattcgccagcccgagatagttgttggcacaaaagttaatgacgtggcttccatcagccacagtgatatctgcttgctgcgcagacgtaataatgcgctcttctttaaacaacccttccgcccgtgcggtttccagatcgttggttaactgctgataaaattctccacgcattgcgattctccagacagggcaaattccagcacatattacccaaacttataggtcgcgacgagataacgcgttaacacttctgcaaaattcaggataaataacgtgtaacttgatgtctctcaacacctacagatagtagaaaaactgtacagttttggctgggcataatgatgattgattttactgcattgatataaaaagaaaaaatgatgccaaagcatcatttttcctatctcagttggtatcaaaacgctacccactaatggagggaaacctattttcttgaaaggaaaattctcagcgcctgcatttttgcccctaaagtgttactcctgaagcagcgaaacaaatcgaaccattttcctctccccagatagtttaggttgaagagatcggggcgtttgtaatagcacatgacaaaaatgccctggtcatcgtccacaatgttattatttagtgttattttttgactttccagaactaatttatagaattctttccatttatgctgtgaaccaacaattgcgcccccaataatatatacatgattgccaatcatgaaatcaaaaacctgttgttgagatgtgacagtaagccctttttttatagtgaaaagatgcatcttactttcatcaaatgggaaatcccaaattttcaatcctcgagttacatttggcttatggcaatagccaaaatctatccacgcaacaagaggcgttttcactaagcccatgttgatagctttatttacaaaataggccttaaggttacataccaaaacatactctggtgaccagtactctgggttttttaattgtcgaggctcaagtctatttgtaaacgactcatctttttgaattttttcgatacgacttctgatatatctaaatttcttttttatatcgataacgataaccgttgttggttttccgttgcgaatcgcttcaacccttggtttcaaatcgggagaagtgaaaataatcatctcattttcaagtgcggccagacgctcaaagtaactaaaataaacatcaactgaacgagctagtttttcacggaaccctttattagcagtccaatcccctctaccaatgtcaaaatatgcagtgataattgtggtggatgatttcattactaataagaccattaatataaaaaaagaattatatcataaatattaatagaatgtatactgtatattatccattcaaatgcttccgttatttatcatacatcggaatattgatactaaagcactattcacatgcaaaaccaacatccgccatgaaggactagctaaaacccaaactagtttgttgcaattagcatccttgcacctctatgtaaagggctgaagggattcggatgtgatggtatgattacagacattcgtgtctgagattgtctctgactccataattcgaaggttacagttatgatcatcgttaccggcggcgcgggctttatcggcagcaacatcgttaaagccctgaatgataaaggcatcaccgatattctggtggtggacaacctgaaagacggcaccaagtttgtgaacctggtggatctgaatatcgcagactatatggataaggaagacttcctgatccagattatggctggcgaagagttcggcgatgtcgaagcgattttccacgaaggcgcgtgctcttccaccaccgagtgggacggcaagtatatgatggataacaactatcaatactccaaggagctgctgcactactgcctggagcgtgaaatcccgttcctgtacgcttcttccgcagccacctacggcggacgcacctccgactttattgaatcccgcgagtacgaaaaaccgttgaacgtctacggttactcaaaattcctgtttgatgaatatgttcgtcaaatcctgcctgaagcgaactcgcagattgttggcttccgttatttcaacgtttatggaccgcgtgaaggccataaaggcagcatggcgagcgtcgctttccatctcaacacccagcttaacaacggtgaatcaccgaagctgtttgaaggtagcgagaacttcaaacgcgacttcgtctatgtgggcgacgtggctgatgtgaatctgtggttcctggaaaatggcgtttccggcatcttcaatctcggtactggtcgtgcggaatccttccaggcggtagctgatgctacgctggcttatcacaagaaaggccagatcgaatacattccgttcccggataaactgaaaggccgctatcaggcgttcactcaggcagatctgacaaatctgcgcgcggcgggttacgacaaaccgttcaaaaccgttgctgaaggtgtaacggaatacatggcctggctgaatcgcgacgcataagagctctgcatgaaaatactggtgatcggcccgtcttgggttggcgacatgatgatgtcgcaaagtctctatcgcacgctccaggcgcgctatccccaggcgataatcgatgtgatggcaccggcatggtgccgtccattattatcgcggatgccggaagttaacgaagctattcctatgcctctcggtcacggagcgctggaaatcggcgaacgccgcaaactgggtcatagcctgcgtgaaaagcgctacgaccgcgcctacgtcttacccaactccttcaaatctgcattagtgcctttcttcgcgggtattcctcatcgcaccggctggcgcggcgagatgcgctacggtttactcaacgatgtacgcgtgctcgataaagaagcctggccgctaatggtggaacgctatatagcgctggcctatgacaaaggcattatgcgcacagcacaagatctgccgcagccattgttatggccgcagttgcaggtgagcgaaggtgaaaaatcatatacctgtaatcaattttcgctttcatcagaacgtccgatgattggtttttgcccgggtgcggagtttggtccggcaaaacgctggccacactaccactatgcggagctggcaaagcagctgattgatgaaggttatcaggtggttctgtttggctcggcgaaagatcatgaagcgggcaatgagattcttgccgctttgaataccgagcagcaggcatggtgtcggaacctggcgggggaaacacagcttgatcaagcggttatcctgattgcagcctgtaaagccattgtcactaacgattctggcctgatgcatgttgcggcggcgctcaatcgtccgctggttgccctgtatggtccgagtagcccggacttcacaccgccgctatcccataaagcgcgcgtgatccgtttgattaccggctatcacaaagtgcgtaaaggtgacgctgcggagggttatcaccagagcttaatcgacattactccccagcgcgtactggaagaactcaacgcgctattgttacaagaggaagcctgacggatgcgggttttgatcgttaaaacatcgtcgatgggcgatgttctccatacgttgcccgcactcactgatgcccagcaggcaatcccagggattaagtttgactgggtggtggaagaagggttcgcacagattccttcctggcacgctgccgttgagcgagttattcctgtggcaatacgtcgctggcgtaaagcctggttctcggcccccataaaagcggaacgcaaagcgtttcgtgaagcgctacaagcagagaactatgacgcagttatcgacgctcaggggctggtaaaaagcgcggcgctggtgacgcgtctggcgcatggcgtaaagcatggcatggactggcaaaccgctcgcgaacctttagccagcctgttttacaatcgtaagcatcatattgcaaaacagcagcacgccgtagaacgcacccgcgaactgtttgccaaaagtttgggctatagcaaaccgcaaacccagggcgattatgctatcgcacagcattttctgacgaacctgcctacagatgctggcgaatatgccgtatttcttcatgcgacgacccgtgatgataaacactggccggaagaacactggcgagaattgattggtttactggctgattcaggaatacggattaaacttccgtggggcgcgccgcatgaggaagaacgggcgaaacgactggcggaaggatttgcttatgttgaagtattgccgaagatgagtctggaaggcgttgcccgcgtgctggccggggctaaatttgtagtgtcggtggatacggggttaagccatttaacggcggcactggatagacccaatatcacggtttatggaccaaccgatccgggattaattggtgggtatgggaagaatcagatggtatgtagggctccaagagaaaatttaattaacctcaacagtcaagcagttttggaaaagttatcatcattataaaggtaaaacatgctaacatcctttaaacttcattcattgaaaccttacactctgaaatcatcaatgattttagagataataacttatatattatgttttttttcaatgataattgcattcgtcgataatactttcagcataaaaatatataatatcactgctatagtttgcttattgtcactaattttacgtggcagacaagaaaattataatataaaaaaccttattcttcccctttctatatttttaataggcttgcttgatttaatttggtattctgcgtttaaagtagataattcgccatttcgtgctacttaccatagttatttaaatactgccaaaatatttatatttggttcttttattgttttcttgacactaactagccagctaaaatcaaaaaaagagagtgtattatacactttgtattctctgtcatttctaattgctggatatgcaatgtatattaatagcattcatgaaaatgaccgcatttcttttggtgtaggaacggcaacaggagcagcatattcaacaatgctaatagggatagttagtggcgttgcgattctttatactaagaaaaatcatccttttttatttttattaaatagttgcgcggtactttatgttctggcgctaacacaaaccagagcaaccctactcctgttccctataatttgtgttgctgcattaatagcttattataataaatcacccaagaaattcacttcctctattgttctactaattgctatattagctagcattgttattatatttaataaaccaatacagaatcgctataatgaagcattaaatgacttaaacagttataccaatgctaatagtgttacttccctaggtgcaagactggcaatgtacgaaattggtttaaatatattcataaagtcacctttttcatttagatcagcagagtcacgcgctgaaagtatgaatttgttagttgcagaacacaataggctaagaggggcattggagttttctaacgtacatctacataatgagataattgaagcagggtcactgaaaggtctgatgggaattttttccacacttttcctctatttttcactattttatatagcatataaaaaacgagctttgggtttgttgatattaacgcttggcattgtggggattggactcagtgatgtgatcatatgggcacgcagcattccaattatcattatatccgctatagtcctcttactcgtcattaataatcgtaacaatacaattaattaagaataaacaagtttaagaagtgagttaaaactcacttcttatctatacaacttaatctctttactgaattagttaaagtttcagtatcgatatcttttaccgtatatgttggggatactatttgtatagatttatgatgattcggggaccaaattaaatgcgagggatattccggagtacgtgaattagggtaaaatgcaagcgttggtttatgataagccgcagcgatatgaacaagagctgtatcaacagaaatgacaaaatcactatacttggtcaacgcaacggtataaataaactcatcaaatggtagtgtttcgatttcaagtattggtattgtcaataaatcttgcggtaacccggtaaatataatccgataattttcaaagtgtgttttcacttcttgatatataacttttatttgctcaaacgtaagacggcatattttttttgcacctaatggattaataatgactattcttgtatctccaataaattcttttattttatcttcaacatctactggtaaatgcaagtcgtagttggtggaaaatttaccctcaccataaatatgcttcagtatttctattgctcgtgtactcatatgttcttttaaacattcatcgtggggatggtaaaatgaatagtaacgcttataccaatgatcaaaacccagaatgtaagaatcttttaaacttgataatattaagctatgcttaaatgagggcatagtttcaaaggggtctaatacaatatcgaactgtaaatcccgcagatgcttacatagagtaagcatttcaagaaaaccggttgattctttaatacagaactcaaatatatttttattattagagagaaattccccaccctttctatttgtgagaagagttattttaacccctttactataaagttcacgataaatcgaacttaatacaattagatcaccaagtttattattatcatgaataataaggcatgatttaacttgtgctggatctgtaatttgattatttattttattacgaaataaaaaagaaaggaaattaatcttgattttgtttatataaaatcttttctttttgtgaaaagttcctaagcgcatttttataccatattattttagtttcaggatgattaattagcataagaatcggttgaagttctatattgcattttttttcttgtcatatcttttgattcttctgcactgatgtcttgaagtttaataaatggaattacatcgtaagaaatagctgtatcatctgataaattataaatattaatatcttttacattatcatgcataaaacgaaaaaatggcaatattttgaataaatccctacttaattccgagggcatgggatttttattctcatcatagaaacgagaacagctacccgttaaatcaagaccagaacaaataatccgcgcatacttaagtgaatatgcgatttgaattgcagcaaaggcaatagtatggcatgagcaataaccaagactaatgtccttgcaaaatccaaccagacgaccttttttagacaacggtacagagatcagcagttctttgtgaatctgtctcaaaatattaaatttaatcttctttataaaaccacctttttcccgacggtaaaaggaccgtaatacgaggcagttctggaggatataaagtttatcttctttggaagcgtgttcataaacgtcaacgtttactatggtataacgacttctctggctaaatttataaaaatcatcacgacgctgatgtaaaaatcggacatctgtaagtacatatataaaaggaacgatattattacttaacagatattgcgcagaaccattgacagcaataatatcctttgttcgtaatactgacaaaggtgttttttgcgatgtagggcccgaaagaaaaataataacatcatcagatattttattttcaatcaggttttcaacatcttttttgtcaatgtatctaatattcttcatgataaacctgtgaaataaataactccgcttaaaactgtcctggtgaagacatgtaattgtgggattttttttagcgcgctggtttccctttcaaacgccgcataaaattgcgcatttttttacgatatactaaaagataatagcctagatctctaatctcatttttaataccgtaatgacgctctaagtcaatacgatctttcgctttacgctgcgctgaagcacgctttccggagagatcgataattcgaacctcaccattttttataatgaagttaccacgatgggggtcgccagaaaccatgccatgttgatgtaaggcattaattgattgctgaattttattttttagcgcatcatcaatatcgggcatatcacacaactctatgccatcaatatactcgatgatcatgatataagtatggacaaaacgtaaggttttccgttcagccaataaataaaagtcattgagtgtatttaacccttcatttcgtactttttgggtttgctcaaaaaggcgttcgtaataatcaccttttaacagagacttaaagaaacgttcgttacgcttaactttcggagaaaaaaccttaagaatcaatttaccgtaatcggtatcaataagcataacttttgtatcatcaatagaacgaaaaaccttgatgatatttatattataagacaagaagtcatttaatacattgaggtactttgaattgttttcatcggtaaaaacaaccaagtctttgatcttgctcttctgaatcataataaaccagttaaatgttatttacggtaatattttcggcaaagataacagactcctgctataattcctgagatataatgatgttgcactaaaagatgtttatatctttttttaaattcaataattgatttcgcatctcgtggagagtcatctttccagggggaattttctaaagctattttatagtattttaccgatggataaattgcccatttgtgccacggtttagttgcacctgtataatgaataagaagagtactttctgtaatcagctttttatagttttgatgtgttttgtcttttaattcacttttaattgtataaattgtattgtactcacgaggcaaaaataatgtcatccctttcagtaagacattcataacatcctgatcagggtatttataaacattatctttactcataagaatagacaacgctttttctgttagttttgcgtcagcccatttttttaagtctaaataaacgacaccggaattaaagtactgcccaagtaattcaggatcagacaacctggataccgccttttcttgcattggctcaacatctttaacaacagcagcaaccgctccatttaaacccagatgtaatagttggctaatatcgcctttacaaacaacatctgcatcaagataaagcaaacgatcaagcgttaaacccaataattgaaatgcaaataaacggaagtacattgctcttgaccagacctgtgtacaaggcaagcactggagcttatcagtgttaattctatataacgtgattcttaattggttttgctctgcaagctttgcaattttttgaaaaaaaccatcattataaacatcagcaataatataaaaatcaagattaatatgtcgattatttaggacaattgatgtgatggaaacacctacaccatcaagataattagcatcgacaccataggcaacatttaaacattcagaagtatttatattagctagccgaaaatcccaggctttaactttatctatctctatggcaggaaatgagtccacaatgctacccttatatcattactttatagtttcccagttttaatgctttatcttttcaataaaataaaaaagatagttgctaaatccttttagatatctatgctttttaagcatatgttttgcgctatatcttaattgattgctattgttcggtttcagcaacgccgtattcttccatggcgaagcattttttgcctccataaaggcttgtgatacaggataatcccaggcccaatcatgccagggcttggttggcccgatataatggataaaaatagtatcgttggttactgggtttataaagctttctttgagttgataatttaagctgaactgggtgttatatttaatatcagcgaaaataagtttatccgccagcaacatatttaacacatcctgatcaggatgtgttatttttttgattatttctggctcatttagcattgcaatagctcgtgcagaaacctgctgagccgcccattgggcagtattaatcaataaaaaaccggagttaaagtaacctttagcaattcccgcaacacctaacgaatgggcgcgtttttcccaccagtcagcttgcccttctgtaacaaccattgcgactttatcgtcaggaaatgagaaattaattagtggctcaatagtcccctgacaaatgatatctgcatccagataaaggactttaggcgccttattaataaagtaatctgcaataacaaaacgaaaatatattgcatgagtccaattcttagtgctaggcaatgagcgcagtcgatcaccattaatcagatatattttaattctggttttatactgcaacgccagggcatcaaaatacttacgatcatcatcaccaaaataatcagtaaaaatatggaaacacaatcgacttccttcattatattttaatattgaagcaatcgaaattccgcaaccaaatagaaagtttttgtcagttccataagcgatgtccagacaaagattttctgtttctactttatgatcataatcaataactgaattaagaaactcagtttcctggaaaaacacctgctgcattatttcctccgggaaatagcagaaataattaccttatgtaatctatcgtaatacttcgattggtaaaattcatcgatcgacgcaggaattttttcatgttcgatatgaatttcacctgctatatatttatttagaagagttacaaaaccagcaatatctcccggttgatacagatggccattgacatcaggttgaataatgtcagcaggcccggagacacaatcggcactgatacaaggaatcccccacgacaaggcttcaagtagggtcattgggaaaccttcaaaagatgacgtgagcaataacgcactcactttttcaatatcttgctggaccaattcccagggatattgttgccaaccataccagacaattcgatcatcaatatttaattctctaccataagcctggcatttttcgaaatcggagccatcacccaatacatggagtttccagttacctttcgcttgtgataagccatcaagcaggtctttaactcttttctggccttcaaatttcatacgcccaacataaataaacgttgccgtttcaccttcctcgggcgcgggaatgactgagtctttagtttcgacgggattaaaaataacatttatcgtcgattctgctacacctcgattaatcatttgctgtttaatgccagagctgattgctaaatgatagtcggcacaggtgatatattcagcatgttttttgtgatctaaagaaaaatgtggccatgaaaatactggcatatcaattcctgattttttacgtgcttttgcggcaaacaggcaggagatcacatcaatacaaataacgatatctggttggtactcctgaagccatttacttagagcatgaatatgtttcgcccgacgcaaaaaacctaaacgaatattggaaaatgaacatgagtatttaataccttccagccatcccttatccattttgtcattacgacaaaagaaaaacatttcactttggatatgttgttgcctgaaggtagtaataacatcacggatgacagtttccatgccgccaaatccagaaacagcttcgccgataaacgctattttcatagaaactctcattaattgagtaaaactcactgttttaacggttttatttgtctataaaatcagaaacaatcgttgacatcattttatctggactgaatttatataaactatcataatccattggtttaacagatgagttaataaaatactctaacttatcccaatcatcatgacctattataaaaaagcgagattcactatagatttctgaaccaaatacatttatattattagtaattaattttttattgaaaaatagtgcctcaagtatacgaagagtccagccagattggttttctttggttatatcaacaattatattagcatttaatgttcttctaatattctcttcataagatatttgtttttcaatcaaatactttgaagtcgtagatgatgtcttatctttgacaacattaaaatctagcttacatcctagtgttgttaatctctcggctaactcattaattatttgaagacgccctttatcacgaccaaggaaaaaacatattggctggctgttatttttgtcagataaactataatttctaatttcatccattcctataggaaaaaattgttctattgccttgatcttttcattccctataaatctatgctcaaaatcatatataatatcgaaataattcgcgttatcaagaataaaatcttcgccaacagtatttcttagaagcaaaactttatgacagttaatattttttaatatttgtttattgatacctttattaacaacactgtcattaatgataattatgtcatcttttttaatatcattgaggtaatgcttgatgaataatcgccccagccatgcattatccatccctatttttgatatttttttattaatccagttatatttttttggtgttgttatattttttatcttgtacttttttttcaggtactgaatcatttttaattcataatctgcaacccaatttataaaataaatagtcataataaagttagttccagtacatactaataaatatttttataatcctttgcgttgtgttcgctctttaatacgctcggccttaacgcttgccatgttcaataaattctgttcaagagacaatattttgcgtaaaggcatcccaaaataaaccttcataaatcgccagatatctctttgcgtcaggccaatattcattgatgagaaatataaaccaatcaggtctttatcgcgccagcggcgcggtacttttgcacgtatctgtgcccgatgcagatcgataactgaaatttttaattcatcttcccggccagtaaatggcaaatgaagcaaaaagtggcaaatgtaacagtcgcggtgatttatccctgcagtatgcattttacgcaccatagttgctacacgtgcgatcagcatacgcttaacacgtatatcaggcgggttgactgcccaatcggcacaataatcttcaaggctaattgtgggagtgagatcttcggtaataataaatgatgcgcgagttaatggatttaaccctttttcgccaaacccaatgcccttcattgtatcaacgccaacatcactcaggcgatgaatagcgtgccactctctgtctgcgcccaaaacgggcatccgcaatgagagtagattttttataatctcttttaatgtcgtccccttgtgccatttaagaaaatagcttttcccggacagttcaaagcgtaatgtacgacgagtctccagttcacgaaagacctcgccgttcagttttttgacctctgcaaaagcatctttaccacgccaaagtgtggcaagcggctcttttaattcaaccatctaaaccacctgtaatgatatccgcggctttttctggcaagctatacaaatcctgagtatcggcataatggcgagcattctccgcccaggccattcgcaatggcgactgagttaacgctttacgtaaaacttcatttaattgttcctgagagaaaggttcagcgatgaccgttccacaattggcatccgcaatataatgcgcgtacccacataccgctgttgttaaaacaggtaacccagcagtgatcgcttctagaagaacgatacccgcggcttcctgataagcgggatgcagtaataaatcagcggctgccattaattctgacacatcattgcgaccggagaagaaatgcacattgctccgcacgccgagtttttctgccagcgcttcaaattttcgcggcttatcctgaccaacaacaaataaaagcgtattgtgacgtaatgattccggtaacgatgccaaagcttcaattgagcgatctacacctttacggccaaaatctgatccaacctgcagtaataagttttgttgctcttttatgccatttttctggcgataaatttcacggctgtttgggatttgctcactgtattttctgtccggataaataccgggaggaagaatttgaaaacgttcaggttcagtttgataatgcttctggaaatcggcgatttgcttatcggtcagcatcataagtttcgtcgatttaccctgctcgaaagtcgctcgctcaaatgcggcataatggcgatatcgtgatgttaaacgatataaaaaacctttttcttgcgcaactttctcggcgtaacaaacatcagcggcaaaataaacatccaggccaggcatcttattaaacccaacaacgcgatctgcgggatgctctttgagatgattttgtacccaggcataatattctgcattgcgtccatggttggtatgggacttaactggcacctgaataagctcaaatgctttcgggcaatcgccttcccacgactgtgtatatacccgaacatggtggccccgtgcggcaactgttgatgcaatgcgcataaagtcacgttgaagcccaccaaatggaaaatatttatataaacaaaacgccacgatcataattgtgcattcctgtcagctgaaggggcatcttctggcaacagcttttccgtagcggcgatcacatcctccgctgggataacagaaagatattttttgttgcggtcaagttcatgccgggtcggcattttctgataattccccgcccagaattgaataatattctcggtccagggacgccagaatacgtgatccgttgcaccaaatagactaatgactggcgttttcactgccgctgcaatatgtcccggcgcagaatccacaccaataaaaagcactgcatgatcaattaatgcacccagttcaggaaaacgtgttttacctgcaaggccagtaatgggttttgtttcgcaacctcgtgcaatctcatctacacaagcgagatcatctgccgagggcccacaggttagcacaacctgatagcctcgctgttgcagcgcatcgataaccttagaaaatttatcgttatcccaacacttaaatatctgacgcgctgtcggttggatgacaacataatgatcttttacgcccagggcatctaattcccggcgcatcttcttccagcaatcttcggcgtaactcattgttgtgtcggtgtagaaatcggtaatacctaatggctcaaggaccgataaattacgctcaacaatatgtgtaccgtgtattggcgctaagtgtgtgaagctttttttccaaataccatgctgccgatgaccataaagttgcgatattttcatccgtgcaggtaaacaacgtaccagcagcgccaccatccactgatccgtaagattaatgaccaggtcataattattcgcacgcagagtttttatcaacgaaagcacatttttaattttatcgaaagttcccgcacctttattgcttatcccatagagcgcattaatttccgggttttcagacaaaatagggatggtgtcctgataaagcagcatatcgatttttgcatcaggataattctgcttgagcgtactgatgacaggagtagttaataacatatccccatgatatcgcatctttatgaccaggatttttcgaaatggcttttccactagcgactcttttgtgtgattgtctggttaagttaagcagaaaaaagcacgctaccgccccaggctcaacagctacctgaatactgataacgcacttactttgacgtgctagtgtatcatttctttcgcagcaatccgacccgaatgatttttatacacaaaatatactttaatcataaaaatcaaatagataaaaaatagcatttcgataatgtcagtacggcctatgtagatttgaaaatggggccgagtttcaatgaatcgcataaaaatacaaaaaaaatgaagatgtagcggcagatcagaccaaactgaagctatttaagtcaaaaacgggaaaagtaatggtaaagccacagctaaatacatagaatccccagcacatccataagtcagctatttactatgctcgaattgctttacaccgcccttctctaccttattcagccgctgatctggatacggctctgggtgcgcggacgtaaggctccggcctatcgaaaacgctggggtgaacgttacggtttttaccgccatccgctaaaaccaggcggcattatgctgcactccgtctccgtcggtgaaactctggcggcaatcccgttggtgcgcgcgctgcgtcatcgttatcctgatttaccgattaccgtaacaaccatgacgccaaccggttcggagcgcgtacaatcggctttcgggaaggatgttcagcacgtttatctgccgtatgatctgcccgatgcactcaaccgtttcctgaataaagtcgaccctaaactggtgttgattatggaaaccgaactatggcctaacctgattgcggcgctacataaacgtaaaattccgctggtgatcgctaacgcgcgactctctgcccgctcggccgcaggttatgccaaactgggtaaattcgtccgtcgcttgctgcgtcgtattacgctgattgctgcgcaaaatgaagaagatggtgcacgttttgtggcgctgggcgcaaaaaataatcaggtgaccgttaccggtagcctgaaattcgatatttctgtaacgccgcagttggctgctaaagccgtgacgctgcgccgccagtgggcaccacaccgcccggtatggattgccaccagcactcacgaaggcgaagagagtgtggtgatcgccgcacatcaggcattgttacagcaattcccgaatttattgctcatcctggtaccccgtcatccggaacgcttcccggatgcgattaaccttgtccgccaggctggactaagctatatcacacgctcttcaggggaagtcccctccaccagcacgcaggttgtggttggcgatacgatgggcgagttgatgttactgtatggcattgccgatctcgcctttgttggcggttcactggttgaacgtggtgggcataatccgctggaagctgccgcacacgctattccggtattgatggggccgcatacttttaactttaaagacatttgcgcgcggctggagcaggcaagcgggctgattaccgttaccgatgccactacgcttgcaaaagaggtttcctctttactcaccgacgccgattaccgtagtttctatggccgtcatgccgttgaagtactgtatcaaaaccagggcgcgctacagcgtctgcttcaactgctggaaccttacctgccaccgaaaacgcattgaggttgttatgcaaaaacgggcgatttatccgggtactttcgatcccattaccaatggtcatatcgatatcgtgacgcgcgccacgcagatgttcgatcacgttattctggcgattgccgccagccccagtaaaaaaccgatgtttaccctggaagagcgtgtggcactggcacagcaggcaaccgcgcatctggggaacgtggaagtggtcgggtttagtgatttaatggcgaacttcgcccgtaatcaacacgctacggtgctgattcgtggcctgcgtgcggtggcagattttgaatatgaaatgcagctggcgcatatgaatcgccacttaatgccggaactggaaagtgtgtttctgatgccgtcgaaagagtggtcgtttatctcttcatcgttggtgaaagaggtggcgcgccatcagggcgatgtcacccatttcctgccggagaatgtccatcaggcgctgatggcgaagttagcgtagcgtttatgccggatggtatgccatccggcgcgcatgaattacttctggcactgccgacaataaaacgttgcccgctgcgcatgtttagtcgccacaatcggcgtaccgcacacccgacacggctcaccttttcgcccgtaaacctgcaattcctgagcgaaatagcccggtttaccatcactttgcagaaaatctttcagcgttgtaccaccctgctcaatcgaacgcagcaacaccgctttaatcacccgagctaacaattcacactctgccagcgacagtgatgacgccagccgatccggatggatccccgccgcaaacagtgattcgctggcatagatattccctacccctaccaccagcttgttatccatcagccacggtttaatcgccgtttttttcttcgcgcacttctgatgcagatactcaccattgaaatcgtcgctaagcggctccggtccaagatgggtcagcacattatgcccttccagctctttggtccacagccaggcaccaaagcggcgcggatcggtgtagcgcagcactttgccgttgctcatcaccaaatccacatggtcatgcttttcagggggaagttcttctggaaggatgcgcaggctgccagacatccctaaatgaatgataatccagccctcaggcagctccagcagcagatatttagcccgccgctgcacgctaagcactggttggtcgcttaaacggtagatctcttctgaaaccggccagcgcaagcgtccgttgcgcaccactgcatgaagaatggttgcaccaacgagatgcggttctatgccgcggcggctggtttcaacttcgggtaattcaggcatagcatctccaggaatgaacagatgcagtcaatatgggggcaagcagataacaaaaaaccccgccggagcgaggttttttgttacatcaaagcgagaattatttgattttcgcttctttgtagatcacgtgctggcgaacaactggatcgaattttttcagttccagtttttccggcttagtacgtttgttcttcgtagtggtatagaagtgaccagtaccagcagaagaaaccagcttgattttctcacgaatacctttagccatgatttatttcctctaagtacttagtacttttcgccacgggcacgcagttcagccagaactgtatcgatgccttttttatcgattacacgcatacctttagcagatacgcgcagggtgacaaaacgcttctcgctctcaacccagaaacggtgagagtgcaggttcggcaggaaacggcgtttagtcgcgttcagtgcgtgggaacggttgttaccggtcaccggacgcttgccagtaacttggcagactcgggacatgtctattctccaaaaatcaaattagctcgagcttcgtatggggtattggcgcctcgtcaggctttacagcccggtcatcgcagttctatgtgaactctcgattgccaggcccaaatgccaaacccgagattctcaaaggtggcgtagtatacgctgactcagcgatgtgctcaagtcccgaacagacaaagatcccgaaggatcgcgcatagcgggttaaatccagccgcgttcggcaaaagaaacatactctccacgcccaatcacgatatggtcgagcacgcgtaaatccatgaactgacaactctttattatccgttcagtaatgagtttatccgctttactgggttcagcacaacccgaagggtgattatgtgcaaggatcagcgccgaggcgtttatttttatcgcttcgcggataatttcccgaggatggacttcaacatggtttagcgtgccggaaaaaagacgcctatgcgttataacccggtgttgggagtcgagaaagatcaccataaagatctcccgctcctcacccgtgagctggctttgtaaaaattccctcgtcatctccgggctgagtaaagggctttcttcacgcatccgcacgttgtagtaacgccgcgccagttcagcaatcccctttaactgggcaaatttcgccacgccaattccatgaacgccactaaattgttcatattcagaggttaacaagccataaagagagccgaaattctccagcatctcttttgccagggttaatacatctttaccgcgcgttccggtacgcagaaatagcgccagcagctcgacatccgttaaggcgctaataccaaacttcagcattttttcgcgcggcatcaacagctgtgaattgtttttcaccttcacctcctttgtggtgctcgcatcctgtcatagccgtttcgttaaatcgacggccagttttcaatcctggaaagcgcctcgcaaagtgaatctcaggtgaaggcacgacaacaaaagtattgtgataaaatcgccaacttctggtgtcaccctacaggaaaaatcatcatgagcctggccggtaaaaaaatcgttctcggcgttagcggcggtattgctgcctataaaacccctgaactggtgcgtcgtttgcgcgatcgcggggccgacgtccgcgtagccatgaccgaagcggcaaaagcctttatcaccccacttagcttgcaggcggtttctggttatcccgtttccgacagtctgctggacccggcagccgaagccgctatgggccatattgagctgggtaaatgggctgatttagtgattctcgcccctgccacggcagatttgattgcccgtgttgctgccggaatggcgaatgacctggtatcgacgatttgtctggctacacctgcgcctgtagccgtgctccccgccatgaaccagcagatgtaccgtgccgctgccacgcagcataatttagaggtgcttgcttcccgtggtttgctcatctgggggccagacagtggcagtcaggcttgtggtgatatcggtcctgggcgaatgctcgatccgttaaccattgtggatatggcggtagcgcatttttcgcccgtcaacgacctgaaacatctgaacattatgattaccgccggcccgacgcgtgaaccgctcgatccggtgcgttatatctctaatcacagctccggcaagatgggttttgctatcgccgccgccgctgcccgtcgtggcgcgaacgtcacgctggtatcaggtccggtttcactaccgacgccaccgtttgttaaacgtgttgatgtgatgaccgcgctggaaatggaagccgccgtgaatgcttctgtacagcagcaaaatatttttatcggctgcgccgccgtggcggattatcgcgcagctaccgtggccccagagaaaatcaaaaagcaggccacgcagggtgatgaattaacaataaaaatggttaaaaaccccgatatcgtcgcaggcgttgccgcactaaaagaccatcgaccctacgtcgttggatttgccgccgaaacaaataatgtggaagaatacgcccggcaaaaacgtatccgtaaaaaccttgatctgatctgcgcgaacgatgtttcccagccaactcaaggatttaacagcgacaacaacgcattacaccttttctggcaggacggagataaagtcttaccgcttgagcgcaaagagctccttggccaattattactcgacgagatcgtgacccgttatgatgaaaaaaatcgacgttaagattctggacccgcgcgttgggaaggaatttccgctcccgacttatgccacctctggctctgccggacttgacctgcgtgcctgtctcaacgacgccgtagaactggctccgggtgacactacgctggttccgaccgggctggcgattcatattgccgatccttcactggcggcaatgatgctgccgcgctccggattgggacataagcacggtatcgtgcttggtaacctggtaggattgatcgattctgactatcagggccagttgatgatttccgtgtggaaccgtggtcaggacagcttcaccattcaacctggcgaacgcatcgcccagatgatttttgttccggtagtacaggctgaatttaatctggtggaagatttcgacgccaccgaccgcggtgaaggcggctttggtcactctggtcgtcagtaacacatacgcatccgaataacgtcataacatagccgcaaacatttcgtttgcggtcatagcgtgggtgccgcctggcaagtgcttattttcaggggtattttgtaacatggcagaaaaacaaactgcgaaaaggaaccgtcgcgaggaaatacttcagtctctggcgctgatgctggaatccagcgatggaagccaacgtatcacgacggcaaaactggccgcctctgtcggcgtttccgaagcggcactgtatcgccacttccccagtaagacccgcatgttcgatagcctgattgagtttatcgaagatagcctgattactcgcatcaacctgattctgaaagatgagaaagacaccacagcgcgcctgcgtctgattgtgttgctgcttctcggttttggtgagcgtaatcctggcctgacccgcatcctcactggtcatgcgctaatgtttgaacaggatcgcctgcaagggcgcatcaaccagctgttcgagcgtattgaagcgcagctgcgccaggtattgcgtgaaaagagaatgcgtgagggtgaaggttacaccaccgatgaaaccctgctggcaagccagatcctggccttctgtgaaggtatgctgtcacgttttgtccgcagcgaatttaaataccgcccgacggatgattttgacgcccgctggccgctaattgcggcacagttgcagtaatatgacgccggatgacttttcatccggcgagtttctttaaacgccaaactcttcgcgataggccttaaccgccgccagatgttccgccatttccggcttctcttccaggtaagcaatcaggtctttcagggtgatgatagagatcactttgcagttgtaatcacgctcaacttcctgaatcgccgaaatctcgccgcgcccgcgttcctgacgatcgagcgaaatcaacacgccagcaagcgtcgcgccattggcctgaataatctccatcgactcgcgaatcgccgttccggcggtgatcacatcatctaccagcattacgcgtccttgtaacgcgctaccaaccagattgccgccttcaccgtggtcttttgcttctttgcggttaaagcagtacggcaggtccaggtcgtgatgctccgccagtgccacagcggttgtggtggcaatcgggatccctttgtaagcagggccaaacagcagatcgaactcaatgccggaatccaccaacgcttcagcgtaaaaacggcctaacagtgccagatcgcgcccggtattaaacagcccggcgttgaagaaataggggcttttgcgcccggatttcagcgtaaactcgccaaactttaacacctgcttgctaagcgcaaattcaataaactggcgctgatatggtttcatgccttcgctcctcatcttacttttctacagacaaaaaaaaggcgactcatcagtcgccttaaaaatcagtttgccagcgccgccttctgcgtcgctacaatggattcgattcccctcgggccagagccaacaagatgagtagctcttcatgggtgaacggctcgccttctgccgtcccctgcacttcaatgatgcgcccgtcttcggtcatcactacgttcatgtcggtctctgcggcagagtcttcaacgtattccagatcgcaaaccgcttcgccgttcacaattccgacagaaactgcggctaccatccctttcatcggattggttttcagcttgccgttttccaccagcttctgtagcgcatctaccagcgccacgcaggcacccgtaatcgacgcggtacgcgtgccaccatcagcctgaagcacgtcgcagtccagcgtaatggtgaactcacccagcgctttcaaatctactgccgcgcgaagagcacgggcgatcagacgctggatttccattgtgcgtccaccctgcttacctttcgccgcttcacgagcgttacgggtgtgggtagaacgtggcagcatgccgtactctgcggtgatccagccctggccctgacctttcaggaagcgcggcacgccttcttcaatagaggcggtacacaacactttggtatcgccaaattcgaccagcaccgagccttctgcatgttttgtatagttacgagtcagggtaacgggacgcacctgattattgctacggcctgctggacgcatattgaaatctccggcttgaaacaaatgtggctgcgcattatacggacttccggcggttattcctatcctgacaaggcatcgatggctataatccttccacctctccttttataaacaggaacgtctatgatccgcagtatgaccgcctacgcccggcgtgaaatcaagggtgaatgggggagcgcaacctgggaaatgcgctcggtaaaccagcgttatctggaaacttactttcgtctgccggagcagttccgtagccttgaacctgtcgttcgcgagcgtattcgttctcgcctgacgcgcggtaaagtggaatgtaccctgcgctatgagccagatgttagcgcgcaaggtgagctgatcctcaacgaaaaactggctaaacagctggtaactgccgcgaactgggtaaaaatgcagagtgacgaaggggaaatcaacccggttgatattctacgctggccgggcgtgatggcagcccaggagcaggatcttgacgccattgccgctgaaattctcgcggcgctggatggtacgctggacgactttattgtcgcgcgcgaaaccgaaggtcaggcactgaaagcattgatcgagcagcgtctggaaggcgtcaccgccgaagtggtcaaagtccgctcccatatgccggaaatcctgcaatggcagcgtgagcgtctggtcgcgaagctggaagatgctcaggtgcaactggaaaacaaccgtctggagcaggaactggttctgctggcacaacgaattgacgttgccgaagaactggatcgcctcgaagcgcatgtcaaagagacctacaacattctgaagaaaaaagaagcggttggtcgtcgtctggattttatgatgcaggagttcaaccgcgagtcgaacactcttgcgtcgaagtctatcaatgccgaagtgacaaactccgccatcgagctgaaagtgttgattgagcagatgcgcgagcagattcagaacatcgaataactcgtaacgccaattcttacttttccgccttcacaaatgccgccactcaaacagagcggcatttttcttccccgcaacattcaattctgttttgcgtgcctgctccagattttgcgatgtttttttgcccagcacactgagaacgtgagatactcacaactgtatataaatacagttacagatttactttctttgcaattgatatcacatggagtgggcaatgaacgaacatcatcaaccttttgaagagataaaactgattaatgcaaacggagcagaacaatggtcagcaagacaacttgggaaactactgggttattcagagtatcgtcactttatacctgtattaacgcgcgccaaagaagcctgtgagaacagtggtcacacaattgatgaccatttcgaggagatcctcgatatggtcaaaattggctcaaatgccaaaagagcattaaaagacatcgtactctcccgctatgcctgttacctggtagtacaaaacggcgaccctgcgaaaccggtcattgcggcagggcagacttattttgctatccagacccgacggcaggagcttgctgacgatgaagcatttaagcaacttcgtgaagacgaaaagcgtctgtttctgagaaatgagttgaaagaacataacaaacaattggttgaggcagcacagcaagctggggtagcgacagctactgatttcgccatatttcagaatcatggttaccaggggctgtatggtggattagatcagaaagctattcatcagcggaaggggctgaaaaagaatcagaagatcctggatcatatgggttcaacagaactggcggctaatctctttcgagctacccaaacagaagaaaaactcaagcgggatggcgtgaattcaaaacagcaagcaaacaccacacactttgacgtgggtcgcaaggtgaggcaaaccattcaggaacttggcggaaccatgcctgaggagttgccgaccccgcaggtcagcatcaagcagttggaaaacagtgtaaaaattacagagaagaaatagcagaaactaaaaactctttttgttgattgagacacccgatgcgtaagccaaggtccaggtgcagtgaacacaatggctaaatattgcacctttcttttccccctcagttttaacctattttttcttatgcattttctcagacaagaagtcagaagaatgcatctctgctacagaaaatagcgatttcacataactacaagttatcaatttcccctccccttaaaaaatctcaatcgtgacaatgcgcacaaatcgctaccctgccagacagatttttagggagagaaccatgctgttacacattttgtatttggttggcattactgccgaagccatgacgggggcgctggcggccggacgacggcgcatggatacatttggcgtaattattattgcgaccgccaccgcaattggcggagggtcagtgcgcgatattctgctgggccactatccgctcggctgggtcaaacacccggaatatgtgattatcgtcgctaccgccgcagtactcaccactatcgttgctcctgtaatgccttacctgcgcaaagtgtttctggtgctcgatgcgctcggactggtggtcttttctatcatcggggcacaggttgcactggatatggggcacggcccaattattgccgttgtcgcggcggtaaccaccggcgtgtttggcggcgttttgcgcgatatgttctgtaaacgtatcccactggtattccagaaagagttgtatgccggtgtctcatttgcctccgccgtgctgtacatcgcgctgcaacactatgtttctaaccatgatgtggtaattatctccaccctggtattcggcttttttgcccgcttactggcgctacgccttaagctgggattaccggtcttttactacagccacgaaggacactaaggttcaaaacctgtgatctgctgggcagccagccaactgcccagcttcttgatttgcgcattttccttccattcaataacctgtctggcgcgtcccgatccagtccccggcagctgctgccagaactgctccgtgctaaataaaagttgcgaccaggaccgttcatcactggcattaagcgccgcccgggttagcggtattcccattgccatcacccagcgagtaaaaggctgcttacgagccagattaaactgatgccatagctgcgcacttttacttttcgcgatccccggcgtgttctgtaattgctctggcgttaataaaagccaggaaaagatatgttcaaagcgatgagtctgatgcagcgcgcgccaaccggcctcaccaatgccatccagcccaagaacctgttttgcccccagccagactaagcgtgaaatgaactgttcctgacaaacatcagaagcaaagtagcaggtcaacgagttaaagcggttttctggcggtgtcggttttgtacgttctgcaccgcgccacaccacatcatcaatgcgaggaataccctgaccggcaaggctgacgagaatctgatcaccaggcgcaatatcccactcctgccagcgcctgacggaaccaatattcacccgctggacttttttatcatccagcatgacaggtgcgagtgacgcaaccaccgatattttaccgctcttacccaccgcaaactgaattgccttcacttcggcaacctgagctacaggttgatatttccaggccaccagccactctgcctggcccggtagccaatggcgggattctggctctttcgccgctcgtacaactacgccatcggtgacgaagggtaattccgctttccaccactcattgcgtacgcgcgcaacttcatcagcatttttcaccgcacgggtatacgtctgcgttagagtaaaacctgcggtagccagctcttttaaacgatcagacattaactgcggtccatccggccatgcccagacaaaaacgcccagagaattcagcgtgtcgctatcgtcctggcgcatcatcaagccagcaacttttgcgcgggcatttattccccccatttgttgttggatatgcccctcgcgctggagaaatatttccccctgaagcgtactgttggctaaaggcccgctaacggtttgcggcacagcggaaattaagctaactttctgcgtccagtcctcgcctttcaggccattaccgcgactgattgctttgttcagtttcccgtcccgataaaccagggttaccgcaacgccatcaacttttggctgcacccaaagatcgctacgttctcgcatccacagacttaatgcgtttttatccaccattttgcgtacacccgtatgggcaaccggatgcataaccgcaccatttaaaggcggcatcatcacgtcgcggggctcgctcccaaagcagcgttgccactgcgtaagacgggcgcttaactgatcgtaaacaccgtcttccacctcactttttccttccttccagtagtcatcgtcccactgttttatttgctgttgcaggcgggaaatttcttcctgtgctctggctggcgaccaggccggacagaccgcccacacagatgattgccagcacaagatacctattaatatcgccatccatactttcatcatcacctccgctgtagatagtcaggcagatatacaacgtgatgaaagcaaagccgagtggcaaaaacggagtctgcgaggacgcttcctgaaaatcgtctttattgcagtgaatgacaggcaaatgcggaagcagctacgcaaaacgcaacaactttgcgcaaaaagtgtgagcaagggctacgtcacatggccgcgccgtgtataataagctcgtatgtaggctttatttcgctaatcacatacgaaagatactcatggctcaaggcacgctttatattgtttctgcccccagtggcgcgggtaaatccagcctgattcaggctttattaaaaacccaaccgttgtatgacacccaggtttctgtttcacacaccacacgccaaccgcgtcctggtgaagtccacggtgaacattatttctttgttaatcatgatgaatttaaagaaatgattagcagagatgcgttcctcgaacacgcagaagtttttggtaattactatggcacttcgcgtgaggccattgagcaagtactggcgaccggtgtcgatgtttttctcgatatcgactggcagggcgcgcagcaaattcgccagaagatgccgcacgcgcggagtatctttattttaccgccgtccaaaattgaactggaccgccgtctacgcggtcgcggtcaggacagcgaagaggtcattgcaaagcgtatggcgcaagctgttgcagaaatgagccattacgccgaatatgattatctgattgtgaatgatgacttcgataccgcgttgaccgatttgaagaccattattcgcgccgaacgtctgcgcatgagccgccaaaagcagcgtcatgacgctttaatcagcaaattgttggcagactgaacctgatttcagtatcatgcccagtcatttcttcacctgtggagctttttaagtatggcacgcgtaactgttcaggacgctgtagagaaaattggtaaccgttttgacctggtactggtcgccgcgcgtcgcgctcgtcagatgcaggtaggcggaaaggatccgctggtaccggaagaaaacgataaaaccactgtaatcgcgctgcgcgaaatcgaagaaggtctgatcaacaaccagatcctcgacgttcgcgaacgccaggaacagcaagagcaggaagccgctgaattacaagccgttaccgctattgctgaaggtcgtcgttaatcacaaagcgggtcgcccttgtatctgtttgaaagcctgaatcaactgattcaaacctacctgccggaagaccaaatcaagcgtctgcggcaggcgtatctcgttgcacgtgatgctcacgaggggcaaacacgttcaagcggtgaaccctatatcacgcacccggtagcggttgcctgcattctggccgagatgaaactcgactatgaaacgctgatggcggcgctgctgcatgacgtgattgaagatactcccgccacctaccaggatatggaacagctttttggtaaaagcgtcgccgagctggtagagggggtgtcgaaacttgataaactcaagttccgcgataagaaagaggcgcaggccgaaaactttcgcaagatgattatggcgatggtgcaggatatccgcgtcatcctcatcaaacttgccgaccgtacccacaacatgcgcacgctgggctcacttcgcccggacaaacgtcgccgcatcgcccgtgaaactctcgaaatttatagcccgctggcgcaccgtttaggtatccaccacattaaaaccgaactcgaagagctgggttttgaggcgctgtatcccaaccgttatcgcgtaatcaaagaagtggtgaaagccgcgcgcggcaaccgtaaagagatgatccagaagattctttctgaaatcgaagggcgtttgcaggaagcgggaataccgtgccgcgtcagtggtcgcgagaagcatctttattcgatttactgcaaaatggtgctcaaagagcagcgttttcactcgatcatggacatctacgctttccgcgtgatcgtcaatgattctgacacctgttatcgcgtgctgggccagatgcacagcctgtacaagccgcgtccgggccgcgtgaaagactatatcgccattccaaaagcgaacggctatcagtctttgcacacctcgatgatcggcccgcacggtgtgccggttgaggtccagatccgtaccgaagatatggaccagatggcggagatgggtgttgccgcgcactgggcttataaagagcacggcgaaaccagtactaccgcacaaatccgcgcccagcgctggatgcaaagcctgctggagctgcaacagagcgccggtagttcgtttgaatttatcgagagcgttaaatccgatctcttcccggatgagatttacgttttcacaccggaagggcgcattgtcgagctgcctgccggtgcaacgcccgtcgacttcgcttatgcagtgcataccgatatcggtcatgcctgcgtgggcgcacgcgttgaccgccagccttacccgctgtcgcagccgcttaccagcggtcaaaccgttgaaatcattaccgctccgggcgctcgcccgaatgccgcttggctgaactttgtcgttagctcgaaagcgcgcgccaaaattcgtcagttgctgaaaaacctcaagcgtgatgattctgtaagcctgggccgtcgtctgctcaaccatgctttgggtggtagccgtaagctgaatgaaatcccgcaggaaaatattcagcgcgagctggatcgcatgaagctggcaacgcttgacgatctgctggcagaaatcggacttggtaacgcaatgagcgtggtggtcgcgaaaaatctgcaacatggggacgcctccattccaccggcaacccaaagccacggacatctgcccattaaaggtgccgatggcgtgctgatcacctttgcgaaatgctgccgccctattcctggcgacccgattatcgcccacgtcagccccggtaaaggtctggtgatccaccatgaatcctgccgtaatatccgtggctaccagaaagagccagagaagtttatggctgtggaatgggataaagagacggcgcaggagttcatcaccgaaatcaaggtggagatgttcaatcatcagggtgcgctggcaaacctgacggcggcaattaacaccacgacttcgaatattcaaagtttgaatacggaagagaaagatggtcgcgtctacagcgcctttattcgtctgaccgctcgtgaccgtgtgcatctggcgaatatcatgcgcaaaatccgcgtgatgccagacgtgattaaagtcacccgaaaccgaaattaatgttttatgaacccaacacgttatgcacgcatctgcgaaatgctcgccaggcggcagcctgatctgaccgtctgcatggagcaggtccacaaacctcataacgtttctgcgattattcgtaccgcagatgccgttggcgtacatgaagttcacgccgtctggcctggtagccgcatgcgcaccatggcttcggcagcggcgggtagtaacagctgggtacaggtgaaaacacaccgcaccattggcgatgccgtcgctcatctcaaaggccagggcatgcagattctggcaacccatctttctgataacgctgtcgatttccgcgaaattgattacactcgcccgacctgcattttgatgggacaggagaaaacgggcatcacgcaggaagcattggccctggcggatcaggacatcatcattccgatgatcggcatggtgcagtcgctgaatgtttccgttgcctcagccctcattctttacgaagcccagcgtcagcggcaaaatgcaggcatgtacctgcgtgaaaacagcatgttgccggaagcagagcaacaacgcctgttgtttgaaggcggctatccggtgctggcgaaagtcgcaaaacgcaaaggcctgccttatccccacgtcaatcagcaaggcgagatcgaagctgatgccgactggtgggctactatgcaggctgcagggtaagtgccatgaaaggtcgcctgttagatgctgtcccactcagttccctaacgggcgttggcgcagcacttagtaacaaactggcgaaaatcaacctgcataccgtgcaggatctactcttacaccttcccctgcgctacgaagatcgcacccatctctaccccatcggagaactactgccgggcgtttatgccacggtggaaggcgaagtgctgaactgcaatatctccttcggcggtcggcggatgatgacctgccagatcagcgacggttccggcatcctcaccatgcgctttttcaatttcagcgcggcaatgaaaaatagcctggcggcgggccgccgtgtactggcttatggcgaagcaaagcgcggtaaatatggtgcggagatgatccacccggaataccgcgtgcagggcgatctcagcacgccagaattacaggaaacgctcacgccggtttatccaacaacggaaggcgtaaagcaggccacgctgcgtaaattaaccgaccaggcgctggatctgctcgacacctgcgccattgaagaactcctgccgccggaactgtcacaaggaatgatgacgctaccggaagcgttgcgcactttgcaccgcccgccaccgacgctacagcttagcgatctggaaaccgggcagcatccggcgcaacgtcgtctgattctggaagaactgctggcgcacaacctcagcatgttagccttacgtgccggagcacagcgttttcatgcccagccgctgagcgccaatgacacgctgaaaaataaactcctcgccgccttaccgttcaagccaacgggcgcacaggcacgcgtagtggcggagatcgagcgcgatatggcgctggatgtgccgatgatgcgtctggtgcagggcgatgtaggttccggtaaaacgctggtcgccgccctcgccgcgttgcgtgcgattgcccacggcaaacaggtagcattgatggcaccaaccgaattactcgccgagcagcacgccaataacttccgcaactggtttgcaccgctcggtatcgaagtgggctggctcgccggtaagcagaaaggtaaagcacggctggcacagcaggaagccatcgccagcggtcaggtgcagatgattgtcggtacacacgccatcttccaggaacaggtgcagtttaacggcctggcgctggtgattatcgacgaacagcatcgttttggcgtgcatcagcgtctggcattgtgggagaaaggccagcagcagggcttccatccgcatcagttgatcatgaccgccacgccgatcccccgcacgctggcaatgactgcgtatgccgatctcgatacctcggtgatagatgagctgccgccaggccgcacgccagtgactacggtcgctattcctgatacccgccgtaccgacatcattgaccgcgtgcaccacgcctgcataactgaaggtcgtcaggcatactgggtttgtacgttgattgaagagtcggaattgctggaagcgcaggcggcggaagctacctgggaagagttgaaactggcgctaccagagttgaacgttggcctggtacacgggcggatgaaacctgccgagaaacaggcggtgatggcgtcgtttaaacaaggtgagctacacctgctggttgccacaaccgttattgaagtcggcgttgatgtgcctaacgccagtctgatgattatcgaaaacccggagcgtctgggtctggcgcagttacaccagctgcgcgggcgcgtaggtcgtggcgcggtggcttctcactgcgtgctgctctacaaaacgccgctttctaaaacggcgcaaattcgcctgcaagtgctgcgcgacagtaacgacggttttgtgattgcgcaaaaagatctggagattcgcggccctggcgaattgttaggcacgcgtcagacgggtaatgctgaatttaaagtggcggatttactgcgcgatcaggcgatgatcccggaagttcagcgcctggcacgccatattcacgaacgttacccacaacaggcaaaagccctgatagaacgctggatgccggagacggaacgttactcgaatgcgtaaaaggcggcagtgagaagaccgccatttcaggttaccctaccttcctgccggatgcgattcatcaccctacaaattcaataaattatgaatcaatacgcaggcttgataagcgaagcgtatcaggcatttgtctttgttgcggcggcacttctaccgccgcttcatcggttaaccggcaaaaatcggcaacatcaaatacaacttaattaccagcgcattgacgatatcgataaagaacgcaccgaccatcggcaccaccaaaaacgccatgtgcgacgggccaaagcgttcagtgatcgcctgcatgttggcgattgccgttggcgttgcaccgaggccaaaaccacagtgacccgcagccagcactgccgcatcgtagtttttgcccatcatgcgccaggtaacgaagatggcatacaacgccatgaagatggtctgtaccaccagaatcgccagcatcggcagcgccagcgaagccagctcccacagtttcagccccatcaacgccatcgccaggaacaacgacaagcttacgttacccagcacggataccgcacgctcaaagacgcggtaaaagcccattattgacagaccgttgctcagaatcacgccaacaaacagtacacagacgaaggtcggcagttcaaaagcagtgccagccaaaagttgcgcaacaattttccccaccgtcaggcagatagcaatcagcgcgatagtttcaatcagcaccaacgaggtgatcatgcgtcccacatccggcttttcaaacgccgtcgggacttcctggtcatccggaataccgttcggcgtggtggagtgtttcaccagatagcgcgccaccggaccgccaatcaagccgcccagcaccagaccgaacgttgcacaggccatcgccacttccgtcgcattggtgaagccataacgttcaatgaacaatttactccacgcagcgcccgtaccgtgaccgccggaaagagtaatagaaccggccaacagccccatcagcggatcaagccctaacaagctagccataccaatgccaatggcattttgcatcaccaacagaccaacaaccacaatcaagaagatgccaaccacacgcccaccggcacgcaaactggcaatgttggcgttcaggccaatggtggcgaagaaagccagcattaacggatcgcgcagggacatatcaaagttgacttcccagcccatgctttttttcagtactagtagcgccagcgccaccaacaaaccacccgcaacaggttccggtatggtgtatttcttcaaaaaggagacggaatggaccaacttacgcccgagcagcaacgtcagcgttgcggcaacaagcgttgctaaagtatcgagatgaaacatagttactcctttgtatccgcatcactctttcatactcgtcatacttcatcgcgcagtggcaacttcatgaactatgacgggtatcgagttatgctttcctgggtcaaattctcagctgttaatgaacaaatggcatggattttaagcagaaaaataccaaaagttatataaaaaagtgcatttatctcatttaaatatttagatgaggatgtggcaaacgtttgcttttctctttcggtcagctaaaatgcccgctttgctaccacgggattgttttcgatgtctgtttccaccctcgagtcagaaaatgcgcaaccggttgcgcagactcaaaacagcgaactgatttaccgtcttgaagatcgtccgccgcttcctcaaaccctgtttgccgcctgtcagcatctgctggcgatgttcgttgcggtgatcacgccagcgctattaatctgccaggcgctgggtttaccggcacaagacacgcaacacattattagtatgtcgctgtttgcctccggtgtggcatcgattattcaaattaaggcctggggtccggttggctccgggctgttgtctattcagggcaccagcttcaactttgttgccccgctgattatgggcggtaccgcgctgaaaaccggtggtgctgatgttcctaccatgatggcggctttgttcggcacgttgatgctggcaagttgcaccgagatggtgatctcccgcgttctgcatctggcgcgccgcattattacgccgctggtttctggcgttgtggtgatgattatcggcctgtcgctaattcaggttgggttaacgtccattggcggcggttacgcagccatgagcgataacaccttcggcgcaccgaaaaatctgctgctggcaggcgtggtcttagccttaattatcctgcttaaccgtcaacgtaacccttacttacgcgtggcctcactggtaattgcgatggcggccggatatgcgctggcgtggtttatgggcatgttgccagaaagcaacgaacctatgacgcaagaactgattatggtgccaacgccgctctattacggtcttggcattgaatggagtctgctgctgccgctgatgctggtctttatgatcacttcgctggaaaccattggcgatatcacggcgacctctgacgtttccgaacagccagtgtccggtccgctgtacatgaaacgcctgaaaggcggcgtgctggcaaacggcctgaactcgtttgtttcggcggtgtttaacaccttcccgaactcctgcttcgggcaaaacaacggagtgatccagttgactggtgttgccagccgctatgtcggttttgtcgtcgcgctgatgttgatcgtgctgggtctgttcccggcagtgagcggttttgtacaacacattccagaaccggttctgggcggcgcaacgcttgtaatgtttggcaccatcgccgcctccggtgtgcgtatcgtttctcgtgagccgctgaaccgtcgggcgattctgattatcgcgctgtcgctggcggttggtctgggcgtgtctcagcagccgctgattttgcagtttgcccctgaatggctgaaaaacctgctctcctccgggatcgccgcgggcggtattactgccatcgtgctgaatctgattttcccaccagaaaaacagtaattcactggcggcggtaagataattaccgccgcagtctcacctctttaaccattcccgccttgaggattgcgcgtaaatcgtgcataactcccttatgtgcatttcacgggatggaagaccatgaaatttattgggaagctgcttctctacattctcatcgctctgttagtggcgatcgctggcctctattttcttctgcaaacccgctggggagcagaacatatcagcgcatgggtttccgagaatagcgactatcatctggccttcggggcgatggatcaccgtttttccgcgccatctcatatcgtgctggagaacgtcacgtttggtcgtgatggccagcccgcgaccctggtggccaaaagtgtcgacattgcgctaagcagtcggcaactgaccgaaccacgccatgtcgataccatcctgctggaaaacgggacgctgaatctcaccgaccagaccgcgccgctaccgttcaaagccgatcgtctgcaactgcgtgatatggcgtttaatagcccgaatagcgaatggaaactgagcgcgcagcgggtaaatggcggcgtagttccgtggtcaccaaaagccggtaaagtgctgggtacgaaggcgcagattcagtttagtgccggatcgctttcgctcaatgatgttcctgccaccaatgtactgattgaaggcagtattgataacgatcgcgttacgctgactaacctgggtgccgacatcgcccgcgggacattaaccggaaacgcgcagcgtaacgccgacggcagctggcaagtggaaaacctgcgcatggcggatatacgtctacaaagcgaaaaatcgctaaccgacttctttgcgccattacgctctgtcccgtcgttgcagattggtcgcctggaagtgatcgatgctcgtttgcaaggtccggactgggcggtgaccgacctcgatctcagcttgcgcaacatgaccttcagtaaagatgactggcagacacaggaaggcaaactgtcgatgaacgctagcgagttcatttatggttcgctgcatttatttgacccgattataaacacggaattttccccgcagggcgtagcgctgcgccagttcaccagccgctgggaagggggtatggtcagaacgtcagggaactggctgcgtgacgggaaaacgttgatccttgatgatgcggcaattgccgggctggaatataccttgccgaaaaactggcaacagttgtggatggaaacgacacccggttggttaaacagcctgcaactgaagagatttagcgccagccgcaatctgatcattgatatcgaccctgacttcccgtggcagctcaccgcgctcgatggttacggtgccaacctgacgctggttaccgatcataaatggggcgtctggagtggctcggcgaatctgaatgccgccgccgcgacattcaatcgtgttgatgttcgtcgcccgtcgctggcgctgaccgccaacagcagcacggtgaatatcagcgaactgagtgcatttactgaaaaaggcattctggaagccaccgccagtgtttcacaaacgccacaacgtcagacacatatcagcctgaatggacgcggtgtgccggtgaatattttgcaacagtggggatggcctgaattaccgttgactggcgacggcaatattcagcttaccgccagtggcgatattcaggccaatgtcccgttgaaacctacggttagcgggcaattgcatgccgtgaacgccgcaaagcagcaagtgactcaaaccatgaatgctggcatcgtttccagcggtgaagttacatcgacggagccggtgcggtaaacatcaatctcgccgggtacgactcagacgtacccggcattccatcaatagattacaacgtaattgtcagcgcattcccttgaggcttcaccaccagcccctgctcactttcagcctgcgaaccgtcttgcagaccatttactttcacaacattgcgcaggcacagtgtccagttcttcgcctcgcccgcaccagtcacagtaatcgtgttgccagtacgtgctgcttttaaagtaaagatcaccgatccgtcagcagcgggcacttcacagacggcttcatgcccgtcttgcagattgaagaggtggaatgccgtgccttcgtgccacacgtaatcgggacgttgatcgttgttgcccagcgccagtagagtgttatcacgcacataaacgggcagactcaggaagccgtgctgctgtttatgccagcgactaccgtcgagttcatcgttgtgccacaggtgtgtccagcgaccttccggcaggtagaactgcacatcgcccgcttcagtgaacaccggcgcaaccatcacgttgtcgcctaacatgtattgacggtcaaggtaatcacaagccggatcgtccgggaactccatcatcatggcccgcatcatcggcgtaccccgcgcgttcgcacgcgcagcttcacgatacagatacggcatcatgcggcatttcagttgcgtgaagaagcgcaccacatcacaggactcatcatcgtaggcccacggcacacgataagatttgctaccgtgtaaacggctatggctggagagcaaaccaaacgcgcaccagcgtttgtaaacgtgcgccggagcggtattttcaaagccgccgatatcgtggctccagaagccaaaacctgaaaggccaatagacaaaccaccgcgcaggctttccgccattgattcgtagttagcgtaacaatcgccaccccagtgtaccgggaatttctgcgcaccgacggaggccgagcgggcaaacaagacagcttcttcctcaccaacggtgtccttgagcacgttccacaccagttcgttgtagatgtacgcataatggttatgcattttctgcggatcggaaccgtcaaaccactgaacatcagttgggatacgttcgccaaagtcggtcttaaagcaatcaacgcccatcgcgaccagacctttcagtttgtcggcgtaccatttgcaggcatccggattggtaaagtcataaatcgccagacctggctgccatttatcccactgccatagcgaaccgtccgggcgtttgagtaaatagcctttctcttgtaactctttaaagacgggggatttttgaccgatataggggttaatccagacgcagattttcagtcctttcgctttcaggcggcggatcatcccttccgggtcagggaaagtcagcgggtcccactcaaaatcgcaccactggaaggctttcatccagaaacagtcaaagtggaaaacatgcagcggcagattgcgttccgccataccatcgataaagctgtttaccgtcgcttcgtcgtagttggtggtaaatgaagtggttagccacaggccgaaggaccacgcgggcggcagcgccggacgaccagtaaagcgggtataacgatcaagtaccgctttcggcgtcgggccgtcgataacaaagtattcgagatattcactctcaacgctgaactgcactttggagactttctccgatcccacttcaaaagagacacactggggatgattgaccagtaccccataaccacggttagtcatgtagaacgggatatttttatacgcctgttcagtacttgtgccgccgtcccggttccaggtctctaccgtctggccattgcgcaccagggcagtaaagcgctctcccagaccgtaaactgtttcgccaacgccaagatcaagccgctcaaacatataattgcgttgattattcgtgtcctgcacgtagccattatttttcacctgactaccggtaatacgttcgccgttgcgcagaaaatccagtgaccagaactcacctttgctgacacgcgcgcttaagttgccacttttaaactcagcataacgttctgtgttttcgattgtgaccttcacgtcctgcaaaatattgagcggataatgaggaccgttattcagcgccccctgaaaatgctcaatccgcacaccgacaataccttcctgtggggagaaaaagcgcaacgtaaataaaggcgtatcaagctgccaggtacgttcacgcacatcacggggggcagcatagaccaccatttcattatcctgctgttcaacctcgaacacctgaagcgggtgaatcaaattgaggccaggttgaatcaaccagtttccatcgctaattttcattgccgttccttagttctgcacttcttgagaggtgaattgttgctggcaacggcgtttaccctgagccagctgttccataacggttttcagattgtgcgtcgtgagtgagtagtagcgtttagcgataatcgcgctcagcaaataacagatcgccggaacaatcgtgaatagcgcaataatgatgctaatcgtggcgctgttctgcgctttttctgccgcatcatatccgccataagccagcatccagccgataagagcgccgccgaaggccaaccccagtttgagcacaaacagcgtgccagcaaaactgatcccggtcaggcgtttaccattgcaccactcgccgtagtcgacggtatcggacatcattacccactggataggtgtcaccagttgatgcaacacaccaatcacgaagatgaagacaaacatagtgatgctggcctgcatgggaacaaagaacatcgcgaggctaatcactgccagcagggcgttcgtccaccagaagatagtgactttacatttccagtcggtcagaggttttgccagtgcggaaccaatcaggttacccacgcaataagtggtgagaaaagcgacaaacacttccggcgtgcccaaaatccatgtgacgtaatacatcatcgccccaccgcgtacgcacaccgccaggatattgaaaatggttagtaaaccgacaatccgccactggtcgttttgccagatatcacgtaaatcttcccgcatagacgttgttgtaggtggtgcttcaacgcgttctttagtggtgaagaaacaaaatgccagcatcatgaatgccaccacggaaaggaccgcgataccgccctggaaaccgagtggtttattatcaccgccaattaaattaaccagtggcatcatcagaacagtagaaagcatgcctcccgcggtcgccagcacaaaacgccaggattgcagcgagatacgctgagtcgggtcattggtgattacaccacccaatgcgcagtaagggatattgacgacggtataaagtaaggtaagtagggtgtaagtaattgctgcatagatcattttgccgttcatactgagatctggcgtgctataggccagtacacagacgatcccgaatggcagtgcgccaaacagtacccacggacgaaatttaccccagcgagagcgcgttcgatcggccaacaaccccatgcaaggatcggaaatcgcatccagtgcacgagcgaccaaaaacatggttccgacaaaaccggcaggaatgccaaaaatatcggtataaaagaacatcatatataacattacgttatcgaaaataatgtggctggcggcgtctcccatgccataaccaattttctctttaacggacaacacttcactcttcatctgcttttccttgatgctataggggtgctgagaccgataacgcattttgtaaaccatccctgtgagagcgaatattccgatatctggttattaatttatgattcttgttttatgtgatcgtggtagcgttaattccgctcatatatcattgtaaaatatgggttttatatgaactataatgctttcgtgataatacgctgcgtgtattaggcggaaaaaactgatctgggggatgtagaaactcaaggaagtagctataatgcgccccgcctccatgtagcaatcgaggcgcggaagatcgtcgtctccggtgaggcggctggacttcaaatccagttggggccgccagcggtcccgggcaggttcgactcctgtgatcttccgccaaaatgcctctcctgacgttctccaaccccttgtaatactgtcaatccagatattttctactgctcaatattcaatcggcttcaggaatacctggtctaaggttttgtgatggacgatgagcggctgaagaatccgcctgtcggttcttctgtcctcgaacgcatccgcgatattcacgccagtatgcgccgtgtttatttgcaggtgatttgcccccctgctgactctcagccaactgtatcgccattaaggtgaagatgttgttttactcgccccagaacacccttttttatacgactattctatttctttaaccgctggcgaaaaaaactgactataaacttcaccaataatcagactgccatcaagattaatttgttcatttaatatatcaaatcaacttgttttatttttactatcaaaaatagctcattgccttactataattaatatataaattcggtaattaattcttaacatgcttttactaataatctcaattgctggccctataatattgcgctagcattgctttctggttgtatcagcgatactcaaaaattcttaatacaatactcattcgactggtacttatttgtaactcagttatattttttcgcccggtgattcagaagaatgcaaaaaacggctaccactccatcaaaaatacttgatctcactgccgcggcatttttacttgtcgcctttctgacgggtattgcgggcgctcttcagactcctaccctaagtatattcctcgcagatgaactgaaagcccgtcctataatggtaggttttttcttcaccggtagcgctattatgggaattctggtcagtcaatttctggcaaggcactccgataaacaaggcgaccgtaaattactgattctgctatgttgcttatttggagtgctggcctgcacgctttttgcgtggaatcgcaactacttcattctcctctcaacgggcgtacttctgagtagttttgcttccaccgcaaacccgcaaatgttcgccctcgcccgtgaacacgccgacagaacaggccgtgagacggtcatgttcagtacatttttacgtgctcagatctcgcttgcctgggttatcgggccaccgctcgcttatgaactggcaatgggatttagttttaaagtgatgtatctcaccgctgccatcgcatttgttgtttgcggactgatagtctggttgtttttgccatcaatacaaagaaatattcctgtcgttacccaacccgtagaaattttaccctccacccacaggaagcgggatacgcggctactttttgtggtctgttcaatgatgtgggcggcgaataatctctacatgataaatatgccgctatttattattgatgaactgcatctaaccgataaactgactggagaaatgattggtatcgctgccggtctggaaattccgatgatgttaatcgcaggctattacatgaaacgtattggcaagcgactattaatgctcattgctatcgtgagtggaatgtgtttttacgccagcgtactcatggcgacgactccggcggttgagctggaattgcaaattcttaatgccatcttccttggtattctctgtggtatcggcatgctttattttcaggacttgatgcctgaaaaaataggctctgcgacaacgttatatgcaaatacttcacgcgtcggctggattatcgccggctctgttgacggaattatggttgaaatctggagctaccatgcgttgttctggctggcgatagggatgttgggtattgcgatgatttgcctgctgtttattaaagatatttagctcaccagtctgggctaagaaaaatcggcgtggcgcaaacagagccatcctcgccatttttgctatcatgcctgcatacataaacgacaaaacagtatgcagagggaaaaatgggttccaccagaaaggggatgctgaacgttctgattgccgccgtgttgtggggaagttcaggggtctgcgcgcaatacatcatggagcaaagccagatgtcgtcgcagtttttgactatgacgcgtttgatattcgccggtttgattctactgacgctgtcatttgttcatggcgataaaatcttttctattattaacaatcataaagatgccattagcctgctgattttttccgtggttggcgcgctaactgtacagctcacttttttgctaaccatcgaaaaatcgaacgcagccacggcaacggtgctgcaattcctctcaccgacgattatcgtcgcctggttctcactggtgcgtaaatcgcgcccgggcattctggttttctgcgctattttgacatcgctggtcgggacttttttattggtgacacacggtaatccgacgtcattatcgatctctcctgccgcgttgttctggggcattgcctcggcatttgctgctgcattctataccacctatccctcaacgctaattgcccgctatggcacgttaccagtcgtcggctggagtatgctgattggcggtctgattctgttgcctttttatgccagacaaggaacaaactttgtcgttaacggcagtttgattctggcgtttttttatttggtggtcattggtacgtccctgacatttagtctgtacctgaaaggagcacaattaattggcggtccaaaagccagcattttgagctgtgcagaaccattaagtagcgcgctactctctttgctgttgctggggatcacgttcacattaccggactggctgggaacgctgctgattctgtcatcggtgattttgatttcaatggattcccgtcgccgcgccagaaaaataaatcgtccggcgcggcataagtgagaattaccagccaggcaccgcgccaccgttaaaaatggtttctgccgctttagcgacttcgggtgattgataagattgcagaaattccttcacgttttctgcattcttattatcttcccgtgccaccaaaatattcacatacggcgaattcttatcttcaataaatacgctgtcgtgcaccggagaaagcccggtctgctgaatgtaagtggtgctgataatcgctacatcaactttgggatcatccagtacgcgcgggagctgcgccccctcgagttccataatctgcaaatgacgaggattatcggttatatccagcgcggtaggtaataacccttttccctctttcagagtaattagcttctctttttgcaacagtaaaagtgcgcgaccaaggttggtcgggtcgttggggatcgccactgtcgcgccttcttttatttgcgccacggttttgatttttttggaataacccgccatagggaagacaaacgtatttcccaccgctaccagtttataaccatgcgcctgattatcttgttcaagaaagggtcgatgctggaagacattcgcatcaagttcgccatgatttgtcgcatcgttcggtagcaacgaaccgctaaatcctaccagttcaacatcgaggccatatttctcttttgccacctttttagcgacttccgcgacatcttgttctgcgccatttataacgccaactttaatgtgttttgcatcgctgctactctggtcgcaacctgccagcagaattccggccagcaataatgcggcccctgtccgtagatgatgtgttgtcagtttcatttttttatccttttattaatgattacctgactatagcggtaaggtcgctgcggtttaaaaaacgaaacgctatcgataagaataaaaaggaataaaagtggaatataaagtctggcacttcttactgaccacgcaagcgcgtttcgtacagcatgatgagagcgatgaaagcaaactacacttatgcttcattcgatacacatttgtaaaaggttgaatccatgaaaccaacgacactactgcttattttcacttttttcgctatgccaggcatcgtatacgccgagtcgccttttagctcactgcagtccgcaaaagagaaaaccacggtattacaagatttacgtaaaatttgcacgccacaggcgtcattatcagatgaagcgtgggaaaagttaatgttgtcagatgaaaacaataaacaacatatacgcgaggccatcgtggcgatggaacgtaataatcagagcaattattgggaagcgttgggtaaggtagaatgcccggatatgtaagaacagcaacaactactgaccaacgcttctttacctgatatcaggatttcttcattttcacctttgcagtaaccaacaatgcagtcagcaacatcaatgtgccggacaacatcaacggcgaagtcagaccaatattatccagcgcataaccgccgattgccgcgccacaggtattagcaagctgaataaccgccacctgaatagacccggctttttctgcctgatcggccagcgagcgggtgatccacgttgaccagccgacgggaaccaatgcaaaagttagcccccagataatcgccacgccggtagcaacgattttatcgcttccccacaacgtcagtaccaacgcactcacagccagtattaacggcgcgcctgctaaggccagttttaccgaacgtttaagaatgaacgacgaaagcgacgtaccaataaagctggcgataccaaaactcaacagcaccagcgttaagccatccacgccgaatcccgccaggttcatatacaccgggcgaatatacgtgaagaaagcaaactgcccggcgaaagacatgaagatggcgatcatccctgccatcacacccggacgttgtaataagcggaaagtattttgtttctgatgcgagggttcgcctggcagtgaaggcaatgatttgataatccagaaaatacacagcacgcccatcaccgccgccgcattaaagacattgcgccaaccgataagctcgcctaaaaaactgcccaacggcgcggcaatcaccagcgcaatagaaaccgcgccgaagatcaccgacagcgccttcggcaccgtacgcggcggcaccagacgcatggtcagcgacgccgacatcgcccagaacccgcccagcgccagccccagacaggcacgaccgattaaaagcaaactgaatgagttagcaaaggaaaccagcaagcaggagagcgtcagcaaaacggcaaacaaaataacaacgtagcggcggtcagtagcctgaattgtctgggtaataaacaaactggcaaacattgccacaaaggcggtcacggtcaccgattgcccggcaaccccttccgaaatgcctaaatcctgggccattggcgtcaacaaactgacgggcaaaaactcaacgataatcagacaggcgacacaaaacgccaccgagaaaacggctgaccagttcggtcgggtgatggcatccgcgccgcggttttcggcaataaattcactcatggtgttacccgtggcatgtttcaggggaaaagccgaccactttaacattgaaatgtgtgacgcatttaacgtttttgcaacttttacggtgttgcttgagctggagttaagatcgaaacggaacagggcaaagattaccggatgcggcgtgaacgtcttatccacccgacaggtcaggcgcggtctgtaggctgataagacgaaacggtttcaatgcaaccagtgaacgccctcggcaggctgaaagaacgcgttatagcgcatctgaaaagcattaatatcctgcatttcaggttcggtttcgcgcagaaaacctagcgccagcctgacctgagcgtcggtaatcggcgcggcgaggcgagctttttgtaaaatccgatgccattgcagcaggttctgttcgctaccatcgacaatgacaatttgccagatgagcaacacctgcgcggcgttttgcaggtgcgactcatccggacgatgcaaataacgtaaaaattcgtcaccagctgactttcccatttgatcgaccatcgactccacgggtacgacatcgatgttcagccgatcgctgagacggcgaatcgcttttctggccccggatgtcagcacccgaaaaccaaccacaaacactaccgccagcgtggcgagcattatccagatcatgagttctcctgcgtaatcagaactcatgatatctggaaaccctcgccagttactaatccaccagaataatcttcagtgcaaacagagctgcgaccaccaccacacacaggttcagatcgcgccagcgcccggtgcatactttcatgatgcagtacgacataaagccgagtgcaatcccttcggtgatcgagaaagtaaagggcatcatcaccgtggtaataaacgcaggcaccgattcggtaaaatcatcccagttaacgcgcgccaggctcgaagtcatcagcacgccaacaaagattaacgctccggcggttgcgtaaggaggaactatcgccaccagcggtgagaagaacataaccaacaggaacataacgccaaccacaaccgcagtcagccccgtgcggccaccgactgccacaccagaagtactttcaatataggcagtaacagacgaggtgccgataaacgcacccgccaccgaactgacgctatcaacatacagcgccttattcatattggggaatttaccgttaccatctattaagcccgctttatcagttacaccaattaatgttcctgatgaatcaaataggttgatcagcataaaggagaaaatgataccggcgagttcaagtgttaacgcgccgctcaaatctacttcaccaatgacgccgctaatatcaggcggaatggaatagacgccgctaaaatgaacatcaccgaaaaataatccacagcaagacgtcaccacaatagaaaccagcaccgcggcatgaaaatgacgtgatgacaacacggttataataaaaaaccctaaaatacctaacaacacgccgtgagaacttaaatcgccaatcatcaccagcgtgtctttattggcgacaataacgccagtattttttaatcccattaaggcgataaataatccaattccgctggtgataccaatacgtaaacttaagggaatgttggagatcatccagtaccggatacgaaacagcgtgagcaaaaatagtccaactgcgccccagaatattgcgcccatcccggtctgccaggagatgcccatcgcccccacgaccacgaaggcaaagaaggcgttcagccccattgccggagccagcgccacgggtaagttagcaaatatccccatcgcaatactgccgataccggcaatcaaacaggtggtaacaaacaccactttcgggtccatttgtgccgcgccgaggatttgcgggttcacaaaaacgatgtacaccatggttaaaaaagtggtcatccccgcaatcaattctgtgcggacggtggtcccatgctgaggtagtttaaataatcgcgaaagcgtccctgattcattactcacgtaatcggtattgtcattattcatttttttgtccattggaggagatttaatcccttgcttttgtaaaacaaatgacaacaacggttcagtgataattatcacatttcaattgcacattaatggatattctttaataatctcgcgacgtttctttatgataaataataatcaaattgataaaatcaaaatgagaaaaatatgaataattctattaaccataaatttcatcacattagccgggctgaataccaggaattgttagccgtttcccgtggcgacgctgttgccgattatattattgataatgtctctattctcgacctgatcaatggcggagaaatttccggcccaattgtgattaaaggacgttacattgccggtgttggcgcagaatacactgatgctccggctttgcagcggattgatgctcgcggcgcaacggcggtgccagggtttattgatgctcacctgcatattgaatccagcatgatgacgccggtcacttttgaaaccgctaccctgccgcgcggcctgacgaccgttatttgcgaccctcatgaaatcgtcaacgtgatgggcgaagccggattcgcctggtttgcccgctgtgccgaacaggcaaggcaaaaccagtacttacaggtcagctcttgcgtacccgccctggaaggctgcgatgttaacggtgccagttttacccttgaacagatgctcgcctggcgggaccatccgcaggttaccggccttgcagaaatgatggactaccctggcgtaattagcgggcagaatgcgctgctcgataaactggatgcatttcgccacctgacgctggacggtcactgcccgggtttgggtggtaaagaacttaacgcctatattactgcgggtattgaaaactgccacgaaagttatcagctggaagaaggacgccggaaattacaactcggcatgtcgttgatgatccgcgaagggtccgctgcccgcaatctcaacgcgctggcaccgttgatcaacgaatttaacagcccgcaatgcatgctctgtaccgatgaccgtaacccgtgggagatcgcccatgaaggacacatcgatgccttaattcgccgcctgatcgaacaacacaatgtgccgctgcatgtggcatatcgcgtcgccagctggtcgacggcgcgccactttggtctgaatcacctcggcttactggcacccggcaagcaggccgatatcgtcctgttgagcgatgcgcgtaaggtcacggtgcagcaggtactggtgaaaggcgagccgattgatgcgcaaaccttacaggcggaagagtcggcgagactggcacaatccgctccgccatatggcaacaccattgcccgccagccagtttccgccagcgactttgccctgcaatttacgcccggaaaacgctatcgggtcattgacgtcatccataacgaattgattacgcactcccactccagcgtctacagcgaaaatggttttgatcgcgatgatgtgagctttattgccgtacttgagcgttacgggcaacggctggctccggcttgtggtttgcttggcggctttggactgaatgaaggtgcgctggctgcgacggtcagccatgacagccataatattgtggtgatcggtcgcagtgccgaagagatggcgctggcggtcaatcaggtgattcaggatggcggcgggctgtgcgtggtacgtaacggccaggtacaaagtcatctgccgttacccattgccgggctgatgagcaccgacacggcgcagtcgctggcggaacaaattgacgccttgaaagccgccgcccgtgaatgcggtccgttacccgatgagccgtttattcagatggcgtttctttctctgccagtgatccccgcgctaaaactaaccagtcaggggctatttgatggcgagaagtttgccttcactacgctggaagtcacggaataataaaaaaagcccggcgtcatgccgggcaaaagtcaccagttacgtttatgccactgtcaactgctgaatttttttctcgcggcggattttgcgttcttccattaccgccactatcgccatcaggcagatacaaccaatcgcggcgatatccagcgcggcgaaggtgcctgcccagccggtaaggccgaataccggcgtcccatcggcaatcattcccagacctaacttggcaaagctgtcaccaatcaggtaagcaaaggtgcctttaataccatcggcagcgccaatcgcttttttaggtacaaagccaacagcagccacaccaatcaacaattgcgggccaaagaccaggaaacccaacgcaaagagagaagccagatagatatattcgttactggcatgttgatacacaccgagcgtggcgataatcagcgccagcgcgatgcaggccaccaggccacggcgaccgttcgccaggtcagagagccagccccacagcagcgtaccgaccagcgcaccagcttcaaacagcgtaaagccctgaatcgccaccgctttagagagtttcagttcctggaacgcgtatacggttgaccactggtcgataccaatacgtaccacatagaggaaaatgttggcgaagcacagcagccagatcactttgtttttcagcacatactcaacaaagatctgccacttggtcatatcggtagattctgtctctttgtcctcttcgctgatctcctcgccgaacagttcttcagctttgccgaggccataagattccggggagtcgctgccgtaacgcaggccgataaaaccgacaatcagcgcgataatcgacgggaagataaacatgccgatgacatggccatcgaacaggtaatttgccccgaacagcgccacacctgctgcgcctgcaccgccaaggttgtgagaaatattccagaaaccgaggaatgtcccgcgtttacgacgcggcgtccatttggtgatggtggagtaactgcacgaaccgccggtactctggaaaaagccgcttaaggcgtagaaggcaatcatcaggaacaggctaaccgagccgctgcccatactggcactgaagcccagcatacaaatagcagagaggatcagcatgaacggcaggaattgtttggtgtttttgccgtcggcgtagtaggaaaccagcgttttacccacgccataagtgatggagaaacccaggccgatcatccccagctgcgtcatgctcaacccgtaggtcgaaatcatatcgttctgcgcgatgttaaagttcttgcgaatcaggtacatcgtcaggtagccgataaagaccaccaggtaggattgcatgaacggtttgaaccacattttgcgccgcacttcgagcggaaggtccagggtcggcttgcgaacctggtttaagaaagccagcatgggttactcctgaaatgaatacctgcgtgaggcatgcattgtaaaaatcagcagcaaatcaggcctgagatagcgtccaggcaaaacctggaaaatttcttagttttgccggatatgaagtgaaaaggtgagatgcatcacgcttcgcgcggtgtctgggcgttcaaaaagggcagtaacagcagtgcggaaatcccggcggcgatagagataaccacaaaaaatccgctccagtgccaggtatcgagtactttcgccagcggccaaccagcaagcgacgcccccagataagcaaacaagccgacaaaccccgtcgccgcccctgccgcctctttgtgggaacactctgccgccgccataccgattaacatctgtgggccaaagacaaaaaaaccaatggtgaagaagcaggttgcctgcatcacgtagctggcaaatggcatcagccacagggagccgactgaaagcaaaattccggcggcgaaaatcaaattcatcggccctcggttgccgttaaacaatttgtccgagccccaaccggctaccagcgcaccgataaatccgcccagttcaaacatcgtcactgccgtattcgccgtgaccagatcgacgcccagtgtctcggacatatacaaattgccccagtcgttgatcgccgcccggaccacatagaccagcacatagcaaaacgaaagcagccagatatacggattcagcaacacatatttggtgaggatctctttacgcgtcaaccctgccccttcttgttgttgagcaatttccagcgcgtcgtgtcgccattcaccgaccgccggtaaacctaacgcctgcgggcgatcgcgtagccgccagcagagaaaaatccccacgactatcgccatacaaccagcaatcatcatcccggcacgccagccgtaatgcagcgcagccgctgccatcacaatgggaatgagtgcgccgccgacgttatgcgccgtgttccataatgcccaccaaccgccgcgctcggtacgtgaataccaggccgttaacagacgcgcacacaccggtgaaccccagccctggaaaaaggcgttcagcacccagagcacggcaaacgcccatagcgacgtcgagaagccaaacagaatgttgataatgcccgtggcgataagccctatccccataaaataacgggcatttgagcgatcgctgacaatgccggagacaaacttcgacacgccataggtaatgtaaaacagggtcgctaacaggccgatatcgctacggctgagcacgccgttagcaaggatttctggtacggcggcgttaaaacttttccgcgtgaagtaaaacagcgcgtaacccagccagatggtcagcagaatatgccgacgccagtagcgatagcgggcatcaatttcatatttatcagtcattaatggcgcatcggcaggcgctttcagaaacggcaacatcatcaaaccttagacatagcgttgaggtagagaaacgctgacacgcgtgccgtgcagacaggaaatgtgtaatgtgccacccagcgccgttacgcgctcgcgcattccggtgaggccaaaaccttgttgcccggaacccggcggcaaaccgctgccatcgtcttcaataaccagcatcaaccgttcatcctgctgccagccttgcagggtgaccgcgctggcatcagcatgtttcacaatgttgttcagcccttcctggcagacacgaaacagcgtcacgcgctggttttcgcttaacgctgattcatcgattcgccattcgagatggctgacaataccgcgcccttccagctccatttcccgcatcagtgagcggatggcctgctccagggtgagatcatccaactggcgcggacgtaaccgacccaacaaacggcgcaccgcgtcgtaaacgcccagcgatagttgttcgatgagctgcccgctctgcttcacgctggcgttatctgccgccagccgctgaacaatgcccgcctgagtacgaatagcagtgatggtctgaccgatatcatcatgcagctcacgcgccacatcacggcgcacgctctcttcggtttccagcaaccgttcagccagatgctgattgcgcgccagttccttttgcagcgactggttaagttcacgcaaccgctggatgccagcgccaagcaacaaccctgtcagactttgcaccagcagcgagagcaataaatccaccggatgatcgcgccaggtttgactggcgatcagcgcgatggcgttcatcaacgtcgcaatcagcgccccttgccaaccatagtgccaggccagcgcgataatcggcagcgccagacagaatggcgtaaagcgcgacagttcgtccggcaatcccaactggagccagagactgataacaaacagcagcaagtaccagaccagatgtcgcccgcgccagttgattggctgagaaaccagtgacggaccgagcggcagccaggtgttattggcgagatagtgccagaacaccagacatatcggggccagcgtcaggccgccagttaaagtcagcaacagcgcattccacgactctttgccgtgccaaagccagggcagcgactgcaacaacgccgccgccgttaacgccgccccctgtaacagcaaggtgcgccagtcacgctgatggcgatagcgcgagatcagcgctacgggcagtaacgtcagtaaactaccgatcatcaataacggaaaatgggttaaaccgaccgcctgcgttagccagtaaatcagcagccactccgcgcccagcaatacgggccagtatccgcgcgggcattgcagcattagccccagacgcagaccaaacggaaataacagcaccgccatatcagggcgctcaaccagatgcaggctgatactccacaggcaaaaccatgcggcagagaagataaaaaagcaggcaataacggtaattaagcgggagaacaacgtcttcatcaccagccatcaaacatgcggcgcgccagctctacgtcgttactgacgcccagtttttccatcagattggcgcgatggacgtgtaccgttttcggtgacaagcccagttcggcggcaatctctttcaccgccattccttgcgccagtttttccgccacctggcgttcacgtttggttagcgggtcctgacgaccggatgccagtttaatggcaatatccggcgtcagataacagccgcccgtggcaaccgtatgcaccgcagcaatgagttcatccgggctacagcgtttggaaagaaagccgcgtgcccccgcgttaagcgcctgctcaaccagcgcaggactgtcgtgaacggagagcataatcgtcgccatacctttcggcagctggcttagcagctccagaccggagatatcgggcatggagatatcgcaaatacacacctgcacaccgcgccccggcagccccgccagcgcctcgcgccccgaaccaaactcggcaactacctgcaaatcaggttccagccccagcagctgcgcaaagccggagcggacgatgaggtgatcgtctataagggcaacggtgatcatggtcttgtcctggcgggtaaaaaaaatacgcgcttaccttaacgataagcgcgatgttgttcaagccttgagcggttactgaaaaaacaccgcgatcttgttaaacatcgtcggatcggactgattacgctgcactttcacgacatcttccagcttatcgatttggcttatcatctgctccagacgctggtcgtcattgaccagtagccagatatggcttttgtcgctgtcctgaatcggcagacaaagaatgccttcaacgttaaaagcgcggcgggcaaaaaggccacaaacgtgggtcattacgcccggatggttgcgaacggtgagctccagaattacgttgtcatgagttgtgttttgcatggcttattcccccaccatttcagtattcgccgcacctggcggcaccatcgggtaaactttttcttcggcatcaatgcgcacatggatcagcgccgggccagggcgattgatgatttcctgcaatgaagcctgcggatcggcttcgttattcaaatcacaggtttcgaggccgaatccggcggcaatctgcataaagttgattttgcccggataggtggcggcaaaaacgccttgctcgtagaacagactctgttgctgatgcaccagccccagcgcttcgttgttcatcagaatgattttgacatccagctgattttcactggcggtcgccatctcctgaatattcatcatcaggctgccgtcgccggagaaacacaacactttgcgatccgggttcgccagcgcagcgccaatcgccgcaggcaggccaaaacccatcgtgcccagcccaccggaggtcagccactggcgtgggcgattgagcggataagcttgcgcggtccacatctgatgctgaccaacgtcggtggtgataattgcattgtcatcgacacaggcggcaacggcgttgatcaggccgtaatggcttaacggatcgcacgctttcgggattggacacggaaactcacgctgcaaatccgctaccaactggtgccactctgcacgcggttgcgcttccaccagcgggatcaactgcgccagcacgtcatcaacatccgcctgaatcgccacgtgcggctgcttgattttacccagctctgcacggtcgatatcgacatgaatgattttggcattcggacagaactgctcggttttgccaatcgcccggtcatcaaaacgcgcaccgagcactatcaacaaatccgcctcctgcaaaatatagttggtgctgcgcacgccgtgcatccccagcatacccagcgacaacggatgcgcttttggcaacatgcccagcgccattaaagtcatggtggtaggcagttgcgctttctccgccagttcacgcacccgtgcgggcgcattgatcacaccgccgcccagataaagcaccgggcgtttggcagcgttaatcatcgccgctgcgtcacgaatgctttcttcgctaaaggcgggggcggcggctttttctgccatagcgggctgtgtttcaatctcaaaaactgccgtttgcacatccttaggaatgtctatccacaccgggcctgggcggcctgattgcgcaatgcggaaggcatcgctcatgacctgcgggagttcttcgatatgtctgaccagatagttgtgtttggtgatggggatagagatgccgtaggtgtccacttcctggaaggcgtcggtgccgatcatcgaggcgggaacctgaccagtgatgcaaatcagcgggatggagtccagccgcgcatcggcaatggcggtcaccaggttagtcgcacccggtccgctacaggccatacagaccgccggtttaccgtcggtgcgcgccattccctgagcgataaagcccgcgccctgttcatgacgggccagaatatggcggatttgcgtgctttggcttaaggcatcgtaaacaggcaggatagaaccgcccggaatgcctgtcacaatcttaatgccctgctgttccaggaaatgaacgataaattctgcgccggtaaagcgcttacgcgtcgatgttgtgcccgaacttgccatgctccagtccttttcttctgggccgactttccgggaggtgcttaaacgaaaaaccccgcccggtttgcgccggcggggttttggaatcgtgtgttgttccagtccctacggcgcattgccgacgaccaccaccacacgcacgacgaccactgcggcggatggcgcagttggtagtagttttgcgttgagcatggaagtagtcattggggaccttgttggttttgtgtttaacaatatttatacaagcacagctttacaggggagacaatggaaaatttttcagcaagggaaaattgaggggttgatcacgttttgtactgaattgcagataacaaaaaaccccgccggagcgaggtttcgtcagtcgcctgcggctggtaaccgcaaagcacactgtattatgtcaacactgaaagtatacgtgttccgcgcagaacgcgcaatttcggcacgaattttgacgtatttagtgcatagttgagtatcgatcacagtttgcgttttgtccaaatattactgtttatttatacagtaaacttctataatatcactgtacgcaatgtgttatgcgggggccgcatcgttacccggcgcactaagtcctggctgaaacgggtggtgccgtcagcgccttaaccccgcgtgagcacactgtgttatgtcaacaagcacaacgtttctccttgagataccgcgtgcacaacagctggcaacaggcagcggaaaggtacgtcagctggcagtgctcctgaaccacaggagacgcgtatgaacctggtggatatcgccattcttatcctcaaactcattgttgcagcactgcaactgcttgatgctgttctgaaatacctgaagtaattcagattcaagtcgcaccaaaggggagcgggaaaccgctccccttttatatttagcgtgcgggttggtgtcggatgcgatgctgacgcatcttatccgccctaccatctctcccggcaacatttattgccgcttttgtttacatattctgccgctaaacaattccccattcctggcgtatatctggctaacattcatcaatgtgatagattcctctcccgcatttatgggaatgcgtagtgacttattctaattatttttataaaagcatccgtgataatgaaaaggcaaagaaacgtcaatttgttattgatgttggtattactcgtggccgtcggtcagatggcgcaaaccatttatattccagctattgccgatatggcgcgcgatctcaacgtccgtgaaggggcggtgcagagcgtaatgggcgcttatctgctgacttacggtgtctcacagctgttttatggcccgatttccgaccgcgtgggccgccgaccggtgatcctcgtcggaatgtccatttttatgctggcaacgctggtcgcggtcacgacctccagtttgacggtgttgattgccgccagcgcgatgcaggggatgggcaccggcgttggcggcgtaatggcgcgtactttaccgcgagatttatatgaacggacacagttgcgccatgctaacagcctgttaaacatggggattctcgtcagtccgttgctcgcaccgctaatcggcggtctgctggatacgatgtggaactggcgcgcctgttatctctttttgttggttctttgtgctggtgtgaccttcagtatggcccgctggatgccggaaacgcgtccggtcgatgcaccgcgcacgcgcctgcttaccagttataaaacgcttttcggtaacagcggttttaactgttatttgctgatgctgattggcggtctggccgggattgccgcctttgaagcctgctccggcgtgctgatgggcgcggtgttagggctgagcagtatgacggtcagtattttgtttattctgccgattccggcagcgttttttggcgcatggtttgccggacgtcccaataaacgcttctccacgttaatgtggcagtcggttatctgctgcctgctggctggcttgctgatgtggatccccgactggtttggcgtgatgaatgtctggacgctgctcgttcccgccgcgctgttctttttcggtgccgggatgctgtttccgctggcgaccagcggcgcgatggagccgttccccttcctggcgggcacggctggcgcgctggtcggcggtctgcaaaacattggttccggcgtgctggcgtcgctctctgcgatgttgccgcaaaccggtcagggcagcctggggttgttgatgaccttaatgggattgttgatcgtgctgtgctggctgccgctggcgacgcggatgtcgcatcaggggcagcccgtttaagcgcacgtcaccgcagcatcgtcatcagctccatgggagaacgatgctgctttatcagatcacgcatcacccgcatatgcggtgcggagtaagaataaaacgcctgatagcccgcacaaagcacgctgtctggcgtctcctgccgagcgtgcgggcacaggcgatgccagtcgcacgcctggcagtcacagcgcggttgcgggttttcgctgccacaccatttttgtaaggtggcgtcaaaaagctcaatcgagatacgactgatatctgcccgcacccaacactcgaacagggcaattaaaaatttcccccacagctctgctgtcaccgaagcggccgtcagatcgccccggtcatcaaattcaagatagggaatgagctgtacggagcggatgccccgctgtttgaaattgtgataaaaatcggcaggttgcagagcatccttgtactctacaaccagtttatgcctgtcctcttcagcatcaatgacctgacttcctgtcatgcgactctctcaataaatacgataagttgatgtatatgcgttacagcaaacagtattgcgagagataacaccgcgagggagatcaaaaatttgtcacggactacgtgaaattgggaaaaatcgctattcgtgacatccattaaattgcgattacgggtgtagtgccagaggatcagcgccacgatggcgagaatgccaatcgaaatccagaataacatgcccgcctggtgccagttgtgtttgatagccaacgccatcaacgcgccgtagcccagcatggtacgaaaccacgccagtgatgtgcgctccggctgcagtcctgggtcggcaatgcgtctggctttgcggctatccggcatacaacaccagtcccataacgatcaccgccacgaccatcaatattaagctaatgattaataagctgttggtgtagggcaggtcctctttcagacgcatcgctttttcattgcgtaaccagcgcaagtagccatacatcgctaacccgccggaaaacagacacaacaacaacgccagcagttcgcgaatgacgggcgtggcgaaatctggcgcaagttgatcaagcccaacccccgccgccagaaatcctagtgcagtacggatccacgccagaaaagtacgctcattagccagcgagaagcggtaatcaggcgcttctccgaggcgggaaattttcattgttgctcctttgcaatttcactaacgctctacctttagcggtttttttaagaatttcgtccgcccgtttcctgatatgcttttgccatccgctacaaggaggtcagatgggtatcatagctcaaaataaaatcagttcattgggcatgctgttcggtgccatcgctttaatgatggggattatccacttttcattcggccctttctccgcaccaccgccaacgtttgaaagcatcgtggcggacaaaacggctgaaattaaaagaggtcttctcgccggaataaaaggcgaaaaaattaccaccgtggagaaaaaagaggacgtagatgtcgataaaatcctcaatcaaagcggtatcgcactggccattgctgcgctactttgcgcatttattggcggtatgcgtaaggaaaatcgctggggcattcgcggcgcgctggtttttggcggcgggacgctggctttccataccttgctttttggtatcggcatcgtgtgcagcattttgctgatattccttatcttttccttcctgaccggcggttcactggtttaagcagcctgaataatgcccgccgggtgatcatcagcgggcattatcgtcagaacttctgttttttctcctccaccttcaccccttgtgtcggtaggccggtgtcatagtcgcgtacaactggcgaatagccatcttgtggacgtggacgaaacgcccccatccagcgcggccgtgcatctttacgccacggacgcagactccattggtaactgcggaacggatcgcgaattttgtccatgtaatccaataaggcgtcatgcattttgctgcgaacgtctgcaaaacggatatcatcgatcaggttatgcatttcatttgggtcattacggcgatcgtaaagttcatcactggtgaagaggttgagtaccagtttaaagtcatccgtcacccagcaacgcaccggaataaaaccgccaaagctgtcatgctcaatctcgtagcggttaaattccaccatcacgccgcgtggctctttcacggcaaggatattttcccccggcagaatctctggtttttcaatatctgccagcgccatcattgtcggcagtaaatcgatatgactgactggcgtatcgacctgtcgccgctccccttgcggcgaacggatgatcagcggaatgcgggtgatgtcgtcatacatcgccgcccctttactgatcagcttatgtgcgcccatcatttcgccgtgatcggaggtataaataacccacgtattttcacgttgctctggcgttaaggcattgatgacccgtccgatttggtcatcaacaaagtcattacaggcaaaatagagcggatggtgataaagcccgtcatcaccgactggcgatggcatcgcctgcgcccataagcggtgatgttccggtttgttagccaggtcatcctgtgctttctcgcccagctcgtagtaaaaatcagcgtatttctctaaatactccaccggacaggtgaacgggtgatgcggctcatcatacgaaaccaccatcaggaaaggctcgtctgcgcgcgcaggctgttgcagaaaatccaccgcccgattgctgatacgatgcgcccaggtgaaggtttcgtcgatatggttcgcctgtaaatcttcgacgctgtttaggccattgcgccacaggctaatctctttttccgtcagttcgctaagatagttcgccccatcgaaccagtaatcagcgtcccactccggcggacactcgccagtgccgaaatagtcatgaccgtcgagatgccatttgccgatgtaacaggtgtgatagccggcatccttaaagtagcgccccatagtggagatgtttttgcctggcgcgacgttgttggtccacgggccggactggttagcgtagataccggtaaatagtccggcccgtgcaggcgtacaaaccggtgaacaggtgtaggcggaattaaagcgaataccttccgccgccagactatcaatattttgcgtattcagcggtttaccgctatagcaaccgaccatattggtggcctgggtatcggtcatgacgaacagaaaattggggcgtttcataggctatccttcccgtcgggagtaaaggttacggctgggtcgtgacgatgccgccagctgtcaaaaatcaggtagacaatcactacggcggcaatgaaataactgatcatcgctaaccagcgcgtaccgtagccgccgaattcagccagcccggcatagacgccaatcatcgcgaacaggatgccaattgacgcgatcttgacgtttttccacggtttcatgtccaccgcaaacgcatctttgaaggtgaacggcgtggcgcgcggtttgataaaaccgatcaccagcatcacgaccacgttgatgcagaacgtacaggccagcacatagaggaaatggaagtcgaacttcaccagatagttgatggtgatgtagctgattatgccaatccccatcgctacttttgccgccagcgccgggatgcgcgggaagaaaaagcccataatgatgatggtaaccagcggcacgttgtaaatgccgttgagctgtttcatccagctatacagcccctgcggcgcgttggcgatccacggcgcgaccagcaccgaaacgatagcgataaagaaaccaaatttgcgcccgacggtgaccagctgctgcggctcggcattctggttaatgatgcgacggtaaatacccatactgaataacgtactggcgctattcagaaagccgttgaaggtactgatcaccgcaccaaataacaccgcgccgaagaaacccaccattggcactggcagaacgttattgaccagcgtcgggtaggccatgtcggctttcggtaaatcctgatacagatgaaacgcaatcaaccctggcagcaccagtaccagcgggtcgagcattttcagcaccgccgttaacagcgcccccttttgcccttccgccaggctttttgacgccagcgtgcgttgcacgatgccctgatttgtacaccagtaaaaggtgttcaccagaatcaaaccggtaaatgccgcgccaatcggcaagggatcggtcgggccaccgattgagtttaatttctcggcgtgaacggtggtgagttgctcaatgccctgcataaagctgcccttgcccatcgcgattaggccaaataccggcaccatcaacccgccgataaccagcccaataccgttgatggagtccgccactgccattgcgcgcagtccgccgatcaccgcatacaaaattcccgccagaccaagcaaaattaccagtagccagatagccgcaccgtgagaaatctgtagcgattccccgacgtgaaacaggctgttgagcgccaacgcgccggagtagagaacaatcggcagaaagcagacgccggtggcaattaggaagcagaagtcgatgataatacgcgtcgttttatcataacgttcctccagaaaatcggggatggtggcaatgccgcgcttcagatagcgcggtaaaaagattagcgcgaggaagatcagcgtcaccgctgaagtcacttcccagcccatcaccgacatgccgcttttgtaggcctgcccggaaaggccgaccagttgttccgtggaaaggttggttagcattaacgaagcggcaataaccggcgcttttagtgaacgtccggcaagaaaatagccttgttgcgatccggtatctgttttgcggaccttccaccaggtgatcaccgccaccagcagcgtaaaaccgacaaaactcaagatttgtaacgaattcatctcatagcccttatttatgtttatgtcccggacgcatgaatatagggagaggtaaaatgcgtcgggtcaggcagtcagattcttaaaatacaaacgtcgtatccctgaacggattgttttctgttaagttcaggttgtgagcataattcgccggagggatattaaaatgaatggaaaattgcaaagttcagatgtaaaaaacgaaactccgtacaatattcccttattgattaacgaaaatgtgatctccagcggaatttctctgatctcgctctggcatacctacgccgacgagcattaccgggtgatctggccgcgggacaagaagaaaccgcttatcgccaactcatgggttgcggtgtataccgtacaaggatgtgggaaaattcttttaaagaatggcgaacaaataacactgcatggcaactgtattatattcttaaagccaatggatattcactcttatcactgtgaaggtttagtctgggaacagtactggatggaatttacccccaccagtatgatggatattcccgttggtcagcaaagcgttatttataatggcgaaatttataatcaggaactcaccgaagttgctgagttaataacttcaccagaagcaataaaaaataatctggcagtcgcttttctgacgaaaattatttatcagtggatttgtcttatgtacgcagatggtaaaaaagatccacaacggcggcaaattgaaaaattaattgccactttacatgccagtctgcaacaacgctggagcgtagctgatatggctgccacgatcccctgtagcgaagcctggttgcgtcgtctgtttttacgctataccggcaagacgccgaaagaatattacctcgatgcgcgtctggatctggcgctatcgctattaaagcaacaaggaaactcggttggcgaagtcgctgatacgctcaacttcttcgactcctttcatttcagcaaagcctttaaacataaatttggttatgcgccgtcagccgtgctaaagaatacggaccagcacccaacggatgccagtccacacaattaacgtaactctggccagtacgctttgttggcctccagcaactcatccagaatagctttggcgaccgaggcgctcggtaccgttttcgacaacgtaatcgcctgccacaggtgctgatatgaacgctgttcccaggcgtccacgaccagtttttccaccgccacttgctgactcattaaccctttctgaaactgcgggatatcgccgaccaccagtggttcaggccgtagtagcgcacgcgcatctgtttgcgatcttgcagcccaacaatttgcgccatccggctttcaataccgattggcatgtcacagatgttgaggattttcgcattcgggcgcagacgacgcgtggcttctgcgacaatggctgccgggttggagtagttgagcatccaggcatttggtgaatatttttccatataatccaccagttccaggacgccgccaatggaacgcatgccgtacgctattccgccgggtccgcaagtttcctgaccaacaacgccgtggcgcagcgggattttttcatccagttcgcgcatcgggtatttgccgacgcggatgtgcgccatgacaaaatcaacgtcgctgaatgccacttcaggatcggtggtgtaactaaacgcaatgtccggcgctttttctttaaggatgactttacaggcttcggcaatcacttcctgccgcgcaccatcgttatcataaaatttcagtgcacgaagcgggaaacggtcctgattcgccaggagcatcaacacgatgcctggcgtaaaggtgcttccaccgcctgcgacaaccactgagaatttggtcattatactgcctccgtaatggcaacattttctgctgattgatgagaattaattaagctatcgagctgttcacgcagctgagatacatgcagaccaatgatcacctgaatggcatcgccactacggaagacgccgtgcgctcccagctttttaaagacttcgtcatccagcgtttgtgacatgtcatgcagtgcaatacgtaaacgcgtcgcgcaattgttaatgctggagatattgccgaccccgcccagggcttgcaggataccggcagcctgatccagctctttttttggctctgccgcggtggtttggcctcgcgaggctttgtattcggcttttgagtagagtttcacttccgcatcttcacgtcccggcgtgcacatgttgaactgcagaatcagtgtgcggaaaaccacgaagtacagcagggtaaagcacaacccaatggcgatttgggtcagcatcatatccgcgtggttgctgaacatcgggatccagttttgcggtaaaacctagtcaatcagacctccgcccatgttgcccaccacaccaaagagatacattacggtcgacattgaggccgccagcacggcgtgtaccgcaaacagcaacggtgaaatgaacaggaaggtaaattccagcggttcggtaattcccaccagcatggcggttaaggttgcgggaatcagcaagcccgccacttttacccgattttccggtgcggcagtgaagtacatcgctaaagaaatgcccacggcaccaaagatttttgagttaccgtgcagggcaaaaccgccttccgggaacaacgatttcagcggctcggcgctcaaactgaactcttgcagatgctgcgcccagtacatctgaatgccgccttcaacagctgccggaccaaagataaactgtccgtagatgaagtggtgtaaaccggttgggatcagaatacgttcgaggaaggtgtaaacccagaccccaagtgcacccgccgaacgcaggaacgcttgcagagattcaatccccatttgtacttttggccagccgagcaacgtcagccaggcacaggggatcatcaccaggaaggcgataatcaccacataagacgtcccctggaaaatgccgagaaaaaccggcagttttttatcgaacagacggttatgcagcgccgtcacaatgccggaaatgataattgcgccgataatgctggtatcgagggttttaatcccggccatcattgtcagaccgctacctgccaccgcgtcctgagtgaaatcgacgccgaagtagcttccccaggtcattcccatcgcgttgatgaaatagttccaggtcaggaaactcaccatcaccgccagacaagcacgcccctgcgcttgcttagcaaggccaatgggtaaaccgacagcaaaaatcagcggcatattacggaataccgtccaaccgccctcttcaataatgtgtacgatttgcgcgaataaactgttcggatcggtcagtgattccccgacaaacatcgggttttgcagcaagatggcaagacccaccacaatcccggcgaagggaaacagcagcactggcgtgaacatcgcgccgccaaagcgttgaatttgactgagcatttccacatcctcttttctcaattctgtaagtaggaagcctgattggttatgcggcaggcctggagcgaggataggaagatgcgatcggcagaacatgacgacccaatgggattcgtgatcgctttcatgcttttcgttgggcggtagagatctacgttttcgcgaaaaagtagacctctgtgagcacaggtacacagcatcgaacacatctttaaaaaaaagatgttttttcaatcgattaagcagaacttgtgtgcgcattacccgggcttgcaggcaaaaaagagatctagagatgatctacaaaagcattgcggagcggttaagaattcgacttaactccgcagatttcacgctaaacagccttcttcccggtgaaaaaaagctggcggaagagtttgcggtatcgcggatgaccatccgtaaagccattgacctgctggtagcgtgggggctggtggtccgccgccacggtagtggcacttacctggtgcgcaaagatgtactgcatcaaaccgccagtctgaccgggctggtggaggtgttaaaacggcagggaaaaacggtcaccagccaggtgctgatttttgaaatcatgcctgcgcctccggccattgccagccagttacggattcaaatcaacgagcagatctacttctcccgtcgcgttcgttttgtggaagggaaaccgctgatgctggaagacagctatatgccggtaaaactgttccgtaatctttcgctgcaacatctggaagggtcgaagtttgaatatattgaacaagagtgcgggattttgattggcggtaattatgaaagcctgacgccagtgctcgccgatagactgctggcgcggcaaatgaaggtagcggaacacacgccactgctgcggatcacctcgttgtcatatagcgagagcggggagtttttgaattattcagtgatgttcagaaatgccagcgaataccaggtggagtaccatttacggcgactccacccggaaaagagttaaccgatactccagaagagcaccgccagtaattggggggtgataatgcgcaggaacattaccaacggatagacagtggcgtaagagagcgccgccgcaccgctggttggatgaagattattagcaaacgccagcgccggaggatcggtcatggaacctgccagcatcccgcacatggtcaggtaattcattttggctaacatccgcgccagaatgccaacagtaatcagcggaacggcggtgatcagggcaccataaccaatccagcttagcccttcgccattgaccagggtattcacaaaatccccaccagatttcagaccaacgaccgagaggaacagcacgatccccagctcccgcagcgcgaggttggcgcttggcggcataaaccagtacagcttgccgatactgccgatacgcccgaggatcaacgccataatcagcggtccgcccgccagccccagtttcaacgcggccgggaatcctggcacaaagacgggaatagaacctaacaatacgcctagcccgatgccaataaacactggcagcatctgaacctgttgcagtttttgctgcgcattccccagcacattggcaacggcatcaattgcggacggacgccccaccagattgaggatatcgccgaactgcaggctgatatcgccactggcgaccagttcgaccccggcacggttcaggcgcgagataacaacgtcatagcgttctttaaagtgcaggtcgcgaatacgttttccgagcacgttttcattggtgaccaccacacgctcgacgcgcaaatcagtgcctttcgtggacagcgaagtatcgacctcctgaccaatcaccagttgcgcattatgtaaatccgctggctgacccaccagatgcagcaaatcgcccagttggataatggtatctggcgaaggaacttttagggtttcttcgcgtttcagacgcgagcagataattttgtcgccgttgagaatcggtacatctttaatggctaaatcatgcaggttagggttctcaacgcgaatattgatagtcttgatcagcgcgccgccattggtgcgtgaagactcgtgctgctgagcttctgtctcgacattgacgcggaaaataacccgcaacatccacatggtgaacaaaatcccgcaaatgccgaatggatacgccatcgcgtaactcatccccatctgatcgaccatttccattggtgtacccaggtcgcgcaaaatctgctgccctgcccccagcgctggcgtattggtaaccgcaccggagaaaatccccagcactaccggcagtggaatatcaaacagtttatgcaggatggcggtaaccagaccaccgatgatgacgatcagaacagcaaacaggttgaggcgtaatccggagacgcgcaatgaggcaaagaagcccggccctacctgaatcccgatagtataaacgaacaggatcaggccaaattcctgaataacatgcagcatatcgctacttaatgtcatccccgcctgagaaacaaaatggccgacgatgatcccaccaaacagcacgccgccaatacctaatcctatgccgcgaaatttgacgttgccgataaacaaaccgacgactgccaccaaagccagaatactgaccgttaatgctatatcactcatcgtccatttctcttgagataacattttaattgctacggattatggctgaatcggtgaagcagatttgccttatagcgcacattatcacgggaaagaacgtgccgaaatatcttaaacagtcgaaatttaacgcattgttgagtaagtaagacaaaaaaagccccaccagaatggcggggcaaagagaatagctagttagctatttaacgcgggacgttcgctgatagcgatacgctgcgctgcgatgggttcaggctcattacgaattaaatcaatatgcagtaaaccgtttacgaaggttgcgccagagacttccatattttcagccagcgtaaagctcaggctaaatggctgattcataagcccttgatgcagccattttttctcttcttttggctgctccggcgtgccttttacgctcaggcgcgtaccttccagttgaatctctaaatcttcctgacggaaacctgccagcgcaagggtaatgcggtagtggttatcgtcgcttttctcaatgttgtacggcgggaagctctggctttcaccggcgttttgcagtgcgttggccagtttgtcaaaaccgatccattgacgcatcagtggggataaatcgaagttacgcatagtcatttctccttctaagaagcgagtaagtacctgcaaatccgaagattcgcatatgctccctgacggcgagcatggagatgtcaggccgcgccaggcggccttagggaattagttgatttcgatacggcgcggttttttcgcttccggaatcacgcgttcgagatcgatatacagcaaaccatttaccaggttagcaccacgaacatgaatgttctcagctaactggaatttgcgttcaaagttgcgttcagcgatgccctggtacagataggtgcgctctttttgttcgtcggcgtgagcacctttcaccaccagcagattatcctgggcggtaatttccagttcgctctcagcaaaaccagccacagcgatagcaatgcggtaatggttttcgtctaccagttcaacgttatacggagggtagccgccattactctggctctggttgttttctaagtggttaaacaaacggtcaaatccaatagcagaacggtaaagcggggataaatcaaagttacgcataatcaatagctcctgaaatcagcgagaatgtaagaccttccacaatggacaggtcaggtagccagaacacccatcaggcgcgtcctcatcggctacgatgtaaaaatgggtctggaaatgaacttttcaagccttatcagcggacttttttttgcagtttatggtctattgcatagactgagggggcagcacgaaacgttaaagtgcgatagccgccacagtgcgacgtaatgatgatgttattttcagcaagggatcgctataactcatcaggccaacacccacgatcaacagatgaatttattatgataagaaatgtgttgttagcgttcatgatatgcagcggaatgacattactcggaggatgctccagcgtgatgtcccataccggagggaaagaaggaacgtatcccggcacccgcgccagcgcaaccatgattggcgacgatgaaaccaactggggcactaagtcgctggcgattctcgatatgccgtttaccgctgtgatggacacgcttttactgccgtgggatgtgttccgcaaagacagctcggtgcgctcgcgcgttgaaaaaagcgaagccaacgcgcaagccaccaatgcggttattccaccggccagaatgcctgataactgatttagcgatcagtttcggtgatccacagctggccgccttccatccacgccagccactgaccatccggcgagaagaccacggcgtccgcagaaggtgaattggcgtggtgttcggttaaatactcaacctcgccgctttgcgcatgggcacaagcaattcgattatccagcacaaagcccaaccattctcctgacggatgccagttaaatgcagactgaatatccgttttgttatgggttaactggcgcggctcgccgccctgtggcgagataagccacagttgcacaatgccgttatcatctcgcattaaaaacgcgatttgtgtaccctgcggattacagcgcacccagtggcgcgggacgttgactaaccccggataagcccgatggtgggtaaaggttaaacgtcgctgcacgacgccacgcggtggcgcgggcagggttgtttccgttccgcttaacggcgcatcacctgccgctttccagccagcttcatcttgcggtaactcaacgataaacagctccggcactttctcgccctttggcgaaagtgtgtcgccaataaatgccagcgcgtgatttcctacccatccttcttcataagcacgattgatttcatcactgccaggctgtggcgtgggcgtggttttgctcaccagcacgcaccagtggctaccgctgtattcacgcggatgctgcttttgtacgttgaccgggccaaacggcgcagcaacaccgacgtttcgcaaatccagcgccggatcgagttcatgcattacatggtcgttataggtaaagctcaccctttcaccgttcgggctaaagacatgcacatggctgccgccgcgcagcactcctggcgtatacggcgcggtaatatccatcgcatcaaggttactcatcttgccgccttcaacaatcactccgcgccgatgatggaagtcgtaatgccatgtttcatcaggattttccgggccgtggatgaaaacatatttctctgacttcggatgaacggtcaccacgccgacgtgtgcgccctgtgacgcgcgatagataacctcgacctcgccggtatggatattcacacgctcaatggtctcgccggtaaacgacgcgccagaaggacgcacgtcaaataccagccactggctgtcgggcgtccaggtattggtattggtgagcaggtgattacggggagcaaaggttatctgtttcatggcgcggtcctgatacaaaacgggtcccgccatcatacttcacaaggacttcactttcagacaatagtcttttgccatcgtgatgaatgtgagtgaaaagatggaacatttcgacgtggcgattattggcctcggcccggcaggatcggcgttggcacgaaagttagcaggcaaaatgcaggtgatcgcgctggataaaaagcaccagtgtggtactgaaggtttcagcaaaccctgcggcggtctgctggcaccggacgcgcagcgatcttttattcgcgatgggctgacgcttcctgtcgatgtgatcgctaatccgcagattttcagcgtcaaaaccgtcgacgtcgccgcatcgctcacgcgtaactaccagcgaagctatatcaatattaatcgccatgctttcgacttgtggatgaaatcgctgatccccgccagcgttgaggtttatcacgacagcctgtgccgaaaaatctggcgtgaggatgataaatggcatgtcatttttcgtgcagacggctgggagcaacatattaccgcccgctatctggtcggtgccgatggcgcaaactcgatggtgcggcgacatctctacccggatcatcaaatccgtaaatatgtcgctatccagcagtggttcgcggagaaacatccggtgccgttctactcctgcatctttgataattcgataactaactgttattcatggagtatcagcaaagacggttattttatctttggcggtgcctatccaatgaaagacggtcagacgcgtttcacgacgctgaaagagaaaatgagcgcctttcagttccagtttggtaagacggtgaaaagcgaaaaatgcacggtgctgtttccctcgcgctggcaggattttgtctgcggtaaggacaacgcctttctgattggtgaagcggcgggatttatcagcgccagctcgctggaggggattagctatgcgctggatagcacagacattctgcgttcggtgttactgaagcagccagagaagctcaataccgcttactggcgcgccacccgcaaactgcgtttaaaactcttcggcaagatagtaaaaagccgatgcctgaccgcaccggctttaagaaagtggattatgcgcagtggtgtggcacatattccacagttgaaggattagccaacgcgcttcacatcgcccaccagcaggatataagagagcgcgccaatcaacgcgacggcggagatataaaccagtgcaggtgcgaaaccgtaaccctgcgccaggtaccccaccaccagcggaacggtgatgccgcccagaccaccggcgaagttaaacacgccgccggttaaaccaatcaggcgcatcggtgccagagaagaaaccagcgaccaggtaatcgaagcaaaaccgttaccgaagaatgccagcgccatcaggcacataatcatcatcggatcgttagtgtagttagcgcccataatgcaggtggagatcagcaagccgcagataatcggcgttttacgcgcaaagcccagtgaaaagcccttacgtaccagcagatccgctacccagccagagagcaggacgccgacaaacgccgcgaggaatggcaccgtggtcataaagcctgctttcagcgccgtgattcctttttcctgggttaaatagttcgggaaccaggttaagaaaaaccacagtgtagaagccaccgcaaattgcccaagataaacgccgatcagtttacgatggaacaccagtttccagtctttggctgttaacggctgacgcgcctctttcttcaccggcgcatcaccatccaccagaccgccgccatcacgaatgtaatccagttcagctttgctgatacctttggtcaggcgcggcggctgataaaccttaaaccaaatcagcgaccagataatgccgataccaccagtgacaatgaacacccagtgccagctcaacatctcctgaatccagatcagcagcggcgtcagaaacgccagaccgacaaactgaccagacgtataaaaaccaacggcagaagcgcgttcatgttccgggaaccagctggtcaccatccggttattggtcgggaaagcaggcgcttcgaaaataccggttatcgcgcgcagaccaattaatgacattaagcccgtggcaaagccctggaataaagtcgccactgaccagccaaatatcgcaataaaataagtcacgcgagaacctacgcgatctaaaaaccaaccgccggggatctgacatagcgtataaagccaggcgaaggccgaaaatacatagcccatttccgctttggtaatgccgaactcttcctgaatatgggcggaagccacggccaggttggcgcggtcgacataacaaatgactaccgtaataaagatcatcaccagcgtcagataacgccgacgccccggctttgctgcattaacgggaatatccatagcgagctttctccagattttgggcatagcgaagccgctcaccatgccctgtaatttacagagggttatatttttgtattgctgttttagtgcccgatgaggggcttacgtggcaggaattaccactctgctacgctgttatcttcatgacgccagagcggattacgccagtccggggcatttttactgaactcaatcactttagcttcgtcgatttccacgcctaagcccggtttcgttaacggtttaaagaagccgccgaccatgctgaagtcttctttgtttttcacaaagtcgagtaactccgcgcctttgttgtaatgaattcccatactttgttcctgaagtacggcgttataggaaacaaagtcgatatgcaggcaagccgccagtgcaatcggtccgagcggacagtgcggcgcaagggtcacgtcataggcttctgccattccggcgattttgtagcattcggtaataccgcccgcgtgggagagatccggttgcagaatcgaaataccacctgcctccagcacgcgtttaaaatcgaagcgtgagaacatgcgttcacccgccgccagtggaatatgcgtttgtgccgccagtttcgggtagtattcggcttgttccgccagcaccggctcctcaataaacagcgggcgatacggctccagttctttaatcagcactttcgccatcggcgcgctgacgcgaccgtggaaatcaagaccaaactcaatctgattgccaaaagcttcacgaatttgtgccacggtgttaaccgccgcatctaccgcgcgggagttatcaattagccccagttcttcacaaccgttcagtttgaaggtatcgaagccgatttcgcgtagcgttttaatgccgtcgataacatccgccggacgatcgccgccaacccaactgtaggctttaattttgtcgcgaaccaggccgcccatcagttgccagaccggcgcattcagcactttacctttgatatcccataacgcctggtcaatcccggcgatggcgctcatcaggatcggaccgccgcgatagaatccggcgcgatacatcacttgccataagtcattgatgcgcgatggatcctgaccaatcaaatagtcacccagctcgtgaactgccgcttccaccgtacgggcgcggccttcgatcacgggctcgccccaaccgaccacgccttcatcggtttcaattttcaggaacatccagcggggaggtaaacgatacgtggtaattttggtgattttcattgcactgcctctcgatacgccttaacaaatgctgctgcctgctgcgcggtgcgctctacggattgcccggcgcgatagagatcgctgcctaagcccgcccctgcacaacctgcgtctatccactgcgccaggttttctggcgtcacgccgccaacggcaaagactgcgatgtccgatggcaataccgcttttaacgctttgatgtattgcggaccaaaagccgatgacggaaatattttcagcgcctgcgcgcccgcttcgagcgcggtaaaggcttcggtcgccgtcgcgcagccggggcagacggtcatgccgtagcccaccgcacggcggatcacttcactatggatattgggcgtaacgatgagctgacagcccatcctggcgagcgcatcgacctgttcaggtttcagtaccgtacctgcgccaatcaacgccttgtcgccgtacgcatcaacgatggcgggaatgctttgctcccattgtggggaattcagcgggatttcaaccgcgtcgaacccggcgtcaatcaccgcgccaacatgcgccagcgcctcgtcgggcgtaataccgcgcaaaatggcgatcagcgggagtttagtttgccactgcatgagcgatgctccttataccagcctgaaatgccgtgtcgcccgccaccgccgtcacgtcgcaacccatcgcctgaaaggcttgctggtagcgcgcggtcagcgatgttccggcgacaagggtgatggcgtgttgatgggccacatagtcgcgcatactggcgacctctgcgccaatcaacaaaccagagagaaattcgctgacctgttcgcggggaagtgttcccagcacatgcgaggcgcgaacttcaaaaagctgcggcaatatggcgggcgtattaagaccacgctcaaggccagctgtgaaggcatcggcagagttttcctgcggcggcaaacctgcgccaatcaatgagtgatttaacagtaaatgatgtaattcaccggtcatcacggtgcgaaaatcgttgatttgctggctatcggcctgcacccatttgcaatgggttccgggcatgacataaagagaggaaggagccagagctcgcgcgccgatcaattgtgtttcttcgccgcgcatcacattgtggttatcgtcatgagagacacataatccgggaataatccagatattgtcgccaactgacgttaattgttcgccaatagacgaaaaacaggcaggaacagataaatacggtgcaactttccagccgacgttgctgccaaccattcctgccattaccactggcgttttctcttcacgccagtcggtcgtgacttctgctaacaccgcagccggagattttccgttcaggcgcgtgacgcctgcttctgattgcctgctctccaggcagtggtcgccctgataaagccaggcgcgcagattggtcgatccccagtcaattgcgatgtagcgagctgtcatgtgatttcctttaaccttcgtgtcgagctggcgatcatggtaagcgccgcctgctctgccgcatcgccgtcctgatgtcgtatcgcatcgaacagcgccttatgttcctggagcgtttgcggcatgttggcctcatcgcccatccaggttcgttcaaaaaccgcccgctgcagcgaactgatcgcaatgctaagttgctgtaacaccgggttatgcaccgactgcagcaccgcctcgtggtagcgaatatccgcttcgttaaacgcttcgcggtcctgattgttggcaatcatctcgttcagcgccgattcaatctgcgccagatcgctggaagtcgcgcgctctgctgcccaacgggcaatcgccggttccaccagatttcgcacttcgctcatggcactgataagccgtgggtcgtagtcattttccagcacccattgcagtacgtcagtgtcgaggtaattccactggttacgcggtgccacaaacgccccgcgataacgtttcatttcaatcagccgcttcgccatcagcgaacggaacacctcacggatgatgttgcgcgaggttgcaaactcctcacagagttccgcctcagccggaagcggcgagcctggcacgtatttgccgtgaacgatctgtttacccagcgtaatgacaatgcgatcggttttattgagagtcatggagagtccttgtgctctgtatgttcttctctactttaccccgatcgatgcataacgcggcaactttgtagtaccagcgtgatgacgttcgcgtttgccgtgcgtgtaatgtagtacaaacttatattgttgtactacaatttagatcacaaaaagaacaatgcataaaaaaatgacatgcgtcgggcagaaatctgaaaagggatatcaggcgctaaacaggagggaaagaagagtatgctttcaacggcttagctactcgtttaaaggattaatcatgaagttgaattttaagggattttttaaggctgccggtttattcccactggcgctgatgctttcaggctgtatctcgtatgctctggtttcccataccgcaaagggtagttcaggaaagtatcaatcgcagtcagacaccatcactgggctatcgcaggcaaaagatagtaatggaacaaaaggctatgtttttgtaggggaatcgctggattaccttatcactgatggtgccgatgacatcgttaagatgctcaatgatccagcacttaaccggcacaatattcaggttgccgatgacgcaagatttgttttaaatgcggggaaaaagaaatttaccggcacaatatcgctttactactactggaataacgaagaagaaaaggcactggcaacgcattatggttttgcctgtggtgttcaacactgtaccaggtcactggaaaacctaaaaggcacaatccatgagaaaaataaaaacatggattactcaaaggtgatggcgttctaccatccatttaaagtgcgattttatgaatactattcacccagaggcattccggatggtgtttccgcagcattactgccagtgactgttacgctggacatcattactgcaccgctgcaatttctggttgtatatgcagtaaaccaataatcagtaagcgggcaaacgcgtttatgctgtttgcccgcccacagattaattcagcacatacttctcaatagcaaacgccacgccatcttcaaggttagatttggtgacaaagttcgccacttctttcactgaaggaatagcgttatccatcgccacaccgacgcctgcatattcaatcattgcgatatcgttttcctgatcgccaatcgccatgatttcttccggtttaatacctaacacgtcggccagtgatttcacccccgtacctttgttaacgcgtttatcgaggatttcgaggaagtacggcgcacttttcagcacggtatatttctctttcacttcctgcggaatacgcgcgatagcctggtcgaggatggcgggttcatcaatcatcatcactttcaggaactgggtattggggtccattttctccgcttcgcagaacaccagcggaatggtggcaacgaaggattcatgcaccgtgtagtagctgatatcacggttggcggtgtacagcgtggtgcggtccagggcgtggaaatgagaaccgacttcgcgagagagtttttccaggaaacgatagtcgtcatagctgagagcagtttgcgccacggtgctaccatcagcggccttctgtaccagcgcgccgttataagtaatgcagtagtcgcccggctgttccatatgcagctctttcaggtagttgtgcacacctgcatacgggcgacccgtcgttagcacgacattcacgccacgggcgcgagctgcggcaatcgcatttttaacggcgggtgaaatggtgtgatcgggcagcagaagggtgccatccatatcgatagcaatgagtttaatagccatgagttccccaggtagattggttcctgacccatgctaacgcgattccgctcaaaaatcagtacaacacccgagggaaaagggggatgcaacgcgcgttgcgtgctccctttttgcttagcggaagagtttccctttcagcagttccatgcctgcggaaagcagatcgttattggcttgtggtgacacttcaccttgcggtgagagcgcatcaataatcttcggcaattgttctgccagtaaactggaagctgtactggtatccacgccaagtttttgcccgagatcggacaccgcatttgtgccgagcgccgattccagttgctcgccactaaccgattgattgccctgttgattactcagccaggttgagagaatggcccctaagccgccactttgcagtttttccagcagcacctgaatgccgccctgctcctcaacccaacttaaaatagcctgatatttccccgcatcgcctttcagaaaggcaccgacaacttcatcaaaaagccccatgataatcacctgtaaagcgttacgtgttgacccaaaaagtatagatttgcgggatgataattgcggattgcagaaataaaaagggcggagatgatctccgcccttttcttatagcttcttgccggatgcggcgtgaacgccttatccggcctacaaaatcatgaaaattcaatacattgcaagattttcgtaggcctgataagcgtagcgcatcaggcacgctcgcatggttagcgccattaaatatcgatattcgccgctttcagggcgttctcttcaataaacgcacggcgcggttcaacggcgtcgcccatcagcgtggtgaacaactggtcggcagcaatcgcatctttaacggtaacgcgcagcatacgacgactttccgggtccatagtggtttcccacagctgttccgggttcatctcgcccagacctttataacgctggatggagaggccgcgacgggactctttcaccagccagtccagcgcctgctcgaagctggctaccggctgacgacgctcgccacgttcgataaacgcatcttcttccagcaagccacgcagtttctcacccagcgtgcagatacgacgatattcgccaccggtgataaactcgtgatccagcggatagtcagtatccacaccgtgggtacgcacgcgaacaatcggctcgaacaggttttgctcagcattggtgtgaacatcaaacttccactggctgccgtgctgttctttgtcgttcagttcgctgaccagcgcgttcacccagcgggtaacggtctgctcatcagaaaggtcagcttccgtcaacgtcggctgatagataagctctttcagcattgctttcggataacgacgctccatacgattgatcattttctgcgtcgcgttgtactcagataccagtttctctaacgcttcgccagccaatgccggtgcactggcgttggtgtgcagcgttgcgccgtccagcgcgatagagatctggtactgatccatcgcttcgtcgtctttaatgtactgttcctgcttgcctttcttcactttgtacagcggcggctgagcgatgtagacgtgaccgcgttcaacgatttccggcatctgacgatagaagaaggtcaacagcagcgtacgaatgtgcgagccgtcgacgtccgcatcggtcatgatgatgatgctgtgataacgcagtttgtccgggttgtactcgtcacgaccgataccacagccaagcgcggtgataagcgtcgccacttcctgagaagagagcatcttatcgaagcgcgctttctcgacgttgaggattttacccttcagcggcagaatcgcctggttcttgcggttacgcccctgcttcgcagagccgcccgcggagtccccttccaccaggtacagttcggaaagcgccggatcgcgttcctggcagtctgccagtttgcccggcaggcccgctaagtcgagcgcacctttacggcgggtcatttcacgcgcgcgacgcgccgcttcacgggcacgggcagcatcgataattttgccaaccacgattttcgcgtcggttgggttttccagcaggtattctgccagcagttcgttcatctgctgttcaaccgccgatttcacctcagaagaaaccagtttgtctttggtctgggaggagaatttcgggtccggcactttcacggaaacgaccgcaatcaggccttcacgcgcatcgtcaccggtggcgctgactttggcttttttgctgtagccttctttgtccatgtaggcgttcagggtacgggtcatcgccgcacggaagcctgccaggtgagtaccgccgtcacgctgcggaatgttgttggtaaagcagtagatgttttcctggaagccatcgttccactgcaacgccacttcgacgccaataccgtctttttcagtggagaagtagaagatattcgggtggatcggcgttttgttcttgttcagatattcaacgaacgccttgatgccgccttcatagtggaagtggtcttctttgccgtcgcgcttgtcgcgcagacgaatggaaacgccggagttgaggaacgacaactcacgcagacgtttcgccagaatttcatattcgaactcggtcacattggtgaaggtttcgaggctgggccagaaacgcaccatggtgccggttttttcagtctcgccggtaaccgccagcggggcctgcggtacaccgtgttcgtagatctgacggtgaattttaccctcgcgctggataaccagctccagtttttgcgacagggcgtttactaccgaaacaccaacgccgtgcagaccgccggacactttataggagttatcgtcaaatttaccgcctgcgtgcagaacggtcatgatcacttccgccgccgatacgccctcttccgggtgaataccggtcggaatgccgcgcccgtcatcctgtacagagacagagttatcggcgtgaatggtgacgataatttctttacagtgacccgcgagcgcttcgtcgatagcgttatctaccacctcgaataccatgtggtgcagaccggtgccgtcatccgtgtcgccgatatacatacccgggcgcttacgcaccgcatccagccctttcaggactttgatactggaggagtcataagaattcgacatcaacgtttctcgctcatttatacttgggttaatccgttattttacccttttccacggtaaacatcttcgaattttcgtccgacatgtctataacgtgttcagcactgatcgcgctgacaaagacctgtgattgcgtcgcttttaagcggctggcaagcagcccgcgacgctcatcatcaagctcagaggcaaaatcatctatcaggtagagacaccgccgcccgctttcacgggtgaggaactctccttgcgccagacgtaaggcgcacatcaacagcttaagctgcccacgcgataaggtatcttccaccggcgcaccgtcggcgcgaatgcgtaagtccgctttgtgcgggccgtgcgcggtgtaggttagctggcgatcgcgttcaaaattacgttccagcacctcagcatattctgtctctttctcccagccgcgctggaaagagaaagtcagagaaaactcagggagaaattgcttacaggtatcagccatatcggccgcgataccggcgctatactccgcgcgccaggtgctgatttgctccgccagcgggatcagctctttatcccacgggcgtagctgttcgtaacgtgtcacctggcgcagcgccgcattgcgctgcttgagcaatcgcttgagattgctccaggcggtgaaaaatccgggttcgttgtgaaagcatccccagtcgaggaatgctcttctgtatttggggccgccgttgagtaaagtaaacccttctggcgttatcaactgcattggcatcaggtgcgccagttccgcgaccttatgcccgtctgtaccgtcgatgcggactttgctgtcgccctgtttgtctttggttaagccaatcgctgtctcgcgctcttcgccctgtaatcgcccgtggagaacaaacgcctcctgctcatggcgaatgacgcgaccaatctgcaaactgcgaaacgcccgaccatggccgagcgtatagatggcttccagcacgctggttttgccactgccgttggcacctaccagaaagttaaagccgggagataaggcgagatccgcggtttcaatgttgcggaaatcgcggatcaacaagcgggtgagggacattacagtctcattggcatgacaacataagccgcgctctggctggccgcatcttcaatctgcacgctggaaaccgaatcggtcagcatcatgcggacgttttcgcatttcagcgcgttcagaacatccagcacataactgacgttgaagccgatttccatctccgcaccgctataggtaacgtcgaggatctcttccgcttcttcctgttccgggttgttggcggtgattttcagctggttttcgctgacataaagacgtacgccgcggaatttctcgttagagagaatcgccgcgcgagcaaacgcctgcttgagcagatcgcagccagcttccagatgtttgtccgggttcttcggcagaacgcggcgataatccgggaagcgaccatccaccagtttggaggtgaagataaagtcgccaacgtgggcgcgaatgttgttgctgccaatctgtacgcgcagcggattgtcgccgccgtcgagcatacgcatcagttcaatcacgcctttacgcggtacgatcaccgaatggcttggcaaagattgaccaattggcattgaacagaccgccagacggtggccgtcggttgccacggtgcgcagttcttcaccttcggtttcaaacagcataccatttaagtaatagcgaacgtcctgatgcgccatagaaaactgggtcgcttcaatcagacgcttcatcgttgcctgcggcagggtaaattcgacttcactctgccagtcatcgaggttcgggaaatccgccgctggcagggtagacagcgaaaaacggctacgcccggagcgtaccagcatccgttcaccttccagctgcacggcaatttccgcgccttcaggcagaccacggcagatatcaaagaatttgcgcgccggaacggtcgtcgctcctggctcgtgtggctgaaccagcgcaacacgtgccaccatttccatctcgagatcagtaccggtcagcgacaacgtaccgtcagcaacctgtaacagcagattaccgagaatcggtagcgtaggacgaccacctaacggaccgctcacctgttgtagcggttttaataaatgctcacgttctacggtaaatttcataggtttacgatgacaatgttctgattaaatttgaaaaatcttctttgatatcgtggctctcttcacgcaactgctcgatcttacggcaggcatgaagcaccgtcgtgtggtcacggccaccaaacgcatcgccaatctccggcagactgtggttagtcagctctttcgccagcgccatcgccatctggcgcggacgcgccaccgagcgggatcgacgcttggaaaggagatccgcgactttgatcttgtagtactccgccaccgtcttctgaatattgtcgatggtgaccagtttttcctgcaatgccagcaagtcgcgcagcgcctcacgcacgaagtcgatggtgatcgcccgtccggtaaagttggcattggcaatgacgcggttcagcgccccttccagctcacgtacgttagatcgtagacgcttggcgataaagaacgccacttcgcccggcaaacgaatgtcgttttcgtcggcctttttcatcaggatcgccacacgggtttccagctctggcggttcgatcgccacagtcagtccccaaccgaagcgggatttcaaacgatcctcaacgccgttgatctctttcggatagcgatccgaggtgagaatgatctgttgattaccttccagcagggcgttgaaggtgtggaaaaactcttcctgagatcgttctttattagcaaaaaactgaatatcgtcgatcagcagtgcatctacggaacggtagtagcgtttaaactcttcgatcgcgttgttttgcagggctttaaccatgtcctgaacaaagcgctcggagtgcatataaaccactttggcattcggcttgcgcgccataatgccgttacccaccgcatgcagcaggtgagttttacccagacccgtgccgccataaaggaacaacgggttataggcaccgccagggttatccgccacctggcgagccgccgcgcgcgccagttggttagatttaccttcaacgaagttatcaaacgtgtgtttgacgtttacgttagaacgataggtcggttctgccggggccgggacgttatcccaacctgagcgcgtagaaggcgcagcacgttgcggctgcgtttgcgccacctgtgcaggggccgcgacgttgctcgtcactgccgcttgtggcgtttgcgtcaccggtttggtgccgacttcaaaacgcagctgtggggcatccgctccgcagaaactggttagcagtccattgatattattaaggtacttgtcccgtacccaatcgaggacaaaacggtttggcgcgtacagggccagcgtgttatcgctcagttccgcctgcaatgggcgtatccacatactgaattctgtggctggtaactcatcctgcaatcgggcaagacactgctgccaaagcgaaagtgacacggcggactccactcgaacaaaagtcgataatgactaaggctgaaacattcatgattgttgacgtacgtcgaaaagaccctgcttgagggtgacgcacgaaccgctgtctgcggttatatgcccgatcaagatcctgcaaaacgatcgggaccgcggatcatagcctaaactgcgcaagagatcttctgtttctcacagattttcccgatttatccacaggactttccagaactcgctaagtgtaaacgatcctgccgcgaggcgggcacgatttacgccgcatattggaaaatttaatgaccatagacaaaaattggcttaatcgatctaataaagatccaggacgatccttgcgctttacccatcagcccgtataatcctccacccggcgcgccatgctggtttccactggtgtgaggtcgtacattttccctgcgaaaaggtgcggaaaagcgcggtaaataaggaaagagaattgactccggagtgtacaattattacaatccggcctctttaatcacccatggcttcggtgtccatcgtttcatttttcggcggatatccaataaagccattgaatttattcaagtttaggtagaaatcgccatgaaacgcacttttcaaccgtctgtactgaagcgcaaccgttctcacggcttccgtgctcgtatggctactaaaaatggtcgtcaggttctggcacgtcgtcgtgctaaaggccgcgctcgtctgaccgtttctaagtaataaagctaacccctgagtggttaagctcgcatttcccagggagttacgcttgttaactcccagtcaattcacattcgtcttccagcagccacaacgggctggcacgccgcaaattaccattctcggccgcctgaattcgctggggcatccccgtatcggtcttacagtcgccaagaaaaacgttcgacgcgcccatgaacgcaatcggattaaacgtctgacgcgtgaaagcttccgtctgcgccaacatgaactcccggctatggatttcgtggtggtggcgaaaaaaggggttgccgacctcgataaccgtgctctctcggaagcgttggaaaaattatggcgccgccactgtcgcctggctcgcgggtcctgatagccctcattcgggtctatcaacgcctgattagtccgctactcgggccgcattgtcgtttcactccaacctgttcaagctacggaattgaggcattgcgcaggtttggagtgataaaaggcagttggttgacggtgaaacgcgtattaaaatgccaccctttacaccctggtggtgacgatcccgtcccgcccggaccatttgataccagagaacactaacgatggattcgcaacgcaatcttttagtcatcgctttgctgttcgtgtctttcatgatctggcaagcctgggagcaggataaaaacccgcaacctcaggcccaacagaccacgcagacaacgaccaccgcagcgggtagcgccgccgaccagggcgtaccggccagtggccaggggaaactgatctcggttaagaccgacgtgcttgatctgaccatcaacacccgtggtggtgatgttgagcaagctctgctgcctgcttacccgaaagagctgaactctacccagccgttccagctgttggaaacttcaccgcagtttatttatcaggcacagagcggtctgaccggtcgtgatggcccggataacccggctaacggcccgcgtccgctgtataacgttgaaaaagacgcttatgtgctggctgaaggtcaaaacgaactgcaggtgccgatgacgtataccgacgcggcaggcaacacgtttaccaaaacgtttgtcctgaaacgtggtgattacgctgtcaacgtcaactacaacgtgcagaacgctggcgagaaaccgctggaaatctcctcgtttggtcagttgaagcaatccatcactctgccaccgcatctcgataccggaagcagcaacttcgcactgcacaccttccgtggcgcggcgtactccacgcctgacgagaagtatgagaaatacaagttcgataccattgccgataacgaaaacctgaacatctcttcgaaaggtggttgggtggcgatgctgcaacagtatttcgcgacggcgtggatcccgcataacgacggtaccaacaacttctataccgctaatctgggtaacggcatcgccgctatcggctataaatctcagccggtactggttcagcctggtcagactggcgcgatgaacagcaccctgtgggttggcccggaaatccaggacaaaatggcagctgttgctccgcacctggatctgaccgttgattacggttggttgtggttcatctctcagccgctgttcaaactgctgaaatggatccatagctttgtgggtaactggggcttctccattatcatcatcacctttatcgttcgtggcatcatgtacccgctgaccaaagcgcagtacacctccatggcgaagatgcgtatgttgcagccgaagattcaggcaatgcgtgagcgtctgggcgatgacaaacagcgtatcagccaggaaatgatggcgctgtacaaagctgagaaggttaacccgctgggcggctgcttcccgctgctgatccagatgccaatcttcctggcgttgtactacatgctgatgggttccgttgaactgcgtcaggcaccgtttgcactgtggatccacgacctgtcggcacaggacccgtactacatcctgccgatcctgatgggcgtaacgatgttcttcattcagaagatgtcgccgaccacagtgaccgacccgatgcagcagaagatcatgacctttatgccggtcatcttcaccgtgttcttcctgtggttcccgtcaggtctggtgctgtactatatcgtcagcaacctggtaaccattattcagcagcagctgatttaccgtggtctggaaaaacgtggcctgcatagccgcgagaagaaaaaatcctgattcggtgagttttcgctaaaataagggcggtcagttgaccgccttttttcttttcgtagggcggataagcaccgcgcatccgccacacaaagcaacaggaacatcatgagcgataatgacactatcgtagcccaggccacgcctccgggacgtggcggcgttggcatcctgcgcatctccggcttcaaagcccgtgaagttgccgaaaccgtgctgggtaaactgcctaagccgcgctacgccgattatcttccgtttaaagacgccgacggcagcgtgctcgatcaggggattgcgctatggttccctggcccgaactcgttcaccggcgaagatgtgctggaactgcaaggtcatggcggtccggtgatcctcgacctgctgttaaaacgcattctgaccattcccggcctgcggattgctcgccctggtgagttttccgaacgcgcgtttcttaacgataaacttgacttagcccaggccgaggcgattgccgatcttatcgacgccagttcggaacaggcggcccgttcggcacttaactcgctgcaaggcgcattctccgcacgggttaatcatctggtagaagccctcacccacttgcgcatttacgtcgaagcggcaattgatttccccgatgaagagatcgatttcctctccgacggaaaaattgaagcccagctcaatgacgttattgccgatcttgatgcagtgcgtgctgaagcacgtcagggtagtttgttgcgcgaagggatgaaagtggtgattgccggacgtcctaacgccggtaaatcgagcctgttaaacgcgctggcggggcgtgaagcggcaatcgtaaccgatatcgccggaactacgcgtgacgtgctgcgtgagcatatccacattgacggaatgccgctgcatatcatcgataccgccgggctacgtgaagccagtgacgaagtagaacgtattggtatcgagcgcgcgtggcaggaaattgaacaggccgaccgcgtgctgtttatggtcgatggcaccacaacagacgccgtggatccggcagagatctggccggaatttattgcccgtctgccagcgaaactgccgatcaccgtggtgcgcaataaagccgatatcaccggcgaaacgctgggaatgagtgaagtgaacggtcacgcgttaattcgtctctcggcaaggactggtgaaggcgtggacgtgctgcgtaaccatctcaaacagagcatgggctttgacaccaacatggaaggcggcttcctggcgcgtcgtcgccacctacaggcgctggaacaggcagcggaacatctacaacagggcaaagcgcaactgttgggagcctgggcaggtgaactgctggcggaagagttgcgtctggcacagcagaacttaagcgaaatcaccggggaatttacttcagacgacctgctggggcggattttctccagcttctgtattggtaagtaaccgcgcttacgaagccgcattctgactgtcagatgcggcttcgcttcattgttaccactcctgttattcctcaaccctttttttaaacattaaaattcttacgtaatttataatctttaaaaaaagcatttaatattgctccccgaacgattgtgattcgattcacatttaaacaatttcagaatagacaaaaactctgagtgtaataatgtagcctcgtgtcttgcgaggataagtgcattatgaatatcttacatatatgtgtgacctcaaaatggttcaatattgacaacaaaattgtcgatcaccgcccttgatttgcccttctgtagccatcaccagagccaaaccgattagattcaatgtgatctatttgtttgctatatcttaattttgccttttgcaaaggtcatctctcgtttatttacttgttttagtaaatgatggtgcttgcatatatatctggcgaattaatcggtatagcagatgtaatattcacagggatcactgtaattaaaataaatgaaggattatgtaatggaaaactttaaacatctccctgaaccgttccgcattcgtgttattgagccagtaaaacgtaccactcgcgcttatcgtgaagaggcaattattaaatccggtatgaacccgttcctgctggatagcgaagatgtttttatcgatttactgaccgacagcggcaccggggcggtgacgcagagcatgcaggctgcgatgatgcgcggcgacgaagcctacagcggcagtcgtagctactatgcgttagccgagtcagtgaaaaatatctttggttatcaatacaccattccgactcaccagggccgtggcgcagagcaaatctatattccggtactgattaaaaaacgcgagcaggaaaaaggcctggatcgcagcaaaatggtggcgttctctaactatttctttgataccacgcagggccatagccagatcaacggctgtaccgtgcgtaacgtctatatcaaagaagccttcgatacgggcgtgcgttacgactttaaaggcaactttgaccttgagggattagaacgcggtattgaagaagttggtccgaataacgtgccgtatatcgttgcaaccatcaccagtaactctgcaggtggtcagccggtttcactggcaaacttaaaagcgatgtacagcatcgcgaagaaatacgatattccggtggtaatggactccgcgcgctttgctgaaaacgcctatttcatcaagcagcgtgaagcagaatacaaagactggaccatcgagcagatcacccgcgaaacctacaaatatgccgatatgctggcgatgtccgccaagaaagatgcgatggtgccgatgggcggcctgctgtgcatgaaagacgacagcttctttgatgtgtacaccgagtgcagaaccctttgcgtggtgcaggaaggcttcccgacatatggcggcctggaaggcggcgcgatggagcgtctggcggtaggtctgtatgacggcatgaatctcgactggctggcttatcgtatcgcgcaggtacagtatctggtcgatggtctggaagagattggcgttgtctgccagcaggcgggcggtcacgcggcattcgttgatgccggtaaactgttgccgcatatcccggcagaccagttcccggcacaggcgctggcctgcgagctgtataaagtcgccggtatccgtgcggtagaaattggctctttcctgttaggccgcgatccgaaaaccggtaaacaactgccatgcccggctgaactgctgcgtttaaccattccgcgcgcaacatatactcaaacacatatggacttcattattgaagcctttaaacatgtgaaagagaacgcggcgaatattaaaggattaacctttacgtacgaaccgaaagtattgcgtcacttcaccgcaaaacttaaagaagtttaattaatactacagagtggctataaggatgttagccactctcttaccctacatcctcaataacaaaaatagccttcctctaaaggtggcatcatgactgatcaagctgaaaaaaagcactctgcattttggggtgttatggttatagcaggtacagtaattggtggaggtatgtttgctttacctgttgatcttgccggtgcctggtttttctggggtgcctttatccttatcattgcctggttttcaatgcttcattccgggttattgttattagaagcaaatttaaattatcccgtcggctccagttttaacaccatcaccaaagatttaatcggtaacacctggaacattatcagcggtattaccgttgccttcgttctctatatcctcacttatgcctatatctctgctaatggtgcgatcattagtgaaacgatatcaatgaatttgggttatcacgctaatccacgtattgtcgggatctgcacagccattttcgttgccagcgtattgtggttaagttcgttagccgccagtcgtattacctcattgttcctcgggctgaagattatctcctttgtgatcgtgtttggttcttttttcttccaggtcgattactccattctgcgcgacgccaccagctccactgcgggaacgtcttacttcccgtatatctttatggctttgccggtgtgtctggcgtcatttggtttccacggcaatattcccagcctgattatttgctatggaaaacgcaaagataagttaatcaaaagcgtggtatttggttcgctgctggcgctggtgatttatctcttctggctctattgcaccatggggaatattccgcgagaaagctttaaggcgattatctcctcaggcggcaacgttgattcgctggtgaaatcgttcctcggcaccaaacagcacggcattatcgagttttgcctgctggtgttctctaacttagctgttgccagttcgttctttggtgtcacgctggggttgttcgattatctggcggacctgtttaagattgataactcccacggcgggcgtttcaaaaccgtgctgttaaccttcctgccacctgcgttgttgtatctgatcttcccgaacggctttatttacgggatcggcggtgccgggctgtgcgccaccatctgggcggtcattattcccgcagtgcttgcaatcaaagctcgcaagaagtttcccaatcagatgttcacggtctggggcggcaatcttattccggcgattgtcattctctttggtataaccgtgattttgtgctggttcggcaacgtctttaacgtgttacctaaatttggctaaatccttcaagaagccagccattcgctggcttcttgcctctcaggaaatcacttatgtccaaatggcaactcgcctgatcctccttcaccacgtatgctttgcgtcaccttactatcaggacgctttagcccatgtcccgctttttgatttgtagttttgccctggttttactttatcccgccgggattgatatgtacctcgttggtttaccgcgcatcgccgccgatctcaatgccagcgaagcgcagttgcatattgcgttctccgtatatctggcggggatggcagctgcgatgttatttgccggtaaagtggccgatcgttcagggagaaagccggtcgccatacccggcgcggcgctatttattattgcctcggtgttctgttcactggctgaaaccagcacgttatttcttgcaggccgatttctacaggggttgggcgcaggctgttgttacgtagtggcgttcgctattttgcgcgacacgctggatgatcgacgtcgggctaaagtgctgtcattactcaacggtattacctgcatcattccggtgttagcgccagtgctcggacatctgattatgcttaaattcccgtggcagagtctgttctgggcgatggcaatgatgggcatcgcggtactgatgttgtctttgtttattttaaaagaaacgcgcccagcggcccccgcagcttcggataaaccacgagaaaatagcgagtcgctgcttaaccgttttttcctcagccgtgttgttatcaccaccctcagcgtttcggtgatcctcactttcgtcaacacgtcaccggtattgctgatggaaatcatggggtttgagcgcggtgaatacgccaccattatggcgctgaccgctggcgtcagcatgaccgtttcattctccacgccatttgcgctgggaatttttaagccacgtacgttgatgatcacctcgcaggtgttattcctggcggcggggatcactcttgccgtttcaccttcccatgcggtttctctgtttggtatcacgctgatttgcgccggtttctcggtaggttttggtgtggcgatgagtcaggcgttagggccgttttcattacgcgcgggcgtagccagctcgaccttaggtattgcgcaggtttgcggttcgtcactgtggatttggctggcagcggtggttggtatcggcgcatggaatatgctgatcgggattctgattgcctgtagcatagtgagcctgttgctgattatgttcgtcgcgcctggacgccccgttgccgctcatgaagaaatccatcaccacgcttgatctcaatctgctgctttgtctgcaactgctgatgcaggagcgcagcgtaaccaaagcggcgaagcggataaacgtgacaccttcggcggtgagtaagtcgctggcaaagttaagagcgtggtttgacgacccgctctttgtgaactcaccgctgggtctgtcgcccacaccgctgatggtcagcatggagcaaaatctggcggagtggatgcaaatgagcaacctgctgctggataaaccgcaccaccagacaccgcgcggcctgaagtttgagctggcggcggaatcaccgctgatgatgatcatgcttaatgcgctgtcgaaacagatctaccaacgttacccgcaggcgaccatcaaattacgtaactgggattacgattccttagatgccattactcgtggtgaagtggatatcggtttttccggtcgcgaaagccatcctcgctcgcgggagctgttaagctcgctaccgttagccattgattatgaagtgctgtttagtgatgtgccctgcgtctggttacgcaaagatcatccggcactgcatcaaacgtggaatctggacaccttcttacgttatccgcatatcagcatttgctgggaacagagcgatacctgggcgctggacaatgtgttacaggagctgggacgcgaacgcacgattgctatgagcctgccggaattcgagcagtcactgtttatggcagcgcaacccgacaatctgctactggcgaccgcgccgcgctactgtcagtactacaatcaactccatcaactgccgttggttgctcttcctctcccgtttgacgaaagccagcaaaaaaagctggaagttccttttaccctgctgtggcataaacggaacagccataatccgaagatcgtctggttacgggaaaccattaaaaacctttacgcgtcgatggcataaccgaatcgtatgaaacgcgacccaatttcacaataaaatgtaaaaaagttgtaataagcttgtctgaatcgaacttttagccgctttagtctgtccatcattccagtaaatgattactcttgtattcataatggaccattaagcatggagcgaaaaatggcgactcactttgcccgagggattttaacggaaggacatctgatttctgttcgtctcccctcccagtgtcatcaagaagcccgaaacattccccctcatcgtcaaagccgttttctggcgtccagaggtttactcgcagaactgatgttcatgctgtatggcattggcgaattgccggaaatcgtcaccctgccgaaaggtaaaccggttttcagtgataaaaatttgccttcgttttccatttcctatgccgggaatatggttggcgtggcgttaacaaccgaaggtgaatgtggcctcgatatggaactacagcgtgcgacgcgcgggtttcatagcccacacgcgcccgataaccacaccttttccagcaatgaatcgctatggatcagtaaacaaaacgatcctaacgaagcgcgggcgcagctcatcacgctgcgccgaagcgtgctaaaactaaccggtgatgttttgaatgacgatccgcgcgatctgcagctgctgcccattgccggacgcctgaaatgtgctcatgtaaatcatgtagaagcgttatgcgacgcggaagacgtgctggtgtggtccgtggcggtcacgcccacgattgaaaagctcagtgtctgggagttagatggcaaacacggctggaaaagcctgccggatattcacagccgcgccaacaatcctaccagccggatgatgcgttttgcccaactctctaccgtgaaggctttttcgccaaattgatagacaaccacaggagtcatcatgtctgaaaaattgcaggtggttacgttactggggagcctgcgcaaaggctcatttaatggcatggttgcacgtaccctgccgaaaattgctccggcgagcatggaagtcaatgcgttaccatccattgccgacattcccttgtatgacgctgacgtacagcaggaagaaggttttccagcaacggttgaagctctggcggaacagatccgtcaggctgacggtgtggtgatcgtcacgccggaatataactactcggtaccgggtgggctgaaaaatgccatcgactggctttcccgcctgccggatcaaccgctggccggtaaaccggtattgattcagaccagctcaatgggcgtgattggcggcgcgcgctgtcagtatcacctgcgccagattctggttttcctcgatgcaatggtgatgaacaagccggaatttatgggcggcgtgattcagaacaaagttgatccgcaaaccggagaagtgattgatcagggtacgctggaccacctgaccgggcaattgaccgcatttggtgagtttattcagcgagttaagatctaaataaaaaacccgccagcaatcatgcatggcgggtttttaacgcgctatcgattttagtgagcgtcgataaagacaatcttcaggataaacagcagcgcaacgatgattacgcacgggcttagatcacgcagacgtccggtaccgattttcatcacgcagtaggagataaagcccagcgcgataccttcggtaatcgagaagctgaacggcatcatcacggcggtaataaacgccggaacagattcagtaagatcctgccagttcacgcgtgccagactggaagtcatcagcacgccaacgtaaatcagcgcaccagctgcagcgtagcctggcaccatccccgccagcggcgacagaaagataaccagcaggaacagcagaccaacaaccactgccgtcagaccggtacgaccgccaaccgatacgccggaagaggactcaatataagccgtaacggaagaagtaccgataaacgaaccggtcacggaagagatactgtcgacatacagcgcctgcttcatgcgcgggaatttccccttctcatccgccagacctgctttatcggtcacgccaatcagcgtaccggaggagtcaaacaagttgaccaacatgaaagagaaaatcacccctgccagcccgaggttaaacgacccggctaaatctacatgacccacaactgtcattacgctcggcggcgcagaaacgatgccattgtagtgcacatcacccagcatccagcccagcagcgtcgtcaccacgatagaaaccagcaccgctgcgtgaatgttgcgcgaggccagaatagcaatgatgaagaagccgaggatacccagaagtacgctgtgagaagtcagattaccgatgctcaccagcgtttccgggttagcgacaatcacacctgcgtttttcagccccatcatgccaatgaacagaccgataccgctggtaatacccacacgcagactcaccggaatgttggctatcatccagtagcgaacgcggaaaatcgtcagtaacagcagacctatcgcgccccagaagattgcgcccatcccgacctgccacggcaagcccatcgcctgtacaacgacaaaagcgaagaacgcattcaggcccatagcgggtgccagtgcaactggcaggttagcaaacagtcccatcataatactgccgaatgcagcgatcagacaggtagtgacgaagacggcgctggtatccatgccagcaacgccaagaatttgcgggttaacaaaaacgatgtaaaccatcgtcaggaaggtggtaaaaccggcgatcacttcggtccgtgccgtcgtgccatgttcgcgcagtttaaacacgcgttccagcatcccctgaccagaagtctgggtggtatgttgatgactcattatctatttccgaacaaggagggaaaatccgtcgctatcgtataccaaaatgcgacaataggcgcgtttgtgagagacttttttattggatttacttatacggcaacgattgcgttgcgcaaatcggctctacgaaaacgttaaactgattaaaaaggaaaggcatgtcccggatagaagcggtatttttcgactgcgacggtacgctggtcgacagtgaagtcatttgctctcgcgcatatgtaacgatgtttcaggaatttggtattacgctcgatcctgaagaggtattcaaacgtttcaaaggtgtaaaactgtacgaaattatcgatattgtttcccttgaacatggtgttacgttagcgaaaacagaagctgaacacgtttaccgtgcagaagtcgctcggctgttcgattcagaactggaagccatcgaaggggctggagcgctcctgtcagcgatcactgcgccaatgtgtgtggtatctaacggcccaaataacaaaatgcagcattctatgggcaagctgaatatgttgcactacttcccggataaactgttcagcggctacgatattcagcgctggaagccagacccggcgttaatgttccatgcggcaaaagcgatgaatgtaaatgtagaaaactgcattctggttgatgactcagttgccggtgcacaatctggtatcgacgcaggtatggaagtgttctacttctgcgccgacccgcacaataagccgatcgttcacccgaaagtcaccacctttacccatctttcgcagttacctgaactgtggaaagcgcgtggttgggatattacggcatagttcttcacactcccttcacttaccccgcttaaattggcgctcaaaggtaagtaaagggagtttgatatgtctgtttcacgtcgggtaatacatcacggactttattttgcagttttaggaccgttaattggtgttctgtttcttgtcctctacatattcttcgcaaaagaaccgctggttctttgggtgataatacatccaatttttctcttattgtcgataactacgggagctattcctgcgttgttaaccggtgtaatggttgcctgtctgccggaaaagatcgggtcacagaaacgttatcgttgtctggctggtggcataggtggcgtcgttatcaccgagatctattgtgcagttattgtacatattaagggcatggcttcctcggagttgtttgaaaacattctttctggtgacagtctcgttgtccgcatcattcctgcattgctggcaggtgtggtgatgagcagaatcattacccgtctacccggattggatatttcatgtcctgaaacagactctttaagttaagcgggatactttatctttgggctactcaaaagcagacaggatgtttctatgactcaaaatatcaggccgttaccccaattcaaatatcatcccaagccactggaaacaggcgcatttgaacaggataaaaccgtagagtgcgattgctgtgaacaacagacgtcagtttattactcgggtcccttttattgcgttgatgaagttgaacatctctgtccgtggtgtattgcggacggttctgctgctgaaaagtttgcaggtagttttcaggatgatgccagcatagaaggtgttgaatttgagtatgatgaagaggacgaatttgccggtattaagaacacatatcctgatgaaatgctgaaagagttggttgaacgcacgccaggttatcatggatggcagcaggaattctggctcgcgcattgtggcgatttctgtgtttttatcggctatgtgggctggaatgatataaaagatcgcctcgatgaatttgccaaccttgaagaagattgtgagaatttcggtattagaaattctgatctagctaaatgcctgcaaaagggtggtcattgtcagggttatctcttccgctgtctccactgcggcaagctgagactgtggggtgatttttcgtagttatttaaataatgagaacaggccggagcgtaattcacacatccggccttatttcttaagcttaaccgagtgctaattctgcggcagcggctttatcagcgattaccatcagcgaaggatgcagctgcaacacggaagctggaacatcttcggtaaccggaccttgcagaacatttttcagtgcctgcgctttacccgcgccgctgacaattatcagcaagtttttcgccgccatgatgcttttcggccccatcgtcacgtagctgtcaggcactaacgaaaagtcgccgcccaactcgccatgcgccacaatatcaaccatctctccctggatcgggaactccacggtttgctcatggaaatgggtcgtattcggcaaattgccacaaaaatgaccatctgcacctaatcccagcaccaccaaatccagtccgccttcacgcgccagtttctgatcatgctcgcggtagttatcaatagtgagcttctggatattctcttctttgatccccgcaggggtgaaaaacagattacgcagattggtaatcgttacgccttctccctctttgccgcgaaatggaatttcatcaaaattatagaaatagcagttatcgtaccagggcttacctttaaccagggtggtgaggtattcatacatgcctttgggcgtgctaccggcggtaattgccaggttaacacgacgcgtcttcgacatataaccaagcagatggtgtgccgcgacacggctcatttcctggtaatcttcggtaatgattaatttcatcttaatgccttattttatttaaataatttctgtacaaaggctgcataggctggtcgccagacatccatttcatggttcagacccggatattcctggtaatcaaagttaatttttttctgctcaagctcagttttcagcccggcgatatccttgccggttacgacatctttatcccccacaaccacagtaaaattacgtagttgctggttgatagctgccggatcgttcagtcgggccgcgacaccttcatccggtacggttgtcgtggtaacaccactgaatgtggccagccagccaaagctttccagatgattcattccggaaaccagcgcctggtacccgccttgtgaaagccctgccagcgcgcggccatcggcatctttacggacattaaaacgcttgctaatcagcgggataatatcgttcatcagttcgcgatctgccgctttagcattcagcggataaaagactttacgtctttcctgaggcacgaaatcttcgggaataatgcccttcgcatcggtttctgtatccgggatcaccaccagcatcggtttaattttcccttcagcaagcaggttatccatgatttgcgggatacgcccctgatcgatagcggaacgtccggtatcaccaaagccgtgatagaaatagagcactggcaaaggctcgcccatgccggtgtatcctggcggggtccagacatacatctgacgttcagattgcaatgcgttggagtggtaagttatggcgatcaaatcaccatgcgcaacagaacgcgtatccagataactgcctggcaccagaatcatactggagttaacctggcgctgaggattagtcattgcggtgcctgtatcaatgctgcgtacaccatcaacattgaaaaaatactcgtacaggttgcctttcaggataggtgtgcgccacgaccagactcctgcttcgtctttggtcatcgggtgaatattgtccggaaccggaacacccaccactacagagacattttttgccccaggggcaaagtagcgaaaggtcacgctgttatcggcattgacctgagtcacatactgtttcaccgggatagtgggtgccgggctggctggcatatccgctgctatggcccactgagcagaaataccgctggcaatagccagcgttaaagcagcaatttttatattcatcgtaatattcctttcattaagttccattaccaccagatttcagcctgggcaccgacagcaaactggtcgtctttattgtcttcaaaggtgaagccatccagttcgttttccagggctttgatatacgtggcgtagaaacgaatttccggacgcgaggtcaacatactggtattgactttaaaggtatggaagagcgtggttttataaccagactcattaaatttattactattcgcatctttgttttgctgggtgaaatagcccagttcaacacctgtctggttatattggtcccaaatataggccgggcgaacaaccgcacgaatagattcgaaatcagagtgggcgcctgtttcgtagctatatatatcgttaccgaaggagtaaacaatcgcgttagctacaatgaaatgatcgccaatataggcttcgccctgcgaagtcagacgtaccgctgttccgccggtgtgatcaccataataacgaccattaaaggtggtaaatggacttgcgccagcataacggccaaagttactggcgatagagttattcgcgaccaggaaggagaattcgttgaagccacctttatcaaatttctgcgttaaagatgtgccaaacatccaggtatctttccagtcataatacccgttattatcctgattatctttttccgatgcgctttcgtttgccgtgacataacgaccacttaccattaaggtggctttatcccataacgggatatctttatagcgtaaatcaatggtattggtattaatctgctgtttgttttgcaggctgcgatcgtaatcatcgacatcttcgcgaaccagcgcgatatcaattttacccggaccgactttccagttttccagacctacacccgctgcggcatcagtacgctgcgttttccagtcaagcatctggatttcaattttcggcgcaccgtgtttacccacccagaaatcagcctctggcgcaaagggcaggaaacctttggtggtaacgtacatatcggagaactgcatatagttctcgccaccggcgttatcgccaaaccagccggtagagtactgctgaccaacgttaccatccatcatcacaacggcatcaacccgtttgccgttttcgttgtagacacgttgttttaactgcaaatcaaaccagccggagtattcgttaccaaagcggcccagagaaccaatcgcccatgatttaggtgaaccatgagaggcggtcccccaaccagaacggtaatagccgttgtaactaaagccaatttcatctttcacaaatttactgaaatctttcagagtcatggaagaataaatcgagcctgtctcactggcatttttctcttcatttttgaccagtacagcatcaggttttgcggcactactggtcgggaacggattggcggcatacccttgatcattcgtacttacgctacgattcaccgtcgctggcgtatactttttcttctcttcatctttatactttttgagttcgctttgcgtttctcttaacgccttttctaataactcaaggcgttgttccaccgttaatgattcagccaatgattgtgcagaaaaggctaacggtgccattaataagatggcagaggtaataagatttcgtctaaacataatatccctttatggtgcaaagaaagaattaacgcatcgcatccagactgttctgaatgcgacgataattaaggtgctttaatggttattttttttaatgacagcccccgcgtcttgatcacctctgcataccatccgaagcttttcttgcgtgttcttgtgaggcttccttcgccattatcatcacgatccacataaataaagccgtagcgcttagacatttgtgaatgagatgcactgactaaatcaattggcccccaactggtgtaccccataatatccacaccatcggcaatcgcttcatttacctgtaccaggtgatcgtttaaataggcaattcgataatcgtcctgtatcgaaccatccgcttcaacgctgtcttttgcgcctaatccgttctcgacaataaataacggtttttgataacgatcccaaagcgtatttaacagaacccgtaatccaaccggatcaatttgccacccccactctgaacttttcagatgcggattggggatcatattcagtatgttgccctgcgcatttttattaatgctttcgtcgtgggaaacacaaccagtcatgtaataactaaaagagatgaaatcgacggtatgttttaaatcttctgcgtcactttcagtcatctcaatggtgatattgtggtcgcggaagaaacgctgcatatagccgggatactggccacgcgcctgaacatcaccaaagaacatccagcgccggttctcttccatggcctgcaacatatcctgtggctggcaggtgagggggtaaaccagcccaccgagaagcatattgccgattttcgcttcggggagcaggctatgacaggctttaactgcccgcgcactggcaaccagttgatggtggatagcctgataaacttccgcctcgccactctcttctgccagccccacgcccgtgaatggcgcgtgtaacgacatgttgatttcattaaacgtcagccataacgccactttatgttggtagcgagtaaagaccgtgcgggcgtaatgctcgaagtgatcgatgaccgctcgattagcccaaccgccgtagtttttcaccagcccatatggcatttcgtaatgggataacgttaccagcggcttgatccccgcctgcgccatttcatcaaacagccgatcgtaaaacgctaaccccgcttcattcggttcgacttcgtcgccctgagggaaaattcgcgcccaggcaatggaaatacgcagacaggtgaagcccatctcggcaaataacgcgatatcttccgggtaacggtgataaaaatcgatggcgacatctttgatattctctttccccaggatgcgcggttccatttttcccattacgccatgaggctgtaaatctgaggtcgagatccctttgccatcttcctgccaggcaccttccacctgattggcagctgttgcgccaccccaaagaaatgtttctggaaatgctttcataattaactccttttatcgttagcgaatgatggataacagcggttcacctgcgcttatctgcgccgtgccgtggggtaatacgtccgtaaaatcatcgctattactgattaataccggcgtcgtcagatcaaatccggcctcgcgaatagcagggatatcaaaagaaatcagccgatcgcctgtattgaccttgtcacccacgttgacgtgagcggaaaagaatttgccgtccagttttacggtgtcgataccgacatgaatcaggatctccacaccatcatctgactcaatgccaatggcgtgtaatgtggcgaacaacgaagcaattcgacccgcaaccggagaacgcacttcaccaaccgagggcagaatggcaatacctttacccaacaggccactggcaaacgtggtatcagcgacgtgaatgagcggcacaatctctcccgtcatcggtgaacagataccgccctgctcaggtggtgtaataacctctggtgttttctcttgcggggcaccctgcgctggctgacgtttagcggtgatgaaatgaagcatcaccgtaccgacaaatgcgcaaccgatggcaatgacaccgccaataacgctggcccagacggtgaaatcaattcccgttgacgggatggtttgcatgaaggtgaaaatacttggcaaaccaaaggagtagactttcgtttgcgcgtagccaataatggtggcccccaaagccccactgatacaggcgataacaaaggggtacttacgcggcaggttgacgccatataccgctggttcggtgataccaaacagactcgtcaacgccgctgatcccgccaccacttttttctgcgcatcgcgttcgcagaggaagacgccgagcgccgccccgacctgcgccataatggcgggcattaacagcgggatcatggtgtcgtagcccagcacggtgaagttattgatacacagcggcaccaggccccagtgcagtccgaacatgacgaagatttgccagaagccgcccattaccgcgcccgcaaatgcaggaaccgcctgataaagccagagataaccggcggcaatcagttcgcttatccaggttgatagcggccccaccagcagaaaggtgacgggtgtgataaccatcagacatagcaatggtgtgaagaaatttttgattgccgacggtaaccacgcattaagtcggcgttccagaatgctgcacaaccaggcagaaaaaataatgggaataaccgatgacgagtaattcaacaatgtgaccggaatacccaggaaatccagccccagcgcatccgctttttgcccgttctcgaaagcagtcagaattaatggatgcactaacgctccaccaatcaccatggcagtaaatggattaccgccgaagcgtttccccgcggtgtatcccaggattatcgggaagaaccaaaacaaggcatcactggcgctgaataaaattaaataagtaccactttgttcggtcgtccactgaaaagtgagcgccagagccagcatacctttcaagatcccggttgccgccatcaaaccgatcagaggcgtaaaaatacctgaaataacataaacaaagcggtttagcagattacctttatcatcattttccggtgcctgttgcgctttttcgtcaaggcctgccacactgttaaccgccaggaagacatcggccacatggttacctatgaccacctgaaactggccaccgctttccaccaccataataataccgggggtctttttcagtacctctgcttgcgctttgctttcatcctttaatttaaaacgtaatcgcgttgcgcaatgcatcagactcacaatgttatctgcgcccccgactcctgcgactatttttctggctaactccgtcataacttgccctctaccgctttgcggcaaaactccaaaaaaaaacctgaaaaaaacggcctgacgtgaatcaagcaatttttttcaggttttgcccgcttagtgcggtaacaatcctttactcagtaataatatttcagtgttctttgcgcacgcgctctatatttatggctaaaaacataatctctgcgggtgaaattttacgttgatactgcaaaccaataaaaatggcgatccgttccgcacattgccatgcttgcgggtaattttgttttactgcttgttgtaatgattcatcactatcgttaattgaagcatgttcaagaatacgccaggataaaaacttcagatgtgtaaccagtcgctgataactcaagctttcttcctggtaattaaggctgaactgaaattttattaattgcagcatttcgcgcattaactgcgtgacacctgcaacatcctccatatttccgctcatttgggcactgaccagatgcatggcaataaagcccacttcatctttcggtaactgcacgcccaaccgtttatcaataatggttaacgcttcttcccctagctggaactctttcgggtaaagccgctggatatcccacagcaacgggttgggcagcaacacgttttgctgaaagcgtttaatcgcaaactggcaatggtcagttagcgagatataaatactgtcctgtaattttcccaagcgctcctgcgctaaagagataatacgatcacaggttgccatcacctcaagaggaatatgacttaagagttcgcttaatcgcccgttcagttcatgactgctcaaggcatactctttttctattccacttgagttaattctttcgccagcgcgtttttgaaagccaattccgcgccccatgacgactttttcccgctgttgatcatcaataaccaccacaacattattgttgagaattttggtgatttgcatgttcatagcaaggaccttttttataaacaaaaaaacccgacttcaccagtattctctggttatgtcaggttttgcctgcgaatgcagtaacaatccagtcatttattaatggtttttataacgaacatccaggttcggaaattaatttaattgcgtgcagagaaaatagcaatgcgctattgataaaaatatgaccatgctcgcagttattaactttgtgtaattttaggaatttataaagttatatataacaaatcccaataattaagttattgggatttgtctggtgaattatttgtcgctatctttccccgccagcagtttatccagctcatcgccaccgacgtgacggaaatcctgccccttcacgtagtagaagataaactcacaaatattctggcagcggtcgccaatacgttcgatagaacgcgcgcagaacagcgcagtaagtacgctcggaatggtacgcgaatcttccatcatgtaggtcatcagttgacgaacaataccttcgtattcctgatcgacttttttatcttcacgataaatacgtaccgcttcgtcaatgtccatccgcgcgaacgcgtccagcacgtcgtgcagcatctggatggtatgacggcccagcgactccagacttaccagcaacggctgatgctgctgggagaatttctccagcgcagtacggcagattttgtccgccacgtcgccaatacgctccagctcggcaatggttttactgatcaccataaccagtcgcaggtcgctcgccgtcggctgacgtttggcgataatgcgcacgcaggcttcatcgatcgccacttccatcatgttgacgttcttgtcgccttcgatgacgcgcttcgccagatcgctgtcctggttatgcatcgcggtgattgcatcagaaagctgctgctccaccatgccgcccatggtcatcacctgcgtgcggatactttccagttcggcgttgaactggccggaaatatgtttattaagattgagactgtccataacgcactcctgaatcaaccgtaacgaccggtgatgtagtcttctgtttgtttcttcgctggcttggtgaacagatcgtccgtgttgctgaactcaatcaattcgcccaggtacataaacgccgtgtggtcggaacaacgcgcagcctgctgcatgttgtgggtgacgatcaccacggtgtaatcctgcttcagttcggtgatcagctcttcaatacgcccggtagagatagggtcgagcgccgaacacggttcgtcgagcagcagcacttccgggcgaatggcgataccacgcgcaatacacagacgctgttgctgaccaccagagagagagtaaccgctctggtgcaatttatctttggtttcgttccacaatgcggctttggtcaatgcccactgcacgcgctcgtccatgtcggcacgggagagcttctcaaacagacgaacgccaaaagcgatgttgtcgtagatggacatcggaaacggcgtcggtttctggaacaccatgcccactttcgcacgcagcagtgcgatatcctgagagttggtcaggatgttgtcgccatcaagcagaatttcaccttccgcacgctgctccgggtacagttcaaacattttgttgaaggtacgcagcagcgtcgatttaccgcagccggacggcccgataaacgccgttacctggtttttagcgatatccaggttgatgtttttcagggcatggaatttgccgtagtagaagttcaaattacgaacctgaattttactcggggcagtttcaaccatactcattgcaatcttttcctcatcgtgcctgatgcacttcgctaatcaggcttaccgtaggccggatcaggcgttcacgccgcatccggcaaagtgttaaccgtgtacagagtcaaaaaggcgctcggtcggtcccctcgcccctctggggagagggttagggtgaggggaaaaccgtgtcagcaatatcaaccgtgtttattcttcgcaaaaacaacgcgcgccagaatgttcagcagcagtacgcacagggtaatgatcaataccccggcccaggccaattgctgccattccgcaaacgggctcatcgcaaacttaaagatcgtcaccggcaggttggcgatcggctgcatcatgtccgtgctccagaactggttggagagcgcggtaaacagcagcggcgcggtttcaccagcaatacgggcaatcgccagcaggataccggtcataatcccggacaccgacgctttcagcgtaatcgcagagatcatcttccacttcggtgtacccagcgcataagccgcttcacgcaggctgtacggcaccagtttcagcatgttctcggtggtgcggataacaatcggcacctgcaacaacgccagggcaatcacgcccgcccagccggagaagtgctccatctgcgccaccacaatggtgtaaacaaacagaccaaccacaatcgacggcgcagagagcagaatgtcgttaatgaagcgaatcacttctgccagccaggatttacgaccatattccgccagataaatccccgccataatgcccagcggcgtaccgaataccgtggcccacaaaattaacagcccgctacccgccagagcgttcgccagaccaccaccttccgtattgggcggcggcgtcatttcagtgaacagcgccagcgacataccgtcgataccgcgagtgatggtggacattaaaatccagatcagccagaacaggccgaaggccatcgtcgccatcgagagcgtcagcgcaatacggtttttgaggcggcgacgcgcctgcattttgcggcgagattcagccagcgccgcagtggtttgcatttcaaccatagccattagcgtgccccctcattcttagccaggcgcataatcataaacttcgatgcggcgaggacgatgaaggtaatcacaaacaggatcaggcccagttccatcagtgcggcaacgtgcagaccggattccgcttccgcaaattcgttcgccagcgcagaggtgatactgttgcccggcatatacagcgaggcgctgtcgagctggtaggtgttaccgatgataaaggtcaccgccatggtttcaccgagcgcgcggcccagccccagcatgatgccgccgataacaccatttttggtgaacggaagaacgatacgccagataacttcccaggtggtgcagccaataccgtaggccgactctttcatcatcaccggggtttgttcgaacacatcacgcattaccgccgcaatgtacggaataatcatgatggcgaggatcacgcctgccgcgaggataccgataccaaatgcggggccagagaacagcgcgccaacaatcgggatattcgacatgatattgccgaccggctcctgaaagtaaacggcgaacagcggcgcaaagataaacaggccccacatgccgtaaacgatacttggaatggctgccagcagctcaatggcgatacccagcgggcgtttcagccagccaggcgcaagctcagtcaggaacagggcgataccgaaactcaccgggacggcgatcagcagcgcgataaacgaagtcaccaacgtaccgtagatcggcaccagcgccccgtagatatcgttcggtgcatcccactctttggtccataggaaagccagaccaaatttctgaatgctcggccaggaggagatgatcagagagacaataatgccacccaacatcaatagcacaatcagcgccgccagttttaccagcacgctgaaaattatgtcgccctttttacccggtgggttaaaagcaggcttggttgcagccataagttactcttcagttaaacgcgtttacaaagtcattttgtaatgccggatgcggcgtaaaacaccgtacccggcctggagttttattagtacagcggcttaccgctactgtctttaatattggtcttccacgcagcgcgaacctgttcaactacactatccggcaggctggcgtaatccaggtcgttcgcctgtttagccccggttttgtacgcccagtcgaagaatttcagcacttctgtgccttgttctggtttcttctgatctttgtggatcagaatgaacgtggtagaggtaataggccatgcatcttcgcctttctggttggtcagatcctgagcgaaggttttgctccagtctgcaccttttgctgcattagcgaagttttcttcggtcggactaaccggtttaccatcagcggagatcagtttggtgtacgccaggttgttctgcttcgcgtaagcatattcaacataaccaattgcacccggcagacgctgaacgaacgcggcgataccgtcgttacctttaccgcccagaccgatcggccattttacggtagagccagtaccaacgttgtttttccactcttcgttcactttcgccaggtagctggtgaagacgaaggaagtcccggagccatctgcgcggcgtactacagcaatgttttgtgaaggcagtttcagacccggattcagtttggcgatggcttcatcatcccacttcttgattttgcccaggtagatgtcgccgagggttttaccatccagcaccagttcgccagacttcagccctggaatgttaaccgccagcaccacgccgccaatcacggtcgggaactggaacagaccttcctgagccagtttttcgtcagacagcggcgcgtcagaggcaccaaaatcaacggtattagcgataatctgttttacgccaccggaagaaccgataccctggtagttaactttattaccggtttctttctggtaagtgtcagcccatttggcatacaccggcgcagggaaggttgcacctgcacctgtcaggcttgcttctgcaaacacagagaaagcactcatcgataaggtcgcggcgacaacagttgcgacggtggtacgcataactttcataatgtctcctgggaggattcataaagcattgtttgttggctacgagaagcaaaataggacaaacaggtgacagttatatgtaaggaatatgacagttttatgacagagagataaagtcttcagtctgatttaaataagcgttgatattcagtcaattacaaacattaataacgaagagatgacagaaaaattttcattctgtgacagagaaaaagtagccgaagatgacggtttgtcacatggagttggcaggatgtttgattaaaaacataacaggaagaaaaatgccccgcttacgcagggcatccatttattactcaaccgtaaccgattttgccaggttacgcggctggtcaacgtcggtgcctttgatcagcgcgacatggtaagccagcagctgcagcggaacggtgtagaagatcggtgcaatcacctcttccacatgcggcatctcgatgatgtgcatgttatcgctacttacaaaacccgcatcctgatcggcgaagacatacaactgaccgccacgcgcgcgaacttcttcaatgttggatttcagtttttccagcaattcgttgttcggtgcaacaacaataaccggcatatcggcatcaattagcgccagcggaccgtgtttcagttcgccagcagcgtaggcttcagcgtgaatgtaagagatctctttcaacttcaatgcgccttccagcgcgattgggtactgatcgccacggcccaggaacagcgcgtgatgtttgtcagagaaatcttctgccagcgcttcaatgcgtttgtcctgagacagcatctgctcaatacggctcggcagcgcctgcagaccatgcacgatgtcatgttcaatggaggcatccagacctttcaggcgagacagcttcgccaccagcatcaacagcacagttaactgagtggtgaatgctttagtggatgccacgccgatttctgtacccgcgttggtcattagcgccagatcggattcgcgcaccagagaagaacccggaacgttacagattgccagtgaaccaaggtaacccagctctttcgacagacgcaggccagccagggtatccgcggtttcgccagactgtgacaaggtgatcatcaggctgttacgacgcacggcagatttgcgatagcggaattcagaggcgatttcgacgtcgcacggaatacctgctagcgattcaaaccagtagcgggaaaccataccggagttataagaagtaccacaggcgaggatctgaatatgctcaaccttcgacagcagttcgtcggcgttcggtcccagctcgcttaaatcaacctgaccgtggctgatgcgtccggtaagggtgtttttgatcgcgttcggctgttcgtagatctctttctgcatgtagtgacggtaaatgcctttatcgcccgcgtcatattgcagattggattcgatatcctgacgttttacttccgcgccagttttatcgaagatgtttaccgaacggcgagtgatttccgcaatatcgccctcttcaaggaagataaagcgacgggtcaccggcaacagcgccagctggtcagaagcgataaagttttcgcccatccccaggccaatcaccagcggactaccagaacgtgccgccagcagggtatccgggtgacgggagtccatgatcactgtaccgtacgcaccacgcagctgcgggatagcacgcagaacggcctcacgcagagtcccgccttgtttcagctcccagttcaccagatgggcaatcacttcggtgtcggtttcagaaacgaaggtatagccacgcgcttttagctcttcacgcagcggttcatggttttcgatgatgccgttatgcaccaccacaatgtgttcagaaacatgcggatgcgcattcacttctgaaggttcaccgtgggtcgcccagcgagtgtgagcaataccagtgccgccatgcagaggatgttcttccgctgcctgtgccagcatctggactttaccgaggcgacgcaggcgggtcatatgaccttctgcatcaacaacggccagaccggcagagtcatatccgcggtattccagacgacgtaaaccttcaagaaggatttctgctacatcacgttgcgcgatcgcgccaacaattccacacatagtttttgattccgatttatatcgttgtcggtcaacctgtatgcccgttttttcgggcgccccgagccttgtagagagtggggttatttttatagttactgcttgtgggagggagattatgttatctcctcatcccatgtgaccgggttagccggccagaatcactttttctttaccggacgacgccagccttctttctgagtctgcggcacacggctgatagctaatgcattttcgccgacattacgcgtcacagttgtacccgcagcaatggtcgcgcctttgcctactgttaccggggccaccagctgagtgtcggaaccaacaaacacatcgtcgccgataatggtcttaaatttattcgcaccatcgtagttgcaggtaatggttcccgcgccgatgttaacgttatcgccaatttccgcatcgcccaggtaagtcagatgaccagctttcgagcctttacccagacgcgcttttttcatctcaacgaagttaccgacgtgagcaccttccagcaactcagcaccaggacgcaaacgggcaaacgggccaatggtacaggccgctgccagattcgcatcttccacaacggtatacggactgatttcgcaatcatcgccaatcacgctgtttttaatcacgcaaccggtgccaattttcacgcgatgaccgagagtcacgttgccctcgatgataacgttagtatcaatttcaacatcgcgcccgtgagttagcgtaccacgcagatcaaaacgcgctggatcgcgcagcataacgcctgctaacagcagtttttcagcctgttcggactgataaacacgctccagacgggagagttgcaggcggttattcacgccttctacttcgcttaaacgttgcggatgaacggcgacgatttcacgcccttcctgatacgccagcgcaataatgtcggtgatgtagtattcgccctgagcattattgttggtcagcttcgccagccagcgtttcatatctgcgccgttggcaatcagaatgccggtgttgatctcctgaatctgacgctgctcgtcggtggcatctttgtgctcaacaatgccggtaactttgccgttttcacgggtgatacgtccataaccggtcggatcatccagtttcaccgtcagcagaccaatgccaccctgcggtttagcatcacgcagacgctggagtgtttcgacagagatcagcggcacgtcgccgtagagcattaaaatgtcttcatcatcggcaaagaaaggtgcggcctgctgcattgcatgacccgtacccagctgctctgcctgaagcacccagttaaggttgtcgtctttcagcgcctgttttagcagatcgccgccgtgaccgtacaccaggtgaacgtgcgctgcgcctaattcattcgcagcatcaatgacatgctgaaccatcgctttcccggcaagggtatgcagcactttcggaagatcggaatacatgcgcgtgcctttgcctgcggcaaggatcactacgctcatagcattattcaacatacgcgtcctgactgtaatttgagaacgaatttaaaccgcttcaccttgaaaaaactacatttttttcatcgtgaaatggacagaggataaattgttcaataacggattatccccgctgacgaaagcgccattttcgaccatcgtcacgccttttgtctgcagaaaattaaggcagtaccttaatttaagcgtcaggtggatgtttttgctcttatttcgatcaatgaataaacaggaaaacaggggggttttatatcagcaggatctatgtgaacgctattcaggacgggtcacacgcgcaaaaaaaagccagcctgtttccagactggcttttgtgcttttcaagccggtgttacatcgcttttttggtcaactcgataacgcgcagctgcgcgatcgctttggccagttccgcagacgcctgagcgtaatctacgtcgccgtgagagctgctaatgtgctcttcagccttacgtttcgcttccatggctcgcgcttcgtcgagatcctggccgcgaattgcggtgtcggccagaacggtcacgttgccaggctgcacttcaagaatgccgccagacagatagataaactcttcgtgaccgtgctgtttcacgatgcgaatcataccaggcttaatggcggtgagcagcggtgcgtggccagggtagatccccagttcaccttcgctacccgttacctggattttctcgaccagaccagagaacatttgttgctctgcgctgacgacgtccaggtggtaagtcattgccatatcaccctccgattaaggcgttaaagttttttggctttttccacagcttcttcgatggaaccgaccatgtagaacgcctgctccggcaggtgatcgtattcgccttccatgatgcctttaaagccacggatggtgtctttcagggagacgtatttacccggagaaccggtgaatacttctgccacgaagaacggctgggacaggaagcgctggatcttacgagcacgcgctaccaccagtttgtcttcttcagacagttcatccatacccaggatggcgatgatgtctttcagttcctgataacgttgcaggatggactgaacgccacgcgcggtgtcgtagtgttcctgaccaaccaccagcgggtccagctgacggctggtggagtccagcgggtcaacggccgggtagatacccagagacgcgatctgacggctcagtaccacggttgcgtcaaggtgcgcaaaggtggttgccggagacgggtcagtcaagtcatccgcaggtacgtatactgcctgtacggaggtgatagaaccagttttggtggaggtgatacgttcctgcagaacgcccatctcttccgccagggtcggctgataacctaccgctgaaggcatacggcccagcagtgcggatacttccgtaccggccagggtgtaacgatagatgttgtcaacgaacagcagaacgtcacgaccttcgtcacggaatttctcagccatggtcagaccggtcagagcaacgcgcagacggtttcccggcggctcgttcatctggccatacaccagggatactttgtcgataacgttggagtcggtcatttcgtggtagaagtcgttaccctcacgagtacgttcacctacgcccgcaaacacagagtaaccggagtgctcgatcgcgatgttacgaatgagctccatcatgtttacggttttacctacacccgcaccaccgaacagaccaactttaccgcccttagcgaacggacacatcaggtcgataactttgataccggtttccagcagttcctgagagtttgacagctcttcgtaggaaggtgctgcgcggtgaatcgcccaacgctcttcttcaccgatctcgcctttcatgtcgaccggttcacccagtacgttcatgatacggcccagagtcgctttacctaccgggacttcaatcgggtgttcgaggtcttttacatccagaccgcgacgcagaccgtcggaggaacccattgcgatggtacgtacgataccgccgccgagctgctgctgaacttccagcaccagacgctcattaccattttgcacctcaagagcatcgtacacgcgcggtacggcatcctgagggaattcgacgtcaactacggcgccgattacctggacaatctttccagtagccatcttaaatcctctacgaaataacctgtttaaaccgcggcggcccccgagacgatctcggtgagttcctgagtaatgctggcctgacgagctttgttgtataccaactgcagctctttaatcaggctgccgccattgtcggtcgcggctttcatcgccaccatacgggcggcctgctcgctggccaggttttcaaccacgccctgataaacctgagattcgacataacgacgcagcagggtatccagcaacgccttcggatcgggttcgtacaggtaatcccaggatttatgtttcagatcatcatcatctgatgccggtaacggcagcagctggctgatggtcggaacctgagacatggtgttaataaatttgttgctgacaatgtaaagcttgtccagacggccttcgtcgtaggcctgcaacatcacttttaccggaccgatcagttcggacagggaagggttatcccccatgccggtgacctgggcaacaacattgccgcccacggagttgaagaacgacacgcctttcgagccgatcattgcgaggtcgcattgaacgcctttgtcggtccaggtcttcatttccgccagcagttttttgaacaggttaatgttcaaaccaccgcacaaaccacggtcggtcgacaccaccaggtagcccacgcgtttaacgtcgcggtcttccaggtaagggtgcttatattccagattaccgtgtgcaaggtgaccaatcactttgcgcatggtttctgcataaggacggctggccgccatgcgatcctgcgatttacgcattttggaagcggcgaccatctccatcgctttagtgatcttttgcgtgttctggacgcttgcgatcttactacgtatctcttttgcgccggccatgagcttctcctcaatgccttgcggcctgccctaaggcaagccgccagacgttaccaggattgggttgctttgaaggaatcgaggatgcctttcagcttgccttcgatttcgtcgttgtagccaccggtctggttgatctcttgcatcaacggagcgtgatcacggtcgacgtaagccagcagagcggcttcgaagctgccaattttcgacagttcaacatccgccaggtaaccacgttctgctgcgaacagaaccagagactgctgcgcaacggacatcggcgcatactgtttctgtttcagcagttcggtcactttctgaccgtggtcaagctgcttacgtgttgcatcgtcaaggtcggatgcaaactgagagaacgctgccagttcacgatactgtgccagagcggtacggataccaccggacagttttttcatgatcttggtctgtgctgcaccaccaacacgggatacggaaatacccgggttaaccgcaggacgaataccggcgttgaacaggttggtttccaggaagatctgaccatcggtaatggagattacgttggtcggaacgaacgcagaaacgtcacccgcctgagtttcgataatcggcagtgcggtcagagaaccggttttccctttcacttcacctttggtgaaggcttcaacgtattcggcgttaacacgtgcagcacgctccagcagacgagagtggaggtagaaaacgtcgcccgggaatgcttcacgtcctggcggacgacggagcagcagggagatctgacggtaagcaacagcctgtttagacaggtcatcgtaaatgatcagcgcatcttcaccgcggtcacggaagtattcgcccattgcgcaaccggcatacggtgccaggtattgcagtgcagcggattcagacgcggttgctaccacaacgatggtgttagccagtgcgccgtgctcttccagtttacgtaccacgttagaaatggtggacgctttctggccgatagcgacatagatacatttgataccggaatcgcgctggttgatgatggcatcgatagccagtgcggttttacctgtctgacggtcaccgatgatcaattcacgctgaccacgaccgattgggatcatggagtcaacggctttataaccggtctgtaccggctgatctacggactgacgttcgataacgcccggagcgattgcttctacagcagagaagccgtcgtgatccagcggacctttaccgtcgattggtgcacccagagtgttaaccacacggcccagcaggccacggccaaccggaacttccaggatacggccagtacacttaactttcatgccttcggcaaggtcagcgtacggacccataacaaccgcacctacagagtcgcgctcgaggttcagtgcgatagcgtaacggttacccggcagggagatcatttcaccctgcatacaatcggccaggccgtgaatgcggataacaccgtcacttacagaaacaatagtaccttcgttgtgagcttcactcacaacattgaactgagcaatgcgctgcttgatcagttcgctgatttcggtggaattcagttgcatgctccagtccccttaagactgcaagacgtctgcaaggcgctcaagacgaccgcgtacgctgccatcaatgaccatatcacccgctcggatgataacgcctgccattacagacttatcgattttgcaattcagcttaactttgcgtgacagacgtttttccatcgcagcagaaattttcgcgagctgttgttcactcagtgcggcagcggaaatgacgtctacctcagcggtagcctcactcacggcacgcaggtgaataaactgctccagaacatccgggagcgcgttaagacgaccattttcagccataacccgaatcaggttctgaccgttttcgtccagttgctcaccacaaactgcgataaacgactcggcgagcgtttctggcgcaagcgcgccagagagaagctctgccatttgttcgtttttggttacctcggcggcaaacgccagcatgtcctgccagcgttctacactttggtgttcgacggcaaagtcaaaagctgctttggcgtaggggcgagctaccgtaataaattcagacatcagcccctccctccttacagttcagcgacaagtttatccacgatgtcgctgttagcagcttcatccacggaacgttcgatgatcttctcggcgccagcaacagccaggatagcaacttgcttacgcagctcttcacgggcacgtttacgctcggcttcaatttccgcctgcgcctgggccacgattttagtacgttcctgttctgcctcagctttcgcttcgtccagaatctgcgagcggcgtttgttcgcctgctcgatgattacctgggcttccgctttcgcttttttcagctggtcggtcgcgctggcctttgcaaggtcaaggtccttatgtgctcgttctgcggaagcaaggccgtcagcaatttctttttgacgtttttcgatggctgccattaatggcggccatacgtacttcatgcagaacagaacgaacaggacaaacgcgatggcctggccgaggattgttgcgttaagattcacagcacaatgcctctatttagttaacgttctgatattgctctttaaataaaagcaacgcttactacgcgacagcgaacatcacgtacagacccagacctacagcgatcatcgggatagcatccaccagacccataacgataaagaactgagtacgcagcagaggaatcagatcaggttgacgcgctgcgccttccaggaatttacccccgaggatgccgataccgatcgcagcaccgattgccgccagacccatcatcacagcggcagccatgtacagcagatccatattcaggttttccatgacagtctccagtttgtttcagttaaaacgtagtagtgttggtaaattaatgttcttcagacgccatcgacagatagacgatcgtcagaaccatgaagatgaaggcttgcagcgtaatgatcaggatgtggaaaatggcccacggcacattcaggatccactgtgaccaccacggcaacagaccagcaatcagaatgaaaatcagctcaccggcatacatgttaccgaacagtcgcaaaccgagtgaaactggtttggacagcaggcttaccccttcaaggattaagttgacaggaatgaacgcccagtgattgaacggctgcagcgtcaactctttcgtgaagccgccgatgcctttcattttgatgctgtagaacagaatcaggataaatacgcccagtgccatagacagcgttacgttcacgtccgcagacggaaccacacgcagtgcaggcagacccagtacatgttcagcaatgtacggcagcaggtcgataggcagtaaatccatcaggttcatcaggaatacccagacgaagatcgtcagggccagcggagcaatcagcttgcttttgccatggtacatgtctttcacgctaccattaacaaagccgatcaccagctcaatcgcggtctgaaacttacctggcacaccgctggtcgcctttttggctacgctacggaataaaaccaggaacaacagacccagcaccaccgagaagaacatggagtcaatattgattgtccagaaggtggctggggggttttgtggatccaccagcgagaatgtacgcaggtccagctgaaggttattcaggtggtgtcctatgtaatcctgcggcgtcatattttctgaagccatgatgccttttaccctttgttgttaattacagccggtgccagtatctgaaccaccagcaccaaaacccacgtaacgatcagcggcaagaataccgcctttaaaaccgccaacgccaccaccagtaacaccaacatcgccagaactttgaaagcttcgccaaatgcgaatgtccaggccacccggcctttcgctggtgtatgcgcctggtgacgccaggcaaatatcataaacaaaacgttaggcagaaagactgccaggcccccgcttattgcagagacgccccagaaggggtctttgaggctgaacagcaatccacttgctatcaccaccagtaactgaacgagcagaagcttccgagcaacgtttcgactcacgagcgacacagacatcacgtttttcactcctgctcccttcgaggtatgccgcgtgtcgtataaaactttctttaaggcttagagtcaagcatcaaaaagcggtcaaattatacggtgcgcccccgtgatttcaaacaataagtagccaaaaggtgaataaatgtttaaatatttttccagtgcatacaattgcgacttttctgctaaccctgttcgatcatgaaaaactgtaaataacgcgtaaacactggtgataaagcgtgcttcagatcacatattgcgcatgttcgcgcacagcatatttatttacttggcaaatgatgcctttgcaagtttatgatatttcagtctaaaaacagatactgttttaataaatgacatttacacaacaaaaaccacccattgacatttttaataatgttttaacagccaatgatggttcttagcgccgatttttagcagactgatattttcactaatgacttattttctgcttaccaaaaaaagccacgttatcttgttgatgcaaaagagtgaacgtggcgttaaatgtaaccagttatatcagtagaaaacctggttgttgttaacagtctaaccggtcaattttttatgatttttttgataaaaattaaattttatttgctttaatcaccaccagatgacgttcgccatccagggctggaacctgaagtttaaccactgattcgacctgatattcttcgggcaacaaagcgatttcatcttccggcatttgccctttcagcgcgtagaaacggccttgctcaccaggaagatggtggcaccagctcaccatatcgttcagagaggcaaaagcgcggctaattacgccatcaaatggcggctctgaaggaaactcttctaccctgctctgtactggttcaatattctccagtttaagctcatgttgcacctgacgaaggaaacgcacgcgtttaccaaggctatccaacagagtgaaatgggcttcaggacgcacgatagagagtggaatgcctggcagtcctggtccggtgccgacatcgataaaccgttcaccttgcagatacggtgccaccacaatgctatcgagaatatggcgtaccagcatctcattaggatcgcggaccgaagtcaggttgtacgctttgttccatttatgcagcatattcacgtaggcaataagctggtttttctggtgatcggtaagcgaaatacctgcgtctttcagcagtaaggagagtttgttgagcacggtgattacctgttcttgatgcgttgcctggtaagcgggtgcttaccaggcatttttaatgcgttatgcgctacgacgcagcataccctgttttttcagccacaccagcagaatggagatggccgcaggcgtgacgccagaaatacgcgaagcttggccgatagaggctggtttgtgatcgttaagtttggcgatcacttcgttagaaagaccggatacctggcggtaatccagtgtcgcgggtagcagggtgttctcgttacgcagctgcttttcgatctcatcttgctggcgcgcgatataaccttcgtatttaacctgaatctcaacctgttccgccgcctgttcgtctgtcaacgcaggggcaaacggcgtcagcgtggttaatttttcataagtcatttccggacgacgcagcagatcttcaccactggcttcacgggaaagcggcgcagtcaggtgagcattcacttcggctgcagcttccgccgacggggttacccaggtcgatttcagacgctgacgctcacgctcgatattctcaagtttctcgttaaagcgcgcccaacgttcgtcatccaccaggcccagttcacgaccgatttcagtcaaacgcagatccgcattatcttcgcgtagcatcagacgatattctgcgcgcgaagtaaacatacgatacggttctttggttcctaaagtgcacaggtcatcaactagtacgccgagatacgcctgagaacgtgccggagcccaaccttctttgtcagcagacagacgggcagcgttaagaccggccagcaaaccttgcgcagcggcttcttcgtaaccggtagtgccgttaatctgaccagcaaagaacagcccctggataaacttgctctccagcgtcggtttcaggtcgcgaggatcgaagaagtcatactcaatggcataacccggacgcacgatcttcgcgttttccatcccctgcatagagcggacgatttgcatctgcacatcgaacggcaggctggtggagataccgttcggataaatttcattagaggtcagtccttccggttcaaggaagatctgatgctgatttctgtcggcgaagcgcatgactttgtcttcgatcgacgggcagtagcgtgggccgacaccttcgatcacccctgcgtacattgggctacgatcgaggttactgcggatcacatcatgggttttctcgttggtatgagtgatataacacggcacctgctggggatgctgggacgcattgcccataaacgagaataccggcattgggttatcgccatgctgttgcgccagtacgctaaagtcgatggttcgagcatcaatacgcggtggtgtcccggttttcagacgaccaacgcgcagcggcagttcacgcaaacggcgagaaagcggaatggacggcggatcaccagcacggccaccgctgtaattatccagaccgatatgaattttaccgtcgaggaacgtcccaacggtgagcacgacggctttggcacggaacttcagtcccatttgggtaacagcaccgaccacgcgatcgttttcgacaataagatcttcaaccgcctgctggaagatcatcaggttcggttggttctccagcgccgtacgtaccgcctgacggtagagcacacgatccgcctgagctcgggtagcgcgaaccgccggtcctttgcttgcgtttagtatcctaaactggatacccgcctgatcgatcgctttcgccatcagaccgccgagtgcatccacttcttttaccagatgtcccttcccaataccgccgatcgccgggttgcagctcatctgccccagagtgtcgatattgtgtgtcaaaagcagagtctgttgacccatacgcgccgcggccatcgcggcctcggtgcctgcatgacccccgccaatgatgatgacgtcaaaaggatccggataaaacatggtgattgcctcgcataacgcggtatgaaaatggattgaagcccgggccgtggattctactcaactttgtcggcttgagaaagacctgggatcctgggtattaaaaagaagatctatttatttagagatctgttctattgtgatctcttattaggatcgcactgccctgtggataacaaggatccggcttttaagatcaacaacctggaaaggatcattaactgtgaatgatcggtgatcctggaccgtataagctgggatcagaatgaggggttatacacaactcaaaaactgaacaacagttgttctttggataactaccggttgatccaagcttcctgacagagttatccacagtagatcgcacgatctgtatacttatttgagtaaattaacccacgatcccagccattcttctgccggatcttccggaatgtcgtgatcaagaatgttgatcttcagtgtttcgcctgtctgttttgcaccggaatttttgagttctgcctcgagtttatcgatagccccacaaaaggtgtcatattcacgactgccaataccgattgcgccaaagcggactgcagaaagatcgggcttctgttcctgcaatgcttcatagaaaggagaaaggttgtccggaatatctccggcaccgtgggtggagctgataaccagccagatccctgaggcaggtaaatcttctaacagcggaccgtgcagcgtttcggtggtaaaacccgcctcttccagcttttcagccaggtgttctgctacatattcggcaccgccgagggtgctgccgctgataagagtgatatctgccataaaccgccacctttattaagagtggcgtattgtacgctgtgaacgcgttgggatctacctgtggaaaagtatgggattaaaaaagccgatcagggcttgatggtacgcatgatcgggttttgcaggacgatcaatgtctcggtggactgaatttcatcaattgtttggatcttgttgataagtacatgctggagagcgtcgatcgaacggcacatcacttttataaagatgctgtagtggccggttgtgtaataggcttcagtgacttcatcaaggctttccagctttgccagcgcggaagggtagtctttggcgctctttaatataatgccgataaagcagcctacgtcataaccgagctgcttcgggctgacatcaatacgcgccccggtaatgatccccgcctgcttcattttctctactcgaacgtgaatcgtccccggactgacgccaaattgtttcgccagttcggcgtaagcggtgcgcgcattgcccattaatgcttccaggatgccacggtccagattgtcgatcagataattttccataggattttcttatgcggattgatgattcattctattttagccttcttttttaatgaatcaaaagtgagttaggctttttattgaatgattattgcatgtgtgtcggtttttgttgcttaatcataagcaacaggacgcaggagtataaaaaatgaaaaccgcttacattgccaaacaacgtcaaattagcttcgtgaaatctcacttttctcgtcaactggaagaacgtctggggctgatcgaagtccaggcgccgattcttagccgtgtgggggatggcacgcaggataacttgtcgggctgtgaaaaagcggtgcaggtaaaagtgaaagctctgcctgatgcccagttcgaagtggttcattcactggcgaagtggaaacgtcagaccttagggcaacacgacttcagcgcgggcgaagggctgtacacgcacatgaaagcccttcgccccgatgaagaccgtctttctccgttgcactcggtctatgttgaccagtgggactgggaacgcgtaatgggcgacggtgagcgtcaattctcgactctgaaaagcacggtagaggcgatctgggcgggaattaaagcaaccgaagctgcggttagcgaagagtttggcctggcaccgttcctgccggatcagatccacttcgtacacagccaggagttactgtctcgttatccggatcttgatgccaaagggcgtgagcgggcgatagcgaaagatcttggcgcggtattccttgtcgggattggcggcaagctgagcgatggtcatcgccacgacgtgcgcgcaccggattatgatgactggagcaccccgtcagagctgggccatgcgggtctgaacggcgatattctggtgtggaacccggtactggaagatgcgtttgagctttcctccatggggatccgtgtagatgccgacacgctgaagcatcaactggcgctgaccggtgacgaagatcgcctggagctggagtggcatcaggcgctgctgcgcggtgaaatgccgcagaccatcggcggcggtatcggccagtctcgtttgactatgctgctgctgcaactgccgcatatcggccaggttcagtgtggagtatggccagctgctgttcgcgagagcgtcccttctctgctgtaataatttatcgccgccagcgtctgagcaggcggcttcgcatcccggtatcaaagcgccagatatgatcgaaaatgcgcatgatgccgggtttgccgtgtgccgacatcgccacggcatgaaagcgatgctgatgtacccgctgcagctctttcactttactcgtcacgtcgtcaggcaaccgctgagcgataaaatcagaaatcaccaccgcatcggcatcaaaccattccctgctttgcaagcgttccataatggcgcgaaaacaactggcaagatcggtgccgccacgaaactgctggcttaaaaaacggattgcttgttcgatgccttgtgggcctgaaagctcataacggacgatctcggtggaaaatagcataatatagcagcgccggttttctgcgagagcaatgcgcatcaaggccaggcagaacgctttcgcacactgttcattaaagccgcccattgagccggaagtatccacacagacaataaacggcccgcgcggctgttcatcgtaatctttatgtaccaccggacgttcgatcactttttcacgccacgactcaccgtgcaggcgataggtgagcaactgtttttccaccagccgacggtaaaactcatactccagttccgttatccctagtgtcgccagttctggcggcaggagacgtaaaatatcatcgctttgttgcagaccatcaacctgctcaggaaccgtcgccggttcgcgcaccatggtgcggaaggtttccatctgcgcatcgttgcgcggtattgatttggcttcccgagaacgccccagctgctctgccaggcgtttcagttccggctgttcgttaagaaattcaccgtatttcacaatcaactgatagtcgccacgtttaagctgaccggcgctcatatcccacagacgaccagctgcagtattgttatctgcgagaatcggttcaagttgtccgctcagcgtcatgcgttcctgaacttcactcaacagttgttcgcgttcttcttctaatagctgttgatttaacgtcgttgcttgcacgatcagacttaaacgccaacgctggagaaaaagcgtgtgtaacgctgaagtgatcgtgctgttagcatcaaccaactgtcgggcttgttctgcccatggagaattcagacgatgcagtaagtccaggatctgtggtagctgcacaataaactgtggcgtggagaggagctggctttgctgatagcacatcacctcttcggtgagttccggcgggactcgggcatctttcagccgactgcgcagcgcttcacgccagcggggaacatcatcagtgattgccgccttcaggcgtgggaatttttcaaagaagaccgccagctgcggtgaggccagcagtgcgatgatcatctcttcgatcaatccctcttcgctgacggccagcatcacattaagcgtatccagcgttagcattgttgtgcctggcgaatctgtgcaccgacatcctgtaggctggcttcaatgcgacctaaccagtcgccagggataaacagacatttttgctgttcgctgaataaagcgtgttgcttgcgccagtcgctttcaagctcttccagttgttgttttatttcaccaggcagaccttcagccgatgaaccgggaagtgccagcgtactgccttgtaaacttacatcgcgaacgacaagatgttgggcgctatcaacttccagattcagtttctgggcaaagccgataccgttcagtttaccgcgaatttcaccacctttgctcagccactgttccagcgcgctacgctcaaaggagatatgaaccacttccatatcatgcagttttaacggtttttgcagcagtagagtcagagtggaagcagtaacgttaacaggaagttgatactgctgacgacggctgaaaatgccgcccagacgaattaccgttaaggctgttttatcgctttgttgctgctggagttgcaggtgacgttgcacaatcgcgccaaggcgagtcaacatcccttgctgttgccaggcgtgaccggtcatcaatacatcaatttgttgttgtatcaaattcaggctttgcgcgtcataccacaggcaatctttcagcaaaatgagatctaccggggcaacagcactgcgaccgctaaaaaaggcgctggcctgcaataatcggatcgcttttttccagcgacgatccgagacataaggcgcatccggtaatttatccagttgctggcgcagcataaaaatcagctcaaatacatgatcgggcagcgtaatttcaccaatctctttctgccagcgttcatattcttcatctgtgacctgcaaggcatcaggaaccggattgtcgttttcatcctgttgactggtcagcatggagcggaaattcgctttatcctgcactttatctaaccacagacgaatcagcatgcggtcatataacgcttccagactgctgtctgcttccggcagctcgttggaggccgccaccagcagacgcatcgggattttttctacgtgtgcaccgttgcggaactggcgctcgttaatggcggtgagcaaggtattaagaattgccgggcccgctttccagatctcatccagaaagacaatttctgcttccggcaggtaaccgctggttaaacgttcatagcgcccttcatcttttagcgcctgaatagaaaggggaccaaaaacttcttccggcgtggagaagcgggtcatcagatattcaaacgcgcgggcattctgaaaggcgaattttaagcgccgggcgatcaaacttttggcaatacctggcgggccaaggaggaacacactttcaccacttaatgccgctaataaacacaagcggatggcgtggctacgttcataaagccccttttccaacgaactgctcaggcgggaaattctttccgctaataaatgagggtgagccataatgaagtggcgtcctttcgtcaaaagttctgcgtaaattgcgagtatagacgtttcttgctggtggctaaaatagtctcaaagggggggtatttttctttgagccaggttaatgtggccgcatttaggagtacgattttgccgttaatcgtgcatactgtgcgcttttttgtgggccaagggactaagcacacatttcatatttcaacgaaagactagtctatgagcactgataataagcaatcattgcccgcgattaccctcgcggcgattggagttgtctacggcgatattggtaccagcccgttatatacacttcgtgaatgtttgtccggccagtttggttttggcgttgaacgcgatgccgtgtttggctttttatcgctgatcttctggctgctaatctttgtggtttccattaaatatctcaccttcgtgatgcgggcagataacgccggtgagggggggatcctgacgttgatgtcgcttgccgggcgtaatacgtcggcgcgaaccacatcaatgctggtgattatggggctaatcggcggcagctttttctatggtgaagtcgtcataacacccgctatttcggtgatgtcagccattgaaggtctggaaatcgtcgccccgcagctggatacctggatagttcccctctcaattatcgttctcactttattatttatgattcaaaaacatggcacggctatggtcggtaagctgtttgcgccgatcatgctgacctggtttttgattctggcaggactggggttacgtagcattattgctaacccggaagtgctgcatgcgctgaatccaatgtgggcggtgcatttcttccttgaatacaaaacggtttcttttattgcattaggggcagtggtgttgtcgattacgggggtcgaggcgctgtatgctgatatggggcactttggtaagttccctattcgcctggcgtggttcaccgtcgtattaccttccttgacccttaattacttcggtcagggagcgctgttgttaaagaacccggaagcgattaagaacccgttcttcctgttggcaccggactgggcgctgatcccgctgctgatcatcgccgcactggcgacggtaattgcctcgcaggcggttatctctggcgtcttctcattgacgcgtcaggcggtacgtctgggatatttgtcgccgatgcgcattattcacacctccgaaatggagtcagggcaaatctatattccgtttgtgaactggatgctctatgtcgcggtcgtgattgtgattgtcagctttgagcactccagcaacctggcggcggcgtacgggattgcggtgaccggaaccatggtgctgacgtctattctctcgactaccgtggcacgtcagaactggcactggaataagtattttgttgcgctgatcctgattgctttcctttgtgtcgatattccattgttcaccgctaacctcgataaactgctctccggcggctggttgccattgagcctcggtactgtgatgtttatcgtgatgaccacctggaagagcgagcgtttccgcttgctgcggcggatgcatgaacatggtaactctctggaagcgatgattgcttcgctggagaaatcaccgcctgttcgcgtgcccgggaccgcggtgtatatgtcgcgtgcaatcaacgtcattccctttgcgctgatgcataaccttaaacataacaaggtattgcatgagcgggtgattctgttaactctgcgcaccgaagacgctccatatgtccataacgtccgtcgggtacagattgaacaactgtcgcccactttctggcgcgtggtggcaagttatggttggcgagaaacgccaaacgtagaagaagttttccaccgctgcggtctggaaggattaagttgccggatgatggaaacctccttctttatgtcgcatgagtcgttgatcctcggcaaacgcccgtggtatttgcgtctgcgcggcaagctgtacttgctgctgcaacgtaatgcgctgcgtgcaccagatcaatttgaaatcccgccaaacagggttatcgaactgggtactcaggtcgaaatctaacgccagacgcctcctttcttcataagggggcgtttttgttttcatggttaatcaccatgtaaaacgtttcgaggttgatcacatttccgtaacgtcacgatggttttcccaactcagtcaggattaaactgtgggtcagcgaaacgtttcgctgatggagaaaaaaatgaaaaaaggcaccgttcttaattctgatatttcatcggtgatctcccgtctgggacataccgatacgctggtggtgtgtgatgctggtttacccatccccaaaagtacaacgcgtatcgatatggcattaacccagggtgtaccttcttttatgcaggtgctgggcgtcgtcacaaatgaaatgcaggtcgaggcggccattatcgcggaagagatcaaacaccataatccgcaactccacgaaacgttgctcactcaccttgagcagctgcaaaaacaccagggaaataccattgaaattcgttacaccacgcatgaacaattcaaacaacaaaccgcagaaagtcaggcggtaattcgcagcggagaatgttctccgtatgcgaatatcattctctgtgctggcgtgacgttctgaggccgtcatggaagcattacttcagcttaaaggcatcgataaagccttcccgggcgtaaaagccctctcgggcgcagcgttaaatgtctatccgggccgcgtgatggcgctggtgggcgaaaacggcgcgggtaaatccaccatgatgaaagtgcttactggcatctatactcgcgatgccggtacgcttttatggctggggaaagaaacgacatttaccgggccaaaatcttcccaggaagccgggattgggattatccatcaggaactgaacctgatcccgcagttgaccattgccgaaaacattttcctcggtcgtgagtttgttaatcgctttggcaaaattgactggaaaaccatgtatgccgaagcggataaattgctggctaaacttaacctgcgctttaaaagcgacaagctggtgggcgatctttccatcggtgaccagcaaatggttgaaatcgccaaagtgctgagctttgagtcgaaagtcatcattatggatgaaccgaccgatgcgctgaccgataccgaaaccgaatccctgttccgcgtcatccgcgagctgaaatcgcaaggccgcggtattgtctatatctcccaccgcatgaaagaaatcttcgagatttgcgatgacgttaccgtttttcgtgatgggcaatttattgctgagcgcgaagtggcatcactgaccgaagattcgctgattgagatgatggtgggtcgcaagctggaagatcaatatccgcacctggacaaagcgccgggagatatccgcctgaaagtcgataatctctgcggacctggcgttaacgatgtctcttttactttacgcaaaggcgaaattcttggcgtctctggtttgatgggcgcaggtcgtaccgaactgatgaaagtgctctacggcgcactaccgcgcaccagcggttacgtcaccctggatgggcatgaagtcgttacccgttcaccgcaggatggcctggcaaacggcattgtgtatatctccgaagaccgtaaacgtgacggtttagtgttgggcatgtcagtaaaagagaacatgtcgctgacagcgctgcgctacttcagccgcgctggcggcagtttgaagcatgccgatgaacagcaggctgtgagtgatttcattcgtctgtttaatgtgaaaactccgtcgatggaacaggcaattggtctgctttccggtggcaatcagcaaaaagtggcgattgcccgcggtctgatgacacgccccaaagtgttgatccttgatgaacctacccgtggcgtagatgtcggcgcgaaaaaagagatctatcaactgattaaccagttcaaagccgatggcttgagcatcattctggtgtcatcggagatgccagaagtattaggcatgagcgatcgcatcatcgtcatgcatgaagggcatctcagcggggaatttactcgtgagcaggccacccaggaagtgttaatggctgccgctgtgggcaagcttaatcgcgtgaatcaggagtaaaaaaatgacaacccagactgtctctggtcgccgttatttcacgaaagcgtggctgatggagcagaaatcgcttatcgctctgctggtgctgatcgcgattgtctcgacgttaagcccgaactttttcaccatcaataacttattcaatattctccagcaaacctcagtgaacgccattatggcggtcgggatgacgctggtgatcctgacgtcgggcatcgacttatcggtaggttctctgttggcgctgaccggcgcagttgctgcatctatcgtcggcattgaagtcaatgcgctggtggctgtcgctgctgctctcgcgttaggtgccgcaattggtgcggtaaccggggtgattgtagcgaaaggtcgcgtccaggcgtttatcgctacgctggttatgatgcttttactgcgcggcgtgaccatggtttataccaacggtagcccagtgaataccggctttactgagaacgccgatctgtttggctggtttggtattggtcgtccgctgggcgtaccgacgccagtctggatcatggggattgtcttcctcgcggcctggtacatgctgcatcacacgcgtctggggcgttacatctacgcgctgggcggcaacgaagcggcaacgcgtctttctggtatcaacgtcaataaaatcaaaatcatcgtctattctctttgtggtctgctggcatcgctggccgggatcattgaagtggcgcgtctctcctccgcacaacccacggcggggactggctatgagctggatgctattgctgcggtggttctgggcggtacgagtctggcgggcggaaaaggtcgcattgttgggacgttgatcggcgcattaattcttggcttccttaataatggattgaatttgttaggtgtttcctcctattaccagatgatcgtcaaagcggtggtgattttgctggcggtgctggtagacaacaaaaagcagtaataacgactacaggacatcttgaatatgaacatgaaaaaactggctaccctggtttccgctgttgcgctaagcgccaccgtcagtgcgaatgcgatggcaaaagacaccatcgcgctggtggtctccacgcttaacaacccgttctttgtatcgctgaaagatggcgcgcagaaagaggcggataaacttggctataacctggtggtgctggactcccagaacaacccggcgaaagagctggcgaacgtgcaggacttaaccgttcgcggcacaaaaattctgctgattaacccgaccgactccgacgcagtgggtaatgctgtgaagatggctaaccaggcgaacatcccggttatcactcttgaccgccaggcaacgaaaggtgaagtggtgagccacattgcttctgataacgtactgggcggcaaaatcgctggtgattacatcgcgaagaaagcgggtgaaggtgccaaagttatcgagctgcaaggcattgctggtacatccgcagcccgtgaacgtggcgaaggcttccagcaggccgttgctgctcacaagtttaatgttcttgccagccagccagcagattttgatcgcattaaaggtttgaacgtaatgcagaacctgttgaccgctcatccggatgttcaggctgtattcgcgcagaatgatgaaatggcgctgggcgcgctgcgcgcactgcaaactgccggtaaatcggatgtgatggtcgtcggatttgacggtacaccggatggcgaaaaagcggtgaatgatggcaaactagcagcgactatcgctcagctacccgatcagattggcgcgaaaggcgtcgaaaccgcagataaagtgctgaaaggcgagaaagttcaggctaagtatccggttgatctgaaactggttgttaagcagtagttttaatcaggttgtatgacctgatggtgacataaatacgtcatcgacagatgaacgtgtaatataaagaaaagcagggcacgcgccaccctaacacggtggcgcattttatggacatcccgaatatgcaaaacgcaggcagcctcgttgttcttggcagcattaatgctgaccacattcttaatcttcaatcttttcctactccaggcgaaaccgtaaccggtaaccactatcaggttgcatttggcggcaaaggcgcgaatcaggctgtggctgctgggcgtagcggtgcgaatatcgcgtttattgcctgtacgggtgatgacagcattggtgagagcgttcgccagcagctcgccactgataacattgatattactccggtcagcgtgatcaaaggcgaatcaacaggtgtggcgctgatttttgttaatggcgaaggtgagaatgtcatcggtattcatgccggcgctaatgctgccctttccccggcgctggtggaagcgcaacgtgagcgtattgccaacgcgtcagcattattaatgcagctggaatcaccactcgaaagtgtgatggcagcggcgaaaatcgcccatcaaaataagactatcgttgcgcttaacccggctccggctcgcgaacttcctgacgaactgctggcgctggtggacattattacgccaaacgaaacggaagcagaaaagctcaccggtattcgtgttgaaaatgatgaagatgcagcgaaggcggcgcaggtactgcatgaaaaaggtatccgtactgtactgattactttaggaagtcgtggtgtatgggctagcgtgaatggtgaaggtcagcgcgttcctggattccgggtgcaggctgtcgataccattgctgccggagatacctttaacggtgcgttaatcacggcattgctggaagaaaaaccattgccagaggcgattcgttttgcccatgctgccgctgcgattgccgtaacacgtaaaggcgcacaaccttccgtaccgtggcgtgaagagatcgacgcatttttagacaggcagaggtgacgcttggctacaatgaaagatgttgcccgcctggcgggcgtttctacctcaacagtttctcacgttatcaataaagatcgcttcgtcagtgaagcgattaccgccaaagttgaagcggcgattaaagaactcaattacgcgccatcagctctggcgcgtagcctcaaactcaatcaaacacataccattggcatgttgatcactgccagtaccaatcctttctattcagaactggtgcgtggcgttgaacgcagctgcttcgaacgcggttatagtctcgtcctttgcaataccgaaggcgatgaacagcggatgaatcgcaatctggaaacgctgatgcaaaaacgcgttgatggcttgctgttactgtgcaccgaaacgcatcaaccttcgcgtgaaatcatgcaacgttatccgacagtgcctactgtgatgatggactgggctccgttcgatggcgacagcgatcttattcaggataactcgttgctgggcggagacttagcaacgcaatatctgatcgataaaggtcatacccgtatcgcctgtattaccggcccgctggataaaactccggcgcgcctgcggttggaaggttatcgggcggcgatgaaacgtgcgggtctcaacattcctgatggctatgaagtcactggtgattttgaatttaacggcgggtttgacgctatgcgccaactgctatcacatccgctgcgtcctcaggccgtctttaccggaaatgacgctatggctgttggcgtttaccaggcgttatatcaggcagagttacaggttccgcaggatatcgcggtgattggctatgacgatatcgaactggcaagctttatgacgccaccattaaccactatccaccaaccgaaagatgaactgggggagctggcgattgatgtactcatccatcggataacccagccgacccttcagcaacaacgattacaacttactccgattctgatggaacgcggttcggcttagatttacgctgtcttttgatcaaattattaccatcggttgttttcagaagcatgaacattgctgctgaagcaacagtaataatgcccattgtgataaacgtatagtggaattgttcgacagtcgttgtgccttccattccttcataaacgcgaaggacggccgcacttacagcaacgcctaaactaatcgacagttgctgcgtgaccgccagaacactgttaccgctgctggcattgtcatcggtcagatcggcaagtgtgatggtattcatcgcggtaaactgcgtcgacatagccatccctaatataaacaacggcaagatcagcatccatatagccattgctggtgattgcaaagagaactgagcgatcattagcccaataatcaccgtgatccccactaacgtatggcgatagcccagacgacgtaagacttgggtaaccatcgattttgcaataatggaacctaacgctgtcggtgccatcatacagccagcaataaacgcctgataaccaaatcctacctgtaacatcaatggcataaggaacggtacacagccggtccccagacgggttgcaatattgcctacgataccgatcgagaaagtgcgggttttaaataaatctaatgaaattaatgggtttggcgtgcgtcgtgcatggagaatatagagaagcagtaacccgatgctggtgacaattaccgtcaaggcaatccagctggcgacaatcttttccccgaatagctctattccgcttgagaagagaacaaggctgaggccaaacagcaaaaagccagtgatatcgaatctgcgtcgtgcggtggtgaaattgggcatatgtttgcgcgcgtaaagaaggcccgcaatacctatggggatattgattaaaaatatccagtgccaggttgcccaggtgaccagcacgccgccaagaacggggcctaaaattggccccaccagacccggcatggcgacaaaattcaatactggaagaagttcattacgaggataagcgcgcagtaaggccagccgagcaacaggcatcatcattgcgccgcctatcccctgaataacccggaagacaaccagctgtggtagcgaattagaaagtgcgcaggccagagaacccaatgtgaacagactcacggcaagggtaaaaatgcgacgcgtaccgaagcgatcggctagccatccgcttaccggaataagcatcgccaccgtcagcgtataactgatgatggctgattgcatcgcgagaggagaacgattaaggctatgagcgattgcgggtaaggcggtattaagaatagtggcatcaagtgcctgcatgaagaaggccatcgccgcgatccacggcaaacccgccatactgcgcttctttttatcgctcattcaatgtcctgttatcgggttatcacttatcaggtgagcgtagcagcgcctgacaagctttaaatgccgcgtcgccatcgctttggataatcgcatcgacaatcgcctgatgcagatccagctttatcactgtgtcgctggtaattgacgtgaagtaagtgtgataaaccgaatggaatagcgaggcgaatgaggtcaaaaacggattggcgctcatttcatagatatgctcatgccaggccatatcgacttcgatccagcgttcacggcgaaagttctcttttaatgccgccatttcggccattaacgtattgagatgcgctttctgttccgcggtgccaaccgttgctgccagtaggcaggcttgcggctccagacagatacgcataaccagaaagtgatcgatgacctgatgaaagttctcttctgtcatccaccaggtaagcaattcctgatcaagaaaattccagttcgattgtggcatgacccgagtaccaattcgcggtcgcggtaaaaccatcccttttgccgttaacgttttgaccgcttcgcgtaccgctgtacgactcactccaaattgctcgcccagctcaatctcaccgggcaaaatggtgccgggttcatattcaccttttaagatccgttgcgccagcttctcagccagaacatacgaaaggtttttctgtgcagctaactgttgtgcgcttaaaggcattacttatcttcctttttctttttattcctccttagtatgccaccaggaagtgtgattacggttgcaaaaacggcaaattgcttgttttatggcacattaacggggcttttgctgaaaaaatgcgcggtcagaaaattattttaaatttcctcttgtcaggccggaataactccctataatgcgccaccactgacacggaacaacggcaaacacgccgccgggtcagcggggttctcctgagaactccggcagagaaagcaaaaataaatgcttgactctgtagcgggaaagcgtattatgcacaccccgcgccgctgagaaaaagcaaagcggcactgctctttaacaatttatcagacaatctgtgtgggcactcgaagatacggattcttaacgtcgcaagacgaaaaatgaataccaagtctcaagagtgaacacgtaattcattacgaagtttaattctttgagcatcaaacttttaaattgaagagtttgatcatggctcagattgaacgctggcggcaggcctaacacatgcaagtcgaacggtaacaggaaacagcttgctgtttcgctgacgagtggcggacgggtgagtaatgtctgggaaactgcctgatggagggggataactactggaaacggtagctaataccgcataacgtcgcaagaccaaagagggggaccttcgggcctcttgccatcagatgtgcccagatgggattagctagtaggtggggtaacggctcacctaggcgacgatccctagctggtctgagaggatgaccagccacactggaactgagacacggtccagactcctacgggaggcagcagtggggaatattgcacaatgggcgcaagcctgatgcagccatgccgcgtgtatgaagaaggccttcgggttgtaaagtactttcagcggggaggaagggagtaaagttaatacctttgctcattgacgttacccgcagaagaagcaccggctaactccgtgccagcagccgcggtaatacggagggtgcaagcgttaatcggaattactgggcgtaaagcgcacgcaggcggtttgttaagtcagatgtgaaatccccgggctcaacctgggaactgcatctgatactggcaagcttgagtctcgtagaggggggtagaattccaggtgtagcggtgaaatgcgtagagatctggaggaataccggtggcgaaggcggccccctggacgaagactgacgctcaggtgcgaaagcgtggggagcaaacaggattagataccctggtagtccacgccgtaaacgatgtcgacttggaggttgtgcccttgaggcgtggcttccggagctaacgcgttaagtcgaccgcctggggagtacggccgcaaggttaaaactcaaatgaattgacgggggcccgcacaagcggtggagcatgtggtttaattcgatgcaacgcgaagaaccttacctggtcttgacatccacggaagttttcagagatgagaatgtgccttcgggaaccgtgagacaggtgctgcatggctgtcgtcagctcgtgttgtgaaatgttgggttaagtcccgcaacgagcgcaacccttatcctttgttgccagcggtccggccgggaactcaaaggagactgccagtgataaactggaggaaggtggggatgacgtcaagtcatcatggcccttacgaccagggctacacacgtgctacaatggcgcatacaaagagaagcgacctcgcgagagcaagcggacctcataaagtgcgtcgtagtccggattggagtctgcaactcgactccatgaagtcggaatcgctagtaatcgtggatcagaatgccacggtgaatacgttcccgggccttgtacacaccgcccgtcacaccatgggagtgggttgcaaaagaagtaggtagcttaaccttcgggagggcgcttaccactttgtgattcatgactggggtgaagtcgtaacaaggtaaccgtaggggaacctgcggttggatcacctccttaccttaaagaagcgttctttgcagtgctcacacagattgtctgataggaagtgaaaagcaaggcgtcttgcgaagcagactgatacgtccccttcgtctagaggcccaggacaccgccctttcacggcggtaacaggggttcgaatcccctaggggacgccacttgctggtttgtgagtgaaagtcacctgccttaatatctcaaaactcatcttcgggtgatgtttgagatatttgctctttaaaaatctggatcaagctgaaaattgaaacactgaacaacgaaagttgttcgtgagtctctcaaattttcgcaacacgatgatgaatcgaaagaaacatcttcgggttgtgaggttaagcgactaagcgtacacggtggatgccctggcagtcagaggcgatgaaggacgtgctaatctgcgataagcgtcggtaaggtgatatgaaccgttataaccggcgatttccgaatggggaaacccagtgtgtttcgacacactatcattaactgaatccataggttaatgaggcgaaccgggggaactgaaacatctaagtaccccgaggaaaagaaatcaaccgagattcccccagtagcggcgagcgaacggggagcagcccagagcctgaatcagtatgtgtgttagtggaagcgtctggaaaggcgcgcgatacagggtgacagccccgtacacaaaaatgcacatattgtgagctcgatgagtagggcgggacacgtggtatcctgtctgaatatggggggaccatcctccaaggctaaatactcctgactgaccgatagtgaaccagtaccgtgagggaaaggcgaaaagaaccccggcgaggggagtgaaaaagaacctgaaaccgtgtacgtacaagcagtgggagcacgcttaggcgtgtgactgcgtaccttttgtataatgggtcagcgacttatattctgtagcaaggttaaccgaataggggagccgaagggaaaccgagtcttaactgggcgttaagttgcagggtatagacccgaaacccggtgatctagccatgggcaggttgaaggttgggtaacactaactggaggaccgaaccgactaatgttgaaaaattagcggatgacttgtggctgggggtgaaaggccaatcaaaccgggagatagctggttctccccgaaagctatttaggtagcgcctcgtgaattcatctccgggggtagagcactgtttcggcaagggggtcatcccgacttaccaacccgatgcaaactgcgaataccggagaatgttatcacgggagacacacggcgggtgctaacgtccgtcgtgaagagggaaacaacccagaccgccagctaaggtcccaaagtcatggttaagtgggaaacgatgtgggaaggcccagacagccaggatgttggcttagaagcagccatcatttaaagaaagcgtaatagctcactggtcgagtcggcctgcgcggaagatgtaacggggctaaaccatgcaccgaagctgcggcagcgacgcttatgcgttgttgggtaggggagcgttctgtaagcctgcgaaggtgtgctgtgaggcatgctggaggtatcagaagtgcgaatgctgacataagtaacgataaagcgggtgaaaagcccgctcgccggaagaccaagggttcctgtccaacgttaatcggggcagggtgagtcgacccctaaggcgaggccgaaaggcgtagtcgatgggaaacaggttaatattcctgtacttggtgttactgcgaaggggggacggagaaggctatgttggccgggcgacggttgtcccggtttaagcgtgtaggctggttttccaggcaaatccggaaaatcaaggctgaggcgtgatgacgaggcactacggtgctgaagcaacaaatgccctgcttccaggaaaagcctctaagcatcaggtaacatcaaatcgtaccccaaaccgacacaggtggtcaggtagagaataccaaggcgcttgagagaactcgggtgaaggaactaggcaaaatggtgccgtaacttcgggagaaggcacgctgatatgtaggtgaagcgacttgctcgtggagctgaaatcagtcgaagataccagctggctgcaactgtttattaaaaacacagcactgtgcaaacacgaaagtggacgtatacggtgtgacgcctgcccggtgccggaaggttaattgatggggtcagcgcaagcgaagctcttgatcgaagccccggtaaacggcggccgtaactataacggtcctaaggtagcgaaattccttgtcgggtaagttccgacctgcacgaatggcgtaatgatggccaggctgtctccacccgagactcagtgaaattgaactcgctgtgaagatgcagtgtacccgcggcaagacggaaagaccccgtgaacctttactatagcttgacactgaacattgagccttgatgtgtaggataggtgggaggctttgaagtgtggacgccagtctgcatggagccgaccttgaaataccaccctttaatgtttgatgttctaacgtggacccgtgatccgggttgcggacagtgtctggtgggtagtttgactggggcggtctcctcctaaagagtaacggaggagcacgaaggttggctaatcctggtcggacatcaggaggttagtgcaatggcataagccagcttgactgcgagcgtgacggcgcgagcaggtgcgaaagcaggtcatagtgatccggtggttctgaatggaagggccatcgctcaacggataaaaggtactccggggataacaggctgataccgcccaagagttcatatcgacggcggtgtttggcacctcgatgtcggctcatcacatcctggagctgaagtaggtcccaagggtatggctgttcgccatttaaagtggtacgcgagctgggtttagaacgtcgtgagacagttcggtccctatctgccgtgggcgctggagaactgaggggggctgctcctagtacgagaggaccggagtggacgcatcactggtgttcgggttgtcatgccaatggcactgcccggtagctaaatgcggaagagataagtgctgaaagcatctaagcacgaaacttgccccgagatgagttctccctgactccttgagagtcctgaaggaacgttgaagacgacgacgttgataggccgggtgtgtaagcgcagcgatgcgttgagctaaccggtactaatgaaccgtgaggcttaaccttacaacgccgaagatgttttggcggatgagagaagattttcagcctgatacagattaaatcagaacgcagaagcggtctgatgaaacagaatttgcctggcggccgtagcgcggtggtcccacctgaccccatgccgaactcagaagtgaaacgccgtagcgccgatggtagtgtggggtctccccatgcgagagtagggaactgccaggcatcaaattaagcagtaagccggtcataaaaccggtggttgtaaaagaattcggtggagcggtagttcagtcggttagaatacctgcctgtcacgcagggggtcgcgggttcgagtcccgtccgttccgccaccctaattaggggcgtagttcaattggtagagcaccggtctccaaaaccgggtgttgggagttcgagtctctccgcccctgccagaaatcatccttagcgaaagctaaggattttttttatctgaaataaccctctccgaagtaaatccttctaccggcatccttgccagccattcatattaatacacttcatccagcacgttaattttcaaaagatcgcgaatcaacgcatttttatcgctattttgcagccatatggcataaagcggccgtgaaagtgttgtgctatcgacaacggtatgcaggccgccttttttacgcgcccagctgacgggtagccaggtgcaaccattaagcatcgcaatctgttgctgtgccagttcagcagaactggttgtcagaatgggcacttcgtcagcaccgatcaaacctgcctcatgctgttgaaaatctggcccccactcaagtcgcagataattaagatctccctttagttttgaaggggcactggtataaagcgctaaagtgaaatatcccagcaactgactactaaattcgtccattttgggcgcttcagtggtaataagaagatcaagctggcgttcatgcagctgttttaccagagactgccgttgggcaattcgcgcttcgaactgtaagcctgtatgggcatcctgattttgatacaagcgtcccagccactgattaagcatacattcccacaacgaggcgctggcaccgatagaaaactcgttatgtcgtgaggtatgcgccacctccttacgggcggcctgccaggtgctcatgagcgtttctgcataaggcagtagtttttcaccggcagcggttaaacggatattgtttctgtggcgggtgaaaaggttcacacccagttgattttccagttgtctgattcgaaagctcactgctgactgggtcagatagagcgattcagccgctcgaccaaagtgacgcgttcggctaacttccaggaaagtttttaacaattccgtatccacagtgctctccgcaaaattatttgtcgttatgatttaaatgttttgttttacactctgtcaagcgtaactaatactccgcgccataactagctcggtcaaagaattaggagcgtgcaggatggcggaaagctttacgacgactaatcgatatttcgacaataaacattatccacgtggattctctcgtcatggtgatttcaccatcaaagaggcacaactgcttgagcgtcatggttatgccttcaatgagttggatcttggcaaacgcgagccggttaccgaggaagagaaactcttcgtagcagtatgccgtggcgaacgtgagccagtgacagaagcagaacgcgtgtggtccaagtatatgacgcgtattaagcgtccaaaacgttttcacaccctttccggcggtaaaccgcaggttgaaggtgctgaagactacaccgattctgacgattaataaaaagggcgaaatgccctttttttatgtcagtagtttctgcagatggatgagcaaacggtcaatcgctcgatagctaactgcctcctgcaaatgctgacgtgtgataatgtcagactgatcaatatcagcaatggttcgtgcaactttcaataaccgctgccaggcacgaatcgataaccccagatggatcagtgttccttccaaccacatcgcatcttcgctctcaagtttgcagaattggcgtatttccggactatccagccaggcattcagtttattctgccgcttaaattggcgctctctggcggccattacgcgttgtttaacggtggcgctgctttctcccggcactaccgttttactcaaaatgccggggggtggtaatgggatctccagtgagagatcgaagcggtcgagaaagggccccgagagccggttgagataacgtaatgtctgttctggcgtgcagcggttatggtttccctgataatgtccggtagggctgggattcatcgccgcaacaagctggaaacgggctggataggttatttttgctcgtgtgcgtgaaagatggatctgcccggattcaatcggctctcgcaaggcatccagtgtacgccgttcaaattcaggtagctcatcaagaaaaagcacgccgttatgcgccagcgaaatttcaccgggccctggaattgcgccaccgcctaccatcgcagttaacgatgcactgtgatgaggtgagcggaacgggcgctgccgccattgtttttgtactgattcagcatttaccagacttaatatcgcagcactctccagtgcctcttcattgcttaaatctggcaacaggccattaatacggctggcgagcattgttttacctgttcccggcggcccaatcagtaaaaggttgtgcccgccagcagcggtaatttccagtcctcgctttccttgttcctgaccgataacatcactgagatcatgttgtagcgcccgggatactgcatcagttggtttcgggcgttcgagagcgtgcttaccttccagaaacgcacagacagcttgcagatgatcggctatcaggcatccttcaccgttaattagccccacttcatcttcgttatctttcgcgacgataatttttctgcccgacttaatagcttcagttgcactggagattgcgccgggaacgccacgcagagcgcctgtaagcgccagttctccgactaattcatattcatctaacttattggctgtaagctgttctgaggccgccagcaacgcaatggcgataggtaaatcatatcgtcccccttcttttggcagatcagctggagccaggttgatggtgatttttttcgccggatattcatatccgctattgataatggcgctgcgcacgcgatcgcgagcttcttttaccgttgtttctggtaagcccaccatcgttaagccgggtagacctttactgatatgtacctcaacagtgatcgggggcgcatttactcccagggctgcgcgggtatgaacaattgacagtgacataagccctccttgagtcaccattatgtgcataagatatcgctgctgtagcccgctaattcgtgaattttagtggctgattcctgtttatttgtgcaagtgaagttgagttgttctggcggtggaatgatgctcgcaaaaatgcagcggacaaaggatgaactacgaggaagggaacaacattcatactgaaattgaatttttttcactcactattttatttttaaaaaacaacaatttatattgaaattattaaacgcatcataaaaatcggccaaaaaatatcttgtactatttacaaaacctatggtaactctttaggcattccttcgaacaagatgcaagaaaagacaaaatgacagcccttctacgagtgattagcctggtcgtgattagcgtggtggtgattattatcccaccgtgcggggctgcacttggacgaggaaaggcttagagatcaagccttaacgaactaagacccccgcaccgaaaggtccgggggttttttttgaccttaaaaacataaccgaggagcagacaatgaataacagcacaaaattctgtttctcaagattcaggacggggaactaactatgaatggcgcacagtgggtggtacatgcgttgcgggcacagggtgtgaacaccgttttcggttatccgggtggcgcaattatgccggtttacgatgcattgtatgacggcggcgtggagcacttgctatgccgacatgagcagggtgcggcaatggcggctatcggttatgctcgtgctaccggcaaaactggcgtatgtatcgccacgtctggtccgggcgcaaccaacctgataaccgggcttgcggacgcactgttagattccatccctgttgttgccatcaccggtcaagtgtccgcaccgtttatcggcactgacgcatttcaggaagtggatgtcctgggattgtcgttagcctgtaccaagcacagctttctggtgcagtcgctggaagagttgccgcgcatcatggctgaagcattcgacgttgcctgctcaggtcgtcctggtccggttctggtcgatatcccaaaagatatccagttagccagcggtgacctggaaccgtggttcaccaccgttgaaaacgaagtgactttcccacatgccgaagttgagcaagcgcgccagatgctggcaaaagcgcaaaaaccgatgctgtacgttggcggtggcgtgggtatggcgcaggcagttccggctttgcgtgaatttctcgctgccacaaaaatgcctgccacctgtacgctgaaagggctgggcgcagtagaagcagattatccgtactatctgggcatgctggggatgcacggcaccaaagcggcaaacttcgcggtgcaggagtgtgacctgctgatcgccgtgggcgcacgttttgatgaccgggtgaccggcaaactgaacaccttcgcgccacacgccagtgttatccatatggatatcgacccggcagaaatgaacaagctgcgtcaggcacatgtggcattacaaggtgatttaaatgctctgttaccagcattacagcagccgttaaatcaatgactggcagcaacactgcgcgcagctgcgtgatgaacattcctggcgttacgaccatcccggtgacgctatctacgcgccgttgttgttaaaacaactgtcggatcgtaaacctgcggattgcgtcgtgaccacagatgtggggcagcaccagatgtgggctgcgcagcacatcgcccacactcgcccggaaaatttcatcacctccagcggtttaggtaccatgggttttggtttaccggcggcggttggcgcacaagtcgcgcgaccgaacgataccgttgtctgtatctccggtgacggctctttcatgatgaatgtgcaagagctgggcaccgtaaaacgcaagcagttaccgttgaaaatcgtcttactcgataaccaacggttagggatggttcgacaatggcagcaactgttttttcaggaacgatacagcgaaaccacccttactgataaccccgatttcctcatgttagccagcgccttcggcatccatggccaacacatcacccggaaagaccaggttgaagcggcactcgacaccatgctgaacagtgatgggccatacctgcttcatgtctcaatcgacgaacttgagaacgtctggccgctggtgccgcctggcgccagtaattcagaaatgttggagaaattatcatgatgcaacatcaggtcaatgtatcggctcgcttcaatccagaaaccttagaacgtgttttacgcgtggtgcgtcatcgtggtttccacgtctgctcaatgaatatggccgccgccagcgatgcacaaaatataaatatcgaattgaccgttgccagcccacggtcggtcgacttactgtttagtcagttaaataaactggtggacgtcgcacacgttgccatctgccagagcacaaccacatcacaacaaatccgcgcctgagcgcaaaaggaatataaaaatgaccacgaagaaagctgattacatttggttcaatggggagatggttcgctgggaagacgcgaaggtgcatgtgatgtcgcacgcgctgcactatggcacttcggtttttgaaggcatccgttgctacgactcgcacaaaggaccggttgtattccgccatcgtgagcatatgcagcgtctgcatgactccgccaaaatctatcgcttcccggtttcgcagagcattgatgagctgatggaagcttgtcgtgacgtgatccgcaaaaacaatctcaccagcgcctatatccgtccgctgatcttcgtcggtgatgttggcatgggagtaaacccgccagcgggatactcaaccgacgtgattatcgctgctttcccgtggggagcgtatctgggcgcagaagcgctggagcaggggatcgatgcgatggtttcctcctggaaccgcgcagcaccaaacaccatcccgacggcggcaaaagccggtggtaactacctctcttccctgctggtgggtagcgaagcgcgccgccacggttatcaggaaggtatcgcgctggatgtgaacggttatatctctgaaggcgcaggcgaaaacctgtttgaagtgaaagatggtgtgctgttcaccccaccgttcacctcctccgcgctgccgggtattacccgtgatgccatcatcaaactggcgaaagagctgggaattgaagtacgtgagcaggtgctgtcgcgcgaatccctgtacctggcggatgaagtgtttatgtccggtacggcggcagaaatcacgccagtgcgcagcgtagacggtattcaggttggcgaaggccgttgtggcccggttaccaaacgcattcagcaagccttcttcggcctcttcactggcgaaaccgaagataaatggggctggttagatcaagttaatcaataaatacaaaaaatgggacggcacgcaccgtcccatttacgagacagacactgggagtaaataaagtatgcctaagtaccgttccgccaccaccactcatggtcgtaatatggcgggtgctcgtgcgctgtggcgcgccaccggaatgaccgacgccgatttcggtaagccgattatcgcggttgtgaactcgttcacccaatttgtaccgggtcacgtccatctgcgcgatctcggtaaactggtcgccgaacaaattgaagcggctggcggcgttgccaaagagttcaacaccattgcggtggatgatgggattgccatgggccacggggggatgctttattcactgccatctcgcgaactgatcgctgattccgttgagtatatggtcaacgcccactgcgccgacgccatggtctgcatctctaactgcgacaaaatcaccccggggatgctgatggcttccctgcgcctgaatattccggtgatctttgtttccggcggcccgatggaggccgggaaaaccaaactttccgatcagatcatcaagctcgatctggttgatgcgatgatccagggcgcagacccgaaagtatctgactcccagagcgatcaggttgaacgttccgcgtgtccgacctgcggttcctgctccgggatgtttaccgctaactcaatgaactgcctgaccgaagcgctgggcctgtcgcagccgggcaacggctcgctgctggcaacccacgccgaccgtaagcagctgttccttaatgctggtaaacgcattgttgaattgaccaaacgttattacgagcaaaacgacgaaagtgcactgccgcgtaatatcgccagtaaggcggcgtttgaaaacgccatgacgctggatatcgcgatgggtggatcgactaacaccgtacttcacctgctggcggcggcgcaggaagcggaaatcgacttcaccatgagtgatatcgataagctttcccgcaaggttccacagctgtgtaaagttgcgccgagcacccagaaataccatatggaagatgttcaccgtgctggtggtgttatcggtattctcggcgaactggatcgcgcggggttactgaaccgtgatgtgaaaaacgtacttggcctgacgttgccgcaaacgctggaacaatacgacgttatgctgacccaggatgacgcggtaaaaaatatgttccgcgcaggtcctgcaggcattcgtaccacacaggcattctcgcaagattgccgttgggatacgctggacgacgatcgcgccaatggctgtatccgctcgctggaacacgcctacagcaaagacggcggcctggcggtgctctacggtaactttgcggaaaacggctgcatcgtgaaaacggcaggcgtcgatgacagcatcctcaaattcaccggcccggcgaaagtgtacgaaagccaggacgatgcggtagaagcgattctcggcggtaaagttgtcgccggagatgtggtagtaattcgctatgaaggcccgaaaggcggtccggggatgcaggaaatgctctacccaaccagcttcctgaaatcaatgggtctcggcaaagcctgtgcgctgatcaccgacggtcgtttctctggtggcacctctggtctttccatcggccacgtctcaccggaagcggcaagcggcggcagcattggcctgattgaagatggtgacctgatcgctatcgacatcccgaaccgtggcattcagttacaggtaagcgatgccgaactggcggcgcgtcgtgaagcgcaggacgctcgaggtgacaaagcctggacgccgaaaaatcgtgaacgtcaggtctcctttgccctgcgtgcttatgccagcctggcaaccagcgccgacaaaggcgcggtgcgcgataaatcgaaactggggggttaataatggctgactcgcaacccctgtccggtgctccggaaggtgccgaatatttaagagcagtgctgcgcgcgccggtttacgaggcggcgcaggttacgccgctacaaaaaatggaaaaactgtcgtcgcgtcttgataacgtcattctggtgaagcgcgaagatcgccagccagtgcacagctttaagctgcgcggcgcatacgccatgatggcgggcctgacggaagaacagaaagcgcacggcgtgatcactgcttctgcgggtaaccacgcgcagggcgtcgcgttttcttctgcgcggttaggcgtgaaggccctgatcgttatgccaaccgccaccgccgacatcaaagtcgacgcggtgcgcggcttcggcggcgaagtgctgctccacggcgcgaactttgatgaagcgaaagccaaagcgatcgaactgtcacagcagcaggggttcacctgggtgccgccgttcgaccatccgatggtgattgccgggcaaggcacgctggcgctggaactgctccagcaggacgcccatctcgaccgcgtatttgtgccagtcggcggcggcggtctggctgctggcgtggcggtgctgatcaaacaactgatgccgcaaatcaaagtgatcgccgtagaagcggaagactccgcctgcctgaaagcagcgctggatgcgggtcatccggttgatctgccgcgcgtagggctatttgctgaaggcgtagcggtaaaacgcatcggtgacgaaaccttccgtttatgccaggagtatctcgacgacatcatcaccgtcgatagcgatgcgatctgtgcggcgatgaaggatttattcgaagatgtgcgcgcggtggcggaaccctctggcgcgctggcgctggcgggaatgaaaaaatatatcgccctgcacaacattcgcggcgaacggctggcgcatattctttccggtgccaacgtgaacttccacggcctgcgctacgtctcagaacgctgcgaactgggcgaacagcgtgaagcgttgttggcggtgaccattccggaagaaaaaggcagcttcctcaaattctgccaactgcttggcgggcgttcggtcaccgagttcaactaccgttttgccgatgccaaaaacgcctgcatctttgtcggtgtgcgcctgagccgcggcctcgaagagcgcaaagaaattttgcagatgctcaacgacggcggctacagcgtggttgatctctccgacgacgaaatggcgaagctacacgtgcgctatatggtcggcggacgtccatcgcatccgttgcaggaacgcctctacagcttcgaattcccggaatcaccgggcgcgctgctgcgcttcctcaacacgctgggtacgtactggaacatttctttgttccactatcgcagccatggcaccgactacgggcgcgtactggcggcgttcgaacttggcgaccatgaaccggatttcgaaacccggctgaatgagctgggctacgattgccacgacgaaaccaataacccggcgttcaggttctttttggcgggttagggaaaaatgcctgatagcgcttcgcttatcaggcctacccgcgcgacaacgtcatttgtggttcggcaaaatcttccagaatgcctcaattagcggctcatgtagccgctttttctgcgcacacacgcccagctcaaacggcgttttctcatcgctgcgctctaaaatcatcacgcggttacgcaccggttcggggctgttttccagcaccacttccggcaacaatgccacgccacagccgagtgccaccatcgataccatcgcttcatgcccgccaaccgtggcgtaaatcatcgggttactgattttattgcgtcgaaaccacagttcaatgcggcggcgtaccggcccctgatcggccataataaacggcaccgttgaccagtccggcttctctaccgacacctgattacgcaccgggcagggcagcgcgggggcaatcagcactactgccagattctccagcatcgaaaacgccactgcgccgggcaaggtttccggtttacccgcaatcgccagatccgcttcaccagtgaccaccttttccatcgcatctgccgcatcaccagtagtaagtttaatctccaccgacgggtgttccgcgcggaagcgatccagaatcggcggcagatggctgtaggcagcggtcaccgagcagaagatatgtaattcgccagagagcgacggcccttgctgatcgatggtgtggcgcaactgctgatactgcaacagcgtttgctgggcgaaaacgcgcagctcttcgcccgcttcagtcagcgtcaccgtgcggttatcgcgcacaaacagcggctgaccgagatcttcttccaggcgctgaatctgccgtgagagcgtggatgggctaacgtgcatcgcccgcgcgctgcggccaaaatggcggctttccgccagatgcaggaaggttttcagatcgcgtaaatccacagggacagccctcgatgttgacgttgcaaaaattgcaatgtgacgttgtgaatatatcaatttccgcaataaatttcctgtcatatagtgaattcaatctcgcaaacgcgaaccgaacaataagaagcacaacatcacgaggaatcaccatggctaactacttcaatacactgaatctgcgccagcagctggcacagctgggcaaatgtcgctttatgggccgcgatgaattcgccgatggcgcgagctaccttcagggtaaaaaagtagtcatcgtcggctgtggcgcacagggtctgaaccagggcctgaacatgcgtgattctggtctcgatatctcctacgctctgcgtaaagaagcgattgccgagaagcgcgcgtcctggcgtaaagcgaccgaaaatggttttaaagtgggtacttacgaagaactgatcccacaggcggatctggtgattaacctgacgccggacaagcagcactctgatgtagtgcgcaccgtacagccactgatgaaagacggcgcggcgctgggctactcgcacggtttcaacatcgtcgaagtgggcgagcagatccgtaaagatatcaccgtagtgatggttgcgccgaaatgcccaggcaccgaagtgcgtgaagagtacaaacgtgggttcggcgtaccgacgctgattgccgttcacccggaaaacgatccgaaaggcgaaggcatggcgattgccaaagcctgggcggctgcaaccggtggtcaccgtgcgggtgtgctggaatcgtccttcgttgcggaagtgaaatctgacctgatgggcgagcaaaccatcctgtgcggtatgttgcaggctggctctctgctgtgcttcgacaagctggtggaagaaggtaccgatccagcatacgcagaaaaactgattcagttcggttgggaaaccatcaccgaagcactgaaacagggcggcatcaccctgatgatggaccgtctctctaacccggcgaaactgcgtgcttatgcgctttctgaacagctgaaagagatcatggcacccctgttccagaaacatatggacgacatcatctccggcgaattctcttccggtatgatggcggactgggccaacgatgataagaaactgctgacctggcgtgaagagaccggcaaaaccgcgtttgaaaccgcgccgcagtatgaaggcaaaatcggcgagcaggagtacttcgataaaggcgtactgatgattgcgatggtgaaagcgggcgttgaactggcgttcgaaaccatggtcgattccggcatcattgaagagtctgcatattatgaatcactgcacgagctgccgctgattgccaacaccatcgcccgtaagcgtctgtacgaaatgaacgtggttatctctgataccgctgagtacggtaactatctgttctcttacgcttgtgtgccgttgctgaaaccgtttatggcagagctgcaaccgggcgacctgggtaaagctattccggaaggcgcggtagataacgggcaactgcgtgatgtgaacgaagcgattcgcagccatgcgattgagcaggtaggtaagaaactgcgcggctatatgacagatatgaaacgtattgctgttgcgggttaagtgcgcgctgatgccctcaccccgaccctctcccacagggagagggagaaaacactcaaggccttctcctggagaaggccttgctattagttgcggtacagcaccttaatgatgtgatatccgaactgggtgtgcagcgggccggtcggctccagtaccggacaagagaaaaccactttatcgaacgccggaaccatctgaccctggcggaattcacctaaatcaccgccgcgtttgcctgatgggcaaatggagtgtttcttcgccagcttgccgaaatcggccccgttcttaatctgctcgagaagatccagagccagtttctcttcttttacaaggatatgcagtgctgctgctgtttttgccatgatcgtgccttgagtgaataattgtcaggcggcgattttagcatgatccgcagatgctaacgtaattgtcagtcagggagtggctggtacatatatggcaaaagcccggaaaatccgggcttcgcaggtccctcaaggggagaaaacttagggcctctatgggctacaaagtcattatcggggatggttattttattgtcaatttatgagcgatatggcattgattgacttgatgaccgccctctgtatgtctgcaaccaactcatgtggcaaacattgattaagataccctctgtaagtccttgctctgtttaatctgtttcgactgacttgttgtaccaggtcggctttggcccaacgaatctgctgatcaaagaattgcaggtcattgataacattactggctatttcaacatgcattccacgttttaacttgtctggtcgcgagtggttgataatggaacgacgatgcatgcgttgccattaatttttccgttgagcacgacaactaacctgttttttatcatttcaggaggaatgcggccatcgtaatacgtcgtgctgaacggtccattttggctaacaggatagttaccaaagttgcattccagtatttcaccaaccttagggctgaaattaatcgccacgagtaaacctctccttagtaaactctgaaaaagtaataacacaacgttacgacccgatattttctaagtctaatggattcacgatgaactccgatttcggtcttctctctctgatttaaacatccgcagccaaccggttagcggcttacacgcggtcacattcaaatgcgattctgctacaatcctccccccgttcgaagattgagcaatacacctatgcgtctaaaccccggccaacaacaagctgtcgaattcgttaccggcccctgcctggtgctggcgggcgcgggttccggtaaaactcgtgttatcaccaataaaatcgcccatctgatccgcggttgcggttatcaggcgcggcacattgcggcggtgacctttactaataaagcagcgcgcgagatgaaagagcgtgtagggcagacgctggggcgcaaagaggcgcgtgggctgatgatctccactttccatacgttggggctggatatcatcaaacgcgagtatgcggcgcttgggatgaaagcgaacttctcgttgtttgacgataccgatcagcttgctttgcttaaagagttgaccgaggggctgattgaagatgacaaagttctcctgcaacaactgatttcgaccatctctaactggaagaatgatctcaaaacaccgtcccaggcggcagcaagtgcgattggcgagcgggaccgtatttttgcccattgttatgggctgtatgatgcacacctgaaagcctgtaacgttctcgacttcgatgatctgattttattgccgacgttgctgctgcaacgcaatgaagaagtccgcaagcgctggcagaacaaaattcgctatctgctggtggatgagtatcaggacaccaacaccagccagtatgagctggtgaaactgctggtgggcagccgcgcgcgctttaccgtggtgggtgacgatgaccagtcgatctactcctggcgcggtgcacgtccgcaaaacctggtgctgctgagtcaggattttccggcgctgaaggtgattaagcttgagcagaactatcgctcttccgggcgtattctgaaagcggcgaacatcctgatcgccaataacccgcacgtctttgaaaagcgtctgttctccgaactgggttatggcgcggagctaaaagtattaagcgcgaataacgaagaacatgaggctgagcgcgttactggcgagctgatcgcccatcacttcgtcaataaaacgcagtacaaagattacgccattctttatcgcggtaaccatcagtcgcgggtgtttgaaaaattcctgatgcaaaaccgcatcccgtacaaaatatctggtggtacgtcgtttttctctcgtcctgaaatcaaggacttgctggcttatctgcgcgtgctgactaacccggacgatgacagcgcatttctgcgtatcgttaacacgccgaagcgagagattggcccggctacgctgaaaaagctgggtgagtgggcgatgacgcgcaataaaagcatgtttaccgccagctttgatatgggcctgagtcagacgcttagcggacgtggttatgaagcattgacccgcttcactcactggttggcagaaatccagcgtctggcggagcgggagccgattgccgcggtgcgtgatctgatccatggcatggattatgaatcctggctgtacgaaacatcgcccagcccgaaagccgccgaaatgcgcatgaagaacgtcaaccaactgtttagctggatgacggagatgctggaaggcagtgaactggatgagccgatgacgctcacccaggtggtgacgcgctttactttgcgcgacatgatggagcgtggtgagagtgaagaagagctggatcaggtgcaactgatgactctccacgcgtcgaaagggctggagtttccttatgtctacatggtcggtatggaagaagggtttttgccgcaccagagcagcatcgatgaagataatatcgatgaggagcggcggctggcctatgtcggcattacccgcgcccagaaggaattgacctttacgctgtgtaaagaacgccgtcagtacggcgaactggtgcgcccggagccgagccgctttttgctggagctgccgcaggatgatctgatttgggaacaggagcgcaaagtggtcagcgccgaagaacggatgcagaaagggcaaagccatctggcgaatctgaaagcgatgatggcggcaaaacgagggaaataatcaaggccggaaaagatgcgtcagcatcgcatccggcacttactcattaatgcacttccagcggccagtggacatagctctgccactggctttcctgagcaataatctctttacccagcggatgttgggttagccaaccttgcggaagcgtcaaggtcaacagttcatggttagcctgtaatgtcatctctggcacgagatcgtcacggcgacggctggcaaaaatgatggccaggcgtagtaaacggcagagttgttctgcgacgcgcggcggtacggcattttgctgatgcagcgatgagagatcgaccggattagtctggttgagcagtagcgtcgccagcaattttttctgtgcgggggtaaaaccgggaagatccagattacgcaccagataagcagcgtgttgcggcgcttgtttgaagtcaacgctcaggccgatttcatgaagctgacaggcgctgatgagcaaatcgcggcttattgcttcaagatgccattcgttttccacctgatcgaagaagttagccgcaactttggctacgcgctgtgcctgatcaatatcgatcataaagcggcgttgaatattacgcagcgtacggctgcgaatatcctgctcgacggccagatgcaacatgccgtagaccaggccttcacgcagcgcaccgcccgccagggtcatacactgaatattcagttcggtaaaaatggcgatcaggatcgccagaccactcgggaacactaacgcacgttccagcgtcagcccgtcaatctccagttcctccagccgaccgcaatgaatggctcgctgtttcaattgctgcaacttttccagggtaatgcgttcatccatcccctgtgccatcatgatttcctgtaacgcctgcacggtgccggaagcaccaacgcacactttccagccgtgataccgtaattcatcggcaaccggacgtaacacttcgcgtgccgctttttctgcagcatcaaaattttcctgccccagattacgatcggcaaaatagcgttccagccaggtgacgcagcccatcgacaggctgaacaacgaggtggtttgtgcacccgtgccggttaccagttcagtactggctccgcctatatccaccaccaggcgctgatcggcaccaccagtggtgtgagcaacgccctgataaatcagacgtgcttcctcttcaccgctgatcacctgtaccggacaaccgagaatttcctgcgctttggcaataaaatcacccgcattgacggcaaggcgtaacgtcgccgtagcgacaacgcgaatttgcgagggaggaatatcttgcagacgttcagcaaacaggcgcaaacattgccaaccgcgctccattgcttcattggagagggcattttcgctattcaggccagcagccagacgcactttgcgttttattcgcgtcagcgtctggatgcttccagccacctcgcgcacaaccagcatatgaaaactattcgaaccgagatcaatggctgcatacagcgacgaggtggaacccatactcttcatccttcaatctgtctctgtgttggctgcattctttcacctgaatcacttactacagtaagctcatcgggattcattctcttgccatcttgatacagtttgaatgattttgagtatgacattttttatttaacctgaacgacgacgattacgcggagcgccagtacgacgcggaccattgcctgtgcgcgggcgcgtgaggcgcagcggttttggcagatcggtcatcaatgcgtccggattgtatttgcttaccggaattgagtgaccaatataggtctcaatagcaggcaaattcaatgcatactcttcacacgccaggctgatagagtgaccgcttgcgcctgcgcgacctgtacgaccaatacggtgaacgtaatcttcacagtcatcgggtaaatcgtagttaaagacgtgcgtcactgccggaatatgcaaaccacgcgcggcaacgtcggtggcaaccagaatatccagatcgccacgggtaaattcatcaagaatacgcagacgttttttctgcgcgacatcgcctgtcaataaaccgacacgatgaccatctgctgccaggtggccccagatctcttcacaacggtgtttggtgttggcgaaaataatcgctctgtctggccactcttcttcgatcagcgtttgcagcaaacgcattttttcttcgttagaagggtagaaaagctcttctttaatacggtggcccgttttctgttccggttccacttcaatatattcggcattgttcatctgctcgaacgccagttcacgtacccggtacgaaagcgtggcggagaacagcatgttgaggcgctggtttgcaggcggcatacggcggaacagccagcggatatctttaataaagcccagatcgtacatgcgatcggcttcgtccagtaccaccacctgaatggcaccgaggttaatgtggttctgcttggcgtagtcaattaaacgccccgtggtgccaatcagaatgtcaacgccgctttccagcactttcagctgtttgtcgtagccatcaccaccgtaagccagacccagcttcaggccagtagcttccgccagcggttctgcgtcggcatggatctgcacggcaagttcacgcgtcggtgccataattaaggcacgcggctgattcaccttgcgatcggcaatcgcaggatgagagagaagataatgaaacgttgacgtaagaaacgccatcgttttcccggtaccggtttgcgcctgcccggctacgtcacgacccgccagcgtcagcggaagggccagtgcctgaatgggcgtacagttatgaaacccttttttttcaagggcttctacaaccttcggatgcagggcgaagtcggaaaacttctgttctgttaaatgtgttttgctcatagtgtggtagaatatcagcttactattgctttacgaaagcgtatccggtgaaataaagtcaacctttagttggttaatgttacaccaacaacgaaaccaacacgccaggcttattcctgtggagttatatatgagcgataaaattattcacctgactgacgacagttttgacacggatgtactcaaagcggacggggcgatcctcgtcgatttctgggcagagtggtgcggtccgtgcaaaatgatcgccccgattctggatgaaatcgctgacgaatatcagggcaaactgaccgttgcaaaactgaacatcgatcaaaaccctggcactgcgccgaaatatggcatccgtggtatcccgactctgctgctgttcaaaaacggtgaagtggcggcaaccaaagtgggtgcactgtctaaaggtcagttgaaagagttcctcgacgctaacctggcgtaagggaatttcatgttcgggtgccccgtcgctaaaaactggacgcccggcgtgagtcatgctaacttagtgttgacttcgtattaaacataccttattaagtttgaatcttgtaatttccaacgcttcccgttttatcttaaatgcgaagtgaacagatttctggctcgtcactcaatccgtcttgtcgtttcagttctgcgtactctcctgtgaccaggcagcgaaaagacatgagtcgatgaccgtaaacaggcatggatgatcctgccataccattcacaacattaagttcgagatttaccccaagtttaagaactcacaccactatgaatcttaccgaattaaagaatacgccggtttctgagctgatcactctcggcgaaaatatggggctggaaaacctggctcgtatgcgtaagcaggacattatttttgccatcctgaagcagcacgcaaagagtggcgaagatatctttggtgatggcgtactggagatattgcaggatggatttggtttcctccgttccgcagacagctcctacctcgccggtcctgatgacatctacgtttcccctagccaaatccgccgtttcaacctccgcactggtgataccatctctggtaagattcgcccgccgaaagaaggtgaacgctattttgcgctgctgaaagttaacgaagttaacttcgacaaacctgaaaacgcccgcaacaaaatcctctttgagaacttaaccccgctgcacgcaaactctcgtctgcgtatggaacgtggtaacggttctactgaagatttaactgctcgcgtactggatctggcatcacctatcggtcgtggtcagcgtggtctgattgtggcaccgccgaaagccggtaaaaccatgctgctgcagaacattgctcagagcattgcttacaaccacccggattgtgtgctgatggttctgctgatcgacgaacgtccggaagaagtaaccgagatgcagcgtctggtaaaaggtgaagttgttgcttctacctttgacgaacccgcatctcgccacgttcaggttgcggaaatggtgatcgagaaggccaaacgcctggttgagcacaagaaagacgttatcattctgctcgactccatcactcgtctggcgcgcgcttacaacaccgttgttccggcgtcaggtaaagtgttgaccggtggtgtggatgccaacgccctgcatcgtccgaaacgcttctttggtgcggcgcgtaacgtggaagagggcggcagcctgaccattatcgcgacggcgcttatcgataccggttctaaaatggacgaagttatctacgaagagtttaaaggtacaggcaacatggaactgcacctctctcgtaagatcgctgaaaaacgcgtcttcccggctatcgactacaaccgttctggtacccgtaaagaagagctgctcacgactcaggaagaactgcagaaaatgtggatcctgcgcaaaatcattcacccgatgggcgaaatcgatgcaatggaattcctcattaataaactggcaatgaccaagaccaatgacgatttcttcgaaatgatgaaacgctcataaatttgtcttatgccaaaaacgccacgtgtttacgtggcgttttgcttttatatctgtaatcttaatgccgcgctggcgatgttaggaaaattcctggaatttgctggcatgttatgcaatttgcatatcaaatggttaatttttgcacaggactggtgggtttggaacggactttcccttctgaataaaggtcttcgtggttatacttctgctaataattttctctgagagcatgcattgtgaatttactgacagtgagtactgatctcatcagtatttttttattcacgacactgtttctgttttttgcccgtaaggtggcaaaaaaagtcggtttagtggataaaccaaacttccgcaaacgtcaccagggattgatacctctcgttggggggatttcggtttacgcagggatttgcttcacgttcggaattgtcgattactatattccgcatgcatctctctatctcgcttgtgccggtgtgcttgttttcattggcgcgctggatgaccgttttgatatcagcgtaaaaatccgtgccaccatacaggccgctgttggcattgttatgatggtgttcggcaagctttatctcagtagcctgggttatatctttggctcctgggagatggtgctcggaccgtttggttacttcctgacgctatttgccgtctgggcggccattaatgcgttcaacatggttgatggcattgatggcttgctgggcgggttgtcctgcgtctcgtttgcagcaatcggtatgattttgtggttcgacgggcaaaccagcctcgcaatctggtgctttgcgatgatcgccgccatcctgccatacatcatgcttaaccttggtatcctgggtcgccgctacaaagtctttatgggtgatgcgggcagtacgctgattggttttaccgttatctggatcctgctcgaaacgacccagggcaaaacccatcccatcagcccggttaccgctttgtggataatcgccattccgctaatggatatggtggcgattatgtaccgtcgcctgcgtaaaggcatgagcccattctctcctgaccgtcagcatattcaccatttgatcatgcgtgccgggtttacttcccgtcaggcgtttgtgctgattacccttgccgcagcactgctcgcttccattggcgtgctggcagaatattctcattttgtcccggagtgggtcatgctggtgctctttttgctagcattcttcctctatggatattgcattaagcgtgcctggaaagttgctcgctttattaagcgcgtaaaacgcagactgcgtagaaatcgtggtggcagccccaatttaaccaaataaatgaggatgtgatgacacaaccaatgcctgggaaaccggccgaagacgctgaaaatgaactggatattcgtgggttgtttcgtaccttgtgggctgggaagctatggattattggcatggggctggcgtttgcgttaatcgcgctggcgtatacgttttttgctcgtcaggagtggagctcgacggcgattaccgatcgtccaacggtgaatatgctggggggatattactcgcagcagcaatttttgcgtaacctggatgtccgttcaaacatggcttctgccgaccaaccatcggtcatggacgaagcctataaagagtttgttatgcaactggcctcgtgggatacccgcagagagttctggctgcaaaccgactattacaaacagcggatggtgggcaacagcaaagccgatgcggcgttgctggatgaaatgattaacaacatccagtttatccccggagactttacccgcgcggtcaatgacagcgtgaagcttattgccgaaaccgcgcctgacgctaataacctgttacgtcagtatgttgcttttgccagccagcgtgcagccagccatctgaatgatgagctgaaaggcgcatgggcggcgcgtaccatccagatgaaagctcaggtgaagcgtcaggaagaggtggcgaaagccatctacgaccgccggatgaacagcattgagcaggcgctgaaaattgctgagcagcataatatttcgcgcagtgcgacagatgtacctgccgaggaattacctgattcagaaatgttcctgcttgggcgtccaatgcttcaggctcgactggaaaatttacaggccgtcggtccggcctttgatctcgactatgatcagaatcgggccatgttaaacaccctgaatgttggtccaaccctggatccgcgttttcagacctatcgctatttgcgtacgccggaagaaccggtaaaacgcgatagcccacgtcgtgccttcctgatgattatgtggggcattgtcggggggctgatcggggctggtgtcgcattaacccgccgttgctcgaaatagcaacactgctgcggtgagcgcaaaggcgctcgccgcttattcgaagagaatcgatgtgaaagtactgactgtatttggtacgcgcccggaagccatcaagatggcgccgttggtgcatgcgttggcaaaagatcctttttttgaggctaaagtttgcgtcactgcgcagcatcgggagatgctcgatcaggtgctgaaactcttttccattgtacctgactacgatctcaacataatgcagccaggacagggcctgacagagataacctgtcggattctggaagggctaaaacctattcttgccgagttcaaaccagacgtcgtgctggttcacggcgatacgacgacgacgctggcaaccagcctggcggcgttttatcagcgtattcctgttggtcacgttgaggctggtctgcgcacgggcgatctctattcgccgtggccggaagaggctaaccgtacattgaccgggcatctggcgatgtatcacttctctccaaccgaaacttcccggcaaaacttgctgcgtgaaaacgttgcggatagccgaatcttcattaccggtaatacagtcattgatgcactgttatgggtgcgtgaccaggtgatgagcagcgacaagctgcgttcagaactggcggcaaattacccgtttatcgaccccgataaaaagatgattctggtgaccggtcacaggcgtgagagtttcggtcgtggctttgaagaaatctgccacgcgctggcagacatcgccaccacgcaccaggacatccagattgtctatccggtgcatctcaacccgaacgtcagagaaccggtcaatcgcattctggggcatgtgaaaaatgtcattctgatcgatccccaggagtatttaccgtttgtctggctgatgaaccacgcctggctgattttgaccgactcaggcggcattcaggaagaagcgccttcgctggggaaacctgtgctggtgatgcgcgataccactgagcgtccggaagcggtgacggcgggtacggtgcgtctggtaggcacggataagcagcgaattgtcgaggaagtgacgcgtcttttaaaagacgaaaacgaatatcaagctatgagccgcgcccataacccgtatggtgatggtcaggcatgctctcgcattctggaagcgttaaaaaataatcggatatcactatgagttttgcgaccatttctgttatcggactgggttatatcgggctgccaacggcagcagcgtttgcctcacggcaaaaacaggtaattggtgtcgatatcaaccaacatgcggttgataccatcaatcgtggcgaaatccatatcgtcgaacctgatttggcgagtgtagtaaaaactgccgtagaaggcggttttttacgagcgagcacgacgccagttgaagcggatgcctggctgattgctgtacccacgccgtttaagggcgatcatgagccagatatgacctacgttgaatcggctgctcgctccattgcgccagtgctgaaaaaaggcgcgctggtgatccttgaatccacctcgccggtggggtcaaccgagaagatggcagaatggttagcagagatgcgtccggatctcactttcccgcagcaggtgggcgagcaggcggacgtcaacattgcttactgcccggaacgcgtgttaccaggacaggtaatggtcgagctgattaaaaacgatcgcgtgattggtggtatgacgccggtttgttcggcccgcgccagcgaactgtacaaaattttcctcgaaggtgagtgtgtcgtcactaactcgcggacggcggaaatgtgtaagctcaccgaaaacagcttccgcgatgtgaatatcgcttttgctaatgaattgtcgctgatttgtgccgatcaggggattaacgtctgggaactgattcgcctggcgaatcgtcaccctcgcgttaatattcttcagcctggccctggcgtgggcggtcactgcattgctgttgatccgtggtttatcgtggcacagaacccccagcaggcgcggcttatccgtaccgcgcgcgaagtgaacgatcacaaaccgttctgggttatcgatcaggtgaaagcggcggtggctgattgcctggcggctaccgataaacgcgccagtgaactgaaaatcgcctgctttggtctggcgtttaaaccgaatattgatgacctgcgcgaaagcccggcgatggaaatcgctgaactgatcgcccagtggcatagcggcgaaactctggttgttgagcctaacatccaccagttgccgaaaaaactgaccgggctttgtactctggcgcagcttgacgaggcgctggcaacggcagacgtgctggtgatgctggtcgatcatagtcagttcaaagttatcaatggcgacaatgtccatcagcagtatgtcgtcgatgccaaaggagtctggcgctgatgagaaaaattctgataacaggtggtgccgggtttattggctcggcgctggtgcgttatatcatcaacgaaacgagcgacgcggtggtagtggtcgataagctgacctacgccggaaacctgatgtcgctggcaccggtcgcgcaaagcgagcgctttgcctttgagaaagttgatatctgcgatcgggcagaactggcacgcgtattcactgagcatcagccagactgtgtcatgcatctggcagccgaaagccatgttgaccgttctattgacggcccggcagcgtttattgaaaccaacattgtcgggacttatacattgcttgaagcggcgcgggcttactggaatgcgctgacggaagataaaaaatcagcgttccgttttcatcatatctccactgacgaagtatatggtgacctgcactcgacggatgatttcttcaccgaaaccacgccgtatgcgccgagcagcccttattccgcgtcaaaagccagcagcgaccatctggtgcgcgcctggctgcggacctatggtctgccgacgcttatcaccaactgctcgaataactacggcccttaccactttccggaaaaactgatcccgctgatgatcctcaacgcgctggcgggtaaatcgctgccggtatatggcaacgggcagcaaatccgtgactggctgtatgtggaagatcacgcccgcgcgctgtattgcgtggcgaccaccgggaaagtcggtgaaacctataatattggtggtcacaacgagcgtaagaatctcgatgttgtggaaaccatttgcgagctgctggaagaactggctccgaacaagccgcacggcgtggcgcactatcgtgacctgatcacctttgtcgctgaccgtccggggcatgatctgcgttatgccattgatgcttcgaaaattgcccgtgaacttggctggctgccgcaggaaacctttgaaagtggaatgcgtaaaacggttcagtggtatctggctaatgaaagctggtggaagcaggtgcaggacggcagctatcagggcgagcgtttaggtctgaaaggctaattttcagcggaggcaaacatgaaaggtattatcctggcgggcggttccggcacccgattgcatccgattacgcgcggcgtatcgaagcaactgttgccgatttacgataagccaatgatttactatccgctgtcggtgctgatgctggccggtatccgcgaaattctcatcatcactacgccggaagataaaggttatttccagcgcctgctgggcgatggtagtgagttcggtatccagctggaatatgccgaacagcccagcccggacggtctggcgcaggcctttatcatcggtgaaaccttccttaatggtgaaccttcttgtctggtgctgggcgataacatcttcttcggtcagggcttcagtccgaagctgcgtcatgttgcggcgcgcaccgaaggggcgacggtttttggctatcaggtgatggacccggaacgctttggcgtggtggagtttgacgacaatttccgcgctatctcgctggaagaaaagccaaaacagccgaagtcaaactgggcggtgaccgggctttatttctacgacagtaaagtcgtggagtacgcaaagcaggtgaagccgtcggagcgtggtgaactggagattacctccatcaaccagatgtacctcgaggcgggcaacctgaccgttgaactgctcgggcgcggatttgcctggctggataccggcactcacgacagcctgattgaagccagcacctttgtacagacggtggaaaaacgccagggctttaagattgcctgcctggaagagattgcctggcgtaacggctggctcgatgacgagggtgtgaagcgtgctgccagttcattagcgaaaactggctacggccaatatctgctggagttacttcgtgcccgtccgcgccagtattgagccactaacctgggaaaacgccttctttggtgttaacagcgccatcgtgcgcattacgtctgaagcaccgctcctgacgccagacgcgttagcgccgtggtcacgggtgcaggccaaaattgcggcatcaaatacgggtgaactggatgccctgcaacagctgggattctccctggtagaaggtgaagttgatttggcgctacccgtgaacaatgccagtgatagcggtgctgtagtggcacaagagaccgatattcccgcattacgtcagttagccagcgccgcatttgcgcaaagccgttttcgtgcgccgtggtatgcgcctgacgccagcagtcgcttttatgcacagtggattgaaaatgccgtgcgcggcacctttgatcatcaatgtctgattttacgtgcggcgtccggcgatattcgcggctatgtctctttacgggaactcaatgcgacagatgcgcgaattggcctgctggctggacgcggtgcaggtgctgagctgatgcaaacggcgctaaactgggcgtatgctcgcggtaaaacaactttgcgggtggcgacccaaatgggcaacaccgccgcgcttaaacgatacatacaaagtggtgcgaatgtagaaagcaccgcgtactggttatacaggtgatcacatgattccatttaacgcaccgccggtggtgggaaccgaactcgactatatgcagtcggcaatgggtagcggcaaactgtgtggcgatggcggttttacccgtcgctgccagcagtggctggagcaacgttttggcagcgccaaagtgttactgacgccgtcctgcaccgcttcgctggagatggcggcgctgctgctcgatatccagcctggcgatgaagtgatcatgccgagctacacctttgtctccaccgccaatgcctttgtgctgcgtggcgcaaaaatcgtttttgtggatgttcgcccggacaccatgaacatcgacgaaacgctgattgaagcggcgatcaccgacaaaacgcgcgttatcgtgccggtccattacgcgggtgtggcctgcgaaatggacaccattatggcgttggcgaaaaagcataatttgtttgtggtagaagatgccgctcagggcgtgatgtccacttacaaagggcgtgcactgggaaccattggtcatattggctgctttagcttccatgaaaccaaaaactacacggcgggcggtgaaggcggcgcgacgctgattaacgataaagcgttaatcgaacgagccgagatcatccgtgaaaagggcactaaccgcagccagttcttccgtggtcaggtcgataaatatacctggcgcgatattggctccagctatttgatgtccgatctgcaagctgcatacctgtgggcgcaactggaagcagcggatcgtatcaaccagcaacgtctggcgctgtggcaaaactactacgatgcgttagcgcctctggcgaaagccgggcgtatcgagctgccgtcgattcccgatggctgcgtgcagaacgcgcatatgttctacattaaactgcgggatattgatgaccggagcgcgttgattaactttctgaaagaagcggaaatcatggcggtgtttcattacattccgctgcacggttgccctgcgggggaacactttggtgagttccacggtgaagatcgctacaccaccaaagagagcgagcgcctgctgcgcctgccgctgttctacaacctgtcgcccgtcaatcagcgtacggtaattgcgactttgttgaactacttttcctgatatgtcgttggcaaaagcgtccttgtggacggcggccagtacactggtcaagattggtgccgggttactggtcggtaagttgctggcggtgtcatttggtccggcggggcttgggctggcggcaaatttccgccagttgattaccgtgctcggcgtgcttgccggggctggcatctttaacggtgtaaccaaatacgttgcccagtaccatgataatccgcaacagctgcgccgcgtggtcggcacttcatcagcgatggtacttggtttctctacgctgatggcgctggtttttgtgctggcagctgcgccaatcagccagggattgtttggtaataccgactatcaggggctggtgcgtttagtggcgctggtgcaaatggggatcgcctggggcaacctgttactggcgctgatgaaaggctttcgcgatgccgcaggtaatgcgttatcgctgattgtcggcagcttgattggcgttctcgcgtactacgtcagttaccgtttgggcggttatgaaggggcgttgctgggtctggcgctgattcccgcgctggtggtaattcctgccgccatcatgttgatcaaacgtggtgtcatcccgttaagctatctgaaacccagctgggataacggtctggcagggcagttgagcaaatttacgctcatggcgttgattacgtcggtgaccttgcctgttgcttacatcatgatgcgtaaactgctggcggcgcagtatagctgggatgaggtggggatctggcaaggggtgagcagtatttccgatgcctacctgcaatttattacggcatcgttcagcgtatatttgctgcccacgttgtcgcggctaacggaaaagcgcgatatcacccgggaagtggttaaatcgctgaaattcgtcttaccggcagtggcggcggcgagttttaccgtctggctgctgcgtgattttgctatctggctgctgttgtcgaataaatttaccgctatgcgcgatctctttgcctggcagttagtgggtgatgtgttaaaagtgggcgcttatgtctttggttatctggtgatcgccaaagcgtcactgcggttttatattctggcggaagtcagccagttcactttattgatggtatttgcccactggctaatccctgcgcatggtgcactgggcgcggcgcaggcatatatggcaacttatatcgtctatttttctctttgttgtggcgtgtttttactctggcgtaggcgggcatgactgtactgattcacgtactgggatcggatatccctcaccataaccgaaccgttttgcggtttttcaatgacgcgctggccgcgacgagcgagcacgcgcgcgagtttatggttgttggcaaggacgacggcttaagtgatagctgtccggcgctttctgtgcaatttttccctgggaaaaaatcgctggcggaagcggtcatcgcgaaagcaaaagctaaccgtcagcagcgttttttcttccacggtcagttcaatcccacactgtggctggctctgctgagtggtggcattaagcccagccagtttttctggcatatctggggggcagacctgtatgagctttccagtggcttgagatataagcttttttacccactacgtcgcctggcgcaaaagcgagtcggctgtgtatttgccacccgcggcgatttgagcttttttgccaaaacgcacccaaaggtgcggggcgaactgctgttcttcccgacgcggatggacccttcgctcaatacgatggcgaacgatcggcaacgtgaagggaaaatgaccattctggtggggaactccggcgaccgcagcaatgagcatattgctgccttgcgcgccgttcatcagcaatttggcgatacggtaaaagtggtggtgccgatgggatatccgcctaataacgaagcgtacattgaggaagttcgtcaggcggggctggagttattcagcgaagaaaatctacaaattctgagcgaaaaactggaatttgacgcctatctggcgctacttcgtcagtgcgatcttggttactttatttttgcccgccagcagggcattggtacgctgtgcttactgattcaggcgggcattccttgtgtgcttaaccgggaaaatccgttctggcaggatatgacggaacaacatttgccggtgctgtttactaccgacgatctcaacgaggatattgtgcgtgaagcgcagcgccagttggcgtcggtggataaaaacaccattgccttctttagccctaactatctacaaggctggcagcgggcgttggcgattgccgccagggaggtcgcatgagtctgctgcaattcagtggcctgtttgttgtctggctgctctgcacgctgtttattgccacgctgacctggtttgagtttcgccgtgtgcgctttaacttcaatgtcttcttttcattgctgtttttgctcacctttttcttcggcttcccgctgaccagcgtgctggtatttcgctttgatgttggtgtcgcgccgccagaaatcttgttgcaggcgttgctttctgcgggctgcttctacgcggtttactatgtcacctacaaaacccgcctacgcaaacgcgttgctgatgtaccgcgccgtccgctgtttaccatgaaccgcgtggagaccaatcttacgtgggtgatcctgatgggtatcgcgctggtaagcgtcggcatcttcttcatgcacaacggctttttgctgttccggcttaactcctacagtcagatcttttccagtgaagtctccggcgtggcgttaaaacgcttcttttactttttcatcccggcgatgctggtggtctactttctgcgccaggacagcaaagcgtggctgtttttcctcgtcagcacggtcgcctttggcttgctgacttatatgattgtcggcggcactcgcgccaatatcatcatcgcattcgctatcttcctgtttattggcattattcgcggctggatttcgttgtggatgctggcggcggcgggcgtgctggggattgttggcatgttctggctggcactaaaacgctatggaatgaatgtgagcggcgatgaagcgttctatacgtttctctatctcactcgcgacaccttctcgccgtgggagaatctggcgttgctgttgcagaactacgacaacatcgacttccagggcctggctccaattgtccgcgatttctatgtctttatcccttcctggctgtggccgggtcgcccgagtatggtgctgaactcagccaactactttacctgggaagtgctgaataaccactccggactggcgatctcgcctacgcttataggctcactggtggtgatgggcggcgcgttgttcatcccgctcggggcgatcgtggttggtctgatcatcaaatggttcgactggctgtatgagctgggcaaccgcgagcctaatcgctataaagctgcgatattgcacagtttctgctttggggcgatcttcaatatgatcgtgctggcgcgtgaagggctggattcgtttgtctcacgcgtggtcttttttatcgtggtcttcggcgcatgtctgatgatcgcaaaactgttgtactggctttttgaaagcgccggactcattcataaacgtacaaaatcatcgctccggacgcaggttgaaggataacaatgaataacaacaccacggcaccaacctatacgctgcgtggcttacagttgattggttggcgtgatatgcagcacgccctcgattatctgtttgctgacgggcagcttaagcagggaacgctggttgccattaatgctgaaaaaatgctgactattgaagataacgccgaggtcagggagttaattaacgctgccgaatttaaatatgcggatggcatcagcgttgtacgttcagtacgtaaaaagtacccgcaggcgcaggtttcccgcgttgccggtgccgatctctgggaagagctgatggcgcgcgcaggcaaagaagggacgccggtatttcttgtgggcggtaaacctgaagtgctggcgcaaactgaagctaaactgcgcaaccagtggaatgtgaatatcgttggcagtcaggatggttattttaaacccgagcagcgtcaggcgctgtttgaacgcattcatgccagcggtgcgcaaatcgtcaccgttgcgatgggatcgccaaagcaggagatcatcatgcgcgactgccgtctggtacatccagatgcgctgtatatgggcgttggcgggacttacgatgttttcaccggtcacgtaaaacgcgcaccgaaaatctggcaaacgctggggctggagtggctctaccgcctgctttcgcagccgagccgcattaagcgtcagcttcgtttgctgcgttatttacgctggcactacaccggcaacctatgattttcctctctttgtaaagcgacggagtggtcactccgtcgcctgtctgcttttttattacacaaagcattcaaatttttaatgctttatttgccatttctcctgaattacgaaaacatttgcaacactcgatgtacccataacgataaccggtaacaccggaaagcatgcaaacacaacacgaggatttatggcagataacaaaccagagctacagcgtgggctggaagctcgacatatcgaactcatcgccctggggggcaccattggcgtcggcctgtttatgggggccgccagtaccctgaaatgggccgggccatccgtattgttggcctatatcatcgccgggctgttcgtctttttcatcatgcgttcaatgggcgaaatgttgttcctcgaaccggttaccggttcgttcgccgtttatgcgcatcgttatatgagcccgttctttggctatctcaccgcctggtcttactggtttatgtggatggcggtggggatctctgaaatcaccgccattggcgtttatgtccagttctggttcccggagatggcgcagtggatacccgcattgatcgcagtggcgctggtggcgttggcgaatctggcggcggtgcggttgtacggcgaaatcgagttctggttcgcgatgatcaaagtcaccacgattatcgtgatgattgtcattggcctgggcgtgattttctttggctttggcaatggcgggcagtcgattggttttagcaatctcacagagcatggcggtttctttgcgggtggctggaaagggttcctgaccgctctgtgtattgtggtggcgtcctaccagggcgtggagctgattggcattactgccggtgaagcgaagaatccgcaggtgacgctgcgcagtgccgtaggcaaggtgctgtggcggatcctgattttctacgtaggcgcgattttcgttatcgtcaccatcttcccgtggaatgaaataggcagcaacggcagcccgttcgtactgacttttgccaaaatcggtattaccgcagcggcgggcattatcaactttgtggtgctgacggctgcgctctctggctgtaacagcggcatgtacagttgcggacgtatgctctacgcactggcgaaaaaccgtcagttaccggcggcaatggcgaaagtttcccgtcacggcgtaccggttgcgggtgtggcagtatctattgctattctgctaattggctcatgcctgaactacatcattcccaatccgcagcgtgtgtttgtctacgtctacagtgccagcgtgcttccggggatggtgccatggtttgtgatattgataagccagctgcgttttcggcgtgcacataaagcggcgattgccagccatccgttccgctcaatcctgttcccgtgggccaattacgtaacaatggcattcctgatttgcgttttgatcggcatgtactttaatgaagatacgcgtatgtcgctgtttgttggcatcatctttatgctggcggtgacggcgatttataaagtttttggccttaatcgccacgggaaagcgcataaactggaggaataagcagcaaaacgcacaaaccgtaaccaaacgcgcaatttatttaaaaagggactagacagaggggtgggaagtccgtattatccacccccgcaacggcgctaagcgcccgtagctcagctggatagagcgctgccctccggaggcagaggtctcaggttcgaatcctgtcgggcgcgccatttagtcccggcgcttgagctgcggtggtagtaataccgcgtaacaagatttgtagtggtggctatagctcagttggtagagccctggattgtgattccagttgtcgtgggttcgaatcccattagccaccccattattagaagttgtgacaatgcgaaggtggcggaattggtagacgcgctagcttcaggtgttagtgtccttacggacgtgggggttcaagtcccccccctcgcaccacgactttaaagaattgaactaaaaattcaaaaagcagtatttcggcgagtagcgcagcttggtagcgcaactggtttgggaccagtgggtcggaggttcgaatcctctctcgccgaccaattttgaaccccgcttcggcggggttttttgttttctgtgcatttcgtcaccctcccttcgcaataaacgcccgtaataactcattgccccacggtatgatttcgcccttaacgtattgaaggatgacttcaggcaaggagcgaccatgctgcaacaggttccaacgcgtgcttttcatgtgatggcgaaaccgagcggttccgattgtaatctgaactgtgactactgtttttatctcgaaaaacaatccctttaccgcgaaaagccagtcacgcatatggacgatgacacgctggaagcgtatgtccgtcactatatcgctgccagcgaaccgcaaaacgaagtggcttttacctggcagggcggcgaaccaacgctactcgggctggcgttttaccgccgtgccgtagcgctacaggcgaaatatggtgctggcaggaagataagtaacagcttccagactaacggcgtgctgctggatgacgaatggtgcgcgtttctcgcggagcatcattttcttgttggtttatcgctggatggcccgcctgagatccacaatcaatatcgcgtgactaaaggtggcagacccacgcataagctggtgatgcgtgccctgacgctcctgcaaaaacatcatgtcgactataacgtgctggtctgcgttaatcgcaccagcgcgcagcaaccgttgcaggtatatgattttttgtgcgatgcgggagtcgaattcatccagtttattccggtggtcgagcgcctggctgatgaaacaactgcccgcgatggacttaagttacatgcgcctggtgatattcagggtgagctaacggaatggtcggtgcgccccgaggagttcggtgagtttctggtggcgatattcgaccactggatcaaacgcgacgtcggcaagattttcgtgatgaatatcgaatgggcgtttgccaattttgtcggtgcgccgggtgcggtttgccatcatcagccaacctgtgggcgctcggtgattgttgagcacaacggcgacgtttacgcctgtgatcactatgtttatccgcaatatcggctggggaatatgcaccagcaaacaattgcagaaatgatcgattccccgcaacagcaggcgtttggtgaagataaatttaagcagttaccggcgcagtgtcgcagttgtaacgtgttaaaagcgtgctggggaggctgcccgaaacaccgcttcatgctcgatgccagcggcaaaccgggactgaattatttgtgtgccgggtatcagcgttatttccgccatctaccgccatatcttaaagcaatggctgatttgctggcgcacggtcgcccggccagcgacattatgcatgcgcatttgctggtggtgagtaagtagaaatcggcggccgcctgcggttgattgccggatgcggcgtaaacgccttatccggcctacatgatcgtgcaaattcaataaattgcagcgttctgtaggctggataagatgcgtcagcatcgcatccggcaaaggcagatctcagcgatagcgccggcttagtcagatttaatctgcgcgcgtggtggatattttttcaggatctccatatacgcgtgcatttcggtctgtagcggtacacccatcggaatatggcgcacgccgatggagtcgctttcctgcggatcggtgtagaggttaaacaccgacgatcccgccgtttgcattactgtgccggtgaatccaccctgatatccgctctgggtataagcgtaaggttgctgaatcaggacgtgatacttgaactcatccatacgcacagcagcgagtttaccgttgaggaagtagtgctcggccttacggttagactgaccatttgttcccaggaagaaggatgtctggtccacaccatcgataaaggtggttttcggcactaaattcgccactttcgctccaggatgccctgccagatccagcgcggtagggaagagatctgccagatcgacaataccgtcagatttacgcggttggatcatccctttccagtaaacgaaagtcggtacgcgaacgccgccttcccaggtcgaacctttcgcaccacggaacggggtgcgtccgtgcggcggtacttcggcttccggtccgttatcggaggtaaagacgatcagcgtgttatcaagctgaccgtttttctccagtgttttatacagattagcgaacacatcgttcatctccaccatgcagtcgccatacgaggtgcgtgccggagagctacccgcatatttcgcatttgggtagttatcgaagtggcagccacgagtgccgtagtagaggaagaatggtttatcgctcttcgccatcttgtcgaggaacttaacgccatagtccatccagcgttgatccagatcttccatatatttcggcgtaatgtcggcaatggcctgttgttcgccgccgcgcaccgcatgaacgtcatctttgctgaacggtaattgcttgatgtattcagaacggtccggactcagggccacttccggattgacgtgaacgtcgcgccattcggtgtacatatcagacaccgagttaaagccacggaaatcatcaaagccaacgttctgcggctgcgactctttgttttcccccatatgccattttccgatggcctgagtgacgtagccctgatcgtgcagcaactgcggcagcgtggttaacccttgcagcccgcccggttgcccgtacattggcggcatcagaatgccgtggtggatggagtattgtccggtgagaatggtggcgcgggttggggaagagcttggttgagaatacgccgaagttaaaatcagcccctggctggcaacggcgtcgatatctggtgtagggttacccaccgccacgccgccaccgttaaaaccgacgtccatccagcccacatcgtccagcaagaaaacaaccacattcggtttcttaccggtttttttctcaagttctgccagcttctgctgggtttctttatcctgcgccggatgctgcattactggcatcatattgtcggcaatagtggtcgccggtttaaccagatactggtttgggtgatcgtatccggcaaagcctttgcgtgcggtggcagttgacggggtatctgctgcgctggccatgagaggaagagcggcggcgacagcaacaacaagacgtttgggtgaaaacgaaaattccatgcaaaatgctccggtttcatgtcatcaaaatgatgacgtaattaagcattgataattgagatccctctccctgacaggatgattacataaataatagtgacaaaaataaattatttatttatccagaaaatgaattggaaaatcaggagagcgttttcaatcctacctctggcgcagttgatatgtaaggcaggtttattatatcgcgttgattattgatgctgtttttagttttaacggcaattaatatatgtgttattaattgaatgaattttatcattcataataagtatgtgtaggatcaagctcaggttaaatattcactcaggaagttattactcaggaagcaaagaggattacagaattatctcataacaagtgttaagggatgttatttcccgattctctgtggcataataaacgagtagatgctcattccatctcttatgttcgccttagtgcctcataaactccggaatgacgcagagccgtttacggtgcttatcgtccactgacagatgtcgcttatgcctcatcagacaccatggacacaacgttgagtgaagcacccacttgttgtcatacagacctgttttaacgcctgctccgtaataagagcaggcgtttttttatgtatcaggaaggccccggaggtgcttgcctccgggtgagaaggaactactgtggcgggttattctgcaacgttaacatcaaaccgtcgcgacgcatagctgcagcttcttccggcttgtgcagtctgtccagcgcgtcggcaagccatgcgtaatcgtaggcgtccggacgttgtttcagcgctgcgcggaaggcgagcgatgcttcctgccattctccgtgcttcatcagtgactggcccagtgtgctccacaacagcgggcgatcgccgacgtttttgatttgctggcgcagcactttttccagctgttccggattgtttgttttcagtcgaggaatcggcagcagtaggcgatcgtcgtactggcgtttcaggccatcgatgataatttgctgggcagtatcatgatcgtcacattcaataagatgttccgccattgccacctgcaacgctacctgatgacgcgttttccggctttggtttttccaccagttacgcaaaccttcgctaccgttatcggcacgcgcctgatccatcaggccaatccatgcctgttgttccagcattgcacgatgttcttcatcaccaacatgggctttcgccattgatgggataatatccagcagcgaactccatgcacctgtgcggatatacgcctgttccgccagacgtaatacttccggatggcgtggcgtaacttccagcagcttatccacgccgtggcgtgcagcatggttttcattacgggccagttgcagacgtacgcgggtgatttctaccggaatggtgtcgttgccggccagctccgctgcgcgttccagatgttggttggcgcgtgcttcatcaccacgttgttgcgcggcttcggcagccagtagatagttcaccaccggttgttccgcgtgatcggcatttttcgccatcagcttttcaacttgctgataatcgccttccgccagtttcagcagcgcctgttcggtctgcttacgtgcacggcgacgcttacgtccgacaaaccacccacgggtgtgcgcgccagtgcggaagatccgccgcagtagccactcaatggcaaacagcactaccatcgccagaatcaatatgatcgccaggcccgtgacgctggtttcgatattgtagttgtcggtctggatcagcacataaccctgatggccggcaatcatcgggccaaccacgatccccgcaatcagcaacacaaagagcaataacacttttagcatggttattctccttgcggcgcggctgccggagtatcagcttgcggtgcaggtgcaggtttagcttccgttgtccccgctgccggttgtgccagcaggttacgcacgcgagtctgcatcagtttttccagcatcgcctggctttgcagggtttccggaagatccatcgagatattttgctggcttaactggtccacctcgtcgaggaacgctttggtggtggcatcatcagtatcgtagtaagcacgtacccaggtggagacgttctccagcgcctggcgataagtctcttcctggtgacgcggtacagcttgtgctgcgaccagcaggcgagagcgaatattttcgcgcagatagatatcctgatttggcgctaacagcggtacggcggtgtcatcacgacggcgaatcgtaatgaagttgtccataaagttctgccagcttttttgcagattgatacgccattcgctgatggaactggaaagctcttcaccgtctgaatccatcggcgaaccatcgctgtcattatcggccagacgcaggttatctacctgatttgaaagctgattaagcttaaggatgatgccgtcataatccacctgcgatactgcagaaaggctggcgatatcatcggtaattgcccgacgaacggtaatcagactcgggtcattcatatccgccaggctggcgtctgcacttttcagcaacgctgcagcggtcgtgacgtcctgatcgctccacagcttccgtccggcgagtttcaccagaaaatcggcctgagccagcagccaggttttagcatcgctgccggaaatggtggcgaccttttgttggacttcatccaactgttttgccagcgtttcttgctgacgattcgcctgcttaagttgtgcagcttgttgcttaataatgccttccagctcggctttttggctctcctgggctttttgcaatgccgtcagttggttagccagggcatcgctggtggcggtctgattgacggcctgttgtttaccccagccatacaaaccgatgcccgccgccagagcaatagcgatagccaccgcgctgagaatcaatgcggtattgttcttactctttttttctgttgcgacaggttgtgacgtggtgtccacggcctccctggtctcttcaaccacggcggaggttttttcttgttccgtcattatggcttcctgttatgagagttattgtaatgcccgtaaaagcgcatcgttgtcagcgttatcggcgaccttaatgtcttgccagcccagttcccgggcgagtttcgccaaacgctcactgacgaccaatagtcgacagtgtagtaaccagtgctcacgataccattgtgggatcagcgaccagagttgctgcaacatttcaccgctggtaacaacgaccatcgtcacctcgcgggcttgccagcgcatcgcttcttctgcaccatcgtaatggattgcgcatcgttgataacattcacaaaaagtgacctcagcaccgcgcgccgtcagggtatccccaattagctcacgaccaccattgccacgtaatatcagcgcacgtttgcccgcaatattttgtaattcaggtaattgtagcaagacttcgctgatttcccgatcctgcgggtagagaatcttctgtccacttacggtatgtagtgccagtgcggtggtgcgtccaatggcgaaataatcaggtagtcggggccatttacgatcttgctgatgcagctgtgattgggcaaaagcaaccgcgtgttgcgagagggcaaacaacagatcgctctcccccagcgctgccagttgatcagcaagttgcggtaattgttgacccggagaaaactcaatcagcggaaaatgccaggccacctgccccagtgtgcgcagacggctcactaactcttctccagcgggagacgggcgggtgacaaggatactcatgccggggcgtctccgttatagacttcagcgaggatctcgcgcgcgccgttattcagtagctcttctgccagcgaaatccccatttgttcggcatcttgcggcgcaccgcggcgttcaccgcgaataatctgcgaaccgtccggcgcgccgaccagcgcacgcagccagatttcgccatcaataagctcggcgtagctaccaattggcacctgacatccgccttcgagacgggtattcatggcgcgttctgcggtaacgcgcagtgcagtttcgtggtgattcagcgcggcaagcagctcgcgagtgcgtgaatcatcaaggcggcattcaatacccaccgcaccttgtcctaccgccggaagagaaatctcgggtggcaacgcggcgcgaatacgtgactccagacctaaacgttttagtccggctacggcaagaatgatggcatcgtattcgccgttatccagtttgctcaggcgagtgccgacgttgccgcgcagggagcggataatcagatccggacggcgttcagccagttggcactggcgacgtaaactggacgtcccgacgatactgcctgccggtaacgcatccagactgtcatagttattggacacaaaggcatcgcgaggatcttcacgctcacaaatagtgaccagtcccagaccttgcgggaattcaaccggcacatctttcattgagtgtacggcgatatcggcgcgattttcgaggagcgcgacttccagctcttttacaaataagccttttccgcctactttcgccagcggcgtatcaagaatcacatcgccgcgcgtcaccatcggtaccagttcaacgaccaggcccggatggctcgccatcaacttgtctttgacatagtgtgcctgccagagtgcaagtgggctttggcgtgtggcaattcttaaaacattgtctaacatgcttgttaccgtcattatcatccgtggtccatcctaacatccttgccagagtgatgtcagtgttgtggtgaaacgtagacgcctgcgcaaaccgtaaaatgaggtctggcagtggatcctgacaggcgtttcacgccgttgtaataaggaatttacagagaataaacggtgctacacttgtatgtagcgcatctttctttacggtcaatcagcaaggtgttaaattgatcacgttttagaccattttttcgtcgtgaaactaaaaaaaccaggcgcgaaaagtggtaacggttacctttgacatacgaaatatcccgaatgccgcgtgttaccgttgatgttggcggaatcacagtcatgacgggtagcaaatcaggcgatacgtcttgtacctctatattgagactctgaaacagagactggatgccataaatcaattgcgtgtggatcgcgcgcttgctgctatggggcctgcattccaacaggtctacagtctactgccgacattgttgcactatcaccatccgctaatgccgggttaccttgatggtaacgttcccaaaggcatttgcctttacacgcctgatgaaactcaacgccactacctgaacgagcttgaactgtatcgtggaatgtcagtacaggatccgccgaaaggtgagcttccaattactggtgtatacaccatgggcagcacctcgtccgtagggcaaagttgttcctctgacctggatatctgggtctgtcatcaatcctggctcgatagcgaagagcgccaattgctacaacgtaaatgtagcctgctggaaaactgggccgcctcgctgggtgtggaagtcagcttcttcctgattgatgaaaaccgcttccgtcataatgaaagcggcagcctggggggcgaagattgtggctccacccagcatatactgctgcttgacgaattttatcgtaccgccgtgcgtctcgccggtaagcgtattctgtggaatatggtgccgtgcgacgaagaagagcattacgacgactatgtgatgacgctttacgcgcagggcgtgctgacgccaaatgaatggctggatctcggtggcttaagctcgctttctgctgaagagtactttggtgccagcctttggcagctctacaagagtatcgattccccatacaaagcggtactgaaaacactgctgctggaagcctattcctgggaatacccgaacccacgtctgctggcgaaagatatcaaacagcgtttgcacgacggcgagattgtatcgtttggtctcgatccatactgcatgatgctggagcgtgttactgaatacctgacggcgattgaagattttacccgtctggatttagtacgtcgctgcttctatttaaaagtgtgcgaaaagctcagccgtgaacgcgcctgcgtaggctggcgtcgcgcagtgttgagccagttagtgagcgagtggggttgggacgaagctcgtctggcaatgctcgataaccgcgctaactggaagattgatcaggtgcgtgaggcgcacaacgagttgctcgacgcgatgatgcagagctaccgtaatctgatccgctttgcgcgtcgcaataaccttagcgtctccgccagtccgcaggatatcggcgtgctgacgcgtaagctgtatgccgcgtttgaagcattaccaggtaaagtgacgctggtaaacccgcagatttcacccgatctctcggaaccgaatctgacctttatttatgtgccgccgggccgggctaaccgttcaggttggtatctgtataaccgcgcgccaaatattgagtcgatcatcagccatcagccgctggaatataaccgttacctgaataaactggtggcgtgggcatggtttaacggcctgctgacctcgcgcacccgtttgtatattaaaggtaacggcattgtcgatttgcctaagttgcaggagatggtcgccgacgtgtcgcaccatttcccgctgcgcttacctgcaccgacaccgaaggcgctctacagcccgtgtgagatccgccatctggcgattatcgttaacctggaatatgacccgacagcggcgttccgcaatcaggtggtgcatttcgatttccgtaagctggatgtcttcagctttggcgagaatcaaaattgcctggtaggtagcgttgacctgctgtaccgcaactcgtggaacgaagtgcgtacgctgcacttcaacggcgagcaatcgatgatcgaagccctgaaaactattctcggcaaaatgcatcaggacgccgcaccgccagatagcgtggaagtcttctgttatagccagcatctgcgcggcttaattcgtactcgcgtgcagcaactggtttctgagtgtattgaattgcgtctttccagcacccgccaggaaaccgggcgtttcaaggcgctgcgcgtttctggtcaaacctgggggttgttcttcgaacgcctgaatgtatcggtacagaaactggaaaacgccatcgagttttatggcgcgatttcgcataacaaactgcacggcctgtcagtgcaggttgaaaccaatcacgtcaaattaccggcggtggtggacggctttgccagcgaagggatcatccagttctttttcgaagaaacgcaagacgagaatggctttaatatctacattctcgacgaaagcaaccgggttgaggtatatcaccactgcgaaggcagcaaagaggagctggtacgtgacgtcagtcgcttctactcgtcatcgcatgaccgttttacctacggctcaagcttcatcaacttcaacctgccgcagttctatcagattgtgaaggttgatggtcgtgaacaggtgattccgttccgcacaaaatctatcggtaacatgccgcctgccaatcaggatcacgatacgccgctattacagcaatatttttcgtgatgaacgtgccggaaagcgaggcttatccggcatgcaatcttagcggaaactgactgtttcacccgcctgctgcgtcgccgcctgttccagcaaatcccagaaggtttcgccgctgcgatcacaaatccactcatcgcctttcaggtcaaaatggtagccgccctgtttggttgccagccatacctggtgcagcggctcctggcggttgataatgattttgctgccattctcaaaggtaatggtcagtacgccgccgttgatttcgcagtcgatatcgctgtcgccatcccagtcgtccaggcgttcttcaatggtcagccagagttgatcagccaggcgatgaaattcactgtcgttcattgttgtatcctgtttttaagtgatggcggcagtatagcggcatggggtcagggcttcaaagtttgcacctctgcggctgcgttccggcacgattcatccgtcaccggaataatgatgtctctgtgtagcgaaagatttgtctcttcattagggcgcagttacaccacgtctttccctgtttctggtaaacattatgatcaggtttaccgagcgagcatcctcacgctgacggaactaaaaaagacaacaaacaaaccacattgcgatagtgcataaagccatcctggcgcgaggtgccgatcacgaaactaccagcaaaacataaatccccacgagtaagcgttatactcgcagcatttcctcacttttcagacttcataaagagtcgctaaacgcttgcttttacgtcttctcctgcgatgatagaaagcagaaagcgatgaactttacaggcaatccataatgaaaaacgtgtttaaggcactcactgtattacttactctcttcagcctgacgggctgcggtctgaaaggtccgctctatttcccgcctgcagataaaaacgcaccgccgccgaccaaaccggtagagacgcaaacgcaatccacggtgccggataaaaacgatcgcgccactggcgatggtccatcccaggtgaattactaaaagtcagtttctgtacccgcgtgattggagtaaatgatgcagttctcgaaaatgcatggccttggcaacgattttatggtcgtcgacgcggtaacgcagaatgtctttttttcaccggagctgattcgtcgcctggctgatcggcacctgggggtagggtttgaccaactgctggtggttgagccgccgtatgatcctgaactggattttcactatcgcattttcaatgctgatggcagtgaagtggcgcagtgcggcaacggtgcgcgctgctttgcccgttttgtgcgtctgaaaggactgaccaataagcgtgatatccgcgtcagcaccgccaacgggcggatggttctgaccgtcaccgatgatgatctggtccgcgtaaatatgggcgaacccaacttcgaaccttccgccgtgccgtttcgcgctaacaaagcggaaaagacctatattatgcgcgccgccgagcagacaatcttatgcggcgtggtgtcgatgggaaatccgcattgcgtgattcaggtcgatgatgtcgataccgcggcggtagaaacgcttggtcctgttctggaaagccacgagcgttttccggagcgcgccaatatcggttttatgcaagtggttaagcgcgagcatattcgtttacgcgtttatgagcgtggggcaggagaaacccaggcctgcggcagcggcgcgtgtgcggcggttgcagtagggattcagcaaggtttgctggccgaagaagtacgcgtggaactccccggcggtcgtcttgatatcgcctggaaaggtccgggtcacccgttatatatgactggcccggcggtacatgtctacgacggatttattcatctatgaagcaaccaggggaagaactgcaggaaacactcacggagcttgatgaccgggcggttgtcgattatctgattaaaaatcctgagttttttatccgtaatgcgcgcgcagtagaagcgatacgtgtgccgcatccggtacgcggcaccgtttcgttggtcgagtggcacatggcccgcgcacgtaatcatattcatgttctggaagagaacatggcgctgttgatggaacaggctatcgccaacgaaggcctgttttatcgcctactctacctgcagcgcagtctcaccgccgccagcagtctcgacgatatgctgatgcgctttcaccgctgggcgcgcgatctcggcctggcaggtgcgagtctgcgcctgtttccggatcgctggcgcttaggtgcgccgtcgaaccacactcatctggcattaagccgtcagtctttcgaaccgctgcgtattcagcgtttggggcaggaacagcactatcttgggccgcttaacggaccagagctgctggtggtgctaccggaagcgaaagcggtgggatcggtggcgatgtcgatgctgggaagcgatgctgatttgggtgtcgtgctgtttaccagtcgcgatgccagtcactatcaacaagggcaaggaacgcagttacttcatgaaattgcgctgatgttgccggagcttctggagcgttggattgaacgcgtatgaccgatttacacaccgatgtagaacgctacctacgttatctgagcgtggagcgccagcttagcccgataaccctgcttaactaccagcgtcagcttgaggcgatcatcaattttgccagcgaaaacggcctgcaaagctggcagcaatgtgatgtgacgatggtgcgcaattttgctgtacgcagtcgccgtaaagggctgggagcagcaagtctggcgttacggctttctgcgctacgtagcttttttgactggctggtcagccagaacgaactcaaagctaacccggcgaaaggtgtttcggcaccgaaagcgccgcgtcatctgccgaaaaacatcgacgtcgacgatatgaatcggctgctggatattgatatcaatgatcccctcgctgtacgcgaccgtgcaatgctggaagtgatgtacggcgcgggtctgcgtctttctgagctggtggggctggatattaaacacctcgacctggagtctggtgaagtgtgggttatggggaaaggcagcaaagagcgccgcctgccgattggtcgcaacgctgtggcgtggattgagcactggcttgatttgcgcgacctgtttggtagcgaagacgacgcgctttttctgtcgaaactgggcaagcgtatctccgcgcgtaatgtgcagaaacgctttgccgaatggggcataaaacaagggctgaataatcacgttcatccgcataaattacgtcactcgttcgccacgcatatgctggagtcgagcggcgatcttcgtggtgtgcaggagctgctgggtcatgccaacctctccaccacgcaaatctatactcatcttgattttcaacaccttgcctcggtgtacgatgcggcgcatccacgcgccaaacgggggaaataatgcgtttttaccggcctttggggcgcatctcggcgctcacctttgacctggatgataccctttacgataaccgtccggtgattttgcgcaccgagcgagaggcgcttacctttgtgcaaaattatcatccggcgctgcgcagcttccagaatgaagatctgcaacgcctgcgccaggcggtacgggaagcggaacccgagatttatcacgacgtgacgcgctggcgttttcgttcgattgaacaagcgatgctcgacgccgggctgagtgccgaagaagccagtgcaggcgcacacgcagcaatgatcaactttgccaaatggcgcagccgaatcgacgtcccgcagcaaactcacgacaccttaaaacagctggcgaagaaatggccgctggtggcgatcaccaacggtaacgcccagccggagctgtttggtttgggggattattttgagtttgtgctgcgcgctggcccgcacgggcgctcaaaaccgttcagcgatatgtactttttggctgcggaaaaactcaacgtgccgatcggcgagatcttacatgttggggacgatctcaccactgacgtgggtggggcaattcgcagcggaatgcaggcttgttggatcagaccggaaaatggcgatctgatgcaaacctgggacagccgtttactgccgcatctggaaatttcccggttggcatctctgacctcgctgatataatcagcaaatctgtatatatacccagctttttggcggagggcgttgcgcttctccgcccaacctatttttacgcggcggtgccaatggacgtttcttacctgctcgacagccttaatgacaaacagcgcgaagcggtggccgcgccacgcagcaaccttctggtgctggcgggcgcgggcagtggtaagacgcgcgtactggtgcatcgtatcgcctggttgatgagcgtggaaaactgctcgccatactcgattatggcggtgacgtttaccaacaaagcggcggcggagatgcgtcatcgtatcgggcaactgatgggcacgagccagggcggtatgtgggtcggcaccttccacgggctggcgcaccgtttgctgcgtgcgcaccatatggacgccaatctgccgcaggatttccagatcctcgacagtgaagaccagctacgcctgcttaagcgtctgatcaaagccatgaacctcgacgagaagcagtggccgccgcggcaggcaatgtggtacatcaacagccagaaagatgaaggcctgcgtccgcatcatattcaaagctacggtaatccggtggagcagacctggcagaaggtgtatcaggcgtatcaggaagcgtgtgaccgcgcgggcctggtggacttcgccgagctgctgctgcgcgctcacgagttgtggcttaacaagccgcatatcctgcaacactaccgcgaacgttttaccaatatcctggtggacgaattccaggataccaacaacattcagtacgcgtggatccgcctgctggcgggcgacaccggcaaagtgatgatcgtcggtgatgacgaccagtcaatctacggctggcgcggggcgcaggtggagaatattcagcgtttccttaatgatttccccggtgccgaaactattcgtctggagcaaaactaccgctctaccagcaatattctgagcgccgctaacgccctgattgaaaacaataacgggcgtctgggtaaaaaactgtggaccgatggcgcggacggtgagcctatttccctctattgcgcttttaacgaactcgatgaagcgcgttttgtggttaaccgcatcaaaacctggcaggacaacggcggagcgcttgccgagtgcgccattctctaccgcagcaacgcccagtcgcgggtgctcgaagaggcgttattgcaggccagtatgccgtaccgtatttacggcgggatgcgcttcttcgaacgccaggaaatcaaagatgcgctctcgtatctgcgcctgattgccaaccgcaacgacgacgcggcctttgagcgtgtggtgaatacgccaacgcggggtattggtgaccggacgctggacgtggtacgtcagacatcgcgcgatcgccagttaacactctggcaggcatgtcgtgagctgttgcaggaaaaagccctcgccgggcgagctgccagcgccttgcagcgatttatggaattaatcgacgccttagcgcaggaaactgccgatatgccgctgcatgtacagactgaccgggtaattaaagactccggcctgcgtaccatgtatgagcaggagaagggcgaaaaaggtcagacgcgtatcgaaaacttagaggaactggtgacggcaacgcgccagttcagctacaacgaagaagacgaagatttaatgccgctgcaggcgttcctctcccatgcggcactggaagcaggtgaagggcaggcggatacctggcaggatgcggtgcagttgatgacgctacactcggcgaaaggcctggagttcccgcaggtgtttatcgttggtatggaagagggcatgttcccaagccagatgtcgctggatgaaggcgggcgtctggaagaagaacgccgtctggcctacgttggcgtaacccgcgcgatgcagaaactgacgctgacctacgcggaaacccgccgtctgtatggtaaagaggtttaccatcgcccgtcgcgctttatcggcgagctgccggaagagtgtgtggaagaggtgcgcctgcgcgccacggtaagccgcccggtcagccatcagcggatgggtacgccgatggtcgagaacgacagcggctacaagctcggccagcgcgtacgccacgctaagtttggtgaaggcaccattgtcaatatggaaggcagcggtgagcatagccgtttgcaggtggcatttcagggccagggtattaaatggctggtggcggcatacgcccggctggagtcggtgtaacgttgccggatgcggtgctgcgcaccttatttggcctaaaaaatcattcagattcaataaattgcaacgtcatgtaggccggatagggcgtttacgccgcatccggcatctgcgccatcttcagtatctgacacaaaactatcgttttaacctttccgctcgacggaaatcatggtgacaaaaggatagcgttgccacgggattgccccgcctttcatatacatatgtgaaatcgtgccatcaagataaagcagctgctcaacgttcagtttcgctttggcataacaggcaaaatcataaaaatttgttgcctgctggctcaacaaaaacacggcgttcccatgtttattaatcccaacaccgttacgaattttgcttgaggcgacgttgggatgaatacgcggattaattacaccgttttccatcaacattggccctgactgcaccgcaaactgaatctctttactggttttgaaggcatccagacgaacgatgccgactttatctcccgcgacataaaacacgccgccaggacggataaagaaattcccttcacctgaagcgagatttaacgccaccttctgctgaccgttttcgatgtacaaaccgagcggcgcatagctttcatcatagatgccgccgttcatcgccatctgcacctgaccctgactattaatatccgccagcagagcatgtaacgttccccacgcttcgccattggctttttgccagtacattttcacccgctctgtttgaggattaacggtatacgcctgtacggtcagcgtcggatctgagagtgcgcaatcatcagcggcaacagcaaacaagggaagtaaggtgagggcgagaaaaatccgtttgagattcaaggtgatcattcctttaccaatgagtagctgatgcgccattataggtcctggatgtgggatttttttatcctgttagcgaccttgacgagtaccaaaaagcgcgaagttcaactattgttctgtggtgttctgttgcgtgttgacggcaaaattttgctggcgtaacatgcgcgcacgatcactctaagaggacattcgccttggacacacccagtagatactggctcactatcctgtcatccaggatcaactcctaaggctatccctttttgctgatagccttagcggttgtcagcgacctcaatttttcccgtcgcgctgagtcaggctgtttaatggtctgaaacccaatttgtttctgtgtgcccaccgaactgtccgatattttaagcattgggagtcccggtcatgctgagcgcatttcaactggaaaataaccgactgacccggctggaagtcgaagagtcacaaccccttgtaaatgcagtatggattgatcttgtcgaaccggacgacgacgagcgactgcgcgtacaatctgaacttggccagagcctggcaacccgcccggaactggaagacatcgaagcatcggcacgtttctttgaagacgacgacggcctgcatattcactccttcttcttctttgaagatgcggaagatcacgccggtaactccactgtggcatttaccatccgtgatggtcgtctgtttactctgcgtgagcgtgaactgcccgcttttcgtctgtatcgtatgcgtgcccgtagccagtcgatggtagacggtaacgcctacgagttgctgctggatctgttcgaaaccaaaatcgaacagttggcagatgaaattgaaaatatctatagcgacctggagcagttgagccgggtgattatggaagggcatcagggcgatgagtacgacgaggcgctctccactctggcggaactggaagatatcggctggaaagttcgcctgtgtctgatggatacccagcgcgcgctcaacttcctggtgcgtaaagcgcgtttaccgggtgggcaactggagcaggcgcgtgaaatcctgcgagatatcgaatccctgctgccgcataacgaatccctgttccagaaggtgaacttcctgatgcaggcggcaatgggttttatcaacatcgagcagaaccgcatcatcaaaatcttctcggtggtatccgtggtattcctgccgccgacgctcgttgcttccagctatggcatgaactttgagtttatgccagaactgaagtggagcttcggctaccctggcgcgattatctttatgatcctcgcgggcctggcaccgtatctgtactttaagcggaagaactggttgtaaaaaacgagagcggtggcttagtctggctaagccacctgttattcaaaggctccaggtatttaacccttttacctctttctcatagaaccatttgttcgtgttaacagcaacataggctgctacggcaattcccagaatgttaacgccaattagtgcaccaacaaatagagatagaataccaagtaatagaactataattgcttttttccataaccccaggacaaataaatatatccaggaacagaagaaagcaatgaaattcatttgaatagttaagcgttgtcttacttttaatgctttaaatgctgctttatattctggtgttgccccccagaatccaggaaaaccatgttgatcataaaaattaaatcggtatttccatttttcacttaatgaaccatcgttcatatattccttactcataaatactccataactattgttttgatgaatcagtaggtgcaagcattagcatactgaaagtggaaaaataacaaatcaaaaaaatcatcgaaccattgcctgaacaggcaaaatcttcggctatcattgtgatgatagagatgatatatactgctaatgtaccaaaaacataagtttttatatagatgaaaccactatcacggagtcgctggcaattcatgttgatgacgagataatggagtacgatggtagagactataacaagaaagcctgcttctccatcgttaaaaaagataataagaaaggcaaaaatgaaatttattaaaataaatgaaaatatataacgacgtctggaaatcttaccgttagatgttgggataaatatacgtaacataaattttacatccttgtatgagtctccggtcagcatggcaatatgcccactctcatgcaagagtcggcatattttttcagaatatatttattttttatttggacgttctacgctgcgtataaatcgcatccatcacaaaaattgccagcgccacccaaataaaggcgaaagtcaccatcttatcggcacccggtttttcaccataaaacgtcacagccagcaggaacatcagcgtcgggccaatgtactggaaaaagcctaacgttgagagacgcaagcgcgtggcagcggcggtaaaacacaacagcggtacggtagtgacaataccggcggcgatcagcagtaaattcagcgacatcgggttttgccccatatggctggttgagctgtcggcaatagcaaacaggtaaattgccgccacgggcagcagccacatggtttcgattaacatgccggtttgcgcttcaacggcaatcttcttgcgtaccagaccgtagaaggcaaaactaaatgccagtcccagcgcgataataggtagcgaaccaaaagtccacagctggactaacacgccacatatcgccagaatcaccgccagccattgcatccggcggaatcgctcgccgaggaaaatcatccccagcacaatgttcaccagcgggttaataaagtaaccaaggctcgcttccagcatatggtgattgttcaccgcccagataaacagtagccagttgccaccaatcagcacggcagagactgccagcataaaaattttctgtggcgtctgaatcagcgtttttaaataggaccactggcggcaaatgctcatcagcaccaccataaagaaaaacgaccagatcacgcgatgcgtcaggatttcatcggcgggcacgtagtaaatcaacttgaagtacgctggcgctataccccaaataaaataagcggcaagagcgagtaatacgccctgccgcgtttgttttgcatccatcgggaatactcatttttaattggtaacagcagtttacctgcttttatgtcttcaacctaccatataggtggcggtggcactggcaatataaagctgttcttcattgtgtaattcaacgcgggcgacggcgactttattgcctgcacgcaacaggctactagtagcagtaaaacgctcgcccctgcctgggcgcagataatcaacgcgaagatcaatggtccccatccgcgatagccgctggcgtagttcatcttcactgatggtttcgtggcgggttaaggtacttcccacgcacaccagaccggcggcgacatccagcgccgacgcaatgaccccgccgtgcaaaatgctttgcgcccagttgcccaccatcattggctgatttttaaaggccagctgtgcgaactctttttcgtaacgctccagttccatccccaatgcgcggttaaatggcatgtgataaacaaacatctcacccactaatttcagggcttgttcagcggtcagtacggcagacatatcatccttacacttcattggttaatgaaatgttgattttatgcttctttgttgttggtttctactttaggaagggataactaacggctatggagttaagtatgtaaaatagcccgcagaaaaatattcaccttatcaataattcgttacggagaacacgaccgatgcggactctgcagggctggttgttgccggtgtttatgttgcctatggcagtatatgcacaagaggcaacggtgaaagaggtgcatgacgcgccagcggtgcgtggcagtattatcgccaatatgctgcaggagcatgacaatccgttcacgctctatccttatgacaccaactacctcatttacacccaaaccagcgatctgaataaagaagcgattgccagttacgactgggcggaaaatgcgcgtaaggatgaagtaaagtttcagttgagcctggcatttccgctgtggcgtgggattttaggcccgaactcggtgttgggtgcgtcttatacgcaaaaatcctggtggcaactgtccaatagcgaagagtcttcaccgtttcgtgaaaccaactacgaaccgcaattgttcctcggttttgccaccgattaccgttttgcaggttggacgctgcgcgatgtggagatggggtataaccacgactctaacgggcgttccgacccgacctcccgcagctggaaccgcctttatactcgcctgatggcagaaaacggtaactggctggtagaagtgaagccgtggtatgtggtgggtaatactgacgataacccggatatcaccaaatatatgggttactaccagcttaaaatcggctatcacctcggtgatgcggtgctcagtgcgaaaggacagtacaactggaacaccggctacggcggcgcggagttaggcttaagttacccgatcaccaaacatgtgcgcctttatactcaggtttacagcggctatggcgaatcgctcatcgactataacttcaaccagacccgtgtcggtgtgggggttatgctaaacgatttgttttgatgaacggttgagtggttggcaaatctggaatccagcatccaggattaccctctcagagactaaaagcattgcagtttctcgcgcaggcgctgaaaatagcgcctgtttttatttcaggcaatcggggtgaatgtggcgcaggcggaagtgttgaatctggagtccggagctaaacaggttttacaagaaacctttggctaccaacagtttcgccccggccaggaagaaattatcgacactgtgctttccggccgcgattgcctcgtcgtcatgcccactggtggcggaaaatccctttgctatcaaatccctgccttattgctaaacggccttaccgtggttgtttcaccgctgatttcgttgatgaaagatcaggtggatcaactgcaagccaacggcgtggcggcggcgtgccttaactcgacgcaaacccgcgaacagcaacttgaagtgatgacaggctgccgcaccgggcaaattcgtctgctttatatcgccccggaacgcctgatgctggataactttcttgagcatctggcgcactggaatccggtgttattagccgttgatgaagcgcactgtatctcccaatggggccacgatttccgcccggaatatgccgcgctcggtcagttgcgccagcggttcccgacgctgccgtttatggcgctgaccgccacagccgacgacaccacgcgccaggatatcgtgcgcctgctggggctgaacgatccgctgattcaaatcagcagttttgaccgtccgaatattcgctacatgctgatggagaagttcaaaccgctcgatcagttgatgcgctacgtgcaggaacagcgcggtaagtcaggcattatctactgcaacagccgcgcgaaagtagaagacaccgctgcgcgcctgcaaagcaagggaattagcgcggcggcctatcatgccgggctggaaaataatgttcgcgccgatgtgcaggaaaaattccagcgcgatgacctgcaaattgtggtggcgacggtggcgttcggcatgggcatcaataaaccaaacgttcgcttcgtggtccactttgatattccgcgcaatatcgaatcctattatcaggaaaccggacgcgccgggcgtgatggcctgcccgcggaagcgatgctgttttacgatccggctgatatggcgtggctgcgccgttgtctggaagagaagccgcaggggcagttgcaggatatcgagcgccacaaactcaatgcgatgggcgcgtttgccgaagcgcaaacttgccgtcgtctggtattgctgaactattttggcgaagggcgtcaggagccgtgcgggaactgcgatatctgcctcgatccgccgaaacagtacgacggttcaaccgatgctcagattgccctttccaccattggtcgtgtgaatcagcggtttgggatgggttatgtggtggaagtgattcgtggtgctaataaccagcgtatccgcgactatggtcatgacaaactgaaagtctatggcatgggccgtgataaaagccatgaacattgggtgagcgtgatccgccagctgattcacctcggcctggtgacgcaaaatattgcccagcattctgccctacaactgacagaggccgcgcgcccggtgctgcgcggcgaatcctctttgcaacttgccgtgccgcgtatcgtggcgctcaaaccgaaagcgatgcagaaatcgttcggcggcaactatgatcgcaaactgttcgccaaattacgcaaactgcgtaaatcgatagccgatgaaagtaatgtcccgccgtacgtggtgtttaacgacgcaaccttgattgagatggctgaacagatgccgatcaccgccagcgaaatgctcagcgttaacggcgttgggatgcgcaagctggaacgctttggcaaaccgtttatggcgctgattcgtgcgcatgttgatggcgatgacgaagagtagtcagcagcataaaaaagtgccagtatgaagactccgtaaacgtttcccccgcgagtcaaatgtatgttgatgttatttctcaccgtcgccatggtgcacattgtggcgcttatgagccccggtcccgatttcttttttgtctctcagaccgctgtcagtcgttcccgtaaagaagcgatgatgggcgtgctgggcattacctgcggcgtaatggtttgggctgggattgcgctgcttggcctgcatttgattatcgaaaaaatggcctggctgcatacgctgattatggtgggcggtggcctgtatctctgctggatgggttaccagatgctacgtggtgcactgaaaaaagaggcggtttctgcacctgcgccacaggtcgagctggcgaaaagtgggcgcagtttcctgaaaggtttactgaccaatctcgctaatccgaaagcgattatctactttggctcggtgttctcattgtttgtcggtgataacgttggcactaccgcgcgctggggcatttttgcgctgatcattgtcgaaacgctggcgtggtttaccgtcgttgccagcctgtttgccctgccgcaaatgcgccgtggttatcaacgtctggcgaagtggattgatggttttgccggggcgttatttgccggatttggcattcatttgattatttcgcggtgatgccagacgcgtcttcagagtaagtcggataaggcgtttacgccgcatccgacattatttttcacgcatgcctcgccgatgctaacagcgctcccaccagcataaacaacgagccgaaaatcttattcagcgccttcatctgctttggtcctttaatccatagagcaatccgttgagcaagggtggcgtaaccgatcatcacaataatatcgaccacaatagtggtgacgccgagcacgatatactgcatcagttgcggctgttgcggcatgatgaattgcggaaatagcgccgccagaaacacaatacttttgggattggtgagattcacaaaaactgcgcgctggaacaaatgtcgacgcgattgagtagaggccagcgatttaaggtcaattgcaccagcggcgcgccactgctggattcccagccaaatcaagtaagccgcgcctgcccacttcaacacttcaaacgcaatcactgagcgggaaaatagcgtccccaaccccacgccaaccagcacaatatgaatcgccagtccggtctgaagcccagcaatagacgccaccgcgccgcgataaccgtggttgagcgaggtggtcatagtgttgattgcaccagagcctggcgacaggcttaaaatgatcgatgtcagcaggtaggcaaaccaccattctaaggtcatgatgaactcccggtgtgtctatttttgtgccacaatacgctactgtcgcagcgttgtgtcaggcacgctaaaaaaaacgattttacgtggtttaagaggcagattacccgatgtttcagcagcaaaaagactgggaaacaagagaaaacgcgtttgctgcttttaccatgggaccgctgactgatttctggcgtcagcgtgatgaagcagagtttactggtgtggatgacattccggtgcgctttgtccgttttcgcgcacagcaccatgaccgggtggtagtcatctgcccggggcgtattgagagctacgtaaaatatgcggaactggcctatgacctgttccatttggggtttgatgtcttaatcatcgaccatcgcgggcagggacgttccggtcgcctgttagccgatccgcatctcgggcatgttaatcgctttaatgattatgttgatgatctggcggcattctggcagcaggaggttcagcccggtccgtggcgtaaacgctatatactggcacattcgatgggcggtgcgatctccacattatttctgcaacgccatccaggtgtatgtgacgccattgcgctaactgcgccaatgtttgggatcgtgattcgtatgccgtcatttatggcacggcagatcctcaactgggccgaagcgcatccacgtttccgtgatggctatgcaataggcaccgggcgctggcgcgcgttgccgtttgctatcaacgtactgacccacagcagacagcgatatcgacgtaacttacgcttctatgctgatgacccaacgattcgcgtcggtgggccgacctaccattgggtacgcgaaagtattctggctggcgaacaggtgttagccggtgcgggtgatgacgccacgccaacgcttctcttgcaggctgaagaggaacgcgtggtggataaccgcatgcatgaccgtttttgtgaactccgcaccgccgcgggccatcctgtcgaaggaggacggccgttggtaattaaaggtgcttaccatgagatcctttttgaaaaggacgcaatgcgctcagtcgcgctccacgccatcgttgattttttcaacaggcataactcacccagcggaaaccgctctacagaggtttaaatttcttatgtaccaggttgttgcgtctgatttagatggcacgttactttctcccgaccatacgttatccccttacgccaaagaaactctgaagctgctcaccgcgcgcggcatcaactttgtgtttgcgaccggtcgtcaccacgttgatgtggggcaaattcgcgataatctggagattaagtcttacatgattacctccaatggtgcgcgcgttcacgatctggatggtaatctgatttttgctcataacctggatcgcgacattgccagcgatctgtttggcgtagtcaacgacaatccggacatcattactaacgtttatcgcgacgacgaatggtttatgaatcgccatcgcccggaagagatgcgcttttttaaagaagcggtgttccaatatgcgctgtatgagcctggattactggagccggaaggcgtcagcaaagtgttcttcacctgcgattcccatgaacaactgctgccgctggagcaggcgattaacgctcgttggggcgatcgcgtcaacgtcagtttctctaccttaacctgtctggaagtgatggcgggcggcgtttcaaaaggccatgcgctggaagcggtggcgaagaaactgggctacagcctgaaggattgtattgcgtttggtgacgggatgaacgacgccgaaatgctgtcgatggcggggaaaggctgcattatgggcagtgcgcaccagcgtctgaaagaccttcatcccgagctggaagtgattggtactaatgccgacgacgcggtgccgcattatctgcgtaaactctatttatcgtaatcgttctttatttggtcagttgtcaacctgatacttcgctacaatggatacccgttaatcaaagagttttccattgtggcgctacttatcatcaccacgattctgtgggccttctcctttagcttttatggcgagtaccttgcggggcacgtcgatagctattttgcggtgctggtgcgcgttggcctggcggcactcgtttttctgccgtttctgcgtacccgtggcaatagcctgaaaacggtcggcctgtatatgctggtgggcgcgatgcagcttggcgtgatgtatatgctgagtttccgcgcttatctctacctgacggtttccgagctgctgctgttcaccgtgctgacgccgctctacatcacgctgatttatgacatcatgagtaagcgccgtctgcgctggggctatgcctttagcgccttgctggcggtgattggtgccgggattattcgctatgatcaggtcaccgaccatttctggactggcttgctgctggtgcaactctccaatatcacttttgccattggcatggtgggttacaaacgcctgatggaaactcgcccgatgccacagcataacgcctttgcgtggttctatcttggcgcgtttctggtggcagtgattgcatggttcttgctgggaaatgcgcagaaaatgccgcaaaccacgctgcaatggggcattctggtgtttcttggcgtggtggcttccgggattggctactttatgtggaactacggcgcgacgcaggtggacgccggaacgctgggcattatgaataatatgcacgttccggcagggctgctggtaaacctggctatctggcaccaacagccgcactggccaacgtttattacaggcgcgctggtgatcctggcctcactgtgggtgcatcgtaagtgggtcgctccgcgctcttcacaaacggcagatgatcgcaggcgtgattgcgcgctgagcgaataaacgcttccgtaactggctgacgctgctcgccatcgcgcacggcggcgtacagtcggctccacaagccttcgcccagggttttggtcaccaccagaccctggcgctcaaaactctctactacccaatgcggtagcgcggcaatacccatccgcgcggcaaccatctgaatcaacaataaggtgttatcgacgcttttcagtgacgggctgacgcctgccggctgaagaaaatgccgccagacatccagtcgactacgctgcaccggataaattaatagcgtctcgctggcgagatcttccggtgtaattcgcgttttcgccgccagtggatggtcaggtgctaacaccagacgcacttcatagtcgaacatcggcgaataatgcaggccactgcgcggcagaatatcggacgtcattaccagatccagctctccctgttgcaaggcgggctgcgggtcaaatgtcacgcccgatttaaaatccatctctacctgcggccagttcttatggaaattttctaacgcgggtgtcagccactgaatacagctatggcactcaatggcaatgcgcagacgcgtctgctgcggttcattgcaggcttgcagggcctggctaatttgcggcagtacctggtttgccagttgcaacaggatttctccctgcggtgtaaagcgtagcggctggctcttacgcacaaatagccggaagccaaggcgttgttccagatcgctaaactggtgagacagggcggattgcgtctgatgcaacgtcgccgcagcggctgcgagcgagccgcagttccgcaacgcttgtagcgttttcaggtgttttacttcgatcatgaaagtccttcacttcggcatgaataatttgcgcttgaggaatatacagtaaccgccaattatggatgtgtaaacatctggacggctaaaatccttcgtcttttaaatttatggtgcgttggctgcgtttctccaccccggtcacttacttcagtaagctcccggggatgaataaacttgccgccttccctaaattcaaaatccataggatttacatataattagaggaagaaaaaatgacaatattgaatcacaccctcggtttccctcgcgttggcctgcgtcgcgagctgaaaaaagcgcaagaaagttattgggcggggaactccacgcgtgaagaactgctggcggtagggcgtgaattgcgtgctcgtcactgggatcaacaaaagcaagcgggtatcgacctgctgccggtgggcgattttgcctggtacgatcatgtactgaccaccagtctgctgctgggtaacgttccggcgcgtcatcagaacaaagatggttcggtagatatcgacaccctgttccgtattggtcgtggacgtgcgccgactggcgaacctgcggcggcagcggaaatgaccaaatggtttaacaccaactatcactacatggtgccggagttcgttaaaggccaacagttcaaactgacctggacgcagctgctggacgaagtggacgaggcgctggcgctgggccacaaggtgaaacctgtgctgctggggccggttacctggctgtggctggggaaagtgaaaggtgaacaatttgaccgcctgagcctgctgaacgacattctgccggtttatcagcaagtgctggcagaactggcgaaacgcggcatcgagtgggtacagattgatgaacccgcgctggtactggaactaccacaggcgtggctggacgcatacaaacccgcttacgacgcgctccagggacaggtgaaactgctgctgaccacctattttgaaggcgtaacgccaaatctcgacacgattactgcgctgcctgttcagggtctgcatgttgacctcgtacatggtaaagatgacgttgctgaactgcacaagcgcctgccttctgactggttgctgtctgcgggtctgatcaatggtcgtaacgtctggcgcgccgatcttaccgagaaatatgcgcaaattaaggacattgtcggcaaacgtgatttgtgggtggcatcttcctgctcgttgctgcacagccccatcgacctgagcgtggaaacgcgtcttgatgcagaagtgaaaagctggtttgccttcgccctacaaaaatgccatgaactggcactgctgcgcgatgcgctgaacagtggtgacacggcagctctggcagagtggagcgccccgattcaggcacgtcgtcactctacccgcgtacataatccggcggtagaaaagcgtctggcggcgatcaccgcccaggacagccagcgtgcgaatgtctatgaagtgcgtgctgaagcccagcgtgcgcgttttaaactgccagcgtggccgaccaccacgattggttccttcccgcaaaccacggaaattcgtaccctgcgtctggatttcaaaaagggcaatctcgacgccaacaactaccgcacgggcattgcggaacatatcaagcaggccattgttgagcaggaacgtttgggactggatgtgctggtacatggcgaggccgagcgtaatgacatggtggaatactttggcgagcacctcgacggatttgtctttacgcaaaacggttgggtacagagctacggttcccgctgcgtgaagccaccgattgtcattggtgacattagccgcccggcaccgattaccgtggagtgggcgaagtatgcgcaatcgctgaccgacaaaccggtgaaagggatgctgacggggccggtgaccatactctgctggtcgttcccgcgtgaagatgtcagccgtgaaaccatcgccaaacagattgcgctggcgctgcgtgatgaagtggccgatctggaagccgctggaattggcatcatccagattgacgaaccggcgctgcgcgaaggtttaccgctgcgtcgtagcgactgggatgcgtatctccagtggggcgtagaggccttccgtatcaacgccgccgtggcgaaagatgacacacaaatccacactcacatgtgttattgcgagttcaacgacatcatggattcgattgcggcgctggacgcagacgtcatcaccatcgaaacctcgcgttccgacatggagttgctggagtcgtttgaagagtttgattatccaaatgaaatcggtcctggcgtctatgacattcactcgccaaacgtaccgagcgtggaatggattgaagccttgctgaagaaagcggcaaaacgcattccggcagagcgcctgtgggtcaacccggactgtggcctgaaaacgcgcggctggccagaaacccgcgcggcactggcgaacatggtgcaggcggcgcagaacttgcgtcgggggtaaaatccaaaccgggtggtaataccacccggtcttttctcattacagcgacttcttcccaccatactgcttaaaccattccagcatacgctgccagccatcttctgcagatgcggcatgatagctcgggcgataatcagcgttgaatgcatgcccggcgtccgggtacacgataatctctgctttcgcattagcagcccgcagcgcctggcgcatggtttcaacgctctcctgcggaatgctgttatcctgaccaccatataagccgagaatcggcgcgttaagatcggttgcgatatcaacaggttgtttcggtgaattcagcgacttgtcgcccgtcagtttgccgtaccacgccactgcggcttttagctgtggattatgcgcggcatacagccaggtgatacgtccaccccagcagaatccggtgatcattaaacgatgaacatcgccgccgttgcgggaagcccaactggcgacatgatcgagatcggccagcacctgcgagtcaggcacttttgctaccagaccgctaagcaacgtggggatatcggcaaaatcattcggatcgccttcgcggaagtaaagttcaggtgcgatagccagatacccctccagcgccagacggcgacaaatgtcgcggatatgttcatgcacgccaaaaatttcctgcactacaatgaccactggcagtgggccatcgctttgctttggtctggcatggtaagcaggcatgttatccccttgtgaagggatagaggtgaagcccgccacaatcgcgtcgtccggggtctgaacgatggtcgaagcgagaggcgatgcagcaggtgcaaatccagattgttgtgttgttgccatggtattctccgtacccttataaaaatgttgcgcaatgttaactatagtcagcatgcaacaaatcacattgcctgaatcggctcatcttttatgcagtcctgcagaatgaagggtgatttatgtgatttgcatcacttttggtgggtaaatttatgcaacgcatttgcgtcatggtgatgagtatcacgaaaaaatgttaaacccttcggtaaagtgtctttttgcttcttctgactaaaccgattcacagaggagttgtatatgtccaagtctgatgtttttcatctcggcctcactaaaaacgatttacaaggggctacgcttgccatcgtccctggcgacccggatcgtgtggaaaagatcgccgcgctgatggataagccggttaagctggcatctcaccgcgaattcactacctggcgtgcagagctggatggtaaacctgttatcgtctgctctaccggtatcggcggcccgtctacctctattgctgttgaagagctggcacagctgggcattcgcaccttcctgcgtatcggtacaacgggcgctattcagccgcatattaatgtgggtgatgtcctggttaccacggcgtctgtccgtctggatggcgcgagcctgcacttcgcaccgctggaattcccggctgtcgctgatttcgaatgtacgactgcgctggttgaagctgcgaaatccattggcgcgacaactcacgttggcgtgacagcttcttctgataccttctacccaggtcaggaacgttacgatacttactctggtcgcgtagttcgtcactttaaaggttctatggaagagtggcaggcgatgggcgtaatgaactatgaaatggaatctgcaaccctgctgaccatgtgtgcaagtcagggcctgcgtgccggtatggtagcgggtgttatcgttaaccgcacccagcaagagatcccgaatgctgagacgatgaaacaaaccgaaagccatgcggtgaaaatcgtggtggaagcggcgcgtcgtctgctgtaattctcttctcctgtctgaaggccgacgcgttcggccttttgtatttttgcgtagcgcctcgcaggaaatgcctttccaactggacgtttgtacagcacaattctattttgtgcgggtaagttgttgcgtcaggaggcgttgtggatttctcaatcatggtttacgcagttattgcgttggtgggtgtggcaattggctggctgtttgccagttatcaacatgcgcagcaaaaagccgagcaattagctgaacgtgaagagatggtcgcggagttaagcgcggcaaaacaacaaattacccaaagcgagcactggcgtgcagagtgcgagttactcaataacgaagtgcgcagcctgcaaagtattaacacctctctggaggccgatctgcgtgaagtaaccacgcggatggaagccgcacagcaacatgctgacgataaaattcgccagatgattaacagcgagcagcgcctcagtgagcagtttgaaaacctcgccaaccgtatttttgagcacagcaatcgccgggttgatgagcaaaaccgtcagagtctgaacagcctgttgtcgccgctacgtgaacaactggacggtttccgccgtcaggttcaggacagcttcggtaaagaagcacaagaacgccataccctgacccacgaaattcgcaatctccagcaactcaacgcgcaaatggcccaggaagcgatcaacctgacgcgcgcgctgaaaggcgacaataaaacccagggcaactggggcgaggtagtattgacgcgggtgctggaggcttccggtctgcgtgaagggtatgaatatgaaacccaggtcagcatcgaaaatgacgcccgctcgcggatgcagccggatgtcatcgtgcgcctgccgcagggaaaagatgtggtgatcgacgccaaaatgacgctggtcgcctatgaacgctattttaacgccgaagacgactacacccgcgaaagcgcgctacaggaacatatcgcgtcggtgcgtaaccatatccgtttgctgggacgcaaagattatcaacagctgccggggctgcgaactctggattacgtgctgatgtttattcccgttgaacccgcttttttactggcgcttgaccgccagccggagctgatcaccgaagcgttgaaaaacaacatcatgctggttagcccgactacgctgctggtggcgctgcgcactatcgccaacctgtggcgttatgagcatcaaagccgcaacgcccagcaaatcgccgatcgtgccagcaagctgtacgacaagatgcgtttgttcatcgatgacatgtccgcgattggtcaaagtctcgacaaagcgcaggataattatcggcaggcaatgaaaaaactctcttcagggcgcggaaatgtgctggcgcaggcagaagcgtttcgcggtttaggagtagaaattaaacgcgagattaatccggatttggctgaacaggcggtgagccaggatgaagagtatcgacttcggtcggttccggagcagccgaatgatgaagcttatcaacgcgatgatgaatataatcagcagtcgcgctagcccattgggagtagttaagccgggtagaaatctagggcatcgacgcccaatctgttacacttctggaacaattttttgatgagcaggcattgagatggtggataagtcacaagaaacgacgcactttggttttcagaccgtcgcgaaggaacaaaaagcggatatggtcgcccacgttttccattccgtggcatcaaaatacgatgtcatgaatgatttgatgtcatttggtattcatcgtttgtggaagcgattcacgattgattgcagcggcgtacgccgtgggcagaccgtgctggatctggctggtggcaccggcgacctgacagcgaaattctcccgcctggtcggagaaactggcaaagtggtccttgctgatatcaatgaatccatgctcaaaatgggccgcgagaagctgcgtaatatcggtgtgattggcaacgttgagtatgttcaggcgaacgctgaggcgctgccgttcccggataacacctttgattgcatcaccatttcgtttggtctgcgtaacgtcaccgacaaagataaagcactgcgttcaatgtatcgcgtgctgaaacccggcggccgcctgctggtgcttgagttctcgaagccaattatcgagccgctgagcaaagcctatgatgcatactccttccatgtgctgccgcgtattggctcactggtcgcgaacgacgccgacagctaccgttatctggcagaatccatccgtatgcatcccgatcaggataccctgaaagccatgatgcaggatgccggattcgaaagtgtcgactactacaatctgacggcaggggttgtggcgctgcatcgtggttataagttctgacaggagaccggaaatgccttttaaacctttagtgacggcaggaattgaaagtctgctcaacaccttcctgtatcgctcacccgcgctgaaaacggcccgctcgcgtctgctgggtaaagtattgcgcgtggaggtaaaaggcttttcgacgtcattgattctggtgttcagcgaacgccaggttgatgtactgggcgaatgggcaggcgatgctgactgcaccgttatcgcctacgccagtgtgttgccgaaacttcgcgatcgccagcagcttaccgcactgattcgcagtggtgagctggaagtgcagggcgatattcaggtggtgcaaaacttcgttgcgctggcagatctggcagagttcgaccctgcggaactgctggccccttataccggtgatatcgccgctgaaggaatcagcaaagccatgcgcggaggcgcaaagttcctgcatcacggcattaagcgccagcaacgttatgtggcggaagccattactgaagagtggcgtatggcacccggtccgcttgaagtggcctggtttgcggaagagacggctgccgtcgagcgtgctgttgatgccctgaccaaacggctggaaaaactggaggctaaatgacgccaggtgaagtacggcgcctatatttcatcattcgcacttttttaagctacggacttgatgaactgatccccaaaatgcgtatcaccctgccgctacggctatggcgatactcattattctggatgccaaatcggcataaagacaaacttttaggtgagcgactacgactggccctgcaagaactggggccggtttggatcaagttcgggcaaatgttatcaacccgccgcgatctttttccaccgcatattgccgatcagctggcgttattgcaggacaaagttgctccgtttgatggcaagctggcgaagcagcagattgaagctgcaatgggcggcttgccggtagaagcgtggtttgacgattttgaaatcaagccgctggcttctgcttctatcgcccaggttcataccgcgcgattgaaatcgaatggtaaagaggtggtgattaaagtcatccgcccggatattttgccggttattaaagcggatctgaaacttatctaccgtctggctcgctgggtgccgcgtttgctgccggatggtcgccgtctgcgcccaaccgaagtggtgcgcgagtacgaaaagacattgattgatgaactgaatttgctgcgggaatctgccaacgccattcagcttcggcgcaattttgaagacagcccgatgctctacatcccggaagtttaccctgactattgtagtgaagggatgatggtgatggagcgcatttacggcattccggtgtctgatgttgcggcgctggagaaaaacggcactaacatgaaattgctggcggaacgcggcgtgcaggtgttcttcactcaggtctttcgcgacagctttttccatgccgatatgcaccctggcaacatcttcgtaagctatgaacacccggaaaacccgaaatatatcggcattgattgcgggattgttggctcgctaaacaaagaagataaacgctatctggcagaaaactttatcgccttctttaatcgcgactatcgcaaagtggcagagctacacgtcgattctggctgggtgccaccagataccaacgttgaagagttcgaatttgccattcgtacggtctgtgaacctatctttgagaaaccgctggccgaaatttcgtttggacatgtactgttaaatctgtttaatacggcgcgtcgcttcaatatggaagtgcagccgcaactggtgttactccagaaaaccctgctctacgtcgaaggggtaggacgccagctttatccgcaactcgatttatggaaaacggcgaagcctttcctggagtcgtggattaaagatcaggtcggtattcctgcgctggtgagagcatttaaagaaaaagcgccgttctgggtcgaaaaaatgccagaactgcctgaattggtttacgacagtttgcgccagggcaagtatttacagcacagtgttgataagattgcccgcgagcttcagtcaaatcatgtacgtcagggacaatcgcgttattttctcggaattggcgctacgttagtattaagtggcacattcttgttggtcagccgacctgaatgggggctgatgcccggctggttaatggcaggtggtctgatcgcctggtttgtcggttggcgcaaaacacgctgattttttcatcgctcaaggcgggccgtgtaacgtataatgcggctttgtttaatcatcatctaccacagaggaacatgtatgggtggtatcagtatttggcagttattgattattgccgtcatcgttgtactgctttttggcaccaaaaagctcggctccatcggttccgatcttggtgcgtcgatcaaaggctttaaaaaagcaatgagcgatgatgaaccaaagcaggataaaaccagtcaggatgctgattttactgcgaaaactatcgccgataagcaggcggatacgaatcaggaacaggctaaaacagaagacgcgaagcgccacgataaagagcaggtgtaatccgtgtttgatatcggttttagcgaactgctattggtgttcatcatcggcctcgtcgttctggggccgcaacgactgcctgtggcggtaaaaacggtagcgggctggattcgcgcgttgcgttcactggcgacaacggtgcagaacgaactgacccaggagttaaaactccaggagtttcaggacagtctgaaaaaggttgaaaaggcgagcctcactaacctgacgcccgaactgaaagcgtcgatggatgaactacgccaggccgcggagtcgatgaagcgttcctacgttgcaaacgatcctgaaaaggcgagcgatgaagcgcacaccatccataacccggtggtgaaagataatgaagctgcgcatgagggcgtaacgcctgccgctgcacaaacgcaggccagttcgccggaacagaagccagaaaccacgccagagccggtggtaaaacctgctgcggacgctgaaccgaaaaccgctgcaccttccccttcgtcgagtgataaaccgtaaacatgtctgtagaagatactcaaccgcttatcacgcatctgattgagctgcgtaagcgtctgctgaactgcattatcgcggtgatcgtgatattcctgtgtctggtctatttcgccaatgacatctatcacctggtatccgcgccattgatcaagcagttgccgcaaggttcaacgatgatcgccaccgacgtggcctcgccgttctttacgccgatcaagctgacctttatggtgtcgctgattctgtcagcgccggtgattctctatcaggtgtgggcatttatcgccccagcgctgtataagcatgaacgtcgcctggtggtgccgctgctggtttccagctctctgctgttttatatcggcatggcattcgcctactttgtggtctttccgctggcatttggcttccttgccaataccgcgccggaaggggtgcaggtatccaccgacatcgccagctatttaagcttcgttatggcgctgtttatggcgtttggtgtctcctttgaagtgccggtagcaattgtgctgctgtgctggatggggattacctcgccagaagacttacgcaaaaaacgcccgtatgtgctggttggtgcattcgttgtcgggatgttgctgacgccgccggatgtcttctcgcaaacgctgttggcgatcccgatgtactgtctgtttgaaatcggtgtcttcttctcacgcttttacgttggtaaagggcgaaatcgggaagaggaaaacgacgctgaagcagaaagcgaaaaaactgaagaataaattcaaccgcccgtcagggcggttgtcatatggagtacaggatgtttgatatcggcgttaatttgaccagttcgcaatttgcgaaagaccgtgatgatgttgtagcgtgcgcttttgacgcgggagttaatgggctactcatcaccggcactaacctgcgtgaaagccagcaggcgcaaaagctggcgcgtcagtattcgtcctgttggtcaacggcgggcgtacatcctcacgacagcagccagtggcaagctgcgactgaagaagcgattattgagctggccgcgcagccagaagtggtggcgattggtgaatgtggtctcgactttaaccgcaacttttcgacgccggaagagcaggaacgcgcttttgttgcccagctacgcattgccgcagatttaaacatgccggtatttatgcactgtcgcgatgcccacgagcggtttatgacattgctggagccgtggctggataaactgcctggtgcggttcttcattgctttaccggcacacgcgaagagatgcaggcgtgcgtggcgcatggaatttatatcggcattaccggttgggtttgcgatgaacgacgcggactggagctgcgggaacttttgccgttgattccggcggaaaaattactgatcgaaactgatgcgccgtatctgctccctcgcgatctcacgccaaagccatcatcccggcgcaacgagccagcccatctgccccatattttgcaacgtattgcgcactggcgtggagaagatgccgcatggctggctgccaccacggatgctaatgtcaaaacactgtttgggattgcgttttagagtttgcggaactcggtattcttcacactgtgcttaatctctttattaataagattaagcaatagcatggagcgagcctcaccatcgggttcggtgaaaatggcctgaaagccttcgaacgcgccttcggtaataatcaccttatcacccggataaggggttgccggatcgacaatgtctttcggtttatataccgatagctgatgaataaccgccgatgggactatcgctggcgacgcgccaaagcgcacgaagtggctgacaccgcgggtcgcgttgatagtcgtggtatgaatcacttctgggtcaaattccacaaacaggtagttggggaacaatggctcactgactgcagtacgttttccacgcacgattttttccagggtgatcatcggtgccaggcaattcacagcctgtctttcgaggtgttcctgggcacgttgaagttgcccgcgcttgcagtacagtaaataccaggattgcataatgactcttatccgtttaatcggggcgcaaggatagcaaaagctttacgctaagttaattatattccccggtttgcgttataccgtcagagttcacgctaatttaacaaatttacagcatcgcaaagatgaacgccgtataatgggcgcagattaagaggctacaatggacgccatgaaatataacgatttacgcgacttcttgacgctgcttgaacagcagggtgagctaaaacgtatcacgctcccggtggatccgcatctggaaatcactgaaattgctgaccgcactttgcgtgccggtgggcctgcgctgttgttcgaaaaccctaaaggctactcaatgccggtgctgtgcaacctgttcggtacgccaaagcgcgtggcgatgggcatggggcaggaagatgtttcggcgctgcgtgaagttggtaaattattggcgtttctgaaagagccggagccgccaaaaggtttccgcgacctgtttgataaactgccgcagtttaagcaagtattgaacatgccgacaaagcggctgcgtggtgcgccctgccaacaaaaaatcgtctctggcgatgacgtcgatctcaatcgcattcccattatgacctgctggccggaagatgccgcgccgctgattacctgggggctgacagtgacgcgcggcccacataaagagcggcagaatctgggcatttatcgccagcagctgattggtaaaaacaaactgattatgcgctggctgtcgcatcgcggcggcgcgctggattatcaggagtggtgtgcggcgcatccgggcgaacgtttcccggtttctgtggcgctgggtgccgatcccgccacgattctcggtgcagtcactcccgttccggatacgctttcagagtatgcgtttgccggattgctacgtggcaccaagaccgaagtggtgaagtgtatctccaatgatcttgaagtgcccgccagtgcggagattgtgctggaagggtatatcgaacaaggcgaaactgcgccggaagggccgtatggcgaccacaccggttactataatgaagtcgatagtttcccggtatttaccgtgacgcatattacccagcgtgaagatgcgatttaccattccacctataccgggcgtccgccagatgagcccgcggtgctgggtgtcgcactgaacgaagtgtttgtgccgattctgcaaaaacagttcccggaaattgtcgatttttacctgccgccggaaggctgctcttatcgcctggcggtagtgacaatcaaaaaacagtacgccggacacgcgaagcgcgtcatgatgggcgtctggtcgttcttacgccagtttatgtacactaaatttgtgatcgtttgcgatgatgacgttaacgcacgcgactggaacgatgtgatttgggcgattaccacccgtatggacccggcgcgggatactgttctggtagaaaatacgcctattgattatctggattttgcctcgcctgtctccgggctgggttcaaaaatggggctggatgccacgaataaatggccgggggaaacccagcgtgaatggggacgtcccatcaaaaaagatccagatgttgtcgcgcatattgacgccatctgggatgaactggctatttttaacaacggtaaaagcgcctgatgcgcgtttgttttgccctatttatcgatccgacagagaaagcgcatgacaaccttaagctgtaaagtgacctcggtagaagctatcacggataccgtatatcgtgtccgcatcgtgccagacgcggccttttcttttcgtgctggtcagtatttgatggtagtgatggatgagcgcgacaaacgtccgttctcaatggcttcgacgccggatgaaaaagggtttatcgagctgcatattggcgcttctgaaatcaacctttacgcgaaagcagtcatggaccgcatcctcaaagatcatcaaatcgtggtcgacattccccacggagaagcgtggctgcgcgatgatgaagagcgtccgatgattttgattgcgggcggcaccgggttctcttatgcccgctcgattttgctgacagcgttggcgcgtaacccaaaccgtgatatcaccatttactggggcgggcgtgaagagcagcatctgtatgatctctgcgagcttgaggcgctttcgttgaagcatcctggtctgcaagtggtgccggtggttgaacaaccggaagcgggctggcgtgggcgtactggcaccgtgttaacggcggtattgcaggatcacggtacgctggcagagcatgatatctatattgccggacgttttgagatggcgaaaattgcccgcgatctgttttgcagtgagcgtaatgcgcgggaagatcgcctgtttggcgatgcgtttgcatttatctgagatataaaaaaacccgcccctgacaggcgggaagaacggcaactaaactgttattcagtggcatttagatctatgacgtatctggcaaaccatgcccgatgcgacgctgtcgcgtcttatcgtgcctacaaatagtccgaaccgtaggccggataaggcgtttacgccgcatccggcaattggtgcatgatgcctgatgcgacgctgtcgcgtcttatcgtgcctacaaatagtccgaaccgtaggccggataaggcgtttacgccgcatccggcaattggtgcatgatgcctgatgcgacgctggcgcgtcttatcaggcctacattggtgccggatcggtagaccggataaggcgttcacgccgcatccggcaagtggttaaacccgctcaaacaccgtcgcaataccctgacccagaccgatacacatcgtcgccagaccaaactgaacgtctttgcgttccatcagattcagcagcgtggtgctgatacgcgcaccggaacaacccagcggatgacccagcgcgatcgcgccaccgttgaggttgatcttctcgtcaatctgctcaattagtcccagatctttaatacatggcaggatctgcgcggcaaaggcttcgttcatttcaaacacgccgatatcgctggcagaaagccccgcttttttcagcgccagtttcgaggccggaaccgggccgtaacccataatcgatgggtcacaaccaacgaccgccatcgaacgcacacgagcgcgcggcttaagacctaattcatgggcgcggctttcactcatcaccagcatggcagctgcgccatcggaaagtgcagaagatgtgcccgccgttaccataccgtttactggatcaaacgccggacgcagcgtggcgagggcttccacggtggtttccgggcgaatcacttcgtcgtaattaaactgcttcaggacgccgtcggcatcgtgaccaccggtcgggatgatttcatttttaaatgcggccgactgcgtggcggcccaggcgcgggcgtgtgaccgcgcggcaaaggcatcctgcatttcacggctgataccgtgcatacgcgccagcatttctgccgttaagcccatcatgcccgccgctttggcgacattgcggctcaggccggggtgaaaatcgacgccgtgactcatcggcacatggcccatatgctccacgccgccaaccagacatgcctgcgcatcgccagtcatgatcattcgtgctgcgtcatgcagtgcctgcatggatgaaccacacaagcgattaacggtaaccgccgggacagagtgtggtacttctgccagcagcgccgcgttacgggcgatattaaaaccctgctccagcgtctgctgcacacaaccccagtaaatatcgtcgagggccgccgcttccagcgccgggttacgcgccagcaggctacgcattaaatgagcggagagatcttctgcacgcacgttacgaaaagcaccgcccttcgaacggcccatcggggtgcgaattgcatcgacaatgacaacctgttccattgtgactccttaagccgttttcaggtcgccaaccggacgggctggctcaaccggaggatagtacggttcgttatgacgcgctttattacgcagaccttccggcacttcatacagcgggccgaggtgctgatattgctgtgccatatcgaggtattttgcgctaccgagggtgtccagccagcggaacgcgccgccgtggaacggagggaagcccaggccgtagaccagcgccatatccgcttccgccggagtggcgataatgccttcctccagacagcgcaccacttcgttgaccatcgggatcatcatgcgggcgataatctcttcttcgctgaaatcgcgcttcggctggctcacttctgccagcaggtcttcaacggcggcgtcttcttctttcttcggcttacctttgctgtcttctttataacgccagaaaccgaggccgttcttctgaccaaagcggttggcatcaaacagcgcgtcgatggcatcgcggtaatctttctgcatccgctgcgggaagcctgctgccatgacagcctgagcgtgatgcgcggtatcaatgcccacaacgtccagcagatatgccgggcccatcggccagccaaactgtttttccatcactttgtcgatcttgcggaaatccgcgccgtcgcgcagcagctggctgaaaccggcgaaatacgggaacagcacgcggttaacaaagaagccggggcagtcgttaaccacaatcggcgtcttgcccatcttgctcgcccaggcgacaactttcgcgatggtttcgtcggagcttttctcgccgcgaataatttctaccaacggcattcggtggaccgggttaaagaagtgcatcccgcagaagttttccgggcgttccagcgcgttggccagttcgctgataggaatggttgaagtgttagacgccagcacggtatcctggcgtactttttgttcggtttctgccagtacggcttttttcactttcgggttttcaacaaccgcttctaccacaatatccacgcggtcaaatccggcgtagtcgagcgttgggtggattgtggagatcacgccagccagtttcagaccatcgatcttgccgcgctcaagctgcttgttcagcagtttcgcggcttcggtcatgccgagggttaacgacttgtcgttgatatctttcatgacaaccggcacgcctttccacgcagactggtaagcgatgccgccgcccataatgcctgcacccagcaccgcggcctgtttcggggtttcaacgtctttggtgagtttcttcgctttgccttttacatattgatcgttaaggaaaatgccgaccagtgcgcgggcttcgttggtatgcgccagcgggacaaaacttttgttttccaggtttaaggcttcttcacgaccaaaacgggccgcagcttcaatggtttttactgcggtgatgggggccggataatgtttccccgctgtttgtgcgaccatccctttagcgatggtgaagctcatggtggcttcaatcttgctcagttttagtggttccagcttcggctgacgttttgctttccagtcgaggtcgccgttaatggcctggcgtaaaaccgcctttgcgccttcaaccagtttttctgctttgactacgccatccaccagaccgattttcagcgcctgatccgcgccgacatctttaccggcggcaatgatttccagcgcactgtcagcgcccagcatacgtggcatacgtacagaaccgccaaagccaggcatgatgcccagtttggtttccggcagaccgatgcgcagatccggcgtcgccagacgataatcggtcgccagcacgcattcgcagccaccgcccagcgcatagccattgacggcagcaatggtcggcaccggcagatcttccaggcgattaaacacgctattggcaaagtgcagccactgacttaactgttcttcaggaacgaggaacagggacaaaaattcggtgatatcagcaccgacgataaaggctgctttgttcgaacgcagcagcagcccttttagatctgattgctgttccagcacgccgatggcctcgccgaggctggcgacggtcgcagtgtcgagtttattaactgaacctggggcatcaaataccagttcggcaatgccatcttccagccagtcaaggtacagggtgtcgcctttgtaaagcatgtcagtctcctgaatccgcaaggtgatctggtcgtaccagatgagtcgaagtgtgtattttgtgttaaaaatatgcaaacaaaagattaaagaaatgccgatctgatcacgctcggcagaaatcacgctctggatgaacgatgtgctaagatgcggagacttaaggtcaaaaaaacagaagggtaaaaaatggaatcactggcctcgctctataaaaatcatatagctaccttacaagaacggactcgcgatgcgctggcgcgcttcaagctggatgcgttacttattcactccggcgagctgttcaatgtttttctcgacgatcatccctatccgtttaaagtgaacccgcaattcaaagcgtgggtgccggtaactcaggtgccaaactgctggttgctggtggatggcgtgaacaagccgaaactgtggttctatctgccggttgattactggcacaacgtcgaaccgctgccgacctctttctggactgaagatgtggaagtgatcgcgctgccgaaagccgatggcattggtagcctgctgcctgctgcgcgcggcaatatcggttatatcggtccggtgccggaacgtgcgctgcaactgggtattgaggccagcaacatcaacccgaaaggggttatcgactacctgcattactatcgctccttcaaaactgagtacgaactggcctgtatgcgtgaagcgcagaaaatggcggtcaacggtcaccgcgcggcagaagaagcgttccgttctggcatgagcgagttcgatatcaacattgcctatctgaccgcgaccggtcatcgtgataccgacgtaccttacagcaacattgtggcgcttaacgaacacgctgcggtactgcattacaccaaactggaccatcaggcaccggaagagatgcgcagcttcctgctggatgccggggcagaatataacggctatgcggctgacctgacccgtacctggtcggcaaaaagtgacaacgactacgcgcagctggtgaaggacgttaatgatgaacaactggcgctgatcgccaccatgaaagcaggcgtcagctatgtggattaccacatccagttccatcagcgcatcgccaaactgctgcgtaaacatcaaatcatcaccgatatgagtgaagaagcgatggtcgaaaacgatcttaccgggccgtttatgccgcatggtatcggccatccgctgggcctgcaggtgcatgacgtcgctggttttatgcaggatgatagcggtacgcacctcgcggcaccggcaaaatatccgtacctgcgctgcacccgtattctccagccgggcatggtgttaaccatcgaaccgggtatctacttcatcgaatcgctactggcaccgtggcgtgaagggcagttcagcaagcacttcaactggcagaaaattgaagcactgaaaccgttcggcggcattcgtatcgaagacaacgtggtgatccacgaaaacaacgtggaaaacatgacccgggatctgaaactggcgtgatggaaagctggttaattcctgcggcaccggtcacggtcgttgaagagatcaaaaagagccgcttcataacgatgttggcgcataccgatggcgttgaggcggcgaaagcgtttgttgaatcggtgcgggcagaacaccccgatgcccggcaccattgcgtggcgtgggtcgcgggtgcgccggatgattctcaacagctgggtttctctgacgacggggagccggcgggaacggcaggtaaaccgatgctcgcccagctaatgggcagcggcgtcggggaaattaccgctgtggtagtgcgctactacggcggcatattgcttggcaccggtgggttagtgaaagcgtatggcggcggcgtgaatcaggcgctgcgccagctaacgacccaacgcaagacgccattaaccgaatatactttgcaatgtgaatatcatcagttaaccggcattgaagcgttgctggggcagtgtgacggcaaaattatcaacagtgattatcaggcattcgttctgctgcgggtggcgcttccggcggcgaaagtggctgaattttccgcaaagctggcggattttagccgtggttcattgcaattgttagcgattgaagaataatccccacttcgttttgcagaactaaggaagcggcagagatgcattttcgcgccattacccgaatcgttggactactggtcatcttattttcagggaccatgattatccctgggctggtagcactcatctaccgggatggagcgggccgcgcttttacccagaccttttttgtcgccctcgccattggctctatgctgtggtggccgaaccgcaaagagaaaggcgaacttaaatcccgtgaggggtttctgatagtggtgctgttctggaccgtgctgggtagcgtcggtgcgctcccttttatcttctcggaaagcccgaacctcacgattaccgatgcgttttttgaatctttctctggcctgaccactacgggagccactacgctggtggggctggattcgctccctcacgccatcctcttttatcgccagatgctgcaatggtttggcgggatggggatcatcgtgttggcggttgcgatactgcctatcctcggcgtgggtgggatgcagctctatcgcgcagaaatgcccggcccgctgaaagataacaaaatgcgcccgcgaattgcggaaacggcgaaaaccctgtggttgatttatgtcttgctgaccgtcgcctgtgcgctggcgttgtggtttgccggaatggatgcctttgatgccatcggccatagctttgcgactatcgctattggcggcttctcgacacatgatgccagtatcggttatttcgatagcccgactattaacactatcattgctatcttcctgctgatctccggctgtaactacggtctgcacttttcactgttaagtgggcgtagtctgaaggtttattggcgcgatccggaatttcgcatgtttatcggcgtacagtttacgctggtggttatttgtaccctcgtactgtggtttcataatgtctacagttcggcgctgatgacaattaaccaggcgtttttccaggtggtgtcgatggcgacaaccgccgggtttacaactgacagcattgcccgctggccgctctttttgccggtactgcttttatgttcagcctttatcggcggttgcgccgggtcaacgggcggtggcctgaaggtgatccgcatcctgctgctgtttaagcaggggaaccgtgagctgaaacgactggtgcatccgaacgccgtctatagcattaagctggggaatcgcgcactgccggaacgtatcctcgaagccgtttggggatttttctccgcctatgcattggtgtttattgtcagtatgctggcgattatcgccacgggcgtggatgacttttctgcctttgcgtcggttgttgcgacattgaataacctggggccagggcttggcgtggttgctgataactttaccagtatgaacccggtggctaaatggatcctgattgccaacatgctgtttggtcgtctcgaggtctttacattgctggtgctctttaccccgactttctggcgtgaatgatggagtaatacgtgaaaacattaattcttttctcaacaagggacggacaaacgcgcgagattgcctcctacctggcttcggaactgaaagaactggggatccaggcggatgtcgccaatgtgcaccgcattgaagaaccacagtgggaaaactatgaccgtgtggtcattggtgcttctattcgctatggtcactaccattcagcgttccaggaatttgtcaaaaaacatgcgacgcggctgaattcgatgccgagcgccttttactccgtgaatctggtggcgcgcaaaccggagaagcgtactccacagaccaacagctacgcgcgcaagtttctgatgaactcgcaatggcgtcccgatcgctgcgcggtcattgccggggcgctgcgttacccacgttatcgctggtacgaccgttttatgatcaagctgattatgaagatgtcaggcggtgaaacggatacgcgcaaagaagttgtctataccgattgggagcaggtggcgaatttcgcccgagaaatcgcccatttaaccgacaaaccgacgctgaaataagcataaagaataaaaaatgcgcggtcagaaaattattttaaatttcctcttgtcaggccggaataactccctataatgcgccaccactgacacggaacaacggcaaacacgccgccgggtcagcggggttctcctgagaactccggcagagaaagcaaaaataaatgcttgactctgtagcgggaaggcgtattatgcacaccccgcgccgctgagaaaaagcgaagcggcactgctctttaacaatttatcagacaatctgtgtgggcactcgaagatacggattcttaacgtcgcaagacgaaaaatgaataccaagtctcaagagtgaacacgtaattcattacgaagtttaattctttgagcgtcaaacttttaaattgaagagtttgatcatggctcagattgaacgctggcggcaggcctaacacatgcaagtcgaacggtaacaggaagaagcttgcttctttgctgacgagtggcggacgggtgagtaatgtctgggaaactgcctgatggagggggataactactggaaacggtagctaataccgcataacgtcgcaagaccaaagaggggtaccttcgggcctcttgccatcggatgtgcccagatgggattagctagtaggtggggtaacggctcacctaggcgacgatccctagctggtctgagaggatgaccagccacactggaactgagacacggtccagactcctacgggaggcagcagtggggaatattgcacaatgggcgcaagcctgatgcagccatgccgcgtgtatgaagaaggccttcgggttgtaaagtactttcagcggggaggaagggagtaaagttaatacctttgctcattgacgttacccgcagaagaagcaccggctaactccgtgccagcagccgcggtaatacggagggtgcaagcgttaatcggaattactgggcgtaaagcgcacgcaggcggtttgttaagtcagatgtgaaatccccgggctcaacctgggaactgcatctgatactggcaagcttgagtctcgtagaggggggtagaattccaggtgtagcggtgaaatgcgtagagatctggaggaataccggtggcgaaggcggccccctggacgaagactgacgctcaggtgcgaaagcgtggggagcaaacaggattagataccctggtagtccacgccgtaaacgatgtcgacttggaggttgtgcccttgaggcgtggcttccggagctaacgcgttaagtcgaccgcctggggagtacggccgcaaggttaaaactcaaatgaattgacgggggcccgcacaagcggtggagcatgtggtttaattcgatgcaacgcgaagaaccttacctggtcttgacatccacggaagttttcagagatgagaatgtgccttcgggaaccgtgagacaggtgctgcatggctgtcgtcagctcgtgttgtgaaatgttgggttaagtcccgcaacgagcgcaacccttatcctttgttgccagcggtccggccgggaactcaaaggagactgccagtgataaactggaggaaggtggggatgacgtcaagtcatcatggcccttacgaccagggctacacacgtgctacaatggcgcatacaaagagaagcgacctcgcgagagcaagcggacctcataaagtgcgtcgtagtccggattggagtctgcaactcgactccatgaagtcggaatcgctagtaatcgtggatcagaatgccacggtgaatacgttcccgggccttgtacacaccgcccgtcacaccatgggagtgggttgcaaaagaagtaggtagcttaaccttcgggagggcgcttaccactttgtgattcatgactggggtgaagtcgtaacaaggtaaccgtaggggaacctgcggttggatcacctccttaccttaaagaagcgttctttgaagtgctcacacagattgtctgatgaaaatgagcagtaaaacctctacaggcttgtagctcaggtggttagagcgcacccctgataagggtgaggtcggtggttcaagtccactcaggcctaccaaatttgcacggcaaatttgaagaggttttaactacatgttatggggctatagctcagctgggagagcgcctgctttgcacgcaggaggtctgcggttcgatcccgcatagctccaccatctctgtagtgattaaataaaaaatacttcagagtgtacctgcaaaggttcactgcgaagttttgctctttaaaaatctggatcaagctgaaaattgaaacactgaacaacgaaagttgttcgtgagtctctcaaattttcgcaacacgatgatgaatcgaaagaaacatcttcgggttgtgaggttaagcgactaagcgtacacggtggatgccctggcagtcagaggcgatgaaggacgtgctaatctgcgataagcgtcggtaaggtgatatgaaccgttataaccggcgatttccgaatggggaaacccagtgtgtttcgacacactatcattaactgaatccataggttaatgaggcgaaccgggggaactgaaacatctaagtaccccgaggaaaagaaatcaaccgagattcccccagtagcggcgagcgaacggggagcagcccagagcctgaatcagtgtgtgtgttagtggaagcgtctggaaaggcgtgcgatacagggtgacagccccgtacacaaaaatgcacatgctgtgagctcgatgagtagggcgggacacgtggtatcctgtctgaatatggggggaccatcctccaaggctaaatactcctgactgaccgatagtgaaccagtaccgtgagggaaaggcgaaaagaaccccggcgaggggagtgaaaaagaacctgaaaccgtgtacgtacaagcagtgggagcacgcttaggcgtgtgactgcgtaccttttgtataatgggtcagcgacttatattctgtagcaaggttaaccgaataggggagccgaagggaaaccgagtcttaactgggcgttaagttgcagggtatagacccgaaacccggtgatctagccatgggcaggttgaaggttgggtaacactaactggaggaccgaaccgactaatgttgaaaaattagcggatgacttgtggctgggggtgaaaggccaatcaaaccgggagatagctggttctccccgaaagctatttaggtagcgcctcgtgaattcatctccgggggtagagcactgtttcggcaagggggtcatcccgacttaccaacccgatgcaaactgcgaataccggagaatgttatcacgggagacacacggcgggtgctaacgtccgtcgtgaagagggaaacaacccagaccgccagctaaggtcccaaagtcatggttaagtgggaaacgatgtgggaaggcccagacagccaggatgttggcttagaagcagccatcatttaaagaaagcgtaatagctcactggtcgagtcggcctgcgcggaagatgtaacggggctaaaccatgcaccgaagctgcggcagcgacactatgtgttgttgggtaggggagcgttctgtaagcctgtgaaggtgtgctgtgaggcatgctggaggtatcagaagtgcgaatgctgacataagtaacgataaagcgggtgaaaagcccgctcgccggaagaccaagggttcctgtccaacgttaatcggggcagggtgagtcgacccctaaggcgaggccgaaaggcgtagtcgatgggaaacaggttaatattcctgtacttggtgttactgcgaaggggggacggagaaggctatgttggccgggcgacggttgtcccggtttaagcgtgtaggctggttttccaggcaaatccggaaaatcaaggctgaggcgtgatgacgaggcactacggtgctgaagcaacaaatgccctgcttccaggaaaagcctctaagcatcaggtaacatcaaatcgtaccccaaaccgacacaggtggtcaggtagagaataccaaggcgcttgagagaactcgggtgaaggaactaggcaaaatggtgccgtaacttcgggagaaggcacgctgatatgtaggtgaagcgacttgctcgtggagctgaaatcagtcgaagataccagctggctgcaactgtttattaaaaacacagcactgtgcaaacacgaaagtggacgtatacggtgtgacgcctgcccggtgccggaaggttaattgatggggttagccgcaaggcgaagctcttgatcgaagccccggtaaacggcggccgtaactataacggtcctaaggtagcgaaattccttgtcgggtaagttccgacctgcacgaatggcgtaatgatggccaggctgtctccacccgagactcagtgaaattgaactcgctgtgaagatgcagtgtacccgcggcaagacggaaagaccccgtgaacctttactatagcttgacactgaacattgagccttgatgtgtaggataggtgggaggctttgaagtgtggacgccagtctgcatggagccgaccttgaaataccaccctttaatgtttgatgttctaacgttgacccgtaatccgggttgcggacagtgtctggtgggtagtttgactggggcggtctcctcctaaagagtaacggaggagcacgaaggttggctaatcctggtcggacatcaggaggttagtgcaatggcataagccagcttgactgcgagcgtgacggcgcgagcaggtgcgaaagcaggtcatagtgatccggtggttctgaatggaagggccatcgctcaacggataaaaggtactccggggataacaggctgataccgcccaagagttcatatcgacggcggtgtttggcacctcgatgtcggctcatcacatcctggggctgaagtaggtcccaagggtatggctgttcgccatttaaagtggtacgcgagctgggtttagaacgtcgtgagacagttcggtccctatctgccgtgggcgctggagaactgaggggggctgctcctagtacgagaggaccggagtggacgcatcactggtgttcgggttgtcatgccaatggcactgcccggtagctaaatgcggaagagataagtgctgaaagcatctaagcacgaaacttgccccgagatgagttctccctgactccttgagagtcctgaaggaacgttgaagacgacgacgttgataggccgggtgtgtaagcgcagcgatgcgttgagctaaccggtactaatgaaccgtgaggcttaaccttacaacgccgaaggtgttttggcggattgagagaagattttcagcctgatacagattaaatcagaacgcagaagcggtctgataaaacagaatttgcctggcggcagtagcgcggtggtcccacctgaccccatgccgaactcagaagtgaaacgccgtagcgccgatggtagtgtggggtctcctcatgcgagagtagggaactgccaggcatcaaataaaacgaaaggctcagtcggaagactgggcctttcgttttatctgttgtttgtcggtgaacgctctcctgagtaggacaaatccgccgggagcggatttgaacgttgcgaagcaacggcccggagggtggcgggcaggacgcccgccataaactgccaggcatcaaattaagcagaaggccatcctgacggatggcctttttgcattggcgcagaaaaaaatgccggatgcgacgctggcgcgtcttatccagcctactcttgcttatccgttctgcttttgcatccactccaccacaaaatcagccagcccctcaacatcattaatatccagtaatgcgacatcaagattaagcggcacatcactggctacagcaataacatgcctgtctatcactaattcttcaggtcgatgtccggctccatcgcgaaacagcacaatctttgcgatctcttcatgcttaaacccttcgaccagaatcaaatccagctttgaggtatccattcgacttgcgagaaactgtagatccagctcttcttcgtctggtgtttccgtcatcaaggcccatcgttgctggctggcaacgatggtttgtgccgcgccagccttgcgcagctcatagctatctttgcctggcttatcaacatccatatcatggtgcgtatgcttaatcagccctggacggatccctctggcgcataatgccgggatcagttttttcaaaagcgtagtttttccggtaccactccacgcggcaaaggcgagtaacggtatcatcgtttttcctgccatcgggcaagctcctctggcgtattcacgttaacaaatgcatctttatgatcgctgaaatcaaccgcatgaccgccagccagacgcataaataccattacccggcgttctcctgcttgcagatattccagtaataaaggctcaatagcgcggtttaccagagcaatagtcgggtgatcgcgttcaccgtcatggacccacacgacaggcgcatctttgcgctgatgattaagcctggctgctaaatcagggggaatgtaaggcgtatcgcacgggcaaaacaaaaaccactcaccagcttcctgctgcattactgaaagcattcctgccagagggcctgggtaatccgccagtgaatcttcaatcactttcagaccgcttgcctgatagatttcctgatgacgattagcattaaccacgacgtgagagagctgcgtcataagcgcgtcagcgacatgttgccataatggtttgccgtttaattcaagcaatcctttatctacgccgcccattcgtctggctttaccgcctgccagcacaacgcctgttatcgtcgtcatcagattcaccgatatcgcctcttttattgtgggattgaccctgctaacgtgtctgtctcaagagtaaggagcatcactatgaaatgtaaacgtctgaatgaagttattgaactcctccagccagcctggcaaaaagagccagaccttaacctgctgcaatttttgcagaaactggcgaaagagtcaggttttgacggcgaactggcggatttgacggatgacattctgatctatcacctgaaaatgcgtgattccgcgaaagatgcggtgatcccgggtttgcagaaagattatgaagaagacttcaaaacggcgctgttacgcgctcgcggcgtaattaaagagtaaaagcttgtaagcggcgccaccaaaatcatcgtgaaatgatatccttcgtcattcgtaatgttttccggatgatgggatgaataacagcgcttttactttccagacactacacccggataccatcatggacgctctgtttgagcatgggatccgggtggattccggtcttaccccgcttaacagctatgaaaaccgtgtctatcaatttcaggacgaagatcgtcgacgttttgtcgtcaaattttatcgccctgaacgttggacagccgatcaaatcctcgaagaacatcaatttgcgttgcagctggtaaatgatgaagttccggtcgcagcacctgtggcctttaacggtcagactttattgaatcatcagggattttatttcgctgtttttccaagcgtcggtggtcgccagttcgaagctgataatatcgatcagatggaagcggttgggcgttatttagggcgtatgcaccagacggggcgcaaacagctttttatccatcgcccgaccatcggtttgaacgaatatctcattgagccacgcaagctgtttgaggacgctacactgataccttccgggttgaaagcggcattcctgaaagcgacagatgagctgattgccgccgttacagcacactggcgggaagatttcaccgttctgcggctacatggagactgccacgccgggaatattctctggcgcgatggtccaatgtttgttgatctggatgatgcacgtaatggtccagccgttcaggatttgtggatgttgctcaatggcgataaagccgagcagcggatgcaactggaaactattattgaagcttatgaagaatttagcgagttcgacaccgctgaaatcggactgattgaacctttacgcgccatgcgtttggtttattatcttgcctggctaatgcggcgttgggctgatcccgcgttcccgaaaaatttcccgtggttaaccggggaagattactggctgcgacagacggcgacttttatagaacaggcaaaagttctacaagaaccccctttgcaattaacacctatgtattaatcggagagagtagatcatgaaaaagatttggctggcgctggctggtttagttttagcgtttagcgcatcggcggcgcagtatgaagatggtaaacagtacactaccctggaaaaaccggtagctggcgcgccgcaagtgctggagtttttctctttcttctgcccgcactgctatcagtttgaagaagttctgcatatttctgataatgtgaagaaaaaactgccggaaggcgtgaagatgactaaataccacgtcaacttcatgggtggtgacctgggcaaagatctgactcaggcatgggctgtggcgatggcgctgggcgtggaagacaaagtgactgttccgctgtttgaaggcgtacagaaaacccagaccattcgttctgcttctgatatccgcgatgtatttatcaacgcaggtattaaaggtgaagagtacgacgcggcgtggaacagcttcgtggtgaaatctctggtcgctcagcaggaaaaagctgcagctgacgtgcaattgcgtggcgttccggcgatgtttgttaacggtaaatatcagctgaatccgcagggtatggataccagcaatatggatgtttttgttcagcagtatgctgatacagtgaaatatctgtccgagaaaaaataattcaatgtaaattacataaagcccgtgaatattcacgggctttttttattatttaataaatataaatacattctgataatgcatcctgccgctggacattatttcagcataagtggatattcaaagttttgctgttttatcagggaatatttatatgatacgtaagtcagctacaggtgttattgttgcgttagccgtaatctggggtggtggcacatggtacacaggtacgcaaattcagcctggtgtcgaaaaatttattaaagattttaacgatgctaaaaagaaaggtgaacatgcctacgatatgacgttaagttatcaaaattttgacaaaggcttttttaattcccgttttcaaatgcaaatgacattcgataacggtgcacccgatctcaatatcaagccaggccagaaagttgtatttgatgtggatgttgagcacggtccgttgcccatcacaatgttaatgcatggtaatgtcatcccagcactggcagcggcaaaagtgaacttagtgaataatgaactgacacaaccgctatttatcgccgcgaaaaataaatcgcccgtggaagcgacattgcgattcgcgtttggtggctcattctctacgacattagatgttgcccctgcagagtatggaaagttttcttttggtgagggccagtttacttttaatggtgatggtagttcattgtctaacctggatattgaaggcaaagtcgaagatattgttctgcaattatcaccaatgaacaaagtaacggcaaaaagttttaccattgattctctggcgcgattagaagaaaagaaatttccggttggtgaaagcgagtcgaaatttaatcagattaacattatcaatcacggggaagacgttgcccaaatcgatgctttcgttgcaaaaaccaggctggatcgcgttaaagacaaagattatatcaatgtcaatctcacctacgaacttgataagttaacaaaagggaatcagcaactcggtagtggtgagtggtcattgattgctgaatctattgatccctcagcagtgcgccaatttatcatccagtataacattgcgatgcagaagcagcttgctgcacaccctgagttagcaaacgatgaagttgctctgcaagaagtgaatgctgcattgttcaaagagtatttaccgttattacaaaaaagtgagccgaccattaaacaaccggtaagatggaagaacgcactcggcgaactaaatgccaatctggatatcagtattgccgacccagccaaatcttcatcatccacaaacaaagatatcaaatcgctcaattttgatgtgaagttaccgcttaatgtcgtcacagaaaccgcaaaacagcttaatttatctgaaggaatggatgcggaaaaagcgcaaaagcaggctgataaacaaatcagcgggatgatgacattaggtcagatgtttcagttaatcacgattgacaacaataccgcctcgctgcagctgcgttatacaccgggtaaagttgtttttaacggacaggagatgagcgaagaagaatttatgtctcgtgccggacgttttgttcattaaaatactcactcgcctctgctcattcagaggcgagtaaaacttacttattctgacgctgtgatgacatgagagacgtcagaagccggtctttttcctgccacaatgagttcagccattgctgaaaatggcgcttaaagcttttgtcattgatgtagtcgccatgtaactcatcggcaataggctgtaaatccacatgtacgacaatccgcgtcagtttaccgcttaacatatcgaagaacggctgacggttattgtccggataacacagcgtaacattaagcagtttatcgaattgtttacccagtacatttagcgccatcgcaatgcctgccgcctttggtggcaacaagttttgaaaagtggagtgggtttgctgatgtttttcttgcgtgaaacgggagccttcaacgaaattgacaatggtggtgggatgcaggcgaaacttttcacaagaacgccgagtggtttcaacatctttaccacgtcgctccggatgacgtaataaataagcgcgggaataacgcttcataaacggcatatccagcgaccagcacgccaggccaagaaatggcacccaggccagctgttgcttgaggaaatatttattcatcggaatgtgcttacgaaacagcacgcacagtacgacaatatctgcccaactacggtggttacaaataagcagataccagttcttcttacttaacccttccagcccgtgaacttcccattgaaggtgtgggttcagatgcagtaataccgccagaccttcacaccagcaatacatcataaaatcacaaaaacgcgaaacctttcgccaaatgactggcacaggtagcaatagttttacaatcccggcaatgatgatcgggacggaacaaaaaatagtgaccaaaatggtcaatacgatactcagcaaaagggttatcgcagcgagtattctcgtcataatgaatttattcaaaaggttagccatagacagtgcgctaaagaagcgcaaggcgcagattttagcagaaaacgacccaaataacggatgatccttaaggagaaaaataattcatatctatccacattagaaaaaatcccattatctcaattattagggatggatttatttttaactgcatgaaaaacaaagacaaacatcatgctgtaaaaagcatgataataaattaaaagcgatgtaaataatttatgcacaaagttatccacatgacgatttgcgagcgatccagaagatctacaaaagattttcacgaaaagcggtgaaaaactcatgttttcatcctgtctgtggcatcctttacccataatctgataaacaggcacggacattatggttcagatcccccaaaatccacttatccttgtagatggttcatcttatctttatcgcgcatatcacgcgtttcccccgctgactaacagcgcaggcgagccgaccggtgcgatgtatggtgtcctcaacatgctgcgcagtctgatcatgcaatataaaccgacgcatgcagcggtggtctttgacgccaagggaaaaacctttcgtgatgaactgtttgaacattacaaatcacatcgcccgccaatgccggacgatctgcgtgcacaaatcgaacccttgcacgcgatggttaaagcgatgggactgccgctgctggcggtttctggcgtagaagcggacgacgttatcggtactctggcgcgcgaagccgaaaaagccgggcgtccggtgctgatcagcactggcgataaagatatggcgcagctggtgacgccaaatattacgcttatcaataccatgacgaataccatcctcggaccggaagaggtggtgaataagtacggcgtgccgccagaactgatcatcgatttcctggcgctgatgggtgactcctctgataacattcctggcgtaccgggcgtcggtgaaaaaaccgcgcaggcattgctgcaaggtcttggcggactggatacgctgtatgccgagccagaaaaaattgctgggttgagcttccgtggcgcgaaaacaatggcagcgaagctcgagcaaaacaaagaagttgcttatctctcataccagctggcgacgattaaaaccgacgttgaactggagctgacctgtgaacaactggaagtgcagcaaccggcagcggaagagttgttggggctgttcaaaaagtatgagttcaaacgctggactgctgatgtcgaagcgggcaaatggttacaggccaaaggggcaaaaccagccgcgaagccacaggaaaccagtgttgcagacgaagcaccagaagtgacggcaacggtgatttcttatgacaactacgtcaccatccttgatgaagaaacactgaaagcgtggattgcgaagctggaaaaagcgccggtatttgcatttgataccgaaaccgacagccttgataacatctctgctaacctggtcgggctttcttttgctatcgagccaggcgtagcggcatatattccggttgctcatgattatcttgatgcgcccgatcaaatctctcgcgagcgtgcactcgagttgctaaaaccgctgctggaagatgaaaaggcgctgaaggtcgggcaaaacctgaaatacgatcgcggtattctggcgaactacggcattgaactgcgtgggattgcgtttgataccatgctggagtcctacattctcaatagcgttgccgggcgtcacgatatggacagcctcgcggaacgttggttgaagcacaaaaccatcacttttgaagagattgctggtaaaggcaaaaatcaactgacctttaaccagattgccctcgaagaagccggacgttacgccgccgaagatgcagatgtcaccttgcagttgcatctgaaaatgtggccggatctgcaaaaacacaaagggccgttgaacgtcttcgagaatatcgaaatgccgctggtgccggtgctttcacgcattgaacgtaacggtgtgaagatcgatccgaaagtgctgcacaatcattctgaagagctcacccttcgtctggctgagctggaaaagaaagcgcatgaaattgcaggtgaggaatttaacctttcttccaccaagcagttacaaaccattctctttgaaaaacagggcattaaaccgctgaagaaaacgccgggtggcgcgccgtcaacgtcggaagaggtactggaagaactggcgctggactatccgttgccaaaagtgattctggagtatcgtggtctggcgaagctgaaatcgacctacaccgacaagctgccgctgatgatcaacccgaaaaccgggcgtgtgcatacctcttatcaccaggcagtaactgcaacgggacgtttatcgtcaaccgatcctaacctgcaaaacattccggtgcgtaacgaagaaggtcgtcgtatccgccaggcgtttattgcgccagaggattatgtgattgtctcagcggactactcgcagattgaactgcgcattatggcgcatctttcgcgtgacaaaggcttgctgaccgcattcgcggaaggaaaagatatccaccgggcaacggcggcagaagtgtttggtttgccactggaaaccgtcaccagcgagcaacgccgtagcgcgaaagcgatcaactttggtctgatttatggcatgagtgctttcggtctggcgcggcaattgaacattccacgtaaagaagcgcagaagtacatggacctttacttcgaacgctaccctggcgtgctggagtatatggaacgcacccgtgctcaggcgaaagagcagggctacgttgaaacgctggacggacgccgtctgtatctgccggatatcaaatccagcaatggtgctcgtcgtgcagcggctgaacgtgcagccattaacgcgccaatgcagggaaccgccgccgacattatcaaacgggcgatgattgccgttgatgcgtggttacaggctgagcaaccgcgtgtacgtatgatcatgcaggtacacgatgaactggtatttgaagttcataaagatgatgttgatgccgtcgcgaagcagattcatcaactgatggaaaactgtacccgtctggatgtgccgttgctggtggaagtggggagtggcgaaaactgggatcaggcgcactaagattcgcctgaacatgccttttttcgtaagtaagcaacataagctgtcacgttttgtgatggctattagaaattcctatgcaacaactgaaaaaaaattacaaaaagtgctttctgaactgaacaaaaaagagtaaagttagtcgcgtagggtacagaggtaagatgttctatctttcagaccttttacttcacgtaatcggatttggctgaatattttagccgccccagtcagtaatgactggggcgttttttattgggcgaaagaaaagatccgtaatgcctgatgcgctatgtttatcaggccaacggtagaattgtaatctattgaatttacgggccggatacgccacatccggcacaagcattaaggcaagaaaattattcgccgtcctgcgtttcttctacaggctgcatctcgctaaaccaggtatccagtttctgccgcagcttgtccacgccttgtttcttcaacgaagaaaacgtttcaacctgcacatcaccgttaaacgccagtacagcttcacgcaccatattcaattgcgctttacgtgcgccgcttgccagtttgtccgctttggtcagcagcaccagaacggcgatattgctgtctaccgcccactcaatcatctgctgatccaaatctttcagcggatggcgaatatccattagcaccaccagaccttgcaggctctgacgtttttcgaggtattcgccgagcgcacgctgccatttgcgcttcatctcttccgggacttccgcataaccgtacccaggcaagtcaaccagacgcttgccgtcagccacttcaaacaggttgataagctgggtgcgccctggggtttttgaggtacgagccaggcttttctggttagtcagcgtgttcagcgcgctggatttacctgcgttggaacggcctgcaaaagccacttcaattccggtatcggaaggtaggtggcgaatatcaggcgcactcatcacaaaatgcgtctgttgataattcaaattagtcaaagcggtcgtctccgtcagtcaaagctttgtggcgattatacctgaaccataataaaaggcggatttttcggcgtgagcgttgtaagtaaaagccatacgctttgtgagacattgccgatagtctttatgcgaaatagcagagaaaattctgcgatgcatgtcaaataagctatataaatcagtgaattgcttttatataaaactctgaaaatgtgcaaatactgatggcggttgattgtttgtttaaagcaaaggcgtaaagtagcacccatagagcgaggacgctaacaggaacaatgactcaggatgagggtcaggagcgccaggaggcgaagacagaggattgtcaggaagacaaacgtccggagacgtaattaaacggaaatggaatcaacacggattgttccggctaaaggaaaaacagggtgtgttggcggcctgcaaggattgtaagacccgttaagggttatgagtcaggaaaaaaggcgacagagtaatctgtcgccttttttctttgcttgctttctgttagattccgccgcaaatctatactgaataaaacggctaaaagacgaaccattatgaaaccatcatcttcaaactcacgcagcaaaggtcatgcaaaagcgcgtcgaaaaacacgcgaggagctggatcaggaagctcgtgatcgcaagcgtcagaaaaaacgtcgtggtcatgcgccgggcagccgcgcagcgggcggaaacaccacgtcaggcagcaaaggccagaacgcaccaaaagatccacgtattggcagtaaaacccctattccattgggcgtgactgaaaaagtcaccaaacagcacaaaccgaagagtgagaaacctatgctttcaccgcaggcggagttggaattactggaaacggatgagcgtctggatgcgctgctggaacgtctggaagcaggcgaaaccctgagtgccgaagagcaatcctgggtggatgctaaactggatcgtattgatgagttgatgcagaaactcggcctctcttatgacgatgacgaagaagaggaagaagacgagaagcaagaagacatgatgcgtctgctgcggggcaactaacggattgccgccgtgggccttcccgttctgctgataacccttccggttatatgttatctggtgtggttattcgttaaactacagcggttgtcgcggcgacaaaagtggctgcgcaaccggctgatgacccgaaacgggcatccgccggtacgccgtagccgccagagacgccatcggaaggagtgagcatgtctgtacagcaaatcgactgggatctggccctgatccagaaatataactattccgggccacgatacacctcgtacccgaccgcgctggagttttcagaagacttcggcgaacaggcgtttttacaagccgtggcgcgctatcctgagcgtccattatctctctacgtacatatcccgttctgccataagctttgttacttctgcggttgcaataagattgttactcgccagcagcacaaggccgatcagtatctggacgcgctggagcaagaaatcgtccatcgtgcaccgctgttcgccgggcgtcacgtcagccaattgcactggggcggcggaacgccgacgtatctgaataaagcgcaaatcagccgcctgatgaagctgctgcgcgaaaacttccagttcaatgccgatgcggagatttcgatcgaagtcgatccgcgggaaatcgaactggatgtactcgatcatttacgcgccgaaggctttaatcgcctgagcatgggcgtgcaggacttcaacaaagaagtgcaacgtctggttaaccgcgagcaggatgaagagttcatctttgcactgcttaaccatgcgcgtgagattggttttacctccaccaacatcgacctgatttacggcctgccgaaacagacgccggagagtttcgcctttaccctgaaacgtgtggcggagctgaaccccgatcgtctgagtgtctttaactacgcgcatctgccgaccatttttgctgctcagcgcaaaatcaaagatgctgacctgccgagtccgcagcaaaaactcgatatcctgcaggaaaccatcgccttcctgacgcaatcgggctatcagtttatcggtatggatcactttgcccgtccggatgacgagctggcggtggcccagcgtgaaggcgtgctgcatcgtaacttccagggctacaccactcagggcgataccgatctgctggggatgggcgtttccgccatcagcatgattggcgactgctacgcgcagaaccagaaagagttgaagcagtactatcagcaagtggatgaacaaggcaatgcgctgtggcgtggtattgcgctaacgcgtgatgactgtattcgccgcgatgtgattaagtcgctcatctgcaacttccgtctggattacgcccctattgagaaacagtgggatttgcacttcgctgattactttgcggaagatctcaagctgctcgccccgttagcaaaagatgggctggtggatgtggatgagaagggaatacaggtgacggcgaaaggtcgcttgctgatccgcaacatttgcatgtgctttgatacctatctgcgccagaaagcgcggatgcagcagttctctcgggtgatttaaatagtgaatggcgcttcgtttacaaagtagaaaacgaaagcgccatcaatgtgctgagaacaagattgcctgatgcgctgggcaacaaaacctgttgaaattattgcttttgtaggccggataaggcgtttacgccgcatcaggcatctgagcatgatgcctgatgcggcgctggtcgcgtcttatcaggcctacgactttctccgcatccggcataaacaacgagcttcagctaaacagcccaatcattgcggcacacagcacggcagcaacggcagtttgcggtgtgtggctgtcaactgcgccactcgataccagattaattattgattccagcataatgactctccccgttttccgggcaagatcatactgaacttatcggaacagtaaagcgtaaaataccagcaatttgcgctcaataatcaatctttacacacaagctgtgaatcactccatccccagctcttttaacttacgcgtcagggtgttgcggccccagccgagtagccgcgccgcttcctgtttatgcccctgcgtatgtcgcaacgcggtcgtcagtaacgtccgctccagctctggctgcgcttcggaaagcagattttgatgaccggaacgcagcgctctgtctgcccactgcgcaagaagcgtcgcccagctgtccggttgcatttgcgaagtactctccgcaaccgttgattcaaacagttcgccgggcaaatcctgaatcaacacttcctgcccggcggccatcaccgttagccagcggcaggtgttttccagctggcgcacgttgcctggccacgccagacgcgtcagagcagcttcggtttccggatgcagtaacttcgcttctacgcccagttcgcgcgcggcaacctgtaaaaaatggcgcgccagacggggaatatcttcccgacgttcgcgcagcggcggcagatgaacgcggataacgttcaggcggtggaacagatcctcacggaacttaccttcctgcactcgctgttcgagattctggtgagtggcagcgataatccgcacatccactttcaccggcgcatagccgccaacgcggtaaaactgaccgtctgccagcacgcgcagcaaacgcgtctgcacatccagcggcatatcaccaatttcgtcgaggaataatgtaccgccatcggcctgttcaaaacgcccctgacgaatggtattcgcgccagtaaacgcgcctttctcgtggccaaacagttctgattcgatcaaatcttttgggatagctgccatattcagcgcgataaacggcgctttggcgcgcggactgtggcgatgcagggcatgagcgaccagttctttaccggtgccggattcgccgttaatcagcacgctaatagaagaacgcgaaagccgaccgataatacggaacacgtcctgcatggctggcgcttcgccgatgatatcggtcgttgggccgttaagctgaacattacgcggctgctgctgttcctggtaatgactgatagcgcgctcaaccagcgccactgcttcgtcgatatcaaacggtttgggcagataatcaaacgccccttgttgataggcgctgacggcagcatccagatcggaatgtgcggtcataatgatgaccggaagcattggatggcgctgtttaatctgcttgagcagcgccagcccgtccattcccggcatacggatatctgaaagcagcacatccggcgttttgctcgccagcgcctccagcacttctgcgccgttctcaaacgtcgtacaggttaaacctgccccagcgagcgcacgttcaagcacccaacggatggaactatcgtcatcgactacccagactatccctcgttgcataaacgtcacctttatttcctgataggcaggtaaaccgagaactcggtatgccctggccaactggtaaattcaattttgcctgaatgctgatcaatcaaattacgagcgatggataagccaagcccggtgccaccttcgcggccgctgaccatcgggtaaaacagcgtatcctgcaaatgaggcggaatgcccggcccgttatcttccacatcaatccgcgccgccagccggtagcgctcgccgtgtaaggtcagttgaaacgcggtgcgggtacgcagaatgatttcaccgccttccggccccagcgcctgtagcgcattgcgcacaatattcagcaagacctgttcaatttgatccgggtcgtgcgccagttccggtaggctgggatcgtaatcacgaatcaaccgcacgttgtccggcagttccatcgacaccagcgttaccacgcgttcagccactttgtgaatactttcggtaacgcgcgtaccgggcagctgcggccccaacagacggtcgaccagatttcgcagccggtccgcctgttcgataatcactttggtatattcgagtagtgatgggtcaggtaacgctttgctgagcagctgcgccgcgccacgtaaaccgccaagcggatttttaatctcatgtgccaggccgcgcactaaatcacgggcagcaacctgctgggcgtgctgtagctgttcctgacttaagcggcgctggttatccatcggagccatctccagcaggatcatgccgtccggcatacgctgggccgtcacagaaaggatatgcgagcgcccgtcgatgaccagcgtcacttcgttatcggtaaaaccttgccccgcctccagactttcttgcatcagctcgatatttaatgagaagtagctcaacagttccggtaacggtgtaccaaacaatttgcgggagctttgggcgagcagttgttgcgcggcagggttggcgtaatggatcgccaggttgtcatcgattaacaaaatactgttaatcagcgagttgaggatctgcccagcatcgggctgcgtgcctgttgccataaagcagtctcctgaacaggttgcaccattttagtgcattatagctttttacggataaaaagcgcgaagcatcagagaattgacggagaaaaaagcccatgcagagatgggctacagatagctgacaaacttcacgttggagagcgactcacctgctccggcctaccacatcatcaccgtgtaggccggataagacgcatttgcgtcgcatccggcgtgatgtgcttgccaccgatcccaggcctgccagagacaggcgaaaagtttccacggcaactaaaacacttagacgctgtagtacagctcaaactctaccggatgcggagtcatacgcacgcggtcatcttcttcgcgacgcagagcgatgtacgcatcaattgcttcgtcagtgaacacgccaccggctttcaggaactcgcggtccagatccagttcgttcagtgcttcttccagagagcctgcaacctgtgggatctctttcgcttcttctggcggcaggtcatacaggtttttgtccatggcttcgcccggatggatcttgttcttgataccatcaagaccggccatcagcagggcagcaaagcacaggtacgggttagctgccggatccgggaaacgtacttcgatacgacgtgctttcggagaagaaaccaccggaatacggatagacgcagaacggttacgcgcagagtaagccagcattaccggtgcttcatagcccgggaccagacgcttataagagttggtggtcgggtttgccagggcgttaatcgctttagcgtgtttgattacgccgccaatgtagtacagcgcctgctcagacagacctgcgtatttgtcgcctgcgaacaggttaacgccgtttttagacagagacatgtggcagtgcataccggagccgttatcaccgaacatcggttttggcataaaggtcgcggttttaccgaagcggtgcgctacgttgtgcacaacatatttgtagatctgaatttcgtcagcttttttggtcatggtattgaagcgggtagccacttcgttctgaccagcagtcgctacttcgtggtgatgggcttcaaccaccagacccatctgttccatcaccagacacatttcagaacgaatatcctgagccgagtctaccggtggaaccgggaagtaaccgcctttcactgccggacggtgacctttgttaccaccttcgtattgggtggaggagttccatgcgccttcgatatcgtcgatagcaacgtgggaaccggagatagatgatccgaaacggatgtcatcgaacaggaagaattcaggttctggcccgaacagtacggtgtcggcaatgccagtggaacgcaggtaatcttcggcgcgcttcgcaatggagcgcgggtcacggtcatagccttgcagggtgccaggttcaaggatgtcgcaacggataatcagggtggagtcggcgaagaacgggtcaatcactgcggtggatgcgtctggcatcagcaccatgtcggactcgttaatgcctttccagccgccaatcgaggagccgtcaaacattttgccttcttcgaagaattcagcattcacctgatgagcagggatagtgacgtgctgttctttacctttagtatcggtgaagcgcaaatcaacaaacttcacttcgtgctcgttcagcatcgtcagtacgtgttcagcggacatactttaactctcctggattggtcatggtcgtcgtggtaacgaaatctgcaattattttggccgtgtcgccgtaaaaaagataaagcgaaatctgtgccaacttttaaattgcccctaaaaggcgttatcatgcgcaccatcgtgcaaaagggctgcaccacgatgtgaatgttgcaccaatatagtgcttcaatggaaacattaagcaccatgttggtgcaatgacctttggataaccctttttatgctccgtgaaagcgatcacaaagggactctgcaatacttgtttgcggaggatgtttgtgatcctgttttgtagtgcgattaatccgtgtacaataacgcgctatttctaatgcctgaggcaaagttgtgatcgaaaaattgcgtaatatcgccatcatcgcgcacgtagaccatggtaaaaccaccctggtagacaagctgctccaacaatccggtacgttcgactctcgtgccgaaacccaagagcgcgtgatggactccaacgatttggagaaagagcgtgggattaccatcctcgcgaaaaacaccgctatcaaatggaatgattaccgtatcaacatcgttgataccccggggcacgccgacttcggtggtgaagttgaacgtgtaatgtccatggtagactcagtgctgctggtggttgacgcatttgacggcccgatgccgcaaacgcgcttcgtaaccaaaaaagcgtttgcttacggcctgaagccgattgttgttatcaacaaagttgaccgccctggcgcgcgtcctgattgggttgtggatcaggtattcgatctgttcgttaacctcgacgcgaccgacgagcagctggacttcccgatcgtttacgcttctgcgctgaacggtatcgcgggtctggaccacgaagatatggcggaagacatgaccccgctgtaccaggcgattgttgaccacgttcctgcgccggacgttgaccttgacggtccgttccagatgcagatttctcagctcgattacaacagctatgttggcgttatcggcattggccgcatcaagcgcggtaaagtgaagccgaaccagcaggtcactatcatcgatagcgaaggcaaaacccgcaacgcgaaagtcggtaaagtgctgggccacctcggtctggaacgtatcgaaaccgatctggcggaagctggcgatatcgttgcgatcacgggccttggcgaactgaacatttctgacaccgtttgcgacacgcaaaacgttgaagcgctgccggcactctccgttgatgagccgaccgtttctatgttcttctgcgttaacacctcgccgttctgcggtaaagaaggtaagttcgtaacgtctcgtcagatcctggatcgtctgaacaaagaactggtacacaacgttgcgctgcgcgtagaagaaaccgaagacgccgatgcgttccgcgtttctggtcgtggcgaactgcacctgtctgttctgatcgaaaacatgcgtcgtgaaggtttcgaactggcggtatcccgtccgaaagttatcttccgtgaaatcgacggtcgtaaacaagagccgtatgaaaacgtgactctggacgttgaagaacagcatcagggttctgtaatgcaggcgctgggcgaacgtaaaggcgacctgaaaaacatgaatccagacggtaaaggccgcgtacgtctcgactacgtgatcccaagccgtggtctgattggcttccgttctgagttcatgaccatgacttccggtactggtctgctgtactccaccttcagccactacgacgacgtacgtccgggtgaagtgggtcagcgtcagaacggcgtactgatctctaacggtcagggtaaagcggtcgcgttcgcgctgttcggtctgcaggatcgcggtaagctgttcctcggtcacggtgcagaagtttacgaaggtcagattatcggtattcatagccgctctaacgacctgactgtaaactgcctgaccggtaagaaactgaccaacatgcgtgcttccggtactgacgaagccgttgttctggttccgcctatccgcatgactctggaacaagctctggagttcatcgatgatgacgaactggtagaagtgactccgacctctatccgtattcgtaaacgtcacctgacggaaaacgatcgtcgccgcgccaaccgcgcaccgaaagacgattaatttcgttttttagtcataaaaaacctgccagcgatggcaggtttttttttgcctgtcgtgagcgcacaccaatgcgagtatctcccttataagtctgtggttacgtcaatagagagctttgtcacaattatctgcaaagtcatacgccgttaattgctttcttttttggcgtaagcgtaagatgcttcatctggtttaaaccaaaaggattaaacaatggcggagaatcaatccaccgtagaaaatgcaaaagagaaactggatcggtggttgaaagatggcatcaccacgccgggtggaaaactcccttcagaaagagagctgggagaactgctgggcattaaacgtatgacgctgcgccaggcgttgttgaacctcgaggcagaatccaaaatcttccgtaaggatcgtaaggggtggttcgtgacccagccgcgatttaattacagtccggagctgtcggcgagctttcagcgggccgcaattgagcaagggcgagagccttcctgggggtttaccgagaaaaaccgtaccagcgatattcccgagacgctcgcgccactgattgcagtgacgccatcaactgaactctatcgcatcaccggctggggggcgctggaaggacataaagttttctatcacgaaacatatattaatcctgaagttgctccgggctttattgaacaacttgaaaaccactcattttctgcagtctgggaaaagtgctaccaaaaagagacggtagtaaaaaaattgattttcaaacccgtcagaatgccgggcgatatcagcaagtatcttggcggttctgcgggtatgccagcgatcttaattgaaaagcatcgcgccgaccagcaaggcaatattgtccaaatagatattgaatattggcgatttgaggccgtagacctcatcattaatctgtaggtgttttatggtgacaataaataacgcaagaaagattctacaacgtgtcgacactcttcctctttatttacatgcttatgcctttcatttaaatatgcggctggaaagagtgttgcctgctgatttacttgatatcgcaagtgaaaataatctacgtggcgtcaaaatccatgttctcgatggcgagcgtttttctcttggtaatatggacgataaagaactctctgcctttggggataaagcccgccgtctgaaccttgatattcatattgaaaccagcgcctcagataaggcatctattgacgaagccgtcgccatcgcgttgaaaactggggcatcgtccgtacgtttttatccacgttatgaaggtaatttgcgcgacgtattatcgattatcgctaacgacattgcctatgtacgggaaacgtatcaggacagcggcctgacttttacgatcgagcagcatgaagatttaaaaagtcatgagctggtgtcgctggtcaaagaaagtgagatggaatctctttccttactgtttgattttgcgaacatgatcaatgcaaatgagcatcccatcgacgctttaaaaacgatggcaccgcatattacccaggtccatatcaaagatgccttgatcgttaaagaaccgggtggcctgggtcataaagcctgtatttcaggtcagggtgatatgccgttcaaagcgttattaacgcaccttatctgcctgggtgatgatgagccgcaggtgacggcatatggcctggaagaagaggttgattactatgcgccggcgttccgctttgaagacgaagatgataatccgtggatcccttatcgccagatgagtgaaacaccattgccagaaaatcatttactggatgcgcggttacgtaaagaaaaagaagatgcaattaatcagataaatcatgtgcgtaacgtactacaacaaatcaaacaagaggcaaaccatcttctgaaccactaataagttttaactcatacgcagttaataaaaccattccatatgaatggtcggtatcttattgcctttaaaacagtgattttaaaaatcgcttaggggatgttatgctcacgaaaaagaaatgggcgttatttagtctattaacactgtgtggcggtacaatttataaattaccgtcgctgaaagatgcgttttatatcccgatgcaggaatatttccatttgaccaatggtcaaattggtaatgctatgtcggtaaactcatttgtcaccacagtgggcttttttctgtctatttattttgccgataaactaccgcgcagatacaccatgtcattctcactcattgcgacaggattactgggtgtttatttgacgacaatgccggggtattggggcatcctctttgtctgggcgctatttggcgttacttgcgacatgatgaactggccggtcttgctcaagtcggtaagtcgattgggcaatagcgaacaacaaggtcggttgtttggcttcttcgaaacagggcgtggcattgtcgataccgtggtggcattttctgcgttggcagtatttacctggtttggcagtggcttattaggttttaaagcaggcatctggttctattcccttattgtgattgccgtaggcattattattttctttgtcctgaatgacaaagaagaggcaccgtccgttgaggtgaaaaaagaagacggagcatcgaaaaacaccagtatgacctcggtgctgaaagacaaaactatctggcttatcgcttttaacgtcttcttcgtttacgcggtttactgtggcctgacattcttcattccattcctgaaaaacatctatctattgcccgttgcgctggtgggggcttacggcatcattaaccaatactgtctgaaaatgattggtggaccgattggtggcatgatttcagataagatcctgaaatcgccaagtaaatatctatgctacacctttatcattagtaccgctgcgctcgtactgttgattatgctgccgcacgaaagtatgccggtctatttagggatggcatgtacgctgggctttggcgcgatagtctttacacagcgagccgtattttttgcacctatcggcgaagcaaaaattgctgaaaataaaacaggtgcggcgatggcgttgggtagctttattggttacgctccggcgatgttctgcttcagtctgtatggctacattctggatttaaatccggggattattggctacaaaatcgtgtttggcattatggcctgcttcgcattcagtggtgcggtggtttccgtaatgctggttaagcgtattagccaacgtaagaaagagatgctggcggctgaagcttaattaatggccggatgtgcttaatccggccaacgaaaaccgtatcaaccgtaggccggataaggcgtttacgccgcatccggcagtttcacatcagaagaaatacttcgtcccgatacggatctggttttgctcgcggtggtacggttcgacgttgcggtctaaccagcgcaattcgaaataagggagccagtgttcattaatacggtaacggaaggtgttagtgatttcccaatgatgatctttcccgttgctactattaaagtcattcactcgcatgaagtaatgtggctcaaatgtataggaaaatttatcggtgattttaaaattccagtaggtgccaatttcataggtgtcattattatccagttccccgctcaaatctgttgaactatagttattatggttatagcgatttcgtactgtcagattaaaccatggtacaaatttatagttgacgtccagatacactgcaccacccgaaccgatactcttatcattaattaagccaccgggctggatggttaatttatcggttggtttaaataacggataccagccttcaatttcgttatatccatgttttagttcatcttctcgctgaaagttgtaggtattggttaacataatacccgcgcccatatcgaagttataacccacacgtagcataacctcgccctgatcggaggcaagattatatgcctccctgttttcgacgtatgcgccagcaaataccgaggcagaggtcagagaagataataaaattattgcattaatctttttcataataagtccattttttaaacgtagggaggccgccacccaccaggatggaaatagcggctattgacatttataacgttacggaagccgttttttcttctgtcgccatctctttatttttgcgttggttgatttcctcaataatcaatgcaaaccgtttttcattgagtgtgtaaaagaatcccatcgtcaatgcagcaataattgccagtgcacaaggccagataaaaatgagctgacgcaaaccctgtaatgtcgcatcgctttgcgcgatgttgggaacataaccaatttgcgtcagcataatgcctggcaagaagccagcaagtgcggcagaaattttacgaaagaaggtataaccggtataaacagaaccttcggcacgaataccggttttccattcaccgtaatctacggtatctggtaccagtgcccagttcaggctgtttacaaaggccgtgccaaaaaaggcgacacaagagaacatgacgaaagtgaaagagttacttccccagaaataattcagtatatcacccaccgcccacagcaccatgccagccagataaacctgttttttaccaaaacattttacagttaatggcaccagtaatacgccgatgaggatgcatcccatactgaagaatcccatccacgacaataaattaatatcattcagcacatactgggtgtaatagacctgaatcgccagtttgatattaaatgccgccagggtacacaagttagcaatgcataaaaccagcaatggcggattccgaaatatcgcgcaaaatgatttgagaatactggctttatgtccggttggcgttgtgtccacataatgctctttgacgcctctgtagcacagcatcataaaaataaagccgccaatggagaacataagtgccgcacaggcataaccgacggttgagtcagaaaaaagcgactgcaacggaataaacgccacggtacaaatcaatagccctatggttgcaccaccctggcggtaagccgcgagctgcgcgcgctcattcgggtttttggtaattgccgggatcatcgcaccatacgagcagttcatcagactgtatgaaagtccaaacatcataaacagcgcggtggcaatcgtcgttttaaccggcaaacaaaaggtggtggcgataaactggagcgttgcaattaacgccgccggaaccgctgcatataaaataaagggacgaaatttgcctttaggcccaatatttttccgcgagtcgagtaaaaatccggtgagcatatcggtaaacgcggtaaaaaacttcgccaccagaaagataatcccgccatagtaagcaggcatccctaattcatcggtataaaatttgaggagatacagagtaccgatgcagagcattaaattcgaaccgacgtcgcccataccataggcgattttttcccgcagattcagttttaatgtcagtggattatggtcagacataatcactccttataacgccccgcagggcgtcgtttattattattacgccgtgcgtttacgggcttctatctcttccacaatgcggacatacatcttctcgttcaggctgtagaagcaacccatcgccacaatggtgactaccgccagtgcgcttgggtagatgaagatcaactggcgtaacccttcaatggtgtggtcagcctgtgcgacgttcggcacatagccaatttgcgtcagcatccagccggggaagaaaccagccagcgcctgagacactttgcgaaagaaggtaaaaccggtgtagaccgttccttccgaacgcacgccggtgcgccactcgccgtactcgacggtgtcggaaaccagcgcccagttcaggctgttaacaaacgctgagccaaagaacgccaggcaggagaacgccacgaagctgaccgaaccgccgccgaagaaatagttgagcagatcgcccagcacccaaatcagcaggccgccgatataaactttcttcttgccaaaacgtctgactgaggcaggcatcaggaatacgccgatgaaaatacagcccatgctgaaaaatcccatatacgacaacaggatgggatcgttaagcacgtactgggtgtaatagacctggatggcgagcttgacgttaaacgcccctaaagtgcagaggttggcaatgcacagaatgaacagcgggcggttacccgcaattgcgcggaaagattgcagcaggcccggcttttgcgccggattagcaggctgggtttcgacataacgctctttcacgcccgagtagcagatccacataaacagcaggccaaacagtgaaaacagcgtggcggcgaagatatagccaagttgctgattaccttcgataagattcataactggcacgaatcccaccgtgcacagcagcaggcccagcgtagcgccgccctgacgccatgccgccagtgaggcgcgttcgttggggtttttggtgatagcgggaaccattgcgccgtaggagcagttcatcatgctgaaaaacagtccgtaaagcataaacagaatagtggccatcaccgttttaccggtgacatcaaacggtgtgccgacaaagttggcgatcgccagtaaggtgaccgggaatgacgcatacagaataaaaggacggaacttaccttttggaccgatcttgcgtcgggaatccaacataatgccggtacccatatcggtaaacgcagtaaagaattttgaaatcaaaaagataatgccgccataggtgcctggcagccccagaacgtcggtataaaacttcaaaagataaagcgtaccgatatccagcaggatgttagaggccaggtcgccaataccgtaagagagtttctctttaaagggcaggcgtaaagttgctggatcttccgttgtgatgtgactcatcgatgttctccctttgcccatgagtttccccacgggcggatgtgattagatgctttttaacgacgcgaacagtgccgcccattcgctatcggcgcgataaaagaccggcggcttgccgatgggcgcattaacggtaacttccccgccccggaacgcttcacccgtccaggcgtggacccagttatcctccggcagatagagcgtccagtcgctacggccttcttcatgcaccggagcgaccagaatgtcgcgacctaacaggtactgatatttcagggtgtaagtgtgcgcatcgtcttcgtaatgcaggaacagcgggcgcataaccggcaggccggacttcgcattcagcgcgacggcctctttcaggtaaggtttcagggtggtgaagacggtggtcatacgggcgaaatgggcgatggtttctgcgtcgccgtcaaactgccagttgtcgccaggacggttaccttcgtgggtgcgcatcatcggcgtgaaggcgctgaaatcgcaccagcgcagcagcagctctttgctgcgcttcatctcaaacagggtggtgtaaccgccaatgtcgctgtggtgcaggccatgtccggtcattgccagcgacagcgccgccgggacaaccgacgccaggccatcgtcgagactccagtcgacgttctggtcgcccgcccacatcatggtggagtatttctggctaccggtagaaccggcgcgcataaagaaaaggatctcgccgagcttgcccgtttcttcaagggcttcgtagttacacttcgcccacagcgcaggccaggcgttatgcataatttcggcactgacgccgttatgcaagtacgtgtcggtgggcagatactcgccgaagtcagccatccagccgccgcagccgagttcaatcatgttctttttgatcacttccttgaaccaggcgtaggcttctggattagtgagatcgacaacgccgccgtaaaactcgccaaactccaccagatagtcaccgccagaggcatcttttgccagatagccgtgttgtgccgcttcttcgcagagatctttatcgctggcaacatacgggttgatataggccaggaactgcacgccctcctgattccactgcttaatgcgtgaatccagttgcgggtagttttcgctgttccacttccagttccacatcacgcgtttgccaaaagaggtcatacgaataccggaccagtcctgcgcccagatgccgttgaccttcacgcccgcgttacgcatggtgtccagtttcttctggcacacttccgtcccgccctgaatgccgagcgttactccgtcataaatccagtcgggcagttctggctggcgtcccagcagggcggttaatttttccagcagggaaatgtatgtgtcagcacattcaaaacgcagcgttgctttgtcttcccacagcgccagttcatggtattccggggcactaaagtcgaagttcatatagcaactgttatcaacatggcagtaatacttctgcgtgctgacaaacgtaggctgtgggaagaaagtccagtaatagtcgccgcccgcattttctttgcagtcggcctgccaggtgacataggtttgtttgttgcgaccaacgccttgttcactggtccatagcgggaacggtttgccacgcagatcgaagtaggaaaactgttcgccgcagccgtagatatggtcctctggttgagcggcaaggcgcagccagatacggttgtggttaaggttgtcgttttgtagttccagcaataaacgcccctgatcgtcggcagagatattcagcgtggcgctaatgtcagaaccacggctgaaatgaattaaccaaccatccggtgactggctgacgatggcgtcggtaagcgcaattttctcctgtagtttatctttaatgctgaaattaccgcggaacatatcgatatccgctatacctgagccaatccataaacaaggattatctttgctatgggttaaaataagacgttgttgaaaatgtagggtaaaactgtcgttattctgatgaaattgaaaatctaataactgtggacgtggcgtatccataactaatctccatagagttgagaacgagattgttgccttcctgttattacaggcttatgtaaaatgattctcataaaactgatatataaaaactttacagaagctgagctgtttttaacttaataaattgaagatacataatgttgcctttagcgagtgaaatgttcttcaatgattttgactgctaatcaatacaagttattttctctgtccgtaaatattaaaaaacaggcggtgcggttttcctgattccagtaataataagtcgatacctgaattaaaggcgttaggcgggcaactcataggttcaactgccagtccctgacgctgtaatttttcaccgctataaacctgcacccagagttgatcggaacaaaggcttaccgaaagcgcctgctgtggatgggtaatggtcatttcccacaaatcattagcggttttaaaggtgtggtcgatttttgtcgcggctatttttttcgcctgcgtgaaatttaaatccagctcatcaacgtggtgaagcgttgtcggattcgcgtgctcatcgacggcataaacctggtttgccggaagctggaacagatattcatcaacagatgttaagttgcaggttaaataaggatgaatacccacgccataaggcgctgcgacagtgccgatattctggcttgcgatctcaacggaaagacccgtgtgtgcgttgagcgaataaacaacttgtgaagccagcataaacggatagccgtaactgggcggcagaaaagctgtcagggtaacgctggtggcggttaattcactaatttgccagtctcgccaggcaagcagcccgtgaatagcggcttttgaactatgttcattaatgggtaactgatattcctgcccctgatagcggtaacagccgttggcgatccggttcggccacggaataagcactttacccagatgcgccagcggcatctcttcgggtttgtgcgggatgactaaatgacaaccctgaaaggttaattcagccagaccagcaccgacggtcacaatggtcgcgtgataatcccccgcggcaagtgaaacggtctgtccactgcaatgcatattggtgatttgcatacaaggcaccttaattaacgacatacagcctcccgtgaggctgatgtcaaacccaaaaactgcaccggacggtcccctcgcccctttggggagagggttagggagaggggaaaacccgcaccctattttcagatcagttatttcgcattaatatccagcagacccgctgcaaccgctggagccatgccgggcgctaacgggatacgcgggatcaccaggcaatgcagcaggtgataaatatcctgtttgccgtcccagactttggtggtgaccttattgtccgcatccagctcctgccaccaggaaccattttcatagtccatcaggtacttaatgcagtactcccaccatgtttgataccaggtttcatactggcgatcgccagtgacggtgtagagcgcgtaggccgtacccattgcttcgacgataggccaacgtacacgttcgcggaccaccggttttccttcccagtcaacggtataaacaatcccgtccgcgccatcgggtgcccaggcatcgcgcacggtggcgttaaacagacctttggcatcttctagcagccatgctggtggttgttcgcaacgggcttccagggcagcatggatgtgcagcattaaacggccccattcgatccagtggcctggtgtacctccgaacgcgcggaagcgatgcgccgggttatctttgttgtaatccggcagcggattccactgggtatcgaagtgttcgttaacgcgataatgattatttctggcgacgtcgtggataatcacggaagccacgcgaatcgcgcgatccagccattttttgtcgtgagtgacgtcataaacaatcaagaaagcttccaccgcgtgcatattggcattgccgccgcggtactcttcggttttgctgaaggcttcgtcccaggattccaggcacatctgctcttcttcgctccagaaatatttctcgataatttcaatggtgtaatcgagcagcttgcgcgcttccgggtgacccgttgtgacggcgctggcggcacccagcagagcaaagaagtgttgatagccctgtttggaggcatccaccacgccctcgtcattcacgcaggcataccagccgccatattttttatcacgcagtgcgccgttcatggctttgataccgtgatcaaccaacgagtaagcgccaggtcgacccatcgccgcagcaacggaataaacgtgcaacatacgagcggtgatccacagatgggtgcccatctcttctttgatttgccctttattgcctaaccagccaaaaccagtcggcactacggaatttttaccaaaatcaaagatgcggtcggtttcctgttccagccaacggttgtggcttagggtgttaaaccatttcattccttttatcctcatcttagcggcgtttagccatcatttcgtcgacgatatcgccaagttgttgtaatttcggtgcgcaaacgtcacgcagcatcagctcgttgtctggtaaaccgacgaccgatgcccagactgcacggcctgccaggaatcccgatgcgcccgccgtcattgccacgcgtacggcacgcgggaacagtttttcgtcgacaccggaagagaggatcacccatggcatattgatatggtcattcagacgttgtgaagcacagagaagctcttgttgcggacctttgccataaagcggcatttcaactttgtagaggtcagcgccactgtcgcccagctctttggcggcatcgatgatcgcttgttcgcgatcgaatttatcgccacgacgcggtgggcggacgactggctcaatgatgcttaccagaccgtgtgagtggcacagttcgttgaactctttcaccatatccagacgttgctgcgcatcttcatcactacgccacagcaccagcagttttaaggctttgccaccgtcttgtttgatctgtagcggattgattttgcggtcaataaccacgctatcgaccggaataccgttgccaggaatgaactcatcggcggcgacaatcatggcgcaacttttggcaatcgcgttttgctcaaccacctggcggtagcagaattgttgatctaccagaatcgccgaggcataaggcgagagggcctttgcagcgttaactttgaaatcagttaaaacgctatcggctaccggagcgggtgccccagccgcggcaaacatcatgcgcatggcttcgcgctgatcgaccgccagcatggcaaaaccgcccgatgcgcgcgtaatgtcgttgatggtgtacttattcattcatttattcctttatccagtcgttacatttttactttggcagtcatcccggcactgacacggacctgttccagaatggcggaccagtcctggcgaccgcgacccgctgcgcgcgcctggctataaacctcccgtgaggcggcccccagcggcattggcacatgcagctggttggcgacatcaagggcgatgccaagatccttatgggcaagatcgatcatgaaggcgggagaaagatctccgctgaggactttgtttggccaggaagtggtgaagtgacctttaccggcggcggtaccgctcatcactttgacggcaacatcgaagggaagattcagggcttcgcacaaaacggcggcttctgccgaaagcgcattgagcgcgatgctcatgtagttgttgatgagcttaacgcggatccccatgcccggaccgccagcgttgatcaactcactgcccatcgccatcaggatcggtgtggcacgttcaacttgttcagcggtgccgccagccagcagtaacagagtaccggtaatggcatttgcagaagtacggcctaccggaacatccatcatgctgaagcctttggcttgcatatcggcaatcaatttatcggtttgcagcggatggatggtggacatatcaatgaccagcgcatcggtagataagccttcgcaaacgccgttttcaccgaacaacacgttgcgcaccagatcgccattcggcaacatggtaatgataaattcggcatctttagcggcctgcgccgggttggcggcgggagtcgcacctttgtctaccagatgccgcacagcttcggcgttcacatcaaagacgcgaagttgatgcccttgctgcaataaattgctcgccattggcgaacccatttgtcctaaaccgataaacgcgattgctgccataaccctctcctgaatacagttatgtcactttttgtcatttatgacatgctttgcttgtctgtttttgatcgtatttgtaatttatcgtcaaaaaattgacagccgtcactttttaaacaattggtgaaattaaaatgaacgcatcccaaaatgtttaaggaatgaccatgattcgtgttgcttgtgtaggtataaccgtgatggatcgcatctattacgtggaagggttaccgacggagagcggtaaatacgtggcgagaaattatacggaagttggtggcgggccagcggcgacggcagcggttgcggcggcaaggctgggggcgcaggtcgattttattggtcgcgtaggtgatgacgacacgggcaacagcctgctggcagagctggaatcctggggcgttaacacccgttacaccaaacggtataaccaggcgaaatcttcgcaatccgccatcatggtggataccaaaggcgagcggataatcattaactaccccagcccggatctgctgcctgacgcagagtggttggaggaaattgatttctctcagtgggatgttgtgctggcagatgtacgctggcacgacggcgctaaaaaagccttcaccctggcccgtcaggcgggtgtgatgaccgttctggacggggacattacgccgcaggatatcagtgagctggtggcattaagcgatcacgcggccttttcagaaccgggtctggcgcgcttaacgggcgtgaaagagatggccagtgcgctaaaacaggcacaaacgctcacaaatggtcatgtctatgtgacccagggtagcgcaggctgcgactggctggaaaatggtgggcgtcagcatcaaccggccttcaaagttgatgtggtagataccacaggtgcgggtgatgtttttcacggcgctttggcggtggcgctggcaacaagtggggatttagcggagtcagtccgcttcgccagcggtgtagcggcgttaaaatgcacacgtcccggtggacgagccgggatccctgactgtgatcaaacccgatcttttttgtcactttttgtataaaatgccagggtgatggtttttcgaggaattttcatgagccttaccgaactaaccggtaacccgcggcacgaccaactcctcatgctgatcgccgagcgtgggtatatgaatattgatgagctggcaaatctgctggatgtctccacgcagacggtccgccgggatattcgtaaattaagcgagcaaggcctgattacgcgccatcacggtggcgcgggtcgggcttccagcgtcgttaatacggcgttcgagcagcgtgaggtttcgcaaaccgaggaaaaaaaagcgattgccgaagcggtggcagactatattcctgatggttcaacaatatttatcaccattggtacgactgttgagcatgttgcccgggcgttacttaaccataatcatttgcggataatcaccaacagcctgcgtgtggcgcatattctttaccacaacccgcgctttgaagtgatggtgcccggcggtacgttgcgctctcataatagcgggatcattggcccttcagcggcgtcctttgtggctgattttcgtgctgattatctggtaacaagcgttggggcgattgagagcgatggcgcgttgatggagtttgatgtaaacgaagctaacgtggtgaaaacgatgatggcgcacgcgagaaatattctgctggtcgccgatcacactaagtatcatgcttcggcggcggttgaaattggtaacgtggcacaggtcactgcgctctttaccgacgagctgccgcccgctgcgctaaaatcacgcttacaagacagccaaattgaaatcattcttccccaggaagacgcgtagatttttgtgaccgttaacctggcttcataccttgccacatagccaaacccatcctttcccgctacagttaatttcttgtggcgcgaaaggaggcaaaaatgctctatatctttgatttaggtaatgtgattgtcgatatcgactttaaccgtgtgctgggagcctggagcgatttaacgcgtattccgctggcatcgcttaagaagagttttcatatgggggaggcgtttcatcagcatgagcgtggggaaattagcgacgaagcgttcgcagaggcgctgtgtcatgagatggctctaccgctaagctacgagcagttctctcacggctggcaggcggtgtttgttgcgctgcgcccggaagtgatcgccatcatgcataaactgcgtgagcaggggcatcgcgtggtggtgctttccaataccaaccgcctgcataccaccttctggccggaagaatacccggaaattcgtgatgctgctgaccatatctatctgtcgcaagatctggggatgcgcaaacctgaagcacgaatttaccagcatgttttgcaggcggaaggtttttcacccagcgatacggtctttttcgacgataacgccgataatatagaaggagccaatcagctgggcattaccagtattctggtgaaagataaaaccaccatcccggactatttcgcgaaggtgttatgctaaaaaccattcaggacaaagccaggcaccgtacccgtccactatgggcctggctaaaactactctggcaacgcattgatgaggacaacatgacaaccctggcaggtaaccttgcctatgtgtcgttgctctcattagtgccgctggttgccgttgtttttgcgcttttcgccgcttttcccatgttttccgacgtcagcattcagttacgtcactttatttttgccaactttctgcctgctactggcgatgttattcagcggtatatcgaacaatttgttgccaattccaacaagatgaccgccgttggggcgtgcgggctgatcgtcaccgcgttattgttgatgtactccatcgatagcgcgttgaataccatctggcgcagtaaacgagcgcgaccaaaaatttactcgttcgccgtgtactggatgattttaacgctggggccgctgctggcaggggccagtctggcgatcagttcctatttgctctccctgcgctgggcgagcgatctcaatactgtcatcgacaacgtgctgcgtatttttccgttgctgttgtcgtggatctccttctggttgctgtacagcattgttcctaccatccgcgtacctaaccgcgacgcgattgtcggcgcgtttgtcgccgcactcctgttcgaagcaggaaagaaaggtttcgcgctttatatcaccatgttcccgtcatatcagctcatttatggtgtgctggcggtgatccccattctctttgtttgggtctactggacatggtgtatcgtcttgcttggcgcggaaattactgtcactctcggggaataccgcaaactaaaacaagcagctgaacaagaagaagacgacgaaccatgattgcattaattcaacgcgtaacccgtgccagcgtcaccgtggagggagaagtgacgggcgaaattggcgcgggacttttggtgttattgggtgtcgaaaaggatgacgacgaacagaaagcaaaccgtctgtgcgagcgtgtgctcggctaccgcatctttagcgatgccgaaggcaagatgaatctcaacgtgcaacaggcgggcggcagtgtgctggtggtttcccagtttaccctcgccgcagataccgaacgggggatgcgcccaagtttctccaaaggtgcatcaccggatcgcgcagaggcgttatatgactatttcgtcgaacgctgccgtcagcaagagatgaacacgcaaacaggacgcttcgctgcggatatgcaggtatcgctggtcaatgatggccccgtgacattctggttgcaggtatgagccagcttccagggttgtcacgggaaacaagagagagtatcgctatgtatcaccttcgggttccacaaacagaagaagaattagagcgttactatcagtttcgctgggaaatgttgcgtaagcccctgcatcaaccaaaaggttcggaacgcgacgcgtgggatgcgatggcgcatcaccagatggtcgtcgacgagcagggtaatctggtggcggtaggccgactgtatattaatgccgacaatgaagcgtccattcgctttatggccgttcatcccgacgtgcaggacaaagggttaggcacgctgatggcgatgaccctggagtcggtggcgcgtcaggaaggcgttaagcgcgtgacctgtagcgcccgtgaagacgcggtggagtttttcgccaagctggggtttgttaatcagggagaaatcaccacgccaaccaccacgccgattcgccattttttgatgattaagcccgtcgccactctggatgacattctgcatcgcggcgactggtgcgcgcagctgcaacaggcgtggtacgaacatatcccgcttagtgaaaaaatgggcgtgcgcattcagcaatataccgggcaaaaatttatcactaccatgccagaaaccggcaatcagaatccgcaccatacgctgtttgccgggagtttattctcactggcgacgctcactggttggggacttatctggctgatgctgcgtgaacgccacctcggcggaacgattattcttgcggatgcgcatatccgctacagcaagccgattagcggtaaacctcatgcggtagccgacctcggtgccttaagcggcgatctcgaccgtctggcgcgcggacgaaaagcacgggtgcagatgcaggtcgaaatctttggcgacgagacgccgggtgcagtgtttgaaggcacgtatatcgttctgcccgcgaagccatttggcccgtatgaagagggcgggaacgaagaagagtagctgatggagaggggcggtgctgcctctctcattcaggtcatttatattagtccttggctatttcggttatattaaataagaactctataaatttttattcttcgttggctccatacgtgtcttgctacatcactgttcaggagcatttaaatattatttgtagaactgagtggcaattatcgcagataatgcttaattcatcatcttagttcatgtttgagcgatttttgatagtcaaaaccccctctggtgccatacttttctcataaatatttttaaaatctatagctaacaaatattatgcaaagataatggactagcatcattgtcagtatcattcatttactgctctgtatgttatgaataattatgttgtatgtttgctcttaaaccgtgggaaggaggctataatggttgccaatattaatctcattaaacaagaaagttattctgttgttaatttagaaaaacaactttcccgaactgttaccaacaaaattataacgatgagcaagtaaagaccggttggtggcagtactgaccggtctgtgatgaaagattaatttcaccttaaatcctggtgctgttaggatgctgacgtttttcggctacaccattcagattatgcaaataaatatctctgaatataatatattcatagcacccataattcatcctgggcgataactaaaccatttttgagtaataaatgaaacaactgcaacactcttattatttctggaaaacgcctcgcaaaaacaaaacaacatgcaaaaatccgctttttttaaatgattttccggcgtaattttcgcacatacattaatgagtaatatatgtaaggtattggtaatggcgatgaatacggtttttcttcatttatcagaagaggcaattaaacggctgaacaagcttcggggctggcgtaaggtttcacgatctgcaattttacgcgaagcggtagagcaatatctggaacgtcagcaattcccggtgcgtaaagcaaagggaggcaggcaaaagggggaggtagttggtgttgatgatcagtgtaaggagcataaggaatgacaaaaatttttcattcttgaatataaaaaacagatgcccttattctggtattaatacaaggctgttttacttgaacttataataactgcaactgttacatcatatctggaaaacgcctcgcaaaaataaaaaatgatgcgtaaatgagctttctttaaagattcggcaagggtacttttctctccatagattcaaaaatgatattggcgagatatttatgaactctctggcaggtatagatatgggcagaattttactcgatttatcgaatgaggtgattaagcaacttgatgatctcgaggtgcagcgtaatcttcctcgtgcggacctattaagggaagcggtagatcaatacctgataaatcaatcgcaaacagcaagaaccagtgttcctggcatctggcaagggtgtgaggaagatggtgtcgaatatcagcgtaagctgcgcgaggaatggtaatgggaaaaaatgatgtcaatcagattgctgacaacgtgcgcgttgttcatgccggatgcggcgtgaacgccttatccggcctacaaagtcgtataaattcaatgtattgcagtttattggtaggcctgataagcgcagcgcatcaggcaatcttacgcttgtcatcagtctcatgcccataaccttattgatgtggtggtgggtaaattgaggccaaaccggcactggcggcatagcttgaggtggtaacgcggaatacgagagatggtgtcgtcacaccctatgagctgtaatccgggcgacctgcgccacccggaaaacgtcagagattactctccttcacccggaaacaggaacgggttgatggaactgcgggcatagccttcttgctccattcgtgcgtccagtaccagagaggcgaggtcatctgctacggcttcgatttttggatctttttcctgatagagaattttcaggtaagtgtcgcagtcatcgcagctttcggctttaatcgcggcctgttcgtcatccagcgaccagtaatgcagtttgccgctctgctcgcagttgctgcattttacgcgcactacgtgccattcagtttcacacaggttgcagtgcaggtaacgtagcccctgagtggtgccaatttgcaccatgctggacaccggcatagaaccacaaaccgggcaatattgacgttgctcgccgtattcagcgcgggctttgccggggatcagattggccatctgcgcccagtagagcgacagtgcagcccagataaacggcgctttatcgctgctgacggacgagaaatcagaggcaaacagcgcgctggccatatcttccagctcctgagtcgatgccttctccagattctcaatcactgccagcgccgggccgctcatttcaggtttcagctcagcaatcagcgccatcagcagcttttgccagtgcttatcacgcggcagaacgtgaatatccagcgggggcttgccttgtgcgctggcttctttaatgcgcgcagtcagatccatctccagcggatggtcgtacagcaccacttcctgggcgtgggcgataagcgcagcaaagcgcaggtaatcacccagaggattattttctgccagctcgcgcagacgctcggcgcggcggttgtataaattcttgagccgagggaacaataacggcggaatcatatccgccgtacgtttctcgcttgaacccagctcatcttgcgggattatgcgaatactcattcagctttcttttccgttgtcttgcggacctcacggtaccagcgcgggtgatgtttcttcgcccaggcgctggtaacccatccttccaccatggcggtaatcgtgcctttcacccaaagggcggcgtagatatgcaccatgataaccacaattaacgccactgcggcaaatgaatgcagcattaacgcgaatcggatcaccgggattgagaaagcaggcgcaaaataaggacgccagataatcacgccgctcaccagcagcagaaccaggaaaataatcgccgcccagaaaacgcatttctgaccgaagttataacgcccggtgtcacctacttcctcgttgacgacgatcttacgaatattcttcgcccaaaagatatcatcccgattgattaggttgtgatgccagtaacggaaaaacatgatgatgaacgaggcaaacataaccacgccgacaaacgggtgcagaattcgcgccagctgcggtgtgcccatgatttgcatcaaccagttgaaggacgggaacaaaaagcccagcccgctcaccgccgccaggatgaagcagaaggcggtgatccagtggttgatacgttccggcgcggtgtagcgcacgatggtgtcacgtcgtttcatttgcgctcctcgtctttctcttcgtgcagattattctcttcctcatccgcacggttcggaccgacacccacgtagtggaagatactggccgcaaaggtagccgcaaagccaacagccgcgagcggtttccagatgcctttccagaatttcacggtttcgctgatttccgggttctccggcaagccatgatacagatttggcttgtcagcatggtgcagcacgtacatgacgtgtgtaccaccgacgcctgccggatcgtacagacccgcattgtcgtaaccgcgggttttcagctcagcaacgcgctcgctcgccagcgttttcatcgactctttcgtaccgaagtgaatcgcgcccgttgggcaggtcttcacgcaggctggttcttgcccaaccaccacgcggtcaacgcacagcgtacatttgtagacgcggttgtcttccgggttgaggcgcggaatgtcgaacggacagcccgcaatgcaataaccgcagccaatgcactgctcggactggaagtcgacgataccgttggcatactgaataattgcaccttccgccgggcacgctttcaggcagcctggatcggaacagtgcatacagccgtctttgcggatcagccattccagtttgtcgttctgctccacttccgagaagcgcattaccgtccacgatttggcgcttaaatcattggggttgtcgtacaccccaatgttattgccgacggtatcgcgaatgtcgttccactctgaacacgccacctgacaggctttacagccgatacaggtggtaacgtcgatgagtttcgccacttcttcctggaagtcccgcgcctgaggcgcgggggtcagaccgttagtcgcggaacgacgaatgatatcttgagattgataagccatatgtcgtctccgttacaccttttccacattcacaaggaaggacttaaactccggcgtctgcgtgttcgcatcaccaacgaatggcgttaaagtattggcaataaagccttttttagctacgccttcatagccccagtgaatcggaataccgatggtatcgatatctttgccgttcgctttcagcgtgcgaatacgtttggtcaccaccgctttggctttgatatagccacggttggaggagactttcacggtatcgccctgggcaatgccaagtttattcgccagcgactccccgatttccacaaactgctctggctgcaaaatcgcgttcaacagcgcgtgtttggtccagtagtggaagtgctcggtcagacgataggtggttccgacatacgggaacttatcggctttacccaatgcttcggcgtcgtctttaaagatacgtgcagccgggttcgagataacgtttggatgcagcgggttagttcccagcggcgtttcaaacggctcgtagtgttccgggaacggaccttccgccatcttatcgagggcaaacagacgccccatgccttcctgctgcatgataaacggcccgacgccgctacccggaggcgctgcgctgtagtccggaatatcccagccggtccacttagtgccgtcccatttcagcaactgacgcttcggatcccacgggttaccctgcggatctgcggaggcgcggttatacagaatgcggcggttaagcggccatgcccatgcccagcccagcgtgttaccgaggccagacggatcggcgttatcacggcgtgccatctggttgccttccggcgtccagctaccggcgaaaatccagcagccacaggaggttgtaccgtcatcgcgcaattgggcgaacgaactaagttgttggcctttcttgacgataaccgcaccggttgccggatcggtaatatcggccagcgccttaccgttgctctccatcgccacttcttctgaagatggctcatgcggaatggcgtagttccatgtcatgttcagcacctggtccgggttcgcgccaccctgttcggcatacatcttgcgcaagcgcaggaagataccggagaggatctcgccgtcagtcagcgcaatccccggggcgtccgcacctttccagtgccactgtaaccagcgacctgagttaacgatagaaccgttctcttccgcgaagcaggtcgatggcagacggaacacttcggtctggatcttcgacgagtcaacttcgttcagctcaccgtggttctgccagaagttagaggtttcagtgttcagtgggtcgatggtgacgaggaacttcagtttcgacagacaaccgatcactttgtttttgttcgggaatgaggcaacagggttaaagccctggcagatatagccattgaccttgccctctttcatcatctcgaagtattgcaggacgtcgtagcctttatcccacttcggcaaccagtcaaagccccagctattttccgccgtcgctttatcaccaaagaaggccttcatcatagagacgaagaatttcgggtagttgccccagtagtttacctggccttccagcagcggttttggcgtgttggcggtaaggtaggtttgcagatcggtctgcttctcgcttggcagcgtcatgtaacctggcaggctctgcgacagcagccccaggtccgtcagcccctgaatattggagtgaccgcgcagggcgttaacgccgccgcctgccatccccatattgccgagcagcagctggatcatcgccatcgtacgaatgttttgcgcaccaacggagtgttgcgtccagccgagggcatacaggaacgaggcagttttatcgtgagcactggtttctgcgatgtattcgcagactttcaggaacgcgtcttttggcgtaccacagatgttttcaaccacatctggcgtgtagcgggaaacgtgctgtttcagcaagttccacacgcagcgcggatgttgcagcgtggtatcgcgtttggcgaagccgttttcgtccagttcataagtccaggaggatttatcgtacttgcgtttttccgcgtcgtagccggtgaacaggccatcttcaaagccgtaatcctcacgcacgatcaggctggcgttggtataggcttcggtgtattcgcggttgaatttttcattgttcagcaggtacagcaatacgcctgacaggaaagcaatgtcagtaccggaacgaataggggcatagtagtcagctaccgccgccgtacgcgtaaagcgaggatcgatcacaatcagcttcgcgccgttgtgaattttggcttccatcgcccagcggaacccgaccgggtgagcttcagcggcgttaccgcccatcaccacgacgaggttggcgttcttgatgtcgacccagtggttggtcatcgcaccgcgaccaaatgttggagcaagacttgctaccgttggtccgtgtcagacacgcgcctggttgtcgaccgcgagcatacccagcgcgcgggagaatttttgcgttaaatagccggtttcgttactcgacgcggaagcacacagcatcccggtggagagccagcggttaacagtcacgccttcggcgttttgcgcaatgtagttagcatcgcggtcttctttcatcagtttggcgatgcgatcaaacgcctcttcccaactgatttgctgccatttatcagaacctggcgcacggtattccggaaacttcagacggctttcggagtggatgaaatccaccaggccagcgcctttcggacaaagtgcaccgcggttgaccgggtgatccggatcgccttcgatatggaagatagatgctttggcgttttttgctccgtcaccgaggctgtacatcaacagcccacagcctacggaacaataggtgcaggtattacgggtttcgcgggtgcgcagcagtttatactgccgggtttccgcgagtgctacgctgggtgcaaaacccagtgccgctgccgtggtgcctgccataccgccagcgcagatcttaaagaactgccttctgctgacctgcatggattgctccttgtttcgacattgtcacgtcccatttacattcgcttgctgcgtgtgcagggagtgggagttatttttctttgcggaaggggccgcaaaggtccagaattggctcaatttccctccatccaggaagggtttgtaacagaataccataatgttggtgtgtgtgttcttatctggttaagagaaagtgaaaaaaacacagcgaaaagaaatcgaaaatgtgacaaatatcacaggtgttcgtcaaattgagttatggcggcgtgatgatttacaacacccacggttagatgaggtcgcggaagaagttcccgttgcgctggtctacaacggcatttcgcatgtggtgatgatggcgtcgcccaaagaccttgagtactttgcgctcggtttttcgctttccgaggggattatcgaaagtccgcgcgatatcttcggcatggatgtcgttccttcctgtaatggtcttgaagtacaaattgagctttccagccgccgctttatggggttgaaggagcgccgccgggcgctggcgggacgtacgggctgtggcgtatgcggcgtggagcaacttaatgacatcggaaaaccggtgcagccgctaccgttcacccagacgtttgatctcaacaaactggatgatgcattacgtcatctcaacgattttcagccagtggggcaactgactggttgtactcacgccgctgcctggatgttgccatctggcgaactggtcggcgggcatgaagacgtgggtcgccatgtggcgctggacaaactgttaggccgccggtcacaagaaggggaaagctggcagcaaggtgcggtactggtttccagtcgtgccagttatgaaatggtgcaaaagtcggcgatgtgcggcgtagagattttgtttgcggtgtctgccgcgaccacgcttgctgtagaagtggctgagcgctgtaatctgacactggtaggtttttgtaaaccgggtcgggcaacggtttatacccatccgcagcgtttgagcaattaattaaaataagtcctgcgaaatatattaaattgcaggacttattcatttcgtgaattttattattttatttataaacaaaatgcgtgtagtggcgttttcttttttcatttattatgttcactctcttatctatatatttataaggcaattaaatgaaaaggaatttattatcttccgctattatagtcgccatcatgtccctcggtctgacgggttgtgatgataaaaaagccgaaacagaaacgctcccgcctgccaatagtcaacctgccgcaccagctcctgaagcgaaacctactgaagctcccgttgcaaaagcagaagctaaacctgaaacacctgcgcaaccggtggtcgatgaacaagcggttttcgacgaaaaaatggatgtctatatcaagtgctacaacaagttacagatcccggtacagcgcagtctggcgcgttatgctgactggctgaaagattttaaacaggggcctaccggtgaagagcgtactgtttatggcatctacggcattagtgaatccaacctcgctgagtgtgaaaaaggcgtaaaaagtgctgtggcgttaacgcctgcgctgcaaccaattgatggcgtggcggtgagttatatcgatgctgccgtggcgttgggtaataccattaacgaaatggataaatattacacccaggaaaattataaagacgatgcgtttgcgaaagggaaaacgctgcaccagacattcttaaaaaatctggaagcctttgaacctgtagccgaatcttatcatgcggcgattcaggaaattaatgataagcgtcagcttgcggaactgaaaaatattgaagaaagagaagggaaaacattccactactactctctggcagtcatgatttcagcgaaacaaattaataacctgatatcgcaagataagtttgatgcagaagcggcaatgaagaaagtgtctgaactggaaacgctagtggcgcaggccaaagaagcggataaaggcggcatgaatttctcgtttattaattcggcaggccagtatcaactcgaggctaaaaaatacgttcgccgcatcagagataaagtcccgtactctgactgggataaagagcaacttcaggacgcaaactcaagctggatggtcgaagactctttcccgagagcattacgcgagtacaacgaaatggttgatgactataatagcctgcgttaaacgtttttgatgataaatgcagtgtcggatgcggcgcatccgacacagttcaccccttgtgaagtaactccataaatgcctcatatcctgttaacccggcaataatctccgccggatgctgacacaatatgcttgccagatagctaaatatttttagctcatgacgcgcatcggcggcggcgcaggcgatcaagacatggttaatgacttcgttattcacctcaactggttgggcgagggtaataaaaaatccacgaaaacgtcgctcctgttcgctccagcaatgtgggatggcgaggcgattaacaatcaggttttcaccttcgccttcgcgggcgatgatgcgttgtgcttcatcggcggtaatatggtgttgtgcgactaattgcgcacaaatttgccgggtaatatgttgccagctttcaccgcgtacattcgaataatgaaaacttccgggggcagagaaaaaacgctccggctgttggcgaataaatgccgtcgccagaaaatgttttatttgttcgataccggcagccgtaatgatattttttacggtgatgtaattatttaccgcgtcatccagtaaataatggctgttgttaatgatcaataacggctcaatctcttcgcgaatggcaacaagttcgcttaagctacgggcaataattacccgacaatttaaaacatcgcgctcaatggcgagctgattaatagtggcaatcgcgttctggtccgagagcaaaatgatcggctggcgttcgttttgatgccgctccagcgcacaggcaaaatacaaaccgatcagatcgctgtcgaaaaggggaatatcgagctgttcacgcagtagcgtaataaagtgcagactcatatcaaaggccgcaggccaggcggctttcaggttattcatgctgctctggcggtgctcagcaatccacactggtgcggcaaggcaacgtaataaatgcccggtaatattctcaaccagctgcgcatcaataatattcaatgacgcgatgcccggcaccctttgcagcaacccctgcacattatcggctgaaattacctgcgcttgctgatgctgtttctctatcaaacccgtcagggttcttacagcgttatcaccaagaaacagaccgctatgttcaacgatttgttttatctcgtcaccgggatattgcggccactcatcggtcagttgattacgcagggcgtaaatcgccagaatcaggctggagagataatcaccctgcatgagcggccagcggtgttggttgtcgcaggccgtggataaatgctgaaggttgtctcgtgttatgcccgccagcggaattaaaaacggatctttgcgcagcaagttcgccagcaagataacgcgtttctcttctgtctcatcaatgaaatggcccaaaccagggcggctggccaggcaacaagtgcgttcataacgctgttttaaccggggcagacgctctgctacccacgtttctggcaaattaagcgccgaggcgagttgcgcacggggagtgaaagtattcagtaataacagcgccagcagccgatcgtcgttatcgtgcttttgcagcaactgaaaaaagctgcggcgctcgaagatttccagctgatagcccgcactgccactggcgaaaatgcgggctttgccgttaagggtgaagttgagatagtcaatatcacgcaggatggtcctgcctgaaacgccagtctgttgcgccagctcgccaggcgtgcgcggctgttgctccagcagatcgacaatctttaactggcgttcgtttagcattaatccacctgacggaactggctaaacgcgttgactttctccgcagttaaggtcgtcagaaaaccccgtatcagcgtgagcagagcttcgtaatcggcttttgaaatcataccgctgttggcgtgcagataacgagttggcagacacagcgcgacaaccggacgcccgccgcccatcacgttgtagcgcccgccatccgtcgcaccggttttcatggtggaaaattgcagcggtaaatcgttatgtgcggcacagctttttaacgctgctaccagtttctggttggggaagtagcgcttgtcaaacagcatcagccccggcccctggcccagtttcagcgggtatttaatgttatcaatgcccggaacatcgcccgctacggcggtatccaacacgatcacgacgtccggtttaatgtgttccgccgaggtttgcgccccgcgtagcccaacttcttcttccacactgccaacgccatacagcgtaatttcgggattattcaccgtctgcaatagttcagccatcattgcgcagccgatgcggttatccaacgccttgccgaccactttatcttcgccccagcaggcaaaattggcttccgggctaataaaattaccaatttccacgccgcgcttttccacctcttcgcgactgttcgcgccaatatcaatgaacatctcatcaaatgacagcggttgttgcttttgcttttccgttaacgcatgaggcgcgacggaaccaatcacaccagggattttcactcccttgtgtgtgcgtatggttacccggtggttgagcatcgactgattccaccagccgccaatggtggtaaaacgcagaaaaccgctctcgtcgatgtgggtgaccataaagccgacttcatccatatgtccgacaacggcaacttttggacctttattccccttacgggcaacaaagctgcccagaccatcgaaggtgatttcattcacgcaaggttccagcgtgtttatcagaatgtcgcgaacttcctgttcatcgccgctgacggcgctggcttcgcacaactgttgcagtaactcaatgttcatggacaagctcctgttgcgcggctttcgctttgcggcgtaaccacaatcctttcaggacgataatgaatgaaatgttcagcgcgaggccaatcgccagcaccagataaaacgaacccaccggcgacatcaggccgatcagcgggtcaaagatacccaaaccaggtgccagacgtttgattccgaaagcgatcaccagcacgccggtaatgccgcccgccagcgtattggcggtaatcatcggcaacggagctgccagagcgtaaggaatagccggttcggttgcgactgtggcaccgaccacaatggcactactggcagcctctttttcctgtcgggtaaacagtttgggcgcaatgaacgtcgcaagacccgccgcgacgggcggcatcagcgcgacaacgccgacgatggcgtaccagtcataaatgtgtttttccagcagtgagaagcagaagaaccaggcggttttattgatggggccgcccatatcgaacgccagcatcgcaccgaccagaaacgctgccgcaaacttcattgatggaggaatggtattcaggaagtggagcagcccgcccatgaggtcggacatcaccggcccgataacgtagtaagtgagcacgccgaaaaccagcagagtaacgaacgggatcagcattgaaccgagcagcggttgtaatgctttgccaaggcgcactttgcggaaccagaagacgaaatagccaatcgccagccccagcaccaccgcgccgaggaatcccgcacccgactgggtgccgagcagcgctttgtcgttcgccagatagcaaaccagaaacgccggagcgaaagccggtttatcggcaatcgacgaggcaatataagcgcccatgatggggatcataaaggtgaagccaaggtaaccgatggattcaactacccaggtaaacgacggcgcgcctttcgacatatcggtatacggcaaaccgaactgcaccagcatgttggcaagcgccaccaggataccaccgccgatgacaaacggcagcgccgcagagacgcccgccatcaggtggctcatcacgctaccgctttgcacttcctgtttgccaagcttcacgccgctatctgcggcaaaaagctgcgagtttgtcggtaattcgctgaaaatctggtcgatatttttcaacgcctgggagatggcaatctcataaactttcttcccggcaaaccgcgcgcgatcatcaccgctcaggccacgcccggtagcgagaatgacgtaatcggcagcggcaatctcttcgctggataagcggttttcaacgccactggacccttgagtttccacttttatggtatgaccgagagaacgggctttctgttccagggcttccgccaccatgtaggtgtgagcgatcccggcggggcagttggtgatcgcgacaatacgtaaggatgactccatcgccacttccttatgagctgagggtttgatttaacaaggcaagcacctggtcggtatcgccctgttgcagttgatgaataaattccttgtgaataattttgcgacacagtgtgccgatgattttgacctgatcctcttcgccgctttgcggcacgccgaggcagatccagcaattgacgtcttcgccatcgctggctttccagtcaatagcctgcgctttgcgggcgaataatacgaacggttgtttaacgcaggcgcttttaccgtgcggcacggcgacaccggaaccaaatccagtagagtgcattttttcgcgcagcagcagggtttgcaggaactggtgtgagtcggtgataaaaccgttttgtaacgctattgtcgccaactgcttcagaacggaataagcgccattgccctgaatattcaggtcaatacagcttgcagtaagagctgccattaatcggactccataaaatatattttaatcaattgtaatggtggagcgattaagtgatgagaggcgatatgtcggtaaacaatgacaatttgagacagagtgaaaggtcagatttgcggagtaatgcacataatggttatttaaataaaccacatgaatcattaatgggttattcattatttttgtgatttactcacaatgtatcagggaaatataacttaccgggagatgtaatatgtttaatttttcaaatcgaaatttaaaatattgtgccggaggcatctctggcacattgggcaattacggcaggtaaaacacttcttgcagctcgctactcaccgggctgttatccgggttagcgggcataacatcggtcatatatttccaccaacgttggcaaacatcagtgctggcaaccgcattccagcgttcttcagattcaatctctaccatggcaaacagcagattacgcgctttgtcgagatagatggcgtagttatgcgcaccgtgagatttcagcactgcttccagttctggccagatgggattatgccgacgctgatactcttcgtgggcgtcggggtttacctgcatgacaaaggctttgcggatcatgtttgctccttacagcgccagcgcactggcgagtggcgtaacgccgaaacgcttgccgagcgctatcaactcttcacggctgatggtctgtttcatgccgcccatcgaataaaccttcactaatacttgtgctgatttttctgcggtgtcgattaaaccgaaggtttcatccagcgtcggtccgctgccgaagacgccgtggaagggccacaacaccagcgaatgtttttgcatctcttgtgcggtcgcctggccgatttcgtccgtgccgggcaccatccacggcaaaatgccaacgccatccgggaataccaccagacactcggtgctgccttcccacagttggcgagtgaagaccgcggtgtcgttttcaagtacataggtgagggcgatcaggttggtggcgtggcagtgcatgatcacccgatctttgccgttggtggctttaatgcgctcgcagtgggaaaggaagtgagccggaagttcggaagtggggacggcttcgttggttaacccccaaagaatgtggtagcccgcgccgtcgctgtcgacttttacgatgcctaagttagccgcaggatcaagctggacgttacggaagaatttgcccgagccggtgacaataaacggtgtatttgccagtaaaggcatgggctggctgagcgggatatagcgcggttgttggtggaaattgtcgtgatatggtgcgatatcggcgtcatccaggcgtagcgtcaggttgccgccgttgcgctcatcccagcctttcagccaggcgtcggtggtggctttgatcattccctggacaaaccaggactgagtaatgttttgcatgttctgtgttcctgtaaattcggtgttgtcggatgcacgacccgtaggccggataaggcgctcgcgccgcatccggcaatcaatgcctgatgcgacgctgtcgcgtcttatcaggcctacaactattgccgacctgtaggcctgataaggcacttgtgccgcatccggcaatcaatgcctgatgcgacgctgtcgcgtcttatcaggcctacaactgttgccgacctgtaggccggataaggcacttgtgccgcatccggcaatcaatgcctgatgcgacgctgtcgcgtcttatcaggcctacaactattgccgacctgtaggccggataaggcacttgtgccgcatccggcaatcaatgcctgatgcgacgctgtcgcgtcttatcaggcctacaactgttgccgacccgtaggccggataaggcgctcgcgccgcatccggcagtgtttacccgcggcgactcaaaatttctttctcataagcccgcacgctctccagccattcgctacctgctggcgtatcgtgacgttggcaatacatttcccagaccgcctgccacggcaacgatttctgctcttccagcagtgccagacgcgcagtgtaatcgcccgccgcttccagcttgcgcagctcagcggtaggttccagcaacgcacgcagcagggcttttttcatattgcgtgtaccaatgacccacgcggcaatgcggttgatagaggcatcgaagaagtcaaggccgatatgcacccggtcaaacagatcgtgacgcacaatctcactggcaattgcctgggtttcatcatccagcagcactacgtgatcgctgtcccagcgaaccggacggctgacgtgcagcagcaactgcggcacatacagcatggcggcggaaatcttgtcggaaatcacttcagtcgggtggaagtgcccggcgtccaggcacagcgcagtctggcggctggtggcataccccatgtaaaactcattggagccaaccgtgtagctctctgcgccaatgccaaacaatttgctctcaacggcgtcgatatggtgcgcagggtttagcttctcgctgatcacctcatccagtgctgccagcagacgctgacgcggggcgagacggtcaacggtgatatctttcataccatccgggatccagatgttcatcaccgatggtgtgccgagttgctcgccaaaataggccgaaacgcgacggctggctttgcagtgatcaatccagaactggcgaatgctgtcgtcggcatgggaaagcgtaaagccatcggcgcttagcggatgcgaaaagcaggaggggttaaaatccagaccgagctgattggctttcgcccattcaacccagtttttgaagtgctctggtttgatctggtcgcgcgagactggcgtatctgattccagatagatggcatgtaaattaagccgtttcggccccggaatcagccgcatagcctgttccagatcggcacgtagctcactggcattacgcgctttgcccggataattgcctgtggcctgaatccccccggtcagcgaaccttccgggttttcaaaaccggaaacatcatcgccctgccagcagtgcattgaaacgggtaaacgatcaagttggcgcagcgcctcctcgacatcaatccccaccgccgcgaaacgctgtttcgctagctcccaggcctgttccagttgagtggtcatgcgcaaagctcctttgtctgtcgtgtagagtgaatctgcgccacatagtgggcaatttcactgtcaggattaggggtaaaggtggtcagattcgcggtggtgctgacgacctgacggaaatcatccacattgttgagttcatccagcgtcattaactggatgccgatattgccgagcgtcgaggcttcaacaggcccggcgatcacccgaataccgcaggcatcggcgcatagctggttgagcagcgtgttctggcagcctccgccgacaatatgcagttgcgagaaatcttcaccgcgcagctgcgccagctcatgcaacacatcggcatacagcagcgccagactgtcgaaaatgcagcgcgccagttcagcatcactttccgggatcggttgcgccgtttcccgacacgcagcctgaatttcgctgcacatcgtctcaggattaataaagcgatcgtcattgggattgataatgaagcggcaagccggaagtgcctgtgtcgcggagataagcgccggaagatcgttgatttgctgctcctgaagcactcgctgaagcagccataagcccataatatttttcagcacccgatagcgaccttccgccccgccttcattggtgatgttggctgccagtgccgtgtcattggtaaatggcgtctggctttcgaagcccatcaatgaccaggtgccagaagagagataagcagcacgtgagccgtttaacggcgaggcgataaccgcgctggcggtatcatggctggcaacggcgaccactggaatctcattaccctgcgggcaaatccagtgacctatgacattacccggatgcgtcgggcgaccaaaccaggctttgttggccccgctccacgccagtagcgactcgtcccagtcgtcgctattgatattgaccagttgcgtggtcgtggcgttggtatattcccagttcatcttgccggtcaggcgataactgaagtaatccggcatcagcagagcgtgagcaatgtgtggaataagttcaggttgttgctccgtcagcgcacgcaactgataaagcgtattgaagggcagaaactggatgccgctacgttgataaatatcgcgtttgccgagttgttgttgtgcctgcgccattaggccattggtgcggctatcgcgataagcaacgggcaggcccacacgctgaccctgttggtcgagcagcacaaagtccacgccccaggtatcaatcccaatgctatcgatacgaatcccttcctcgcacaccttgtttaatccaaggcgaatggcactttcaaggctatccacatcccaggtgacatagccgttctgactatgcagcccattgttaaaacgatggatttcgcgcagcgtcaggctgcggcattcacgctcgtaacgcgccagcatcacgcgcccactggatgcgccgagatcgacggcgacacaattgcgaaaggtcataatgtgatcctgctgaatttcattacgaccagtctaaaaagcgcctgaattcgcgaccttctcgttactgacaggaaaatgggccattggcaaccagggaaagatgaacgtgatgatgttcacaatttgctgaattgtggtgatgtgatgctcaccgcatttcctgaaaattcacgctgtatcttgaaaaatcgacgttttttacgtggttttccgtcgaaaatttaaggtaagaacctgacctcgtgattactatttcgccgtgttgacgacatcaggaggccagtatgaccgtattacatagtgtggatttttttccgtctggtaacgcgtccgtggcgatagaaccccggctcccgcaggcggattttcctgaacatcatcatgattttcatgaaattgtgattgtcgaacatggcacgggtattcatgtgtttaatgggcagccctataccatcaccggtggcacggtctgtttcgtacgcgatcatgatcggcatctgtatgaacataccgataatctgtgtctgaccaatgtgctgtatcgctcgccggatcgatttcagtttctcgccgggctgaatcagttgctgccacaagagctggatgggcagtatccgtctcactggcgcgttaaccacagcgtattgcagcaggtgcgacagctggttgcacagatggaacagcaggaaggggaaaatgatttaccctcgaccgccagtcgcgagatcttgtttatgcaattactgctcttgctgcgtaaaagcagtttgcaggagaacctggaaaacagcgcatcacgtctcaacttgcttctggcctggctggaggaccattttgccgatgaggtgaattgggatgccgtggcggatcaattttctctttcactgcgtacgctacatcggcagcttaagcagcaaacgggactgacgcctcagcgatacctgaaccgcctgcgactgatgaaagcccgacatctgctacgccacagcgaggccagcgttactgacatcgcctatcgctgtggattcagcgacagtaaccacttttcgacgctttttcgccgagagtttaactggtcaccgcgtgatattcgccagggacgggatggctttctgcaataacgcgaatcttctcaacgtatttgtacgccatattgcgaataatcaacttcgttctctggccgaggtagccacggtggcgcatcagttaaaacttctcaaagatgatttttttgccagcgaccagcaggcagtcgctgtggctgaccgttatccgcaagatgtctttgctgaacatacacatgatttttgtgagctggtgattgtctggcgcggtaatggcctgcatgtactcaacgatcgcccttatcgcattacccgtggcgatctcttttacattcatgctgacgataaacactcctacgcttccgttaacgatctggttttgcagaatattatttattgcccggagcgtctgaagctgaatcttgactggcagggggcgattccgggatttaacgccagcgcagggcaaccacactggcgcttaggtagcatggggatggcgcaggcgcggcaggttatcggtcagcttgagcatgaaagtagtcagcatgtgccgtttgctaacgaaatggctgagttgctgttcgggcagttggtgatgttgctgaatcgccatcgttacaccagtgattcgttgccgccaacatccagcgaaacgttgctggataagctgattacccggctggcggctagcctgaaaagtccctttgcgctggataaattttgtgatgaggcatcgtgcagtgagcgcgttttgcgtcagcaatttcgccagcagactggaatgaccatcaatcaatatctgcgacaggtcagagtgtgtcatgcgcaatatcttctccagcatagccgcctgttaatcagtgatatttcgaccgaatgtggctttgaagatagtaactatttttcggtggtgtttacccgggaaaccgggatgacgcccagccagtggcgtcatctcaattcgcagaaagattaattcgccatgccgatgccgacgatgttagcggcgacaataatcaccacacaaccgaggctcaacaccgttaccggacggcgtcctgcattgttccactctttcagcaccagcccgacgataccgccgcacaatacatagaaactcatatgcagcatccaactgatgtagtcatactgcgccggaatgcgggcgtggccccaggcatagaaaaagaattgcagataccacatcaacccgcccagtgtcgagagtaacacattgtgaatgatcagcgattttgccagcgagaagtcggcttttagcgacaaatccttcacttttgccagacgaataaaacagaaaccgaggttaatgatcgcgccgccgcccatgatgacaacatagcttggcagagcgacatacagtggatcgacgccaagtgcggcagcggcttcatgcatcggttttgcggcgttcatcgcaaaggacatcccggcagagaaaatgccgcacatcaccgccagcaccagcccttttttcagattgaactcttcggctttaatgcccatcttgcgctctttcaactgcccggcgcgagttacaatccctacgccaatcagcgccaccagaacgccgagcaacgtcatgcgtccgccttcggtgctaatcaacacatcgaaattgccgttgataattggcgtcatcagcgtaccgacaatcaacgtaatgccaatggcgatgccaattcccatcgacatgccgagataacgcatggtcaggccgtagttgatattaccgatcccccacatagcgccgaacagaaaaacaggcagtcgcgtagagagactaaacgagctgtaatacgcccagaaattcggtagtaacagggcgctgatggcccacggcagaataatccacgaaacaatcccaccgactgaccacatggtttcccatgaccatttttttacttttttgaacggagcgtaaaaacaggctgcactggccgcgccgatcaaatgccaaaatatccccatcgtaatcgcgttactcatcttcttatcctcatcatttttcgtcgcgtcacatctccgacgagatgagtgtaaaaatcgtgctgtcgattaacctttcgcctgttgccgccgttgtcgatttactggcaatcacggcattaagtgggtgatttgcttcacatctcgggcattttcctgcaaaaccatacccttacgaaaagtacggcattgataatcattttcaatatcatttaattaactataatgaaccaactgcttacgcggcattaacaatcggccgcccgacaatactggagatgaatatgagctataccctgccatccctgccgtatgcttacgatgccctggaaccgcacttcgataagcagaccatggaaatccaccacaccaaacaccatcagacctacgtaaacaacgccaacgcggcgctggaaagcctgccagaatttgccaacctgccggttgaagagctgatcaccaaactggaccagctgccagcagacaagaaaaccgtactgcgcaacaacgctggcggtcacgctaaccacagcctgttctggaaaggtctgaaaaaaggcaccaccctgcagggtgacctgaaagcggctatcgaacgtgacttcggctccgttgataacttcaaagcagaatttgaaaaagcggcagcttcccgctttggttccggctgggcatggctggtgctgaaaggcgataaactggcggtggtttctactgctaaccaggattctccgctgatgggtgaagctatttctggcgcttccggcttcccgattatgggcctggatgtgtgggaacatgcttactacctgaaattccagaaccgccgtccggactacattaaagagttctggaacgtggtgaactgggacgaagcagcggcacgttttgcggcgaaaaaataatcatttgccgcctgctgcaatgaggcgtataggccgcatatcagcttaaaaaatgaaccatcgccaacggcggtggtttttttgtgatcaatttcaaaataaaaacaatgatccgataaaaataaaacagcgtttcaattgatgtggttttgatcacttttattgattaaatgaatgtctatcttcgtttccatcaacactgatgctccattgaggaattacgcatcagcccttaaaaatatgccgacaggtgatggaaatgcagataaaacgctcgattgagaaaatcccgggggggatgatgctcgtcccgctattccttggcgcactgtgccacaccttctcgccgggggcggggaaatattttggatcattcaccaacgggatgattaccggtacggtgcccattctggcggtgtggtttttttgcatgggggcgtcaataaaattaagcgcgacgggaacggtactgcgtaaatccggtacgctggtggtaactaaaattgccgtcgcgtgggtggttgcggcaattgcctcgcgtattattccggaacatggtgttgaagttggattctttgccggactttcaacgctggcgctggtggcggcgatggatatgaccaatggcggactttacgcttccatcatgcagcagtacggcacaaaagaagaagctggggcatttgtgttgatgtcgttggagtccgggccgctcatgacgatgattattctgggcactgccgggattgcctcgtttgaaccgcatgttttcgtcggcgcagtattaccgttcctggtgggctttgccctggggaaccttgaccctgaattgcgagaatttttcagcaaagcggtgcaaacgctgattccattctttgccttcgcgctgggcaataccattgatttgactgtgattgcccagactggtttgctggggatcctgttgggtgtggcagtaattatcgtgaccggtattccgttgattatcgccgataaattgattggcggtggcgatggcactgccggaattgccgcttccagttccgcaggggccgcggtagcgacacctgtgctgattgcagaaatggtgcctgcgtttaaaccgatggctccggcagcaacttcgctggtagcgacggcggtcattgtgacttcgattctggtgccaattcttacctctatctggtcacgtaaagtcaaagccagagcagcgaaaatcgaaattttaggtacggtgaaataaacctgcttccttaatccccacagccggatgaactaacgttcgtccggtttgctattgagttcctgcctggatacttaccgcgaaaacagcacgcctgacataaaataaatatggtctaatggggaaatttctcgtggagagggaacagatgcgatatccggttgatgtatacacaggcaagattcaggcttatcccgaaggcaaacccagcgcaattgctaaaatccaggttgatggtgagttgatgctgacggagctggggctggaaggtgacgagcaggcggagaaaaaggttcacggcgggccagacagagcgctgtgtcattatcctcgtgagcattatctctactgggcgcgggaatttccggaacaggcggagttgtttgttgcgcctgcgtttggtgaaaacctctcaaccgacggcctgacggaaagtaatgtttatatgggcgatattttccgctggggagaggcattaattcaggtcagccagccgcgctcgccttgctataaactcaattaccattttgatatcagcgatatagcgcagttgatgcaaaacacaggtaaggtggggtggttgtatagcgtgatagcgccagggaaagtgtctgcggacgcgccgctggagttggtttcccgtgtcagcgatgtgaccgtgcaggaggctgccgccatcgcatggcatatgccgtttgatgacgatcaatatcaccgtttactctccgctgccgggttatcgaaaagctggacgcggacgatgcaaaagcgccgactgagcggcaagatcgaagatttttcccgccggttgtggggaaaataacccccggagtgtaggcctgataagacgctatcagcgtcgcatcaggcatcctgctcaaatgccggatgcggcgtaaacgccttatcctgcctgcaaatgcgaagtttaactccgcttatacagcggcaaccaaatcaccagccgtaaaccgcccagcgggctgtcttctgccttcacccagccacgatgctgctgaatggcggtttcaacaatcgccagccccaaacctgtaccgccagattcacgatcgcgtgcttcatcggtacgatagaacggacggaaaatctgttcgcgatcttccgggctaacgccaggaccatcgtcgtccaccgtaatggtgataccgtctttatctaccgcaaagcccacttcaatcttcgtatgggaataacgcagagcattacgaacaatgttttccagcgcactttccagggcgttcggattgccgtacagcggccacggcccaggcgggaagttaactgtcaacgacttgcccatttgctcggcttcgaacgccgcgttatccagcacttcactccacaactggttggctttgatggtttcgctaaccagcgcgtttttttgctgattacgtgacatcaccaacagatcgttgatcatgctgtccagacgttgcgcttcggtttcaatacgctccagttccttgctttcaccgctacgacggcgcagtaacgccgtacccagttgcagacgcgtcagcggggtgcgcagctcgtgagagatatcagaaagcagacgctgctgagaggtcatcatgcgctccagcgcggtgaccatctggttaaaactggcacctgcggcaaggaattcctgtggccccgcttccagttccgggtgctggcgtaagtttccctgggcaacttcatcggcagcgtttttcagcttacgcgccggttttgccagactccaggccaaccacaacagcagcggcgtactgaccaacatggtgacaatcagcagtaatagcgggcggtcaaacagtaagttaatgaaatcggattgagaactgctggccggacgaatcagataaagttggtaattatcttcgccatcacgcacggagaacggaccgaccagttccacgcggccatactttttcttctgcggatgatcggcgttatcggcctgaccaataaagttacgaatgatctgcatttcgctgcgttcagcgccgatcacgcggccttcggtggtcaccaataacaaacgctgtcctggcggtgcccacttatcaatcgcccggaacagacgccgccaccacattaaatcgttgggcggatcgttcgccagctccgcttcgacatgctgctcaatcatcagcccctgacgctgttcgctatccagaagctcggtcatctggcgtgaatcgagcttgggtaacatcaaaaccaacatcaacaccagcgccagcgtcagccagaagatggcgaagatgcgcgcggttaagctgcctatcatgaagcagaaaccatcagatagccgcgaccacgcaaggttttaaaccacgggtgaccatctttacgatccggcagtttacgacgcaggttggaaatgtgcatatcaatagcgcggtcgaaaggcgtcaggcgtttgcccaacacttcctggcttaaatgttcacgggaaaccacctgacccagatgctgtgccagcaaatagagcagggtaaactcagtaccggttaactccagcgtttgcccgtcgaagctggcttcctgacggcctggattcagcactaaggcatcaacttccagtgtcggtgaaccgttgtcgttgttttgctgttgctcgctccagtgcgaacggcgcaggatcgcgcgaatacgtgccaccagctcacgatcattaaacggtttcgggagatagtcatctgcgcccagctcaaggccgagaacgcgatcaagttcactgccgcgcgccgtcaacataatgacaggcgtctggtgtgtctggcgaagtgcttttaatgtgtcgataccatttttcttcggcatcattacgtcaagcaaaagtaaatcaatgctgtcgtccagaagatcaagcgcctgttccccatcgtgggcaacaatcacgttgaagccttccatctcgagcagctcctttaatagggaagtcagctctcggtcatcatcaactaacaggattttattcattgtttaaatacctccgaggcagaaattacgtcatcagacgtcgctaatccatgactttacgttgttttacaccccctgacgcatgtttgcagcctgaatcgtaaactctctatcgttgaatcgcgacagaaagattttgggagcaaatgatgcgcatagttaccgctgccgtcatggcctcaacgctggcagtcagttcattaagccacgctgctgaagtcggttcaggcgataactggcatccgggtgaagaacttacgcagcgcagtacgcagagccatatgttcgacggcataagtttaaccgaacatcagcgtcagcagatgcgagatcttatgcaacaggcccggcacgaacagcctcctgttaatgttagcgaactggagacaatgcatcgccttgtcaccgcagaaaattttgatgaaaacgctgtgcgcgcacaggcagaaaaaatggcgaatgagcaaattgctcgtcaggttgagatggcaaaagtccgcaaccaaatgtatcgcctgttaacgccggagcagcaagcggttttaaacgagaaacatcaacaacgaatggagcagttgcgtgacgtgacgcaatggcaaaaaagttcatcgttgaagctattgagtagtagcaactcacgttcccagtagtaaaccctgttttccttgccatagacaccatccctgtcttcccccacatgctgtgggggttttttttatcctcaatttgcctgctgcttaatgcattgcagatgatttgcttccgttatactagcgtcagttgatagcgggagtatttatgaatcaatcttatggacggctggtcagtcgggcggcgattgctgcgacggcgatggcttcgctgctattgctgattaaaatttttgcatggtggtataccgggtcggtgagtattctcgccgcgctggtggattcgctggtggatatcggcgcgtcgttgacgaatttattggtggtgcgatattccctgcaacctgccgacgataatcactcgtttggtcacggtaaagctgagtccctcgcggcgctggcgcaaagtatgtttatctccggttcggcactattcctgtttttgacgggtattcaacatctgatatctccaacaccgatgacagatccaggcgtcggggttatcgtgacaattgtggcgctaatttgtacgattatccttgtctcgtttcagcgttgggtggtgcggcggacgcaaagccaggcggtgcgggctgatatgctacattaccagtctgatgttatgatgaacggcgcaattctgctggcgctggggttgtcctggtacggctggcatcgcgccgatgctctgtttgcattgggaatcggcatctatattttatatagcgcgttacgcatgggatatgaggcggtacagtcattactggatcgcgcattgcctgatgaggaacggcaagaaattattgatatcgtgacttcctggccgggtgttagcggcgctcacgatcttcgcacgcggcagtcagggccgacccgctttattcagattcatttggaaatggaagactctctgcctttggttcaggcacatatggtggcggatcaggtagagcaggctattttacggcgttttccgggatcggatgtaattatccatcaggacccctgttccgtcgtacccagggagggtaaacggtctatgctttcataatcagtataaaagagagccagacccgcattttgtgtataaaataccgccatttggcctgacctgaatcaattcagcaggaagtgattgttatactatttgcacattcgttggatcacttcgatgtgcaagaagacttccggcaacagatttcattttgcattccaaagttcagaggtagtcatgattaagaaaatcggtgtgttgacaagcggcggtgatgcgccaggcatgaacgccgcaattcgcggggttgttcgttctgcgctgacagaaggtctggaagtaatgggtatttatgacggctatctgggtctgtatgaagaccgtatggtacagctagaccgttacagcgtgtctgacatgatcaaccgtggcggtacgttcctcggttctgcgcgtttcccggaattccgcgacgagaacatccgcgccgtggctatcgaaaacctgaaaaaacgtggtatcgacgcgctggtggttatcggcggtgacggttcctacatgggtgcaatgcgtctgaccgaaatgggcttcccgtgcatcggtctgccgggcactatcgacaacgacatcaaaggcactgactacactatcggtttcttcactgcgctgagcaccgttgtagaagcgatcgaccgtctgcgtgacacctcttcttctcaccagcgtatttccgtggtggaagtgatgggccgttattgtggagatctgacgttggctgcggccattgccggtggctgtgaattcgttgtggttccggaagttgaattcagccgtgaagacctggtaaacgaaatcaaagcgggtatcgcgaaaggtaaaaaacacgcgatcgtggcgattaccgaacatatgtgtgatgttgacgaactggcgcatttcatcgagaaagaaaccggtcgtgaaacccgcgcaactgtgctgggccacatccagcgcggtggttctccggtgccttacgaccgtattctggcttcccgtatgggcgcttacgctatcgatctgctgctggcaggttacggcggtcgttgtgtaggtatccagaacgaacagctggttcaccacgacatcatcgacgctatcgaaaacatgaagcgtccgttcaaaggtgactggctggactgcgcgaaaaaactgtattaatgatttcggaaaaaggcagattcctttaccctgaaaccgatgacagaagcaaaaatgcctgatgcgcttcgcttatcaggcctacatgaattctgcaatttattgaatttgcaaacttttgtaggccggataaggcgttcgcgccgcatccggcatggacaaagcgcactttgtcagcaatatgaggcggatttcttccgcctttttaatccctcaacatatacccgcaagttatagccaatctttttttattctttaatgtttggttaaccttctggcacgctttgctcatcacaacacaacataagagagtcgggcgatgaacaagtggggcgtagggttaacatttttgctggcggcaaccagcgttatggcaaaggatattcagcttcttaacgtttcatatgatccaacgcgcgaattgtacgaacagtacaacaaggcattcagcgcccactggaaacagcaaactggtgataacgtggtgattcgtcagtcacacggtggctcaggtaaacaagcgacgtcggtaatcaacggtattgaagctgatgttgtcacgctggctctggcctatgacgtggacgcaattgcggaacgcgggcggattgataaagagtggatcaaacgtctgccggataactccgcaccgtacacttccaccattgttttcctggtacgtaagggaaatccgaagcagatccatgactggaacgatctgattaaaccgggtgtttcggtgatcacgcctaatccgaaaagctctggtggcgcgcgctggaactacctggcagcctggggctacgcgctgcatcacaacaacaacgatcaggcaaaagcacaggattttgttcgggcactgtataaaaacgtcgaagttctggattctggcgcgcgtggctccactaacacttttgtcgagcgcggaattggcgatgtactgattgcctgggaaaacgaagctctgctggcagcgaatgaactggggaaagataaattcgaaatcgtcacgccgagtgagtctatcctcgcagagccaaccgtgtcggtggtcgataaagtggtcgagaaaaaaggtactaaagaggtggcggaagcctacctgaaatatctctactcgccagaaggtcaggaaattgccgcgaaaaactactaccgtccgcgcgacgctgaggtggcgaaaaagtacgaaaatgcgtttccaaagctgaagttattcaccattgatgaagagttcggcggctggacgaaagcgcaaaaagagcattttgctaacggcggtacgttcgatcagatcagcaaacgctgatttccccaggataattatcaaacccggtggtttctcgcgaccgggttttttatttgtcacgattttgcgttacccttgcatctctttgaggtacagggaaaaaaagatgaaaaaagcgggtcttctttttttggtgatgatagttatcgccgttgtggctgccggtattggttactggaaattaaccggtgaagagtcggatacattacgtaagattgtccttgaggaatgtttgcccaatcagcagcaaaatcaaaatccttcgccatgtgcggaagtcaaacccaatgccggatacgtggttttaaaagatcttaatggcccactgcaatatctgttgatgccaacgtatcgtattaacggtactgaaagtcctttgttgaccgatccttcaacgccgaacttcttttggttggcttggcaggcgcgtgattttatgagcaaaaaatacggccagccggttcccgatcgcgcggtttctttggcgatcaactcccgcaccgggcgtacgcaaaaccattttcatattcatatctcttgtattcgtcctgatgtgcgcaaacagctggataacaatctggcgaacatcagcagccgctggttgccactgccaggtggtttgcgcgggcatgaatacctggcgcgtcgggtaacggaaagcgaactggtacaacgcagcccatttatgatgctggcagaagaagtacctgaggcgcgggaacatatgggacgctacgggctggcgatggtacggcagagtgataactcatttgtattgctggcgacacaacgaaatctactgacgcttaaccgtgcttcagccgaggaaattcaggatcatcagtgtgagattttgcgttaaggcgaagagttaaggaaagtaagtgccggatatgaaatccggcacctgtcagacttaagcctgtttagccgcttctgcagctttaacgattactgcgaaggcgtcagctttcagagaagcaccaccaaccagcgcgccgtcgatatccggctgagcaaacagttctgcagcgttagacgcgtttacagagccgccgtactgaatgatcacttgttcagcgatgttagcgtcaactttagcgatgtggtcacggatgaatttgtgaacagcctgtgcctgagccggagttgcagatttgccagtaccgattgcccatacaggttcgtaagcgataaccgcaccttcgaatgccgcagcaccctgagttttcagtaccgcgtcgatctgacgtgcgcaaacttcttcagttttgcccgcttcattttcagcttcggtttcaccgatgcacagaaccggagtcaggccctgctctttcagcaccgcgaattttttcgcgatcagttcgtcagattctttgtggtaagtacgacgttcagagtgaccgatgatgatgtactgtgcgccgatgtctttcagcatagcagcagaggtttcaccggtgaatgcgccggacaggttcaggtccacgttttgcgcacccagcatgatgtggctgccttcagcttcgcgcttcgccatatcgatatacatttccggtggtgcgattgcaaccgcacagccagcaacacctgccagctctttacgcaggttagaaaccagctcgtgaaccatgtggcggctgccgttcagtttccagttacccatcactaaaggatgtcgcattttaattctccacgcttataagcgaataaaggaagatggccgccccgcagggcagcaggtctgtgaaacagtatagagattcatcggcacaaaggctttgctttttgtcatttattcaaaccttcaagcgattcagatagcgccagcttaatcggttcaacagcgaaggtcagccccttttcgccgttgtccgcgacaacataacgcagtgcaccttctgtctcggtgtaataacgtttgtttttccccgccgttagtagcgactgcagttttttctggctttgtgttttggtcattaatggggtgagtgtgcggatcaccgctgccatgtattcctgagctttcgctttcgcggctttttgctctggcccctggatgggtagccaggtcatttgaatgcttttgatttttaaggtaccgcgctccagcgctgtagaagcatacaagttctcattaattttacttgcagcacgagtgagattggctttgtcgggactgctgtcgatggcacgaaattcgttcagtggcaggctgggattctggctgttaaagtcttctcgaaactggctgatggagagatcgaaagtaggggctccagccagcagataaggcgcggtcgttgccgtatctggtgtttgtgcatgcgcctctgttgtaacggttaatgcagaacataagagaaaaaacagcgtacaccctggcttcattgacagtaccttttgttatgactggctccgattaaaacgatatctgtcgcccttgtcaaaagggtagaatcctggaaaagacaaccatcaaggaacttacatgaccatacagcaatggttattctcatttaaagggcgtattggacgccgtgatttctggatttggataggcctgtggttcgcaggcatgctggtgcttttctcactggcgggtaagaatctactcgatattcagaccgcggcgttttgccttgtgtgcttgctctggccaacagcggcagtaactgttaagcgcttgcatgatcgcgggcgttccggcgcatgggcatttctgatgattgtggcgtggatgctgctggcgggtaactgggcgattttaccgggtgtctggcaatgggcggtggggcgttttgtcccgacgttgattctggtgatgatgcttatcgatcttggtgcgtttgttggcacacaaggcgaaaataaatatggtaaagatactcaggatgtgaagtataaagccgacaataaatcaagtaattaacctttaatatatctcttactgctatttttttccgggattgttatttccacgatgcaaatgacaatacccggaaaatccttctgaactcttcaccttaagcaatatcaaaaaaaatggtaatccataagatcattacttgtttgttcttcccttaacggcgcattattcttaagtcgtaatcgacagagaggcgaatatacagaggtgccctatgaaagatgtcgtagataaatgcagtactaaaggatgtgcgattgatatcggtacggtgattgataacgacaactgtaccagtaagttttcgcgcttttttgccacccgcgaagaagcagagtcttttatgaccaaactgaaagagcttgccgccgctacatcctctgcagatgaaggggccagcgtggcctataagattaaggatctggaggggcaagttgagcttgatgcggccttcactttctcatgccaggccgagatgattatttttgagttatcactgcgttcgttagcttgatggagttgctttagaaggagttaaacatggcttataaacacattggcgtggcaatttccgggaatgaagaagatgccttactggtgaataaagccctggagctcgccagacataatgacgctcacctgacgttaattcatattgatgatggcttaagcgagttgtatccgggtatctacttccctgcaacagaagatattcttcaattgttgaagaataagtcggataacaagctgtataaactgacgaaaaatattcaatggccgaagacaaaactgcgtattgaacgcggagaaatgccggaaacactgctggaaattatgcaaaaagagcagtgcgacctccttgtctgtggtcatcatcactcatttatcaaccgtttgatgccggcatatcgcgggatgatcaataagatgagtgcggatttgctcatcgtgccgtttatcgataagtaaccgcttaccagtaatgctccgctgtcatatggcccggtcggcgacgtaaatgtttcgtcatctgccgggtctctttcagcaactgttgtgtatcgcgcaccatctgtggattgccgcacagcatcacatggctggtttctttattcatcggcaggccaatcgtgctttccagttccccactttcaattaatgccggtatccgtccggtgagcgaccccgctgccgtttcccgactgaccaccgtctgaatgcgcagttttccttcgtagcgtttttccagttcctgcatcagtggcaaatagcttaagtcggcggcataacgtgcggcgtgcaccaggaccagatttttgaagcgatctaaatctttacctagttgcagaatcgataaataagggccaatcgctgtaccggttgccagcatccatagcgtttcgcagtgcggcacttcatcgagcacaaagaatcctgccgcttcgctaaccacctgcacttcatcgcctggtttcagtgccgccagtcgtgggcttaatttgccatcggggacggtgaccaggtaaaactccagatcgggattatcgggcgagtttacataggagtaggcgcgctggacgcgttcgccgtcgatttcaaggccaagcttggtaaattgcccggcggtaaacggaagcacgggggcgtgaacggtgagactaaacagggcgtcggtccagttctgcactttagtgactttgcctgttacccaatcagccatgtttttctcctgttttgattgacttgccttatcttcgttctccgaacaaaaaaattccagtcccgaaggactggaaggctcaatcgatcaaatcaatcagaggatgtgcacctgcatttccgggtctttgcgatccagatagtggatggactgaatgcggcgaatggtgcgtgacttgccgcggatcagcagcgtttcggtagtcgcgatattgcctttgcggctaatgccttccagcagatcgcctttggtaataccggtggcagagaagatgacgttatcgctgcgcgccatatcgcccaggcgcaatactttaccggcttcgatgcccatcgctttgcagcgtgccagctcctgctcgccaatgcgacgattctcttcgttgtcgcctttgacgtcatgacgcgccagcagacgaccgttcatgtcgccatctaatgcgcggatcaccgccgcagaaactacgccttccggcgcgccaccaataccgtacagcacgtcaacttcgctgtctggcatacaggtgagaattgaggccgcaacgtcgccgtccggaatagcaaatacgcgtacgccgagttgctgcatttcagcgataacggcatcgtggcgtggtttagccagaatcgttaccgtcagttcgctcaacggtttgccgagcgccgccgctacattgcgcaggttatccgccagcggcaggttcagatcaatggtgcctttggctcccggcccgacaatcagcttctccatatacatatccggcgcattgaggaagcagcctttatcgcctactgccagcaccgccagcgcgttagcctggcccatcgccgtcatgcgcgtgccttcaatcggatcaacagcaatatctaccgcgtcgccgcgaccagtaccgactttttcaccaatgtagagcatcggtgcttcgtcgatttcaccttcaccaatgacgatggtgccgtcaatgttgacctggttgagcataatacgcatggcgtttaccgccgcgccgtccgcggtgtttttatcgccgcgtcctaaccatttgtagccagccagcgccgctgattcggtgacgcgggaaaattcgatggcaagttctcgtctcatagcaaactctaagcagtaaggaatggcgcgaagtgtagcacaggggaagggagggattattgatgtgtgcggggttgcccccgcacgtttcgggactaccggatgcggcataaacgcttcattcggcatttacattattcgtcgtgttcttcccacgccatcgcgcgtttaaccgcttttttccagcctgcgtaacggtaattacgctcagtggtttcgatgcctggacggaactcgcgctcaatcaccgctttctcttgcagctcgtcgaggttctgccagaagccaaccgccaggcctgcgagataggccgcacccaatgcggtgacttcgcgcacttccgggcgctcaacgcgggtgccgagaatatcggactggaactgcatcaggaaattgtttgctactgcgccaccatccacgcgcagggcgtgcagacggataccagagtcggcctgcatcgcttccagcacgtcacgcgtctgataagcaatagactccagcgtcgcgcgtataatgtggttagcgttcaccccacgagtcagaccgaaaatcgccccgcgcgcatacgggtcccagtacggcgcacccagcccggtaaatgccggaaccacatacacaccattggtgttttgcactttggtggcgaaatattcggaatcgtaggcgtcgttaatcaacttcatttcatcgcgcagccactgaatggatgcgcctgccataaacaccgcaccttccaacgcatagttcacttcgccagtcgggccgcaggcgatggtggtcagcaggccgttttctgatttcaccgctttctcgccagtgttcatcagcataaagcagccagtgccataggtgttcttcgccatcccttctttcacgcacaactgaccaaacagcgcggcctgctggtcaccggcgatcccggagattggaatacgcgtgccgcctttgccgccaatgttagtctgaccgtatacttcggaagaacgacgcacttctggcagcatctcgcgcggaatatccagcacttccagcattttgtcgtcccagtccagggtatggatgttgaacaacatggtacgagaggcgttggtgtaatcggtcacatggacacggccctgagtcattttccagataagccacgtatcaaccgtaccaaacagcaattcaccacgacgtgcacgctcgcgagagccttccacatggtcgaggatccacttcactttggtgccagaaaagtacgggtcaatcaccagaccggtattgctgcggatataatcttctaaaccgtcacgttttaaatgctcgcagatttctgcggtacgacggcactgccagacaatggcgttatagataggcttgccggtttctttttcccagacaatagtggtttcacgctggttcgtaataccgatagctgcaatttgatcggaactgatatcggctttcgccagcacttctaccagcgtggagctttgggtggcccagatttccattgggtcgtgttctacccaacctggttttgggtagatttgctcaaattcgcgctgcgacacgctaatgatattggcatcgtgatccattacgaccgcgcgggagctggtggtgccctggtcgagcgcaacgatatattttttttcagtcatgtttaattgtcccgtagtcatattacagcgaagctttttgttctgaaggagttgtggtttccttttcttccacaacacagatatcgcaaggcaaatggcgaccaatcagtttgcggtaggcaaatgcacctacaatcgcgccaacgatagggccgaaaagcggcaccaggaagtaaggaatgtctctgccgccggtaaaggcgacattgccccagcccgccagccaggcaaagactttcggaccgaagtcacgcgctgggttcatggcaaaacctgtcaatgggcccatagatgcgccaatgaccgcaatcagtagaccaatcagcaagggagccaaagggccgcgtggtacaccgttgccatcgtccgttaacgccaggatcagccccatcagaatagcggtaatcaccatctcaactgcgaaagcctgcacaaaattgatatgaggattagggtaagtagagaaagtgccagccagatcaacactttcaacgctgccgcgaacaatgtgatgagtctgctcgaagtcgaaaaataaattgtagtaaagcccgtaaactaaagccgcagcacagaaagcgccggcaacttgtgaaacgataaaaggaataactttgcgcttgtcgaaacaggcaaacagccacaatgcaatggtaacagcgggattaagatgcgcgccggaaacccctgcggtcaggtagatggccattgccacccccagtccccaaatgacactgatttcccactgaccaaaagacgcaccagcgacttttagtgctgcaacgcaacccacaccgaagaaaatcaacaacccggtaccgaggaattcagcaatgcactggcctttcaaggttgatgtttgactcataatcggatcctgaagagttaatgtttgttgtatgcgtgaaagtcacggacctccacgatgcttgtaggcatgctgtaaacttatcgttaacgagcaaaaacgagaaatatcgaacttaaaatgtgtgtgcctcgtcataaaatgagcgttatcgcgccatttattccatctgattgtacatgatgcatgtttgttagatcattcgcgcaacaaatttattaacattttcgattgatgtggattatgtcaccaggagaaggatgaaaagtgtggcaaaccgtaatctgcaaggcgtgccgctggacagcgatggcgcggcttcatacaatcggagctaactaaagtgcgctcgtatttattaaggcgtcaccggtaatcgggacgaggatttttatccatcaacgccttgcaattcaggagaggtatgacaatgtcattagaagtgtttgagaaactggaagcaaaagtacagcaggcgattgataccatcactctgttgcagatggaaatcgaagagctgaaagaaaaaaacaactcactgtcgcaggaagttcaaaatgcccagcatcagcgcgaagagctggagcgtgagaacaaccatctgaaagaacagcagaacggctggcaggaacgtctgcaggccctgctgggtcgcatggaagaggtctgattacgcttcatcttccgcgtaatttctttactgtgtaggccaacaggtaacgcagaaaaaaggcaccttgcggtgcctttcttatcattcaatatccagcggatcttctgaaagaataatcccggtattgtcggcataaagatggtcgccggagaagaaggtgacaccgccaaaattgacgcggacatcgctttcgccaatgccttcgccagcggcaccaaccggaattgccgccatcgcctggatgccgatatccaactcttccaggtcatctacctgacgcaccgcgccgtaaatgaccagaccttcccattcattttgtactgccagacgcgccagttcagcatcgaccagtgcgcgacgaacagaaccaccgccatcgacgacaagaacacgaccacggccattctgttcgagcagatcgtacagcaacccgttgtcctcgaaacattttaccgtgattatttgtccgccaaacgacgcccgtccgccaaagttggagaacagcggttccacgacgttaacatcttcttgatagatgtcacaaagctcggaagtatcgtatttcataggcttaacattcagttgctgcgagaattttcagtatatcgcgctatgtgggctgttggcaaaatcatcaattgttaattgatatttgtcagttatgctgcccactggcttaggaatatccctaaaacaaacagcaggttagtcagtaacgctcccttgacagtacgttccagcattggtcgcatcgccaccgggtccatttcccgcatcacataacgggcttgcttcaccagtaatggtgccgccagcaggaacagccagccccacaggctatgcagcgaaaagagattaaacagcgccagacacaccagcgagcccatcagcaggcaggcatgataacgacgcgcgttcacttcacctaagcgcaccaccagcgtgtttttgccattttcgcggtcgctattgatatcacgcaggttattaatattcagtactgccgttgccagcaggccgcatgcggtcgccggaaggatcagtgccggaatcaatgtatgagcctgtaaataccagctccccatgacactcaaccagccaaagaaaaccagtacggaaatatcacccagaccgatataaccataaggacgattgcccacggtgtaggtgatagcggcaatgatcgacaacccgccaagaatcaggaaaccgacaaaatcggccagcgtatggcatgccactgcaaccagtgccagcccggagagacagatgagcacgacggtaataatgagcgcccgtttcatctcttgctgggtaatgacccctttttgcatgccgcgtagcggcccaatgcggtcaggtttatcgctgccttttaccgcatcgccgtaatcattggcgaggttagaaaggatctgtaatagcccggcggtaattagtgccagcagggcgaccagcggatcgaagtgaccttgccaccatgccagcgctgtcccgacgataattgcagcaaaggcgagggggagggttttaggtcgtaaactttccagccacgcctgagttcggctaatttgttgttcagtcataatacgcgccaataaaaatggggcctttcagccccatcaaacaatgatgaaaatgattgaacgcgattataggataaaacggctcagatcttcatctgccaccaacgcatccagatgtttgctcacataatctgcgtcaatagtgatattttgaccgcttaaatcgctggcgtcgtaggaaatctcttccattaaacgctccagaacagtgtgtaaacgacgagcaccgatgttttcggtagattcgttcacctgccatgccgcttccgcgatgcgtttaataccggagtcggtaaactcgatatttacgccttcagtcgccatcagtgctttgtactgcacggtgatagaggcattcggctcggtcagaatacgctcgaagtcgctggtggtcagcgcctgcagttcaacgcggattggcagacgaccttgcagttccgggatcaggtcagacggtttcgcaatctggaacgcgccagaagcgataaacagaatgtggtcagttttgaccatcccgtgtttggtggaaacggtgcaaccttctaccagcggcagcaggtcacgctgaacgccttcacgagaaacatccggaccggaagactcgccgcgcttacagattttgtcgatttcgtcgataaacacgatcccgtgctgctcaacagcgtcgatagcgtcttgcttcagctcttccgggttcaccagtttcgccgcttcttcttcaatcagcagcttcatggcgtctttgattttcagcttacgcgctttttgcttctggccgcccaggttctggaacatggactgcagctggctggtcatctcttccatgcccggaggagccataatttcaacgcccatcggtgctgcggcaagatcgatctcgatttctttgtcatcaagctggccttcacgcagttttttgcggaatgcctgacgagcagcggacggttcctgctgctgttcggtctgtccccagttgtttttagcaggtgggatcagcacgtcgagaatacgttcttctgccagttcttcagcgcgataacggtttttctcgatagcctggacgcgtaccattttcacggcggcatcggtcagatcgcgaataatagaatccacttccttaccgacgtagcccacttcggtgaatttggtcgcttcaactttgatgaacggcgcattcgccagcttagccagacgacgggcgatttcagttttaccgacaccggtcgggccgatcatcaggatatttttcggggtcacttcatggcgcagctcttcgttgagctgcatgcgacgccagcggttacgcagagcaatcgccacagaacgcttggcgttgtcctggccgatgatgtgcttatccagttcgctgacgatttcgcgtggggtcatttcagacatgggagatccttacgctttgtagcttaattcttcgatggtgtggaaatggttggtatagatgcaaatgtcgcctgcaatatccaacgccttttcagcaatttcacgggcgctaagttcagtgttttctaacagcgcgcgcgccgcagcctgggcgtaagggccgccggagccgatagcaataagatcgttttctggctgcaccacgtcaccgttaccggtgatgataagcgatgcagtttcatccgcgactgccagcagtgcttcaagtttgcgcagcatgcgatcggtacgccagtcttttgccagctcaacggcggctttgaccagatggccctgatgcatttccagtttacgttcaaacagttcgaacagcgtaaaagcatccgcagtaccgcccgcaaagcccgcgatgactttgtcgttgtacagacggcggacctttttcacgttgcctttcattacggtattgcccaacgtggcctgaccatcaccagcgatgaccacatggccgttacggcgtacgcttactatagttgtcacgagctgaccccttggttacgaatacagagtacaaaccccgtacaaaagtacggggcataatgcaattatagatgggggggattttgagggtttcaacccccggcggcgagccgaatgcagtttgtatgacccgccatcttcaaccgattgagggtgctgtctgcgttctctttgcctttcaccgggccaatgaccacacgattccagccattgttggtggtgattttcgagtcaaagccttcgaacgccagctgagcacgtaccgtctctgcctgttccgcgcctctgaacgaaccgcactgcaccatccagcggcgttcgtcttttttctccgccgtcggttttggcgcgtcagcggcacgagcaactggcgcagcttgctgcggcttcgactgcgcagtcgtgtgcgcaggagtttgcagcagatcctggtacggctgctgagaagaagccggtttagactggcgcggttgcgcctgtaccggtgcggcttgcgacgtacgcgtctgctgctgccagctttgttcagtcgtacgcgactgctgagccaggcgttgctgttccgctaattgctgcgcctgacgttggcgctgtagcgtttgctgacgctgttccggcgtctgttcattccacggaacttcaaccagctgcgttggctgctggcgcatatcagcctgcatttgttcaagaagctgacgttgttctggtgtcagttgctccggcgttttcacttcaccaccggcagaaggttctgtgggcgcacgcactcccggctggcgactttccagctctttaatgtagcgccagcgttcttctggttttggtggtagtccgtttccggtcactttctggctttgcagcgtctcggactcttctttcttgtgatgcgtaatgaagtacagaccaccgataaaggtcacaagaacggcggcagcaatagcgaccatagcgggagaaaccgcaggcagatttcgttgctttttccgtgaggtgctcttttttcgccgcgaaggtgccggttggctgcggcgtacataatctcgttgtgccactatcgtttcgctgtatttattcgttcgtcagcccgccatgttacttaagcggcgggcctttgaccagtcacggcagtcttaaaggtttactttaaggtaacgcgcgtgttgatccccggatgataagttcgcagtccattaaacgagagccactgccaacgtgttgcccctgcatttgatcaagcaataacagcatagcttcccgaccgatttcgtaacgcggctgcgcgatggttgtcagcggcggatcacaaaattgcgtcaggtcgatgttatcaaaaccgattatggaaaggtcttccgggactttcagcccctggcgttttgcctgagaaagtgcgccgagcgccatcacatcgctatggcagaagacagcagtaggcggttgtggaagatcaagcagctgctgcatcgctttgcttccggcttcgaaggtgaagtcgccacgggcgatgtattgcggatcaaccataatgccgcagcgacgcagcgcctgaacatagccttgcaggcggtagtgacacagcggcatctcttcgggaccggctatacagccaatccgtttatgcccttgctcatataaataatttactgcatcaaatgcggcggtcagattgtcgatatgaactgtaggcagctccagctccggtgcaaattcgttcgccatcaccatcggcggcagattacgctgttcctcaatgctggcatcaaacggcagccttgaacccagcaacaacatgccatcaatttgcttggtgatgatcaaatcgataaaggttttttcctgctgattttgatgcgcacagtcgccaatcagcaccagatatccgtgatttgccgccgtaacttcgataccgcgaataatttcgctaaagaagggatcgcagatatccgggacaatcaccagaatggtgcgggattcattacgcttgacgttgcgccccataggctgcggtaaataacccacttcccgggccgctttttcaacccgattacgggtggcctgggagactttatcgggattcattaatgctcgggagacggtcgctgtagagacttttgccttgagggcaacgtctttcatggtcgcggcagtttcctgcttcttcgctttcacactcactcctcgcctggcacgtcaggcgtactacatccatgtttacttcacatcggcaacatttttagcagatagcgcgtgaaaacggttacagaattttcatgaaaagtgtgatgaatattgaatttttcgatccgcctcgcatcgtgagcggtttaaccctcaatcggatcaacatccagcacccatttcaccttacgggaatccggtattgtattgatgagcgccagcgtaccgttaatgatgtgttgcaagcgcacgcgggaagggtgctgcaacaatatctgccagcgccagcgaccgccacgtttaggtgccagagccggaaccggaccgagaacccacagtttctcgtctgccagtgggctggagaggatcagattacgcagttgttgcaggaacaatggcgcgtgctgattgttatgatcttccgcacgcacaatcacatggctggtccacggcggtagctgcatcattcgccgctcagccagcgcctgttcggcaaaggcgtcgtagcctttatagagcaacgtttgcaacagaggatgttccggatggtgcgtttgcagcaccacttcgccctgtttacccgcacgcccggcacgaccggcgacctgggtgtaaagctgagcgaaacgctctgccgagcgaaaatcggcagaaaacagcgcgccgtccacgtccagtaatgcaaccagcgtcacatccgggaaatggtgacctttcgccagcatttgtgtaccaatcaaaatccgcgcgccgccgcgatgtacttctgccagttgctgttccagcgcccctttgcggctggtggtatcgcggtcgatacgagaaatgggcacgccggggaacaacggcgcgagcgtctgttcaagctgttcggtgcccagccccacggggaccaggtgcgtggaaccgcaggaagggcactggcgcggcaccggacgctgactgtcacagtggtggcagcgcagatggtgctgcgcctgatgcagcgtgtagtagtgatcgcaacgtgggcattcggcaatccagccacagtcgtggcacagcagtgcaggcgcaaagccacggcggttaagaaagagaatgacctggttatcagcctgtaaatgctggcgcatacgagtgattaacgccggagccagacctgcctgcaccttctgaccttttaaatccagcacatgttgaattgccggacgcgcattccctgcccgacgggtcaggcgcagcaggcggtattttttctgctggacgttgcataacgtttccagcgcgggcgttgcggagccaagaataatcgggatttgctcgctgtgcgcacgatacaccgccaggtcgcgggcatgatagcgccagccttcctgctgcttgtaggagctgtcgtgctcttcatcaatgacaatcacgccgagatttttaaacggcgtaaacagcgcggagcgggtgccgatcacaatcgccgcctcaccatttttcgctttcagccacgccgaaagacgctcgctgtcgttcaggccggaatgcagaacttccacgggggcattaaaacgttcacgaaaacgggcgatagtttgcggtgtcaggccgatttccggcaccatcaccagcgcctgtttgccctgagcgagcacgttttccagtacgctgagataaacctccgttttaccggaaccggtaacgcccgccagcagccaggcagaaaaagtatctgccgcgctatgaattgcgccaacggcggtggcctgttcggtattcaatcgcaaccgctcaccagaaacggcatagttcgttcgccagtcgctaaactctggtgtttcacttgctaaatcacacagaccttttttgcgtagcgcctgcaacgcggcatcattaaattcgagcgtggcgacctggtcgcgccagattttgccttgccgtaacgccgccagcgcctgttgttgcttgggggagcgtttcaggctgttcagatccaccgcctggccttgttcagtggcaaaccagtaccacatcggcgcgttcgccgcaggccgcccctggcgtagtaaaatcggcaaggcatgaaacagcacatcgccaatcggatgatgatagtaatctgccgcccatagcagcaatcgccagacggagtgagtaaacaccggctcactatccagcacttcgactaccgcttttagctcattgagcggcagttcgctggcatcgctaactgataccacaatcccgatgcgctcctgctgtttgccaaacggcacgcgcacgcgacacccagctttaaccgtcatgccttctggcagcagatagtcaaaggtacgaggaagcggaacgggcaaggcaacgtgggcaacgggcatagcatcatcctgacttgaaattcggtgggttagtatacacattgccgtagaagagtgcggatcagtttgcatacgctggttaatttctgtatgatttcgcgccttcgtacgaaatgatcgtattgaagctatacttttaacatcgcgtggtgtctggcgttagggctggaagagcgacgcggccttaaaccgaggttttcccatgaaaaaagatattcacccgaaatacgaagaaattactgctagctgctcttgcggtaacgtaatgaaaatccgctccaccgttggtcatgacctgaacctcgacgtgtgcagcaagtgccacccgttcttcactggcaaacagcgtgatgttgctaccggtggccgtgttgaccgcttcaacaagcgtttcaacatcccgggcagcaaataagaccggatttccgaaaaaagcgccgcacggcgctttttttgtgcctgaattttggtcgtattaccacgaaaacagcggccattctttggcgaccgtggtgagttgtggcgcatcgaaaacggcttgtggcgagaccaccgtttcctcaagcggaatattcttgccgtaacgttctttgagctttgcctgaacttgtgggctgctcaggtcgaactctttcaacttctgctgctcgcccacgcgcattcccagcgcgttctggtaaaccttccacaccacttccgaacagtactggcgatcgtcgctccatgagaagctgaaatcatacggtttaccgagataacgttttgccgtttgcgccagtttttgctgttgttcaacactcagtccgccttcaacgcggcgaacaacgtatttgcccttttcaccatgggcgatccactgcttgagcggggtgtatttcaccgggccgactgcttcaaaaacgtagggctttttgttgcgtatcaccagcataccggtgtggctataatcggtatgggtcgccagttggatcgctttactttgcgatgagcgagagatctgaaagatgatgtcgccggtttgtggctgccaggcaaaggcaggtacagaaaccagcaggctgaggatcagcagcctgtttttcatagttaaacgtccatgtataaaaagcggtgggtcgcagacaacgtgctcgttgtttatgccggatgcggcgtgaacgccttatccggcctacaagttcgtgcaaattcaataaattgcaatatgacgtaggcctgataagcgtagcgcatcaggcgattccactccgcgccgctcttttttgctttagtattcccacgtctccgggttaatccccatctcacgcatgatctcttttgccgcttccgggatttcgtcgctgcgctctttacgcagatcggcatcatccggcaaaggttgcccggtaaaggcatgcagaaacgcttcgcacagcagctcgctgttggtagcgtgacgcaggttgttcacctgacgacgcgtgcgttcatcggtgaggatttttaacaccttaagaggaatggaaaccgtaatctttttgacttgttcactcttcttgccgtgctcagcgtatgggctgatatattcgccgctccattcagccatgagatacttaatcctcttcgtcaataaattgagaccagaccacacagttgatgtgggtactgaccgtaaacccgcatagtttaccgtacaggcgttaccgtgacatcgtgtaatgcacctgtcggcgtgataatgcatataattttaacggctatttgggatttgctcaatctatacgcaaagaagtttagatgtccagatgtattgacgtccattaacacaatgtttactctggtgcctgacatttcaccgacaaagcccagggaacttcatcacatgacgcgtaaacaggccaccatcgcagtgcgtagcgggttaaatgacgacgaacagtatggttgcgttgtcccaccgatccatctttccagcacctataactttaccggatttaatgaaccgcgcgcgcatgattactcgcgtcgcggcaacccaacgcgcgatgtggttcagcgtgcgctggcagaactggaaggtggtgctggtgcagtacttactaataccggcatgtccgcgattcacctggtaacgaccgtctttttgaaacctggcgatctgctggttgcgccgcacgactgctacggcggtagctatcgcctgttcgacagtctggcgaaacgcggttgctatcgcgtgttgtttgttgatcaaggcgatgaacaggcattacgggcagcgctggcagaaaaacccaaactggtactggtagaaagcccaagtaatccattgttacgcgtcgtggatattgcgaaaatctgccatctggcaagggaagtcggggcggtgagcgtggtggataacaccttcttaagcccggcattacaaaatccgctggcattaggtgccgatctggtgttgcattcatgcacgaaatatctgaacggtcactcagacgtagtggccggcgtggtgattgctaaagacccggacgttgtcactgaactggcctggtgggcaaacaatattggcgtgacgggcggcgcgtttgacagctatctgctgctacgtgggttgcgaacgctggtgccgcgtatggagctggcgcagcgcaacgcgcaggcgattgtgaaatacctgcaaacccagccgttggtgaaaaaactgtatcacccgtcgttgccggaaaatcaggggcatgaaattgccgcgcgccagcaaaaaggctttggcgcaatgttgagttttgaactggatggcgatgagcagacgctgcgtcgtttcctgggcgggctgtcgttgtttacgctggcggaatcattagggggagtggaaagtttaatctctcacgccgcaaccatgacacatgcaggcatggcaccagaagcgcgtgctgccgccgggatctccgagacgctgctgcgtatctccaccggtattgaagatggcgaagatttaattgccgacctggaaaatggcttccgggctgcaaacaaggggtaaaaatgagtgtgattgcgcaggcaggggcgaaaggtcgtcagctgcataaatttggtggcagtagtctggctgatgtgaagtgttatttgcgtgtcgcgggcattatggcggagtactctcagcctgacgatatgatggtggtttccgccgccggtagcaccactaaccagttgattaactggttgaaactaagccagaccgatcgtctctctgcgcatcaggttcaacaaacgctgcgtcgctatcagtgcgatctgattagcggtctgctacccgctgaagaagccgatagcctcattagcgcttttgtcagcgaccttgagcgcctggcggcgctgctcgacagcggtattaacgacgcagtgtatgcggaagtggtgggccacggggaagtatggtcggcacgtctgatgtctgcggtacttaatcaacaagggctgccagcggcctggcttgatgcccgcgagtttttacgcgctgaacgcgccgcacaaccgcaggttgatgaagggctttcttacccgttgctgcaacagctgctggtgcaacatccgggcaaacgtctggtggtgaccggatttatcagccgcaacaacgccggtgaaacggtgctgctggggcgtaacggttccgactattccgcgacacaaatcggtgcgctggcgggtgtttctcgcgtaaccatctggagcgacgtcgccggggtatacagtgccgacccgcgtaaagtgaaagatgcctgcctgctgccgttgctgcgtctggatgaggccagcgaactggcgcgcctggcggctcccgttcttcacgcccgtactttacagccggtttctggcagcgaaatcgacctgcaactgcgctgtagctacacgccggatcaaggttccacgcgcattgaacgcgtgctggcctccggtactggtgcgcgtattgtcaccagccacgatgatgtctgtttgattgagtttcaggtgcccgccagtcaggatttcaaactggcgcataaagagatcgaccaaatcctgaaacgcgcgcaggtacgcccgctggcggttggcgtacataacgatcgccagttgctgcaattttgctacacctcagaagtggccgacagtgcgctgaaaatcctcgacgaagcgggattacctggcgaactgcgcctgcgtcaggggctggcgctggtggcgatggtcggtgcaggcgtcacccgtaacccgctgcattgccaccgcttctggcagcaactgaaaggccagccggtcgaatttacctggcagtccgatgacggcatcagcctggtggcagtactgcgcaccggcccgaccgaaagcctgattcaggggctgcatcagtccgtcttccgcgcagaaaaacgcatcggcctggtattgttcggtaagggcaatatcggttcccgttggctggaactgttcgcccgtgagcagagcacgctttcggcacgtaccggctttgagtttgtgctggcaggtgtggtggacagccgccgcagcctgttgagctatgacgggctggacgccagccgcgcgttagccttcttcaacgatgaagcggttgagcaggatgaagagtcgttgttcctgtggatgcgcgcccatccgtatgatgatttagtggtgctggacgttaccgccagccagcagcttgctgatcagtatcttgatttcgccagccacggtttccacgttatcagcgccaacaaactggcgggagccagcgacagcaataaatatcgccagatccacgacgccttcgaaaaaaccgggcgtcactggctgtacaatgccaccgtcggtgcgggcttgccgatcaaccacaccgtgcgcgatctgatcgacagcggcgatactattttgtcgatcagcgggatcttctccggcacgctctcctggctgttcctgcaattcgacggtagcgtgccgtttaccgagctggtggatcaggcgtggcagcagggcttaaccgaacctgacccgcgtgacgatctctctggcaaagacgtgatgcgcaagctggtgattctggcgcgtgaagcaggttacaacatcgaaccggatcaggtacgtgtggaatcgctggtgcctgctcattgcgaaggcggcagcatcgaccatttctttgaaaatggcgatgaactgaacgagcagatggtgcaacggctggaagcggcccgcgaaatggggctggtgctgcgctacgtggcgcgtttcgatgccaacggtaaagcgcgtgtaggcgtggaagcggtgcgtgaagatcatccgttggcatcactgctgccgtgcgataacgtctttgccatcgaaagccgctggtatcgcgataaccctctggtgatccgcggacctggcgctgggcgcgacgtcaccgccggggcgattcagtcggatatcaaccggctggcacagttgttgtaatttcagaaatttaataatgcccggtactcatgttttcgggtttatggtttctaatgaaatatattgaattatcataggattaggccggattaagcgtttacgacgaatccggcaagaagcaataagtacatggttagtttatatttgcagtccggtttgctttgcataccggattttctttttcttaccatcctgaagttttttcatcttccctgatttttcctcaccatcattggtcatttttcggttgacgcccttcggcttttccttcatctttacatctggacgtctaaacggatagatgtgcacaacacaacatataactacaagcgattgatgaggtaaggtatgagcttttttcacgccagccagcgggatgccctgaatcagagcctggcagaagtccaggggcagattaacgtttcgttcgagtttttcccgccgcgtaccagtgaaatggagcagaccctgtggaactccatcgatcgccttagcagcctgaaaccgaagtttgtatcggtgacctatggcgcgaactccggcgagcgcgaccgtacgcacagcattattaaaggcattaaagatcgcactggtctggaagcggcaccgcatcttacttgcattgatgcgacgcccgacgagctgcgcaccattgcacgcgactactggaataacggtattcgtcatatcgtggcgctgcgtggcgatctgccgccgggaagtggtaagccagaaatgtatgcttctgacctggtgacgctgttaaaagaagtggcagatttcgatatctccgtggcggcgtatccggaagttcacccggaagcaaaaagcgctcaggcggatttgcttaatctgaaacgcaaagtggatgccggagccaaccgcgcgattactcagttcttcttcgatgtcgaaagctacctgcgttttcgtgaccgctgtgtatcggcgggcattgatgtggaaattattccgggaattttgccggtatctaactttaaacaggcgaagaaatttgccgatatgaccaacgtgcgtattccggcgtggatggcgcaaatgttcgacggtctggatgatgatgccgaaacccgcaaactggttggcgcgaatattgccatggatatggtgaagattttaagccgtgaaggagtgaaagatttccacttctatacgcttaaccgtgctgaaatgagttacgcgatttgccatacgctgggggttcgacctggtttataaatagtgtggcttttgtgaaaatcacacagtgatcacaaattttaaacagagcacaaaatgctgcctcgaaatgagggcgggaaaataaggttatcagccttgttttctccctcattacttgaaggatatgaagctaaaacccttttttataaagcatttgtccgaattcggacataatcaaaaaagcttaattaagatcaatttgatctacatctctttaaccaacaatatgtaagatctcaactatcgcatccgtggattaattcaattataacttctctctaacgctgtgtatcgtaacggtaacactgtagaggggagcacattgatgagcacgtcagacgatatccataacaccacagccactggcaaatgcccgttccatcagggcggtcacgaccagagtgcgggggcgggcacaaccactcgcgactggtggccaaatcaacttcgtgttgacctgttaaaccaacattctaatcgttctaacccactgggtgaggactttgactaccgcaaagaattcagcaaattagattactacggcctgaaaaaagatctgaaagccctgttgacagaatctcaaccgtggtggccagccgactggggcagttacgccggtctgtttattcgtatggcctggcacggcgcggggacttaccgttcaatcgatggacgcggtggcgcgggtcgtggtcagcaacgttttgcaccgctgaactcctggccggataacgtaagcctcgataaagcgcgtcgcctgttgtggccaatcaaacagaaatatggtcagaaaatctcctgggccgacctgtttatcctcgcgggtaacgtggcgctagaaaactccggcttccgtaccttcggttttggtgccggtcgtgaagacgtctgggaaccggatctggatgttaactggggtgatgaaaaagcctggctgactcaccgtcatccggaagcgctggcgaaagcaccgctgggtgcaaccgagatgggtctgatttacgttaacccggaaggcccggatcacagcggcgaaccgctttctgcggcagcagctatccgcgcgaccttcggcaacatgggcatgaacgacgaagaaaccgtggcgctgattgcgggtggtcatacgctgggtaaaacccacggtgccggtccgacatcaaatgtaggtcctgatccagaagctgcaccgattgaagaacaaggtttaggttgggcgagcacttacggcagcggcgttggcgcagatgccattacctctggtctggaagtagtctggacccagacgccgacccagtggagcaactatttcttcgagaacctgttcaagtatgagtgggtacagacccgcagcccggctggcgcaatccagttcgaagcggtagacgcaccggaaattatcccggatccgtttgatccgtcgaagaaacgtaaaccgacaatgctggtgaccgacctgacgctgcgttttgatcctgagttcgagaagatctctcgtcgtttcctcaacgatccgcaggcgttcaacgaagcctttgcccgtgcctggttcaaactgacgcacagggatatggggccgaaatctcgctacatcgggccggaagtgccgaaagaagatctgatctggcaagatccgctgccgcagccgatctacaacccgaccgagcaggacattatcgatctgaaattcgcgattgcggattctggtctgtctgttagtgagctggtatcggtggcctgggcatctgcttctaccttccgtggtggcgacaaacgcggtggtgccaacggtgcgcgtctggcattaatgccgcagcgcgactgggatgtgaacgccgcagccgttcgtgctctgcctgttctggagaaaatccagaaagagtctggtaaagcctcgctggcggatatcatagtgctggctggtgtggttggtgttgagaaagccgcaagcgccgcaggtttgagcattcatgtaccgtttgcgccgggtcgcgttgatgcgcgtcaggatcagactgacattgagatgtttgagctgctggagccaattgctgacggtttccgtaactatcgcgctcgtctggacgtttccaccaccgagtcactgctgatcgacaaagcacagcaactgacgctgaccgcgccggaaatgactgcgctggtgggcggcatgcgtgtactgggtgccaacttcgatggcagcaaaaacggcgtcttcactgaccgcgttggcgtattgagcaatgacttcttcgtgaacttgctggatatgcgttacgagtggaaagcgaccgacgaatcgaaagagctgttcgaaggccgtgaccgtgaaaccggcgaagtgaaatttacggccagccgtgcggatctggtgtttggttctaactccgtcctgcgtgcggtggcggaagtttacgccagtagcgatgcccacgagaagtttgttaaagacttcgtggcggcatgggtgaaagtgatgaacctcgaccgtttcgacctgctgtaatctgaccccgttcagcggctgcttgctggcagtcgctgaacgttctttaccagcgtatagtgggcgaacgaaaactacacactggatctctcatgtctgccgcaggaaagagcaacccactggcaatcagtggcctggttgtgctcacacttatctggagttatagctggattttcatgaagcaagtcaccagttacatcggtgccttcgactttaccgccttacgctgcattttcggcgctctcgttttattcatcgtccttttattacgtggtcgcggaatgcgcccgacaccgtttaaatacaccttagccattgccctgttacaaacctgcgggatggttggtctggcgcagtgggcgttggtcagcggaggtgcggggaaggtggcgatcctgagctataccatgccgttctgggtggtgattttcgccgcgttgtttctcggtgaacgcctgcgacgtgggcaatatttcgcgattctgattgccgctttcggcttatttttggtgttgcagccgtggcaactcgatttctcttcgatgaaaagtgccatgctggcaatcctctccggcgtcagttggggggcgagcgcgattgttgctaaacgtctgtatgcccgtcatccgcgcgtggatttattgtcgttaacatcctggcagatgctgtatgcggcgctggtgatgagtgtggtcgctttactggtgccgcaacgtgaaattgactggcagcccaccgtgttctgggcgctggcctacagtgcgattctggcgacggcactggcgtggagcttatggttgtttgtattgaaaaacttgcctgccagtattgccagcttaagcacactggccgttcccgtttgcggcgtactcttttcctggtggctgctcggcgagaatccgggggccgttgaaggtagcggtattgtgctgattgtgctggcactggcgctggtgagccgtaagaaaaaagaagccgtcagtgtaaaaaggatctgaattttttcttcatgtggggcgatctcttatttaacaaaataacgataatgccccaccatccgccagttaaacagcacatcttcttcctgcgcgcctgcgccaatgttatgtatcaccagcggcgtaccgtcgcgggcgaagccatctgaaaccaccccaatatgtgccagcccgttatccagtcgccaggagacaatatcgcccgcttgatagtcactggggttcttgctggtggggcgtgttttatcatggcggctaaaccaggtttccagattaggcacccgacggtgatcgatgttgctgtccgggcgctttaacttccatttttgcgggtactcagcaaaattcttcgccatatcttcgtgaaccagtttctgcaaatcgaccttctggctgcgcaatgcgcggatcaccacatcggaacatacaccgcgttcttgcggaacatcaccgccaggataagtaagctgcacatacgccggatcgtaaaatagcgtgctgccaatttgctgtctggcaccgtctgcgatggcaaggttggtattggcctggatttgtaccacggttggtggaacggcgggagattttaaggagtggctggtaaatgccgttagcaggctgagcagcgccagtgaagctttcatctggttcgtccgtgaaaataagagtcacagattcgaccttccgggctaacgattgttctgtagagaaaatgtccagaagcggataaaaaattcctgaacaacgtgggagtttcagattactggcacagagtgccggatgcggagtgaacgccttatccggcctacaaaagcacgcaaattcaatatattgcagagattgcgtaggcctgataagcgtagcgcatcaggcaattttgcgttcaaactcccggacaagccgggagtttggagtaggttattcccactcttgcaggaaacgctgaccgtactggtcggctaccagcagagcggcgtaaacctgatctggcgtcgcgccgccaggcatgttgtgaatggtttcaccttctgcacatgccgcttctgccacaattcgcattttcgccgggacatcttctttaatatccagttgagcgagagttattggcaaacctaccgcatggctaagggcagctacggtttcgatttcctccaccggcgcattttccagaaccagctgcgtcagcgtaccgaatgccactttttcaccgtgataatagtgatgcgcgtccgggatagcggtcaggccgttatgcactgcgtgcgccgcagccagaccaccactttcaaaaccaacaccgctcaaataggtgttcgcttcaatcacgcgctccagcgccggagtcactacatgctgttcggcagcaagcatcgctttttcgccttcttccagcagggtgttgtagcacagttcagccagtgccagcgcagcctgggtgcacttgccgcccgccatggtggtcgcgccgctacgagagcaggcacgcgcttcaaaccaggttgccagcgcatcgccgatacccgccgctaacagacgtgcaggtgcgccagcgacgattttggtgtcgacaatgaccatattcgggttatttggcaacagcagatagcggtcaaactcaccctcatcggtgtagataacagacaatgcgctgcacggtgcatcggtagaggcgatagtcggtgcgatcgctaccggaacacccatgaaatgtgccagtgctttggcagtatcgagggtttttccgccaccgataccgagaattgcgccacactgcgcagtctccgcgatgccacgcagacggtcgatctcattttgcgaacattcaccgccaaacggcgcaatttctactaccagtccagcatctttaaagcttttctcgacagtggattgagcaaaacctaaaacaaatttgtcacccaccactaaccagcgttctgccagcggcttcaggtattcgcccagacgattaatcacatcagcgccctggatgtatttacccggtgattgaataatgcggtccataattgctcctttagagatgagtagtgccaaatgcggcattccagtcgtgttcgaacttctctatagctgactctaccgcaggggtgttgagcatttgttgcgctacatctaagggcagggtgatggattcacatcctgccagtaaacagtccagcgcctgacgcggcgttttaaagctggctgccagcaccatgctttctggcgcgtgcatttctaacagcgtttgcagctcctgaaccgtacgaatgccgtctccgccctgggcatctacgcggttaacatacggagcaacgtattttgcccctgccagtgcggctaataacccttgtgcggcgctatatacagcagtgccaagtgtagtaataccctcttttttcagtattttaattgctgccagaccttcggaagtcaccgggattttcaccacaatacccggaatagcgtcgcgcaggcgcttcgcttcttccaccatcccctgcgcgtcgcggctcatggtctgagcaaacagaatgccctcatcaccaatcgctttttgcagacgcggcagcacttcccatatggactccttgctggcagcgataatgctcgggttagttgtcaccccggcaatggggaatatgcgtgccagacgttcgacttctgcgacgttagcggtgtccagatacagttccatgatgtttccttttacagttccagttcatgttgcagcaggctggcgatagcgtcggcagaggcggcgttaaccagcgcgttacggaattcttcgtgcatgatgcggcgagcgaggcgcgagaaaatgcgcatatgctgatcgcccgcagcgtgtttgttcagggttaacataatgatgaattgcgcttcatcatcgccccagcgcaccggcgcttgcagacgcgccacgctgatggtggattgctcaatgtgttctgatttgctgtgtggaatggcaaaactaaagcccagaccggtagagaaaacggcctcgcgcgcccacaagtcggcttccagtttacgcggatagcggcagcggcccgccagcagcaggttatcggtcatgcctttgagcacttcttctttgctgcgccagtcgctttccagtgtgatgcactcggcggtgaccagcggtgcgtcttgttgggtcatgcggaattgcgccagcaggtgttctacttccagcgaagtacggcaggccattgcctggttgagcaacttgcggcactcacggctatcaagttgcgccatccgagctttcgccgccggaattgatggtgcgctcatgctgagttcatccagccctaagccgaccagcaacggcagcacggaacctttcgctcccagctcaccgcacagaccaatccatttgccctggcgatgcaccgcttgcacggcgtaatcgagcgcccgcaagaatgccggattcaggctgttgtagtgacgagtaaccttagcgttatcgcgatccaccgccagcagatactgcgtcaggtcattactaccaatactaaagaaatcaatctcttcgcagcattgatcgatgatgaacatcaccgacggcacttccagcatgatgccgagctggattttctcatcaaacggaatgtgttcgttacgtagttgctgtttggcttccgccagtttttctttcacccataagatctcttccattgaggagatcatcgggatcatgattttcaggctgccgtgagcggaggcgcggaggatcgaccgtagctgcgtggtaaacaacgacgcgtactcttcataaatacgcacggcgcgataaccgaggaacgggtttgcctctgcgggaatgttcagataatcaacgggtttgtcgccgccaatgtccatagtgcgcacaataatgctgcgtccgttggcggattccagcgcctgacaaaaaatgttgtacaactcgctttcgcccggtgcgctggtgcgatccatatagagcatttcagtgcggaacaaaccaacgccttccgcaccattgccgaatgcggcctgcgcttccacggagtgagcgatgttagcggcaatttcaatgcggataccgtcagcggtacgggcttgttgggtcagccagacacgctgttgctcacgcagggcgtcctgtacgcgggcttcttgctgataataacgagctacggcttcccctggctcaaccacaatcgccccggcgttgccgtcgatataaatcgtttgttgctgccacggagtaagggcatcaatatccacaccaaccagcgttggaatgttgaacgaacgggcaaggatcaccgtatgtgaggtggtgccgccgcttttgagcaacaatcctttgaggtgatttttatccagttcgaggaactggctgggggtcagttcatcagccatacaaatggcgggctgcgtcagtttgcccggtgccgggaagcgttgctcaccgtagatttgctggagtaactggaagcagacgtcgcgtacgtccagggcacgttcttgcaggtagctgctgctggaacgggaaaactcttcgcaaaagtgattcgcgctggcaacaattgcttcggcgcagcttaatccggcgctgacgcctgccagtaaatgttcgcgcagggaagtatcgccagccagggatcggtgagcttccagaatcgcgctggtagcaccgtcgctatccagcagacgaaactcaatgtttttcagtaccagcgtcaggccgttttccagtgcggattgctcggcgtcaacgcctttggctgcgggaagattacccagcgcattgagatctaaagaagagatcggcgtcagaatgccgcctgcactaccgctgcacacggtgcgggcgcggataatttgcggattcagattggtcagtgaaaccggcagtggttccagttcgtcagatttaacttccgccagcggcgcatcgcagtgggggaattcatcgcgcagccattggcttaaacgctggtgcgcttcctgttcgtcggccccggaaatcagtaactggcagttatcgcccgccagcgtatcggtgccaatcagcgcaagggcgcttttggcgttgcccttgcggtcagtgcgcaggttatgccactcaatttgtgatgaaaaagtattacacagcgtttcaacgtggcttgccggacgcgcatgtacgccgttaggtagctcacaaataaattccacaatcagggccattgcctctctcccggtacggttttctgtttacaggataagagcgcacggcaacggcctgccatgtgacaaatctgccaaaagctggacaaatgtaatgtaaccgtcaatttgcgacgcgtctcacaagacgctgttttgcggcatgcttccggtttatcgcaagttatgaggcggatcgcatttttgtactgatattacaaaagtccagtaaatggcctttttatccactgtttgctccgcctgcgattgcctattgtttcctccatcaaaaatatggacatgggctttcgcaagcccgggagcagcttatgaatgagttggtgcagatcctgaaaaatacccgtcagcatttaatgacgggcgtttcacacatgattcccttcgtggtatcgggcggtattttgctggcggtttccgtcatgttgtatggcaaaggcgcagtgccggatgccgtagccgatccaaatctgaaaaaactgtttgatatcggcgttgcgggcttgacgctgatggtgcctttcctcgcagcgtacatcggttattccattgcagagcgttctgcgctggctccgtgcgctatcggtgcctgggttggtaacagctttggtgcgggcttctttggtgcactgatcgccgggattatcggcggcatcgtggtgcattacctgaagaaaattccggtgcataaagttctgcgctcggtgatgcctatcttcattattcctatcgtcggcacactgattaccgcaggcatcatgatgtggggcttgggcgagcctgtaggggcgttgaccaacagcctgactcagtggcttcaggggatgcagcagggcagcattgttatgctggcggtgatcatgggtctgatgctggcgttcgatatgggcggtccggttaacaaagtggcctatgccttcatgctgatttgcgttgctcagggtgtttataccgtggtggccatcgctgccgtgggtatttgtatcccgccgctggggatggggctggcgacgctgattggtcgtaaaaatttctccgcagaagagcgcgaaaccggcaaagcggcactggtgatgggctgtgttggcgttactgaaggggcgattcctttcgccgctgccgatccgctgcgtgtcattccttccatcatggtcggttcagtttgtggtgcagtaactgcggcgctggtcggtgcgcagtgctatgcaggctggggtggtctgattgtgctgccggtggttgaaggcaagctgggttatatcgcagcagtggctgtcggagcagtggtgacggctgtttgtgtgaacgtgctgaaaagtctggcgcgtaaaaatgggtcttcgactgatgaaaaagaagacgacctggatttggattttgaaattaattaattgaggaacgagccatgacgaaaattattgcagtaaccgcatgtccttcaggtgttgcccatacctatatggcagcagaggcgctggaaagtgccgcgaaagcgaaaggctgggaagtgaaagtagaaacccaggggtcaattggtctggaaaatgaactgactgcggaagatgtggcgagcgctgatatggtgattctgaccaaagatatcggcatcaagtttgaagagcgttttgctggcaagaccatcgtgcgcgtcaacatcagcgatgcagtaaaacgtgctgacgccattatgagcaaaattgaagctcacctggcgcaaaccgcttaagttcttctcccgctcgcaagggcgggttcgctttcccacaggagttcctcatgacgaatcgtatctctcgcctcaaaactgcactgtttgccaatacccgtgaaatctcgctggagcgggcgctgctttataccgccagccatcggcaaaccgaaggcgaaccggtgatattgcgccgggcgaaagcaacagcgtatatccttgaacatgttgaaatttcgattcgtgatgaagaactgattgccggtaaccgcaccgtaaaaccgcgcgccgggattatgtcgccggaaatggacccttactggctgctgaaagagctggatcaattcccgacgcgtccgcaggaccgctttgctatcagcgaagaagataaacgtatctaccgtgaagagttgttcccgtactgggaaaaacgttcgatgaaagatttcatcaacgggcagatgacagatgaagtaaaagccgcgaccaacacgcagattttcagcatcaaccagacggataaaggccaggggcacattattattgattacccacgcctgttgaatcacgggctgggtgagctggtggcacagatgcagcaacattgtcagcaacagccggagaatcacttttatcaggccgcgttgttactgctggaagcctcgcagaaacacattttgcgttacgccgaactggcggaaacgatggcggcaaactgcacagatgcccagcgtcgcgaagagctgctgactattgcagagatctcccgccataacgcgcaacataagccgcagacgttctggcaggcgtgccagttattctggtacatgaacatcattctgcaatacgaatccaacgccagttcgctatcgttggggcgcttcgaccagtatatgttgccgttctatcagacatcattaacccagggcgaagatgcggcgttcctgaaagaactgctcgaatctttatgggtgaaatgcaacgacatcgtgctgttgcgctccaccagtagcgcgcgttatttcgccggtttcccgaccggctataccgcactgctcggcgggttaaccgagaacggacgtagcgcggtgaacgtgctttcgttcctttgccttgacgcctatcaaagcgtgcaattaccgcaaccgaacctcggcgtgcgcactaacgccttgatcgacacgccgttcctgatgaaaaccgccgaaaccattcgcttcggtaccggtattccgcaaatctttaacgatgaagtggtggtgccagcgttcctcaaccgtggcgtttcgctggaagatgcgcgcgactattccgtagtgggctgtgtggaattatctattcccggcagaacctacggcttgcatgacatcgcgatgtttaatctgctgaaagtgatggaaatctgcctgcatgaaaatgaaggcaatgctgcgctgacttatgaaggtttactggagcagatccgcgccaagatcagccactacatcaccctgatggttgagggcagcaatatttgtgatatcggccatcgcgactgggcacctgtaccgctgctctcatcgtttatcagcgattgtctggaaaaaggccgcgatattaccgatggcggcgcgcgttataacttctccggcgtacaggggatcggtatcgccaacctgagcgattctctccatgcgttgaaagggatggtttttgagcaacagcgtttaagttttgacgaattgctgtcggtattaaaagccaacttcgcaacgccagaaggcgaaaaagtccgcgctcgcttaattaaccgcttcgagaaatacggtaacgatatcgacgaggtggataacatcagcgccgaactgttgcgccactactgcaaagaagtggaaaaataccagaacccgcgcggcggctacttcacgccgggatcgtataccgtttctgctcacgtcccgttgggatcggtggttggcgcgacgccagacggtcgttttgccggagaacagctggcagacggcggcttgtcacccatgctgggccaggacgcacaagggccaacagcggtactgaagtcagtcagtaagctcgataacacgctgctgtctaacggtacgttgctgaacgtgaaattcactccggcgaccctggaaggtgaagcaggattacgcaaactggccgacttcttacgggcgtttacccagcttaagttacaacatattcagtttaacgtggtgaacgccgacacgttgcgggaagcgcaacagcgcccacaagattatgccgggctggtggtgcgcgttgccggatacagcgccttctttgtcgaactgtcgaaggagatccaggatgacatcatccgccggacagcgcatcagctgtaacgttgtggaaacgcgccgcgatgatgtggcgcgcattttcaacattcagcgttattcactgaatgacggcgagggcattcgtacggtggtcttttttaaaggctgtccgcatctttgcccgtggtgtgctaatccggagtcgatctccggcaaaatccagacggtacgcagagaggcgaaatgtctgcactgtgcgaaatgtttgcgtgatgcggatgaatgcccctccggggcgtttgaacggattggtcgcgatatcagccttgacgctctggaacgggaagtgatgaaagatgacattttctttcgcacgtccggcggcggcgtcacgctttctggcggcgaagtgttaatgcaggcggagtttgctacccgttttttacagcgactgcggctgtggggtgtgtcatgcgccattgaaactgccggagacgcaccagccagcaagctattaccgctggcgaaattgtgcgatgaagtgttgttcgatttaaaaattatggacgcgactcaggcgcgggatgtggtgaagatgaacctgccacgcgtgctggagaatctgcgtttgctggtgagtgagggcgtcaacgtgatcccgcgtttaccgctgatccctggtttcacgctcagccgggagaatatgcagcaggcgctggatgtactgatcccgctgaatatcaggcagatccatctgttaccgtttcatcagtacggcgaaccgaaataccgcctgctggggaaaacatggtcgatgaaagaggtgcctgcgccgtcgtcagctgatgtggcaacgatgcgcgaaatggcagaacgggccggacttcaggttaccgtgggaggttaaaatggcatacctggtggcagtaaccgcctgcgtaagcggcgtggcgcatacttatatggcggcggaacggctggaaaagttgtgcctgttagagaagtggggagtcagcattgaaactcagggcgcgctgggaacggagaatcgtttagcggatgaggatatccgccgggcggatgttgctctgttgattacggatatcgagcttgccggtgccgagcgatttgaacattgccgctatgtgcaatgcagcatctacgcattcctgcgtgagccgcagcgggtaatgagcgcggtgcgcaaagtgctttctgcgccgcagcaaacccatcttattctggagtagtcggtttttctgtcagttggctgtggtactgccggcgatattccgacggcgagcgttcggtgtttttacgaaacagacggcagaagtagttgctgtcgacaaagccgcaggcgtgcgccacttcttttaccttcaggtcatagcctttcaataacgtcttagcgtgctccagtcgcgtgtgattcaggtattcgttaaaaccaatggcccccgttttttgaaacaggtgcgagaggtaatttggcgaaatataaaacgcctgtgcaacagattcgcgggtaagcgcggaggcatagcgttcgtcgatataatcgcgaatagcttcaaatagtgcctggctgcgtgaggcggtctggatttggctgccaagcaaatcgcggcagtggctaagcaggctggcgacgataagccttgccgtttgctgctcctgcggctgcatttgcatttcattgagcgtttgtagcagaaaagaacctatgcgtgggccgcgtcgggcgacgtgttgcttcgccagattttgatattgtttgccatcccattgcacgacgctgaagccgagttgctgtttgccaaacagcacgctaaaggtagtagcgggggcttgccattgtggaaaattccagccaccagcaggaacgtacagcacatcgccgggaactaacgttgctccagcgccggtatcaacaaactcaccttccagcacaatttccagccgtggaaaatcgacctgatacgcaagatcgggcaccgggccgttactgctggcaaagtaaatctggcgcagggacagcgggccgttgatcaggcgggagagcagatagctgacgtcgtgatacatgttattcccttaggtatgtagacgggaaaacagtaactggcattattaaaaaaggccacctgaaaagtgtggcctgaggggagttcgatgtaaacattgcggcagttgtattgccggatgtggcgtaaacgccttatccagcctaccgccgcgatctgtaggccggataagacgcgtcaagcgtcgcatccggcaaatagcgcctggctgataattactgattacccacctgatcgccatagggcagtgtgtcgtaatcgatcagtgcgtttttcttatacgggttaccaatccagcgggtagtttctttgaactgcggattcaccactgaacgggttggatcgtaaccgtcgtaagataagcccgccaaatctgaccaggtgtggatcagttccgccaggctgtatttacgatcaacatcctgcgagaaatcacggggatgagtcgcttgccatttttctgacgtccacagcaggaacggaatggtgtacatatgacgcgtcgggttgtcctcattacgcccctgagttttgtgcggcggcgtgtcgtaaacctcttcaccgtggtcagagaaataaaccaggaaaccgttcgggtttgctgctttaaagtctttaatcaggctggcaaccacatgatcgttatacaggttagcgttgtcataatcgttatatgactccagctcttccgcgtttaatcccggcggaacatgatcggtattgccatcaaacttgccctgattttccgggtagcggtatttgtatttgatatgcgtacccagcagatgaacaatgatcagtttcttcggcgcagggtcattcagcacttcctggaacggcttcagcacgttggtgtcgtattcacgcgcactctgcgtacgttgctggttcatgtagtactgcttgtcggtctggcgcgaaaataccgtcagcatggtattgcgggcggtcatcgtctgctggttggtgatccagaaggttttataacccgcctgtttcatcatgttcatcagcgacggctgcgtcagatacagatccgggttcttttcattggcaaaggtcagcgcctgttgcaggatttcaatggtgtacggacgagacgtaactacgttattaaacacggtcagattcggatcggttttatgcagcgcatccagctccggcgtggtttcacgcggataaccgtacagactcatgcgtccgcgctgggtcgactcgccaatcaccagcactaaagtgcgcggttcgttacccgattcatctttgaaattagccagtggcggcaaggcattattttcattcagtaactttgttagcgagtttagttgctgacgatactgataatagccggtcaggaattgccacggtgcggcaggctccatacgcgaggccaggttatccaacgttttctcaaacggcttgtttttgataaacgtattcatggcgatcggatgcagaatcaagccataaagcagggcaaaagagacaacataacgccacggctttggaatatagaccgggcgcaggcgtgtccacagcagaactgccaccgccgtataggccagcgcgataagcacaattttcaggctgaaatactggcttaaatactcgctggcttcgttggtgttggtttcgaacatcacaaacagaacgctctgcgagaactcctgaccgtagatgacgtagtagcacagcgccgccagagaggccgcccatagcaccacgccgattactgcggcaataattttaatccgcttcggaaagaggaataccgggatcaaccacagcgaactgaataacagcgagtcgcgaatgccgttagtgccactataaccactgatgtaaataatggcctgtagcagagtagagaaaaaccaaaagtagagcagtgcccaacccagggctttccagctaaaaagaggtttagcctggacttctgtggaatgcatagtaagaacctgtcttgaaaaaatatcgccgaatgtaacgacaattccttaaggatatctgaaggtatattcagaatttgaataaaatgcagacagaaatatattgaaaacgagggtgttagaacagaagtatttcagaaaaccctcgcgcaaaagcacgagggtttgcagaagaggaagattagccggtattacgcatacctgccgcaatcccggcaatagtgaccattaacgcttgttcgacgcgaggatccggttcctggccttctttttctgcctggcgggagcggtgcagcaactcggcctgcaatacgttcagcgggtcggtgtaaatattccgtagctgaatagactctgcaatccacggcagatcggccatcagatgggaatcgttggcaatcgccagcaccactttgatgtcttcttcttgcaggttgcgtaactctttacctaacggccacagtgctttgtctaccaggcgttggtcatagtattccgccagccacaggtctgctttggcgaagaccatctccagcatgccgagacgcgtcgagaagaatggccaatcgcggcacatagcctccagctcgctctgtttgccgtcttcgaccactttttgcagcgccgtacctgcacccagccaggcggggagcatcagacggttttgcgtccaggcgaagatccacggaatggcgcgtagtgactcgacgccgccggttgggcgacgtttcgccggacgtgaacccaacggcagtttgcccagttcttgttccggcgtagcggagcggaagtaaggcacaaaatctttgttttcacgtacgtagccgcggtagacatcgcaggagatgactgacagttcatccataatgcgacgccagctctctttcggctccggcggtggcagcaggttggcttccagaatcgccccggtataaagcgacaggctgctgacggtgatttctggcagaccatatttaaagcggatcatctcgccctgttcggttacgcgcaggccgcctttcaggcttcctggcggttgtgacagcagcgccgcatgagcaggtgcgccgccgcgaccaatggaaccgccgcgaccgtggaacaacgtcagctcaatacccgctttttcgcaggttttgattaatgcatcctgtgcctgatattgcgcccaggaagctgccatcactcccgcatcttttgctgagtcggaatagccaatcatcaccatctgtttgccctgaatcaggccacgataccagtcaatattgagcagctgggtcatgacatcgttggcgttgttcagatcatcgagggtttcaaacagcggagcaaccggcatcgcaaacccgatacccgcttctttcagcagcaggtggacagccagtacgtcggacggcgttttcgccatcgagatcacgtaggcggcaatggagccttgcggtgcttcggcaatcacctggcaggtatcgagcacttcgcgcgtttcggcgcttggttgccagttgcgcggcagaagcggacgtttggagttcagttcgcggatcaggaacgcctgtttgtcggcctctgaccagctttcgtagtcgccgataccgaggtagcgggtcagctcgcccagcgcttcggtatgacgcgtgctctcctgacggatatcaatacggaccagcggtacgccgaaacatttcacgcggcgcagggtgtcgagcagatcgccgttggcgataatacccatgccacacgcctgaagtgactggtagcaagcgtagagcggttcccacagttcttcgttttgtgtcagcaggccttctggttttggcagttcttcgcctttcaggcgcgcttccagccatgcctgtgtcgccatcaggcgagaacgcaggtttttcatcagatagcgatacggttctgcggcaccttcttcgccaaccagcgccagcagttcaggggtcgcttcaaccatcgacagttcagaaaccagcacctgaatatctttcaggaacaaatcggtggctttccagcggctgagtagcaggacgtggcgggtgatatcggcagtgacgttcgggttgccgtcgcggtcgccgcccatccacgaagtaaaacggaccggaacaaattcgacgggcagtttgtagccgaggttctcttccagttgttcgttcagttcgcgcaggtaatttggtacgccttgccacaggctgttttccactacggcaaagccccatttggcttcatctaccgggcttggacgcagcttacggatttcatcggtatgccatgactgggcgatcaactggcgcaggcgacgcatcagctggttgtgttcgtagtcagcgatatctttgttatcgagctgttttaaacaggcgttcacttccaccattttgtggatcagtgtacgacgggtaatttcggttgggtgagccgtgaggaccagttccagcgacagcgattccactgcttttttgatggtgtcttcgctcagttccggctggtttttcagtttacgcagggtgcgggcgatcacttccgggttgctggcagcttcgcctttcggcgaaatgctgtggtattgctcggcggtgttggccaggttcaggaactgactaaacgcacgcgcaacgggcagcagctcgtcgttcgacaaattttgtaaggtggtgagcaactcctggcggttagcatcattgccagcgcgtgaagatttcgacaacttacggatagtttctacgcgttcaagaatgtgttctcccaacgcatccttgatggtttctcccagcactttgccgagcatactgacattactacgcaatgcggaatattgttcgttcatattaccccagacaccccatcttatcgtttgatagccctgtatccttcacgtcgcattggcgcgaatatgctcgggctttgcttttcgtcgtcttttataaagccacgtaaaagcggtgacgtcaaatgctgcgaaatcgcttcagcaaacgaataaatagcaggaatttacgtcattaaattcacgacgctttaaataagcgtaacttatggaaatgttaaaaaatcgccccaagtaacaccaaaggtgtaggtcggataagatgcgcaagtatcgcatccgacattattgcggcactggagtttggcaacagtgccggatgcggcgcgagcgccttatccggcctacagttgggcatcgtttgagtcactgtcggtcggataagatgcgcaagtatcgcatccgacattattgcggcactggagtttggcaacagtgccggatgcggcgcgagcgccttatccggcctacggttgggcatcgtttgagtcactgtaggtcggataagatgcgcaagcatcgcatccgacattattgcggcactggagtttggcaacagcgccggatgcggcgcgagcgccttatccggcctacgttttaatgccagcaaaaatggtgaattacctgggttatcagttcgcgggtgggcttgataaaccgtgtttccagatattcatcaggttgatgagcctgattaattgagccaggccccaacaccagcgtcgggcataacgtttgaataaacggcgcttcggtacagtagttcaccacttcggtttttgctccgagcaatttctcaaccacttcaaccagttgatgattcggtgggcattcatagccagggatcggcggatgcagctcgtcgaccgtcagacgacccggccagcgttcgctcaccggagccaatgcatcgttgagcaaaccattaagttcattgagtgtcatgccaggcagcggacgaatatccatatgcaactcacagcaagcgcaaatacggttagaagcgtcgccaccgtgaatatgcccgaggttgagcgtagggtatggcacggtaaacgcttcgtagtgataacgttctttcaggttatcgcgcaattgcaaaatatgcccgatggcgtcgtgcattagttcgatagcgttaactccgcgtgctggatcgctggagtgccccgactggccctgaatacggatggcgttagagatatgacctttatgtgcgcgtaccggttgtagtgacgtcggttcgccaatgatggcgcaatccgggcgcagggcggtagtttcggcaaaataacgcgctccggccatactggtttcttcatcagcagtcgccagaatgtagagcggttttttcagtttcgtgacgtcgacatcgcgtagcgcatcaaggataaacgcaaaaaagcctttcatgtcggcggtgcctaagccgtaaagcttgccgtcatgctccgtcagtgtaaacggatcgcgcgtccagcgaccgtcatcaaatggcaccgtatcggtatgccccgccagcaacaagccgccagccccctgtccgatacttgccagcatattgaatttgttgcgagttcctggaacaggctgcacttccacattgaagcccaaatctttaaaccagtccgccagcagagtgattaaatctgcattgctttgatcgagtgcctcttccgtggcgcttattgaaggtgtggcaatcagagcgcggtaaatctcgataaatggcggtaatttgtttttcattgttgacacacctctggtcatgatagtatcaatattcatgcagtatttatgaataaaaatacactaacgttgagcgtaataaaacccaccagccgtaaggtgaatgttttacgtttaacctggcaaccagacataagaaggtgaatagccccgatgttgaatacgctgattgtgggtgccagcggctacgctggcgcagagctagtgacctatgtaaatcgccatccgcatatgaacataaccgctttgactgtttcagcgcaaagcaatgatgcgggaaagttaatctccgatttgcatccgcagctaaaaggcatcgttgatctgccgttgcagccgatgtcggatatcagcgagtttagcccaggggtggacgtagtgtttctcgccaccgcccatgaagttagccacgatttagcgccgcagtttcttgaagcgggctgcgtggtgttcgacctttccggcgcgtttcgtgttaacgacgccaccttctatgaaaaatattacggctttacccatcaatacccggaactgttggaacaggcagcctacggtctggcggagtggtgcggtaataaattaaaagaagcgaatttgattgcggtgccgggctgttatccgacggcggcacagctggcgctgaaaccgttgattgatgccgatcttcttgacctcaatcagtggccggtgatcaacgccaccagcggcgtgagcggtgcagggcgtaaagcggccatttcaaacagcttttgtgaagttagcctgcaaccgtatggcgtctttactcatcgccatcaaccagagatcgccacacacctcggtgctgacgttatcttcaccccacatctgggcaatttcccgcgcggcattctcgaaaccattacctgccgcctgaaatcgggtgtgacccaggcgcaagtcgcgcaagtgttacagcaggcgtatgcccataaaccgctggtgcggctgtatgacaaaggcgttccggcgctgaaaaatgtcgttgggctgccattttgcgatatcgggtttgccgttcagggcgagcatctgattattgtggcgaccgaagacaacttactgaaaggcgcggcggcacaagcggtacagtgcgccaatattcgtttcggctatgcggaaacgcagtctcttatttaagggtgcaatgatgaatccattaattatcaaactgggcggcgtactgctggatagtgaagaggcgctggaacgtctgtttagcgcactggtgaattatcgtgagtcacatcagcgtccgctggtgattgtgcacggcggcggttgcgtggtggatgagctgatgaaagggctgaatctgccggtgaaaaagaaaaacggcctgcgggtgacgcctgctgatcagatagacattatcaccggagcactggcgggaacggcaaataaaaccctgttggcatgggcgaagaaacatcagattgcggccgtaggtttgtttctcggtgacggcgacagcgtcaaagtgacccagcttgatgaagagttaggtcatgttggactggcgcagccaggttcgcctaagcttatcaactccttgctggagaacggttatctgccggtggtcagctccattggcgtaacagacgaagggcaactgatgaacgtcaatgccgaccaggcggcaacggcgctggcggcaacgctgggcgcggatctgattttgctctccgacgtcagcggcattctcgacggcaaagggcaacgcattgccgaaatgaccgccgcgaaagcagaacaactgattgagcagggcattattactgacggcatgatagtgaaagtgaacgcggcgctggatgcggcccgcacgctgggccgtccggtagatatcgcctcctggcgtcatgcggagcagcttccggcactgtttaacggtatgccgatgggtacgcggattttagcttaagttttgttggccggaggcgcagctttccggcattgaatttcaaaataaggaaacagagttatggcactttggggcgggcgttttacccaggcagcagatcaacggttcaaacaattcaacgactcactgcgctttgattaccgtctggcggagcaggatattgttggctctgtggcctggtccaaagccctggtcacggtaggcgtgttaaccgcagaagagcaggcgcaactggaagaggcgctgaacgtgttgctggaagatgttcgcgccaggccacaacaaatccttgaaagcgacgccgaagatatccatagctgggtggaaggcaaactgatcgacaaagtgggccagttaggcaaaaagctgcataccgggcgtagccgtaatgatcaggtagcgactgacctgaaactgtggtgcaaagataccgttagcgagttactgacggctaaccggcagctgcaatcggcgctggtggaaaccgcacaaaacaatcaggacgcggtaatgccaggttacactcacctgcaacgcgcccagccggtgacgttcgcgcactggtgcctggcctatgttgagatgctggcgcgtgatgaaagccgtttgcaggatgcgcttaagcgtctggatgtcagcccgctaggctgtggcgcgctggcgggaacggcctatgaaatcgaccgtgaacagttagcaggctggctgggctttgcttcggcgacccgtaacagtctcgacagcgtttctgaccgtgaccatgtgttggaactgctttctgctgccgctatcggcatggtgcatctgtcgcgttttgctgaagatctgattttctttaacaccggcgaagcggggtttgtggagctttctgaccgcgtgacttccggttcatcattaatgccgcagaagaaaaacccggatgcgctggagctgattcgcggtaaatgcggccgggtgcagggggcgttaaccggcatgatgatgacgctgaaaggtttgccgctggcttacaacaaagatatgcaggaagacaaagaaggtctgttcgacgcgctcgatacctggctggactgcctgcatatggcggcgctggtgctggacggcattcaggtgaaacgtccacgttgccaggaagcggctcagcagggttacgccaacgccaccgaactggcggattatctggtggcgaaaggcgtaccgttccgcgaggcgcaccatattgttggtgaagcggtggtggaagccattcgtcagggcaaaccgctggaagatctgccgctcagtgagttgcagaaattcagtcaggtgattgacgaagatgtctatccgattctgtcgctgcaatcgtgcctcgacaagcgtgcggcaaaaggcggcgtctcaccgcagcaggtggcgcaggcgattgcttttgcgcaggctcggttagggtaagaacatttatatgtataaatttgagcctggcttatcgccgggcttttttatggcaaaaaaaagcggatcctggagatccgcaaaagttcacgttggctttagttattcgagttgagaaactctcgaaacgggcagtgacttcaagggttaaaagaggtgccgctccgtttctgtgagcaattatcagtcagaatgcttgatagggataatcgttcattgctattctacctatcgccatgaactatcgtggcgatggaggatggataatgaatattcgtgatcttgagtacctggtggcattggctgaacaccgccattttcggcgtgcggcagattcctgccacgttagccagccgacgcttagcgggcaaattcgtaagctggaagatgagctgggcgtgatgttgctggagcggaccagccgtaaagtgttgttcacccaggcgggaatgctgctggtggatcaggcgcgtaccgtgctgcgtgaggtgaaagtccttaaagagatggcaagccagcagggcgagacgatgtccggaccgctgcacattggtttgattcccacagttggaccgtacctgctaccgcatattatccctatgctgcaccagacctttccaaagctggaaatgtatctgcatgaagcacagacccaccagttactggcgcaactggacagcggcaaactcgattgcgtgatcctcgcgctggtgaaagagagcgaagcattcattgaagtgccgttgtttgatgagccaatgttgctggctatctatgaagatcacccgtgggcgaaccgcgaatgcgtaccgatggccgatctggcaggggaaaaactgctgatgctggaagatggtcactgtttgcgcgatcaggcaatgggtttctgttttgaagccggggcggatgaagatacacacttccgcgcgaccagcctggaaactctgcgcaacatggtggcggcaggtagcgggatcactttactgccagcgctggctgtgccgccggagcgcaaacgcgatggggttgtttatctgccgtgcattaagccggaaccacgccgcactattggcctggtttatcgtcctggctcaccgctgcgcagccgctatgagcagctggcagaggccatccgcgcaagaatggatggccatttcgataaagttttaaaacaggcggtttaaaccgtttaacgcagctacccgataggcttccgccatcgtcgggtagttaaaggtggtgttgacgaagtactcaatagtgttgccgccacctttctgttccataatcgcctgaccgatatgaataatttcggcagcgcgctcgccaaagcagtgaatacccagaatctcttttgtttcccgatggaacaaaattttcagcgtgcccacgttcatgccgacgatttgtgcgcgtgccagatgtttaaactgggcgcggcccacttcatatggcactttcattgcggtcagctgctgttcggttttgcccacagagctgatttccgggatggtgtaaataccggtagggatatcttcaatcagatgtgcggtggcttcgccttttaccagcgcctgcgcggcaatgcgcccctggtcataggccgccgacgccaggctcggataaccaatcacgtcgcccaccgcgtaaacgtgtggctgtgcggtctgatacatgctgttgaccttcagctgtccgcggctgtcagtttctagcccaatgttctgtaacgccagcgaatcggtattaccggtgcgaccgttggcatagagcaggcagtcagctttcagttttttacccgacttcagatgcatgatcacaccatcgtcacagccttcgatcttctcgtactcttcgttgtgacgaatcactacgccactgttccagaagtgataggagagagaatctgacatctcttgatcgagaaatgccagcaggcgatcgcgggtgttgatcagatccacttttacatccataccgcggaagatcgacgcatattcacagccgatcactccagcaccatagataagtacatggcgcggttcgtggtgcatgctgagaattgagtcgctgtcgtaaatgcgtggatgggtgaaatcaacatctgttggatgatatggacgagagccgcaggcaataacaaatttttcagcggttagtgtttcaacgctgccgtccgggcaatccagcgccaacgtatgctcgtcaacaaagcgagcgtttccctgcaatatttcacagtgattacgttcgtaaaatccctgacgcatgcgcgtttgttgattaatcacgttatcggcatggttaaggatatcggcaaaagaagagcggagcagtcgggaatggtcgctgtaaagtgggttttgattgaattctataatgcggctgacggcgtgacggagagctttcgacgggatggtgccccagtgggtgcaaccgccgccaacattttgataacgctcgataactgcgacgcgcgcaccttgcttaaccaggcccattgcagcgccttcgccgccggggccggaacctattactatggcatcgtaatcgtaggaatgtggcatggtagggcttacctgttcttatacataaaagcaacagaatggtaacattttatcgcgggtaagccaattgatccccgtcatttatctggctatatcctgagcggcctttgctttgtctgtttcttacttttgccctgacgttttattggatttttatcgacgatactctccgtttaagcggcaggtttccgctgtacgtaaaagaaccggccaaagaattgcagtaaatatgttttattgcgttaccgttcattcacaatactggagcaatccagtatgttcattctctggtatagtgccagcagtacttttggcaaggattcagacatcgtgatgggcgtaagagcgcaacaaaaagaaaaaacccgccgttcgctggtggaagccgcatttagccaattaagtgctgaacgcagcttcgccagcctgagtttgcgtgaagtggcgcgtgaagcgggcattgctcccacctctttttatcggcatttccgcgacgtagacgaactgggtctgaccatggttgatgagagcggtttaatgctacgccaactcatgcgccaggcgcgtcagcgtatcgccaaaggcgggagtgtgatccgcacctcggtctccacatttatggagttcatcggtaataatcctaacgccttccggttattattgcgggaacgctccggcacctccgctgcgtttcgtgccgccgttgcgcgtgaaattcagcacttcattgcggaacttgcggactatctggaactcgaaaaccatatgccgcgtgcgtttactgaagcgcaagccgaagcaatggtgacaattgtcttcagtgcgggtgccgaggcgttggacgtcggcgtcgaacaacgtcggcaattagaagagcgactggtactgcaactgcgaatgatttcgaaaggggcttattactggtatcgccgtgaacaagagaaaaccgcaattattccgggaaatgtgaaggacgagtaatgaaacaagcaaatcaagatagaggtacgctgctgctggcgttagttgctggcttatcgattaatggtactttcgcagcgctgtttagctccattgtgccattttctgtattcccgattatttccctggtgctgacggtttactgcctgcatcaacgttatcttaatcgcactatgccggtaggcttgccgggtctggcagctgcctgttttattctcggcgtactgctgtacagcacggtagttcgtgcggaatatccggatatcggctctaacttcttcccggcagtactctccgtcattatggtgttctggattggcgcgaagatgcgtaaccgtaagcaggaagttgctgagtaatcggtattatgccggatgctggcgcatccggcatgggttttacttcgcggtcagtaatacgccgcactccatatggtgcgtgtaggggaactgatcaaacagagccagacgttcgaccttgtgcgtctggcttaatgtttccagattcttgcataacgtttccgggttacaggagatgtacaaaatacgcggatacgcctgcaccattttctcggtttcactgtccagaccgctgcgcggagggtcgacaaaaatggtttcgcactgataactctttaagtcgatcccttgcaggcggttaaactcgcgcacaccattcatcgcctgagtaaattcttctgccgccatacgaataatttgtacgttatcaatatggttagctgcgatgttgtattgcgcagcagcaaccgacggcttagcgatttcggtggctaatacccgatcaaaattacgcgccagcgctaatgaaaagttaccgttgccgcagtacagctccagtaaatcgccttttgagcctttggttacgtccagcgcccattccagcatctgaatattcatcgccgcgttcggctgggtaaagctgttttctacctgacggtagatcatctctttccctgcgaccggcagacgttcatcgatgtaatcctgatccagctcgattttggttttcgttgcccgaccaatcagatgcacattcagattctgcgcgcgcagtgcatcgcgcagggcctccgcttcctgacgccactcatcatccagcttcttatggtatagcagggaaaccaccgcctgattactcagtgtagtgaggtaatcaatctggaacaacttgtggcgcagaacgggattattacgcacacccgcaatcatcgccgtcatcaactggttgataagttcactggcggcggggaagctatccacgcggatgcggcttttggtttgttgatcgaaaatgatgtgatacaggtcatcgccatcgtgccagatgcggaactccgcgcgcatccggtaatgactgaccggcgagcgaaacacttccggaaccaggtcagaaaacggtgccatcatactttgcaaacgtaccactttttcggctaactgcgcttcatactgttctgttggaaggtgttcgggggtcatgatgtatcctgaaaaattaaagtacgcggcgattgtagggattgctcatcagatgtccagatcttgatgaattcctatttgtgagctacgtctggacagtaacttgttacaacctgtagcatccacttgccggtcctgtgagttaatagggaatccagtgcgaatctggagctgacgcgcagcggtaaggaaaggtgcgatgattgcgttatgcggacactgccattcggtgggaagtcatcatctcttagtatcttagatacccctccaagcccgaagacctgccggccaacgtcgcatctggttctcatcatcgcgtaatattgatgaaacctgcggcatccttcttctattgtggatgctttacaatgattaaaaaagcttcgctgctgacggcgtgttccgtcacggcattttccgcttgggcacaggataccagcccggatactctcgtcgttactgctaaccgttttgaacagccgcgcagcactgtgcttgcaccaaccaccgttgtgacccgtcaggatatcgaccgctggcagtcgacctcggtcaatgatgtgctgcgccgtcttccgggcgtcgatatcacccaaaacggcggttcaggtcagctctcatctatttttattcgcggtacaaatgccagtcatgtgttggtgttaattgatggcgtacgcctgaatctggcgggggtgagtggttctgccgaccttagccagttccctattgcgcttgtccagcgtgttgaatatatccgtgggccgcgctccgctgtttatggttccgatgcaataggcggggtggtgaatatcatcacgacgcgcgatgaacccggaacggaaatttcagcagggtggggaagcaatagttatcagaactatgatgtctctacgcagcaacaactgggggataagacacgggtaacgctgttgggcgattatgcccatactcatggttatgatgttgttgcctatggtaataccggaacgcaagcgcagacagataacgatggttttttaagtaaaacgctttatggcgcgctggagcataactttactgatgcctggagcggctttgtgcgcggctatggctatgataaccgtaccaattatgacgcgtattattctcccggttcaccgttgctcgatacccgtaaactctatagccaaagttgggacgccgggctgcgctataacggcgaactgattaaatcacaactcattaccagctatagccatagcaaagattacaactacgatccccattatggtcgttatgattcgtcggcgacgctcgatgagatgaagcaatacaccgtccagtgggcaaacaatgtcatcgttggtcacggtagtattggtgcgggtgtcgactggcagaaacagactacgacgccgggtacaggttatgttgaggatggatatgatcaacgtaataccggcatctatctgaccgggctgcaacaagtcggcgattttacctttgaaggcgcagcacgcagtgacgataactcacagtttggtcgtcatggaacctggcaaaccagcgccggttgggaattcatcgaaggttatcgcttcattgcttcctacgggacatcttataaggcaccaaatctggggcaactgtatggcttctacggaaatccgaatctggacccggagaaaagcaaacagtgggaaggcgcgtttgaaggcttaaccgctggggtgaactggcgtatttccggatatcgtaacgatgtcagtgacttgatcgattatgatgatcacaccctgaaatattacaacgaagggaaagcgcggattaagggcgtcgaggcgaccgccaattttgataccggaccactgacgcatactgtgagttatgattatgtcgatgcgcgcaatgcgattaccgacacgccgttgttacgccgtgctaaacagcaggtgaaataccagctcgactggcagttgtatgacttcgactggggtattacttatcagtatttaggcactcgctatgataaggattactcatcttatccttatcaaaccgttaaaatgggcggtgtgagcttgtgggatcttgcggttgcgtatccggtcacctctcacctgacagttcgtggtaaaatagccaacctgttcgacaaagattatgagacagtctatggctaccaaactgcaggacgggaatacaccttgtctggcagctacaccttctgaaccacgtcccaccgtgctggtgtttgactccggcgtcggtgggttgtcggtctatgacgagatccggcatctcttaccggatctccattacatttatgctttcgataacgtcgctttcccgtatggcgaaaaaagcgaagcgtttattgttgagcgagtggtggcaattgtcaccgcggtgcaagaacgttatccccttgcgctggctgtggtcgcttgcaacactgccagtaccgtttcacttcctgcattacgcgaaaagttcgacttcccggttgttggtgtcgtgccggcgattaaacctgctgcacgtctgacggcaaatggcattgtcggattactggcaacccgcggaacagttaaacgttcttatactcatgagctgatcgcgcgtttcgctaatgaatgccagatagaaatgctgggctcggcagagatggttgagttggctgaagcgaagctacatggcgaagatgtttctctggatgcactaaaacgtatcctacgcccgtggttaagaatgaaagagccgccagataccgttgtattgggttgcacccatttccctctactacaagaagaactgttacaagtgctgccagagggaacccggctggtggattctggcgcagcgattgctcgccgaacggcctggttgttagaacatgaagccccggatgcaaaatctgccgatgcgaatattgccttttgtatggcaatgacgccaggagctgaacaattattgcccgttttacagcgttacggcttcgaaacgctcgaaaaactggcagttttaggctgatttggttgaatgttgcgcggtcagaaaattattttaaatttcctcttgtcaggccggaataactccctataatgcgccaccactgacacggaacaacggcaaacacgccgccgggtcagcggggttctcctgagaactccggcagagaaagcaaaaataaatgcttgactctgtagcgggaaggcgtattatgcacaccccgcgccgctgagaaaaagcgaagcggcactgctctttaacaatttatcagacaatctgtgtgggcactcgaagatacggattcttaacgtcgcaagacgaaaaatgaataccaagtctcaagagtgaacacgtaattcattacgaagtttaattctttgagcgtcaaacttttaaattgaagagtttgatcatggctcagattgaacgctggcggcaggcctaacacatgcaagtcgaacggtaacaggaagaagcttgcttctttgctgacgagtggcggacgggtgagtaatgtctgggaaactgcctgatggagggggataactactggaaacggtagctaataccgcataacgtcgcaagaccaaagagggggaccttcgggcctcttgccatcggatgtgcccagatgggattagctagtaggtggggtaacggctcacctaggcgacgatccctagctggtctgagaggatgaccagccacactggaactgagacacggtccagactcctacgggaggcagcagtggggaatattgcacaatgggcgcaagcctgatgcagccatgccgcgtgtatgaagaaggccttcgggttgtaaagtactttcagcggggaggaagggagtaaagttaatacctttgctcattgacgttacccgcagaagaagcaccggctaactccgtgccagcagccgcggtaatacggagggtgcaagcgttaatcggaattactgggcgtaaagcgcacgcaggcggtttgttaagtcagatgtgaaatccccgggctcaacctgggaactgcatctgatactggcaagcttgagtctcgtagaggggggtagaattccaggtgtagcggtgaaatgcgtagagatctggaggaataccggtggcgaaggcggccccctggacgaagactgacgctcaggtgcgaaagcgtggggagcaaacaggattagataccctggtagtccacgccgtaaacgatgtcgacttggaggttgtgcccttgaggcgtggcttccggagctaacgcgttaagtcgaccgcctggggagtacggccgcaaggttaaaactcaaatgaattgacgggggcccgcacaagcggtggagcatgtggtttaattcgatgcaacgcgaagaaccttacctggtcttgacatccacggaagttttcagagatgagaatgtgccttcgggaaccgtgagacaggtgctgcatggctgtcgtcagctcgtgttgtgaaatgttgggttaagtcccgcaacgagcgcaacccttatcctttgttgccagcggtccggccgggaactcaaaggagactgccagtgataaactggaggaaggtggggatgacgtcaagtcatcatggcccttacgaccagggctacacacgtgctacaatggcgcatacaaagagaagcgacctcgcgagagcaagcggacctcataaagtgcgtcgtagtccggattggagtctgcaactcgactccatgaagtcggaatcgctagtaatcgtggatcagaatgccacggtgaatacgttcccgggccttgtacacaccgcccgtcacaccatgggagtgggttgcaaaagaagtaggtagcttaaccttcgggagggcgcttaccactttgtgattcatgactggggtgaagtcgtaacaaggtaaccgtaggggaacctgcggttggatcacctccttaccttaaagaagcgtactttgtagtgctcacacagattgtctgatagaaagtgaaaagcaaggcgtttacgcgttgggagtgaggctgaagagaataaggccgttcgctttctattaatgaaagctcaccctacacgaaaatatcacgcaacgcgtgataagcaattttcgtgtccccttcgtctagaggcccaggacaccgccctttcacggcggtaacaggggttcgaatcccctaggggacgccacttgctggtttgtgagtgaaagtcgccgaccttaatatctcaaaactcatcttcgggtgatgtttgagatatttgctctttaaaaatctggatcaagctgaaaattgaaacactgaacaacgagagttgttcgtgagtctctcaaattttcgcaacacgatgatgaatcgaaagaaacatcttcgggttgtgaggttaagcgactaagcgtacacggtggatgccctggcagtcagaggcgatgaaggacgtgctaatctgcgataagcgtcggtaaggtgatatgaaccgttataaccggcgatttccgaatggggaaacccagtgtgtttcgacacactatcattaactgaatccataggttaatgaggcgaaccgggggaactgaaacatctaagtaccccgaggaaaagaaatcaaccgagattcccccagtagcggcgagcgaacggggagcagcccagagcctgaatcagtgtgtgtgttagtggaagcgtctggaaaggcgcgcgatacagggtgacagccccgtacacaaaaatgcacatgctgtgagctcgatgagtagggcgggacacgtggtatcctgtctgaatatggggggaccatcctccaaggctaaatactcctgactgaccgatagtgaaccagtaccgtgagggaaaggcgaaaagaaccccggcgaggggagtgaaaaagaacctgaaaccgtgtacgtacaagcagtgggagcacgcttaggcgtgtgactgcgtaccttttgtataatgggtcagcgacttatattctgtagcaaggttaaccgaataggggagccgaagggaaaccgagtcttaactgggcgttaagttgcagggtatagacccgaaacccggtgatctagccatgggcaggttgaaggttgggtaacactaactggaggaccgaaccgactaatgttgaaaaattagcggatgacttgtggctgggggtgaaaggccaatcaaaccgggagatagctggttctccccgaaagctatttaggtagcgcctcgtgaattcatctccgggggtagagcactgtttcggcaagggggtcatcccgacttaccaacccgatgcaaactgcgaataccggagaatgttatcacgggagacacacggcgggtgctaacgtccgtcgtgaagagggaaacaacccagaccgccagctaaggtcccaaagtcatggttaagtgggaaacgatgtgggaaggcccagacagccaggatgttggcttagaagcagccatcatttaaagaaagcgtaatagctcactggtcgagtcggcctgcgcggaagatgtaacggggctaaaccatgcaccgaagctgcggcagcgacgcttatgcgttgttgggtaggggagcgttctgtaagcctgcgaaggtgtgctgtgaggcatgctggaggtatcagaagtgcgaatgctgacataagtaacgataaagcgggtgaaaagcccgctcgccggaagaccaagggttcctgtccaacgttaatcggggcagggtgagtcgacccctaaggcgaggccgaaaggcgtagtcgatgggaaacaggttaatattcctgtacttggtgttactgcgaaggggggacggagaaggctatgttggccgggcgacggttgtcccggtttaagcgtgtaggctggttttccaggcaaatccggaaaatcaaggctgaggcgtgatgacgaggcactacggtgctgaagcaacaaatgccctgcttccaggaaaagcctctaagcatcaggtaacatcaaatcgtaccccaaaccgacacaggtggtcaggtagagaataccaaggcgcttgagagaactcgggtgaaggaactaggcaaaatggtgccgtaacttcgggagaaggcacgctgatatgtaggtgaggtccctcgcggatggagctgaaatcagtcgaagataccagctggctgcaactgtttattaaaaacacagcactgtgcaaacacgaaagtggacgtatacggtgtgacgcctgcccggtgccggaaggttaattgatggggttagcgcaagcgaagctcttgatcgaagccccggtaaacggcggccgtaactataacggtcctaaggtagcgaaattccttgtcgggtaagttccgacctgcacgaatggcgtaatgatggccaggctgtctccacccgagactcagtgaaattgaactcgctgtgaagatgcagtgtacccgcggcaagacggaaagaccccgtgaacctttactatagcttgacactgaacattgagccttgatgtgtaggataggtgggaggctttgaagtgtggacgccagtctgcatggagccgaccttgaaataccaccctttaatgtttgatgttctaacgttgacccgtaatccgggttgcggacagtgtctggtgggtagtttgactggggcggtctcctcctaaagagtaacggaggagcacgaaggttggctaatcctggtcggacatcaggaggttagtgcaatggcataagccagcttgactgcgagcgtgacggcgcgagcaggtgcgaaagcaggtcatagtgatccggtggttctgaatggaagggccatcgctcaacggataaaaggtactccggggataacaggctgataccgcccaagagttcatatcgacggcggtgtttggcacctcgatgtcggctcatcacatcctggggctgaagtaggtcccaagggtatggctgttcgccatttaaagtggtacgcgagctgggtttagaacgtcgtgagacagttcggtccctatctgccgtgggcgctggagaactgaggggggctgctcctagtacgagaggaccggagtggacgcatcactggtgttcgggttgtcatgccaatggcactgcccggtagctaaatgcggaagagataagtgctgaaagcatctaagcacgaaacttgccccgagatgagttctccctgaccctttaagggtcctgaaggaacgttgaagacgacgacgttgataggccgggtgtgtaagcgcagcgatgcgttgagctaaccggtactaatgaaccgtgaggcttaaccttacaacgccgaagctgttttggcggatgagagaagattttcagcctgatacagattaaatcagaacgcagaagcggtctgataaaacagaatttgcctggcggcagtagcgcggtggtcccacctgaccccatgccgaactcagaagtgaaacgccgtagcgccgatggtagtgtggggtctccccatgcgagagtagggaactgccaggcatcaaataaaacgaaaggctcagtcgaaagactgggcctttcgttttatctgttgtttgtcggtgaacgctctcctgagtaggacaaatccgccgggagcggatttgaacgttgcgaagcaacggcccggagggtggcgggcaggacgcccgccataaactgccaggcatcaaattaagcagaaggccatcctgacggatggcctttttgcgtttctacaaactcttcctgtcgtcatatctacaagccatccccccacagatacggtaaactagcctcgtttttgcatcaggaaagcagctatgaaccactccttaaaaccctggaacacatttggcattgatcataatgctcagcacattgtatgtgccgaagacgaacaacaattactcaatgcctggcagtatgcaaccgcagaaggacaacccgttcttattctgggtgaaggaagtaatgtactttttctggaggactatcgcggcacggtgatcatcaaccggatcaaaggtatcgaaattcatgatgaacctgatgcgtggtatttacatgtaggagccggagaaaactggcatcgtctggtaaaatacactttgcaggaaggtatgcctggtctggaaaatctggcattaattcctggttgtgtcggctcatcacctatccagaatattggtgcttatggcgtagaattacagcgagtttgcgcttatgttgattctgttgaactggcgacaggcaagcaagtgcgcttaactgccaaagagtgccgttttggctatcgcgacagtatttttaaacatgaataccaggaccgcttcgctattgtagccgtaggtctgcgtctgccaaaagagtggcaacctgtactaacgtatggtgacttaactcgtctggatcctacaacagtaacgccacagcaagtatttaatgcggtgtgtcatatgcgcaccaccaaactccctgatccaaaagtgaatggcaatgccggtagtttcttcaaaaaccctgttgtatctgccgaaacggctaaagcattactgtcacaatttccaacagcaccaaattacccccaggcggatggttcagtaaaactggcagcaggttggcttatcgatcagtgccagctaaaagggatgcaaataggtggggctgcggtgcaccgtcaacaggcgttagttctcattaatgaagacaatgcaaaaagcgaagatgttgtacagctggcgcatcatgtaagacagaaagttggtgaaaaatttaatgtctggcttgagcctgaagtccgctttattggtgcatcaggtgaagtgagcgcagtggagacaatttcatgaaggataacaccgtgccactgaaattgattgccctgttagcgaacggtgaatttcactctggcgagcagttgggtgaaacgctgggaatgagccgggcggctattaataaacacattcagacactgcgtgactggggcgttgatgtctttaccgttccgggtaaaggatacagcctgcctgagcctatccagttacttaatgctaaacagatattgggtcagctggatggcggtagtgtagccgtgctgccagtgattgactccacgaatcagtaccttcttgatcgtatcggagagcttaaatcgggcgatgcttgcattgcagaataccagcaggctggccgtggtcgccggggtcggaaatggttttcgccttttggcgcaaacttatatttgtcgatgttctggcgtctggaacaaggcccggcggcggcgattggtttaagtctggttatcggtatcgtgatggcggaagtattacgcaagctgggtgcagataaagttcgtgttaaatggcctaatgacctctatctgcaggatcgcaagctggcaggcattctggtggagctgactggcaaaactggcgatgcggcgcaaatagtcattggagccgggatcaacatggcaatgcgccgtgttgaagagagtgtcgttaatcaggggtggatcacgctgcaggaagcggggatcaatctcgatcgtaatacgttggcggccatgctaatacgtgaattacgtgctgcgttggaactcttcgaacaagaaggattggcaccttatctgtcgcgctgggaaaagctggataattttattaatcgcccagtgaaacttatcattggtgataaagaaatatttggcatttcacgcggaatagacaaacagggggctttattacttgagcaggatggaataataaaaccctggatgggcggtgaaatatccctgcgtagtgcagaaaaataagaaaggggagtattcgctcccctgcaaattatttgcgtagtctgacctcttctaccgcatgattagcacttttcgtcaggattaaactggcgcgctcacgagtaggtagaatattttgctttaagttcagccagttgatctctttccacaatgtcatggcagtcttaatcgcttcttctttagttaatttcgcgtagttatgaaaataggaatccgggtcggtaaaagccccttcgcggaatttcagaaaacggttgatataccatgtctgaagtaagtcttccggtgcatcaacatatatcgaaaaatcgacaaaatcagaaacaaatacatgatgtggatcgtgtggataatccatcccgctctgtaagacatttaacccttcaagaattaaaatatcaggctgaacaaccgttttatctccatccgggatcacatcataaataagatgtgagtaaacaggtgctgtaacgtttggcacgccggatttgagatcggaaacaaacttcaccaggcgatgcatatcatacgattccgggaagcctttcttcttcatcagaccacgttctttcagaacctgattagggtgaaggaagccatctgtagtgatcagttcaacacgacgatgttccggccaacggcttaatagcgcctgcaatacacgggcggttgtacttttccccaccgcgacactgccagcaatactgataatgtaaggaatgcgttgcccgttggtaccaagaaactgttccagaactgcctgacggcgcagattcgagcttatatagaagttcagcaaacgtgacaaaggtaaatagatctcggcaacttcttctaacgagagatcttcattaatacctttgagacgggcgatctcatcttccgataacgtcataggtacggaatcacgcagagctgcccactggttgcggtcaaactgtaggtaaggcgtcattaacgtttgctcttttatactcataagcatgtttctggcggtcatagctctatcggcaaagcgatatttgccatggcgcgtcacagttctgttgaatgggttaatgggcaggagggtaacaccagatggggaggaataataagaaaaaatctctgccaggaagctatcgttgaaaagcaatgtgacagatattccatctgataaaaagaattatggtttagcaggagcgcattgttgagcacaatgatgttgaaaaagtgtgctaatctgccctccgttcggctgtttcttcatcgtgtcgcataaaatgtgaccaataaaacaaattatgcaattttttagttgcatgaactcgcatgtctccatagaatgcgcgctacttgatgccgacttagctcagtaggtagagcaactgacttgtaatcagtaggtcaccagttcgattccggtagtcggcaccatcaagtccggtggggttcccgagcggccaaagggagcagactgtaaatctgccgtcacagacttcgaaggttcgaatccttcccccaccaccaatttcggccacgcgatggcgtagcccgagacgataagttcgcttaccggctcgaataaagagagcttctctcgatattcagtgcagaatgaaaatcaggtagccgagttccaggatgcgggcatcgtataatggctattacctcagccttccaagctgatgatgcgggttcgattcccgctgcccgctccaagatgtgctgatatagctcagttggtagagcgcacccttggtaagggtgaggtcggcagttcgaatctgcctatcagcaccacttcttttctcctccctgttttttccttctgtttattgcattcaacaagtcgggcatgttgcctggttgatgtggtgatatcaccgatttatccgtgtcttagagggacaatcgatgtctaaagaaaagtttgaacgtacaaaaccgcacgttaacgtcggtactatcggccacgttgaccatggtaaaacaacgctgaccgctgcaatcactaccgtactggctaaaacctacggcggtgctgctcgcgcattcgaccagatcgataacgcgccggaagaaaaagctcgtggtatcaccatcaacacttctcacgttgaatacgacaccccgacccgtcactacgcacacgtagactgcccggggcacgccgactatgttaaaaacatgatcaccggtgctgcgcagatggacggcgcgatcctggtagttgctgcgactgacggcccgatgccgcagactcgtgagcacatcctgctgggtcgtcaggtaggcgttccgtacatcatcgtgttcctgaacaaatgcgacatggttgatgacgaagagctgctggaactggttgaaatggaagttcgtgaacttctgtctcagtacgacttcccgggcgacgacactccgatcgttcgtggttctgctctgaaagcgctggaaggcgacgcagagtgggaagcgaaaatcctggaactggctggcttcctggattcttacattccggaaccagagcgtgcgattgacaagccgttcctgctgccgatcgaagacgtattctccatctccggtcgtggtaccgttgttaccggtcgtgtagaacgcggtatcatcaaagttggtgaagaagttgaaatcgttggtatcaaagagactcagaagtctacctgtactggcgttgaaatgttccgcaaactgctggacgaaggccgtgctggtgagaacgtaggtgttctgctgcgtggtatcaaacgtgaagaaatcgaacgtggtcaggtactggctaagccgggcaccatcaagccgcacaccaagttcgaatctgaagtgtacattctgtccaaagatgaaggcggccgtcatactccgttcttcaaaggctaccgtccgcagttctacttccgtactactgacgtgactggtaccatcgaactgccggaaggcgtagagatggtaatgccgggcgacaacatcaaaatggttgttaccctgatccacccgatcgcgatggacgacggtctgcgtttcgcaatccgtgaaggcggccgtaccgttggcgcgggcgttgtagcaaaagttctgagctaattgccgataacatttgacgcaatgcgcactaaaagggcatcatttgatgccctttttgcacgctttcgtaccagaacctggctcatcagtgattttctttgtcataatcattgctgagacaggctctgttgagggcgtataatccgaaaagctaatacgcgtttcgatttggtttgcctcgcgatcgcggggtgaaaatgtttgtagaaaacttctgacaggttggtttatgagtgcgaataccgaagctcaaggaagcgggcgcggcctggaagcgatgaagtgggtcgttgtggtggcattgctcctggtggcgattgtcggcaactatctttatcgcgacattatgctgccgctgcgtgcgctggccgtagtaattctgattgctgcagcgggtggtgtcgcgctgttaacgacaaaaggtaaagctaccgttgcttttgcccgtgaagcgcgtaccgaagtccgtaaggtcatttggccgactcgccaggaaacattgcacaccacgctgattgtggctgcggttaccgcagtaatgtcactgatcctgtggggactggatggtattctggttcgcctggtatcctttatcactggcctgaggttctgagatgtctgaagctcctaaaaagcgctggtacgtcgttcaggcgttttccggttttgaaggccgcgtagcaacgtcgctgcgtgagcatatcaaattacacaacatggaagatttgtttggtgaagtcatggtaccaaccgaagaagtggttgaaatccgtggcggtcagcgtcgcaaaagcgaacgtaaattcttccctggctacgtcctcgttcagatggtgatgaacgacgcgagctggcacctggtgcgcagcgtaccgcgtgtgatgggcttcatcggcggtacttccgatcgtcctgcgccaatcagcgataaagaagtcgatgcgattatgaaccgcctgcagcaggttggtgataagccgcgtccgaaaacgctgtttgaaccgggtgaaatggtccgtgttaatgatggtccgttcgctgacttcaacggtgttgttgaagaagtggattacgagaaatctcgtctgaaagtgtctgtttctatcttcggtcgtgcgaccccggtagagctggacttcagccaggttgaaaaagcctaacccagcgatcaaaaaagcggcgatttaatcgttgcacaaggcgtgagattggaatacaatttcgcgccttttgtttttatgggccttgcccgtaaaacgattttttatatcacggggagcctctcagaggcgttattacccaacttgaggaatttataatggctaagaaagtacaagcctatgtcaagctgcaggttgcagctggtatggctaacccgagtccgccagtaggtccggctctgggtcagcagggcgtaaacatcatggaattctgcaaagcgttcaacgcaaaaactgattccatcgaaaaaggtctgccgattccggtagtaatcaccgtttacgctgaccgttctttcactttcgttaccaagaccccgccggcagcagttctgctgaaaaaagcggctggtatcaagtctggttccggtaagccgaacaaagacaaagtgggtaaaatttcccgcgctcagctgcaggaaatcgcgcagaccaaagctgccgacatgactggtgccgacattgaagcgatgactcgctccatcgaaggtactgcacgttccatgggcctggtagtggaggactaagaaatggctaaactgaccaagcgcatgcgtgttatccgcgagaaagttgatgcaaccaaacagtacgacatcaacgaagctatcgcactgctgaaagagctggcgactgctaaattcgtagaaagcgtggacgtagctgttaacctcggcatcgacgctcgtaaatctgaccagaacgtacgtggtgcaactgtactgccgcacggtactggccgttccgttcgcgtagccgtatttacccaaggtgcaaacgctgaagctgctaaagctgcaggcgcagaactggtaggtatggaagatctggctgaccagatcaagaaaggcgaaatgaactttgacgttgttattgcttctccggatgcaatgcgcgttgttggccagctgggccaggttctgggtccgcgcggcctgatgccaaacccgaaagtgggtactgtaacaccgaacgttgctgaagcggttaaaaacgctaaagctggccaggttcgttaccgtaacgacaaaaacggcatcatccacaccaccatcggtaaagtggactttgacgctgacaaactgaaagaaaacctggaagctctgctggttgcgctgaaaaaagcaaaaccgactcaggcgaaaggcgtgtacatcaagaaagttagcatctccaccaccatgggtgcaggtgttgcagttgaccaggctggcctgagcgcttctgtaaactaatgcctttacgtgggcggtgattttgtctacaatcttacccccacgtataatgcttaatgcagacgtatatccgagatattcgggttgtggcaaggcggcaactgagtgagtcgccaggagcatagctaactatgtgactggtgcgaatgaaggaagccaacgccgtcacaagctgaatagcgacggatagaaaagatttgttcgttggagcctggcctatccaggcctccgtcgaagaccgcaggagtttcgcaagaaacttaatcccctgcgtagacggtgacagaacgctaagattattcttttatattctggcttgtttctgctcaccgtaattaagacgctctctccgtttggaggagtgaagtgagttccagagattttctctggcaaacatccaggagcaaagctaatggctttaaatcttcaagacaaacaagcgattgttgctgaagtcagcgaagtagccaaaggcgcgctgtctgcagtagttgcggattcccgtggcgtaactgtagataaaatgactgaactgcgtaaagcaggtcgcgaagctggcgtatacatgcgtgttgttcgtaacaccctgctgcgccgtgctgttgaaggtactccgttcgagtgcctgaaagacgcgtttgttggtccgaccctgattgcatactctatggaacacccgggcgctgctgctcgtctgttcaaagagttcgcgaaagcgaatgcaaaatttgaggtcaaagccgctgcctttgaaggtgagctgatcccggcgtctcagatcgaccgcctggcaactctgccgacctacgaagaagcaattgcacgcctgatggcaaccatgaaagaagcttcggctggcaaactggttcgtactctggctgctgtacgcgatgcgaaagaagctgcttaatcgcagttatctttttaacgcattcgcttacgtataaacttattctgatattcaggaacaatttaaatgtctatcactaaagatcaaatcattgaagcagttgcagctatgtctgtaatggacgttgtagaactgatctctgcaatggaagaaaaattcggtgtttccgctgctgctgctgtagctgtagctgctggcccggttgaagctgctgaagaaaaaactgaattcgacgtaattctgaaagctgctggcgctaacaaagttgctgttatcaaagcagtacgtggcgcaactggcctgggtctgaaagaagctaaagacctggtagaatctgcaccggctgctctgaaagaaggcgtgagcaaagacgacgcagaagcactgaaaaaagctctggaagaagctggcgctgaagttgaagttaaataagccaacccttccggttgcagcctgagaaatcaggctgatggctggtgactttttagtcaccagcctttttgcgctgtaaggcgccagtagcgtttcacactgtttgactactgctgtgcctttcaatgcttgtttctatcgacgacttaatatactgcgacaggacgtccgttctgtgtaaatcgcaatgaaatggtttaagcgtgatagcaacaggcattgcggaaagtgttccattttccggtcaacaaaatagtgttgcacaaactgtccgctcaatggacagatgggtcgacttgtcagcgagctgaggaaccctatggtttactcctataccgagaaaaaacgtattcgtaaggattttggtaaacgtccacaagttctggatgtaccttatctcctttctatccagcttgactcgtttcagaaatttatcgagcaagatcctgaagggcagtatggtctggaagctgctttccgttccgtattcccgattcagagctacagcggtaattccgagctgcaatacgtcagctaccgccttggcgaaccggtgtttgacgtccaggaatgtcaaatccgtggcgtgacctattccgcaccgctgcgcgttaaactgcgtctggtgatctatgagcgcgaagcgccggaaggcaccgtaaaagacattaaagaacaagaagtctacatgggcgaaattccgctcatgacagacaacggtacctttgttatcaacggtactgagcgtgttatcgtttcccagctgcaccgtagtccgggcgtcttctttgactccgacaaaggtaaaacccactcttcgggtaaagtgctgtataacgcgcgtatcatcccttaccgtggttcctggctggacttcgaattcgatccgaaggacaacctgttcgtacgtatcgaccgtcgccgtaaactgcctgcgaccatcattctgcgcgccctgaactacaccacagagcagatcctcgacctgttctttgaaaaagttatctttgaaatccgtgataacaagctgcagatggaactggtgccggaacgcctgcgtggtgaaaccgcatcttttgacatcgaagctaacggtaaagtgtacgtagaaaaaggccgccgtatcactgcgcgccacattcgccagctggaaaaagacgacgtcaaactgatcgaagtcccggttgagtacatcgcaggtaaagtggttgctaaagactatattgatgagtctaccggcgagctgatctgcgcagcgaacatggagctgagcctggatctgctggctaagctgagccagtctggtcacaagcgtatcgaaacgctgttcaccaacgatctggatcacggcccatatatctctgaaaccttacgtgtcgacccaactaacgaccgtctgagcgcactggtagaaatctaccgcatgatgcgccctggcgagccgccgactcgtgaagcagctgaaagcctgttcgagaacctgttcttctccgaagaccgttatgacttgtctgcggttggtcgtatgaagttcaaccgttctctgctgcgcgaagaaatcgaaggttccggtatcctgagcaaagacgacatcattgatgttatgaaaaagctcatcgatatccgtaacggtaaaggcgaagtcgatgatatcgaccacctcggcaaccgtcgtatccgttccgttggcgaaatggcggaaaaccagttccgcgttggcctggtacgtgtagagcgtgcggtgaaagagcgtctgtctctgggcgatctggataccctgatgccacaggatatgatcaacgccaagccgatttccgcagcagtgaaagagttcttcggttccagccagctgtctcagtttatggaccagaacaacccgctgtctgagattacgcacaaacgtcgtatctccgcactcggcccaggcggtctgacccgtgaacgtgcaggcttcgaagttcgagacgtacacccgactcactacggtcgcgtatgtccaatcgaaacccctgaaggtccgaacatcggtctgatcaactctctgtccgtgtacgcacagactaacgaatacggcttccttgagactccgtatcgtaaagtgaccgacggtgttgtaactgacgaaattcactacctgtctgctatcgaagaaggcaactacgttatcgcccaggcgaactccaacttggatgaagaaggccacttcgtagaagacctggtaacttgccgtagcaaaggcgaatccagcttgttcagccgcgaccaggttgactacatggacgtatccacccagcaggtggtatccgtcggtgcgtccctgatcccgttcctggaacacgatgacgccaaccgtgcattgatgggtgcgaacatgcaacgtcaggccgttccgactctgcgcgctgataagccgctggttggtactggtatggaacgtgctgttgccgttgactccggtgtaactgcggtagctaaacgtggtggtgtcgttcagtacgtggatgcttcccgtatcgttatcaaagttaacgaagacgagatgtatccgggtgaagcaggtatcgacatctacaacctgaccaaatacacccgttctaaccagaacacctgtatcaaccagatgccgtgtgtgtctctgggtgaaccggttgaacgtggcgacgtgctggcagacggtccgtccaccgacctcggtgaactggcgcttggtcagaacatgcgcgtagcgttcatgccgtggaatggttacaacttcgaagactccatcctcgtatccgagcgtgttgttcaggaagaccgtttcaccaccatccacattcaggaactggcgtgtgtgtcccgtgacaccaagctgggtccggaagagatcaccgctgacatcccgaacgtgggtgaagctgcgctctccaaactggatgaatccggtatcgtttacattggtgcggaagtgaccggtggcgacattctggttggtaaggtaacgccgaaaggtgaaactcagctgaccccagaagaaaaactgctgcgtgcgatcttcggtgagaaagcctctgacgttaaagactcttctctgcgcgtaccaaacggtgtatccggtacggttatcgacgttcaggtctttactcgcgatggcgtagaaaaagacaaacgtgcgctggaaatcgaagaaatgcagctcaaacaggcgaagaaagacctgtctgaagaactgcagatcctcgaagcgggtctgttcagccgtatccgtgctgtgctggtagccggtggcgttgaagctgagaagctcgacaaactgccgcgcgatcgctggctggagctgggcctgacagacgaagagaaacaaaatcagctggaacagctggctgagcagtatgacgaactgaaacacgagttcgagaagaaactcgaagcgaaacgccgcaaaatcacccagggcgacgatctggcaccgggcgtgctgaagattgttaaggtatatctggcggttaaacgccgtatccagcctggtgacaagatggcaggtcgtcacggtaacaagggtgtaatttctaagatcaacccgatcgaagatatgccttacgatgaaaacggtacgccggtagacatcgtactgaacccgctgggcgtaccgtctcgtatgaacatcggtcagatcctcgaaacccacctgggtatggctgcgaaaggtatcggcgacaagatcaacgccatgctgaaacagcagcaagaagtcgcgaaactgcgcgaattcatccagcgtgcgtacgatctgggcgctgacgttcgtcagaaagttgacctgagtaccttcagcgatgaagaagttatgcgtctggctgaaaacctgcgcaaaggtatgccaatcgcaacgccggtgttcgacggtgcgaaagaagcagaaattaaagagctgctgaaacttggcgacctgccgacttccggtcagatccgcctgtacgatggtcgcactggtgaacagttcgagcgtccggtaaccgttggttacatgtacatgctgaaactgaaccacctggtcgacgacaagatgcacgcgcgttccaccggttcttacagcctggttactcagcagccgctgggtggtaaggcacagttcggtggtcagcgtttcggggagatggaagtgtgggcgctggaagcatacggcgcagcatacaccctgcaggaaatgctcaccgttaagtctgatgacgtgaacggtcgtaccaagatgtataaaaacatcgtggacggcaaccatcagatggagccgggcatgccagaatccttcaacgtattgttgaaagagattcgttcgctgggtatcaacatcgaactggaagacgagtaattctcgctcaaacaggtcactgctgtcgggttaaaacccggcagcggattgtgctaactccgacgggagcaaatccgtgaaagatttattaaagtttctgaaagcgcagactaaaaccgaagagtttgatgcgatcaaaattgctctggcttcgccagacatgatccgttcatggtctttcggtgaagttaaaaagccggaaaccatcaactaccgtacgttcaaaccagaacgtgacggccttttctgcgcccgtatctttgggccggtaaaagattacgagtgcctgtgcggtaagtacaagcgcctgaaacaccgtggcgtcatctgtgagaagtgcggcgttgaagtgacccagactaaagtacgccgtgagcgtatgggccacatcgaactggcttccccgactgcgcacatctggttcctgaaatcgctgccgtcccgtatcggtctgctgctcgatatgccgctgcgcgatatcgaacgcgtactgtactttgaatcctatgtggttatcgaaggcggtatgaccaacctggaacgtcagcagatcctgactgaagagcagtatctggacgcgctggaagagttcggtgacgaattcgacgcgaagatgggggcggaagcaatccaggctctgctgaagagcatggatctggagcaagagtgcgaacagctgcgtgaagagctgaacgaaaccaactccgaaaccaagcgtaaaaagctgaccaagcgtatcaaactgctggaagcgttcgttcagtctggtaacaaaccagagtggatgatcctgaccgttctgccggtactgccgccagatctgcgtccgctggttccgctggatggtggtcgtttcgcgacttctgacctgaacgatctgtatcgtcgcgtcattaaccgtaacaaccgtctgaaacgtctgctggatctggctgcgccggacatcatcgtacgtaacgaaaaacgtatgctgcaggaagcggtagacgccctgctggataacggtcgtcgcggtcgtgcgatcaccggttctaacaagcgtcctctgaaatctttggccgacatgatcaaaggtaaacagggtcgtttccgtcagaacctgctcggtaagcgtgttgactactccggtcgttctgtaatcaccgtaggtccatacctgcgtctgcatcagtgcggtctgccgaagaaaatggcactggagctgttcaaaccgttcatctacggcaagctggaactgcgtggtcttgctaccaccattaaagctgcgaagaaaatggttgagcgcgaagaagctgtcgtttgggatatcctggacgaagttatccgcgaacacccggtactgctgaaccgtgcaccgactctgcaccgtctgggtatccaggcatttgaaccggtactgatcgaaggtaaagctatccagctgcacccgctggtttgtgcggcatataacgccgacttcgatggtgaccagatggctgttcacgtaccgctgacgctggaagcccagctggaagcgcgtgcgctgatgatgtctaccaacaacatcctgtccccggcgaacggcgaaccaatcatcgttccgtctcaggacgttgtactgggtctgtactacatgacccgtgactgtgttaacgccaaaggcgaaggcatggtgctgactggcccgaaagaagcagaacgtctgtatcgctctggtctggcttctctgcatgcgcgcgttaaagtgcgtatcaccgagtatgaaaaagatgctaacggtgaattagtagcgaaaaccagcctgaaagacacgactgttggccgtgccattctgtggatgattgtaccgaaaggtctgccttactccatcgtcaaccaggcgctgggtaaaaaagcaatctccaaaatgctgaacacctgctaccgcattctcggtctgaaaccgaccgttatttttgcggaccagatcatgtacaccggcttcgcctatgcagcgcgttctggtgcatctgttggtatcgatgacatggtcatcccggagaagaaacacgaaatcatctccgaggcagaagcagaagttgctgaaattcaggagcagttccagtctggtctggtaactgcgggcgaacgctacaacaaagttatcgatatctgggctgcggcgaacgatcgtgtatccaaagcgatgatggataacctgcaaactgaaaccgtgattaaccgtgacggtcaggaagagaagcaggtttccttcaacagcatctacatgatggccgactccggtgcgcgtggttctgcggcacagattcgtcagcttgctggtatgcgtggtctgatggcgaagccggatggctccatcatcgaaacgccaatcaccgcgaacttccgtgaaggtctgaacgtactccagtacttcatctccacccacggtgctcgtaaaggtctggcggataccgcactgaaaactgcgaactccggttacctgactcgtcgtctggttgacgtggcgcaggacctggtggttaccgaagacgattgtggtacccatgaaggtatcatgatgactccggttatcgagggtggtgacgttaaagagccgctgcgcgatcgcgtactgggtcgtgtaactgctgaagacgttctgaagccgggtactgctgatatcctcgttccgcgcaacacgctgctgcacgaacagtggtgtgacctgctggaagagaactctgtcgacgcggttaaagtacgttctgttgtatcttgtgacaccgactttggtgtatgtgcgcactgctacggtcgtgacctggcgcgtggccacatcatcaacaagggtgaagcaatcggtgttatcgcggcacagtccatcggtgaaccgggtacacagctgaccatgcgtacgttccacatcggtggtgcggcatctcgtgcggctgctgaatccagcatccaagtgaaaaacaaaggtagcatcaagctcagcaacgtgaagtcggttgtgaactccagcggtaaactggttatcacttcccgtaatactgaactgaaactgatcgacgaattcggtcgtactaaagaaagctacaaagtaccttacggtgcggtactggcgaaaggcgatggcgaacaggttgctggcggcgaaaccgttgcaaactgggacccgcacaccatgccggttatcaccgaagtaagcggttttgtacgctttactgacatgatcgacggccagaccattacgcgtcagaccgacgaactgaccggtctgtcttcgctggtggttctggattccgcagaacgtaccgcaggtggtaaagatctgcgtccggcactgaaaatcgttgatgctcagggtaacgacgttctgatcccaggtaccgatatgccagcgcagtacttcctgccgggtaaagcgattgttcagctggaagatggcgtacagatcagctctggtgacaccctggcgcgtattccgcaggaatccggcggtaccaaggacatcaccggtggtctgccgcgcgttgcggacctgttcgaagcacgtcgtccgaaagagccggcaatcctggctgaaatcagcggtatcgtttccttcggtaaagaaaccaaaggtaaacgtcgtctggttatcaccccggtagacggtagcgatccgtacgaagagatgattccgaaatggcgtcagctcaacgtgttcgaaggtgaacgtgtagaacgtggtgacgtaatttccgacggtccggaagcgccgcacgacattctgcgtctgcgtggtgttcatgctgttactcgttacatcgttaacgaagtacaggacgtataccgtctgcagggcgttaagattaacgataaacacatcgaagttatcgttcgtcagatgctgcgtaaagctaccatcgttaacgcgggtagctccgacttcctggaaggcgaacaggttgaatactctcgcgtcaagatcgcaaaccgcgaactggaagcgaacggcaaagtgggtgcaacttactcccgcgatctgctgggtatcaccaaagcgtctctggcaaccgagtccttcatctccgcggcatcgttccaggagaccactcgcgtgctgaccgaagcagccgttgcgggcaaacgcgacgaactgcgcggcctgaaagagaacgttatcgtgggtcgtctgatcccggcaggtaccggttacgcgtaccaccaggatcgtatgcgtcgccgtgctgcgggtgaagctccggctgcaccgcaggtgactgcagaagacgcatctgccagcctggcagaactgctgaacgcaggtctgggcggttctgataacgagtaatcgttaatccgcaaataacgtaaaaacccgcttcggcgggtttttttatggggggagtttagggaaagagcatttgtcagaatatttaaggaatttctgaatactcataatcaatgtagagatgactaatatcctgaaactgactgaactaattgagtcaaactcggcaaggattcgatactattcctgtgtaactttcttaaggaacgagaatgaaacaggaagtggaaaagtggcgaccttttggacatccggatggtgatattcgtgatttatcatttcttgatgctcatcaggctgtctacgttcagcatcatgagggcaaagagcctttagagtatcgcttttgggttacctactctcttcactgcttcacaaaagattatgaacatcagacgaacgaagaaaaacaatcgttaatgtaccacgcgcctaaagaatctcgtcccttctgccagcaccgttataacttagcgcgcacacacttaaaaagaactattttggcgctgccagaaagcaacgttattcatgccgggtatggtagctatgccgtgattgaggtggacttagacggaggagataaggcattttactttgttgcgttcagggctttcagggaaaagaaaaaactccgtttgcatgtaactagcgcttatcccatttctgaaaaacagaaaggtaaatcagtgaaatttttcaccattgcctacaacttattgagaaataagcagcttcctcagccctcaaaataacaaaacccaccttaaggtgggtttcgccagagaattatctctggtattcagaacgccattaccggactttgccttgaccttgcgataatcgcaggttgcgggatgtctgaatttcttcagtctgctgcatcctggaagatgagaacatgtgttcttattttcgtctctatcatagttgagtatttactctcttacaatcagatctctttcattgctcaacaggcgatggcttcagactttgcattacggaatttttaagaaaggcagggcgaaacgaggaagaagcttttcgccctggacaacattcctgctgacggcactaccataaaaaaacacaacgctttcaacaaccttgcgtttttcatcttccgtagcggctcggaataaatttacgttcttacattccgtctcatagtctttgcgaggcgcgtcccagatagctgtcccagtctttccataccggctgcaaaccctgagcggttaacgcggcagcaaccgcttccggtctgcgatcgtcgtgcggtgagaactgttccaactcggggtgattatcggcatagccacctggctgcgttttcgagaaggcgctgacgttattgatcgccagcggaataacgcgatcgcgaaaccacggtgattcccgcgtggagagtgacagttcaatctccggtgcaagcagtcggaaggcgcagatggtttgcactaactggcgttcatccataatcgacgcaggctcaatgccgccagtacacgggcgcaggcgcggaaaggagacagagtaacggctttgccagtaatgctgttgcagccatagcaaatgttcggcaaccatatagctgtcaacgcgccagttgtcggaaaggccaattagcgcgccgaggcctatcttatcaatccccgcacgccccagccgatccggcgtttccagccgccagaagaagtcctgttttttgcctttcagatgatggcgggcataagtcgcctcgtgatatgtctcctgataaaccatcacgccatccagaccaagttgctttaactcggcgtattccgtctccgccagcggttgcacttccatctgtagtgaagagaactgttcacgaagggcagggagatgacgacgaaagtaatccatccccactttcgcctgatgttcaccagtgactaacagcagatgttcaaagcccatctcccgtatagcggcactttccctggcaatatccgcttcatccagcgttttgcgcttgatgcgattactcatggaaaatccacagtacgtgcagtcgttagcgcaaagattggaaagataaagcgggacgtagaaactaactgtgttgccaaatcgctgacgggtcagacgctgcgcccgttgggccagttgttccagatagccactggcggcaggcgataacagcgccatcatgtcgtcgcgggtgagttgcgaggcatttagcgcccgctctacgtcagcagccgttttgccgttgatacgcaggcggatgtcgtcccagtccagttgtcgccagcgatcgctgaaggttttcatgccgatgcctccagaaatccggtcagcgggctggtggcatgagcaaaataactgcggctgcccggtccggactgacgtgccagtaggcctgcttctaccgccagacgaaatgccttcgccatgttgacgggatcgtccgcgacggcaatcgccgtattcactaacaccgcgtcggcccccatttccagcgcctgcgcggcatggctgggaacgccgatgccagcatcgacaaccaccggcactgtggcctgctggataataatctccagcatggcgcgggtttccagtccctgattcgagccaatcggcgcgccgagcggcatcaccgctgcacagccgacttcttccagacgtttacacaataccggatcggccccgcagtaaggcagcacgacaaatccctgttgtaccagcgtttcggcggctttcagggtttcgatgggatcgggcaacagccagcgggcgtcagggtgaatctctaattttaaccagtttgtgcctaacgcttcacgagccagatgggcggcgaaaatggcttcttccgctgttttcgccccggatgtatttggcagcagggtcacacccgccgcgataagcggttcgaggatagcgtcgttgtgctggcgcaagtcgacacgtttcatcgccagtgtcaccagctggctgccggaagcgcggatcgcctccaccatcagttgtgaagaagcgaatttccctgtgccggtaaacagatgtgaatcaaacgttttgtccgcaatacgtaacatttcaaccccctgcaataacctgaaaaagcaggatctggtcgccatcctgcacgatatgttgcgcccactgctcacgcgggacgatttgctgattaatcgccagagccgcgcccgcttgtcgttggtcgagttgctccagtagttcgtgaacagtttgcccggcggcgcactgcatcgcttgatcgttaaacaggatctgcattgcttcctccgcataccgggcaaccactggcgcggcgcaacgccaggctgcgccactggctcgatttaccgtcgaacagtcggagttctcccgcaggtgtctctataccgcttaataacttaatggcttccagtgcctgcaaagtgcccataaccccgaccaccgggccaaccacgcccgccgtgcggcagttgcgttctggctcctggttatctggccacaggcagcggtaacacccctgctcccagggcggcgtcagtaccatcaactgaccgccaaatccgaccgcgctggcggtgataagcggcgtgttgagtgccacgcaggcggcattaatctcctggcgagtcgccatattgtcggtacagtcgagcaccacatcggcccgtgcaaccgcatcttttaacgcctcacccgttaaccgttgttgtaatgctgtcagttgaatgtcgggattcaactgtgtcagtcgctgttggctgacctgcgatttcgggcgatcgatatcttcagtggtaaagaggatttgtcgttgcagattgcttaaatgcacatcgtcgtcatctgccagtaccagcgtcccgacgccagcgcccgccaggtacagcgcagcaggtgtacccagcccgcccagaccgataatcagcacctggctgtcgagcagtttttgctgcccgtccagagcgatatcgtcgagcaggatttggcggctataacgcataaagtcacggtcattcatcgccaactcctgcaatttccagcaactgtgccgttgccaaacgccagtctgcggcttgagtaatggcgctgacgacggcgatactgccgacacccgttgctatcaccgcaggcgcgcgtgccagactgataccgccaatcgccacggtgggataatccgccagtcgctcaacatgccgtgccagctgttccagcccctgcggtgcagaaggcatctgtttggtttgcgtcgggaacacatgtcccagcgcgatataagaggggcgtgctgccagcgcgacgtcgatttccatatcgtcatgtgtcgaaacgcccagccgcaggcctgccgcgcggatggcattgagatcggtggcttgcaaatcttcctgccccaaatggacgccatacgcctgatgcttgatcgccagccgccagtaatcgttgataaacaatcgcgcgttatagcggcggcccagcgcaattgccgccacgacatcggcttccacctcttcatcgcgccgatctttgatgcgtagctggagagtacgtacgcctgcatccaacagacgttcgatccactgtacgctgtccaccaccgggtacagtcctgaacgaaaaggtacaggaggaaaatcaggctgatacatcacgcttcctccttacgcaggtagatttctccgcctctggcacggaagttctccgacatatccgccattcccatttcaatagtttgcgtggcggcgtaatcacgcacttcctggctgattttcatcgagcagaatttcggcccacacatggagcaaaaatgggcgactttacctgactcttgcggcagggtttcatcgtgataagcgcgggcggtaaacgggtcgagggccagattaaactggtcttcccagcgaaattcgaagcgggctttcgacatggcgttatcgcgaatttgcgcgcccggatgccctttcgccaggtcagcggcgtgggcagcaatcttataggtgataagcccctgcttaacatcttctttattgggcagacccagatgctcttttggcgttacgtaacagagcatcgcgcagccaaaccagccaatcatcgccgcaccaatccccgacgtgaagtggtcatagcccggcgcaatatcggtagttagcggccccagagtgtaaaacggcgcttcgtggcagtgctctaactcctcggtcatattgcggcggatcatctgcatcggcacgtggcctgggccttcaatcatcacctgcacgtcatattcccaggcaattttggtcagttcgcccagcgtatgcagctcggcaaactgcgcttcatcgttggcgtcctgaatagaaccggggcgcagaccgtcgcccagcgacagcgaaacgtcataagcggcacagatttcacaaatttcgcggaagtgttgatagaggaaattttcctgatgatgggagaggcaccatttcgccataatcgaaccgccgcgagagacgataccggtcaggcgtttcgcggtcatcggcacatagcgcagcagtacgcccgcatggatagtgaagtaatccacaccttgctcggcctgttccagcagcgtgtcgcggaacgcttcccaggtaagatcttcggcgatcccgttaaccttctccagcgcctggtagatcggcactgtaccgatcggcaccgggctgttacgcaaaatccactcgcgggtttcgtgaatatagcgaccggtggagagatccatcaccgtatccgctccccagcgcgtggaccataccagcttttccacttcttcttcgatggaagaggtgaccgccgagttgccgatattggcgttaacttttaccaggaaattgcgaccaataatcatcggctccgattccggatgattaatgttggccgggataatcgcacgtccggcagcaacttcatcacggacaaattccgcagtgatattttccggcagatgtgcgccaaagctcattcccggatgctggtggcgtaaaacctcgctacggatgcgctcgcggcccatattctcgcggatggcgatgaattccatttccggcgtgatgatgccctggcgggcgtagtgcagttgggtgacacggcgtcctgctttggcgcgttttggtgttagtacgccgctaaaacgcagttcgtcgaggccatcatctgccagccgcgctttagtgtaatcggaactgcgcacggtaagttcttcggtatcgccgcgcgcatcgatccacggctggcgtagttttgccagcccttgctgcacgttaatggcaatctgcggatcaccatacgggccggaggtgtcgtagaccggaatcgcttcgttttcttcgtactgcggctgttctttgctaccgccaattagcgtcgggctaagctggatctcacgcatcggcacgcgcacgccggggtgtgtgccagtgatataaatgcgttttgagttgggaaaggcggtgccttccagggtgtcgataaaatgttgggcccgggcgcgttgttcgcggcgggtcagttttgttgcagacatagctcattccaaaaagttaaggacgtggcttgtcagacgacggatgaagcaagagacgatcgccgcaggggcgatgcgatagcagattaactcttgttcccttcgcaggtattagcctgatcaggttccgcggatcccgaataaacggtctcagccagttaaggcactccgacaagaaattagccccgcaaatggggcattgaatgtaaattacgcgttaacagcgcagaactcaagcaggatgtttgacgcgggcggcgtcaagcaccagcagaatcagcttatcttccagcacaaagcgcgcttccagcgcctcgccgatgtcagataaaacctgttgaaactcaaggtaattatcatgatcgatggcggtttccagactggaatcgtagtaatccataatctgttgagtattggcttcgagttgcggccaaatcttcgcggcgcgcgcgagttgcccgttgccttccagcttatgaagaatgcgctcataaatactgaaatgtccggcagacaagtaatcgaccaggctctgacaaaaatcatcaagggctttttcgtttagcctcatgtacgattctttgccaggcttaatgccaaccagattgtagtaagccacgagcagatgcttacgtacatgtagccagcgatcaaccagtttgttacttcctctgacgcgctccgtcaggttatcgagctggttaagcatgattgactccgcaagtttgtattcaaaaactgctcagtgagaaatgtaaaaaccatgttaaacatgccagtgatgcaaaggtagtgcaagagctatggatcgtataattgaaaaattagatcacggctggtgggtcgtcagccatgaacaaaaattatggttgccgaagggagaattgccatatggcgaagcggcaaatttcgatcttgtgggtcagcgcgcactacaaatcggcgaatggcagggggaacctgtttggttagtacaacagcagcggcgtcacgatatggggtcggtacgtcaggtcattgatctcgatgttgggctgtttcaactggccggacgaggcgtacaactggcggagttttaccgatcgcataaatactgtggttactgcgggcatgaaatgtatccgagcaaaaccgaatgggcgatgctgtgcagccattgccgtgagcgttactacccgcaaatcgccccctgcattattgttgccatccgtcgcgatgattcgatcctcctcgcccagcatacccgccatcgtaacggtgtccatacagtacttgccggattcgtcgaagtgggcgaaaccctcgagcaggcagtcgcgcgggaagtgatggaagagagcggaattaaagttaaaaacttgcgttacgtgacttctcagccgtggccgtttcctcagtctttaatgaccgcgtttatggcggaatatgacagcggcgacatcgtgatcgacccgaaagaattgctcgaggcgaactggtatcgctatgacgatttgccgttactcccgccgcccggcaccgtagcgcgccgtctgatagaagatacggtggcgatgtgtcgggcagagtatgagtgatgatacactgaccgcctgacgcactaaggaacagccaaaatgaccgaacttaaaaacgatcgttatctgcgggcgctgctgcgccagcccgttgatgtcactccagtatggatgatgcgccaggcgggtcgctatctaccggaatataaagccacgcgcgcccaggcaggcgattttatgtcgctgtgcaaaaacgccgagctggcgtgcgaagtgactttgcaaccgctgcgtcgctacccgctggatgcggcgatcctcttttccgatatcctcaccgtgccggacgcgatggggttagggctctattttgaagccggagaaggtccgcgttttacctcgccagtcacctgcaaagctgacgtcgataaactgccaattccggacccggaagatgaactgggttacgtgatgaacgcggtgcgtaccattcgtcgcgaactgaaaggcgaagtgccgctgattggtttttccggcagcccgtggacgctggcgacctacatggtggaaggcggcagcagcaaagccttcaccgtgatcaaaaaaatgatgtatgccgatccgcaggcgctgcacgctctgctcgataaactggcgaaaagcgtcactttgtatctgaatgcgcagattaaagccggtgctcaggcagtgatgattttcgacacctggggcggcgtgcttaccgggcgcgattatcaacagttctcgctctattacatgcataaaattgttgatggtttactgcgtgaaaacgacggtcgccgcgtaccggtcacgctgtttaccaaaggcggcggacagtggctggaagccatggcagaaaccggttgcgatgcgctgggcctcgactggacaacggacatcgccgatgcgcgccgccgtgtgggcaataaagtcgcgttgcagggtaatatggatccgtcgatgctgtacgcgccgcctgcccgcattgaagaagaagtagcgactatacttgcaggtttcggtcacggcgaaggtcatgtctttaaccttggtcacggcattcatcaggatgtgccgccagaacatgctggcgtgttcgtggaggcagtgcatcgactgtctgaacagtatcaccgctaaggagtgattatggatctcgcgtcattacgcgctcaacaaatcgaactggcttcttctgtgatccgcgaggatcgactcgataaagatccaccggatctgatcgccggagccgatgtcgggtttgagcagggcggagaagtgacgcgagcggcgatggtgctgctgaaatatccctcgcttgagctggtcgagtataaagttgcccgcatcgccaccaccatgccttacattccaggttttctttccttccgcgaatatcctgcgctgctggcagcgtgggagatgctgtcgcaaaagccggatttagtgtttgtcgatggtcatgggatctcgcatcctcgccgtcttggcgtcgccagccattttggcttattggtggatgtgccgaccattggcgtggcgaaaaaacggctctgcggtaaattcgaaccgctctccagcgaaccgggcgcgctggccccactgatggataaaggcgagcagctggcctgggtctggcgcagcaaagcgcgctgtaacccgttgtttatcgctaccggccatcgggtcagcgtggacagcgcgctggcgtgggtacaacgctgcatgaaaggctatcgtctgccggagccaacgcgctgggcggacgcggtggcctcggaacgtccggcgttcgtgcgctatacagcaaatcagccctaattcaggtaaactgcggataatttccgtatttgagaactcaacatgttacaaaacccaattcatctgcgtctggagcgcctggaaagctggcagcatgtcactttcatggcttgcttatgcgaacgcatgtaccccaattacgccatgttctgccagcaaaccggttttggtgatgggcaaatttaccgtcgcattctcgatctcatctgggaaacgctgaccgttaaagacgcaaaagtaaatttcgacagccaactggagaaatttgaagaagcgattccttcagccgacgatttcgatctgtacggcgtttatccggcaatcgatgcctgcgtggcgttaagtgaactggtccattcgcgtttgagtggtgaaacgctcgaacacgcggtggaagtgagtaagacctccatcacgaccgttgcgatgctggaaatgactcaggctggtcgcgaaatgagcgatgaagagcttaaagaaaacccagctgtagagcaagaatgggacattcagtgggaaatattccgacttttagctgagtgcgaagaacgcgatatcgagctgataaaaggccttagggcagacctgcgtgaggcgggtgagagcaatattggtataatttttcagcaataagaccagaaaacgtgatttaacgcctgatttgtcgtacctggagtcttccctttcgccccccgtctggtctacatttggggggcgaaaaaaagtggctatcggtgcgtgtatgcaggagagtgctattctggcatttccgtcgcactcgatgcttagcaagcgataaacacattgtaaggataacttatgaacaagactcaactgattgatgtaattgcagagaaagcagaactgtccaaaacccaggctaaagctgctctggagtccactctggctgcaattactgagtctctgaaagaaggcgatgctgtacaactggttggtttcggtaccttcaaagtgaaccaccgcgctgagcgtactggccgcaacccgcagaccggtaaagaaatcaaaattgccgcagctaacgtaccggcatttgtttctggcaaggcactgaaagacgcagttaagtaagattgcgtggcagtgaacagttttaacgaaggggtggtttcaccccttttgtctttctggcgtcgatcattgatgctggctggcgctctgcttctcactgcctgtagtcataactcttcacttcctccctttaccgccagtggatttgctgaagaccagggcgcggtacgcatctggcgaaaagacagcggcgataatgtgcatctgcttgccgtgtttagcccgtggcgcagtggcgataccacgacgcgagagtatcgctggcagggcgataacctcacgctcatcaatatcaatgtttacagcaaaccgccggtgaatattcgcgcgcgttttgacgatcgcggtgatctgagctttatgcaacgtgaatccgatggggaaaagcagcagctttctaacgaccaaatcgatttataccgttatcgtgctgatcagatccgccagattagcgatgccttacgtcaggggagagtcgtgctgcgccaggggcgctggcatgcgatggaacagaccgtgaccacctgcgaagggcaaaccattaaacctgatttagattcgcaggcgatagcgcatatcgagcgccgccagagccgctcttctgttgatgtcagcgtggcatggctggaagcgcccgaaggttcgcaattactgttagtggcaaactctgatttctgtcgctggcaacccaacgagaaaacgttctgatttaccagtggcccatacccatatgaccgccaccaccgcagccgccgtagcccatgcccattccggctccgcgcggaatacccgcttcagccatcgcgatatctcgtttcacccgtaactcatctaacgactgacgcaaattctccatctctttggcgaccgcgttaattttgctgctatccggtgggttcgcggctaacagggcattgtattcataacgcttcgtcaccagttgctgttgcagtgcgctgctttgagcgtaaaagtcattatggattttctgccacgctgtctgttgttcgctggtcaaaggcgcggcattttgctgccacataccgtgtccgccgtgagcaaatgcagatgtcgatcccatcgccattgctgaaagcgccatcattaccagggcaattttcgtgttccgtttcatggttaatcctccagtggttgtcttacttcgggtattgcatcttccgtgccaacgatgaaacgctgatatgacgggtaatctggcatgataaacgagtaaaaatgactcgcctgctgcgggtagcgagtcatttttactcattgaaacttaagcctttgtgttacagcgcagggtaagcgctgataaaagatggcatgatttctgctgtcagaaagggatgagcaggcaaagaagaagatgcgttttatgcaacgttctaaagactccttagctaaatggttaagcgcgatcctccccgtggtcattgttgggctggtgggattgtttgcggtaactgtgattcgtgattatgggcgggcaagcgaggcagaccgccaggcattactggaaaaaggtaatgtgcttatccgcgctctggagtcgggaagccgcgtagggatggggatgcgaatgcaccatgtacagcaacaggcgcttctggaagagatggcgggacagccgggagtgttgtggttcgcagtcaccgatgcgcagggcatcattattcttcatagcgaccccgataaggtcgggcgtgcgctctattcgccggatgaaatgcagaaattaaagccagaggaaaactcccgctggcggctgcttgggaaaacggaaactacgcctgcacttgaggtctatcgtttgttccagccaatgtcagcgccctggcggcatggaatgcacaatatgccgcgctgtaacggcaaagctgtgccacaagtagatgcacaacaggctatttttatcgccgttgatgccagtgatctggttgcaacccagagtggggaaaagcgcaataccctgattatcctcttcgccctggcgacggtcttgctggcaagcgtattgtcattcttctggtatcgccgctatctgcgctcgcgccagcttctacaagatgaaatgaagcgcaaagagaagctggtggcgctggggcatcttgcggcaggcgttgcccacgaaatccgtaacccactttcctcgattaaaggactggcgaaatactttgccgagcgcgcgcctgcagggggagaagcgcatcaactggcgcaggtgatggcgaaagaggccgaccgtttaaaccgcgtggtaagcgagttgctggaactggttaagccaacgcatctggctttgcaggcggtggatctcaacacgctgattaaccactcattacagctggtaagtcaggatgcaaacagccgggagatccagttacgctttaccgccaacgacacattaccggaaattcaggccgacccggacaggctgactcaggtcctgttgaatctctatctcaatgctattcaggcgattggtcagcatggcgtgattagcgtgacggccagcgaaagcggcgcgggcgtgaaaatcagcgttaccgacagcggtaagggaattgcggcagatcagcttgatgccatcttcactccgtacttcaccactaaagccgaaggcaccggattggggctggcggtcgtgcataatattgttgaacaacacggtggtacaattcaggtcgcaagccaggagggaaaaggctcaacgttcaccctctggcttccggtcaatattacgcgtaaggacccacaaggatgacgcacgataatatcgatattctggtggtggatgatgacattagccactgcactattttgcaggctttactgcgcggctggggctataacgtcgcgctggcgaacagcgggcgacaggcgttggagcaggtgcgggaacaggtttttgatcttgtgctttgcgatgtgcgaatggcggagatggacggcatcgccacgctgaaagagatcaaagcgttaaacccggcaattccggtgctgattatgactgcgtactccagcgtcgagacggcggtagaggcactgaaaactggggcgctggattatctcatcaagccgctggatttcgataacctacaggcgacgctggaaaaagcgctcgcgcatacgcacagtattgatgctgaaacacctgcggtgactgccagccagttcggtatggtcggtaaaagcccggcgatgcaacacctgctcagtgaaatcgccctcgtcgcgccatcggaagccacggtactgatccacggcgattccggcaccggtaaagagctggtcgccagggcgattcacgccagtagcgcacgtagcgaaaaaccgctggtaacgctcaactgtgcggcactcaacgaatccttgctggaatctgaattgttcggtcacgaaaaaggggcgtttactggagccgataaacgccgggaagggcgctttgttgaggcggacggcggcacgctgtttctcgatgaaattggcgatatctcgccgatgatgcaggtgcgtctgctgcgtgcgattcaggagcgcgaagttcagcgtgtcggtagcaaccagattatctcggttgatgtccggctgattgcggcgacccatcgcgatcttgccgcagaggtgaatgccgggcgttttcgccaggatctctactatcgcctgaatgtggtggcgattgaagtaccatcgctgcggcaacggcgggaagatatccctctgctggctggccattttctgcagcgctttgccgagcgtaatcgcaaggcggtaaaaggttttacgccccaggcgatggatctgttgattcattacgactggccgggaaatattcgtgagctggaaaacgcggtggaacgggcagtggtgctgctgaccggggaatatatttccgaacgcgagctgccgctggcgattgccagtacgccgatcccgctgggacaaagtcaggatattcagccgttggtggaagtggaaaaagaggtgattctggcggcgctggagaaaacgggcggcaacaaaaccgaagccgcccgtcagttagggatcacgcgcaaaacgctattggcaaaactgtcgcgttagttctgctcgcgttcgatagcgcgccagccgatatctttccggcagaagcagtcgtcccagtggatatcggtcattaaggcataggcgcgtttctgcgcttctgccacggtatgacccagcgcggtgacgcacagtacgcgcccgccgttggtcactacctgctcgtcatccgccagttttgtgcccgcgtggaacactttgccgcctgccacttcttccagcggcaggccgtggatcacgtcaccggtgcggtaatcacccggatatccacccgcagccatcaccacgccgagagaagcgcgttcatcccactcggacgttttctcgtccagtttgctttcacaggccgccaggcagagctcaaccagatcggacttcatgcgcagcataatcggctgggtttccggatcgccaaagcggcagttaaattcaataaccttcggattgccctgtttgtcgatcatcaggcccgcgtagagaaaaccggtgtaggtgttgccttccgccgccatgcctttcacggttggccagataatacgttccatggtgcgctgatgaacgtcatcggttactaccggcgcgggggagtaagcgcccatcccgccggtgtttggtccggtatctttatcgcctacgcgtttgtgatcctggctggtagccatcggcagcacatgctcgccgtccaccatcacgataaagctcgcttcttcgccatcgaggaactcttcgataacgatgcgatgacccgcgtcgccaaaagcgttgcccgccagcatatcgtgaacagccgcttccgcttcttccagcgtcatcgccacgataacgcctttcccggcagccagaccgtccgctttaatgacgattggcgcgcctttctcacgcagatacgccagcgcaggttctacctcggtgaagttctggtattccgccgtagggatcttatggcgggccaggaaatctttggtaaacgcttttgagccttccagttgggccgcacctgcggttgggccgaagattttcagcccggcggcgcggaaggtatcgaccacgcctttcaccagcggcgcttccgggccgacgatggtcagatcaatcttttcgttttgtgcgaaatccaacagcgccgggatatcggtcacgccaatagcaacgttttgcagcgcgggttccagtgcagtgcctgcattacccggagcaacaaaaacagtctcaaccagcggcgactgggccgctttccaggccagcgcgtgctcgcgcccgccgttaccaatcactaatactttcatctattgctccattaatggcggaagtggcgcatgtcggtgaagagcatcgcaataccgtgctcgtcggcggcggcaatcacttcgtcatcacggatagaaccgccaggctggattacgcaggtcacgcccgcagcggcggcggcatcaataccgtcgcggaacgggaagaacgcgtcagaagccatcgaggaacctttcacttccaggccttcatcggccgctttaataccggcgatttttgcggagtacacgcggctcatctggcccgcgccaatgccgatagtcatattgtttttggcatagacgatagcgttggatttcacaaacttcgccaccttccagcagaacagcgcatcacgcagttcctgttcgctcggctgacgtttggtcaccacgcgcagttcttccgcaccgaccatccccaggtcacgatcctgaaccagcagaccgccgttcacgcgtttgaaatcgaggcccggaacacgctcgccccactgaccgcaggtcagaacgcgtacgttctgtttggcggcggtgattttcagggcttcttcgctggcggacggcgcaataatcacttcgacaaactgacgagaaatgatggcctgtgcggtttccgcatccagctcgcggttaaaggcaatgatgccgccgaatgcggaggttgggtcggttttgtacgcgcgatcgtaagcatcaagaatggaattgccgatagccacgccgcaagggttggcgtgcttcacaatcacacatgccggctcggcgaactctttcacgcactccagcgccgcatcggtatcggcgatgttgttataagagagggctttaccctgaacctgggttgcggtagcaacggaggcttctttcacattctcttctatatagaaggcagcctgctggtggctgttctcgccgtaacgcatatccagcttcttaatgaagttcaggttcagcgtgcgtgggaagcgaccggcggcttctttgctttcaccgtggtaagccggaaccatgctgccgaagtagttggcaatcatgctgtcgtaggcggcagtgtgttcgaaggctttgatggcgaggtcgaaacgggttgcaagcgtcagcgatccttcgttgtcatccatctctttaataatggcgtcatagtcgctgctcttcaccacgattgcgacatctttatggttcttggcggcggagcgcaccatcgttgggccgccgatatcgatgttctcaaccgcatcttccagcgagcaaccttcacgggccacggtctgggcgaacggatacaggttaacaaccaccatatcgataggctggatctgatgttcttccataatggcatcgtcctggccgcgacggcccagaatgccaccatgtactttcggatgcagggtcttcacgcgtccatccatcatctccgggaaaccggtgtaatcggaaacttcggttaccggcagacctttttctgctaacagacgggcagtgccccctgtagacagcagctccacaccgcgtgcggaaagtgcctgggcgaattcgacgataccggctttgtcagaaacactgagcagagcgcggcggactggacgacgttgttgcatggtaaatcccctggatttgactattacagagagcgttagctgaatttttcgcgaaaaactcagctaacgcccctaacggggcatccttatttttcgcccgcattgtaacgaaaacgtttgcgcaacgctcgcgaatttttctctttcaatggtgatcacaattttgactgtggttaccgtgggcaaaatacagaaattacattgatgattgtggataactctgtgcgtaaaaaggtataaagcgggcttttgctggggaatgcagcagtcagtcatttttctgcaatttttctattgcggcctgcggagaactccctataatgcgcctccatcgacacggcggatgtgaatcacttcacacaaacagccggttcggttgaagagaaaaatcctgaaattcagggttgactctgaaagaggaaagcgtaatatacgccacctcgcgacagtgcgctaaagcgcgtcgcaactgctctttaacaatttatcagacaatctgtgtgggcactcgaagatacggattcttaacgtcgcaagacgaaaaatgaataccaagtctcaagagtgaacacgtaattcattacgaagtttaattctttgagcatcaaacttttaaattgaagagtttgatcatggctcagattgaacgctggcggcaggcctaacacatgcaagtcgaacggtaacaggaagaagcttgcttctttgctgacgagtggcggacgggtgagtaatgtctgggaaactgcctgatggagggggataactactggaaacggtagctaataccgcataacgtcgcaagaccaaagagggggaccttcgggcctcttgccatcggatgtgcccagatgggattagctagtaggtggggtaacggctcacctaggcgacgatccctagctggtctgagaggatgaccagccacactggaactgagacacggtccagactcctacgggaggcagcagtggggaatattgcacaatgggcgcaagcctgatgcagccatgccgcgtgtatgaagaaggccttcgggttgtaaagtactttcagcggggaggaagggagtaaagttaatacctttgctcattgacgttacccgcagaagaagcaccggctaactccgtgccagcagccgcggtaatacggagggtgcaagcgttaatcggaattactgggcgtaaagcgcacgcaggcggtttgttaagtcagatgtgaaatccccgggctcaacctgggaactgcatctgatactggcaagcttgagtctcgtagaggggggtagaattccaggtgtagcggtgaaatgcgtagagatctggaggaataccggtggcgaaggcggccccctggacgaagactgacgctcaggtgcgaaagcgtggggagcaaacaggattagataccctggtagtccacgccgtaaacgatgtcgacttggaggttgtgcccttgaggcgtggcttccggagctaacgcgttaagtcgaccgcctggggagtacggccgcaaggttaaaactcaaatgaattgacgggggcccgcacaagcggtggagcatgtggtttaattcgatgcaacgcgaagaaccttacctggtcttgacatccacggaagttttcagagatgagaatgtgccttcgggaaccgtgagacaggtgctgcatggctgtcgtcagctcgtgttgtgaaatgttgggttaagtcccgcaacgagcgcaacccttatcctttgttgccagcggtccggccgggaactcaaaggagactgccagtgataaactggaggaaggtggggatgacgtcaagtcatcatggcccttacgaccagggctacacacgtgctacaatggcgcatacaaagagaagcgacctcgcgagagcaagcggacctcataaagtgcgtcgtagtccggattggagtctgcaactcgactccatgaagtcggaatcgctagtaatcgtggatcagaatgccacggtgaatacgttcccgggccttgtacacaccgcccgtcacaccatgggagtgggttgcaaaagaagtaggtagcttaaccttcgggagggcgcttaccactttgtgattcatgactggggtgaagtcgtaacaaggtaaccgtaggggaacctgcggttggatcacctccttaccttaaagaagcgttctttgcagtgctcacacagattgtctgatagaaagtgaaaagcaaggcgtcttgcgaagcagactgatacgtccccttcgtctagaggcccaggacaccgccctttcacggcggtaacaggggttcgaatcccctaggggacgccacttgctggtttgtgagtgaaagtcacctgccttaatatctcaaaactcatcttcgggtgatgtttgagatatttgctctttaaaaatctggatcaagctgaaaattgaaacactgaacaacgaaagttgttcgtgagtctctcaaattttcgcaacacgatgatgaatcgtaagaaacatcttcgggttgtgaggttaagcgactaagcgtacacggtggatgccctggcagtcagaggcgatgaaggacgtgctaatctgcgataagcgtcggtaaggtgatatgaaccgttataaccggcgatttccgaatggggaaacccagtgtgtttcgacacactatcattaactgaatccataggttaatgaggcgaaccgggggaactgaaacatctaagtaccccgaggaaaagaaatcaaccgagattcccccagtagcggcgagcgaacggggagcagcccagagcctgaatcagtgtgtgtgttagtggaagcgtctggaaaggcgcgcgatacagggtgacagccccgtacacaaaaatgcacatgctgtgagctcgatgagtagggcgggacacgtggtatcctgtctgaatatggggggaccatcctccaaggctaaatactcctgactgaccgatagtgaaccagtaccgtgagggaaaggcgaaaagaaccccggcgaggggagtgaaaaagaacctgaaaccgtgtacgtacaagcagtgggagcacgcttaggcgtgtgactgcgtaccttttgtataatgggtcagcgacttatattctgtagcaaggttaaccgaataggggagccgaagggaaaccgagtcttaactgggcgttaagttgcagggtatagacccgaaacccggtgatctagccatgggcaggttgaaggttgggtaacactaactggaggaccgaaccgactaatgttgaaaaattagcggatgacttgtggctgggggtgaaaggccaatcaaaccgggagatagctggttctccccgaaagctatttaggtagcgcctcgtgaattcatctccgggggtagagcactgtttcggcaagggggtcatcccgacttaccaacccgatgcaaactgcgaataccggagaatgttatcacgggagacacacggcgggtgctaacgtccgtcgtgaagagggaaacaacccagaccgccagctaaggtcccaaagtcatggttaagtgggaaacgatgtgggaaggcccagacagccaggatgttggcttagaagcagccatcatttaaagaaagcgtaatagctcactggtcgagtcggcctgcgcggaagatgtaacggggctaaaccatgcaccgaagctgcggcagcgacgcttatgcgttgttgggtaggggagcgttctgtaagcctgcgaaggtgtgctgtgaggcatgctggaggtatcagaagtgcgaatgctgacataagtaacgataaagcgggtgaaaagcccgctcgccggaagaccaagggttcctgtccaacgttaatcggggcagggtgagtcgacccctaaggcgaggccgaaaggcgtagtcgatgggaaacaggttaatattcctgtacttggtgttactgcgaaggggggacggagaaggctatgttggccgggcgacggttgtcccggtttaagcgtgtaggctggttttccaggcaaatccggaaaatcaaggctgaggcgtgatgacgaggcactacggtgctgaagcaacaaatgccctgcttccaggaaaagcctctaagcatcaggtaacatcaaatcgtaccccaaaccgacacaggtggtcaggtagagaataccaaggcgcttgagagaactcgggtgaaggaactaggcaaaatggtgccgtaacttcgggagaaggcacgctgatatgtaggtgaggtccctcgcggatggagctgaaatcagtcgaagataccagctggctgcaactgtttattaaaaacacagcactgtgcaaacacgaaagtggacgtatacggtgtgacgcctgcccggtgccggaaggttaattgatggggttagcgcaagcgaagctcttgatcgaagccccggtaaacggcggccgtaactataacggtcctaaggtagcgaaattccttgtcgggtaagttccgacctgcacgaatggcgtaatgatggccaggctgtctccacccgagactcagtgaaattgaactcgctgtgaagatgcagtgtacccgcggcaagacggaaagaccccgtgaacctttactatagcttgacactgaacattgagccttgatgtgtaggataggtgggaggctttgaagtgtggacgccagtctgcatggagccgaccttgaaataccaccctttaatgtttgatgttctaacgttgacccgtaatccgggttgcggacagtgtctggtgggtagtttgactggggcggtctcctcctaaagagtaacggaggagcacgaaggttggctaatcctggtcggacatcaggaggttagtgcaatggcataagccagcttgactgcgagcgtgacggcgcgagcaggtgcgaaagcaggtcatagtgatccggtggttctgaatggaagggccatcgctcaacggataaaaggtactccggggataacaggctgataccgcccaagagttcatatcgacggcggtgtttggcacctcgatgtcggctcatcacatcctggggctgaagtaggtcccaagggtatggctgttcgccatttaaagtggtacgcgagctgggtttagaacgtcgtgagacagttcggtccctatctgccgtgggcgctggagaactgaggggggctgctcctagtacgagaggaccggagtggacgcatcactggtgttcgggttgtcatgccaatggcactgcccggtagctaaatgcggaagagataagtgctgaaagcatctaagcacgaaacttgccccgagatgagttctccctgactccttgagagtcctgaaggaacgttgaagacgacgacgttgataggccgggtgtgtaagcgcagcgatgcgttgagctaaccggtactaatgaaccgtgaggcttaaccttacaacgccgaaggtgttttggcggattgagagaagattttcagcctgatacagattaaatcagaacgcagaagcggtctgataaaacagaatttgcctggcggcagtagcgcggtggtcccacctgaccccatgccgaactcagaagtgaaacgccgtagcgccgatggtagtgtggggtctccccatgcgagagtagggaactgccaggcatcaaattagaaaaaccccggtccataaggccggggttttttgcatatcaattatttgcatgatgaagggaatctcatgtcagttctgtatatccaaattcgtcgtaatcaaattactgttcgcgatcttgaaagcaaacgtgaagtgtcaggagacgctgccttcagtaaccagcgcctgttaatcgccaatttctttgttgcagaaaaagttctgcaagatcttgttctgcaactccacccacgttcaacctggcattcttttttgccagcaaaacgtatggatattgttgtgagcgcactggaaatgaatgagggcggtttgtcacaggttgaggaacgcattctccatgaagtggtcgctggggcaacgttaatgaaatatcgccagttccacatccatgcgcaatcagcggtactcagtgatagtgcggtcatggcaatgcttaagcagaaataatcgtgtcaccattggtgggtactaaacctgaagttcagcccaccgggatgagaaaaaatcgcctacgcccccacatacgccagattcagcaacggatacggtttccccaaatcgtccacctcagagcgtcccgtaaccttaaaacccaccttcttatagaacccaaccgcctgctcattttgctcattaacgttggttgtcagttccggtgccatcgagagcgcatgctccaccagcacccgacctacgccgcagccgcgcacatcaggatcgataaacagcgcatccatatgctgcccacttagcaacataaatccaaccggctgatcccgctcattaaccgcgacccacaacggcgcttccggcaggaaggaacgaactaggtcctccagctcggtccgatactctgctgatagaaaatcgtgagtggcatcgacagaacgacaccaaatcgcaacgagttcctccccttcctcatgccgtgagcggcgaatactaataaccattttctctccttttagtcattcttatattctaacgtagtcttttccttgaaactttctcaccttcaacatgcaggctcgacattggcaaattttctggttatcttcagctatctggatgtctaaacgtataagcgtatgtagtgaggtaatcaggttatgccgattcgtgtgccggacgagctacccgccgtcaatttcttgcgtgaagaaaacgtctttgtgatgacaacttctcgtgcgtctggtcaggaaattcgtccacttaaggttctgatccttaacctgatgccgaagaagattgaaactgaaaatcagtttctgcgcctgctttcaaactcacctttgcaggtcgatattcagctgttgcgcatcgattcccgtgaatcgcgcaacacgcccgcagagcatctgaacaacttctactgtaactttgaagatattcaggatcagaactttgacggtttgattgtaactggtgcgccgctgggcctggtggagtttaatgatgtcgcttactggccgcagatcaaacaggtgctggagtggtcgaaagatcacgtcacctcgacgctgtttgtctgctgggcggtacaggccgcgctcaatatcctctacggcattcctaagcaaactcgcaccgaaaaactctctggcgtttacgagcatcatattctccatcctcatgcgcttctgacgcgtggctttgatgattcattcctggcaccgcattcgcgctatgctgactttccggcagcgttgattcgtgattacaccgatctggaaattctggcagagacggaagaaggggatgcatatctgtttgccagtaaagataagcgcattgcctttgtgacgggccatcccgaatatgatgcgcaaacgctggcgcaggaatttttccgcgatgtggaagccggactagacccggatgtaccgtataactatttcccgcacaatgatccgcaaaatacaccgcgagcgagctggcgtagtcacggtaatttactgtttaccaactggctcaactattacgtctaccagatcacgccatacgatctacggcacatgaatccaacgctggattaatcttctgtgatagtcgatcgttaagcgattcagcaccttacctcaggcaccttcgggtgccttttttatttccgaaacgtacctcagcaggtgaataaattttattcatattgttatcaacaagttatcaagtatttttaattaaaatggaaattgtttttgattttgcattttaaatgagtagtcttagttgtgctgaacgaaaagagcacaacgatccttcgttcacagtggggaagttttcggatccatgacgaggagctgcacgatgactgaacaggcaacaacaaccgatgaactggctttcacaaggccgtatggcgagcaggagaagcaaattcttactgccgaagcggtagaatttctgactgagctggtgacgcattttacgccacaacgcaataaacttctggcagcgcgcattcagcagcagcaagatattgataacggaacgttgcctgattttatttcggaaacagcttccattcgcgatgctgattggaaaattcgcgggattcctgcggacttagaagaccgccgcgtagagataactggcccggtagagcgcaagatggtgatcaacgcgctcaacgccaatgtgaaagtctttatggccgatttcgaagattcactggcaccagactggaacaaagtgatcgacgggcaaattaacctgcgtgatgcggttaacggcaccatcagttacaccaatgaagcaggcaaaatttaccagctcaagcccaatccagcggttttgatttgtcgggtacgcggtctgcacttgccggaaaaacatgtcacctggcgtggtgaggcaatccccggcagcctgtttgattttgcgctctatttcttccacaactatcaggcactgttggcaaagggcagtggtccctatttctatctgccgaaaacccagtcctggcaggaagcggcctggtggagcgaagtcttcagctatgcagaagatcgctttaatctgccgcgcggcaccatcaaggcgacgttgctgattgaaacgctgcccgccgtgttccagatggatgaaatccttcacgcgctgcgtgaccatattgttggtctgaactgcggtcgttgggattacatcttcagctatatcaaaacgttgaaaaactatcccgatcgcgtcctgccagacagacaggcagtgacgatggataaaccattcctgaatgcttactcacgcctgttgattaaaacctgccataaacgcggtgcttttgcgatgggcggcatggcggcgtttattccgagcaaagatgaagagcacaataaccaggtgctcaacaaagtaaaagcggataaatcgctggaagccaataacggtcacgatggcacatggatcgctcacccaggccttgcggacacggcaatggcggtattcaacgacattctcggctcccgtaaaaatcagcttgaagtgatgcgcgaacaagacgcgccgattactgccgatcagctgctggcaccttgtgatggtgaacgcaccgaagaaggtatgcgcgccaacattcgcgtggctgtgcagtacatcgaagcgtggatctctggcaacggctgtgtgccgatttatggcctgatggaagatgcggcgacggctgaaatttcccgtacctcgatctggcagtggatccatcatcaaaaaacgttgagcaatggcaaaccggtgaccaaagccttgttccgccagatgctgggcgaagagatgaaagtcattgccagcgaactgggcgaagaacgtttctcccaggggcgttttgacgatgccgcacgcttgatggaacagatcaccacttccgatgagttaattgatttcctgaccctgccaggctaccgcctgttagcgtaaaccaccacataactatggagcatctgcacatgaaaacccgtacacaacaaattgaagaattacagaaagagtggactcaaccgcgttgggaaggcattactcgcccatacagtgcggaagatgtggtgaaattacgcggttcagtcaatcctgaatgcacgctggcgcaactgggcgcagcgaaaatgtggcgtctgctgcacggtgagtcgaaaaaaggctacatcaacagcctcggcgcactgactggcggtcaggcgctgcaacaggcgaaagcgggtattgaagcagtctatctgtcgggatggcaggtagcggcggacgctaacctggcggccagcatgtatccggatcagtcgctctatccggcaaactcggtgccagctgtggtggagcggatcaacaacaccttccgtcgtgccgatcagatccaatggtccgcgggcattgagccgggcgatccgcgctatgtcgattacttcctgccgatcgttgccgatgcggaagccggttttggcggtgtcctgaatgcctttgaactgatgaaagcgatgattgaagccggtgcagcggcagttcacttcgaagatcagctggcgtcagtgaagaaatgcggtcacatgggcggcaaagttttagtgccaactcaggaagctattcagaaactggtcgcggcgcgtctggcagctgacgtgacgggcgttccaaccctgctggttgcccgtaccgatgctgatgcggcggatctgatcacctccgattgcgacccgtatgacagcgaatttattaccggcgagcgtaccagtgaaggcttcttccgtactcatgcgggcattgagcaagcgatcagccgtggcctggcgtatgcgccatatgctgacctggtctggtgtgaaacctccacgccggatctggaactggcgcgtcgctttgcacaagctatccacgcgaaatatccgggcaaactgctggcttataactgctcgccgtcgttcaactggcagaaaaacctcgacgacaaaactattgccagcttccagcagcagctgtcggatatgggctacaagttccagttcatcaccctggcaggtatccacagcatgtggttcaacatgtttgacctggcaaacgcctatgcccagggcgagggtatgaagcactacgttgagaaagtgcagcagccggaatttgccgccgcgaaagatggctataccttcgtatctcaccagcaggaagtgggtacaggttacttcgataaagtgacgactattattcagggcggcacgtcttcagtcaccgcgctgaccggctccactgaagaatcgcagttctaagcaacaacaaccgttgctgactgtaggccggataaggcgttcacgccgcatccggcaatcggtgcacgatgcctgatgcgacgcttgcgcgtcttatcatgcctacagccgttgccgaacgtaggctggataaggcgtttacgccgcatccggcaattctctgctcctgatgagggcgctaaatgccgcgtggcctggaattattgattgctcaaaccattttgcaaggcttcgatgctcagtatggtcgattcctcgaagtgacctccggtgcgcagcagcgtttcgaacaggccgactggcatgctgtccagcaggcgatgaaaaaccgtatccatctttacgatcatcacgttggtctggtcgtggagcaactgcgctgcattactaacggccaaagtacggacgcggcatttttactacgtgttaaagagcattacacccggctgttgccggattacccgcgcttcgagattgcggagagcttttttaactccgtgtactgtcggttatttgaccaccgctcgcttactcccgagcggctttttatctttagctctcagccagagcgccgctttcgtaccattccccgcccgctggcgaaagactttcaccccgatcacggctgggaatctctactgatgcgcgttatcagcgacctaccgctgcgcctgcgctggcagaataaaagccgtgacatccattacattattcgccatctgacggaaacgctggggacagacaacctcgcggaaagtcatttacaggtggcgaacgaactgttttaccgcaataaagccgcctggctggtaggcaaactgatcacaccttccggcacattgccatttttgctgccgatccaccagacggacgacggcgagttatttattgatacctgcctgacgacgaccgccgaagcgagcattgtttttggctttgcgcgttcttattttatggtttatgcgccgctgcccgcagcgctggtcgagtggctacgggaaattctgccaggtaaaaccaccgctgaattgtatatggctatcggctgccagaagcacgccaaaaccgaaagctaccgcgaatatctcgtttatctacagggctgtaatgagcagttcattgaagcgccgggtattcgtggaatggtgatgttggtgtttacgctgccgggctttgatcgggtattcaaagtcatcaaagacaggttcgcgccgcagaaagagatgtctgccgctcacgttcgtgcctgctatcaactggtgaaagagcacgatcgcgtgggccgaatggcggacacccaggagtttgaaaactttgtgctggagaagcggcatatttccccggcattaatggaattactgcttcaggaagcagcggaaaaaatcaccgatctcggcgaacaaattgtgattcgccatctttatattgagcggcggatggtgccgctcaatatctggctggaacaagtggaaggtcagcagttgcgcgacgccattgaagaatacggtaacgctattcgccagcttgccgctgctaacattttccctggcgacatgctgtttaaaaacttcggtgtcacccgtcacgggcgtgtggttttttatgattacgatgaaatttgctacatgacggaagtgaatttccgcgacatcccgccgccgcgctatccggaagacgaacttgccagcgaaccgtggtacagcgtctcgccgggcgatgttttcccggaagagtttcgccactggctatgcgccgacccgcgtattggtccgctgtttgaagagatgcacgccgacctgttccgcgctgattactggcgcgcactacaaaaccgcatacgtgaagggcatgtggaagatgtttatgcgtatcggcgcaggcaaagatttagcgtacggtatggggagatgcttttttgagtaaagcttccatataatttttctccgcaatgtatcgagggttatccgtaaagccaaagctttcagccatcttatttaatgtattaaggattaattcagcaataacccggtgaccaaattcaaaagccaactcaaaggcagagtatttttgtggggctttgtgttgccaaaaatccataatatcttcagcggtaaatccaaacaggcgtgcatggtcagataaagcaagataaaccgtctctacaacattttgttgtttatgctgtatcgctgaaaacaaaccgggatattcattagaattatttgccaggaggaggggcttcatattttttttatcgaatttaaacgtattaaacagagtgggtaatgcgttaaaaatagtattaataacgttcatgtgtccgcgctgcatggccataaacaaacccgtgtcgcgcgcaagacttttagcggtcagaagatctacaatatcggaagctgaaatgttaatttcctgggctaggctgggcaatgcttcaagaataactttcacgatatcgctatgtccattttgcatcgccagatatagtcctgggcaaccataaaaatcctttgccttcaggagatcgagtacctgttctttagtcaaatgacatgtgcgaattaacaaaggtaacgcgttcaaaacaattttcagcatgtcggcatcaccattcgccataacatggtataaaacatggctggacgttctatttttggcactcaggaatttatacacttgttcgttatctaaatgatgtgttgcggccagtttaggtaaggcgttcagaatcgaggttacaacatttttatccttacgtgatatcgctaaaaataatccagaaaaaccatttttatcttttgcctccagaatatgcatgagattttttttcgagagtaatccttcatatcctgtttctgacaatgaattgaaaatagtctcaacgatatccgcattaccataatttatagccaaatataaacctggcaggttaatactattataggcagtcaacatttctgttctatgtagttctggcattttctggagttgaatcatcagttgcgtaagttggtgattctgaccaattgccattagcaaattcatcgttgcaggtgataatggaggggttatttcatccacagatccttttaacatcaatagctgttctttcggaagtgctggaattattgcaacagattgattaataacatgatcatttgaccatttcaggaggctataatctacattcataaaatccatcagagaatagtgtttaatattctctttgctttcgctcataattcttattttatcgttagttacattaggatcataaaccgaaaccacgtaatgggtacatccttcagttgtgttctttattcttagccggaccgtcaaagcatggttatccaccagtaatatggctgccataacactgatgccatttgattccatcttgtcaaaatatgctttcataactagcccgaaatcaccgcaggcagcaacgcaacgcccctcaggacggctggaaaccaacgccaaagtctggtttttgcattttttgttgaagtgcgtgagaaatttttcagctgaagagtaatcatcttgatggggtttgtaatcaacattctgataaatatcattaatatattgtgcagcaatgtgtcggcatactatacggttttggggtcgccccggaaaataacattgaccattaagtttaattcttgggaattctttttcttttctatctgattttaggtttaattcttgtttatcaagagtgtctgagcgttgaggtaaaatttccattaggtatttttcaaatattggggcaatggtttgagtaagtgtcgtgttttcgtttttattaattatcgtaatttctttcttatcagcttgtaagacggacgtggaaaatttaatgacaaaatccttgttgctaaagatatgacgaccattttgtctacagttctctgagaagctttttaatagaggcgtcgccagctccttgccagaaaatttatcctcgagttctttataaaacaattcactcagggtttggtgttcatttgtctgggctgtattattaatatttgcagagaaagaactacgaggaatacgagtaatcatttaaatatctcattgtttattgatgtcttgaattttaactatcagaacagtgaaaaaatttaatatgattacaactaaagaaatatcataaatcgctcaatctcataatgcagccgtaaaagtttcggtggaatgagatcttgcgattttgttaataattaagtggtttgatgtttaaaaataatgctgagttaataaaagtgtgtgaagtgtatgacattaagttattttggcgtcaatgcgattaacagacacccttattctattgccactcaggtatgatgggcagaatattgcctctgcccgccagaaaaagtcagcgcattccaccgtacgccagcgtcacttccttcgccgctttaatcaccatcgcgccaaactcggtcacgcggtcatcggtaatacgtgaaatcggtccggaaatagaaattgcggcaaacggttcacggtgctcatcgaaaatacacgctgcaaggcaacgtagccccagtgcatgttcctcatcgtcaaatgaataaccccgtttgcgcgtttgggcgagatcttcttttaaatgcacaggagacaccagcgttgcgtgggtataggcatgtaaccctttgcggtgcagcagcttcgtcacctgttcttcgctcagttgggctaaaaaggctttacccgcaccggaagcgtgcatcggcaatttaccgccgataggcgcggacattcgcatcagatgcgtacactgtacctggtcgataataatcgcttcgtgatcgctttgatcaagcaccgccatattgaccgtttcgccagactcttccattagattgcgcaggatagggtgaacaatcgctaacaaattacggctctggagaaagctgctgccgaccataaaggcatgtgcgccgattgcccaatgtcccagttcgccaacctgacgcacgaaaccctgctgttgcatcgtggttagcaggcggtgggtcgtggaattgggtaacccggcttgttgcgccagttccgtgagtgccacactgccattggattcggcaatccactccagtaatttcaggccacgcgttaaagactgaacctgtccagtcgctggtgcggtggcaacggcgggttttctgccgcgtttcgcgggaatgggtgcgaccatgacagtctcttttttctgtatcgtggaaatcattttcatttttattgttagctaatgcaatagttactgaactgatccgatgagttaatgttgaacaaatctcatgttgcgtggtggtcgcttttaccacagatgcgtttatgccagtatggtttgttgaatttttattaaatctgggttgagcgtgtcgggagcaagtgtgagcagcaaagtggaacaactgcgtgcgcagttaaatgaacgtattctggtgctggacggcggtatgggcaccatgatccagagttatcgactgaacgaagccgattttcgtggtgaacgctttgccgactggccatgcgacctcaaaggcaacaacgacctgctggtactcagtaaaccggaagtgatcgccgctatccacaacgcctactttgaagcgggcgcggatatcatcgaaaccaacaccttcaactccacgaccattgcgatggcggattaccagatggaatccctgtcggcggaaatcaactttgcggcggcgaaactggcgcgagcttgtgctgacgagtggaccgcgcgcacgccagagaaaccgcgctacgttgccggtgttctcggcccgaccaaccgcacggcgtctatttctccggacgtcaacgatccggcatttcgtaatatcacttttgacgggctggtggcggcttatcgagagtccaccaaagcgctggtggaaggtggcgcggatctgatcctgattgaaaccgttttcgacacccttaacgccaaagcggcggtatttgcggtgaaaacggagtttgaagcgctgggcgttgagctgccgattatgatctccggcaccatcaccgacgcctccgggcgcacgctctccgggcagaccaccgaagcattttacaactcattgcgccacgccgaagctctgacctttggcctgaactgtgcgctggggcccgatgaactgcgccagtacgtgcaggagctgtcacggattgcggaatgctacgtcaccgcgcacccgaacgccgggctacccaacgcctttggtgagtacgatctcgacgccgacacgatggcaaaacagatacgtgaatgggcgcaagcgggttttctcaatatcgtcggcggctgctgtggcaccacgccacaacatattgcagcgatgagtcgtgcagtagaaggattagcgccgcgcaaactgccggaaattcccgtagcctgccgtttgtccggcctggagccgctgaacattggcgaagatagcctgtttgtgaacgtgggtgaacgcaccaacgtcaccggttccgctaagttcaagcgcctgatcaaagaagagaaatacagcgaggcgctggatgtcgcgcgtcaacaggtggaaaacggcgcgcagattatcgatatcaacatggatgaagggatgctcgatgccgaagcggcgatggtgcgttttctcaatctgattgccggtgaaccggatatcgctcgcgtgccgattatgatcgactcctcaaaatgggacgtcattgaaaaaggtctgaagtgtatccagggcaaaggcattgttaactctatctcgatgaaagagggcgtcgatgcctttatccatcacgcgaaattgttgcgtcgctacggtgcggcagtggtggtaatggcctttgacgaacagggacaggccgatactcgcgcacggaaaatcgagatttgccgtcgggcgtacaaaatcctcaccgaagaggttggcttcccgccagaagatatcatcttcgacccaaacatcttcgcggtcgcaactggcattgaagagcacaacaactacgcgcaggactttatcggcgcgtgtgaagacatcaaacgcgaactgccgcacgcgctgatttccggcggcgtatctaacgtttctttctcgttccgtggcaacgatccggtgcgcgaagccattcacgcagtgttcctctactacgctattcgcaatggcatggatatggggatcgtcaacgccgggcaactggcgatttacgacgacctacccgctgaactgcgcgacgcggtggaagatgtgattcttaatcgtcgcgacgatggcaccgagcgtttactggagcttgccgagaaatatcgcggcagcaaaaccgacgacaccgccaacgcccagcaggcggagtggcgctcgtgggaagtgaataaacgtctggaatactcgctggtcaaaggcattaccgagtttatcgagcaggataccgaagaagcccgccagcaggctacgcgcccgattgaagtgattgaaggcccgttgatggacggcatgaatgtggtcggcgacctgtttggcgaagggaaaatgttcctgccacaggtggtcaaatcggcgcgcgtcatgaaacaggcggtggcctacctcgaaccgtttattgaagccagcaaagagcagggcaaaaccaacggcaagatggtgatcgccaccgtgaagggcgacgtccacgacatcggtaaaaatatcgttggtgtggtgctgcaatgtaacaactacgaaattgtcgatctcggcgttatggtgcctgcggaaaaaattctccgtaccgctaaagaagtgaatgctgatctgattggcctttcggggcttatcacgccgtcgctggacgagatggttaacgtggcgaaagagatggagcgtcagggcttcactattccgttactgattggcggcgcgacgacctcaaaagcgcacacggcggtgaaaatcgagcagaactacagcggcccgacggtgtatgtgcagaatgcctcgcgtaccgttggtgtggtggcggcgctgctttccgatacccagcgtgatgattttgtcgctcgtacccgcaaggagtacgaaaccgtacgtattcagcacgggcgcaagaaaccgcgcacaccaccggtcacgctggaagcggcgcgcgataacgatttcgcttttgactggcaggcttacacgccgccggtggcgcaccgtctcggcgtgcaggaagtcgaagccagcatcgaaacgctgcgtaattacatcgactggacaccgttctttatgacctggtcgctggccgggaagtatccgcgcattctggaagatgaagtggtgggcgttgaggcgcagcggctgtttaaagacgccaacgacatgctggataaattaagcgccgagaaaacgctgaatccgcgtggcgtggtgggcctgttcccggcaaaccgtgtgggcgatgacattgaaatctaccgtgacgaaacgcgtacccatgtgatcaacgtcagccaccatctgcgtcaacagaccgaaaaaacaggcttcgctaactactgtctcgctgacttcgttgcgccgaagctttctggtaaagcagattacatcggcgcatttgccgtgactggcgggctggaagaggacgcactggctgatgcctttgaagcgcagcacgatgattacaacaaaatcatggtgaaagcgcttgccgaccgtttagccgaagcctttgcggagtatctccatgagcgtgtgcgtaaagtctactggggctatgcgccgaacgagaacctcagcaacgaagagctgatccgcgaaaactaccagggcatccgtccggcaccgggctatccggcctgcccggaacatacggaaaaagccaccatctgggagctgctggaagtggaaaaacacactggcatgaaactcacagaatctttcgccatgtggcccggtgcatcggtttcgggttggtacttcagccacccggacagcaagtactacgctgtagcacaaattcagcgcgatcaggttgaagattatgcccgccgtaaaggtatgagcgttaccgaagttgagcgctggctggcaccgaatctggggtatgacgcggactgattcacaaatctgtcacttttccttacaacaaacagggcgctcaatgagtgccctgtctctttattaatatgaaacacttatactggaaacaggctggaataatcttagccggaaaaacgaatgtcaaaaggcacagtaaagatgccagtcagcgtgtttccggtcctttggtcattcaattgcttcaggaacatataacgataaggagaacctgaactcgtgttaacgctgcttcacctgctttctgccgtcgccctgctggtctgggggactcatattgttcgaaccggcgtaatgcgcgtcttcggcgcgcgtttgcgtactgtccttagccggagcgtcgaaaaaaagccgctcgccttttgcgcggggatcggcgttaccgcactggtacagagcagtaatgccaccaccatgctggtgacctcgtttgtcgctcaggatctggtagccctcgcaccggctctggtcattgtgctgggtgcagatgtcgggacggcgctaatggcgcgtattctcaccttcgacttatcctggctgtcaccgttacttatttttatcggcgtgatttttttcctcggacgcaaacagtcacgcgccgggcaactgggccgcgtcggtattggtcttgggctgattttgctagcgctggagttgattgtgcaggccgtaacgccgatcacccaggcaaacggcgttcaggtgatctttgcctcgctgaccggcgatattctgctggatgcgctgattggcgcgatgttcgccattatcagctactccagccttgctgctgtactgctgaccgcgactctgaccgccgcaggcattatctccttccccgtggcgctctgtctggtgattggtgctaacctcggttccggtctgctggcaatgctcaacaacagtgccgccaatgccgcagcccgccgtgtcgcgctgggtagtctgctgtttaagctggtgggtagcctgattatcctgccgtttgtccatttgctggcagagacaatggggaagttgtcattgccaaaagcggaactggtgatctatttccacgtcttctacaaccttgtacgttgcctggtcatgctgccatttgttgacccgatggcacggttttgcaaaacgattattcgcgatgaaccggaactggatacccagctacggcctaaacatctggatgtcagcgcgctggatacgcccacgcttgctctggcgaacgccgcgcgcgaaaccctgcgcattggcgacgccatggaacagatgatggaagggttgaataaagtgatgcacggtgagccacggcaggagaaagagctgcgtaagctggcagatgatatcaacgttctctacaccgccattaagctgtatctggcgcggatgccaaaagaagagctggcggaggaagagtcgcgccgctgggcagagatcatcgaaatgtcgctcaaccttgaacaggcctccgatatcgtcgagcgcatgggcagcgaaattgctgacaaatcactggcagcacggcgggcattttcgcttgatgggttgaaggaactggatgcgctctatgagcaattgctcagtaatttaaagctggcaatgtcggtgttcttctctggcgatgtcaccagcgctcgtcgtttgcgtcgcagcaaacatcgttttcgcattcttaatcgccgctattcccacgcccacgtcgatcgcctgcatcagcaaaacgtgcagagcattgaaaccagttcgctacatttaggcttactgggagatatgcagcgcctgaactcgctgttttgttcggtggcttacagtgtgctggaacagccggatgaagatgaaggacgggacgagtattaatattgtgaatcctgtaggcctgataagacgcgtcaagcgtcgcatcaggcactatgaacaagatgccggatcatgcatccggcaattcacttaaaaacggtgaccagcttccagcggaaccgcttcttcaccagccttaaacacataagtggtgttcgggccacccagcgtagcgtgacctttactcactgtgatccagttaccttccggtagaccaataatcgtcagttctggcgcgacgaccagcagttcgcgaatacgctgctcacgggtttcacctttatggccttccggcagcgcgttggtgaagtgcgggttgatttgcagcgggaacagatttagcgcatcgaaaccttgcggatcgacaatcggcatatcgttggtggtacgaatagttgggcaagcaaggttagcgcctgcgctccagccaatatacagagcgccacgtttaaccacgtcagtaattggtgccagcagcccgcgctcgcggcactgtttcagcaactggaaagtattcccgccgccgacaatcacgatctcagcattttcaatcgcggcaacgggatcgacaacgctatgaataccggtgacagaaacacccagcggagcgagaaccgcagccgttttcgctgtgtaatcatcccaggtctgcgttacgccagcgaaagggataaacaccgctgagcggcgaccctgcaactgttcagcaattagcggcagtgcatgttccagccaggctttacccggcagcgtcgagttactcaataaaagcagttccattacttctccggttagtaagaaatcacgggaggcatgctaccactgcgaatttaaccacttactgacatggctcacgatgtcgcacattgcttctggaaagtgatttgagcaggtaacgaattcaagccaatggaaataacaaatagttcgctcatgactattttttatcaacccaaaggtacggtatattccgttttttacaggagaatttatgctgcccgactcatcagtccgtttaaataaatacatcagcgaaagcggaatttgctcacgccgcgaagcggatcgctatatcgagcaaggcaatgtgttccttaatggcaagcgagccaccattggcgatcaggtgaaacccggcgacgttgtgaaagtaaacggtcagttgattgaacctcgggaagccgaagatttggtacttatcgccctgaacaagcccgttggtattgtaagcaccaccgaagatggcgagcgcgataacattgtcgatttcgttaaccacagcaaacgcgtgttcccgattggccgcctggataaagactcccaggggctgattttcctcaccaatcacggcgatctggtgaataagatcctgcgtgctggcaatgatcatgagaaagagtatctggtgacggtcgataaaccgattaccgaggagtttattcgcggcatgagtgcgggggtgccaatcctcgggacagtgaccaaaaagtgcaaagttaaaaaagaagcgccgtttgtcttccgcattaccctggtgcaggggctgaaccgtcagatccggcgcatgtgcgagcatttcggctatgaagtgaaaaagctggaacgcacgcgcatcatgaacgttagcttaagcggcattccgctgggggaatggcgcgatttaaccgacgatgagttaatcgacctctttaagctcattgaaaattcctcttccgaggtaaaacctaaagcgaaggccaaaccgaaaacagcgggcatcaaacgtccagtcgttaagatggaaaaaacggcggaaaaaggcggtcgcccggcgtccaacggtaagcgttttacctcgccggggcgtaaaaagaaggggcgctgattaacgcctcagactgatgaaaacggcccaaaagtgcccggacagtcccctcgccccttcgggaaaagggttagggtgaggggaaaattgtgttcacactgacgagtgaaaatctcaggcgttgattgtggattagcgcctgccgcgcgtcgacgtatttgctgaccagctaaatgacgcttcaggatccggtttataagcctgctttttcttcaactggcgggcttttttcgcttcagcctcacgctcaaccattaatttatcgatgtaatctttcttaatgctgttggtttcggagttggtcaatacgcgaccatgcgcaatccgcgcccgatccagcagtgttttaagttcacgctgctcgcgttcagtcatctctttttgggtaatacgggggagtgccatgatggtgccctcagtgagccagagagttcagtgtacgggaattcgtttgcgagcagaactgataatattcattttgccttctcttaactatttatctctttcgataattaattagagatgcagataaaaaaattaaaggcaattattctccgataaagacgctggttaacagagtacaggctcgtttattgatgagcatagtgacaagaaaatcaatacggcccgaaatatagcttccaggccatacagtatttactcaaacaaattactatgcagtttttgcaccacctgctcggcatcttcgccgggcaccaggaagcacaggttatggctggatgcgccataacaaatcatgcgaatgttgaacggttccagtacgccgaatacctctttgccaacgccgcaggcttttgacaggtcattgccaatcaacgcgaccagcgccagaccttcttccacctccacccgacacagtgcggaaagctccatcagcagagattgcgtcagcaacgtatcgccagtggaggttgaaccggtggtatcaagggttaatgccacgctcacttctgacgtggtgattaagtctaccgaaatattatgccgcgcgaggatgccgaaaacttccgcgaggaaaccgcgagaatgcagcatattcaggctgtgcaaagtgagcagagtctgattgcgacgaagcgccagagcgcggaacagcggcggattttcagttttattgcacaccagcgtaccacctgcgcgtgggtctttgctggagccgacaaagaccgggatatcgctgcgtactgcgggtagcaacgttgccggatgcagtacttttgcaccaaaagttgccatctctgccgcttcggcaaacgcgatttcatcaatgcgttttgctgcggaaactacgcgtggatcggtggtgtagatgcccgggacgtcggtccagatatcaacacgagatgcgtgtaaagcctccgccagcaaggctgccgtataatcgctgcctccacggccaagcgtcgttgtacgacctttattttcgctaccgataaatccctgggtgatcactaagccttcattgagacgtgggagcagctgcagcgcggccagttccgccagcgcggctatatctggctctgcacgaccaaatcggtcgttggtacgcatcactttacgtacatcaaaccactgtgcctgaacatcgcgttcgcgcaggatctcaacaaacagcagggtcgacatcagctcgccgtggctgaccagctcatctgtcagcgccggagacgttgccagcgccgccgcttctgccagaacagtaatgttctccagcagacgttcaatctcttcacggataacgttcgggtaacgcagacgttccagaatggcaaactggatgttgcggatagcgtcgagtttttcgaatcgctcgccaggttccagtccttcagctaaagcgaccagcagattagtgataccagcagaagccgagaggacaactaaacgcacgttggcatcagaaagcacaatatcagcgctgcggttcatggcgtcaaaatcagctacgctggtaccgccaaatttggagacaacaatttcagacataactacctcgtgtcaggggatccattttcagccttggcacaagggaagagcggaagacgggtgggcgcagagcgatacttcgctactattttcacccagaagtgctccaccacttgcgaaacgcccgactgcgaacgcttctggtgacaacccaggggattcagcccctgtagccgatgatgaacgtggccagccgttcaatcacctcggcgatgcaccccctcaggtgttatcacaggactggctcctccaacaccgttacttgggcaacgcgcctcttctggcctgcgctagcgcaggtagtacatttataaataaagggtgagcggggcggttgtcaacgatggggtcatgcggatttttcatccactcctggcggtcagtagttcagctaataaatgcttcactgcgctaagggtttacactcaacattacgctaacggcactaaaaccatcacatttttctgtgactggcgctacaatcttccaaagtcacaattctcaaaatcagaagagtattgctaatgaaaaacatcaatccaacgcagaccgctgcctggcaggcactacagaaacacttcgatgaaatgaaagacgttacgatcgccgatctttttgctaaagacggcgatcgtttttctaagttctccgcaaccttcgacgatcagatgctggtggattactccaaaaaccgcatcactgaagagacgctggcgaaattacaggatctggcgaaagagtgcgatctggcgggcgcgattaagtcgatgttctctggcgagaagatcaaccgcactgaaaaccgcgccgtgctgcacgtagcgctgcgtaaccgtagcaataccccgattttggttgatggcaaagacgtaatgccggaagtcaacgcggtgctggagaagatgaaaaccttctcagaagcgattatttccggtgagtggaaaggttataccggcaaagcaatcactgacgtagtgaacatcgggatcggcggttctgacctcggcccatacatggtgaccgaagctctgcgtccgtacaaaaaccacctgaacatgcactttgtttctaacgtcgatgggactcacatcgcggaagtgctgaaaaaagtaaacccggaaaccacgctgttcttggtagcatctaaaaccttcaccactcaggaaactatgaccaacgcccatagcgcgcgtgactggttcctgaaagcggcaggtgatgaaaaacacgttgcaaaacactttgcggcgctttccaccaatgccaaagccgttggcgagtttggtattgatactgccaacatgttcgagttctgggactgggttggcggccgttactctttgtggtcagcgattggcctgtcgattgttctctccatcggctttgataacttcgttgaactgctttccggcgcacacgcgatggacaagcatttctccaccacgcctgccgagaaaaacctgcctgtactgctggcgctgattggcatctggtacaacaatttctttggtgcggaaactgaagcgattctgccgtatgaccagtatatgcaccgtttcgcggcgtacttccagcagggcaatatggagtccaacggtaagtatgttgaccgtaacggtaacgttgtggattaccagactggcccgattatctggggtgaaccaggcactaacggtcagcacgcgttctaccagctgatccaccagggaaccaaaatggtaccgtgcgatttcatcgctccggctatcacccataacccgctctctgatcatcaccagaaactgctgtctaacttcttcgcccagaccgaagcgctggcgtttggtaaatcccgcgaagtggttgagcaggaatatcgtgatcagggtaaagatccggcaacgcttgactacgtggtgccgttcaaagtattcgaaggtaaccgcccgaccaactccatcctgctgcgtgaaatcactccgttcagcctgggtgcgttgattgcgctgtatgagcacaaaatctttactcagggcgtgatcctgaacatcttcaccttcgaccagtggggcgtggaactgggtaaacagctggcgaaccgtattctgccagagctgaaagatgataaagaaatcagcagccacgatagctcgaccaatggtctgattaaccgctataaagcgtggcgcggttaatcatcgtcgatatgtaggccggataaggcgttcacgccgcatccggcaaccgatgcctgatgcgacgcggtcgcgtcttatcaggcctacaggtcgatgccgatatgtacatcgtattcggcaattaatacatagcacgattgattaaataaccttaataacaatgccgacgttatgtcggcatttttttatcagataaatccccttgtctgtaatttaacggaaatcataccgtgaggttaatcctaaaatagatttttaatcgttgtttatttcggaaaatacgcagattaattgcttttgtttttattttaagtttatgatttttattgttatttaaatataagttgaaacttatatttgatattcattccaattatcctaaaacgccatcgctaattccccgcgccgtaattcgcatgctttagttgtgtatactcgatcccgcccgaaatgtttttgggtaaatctccattcattcaatgaagggaaattgttatgaaaaaagttctgtatggcatttttgccatatctgcgcttgcggcgacttctgcgtgggctgcacctgtacaggtgggcgaagcggcagggtcggcagcaacgtcggtttcggcggggagttcctccgcgaccagcgtcagcaccgtaagctcggcggtgggtgtcgcgcttgcggcaaccggtggcggtgatggttctaataccgggaccaccacaaccacgaccaccagtacccagtaataaagtatgtatccccaaaataattcgagtcattgcatctgtggctagaagtatgaagggattaaccataaccacactccggtgtggttattctgcccctctggagaagagtcgtgaagcgacctgcactcattcttatctgcctgttattacaggcctgttcagccacgactaaagagctgggcaattcactgtgggacagtctgttcggcacgccaggcgtacagctgacggatgatgatattcaaaatatgccctacgccagccagtacatgcagcttaatggcgggccgcagttatttgtggtgctggccttcgctgaagacggacaacaaaaatgggtcactcaggatcaggctactctcgttacccaacatggccgtctggtgaagactctgctcggcggcgacaacctgattgaagtgaataaccttgctgccgacccgctgattaaacccgcacaaatcgttgatggcgcaagctggacgcgcacgatgggctggaccgagtaccagcaggtacgctacgccaccgcacgctcagtcttcaaatgggatggcaccgataccgtcaaagtcggcagcgatgaaaccccggttcgcgtgctggacgaagaagtctccaccgaccaggcgcgctggcataaccgctattggatcgacagcgaagggcaaattcgccagtcggaacagtatctcggcgcggattattttccggtgaaaaccactctcatcaaggcggcaaaacaatgattaaacaaactattgtcgcgttgcttttgagtgtgggagcgtcatcggtcttcgcggcaggaaccgtcaaggtgttcagcaatggcagcagtgaggccaaaacgctaacgggcgcagagcatttaatcgatctggtaggccaaccgcggctggcaaacagctggtggcccggtgcggtgattagcgaagagctggcaacggcggcagcattgcgtcagcagcaggcgttgctgacacggctggcagaacagggcgcagattccagcgccgacgatgccgctgcgattaacgccttacgccagcaaattcaggcgttgaaagtgacgggcaggcaaaaaatcaatcttgatcccgatatcgtccgcgttgccgaacgcggtaacccgccgttgcagggcaactacacgctgtgggtcggaccaccgccgtccacggtcacgttgttcgggcttatcagccgtcctggcaagcagccattcactccaggtcgcgacgtggcgagctatctctctgaccagagcctgctcagcggtgcggatcgcagctacgcgtgggtggtttacccggacggacgcacgcaaaaagcgccggtggcttactggaacaagcgtcacgtagagccgatgcccggcagcattatttatgttggcctcgcggactccgtctggagtgagacgcctgatgcccttaacgccgacattcttcagactctgacgcagcggatacctcaataatgaaaaaaagacatctgcttagcttactggcgctgggcattagcacagcttgctacggcgaaacatatcctgcgcccattggtccgtcgcagtcggatttcggtggcgtaggattattacaaacgcccaccgcgcgtatggcacgggaaggggagttgagtctgaactatcgcgataacgatcagtaccgttattactcagcttcagtgcaactcttcccgtggctggaaacaacgctgcgctacaccgacgtgcgcacccggcagtacagcagcgtcgaagcgttctctggcgatcaaacgtataaagataaagccttcgatctcaaactgcgtttgtgggaagagagttactggctgccgcaagtggcggttggtgcgcgggatatcggcggtacggggctgtttgatgcggaatatcttgttgccagcaaagcctgggggccgttcgattttacgctcggcctgggctgggggtatttgggcaccagcggtaatgtgaaaaatccgctctgttcagccagtgataaatattgctatcgcgataacagctacaaacaggcgggatctatcgacggtagccagatgttccacggtcctgcctcactgtttggcggcgtggaataccagacgccctggcaaccgctgcgcctgaaactggagtatgaaggcaataattatcagcaggattttgccgggaagctggagcaaaaaagtaagtttaacgtcggtgcgatttatcgcgttaccgattgggccgacgttaaccttagctatgaacgtggcaacacctttatgtttggcgttacgttgcgcaccaactttaacgatctgcgcccgtcttacaacgataacgcccgcccgcaatatcaaccgcagccgcaggatgccattttgcagcattcggtggtggcgaatcagttaacgctgttgaaatacaatgccggacttgccgatccacagatccaggcgaaaggcgatacgctgtatgttaccggcgagcaggtgaaatatcgtgattcgcgcgaagggatcatccgtgcgaatcggatcgtgatgaacgatctgccggatgggatcaaaacgatccgcattacggaaaatcgccttaacatgccgcaggtgacgacggaaaccgatgtcgccagcctgaaaaatcatctcgccggagagccgttgggccacgaaacgacgctggcgcaaaaacgcgtcgagccagtggttccgcagtccaccgagcagggctggtatatcgacaaatcacgctttgatttccatatcgatccggtgctgaaccagtcggtcggtggcccggaaaacttttacatgtatcagctgggcgtgatgggaacggcagatttgtggctgacggaccatctgctgaccaccggcagcctgtttgcaaatcttgccaacaactacgacaagtttaactacactaatcctccgcaggactcgcacttaccgcgcgtgcgtacccatgtgcgcgagtatgtgcagaacgatgtctatgtgaataacctgcaagccaactacttccagcatctgggcaacggcttctacggtcaggtctacggtggttatctcgaaaccatgtttggcggtgcgggggcagaagtgttgtatcgcccgctggacagcaactgggcgtttggtctggatgccaactacgttaaacagcgcgactggcgtagtgcaaaagatatgatgaaattcaccgactacagcgtgaaaaccggacatctgaccgcctactggacgccatctttcgctcaggatgtgttagttaaagccagcgtcgggcagtatctggcaggggataaaggcggcacgctggagatcgccaaacgctttgatagcggcgtggtggtgggtggctatgccacgatcactaatgtttcgaaagaggagtacggcgaaggggacttcaccaaaggcgtgtatgtctcggtaccgttggatctcttctcgtctggcccgacacgcagccgtgcggcgattggctggacgccgctgacgcgtgacggtggtcagcaacttgggcgtaagttccagttgtatgacatgaccagcgaccgtagcgtcaatttccgctaagtcatgggaaaggtgccagttttcgcactcactggcaccttcattcttaatggcctgtcgagccatcaggaacgcagttcactcccggtttgcgatctggtgtgtaaaggcgaaaacattctgtcttcctgtccgtcgatatcggttgcaggtctggttgcctgagcgactgggccatcattgggctggagacattgctttgcggtaggtcggctttatcagcagtaccgagcggaccagcataagcaggaagaacagagactgataacatcaaagcagcaaaataaggcttcatttttaccacctttatcaggttacgtttcatttgttccagaggaacattgtcgatttttcgcgcattgctggtggctgggaatcacctgaatgggtgatttttgaattaccggctttggtgcggtttgtcttgccggatgcgccgccaggcgcggcttatccggcctacgggtaggtatatccggctttggtggaggcgcgctccaaatccaggttgaacaaaacatacacaaaaaatatagatctccgtcacatttttgcgttatacaggaagctcgccactgtgaaggaggtactgctatgacgtcactctctcgtccgcgcgtggagtttatctccaccattttgcagaccgtactcaatcttggcctgctgtgcctcggcctgattttggttgtcttcctcggcaaagaaacggtgcatctggctgatgtgctgttcgcgccagaacaaaccagcaaatatgagctggtagaaggactggtggtttactttctctatttcgaatttatcgcgctgattgtgaagtactttcagtccggttttcacttcccgctacgttactttgtctatattgggatcaccgccattgtgcgcttgatcatcgtcgatcataaatcgccactggatgtgttgatctactcggctgcgatcctgttactggtgatcaccctgtggctgtgtaattcgaaacggctgaagcgggagtaaaaagtcagcacgccgaaatggcgcggcgtgctggacaggaagattacagcgtagcagtttgttgtgttttcttcgtttccggttcccagagcgcttccagctcctcaagggttttacctttggtttccgggacaaatttccacataaacagtgctgccagaacgcccatacaaccgtaaatccagtaggagaaaccgttgtggaaatgggccaccagccaggagtttttgtccatcatcgggaaggtccaggagacgaagtagttcgccagccactgggccgccaccgcgattgccagcgctttaccacgaatagcattcgggaagatttccgacagcagtacccagcataccggaccccaggacatggcaaaggcggcaacatagaacagcatcgacagtagcgccacaatacccggtgcctgagtgtaaaacgcggtaccgaggctaaacataccgattgccattccgagtgcgccgataatttgcagtggcttacgaccaaatttatccaccgtcataattgccagaacggtgaaggtgaggttgataactccgacaataatggtctgcaacagcgcgatatccgtgctggcccccagcgttttgaacacttccggcgcgtagtacagcaccacattgatgccgacaaattgctggaagatggagagcattacgccgattacaatcacgcccacgccaaacatcagcagacgaccaccggttttgcggccatgatccagggagtgtttaatttcctgtactgcctgagttgcaagcgtgttgcccataattttgcgcaggataccttccgcctgttcttgcttgccgcgcgacatcagccagcgaggactttctggcacggtatacagcagcattaagaacagcagtgcagggatacattccgaggcaaacatataacgccagccgtcagtattcagccagctggcatcaccggaacgggcaataaaatagtttacgcagtaaactaaaagttgcccgaaaataatcgcaaactggttaaaagagaccagtttcccgcgaatatgagctggagccagttccgcaatatacattggcgagagcattgaggctaaaccaacgccaataccgccaataatgcgataaataacaaattccgggacataacctgccagataaacaggcacagtgttgtccgggtttatagaggtaaaaccaagttctggccaggcagaacctacaccagaaataaaaaacaggacagcagcaatcttaagtgaatcacgacgaccgaagcggttactgcaataaccaccgagggcaccgccgatgatgcaaccaatcagagcgctggccacgcaaaaccctaacagggagttggcagcggattcacttaagttttgtggagcaacaaagacggtattgagtgactcaacagtaccggaaataacggcggtgtcgtagccaaataataaaccacctaatgtagcgactaaggtaatcgaaaatatataactggaattatactgggtattcattcagacctgccttagaccattctgatcttttatcagtgcattgatgttggaattgtcaggcagttaaggcaattatcattttttacaatgcgtttacgtaatgtcttttctgtgatcttaattgtgataattatccaaaattgataaaaacaatactattgccgtgactcagagcacgaaagagaattatcgtaagtgggaaaacaaataacgtaaaaataataagctctatgatggaaatattaaccggcgaacgattcagattgcagacgaaagaaaaaaaggcgctccgtggagcgccgaataacagtcacaagttgggataacgtaagttgagggtgcagcggcataacattggcagaacaacatctttaacctttcacaccacctgccgtcaggccgttgaccagccagcgttgagccagcaagaagacgatggtgatcggtaatgcagacatcacggcagcggcggcaaagtcaccccacaggtagttttgcgggttgaggtattgctgcatccccacggccagggtgtagctgtttacgtcacgcagtaacagcgacgcgaccggaacttcagtaatggcagcgataaacgacaggatgaataccaccgccagaatcggtactgacagcggcaacaggacaaggcggaaggcctgccacggtgtcgcaccatccagcgcagcagcttcttccagcgaactgtcgatggtttcgaaatagcctttgatggtccagacatgcagcgcaatcccacccagatacgcgaaaattacgccgccgtgagtattcaggccaatgaatggaatgtactcacccagacgatcaaacaacgcatacaacgcgaccagtgaaagtactgccgggaacatctggaaaatcagcattcctttcagcagcgtcgctttgcctggaaagcgcatacgggcgaaagcgtaggcgcaggtggtggagagcgccacaatgccaatcgcggaaatcccggcgacctttaccgagttccacagccacagcagtaccgggaatggcggtggcgtaatgcgaccatcagcctgttcaacgctaaaacctaacgccagtttccagtgatcccaggagatttgctccgggatcaggctgccggtcgcaaagtttccctgacgcagcgagatagcgacgaccatcagcagcgggaacataatcgctgcgataaaaagtagcagtagcaggtgagtaataaataaacgagctttttgcgatttcggttggaccattgccatttttgttatctcccttaatcaaacttcattcgcgtggctttcaggttcactatcgccagcgcacccaccagcaggaagatcagcgtggcaattgctgccgccagaccgaagtcctgacccccgccgccttcaaaagcgatgcggtaggtgtagttaacaagcaggtcggtataaccggctggcgtggtcgtgccaagacgatccgggccgccgttggttaacagttgaatcagcacgaagttgttaaagttaaaggcgaagctggcgatcatcagcggcgtcagcggtttaatcagcagcggcagcgtaatcttaaagaagttctggaacggacctgcgccatccattgctgaggcttcatacaaatcgtccggaatcgctttcagcaagcccatgcagaggatcatcatgtacggataacccagccaggtattgacgataattagcatcgtgcgggcggtggtcggatcgctgaaccaggcgggcttcacgccaaacagcgcgctcaacatcatgttgatttcaccgaagctctggttaaacaaccctttgaaaatcaagattgaaatgaacgatggcaccgcgtagggcagaatcagcaggacgcgatagaccgctttgccgcgcaacgcttcccactgcaccagacacgccagaaccatgccgaccgccaccgttaaaaagacagtgatcagcgagaacaccacggtccagacgaaaatggcgaggaacggtttctgaatgccttcgtcggtaaagacgcgggtaaagtttttccagccggtggtcacggtgtaaccggggcttagcttttcatcaccccagttgccgtcggcggtaatggactggtaaaagccaatttggttattcggacgatatttcacgccgctctgattattcgtcaacgtgccgtcaccgtcgagtgtgtagagcggctgcgtgccagaaaactggcgcagggagctcatcatcactttgttgccatccggcagaatggcggtaatgtcactcagcgcctgacgattctgggtaatcacgcgcagattcgcgcgttcgccttcgggctgggcggtcgtttctttcagttgcagtttttgctcgccgccaaatttaaaagcgtcggagaggtaatttttgccggtttcgccgtcgctgagcgccagttgccactcatcgcccgccgggtaaagaccaaagttataggttttgcctgcttgccaggagcgatctaacaacacttcctgcgcacgttcaaaagtcagctggttagtgctgctgtagttggtgaaggcaatggcgatggtgcagaccagagggaagaggacgaataatcccattccagccattcccgggtaaacatagcgccaggcgtaggctttacgattggcgaaaatatacagccccgctgaactcaatatcagcgtggtaatggcgaacaggtattccccttgtgcgtacattaaaacaacaaggtaacccaccagcaggccgagcagacctagcactgaccatttcagcgcgtcgctttgccaccaatgtttctttttaatgacatccatggggttcttcctcattccaggacggataaggctttcacgccttatccgacaacaactgcctgatgcgacgctgacgcgtcttatcaggcctacatacgtttcggttttgtaggccggacaaggcgttcacgccgcatccggcatttcacagcattacttggtgatacgagtctgcgcgtctttcagggcttcatcgacagtctgacgaccgctggcggcgttgatcaccgcagtacgcacggcataccagaaagcggacatctgcgggatgttcggcatgatttcacctttctgggcgttttccatggtggcggcaatacgtggatctttcgccaactcttcctcgtaagacttcagcgctacggcacccagcggtttgtctttattaaccgcttccagaccttcatcagtcagcagatagttttcgaggaactctttcgccagctctttgttcggactggcggcgttaatacctgcgctcagcacgccaacgaacggtttggatggttgacccttgaaggtcggcagtaccgttacaccataattcactttgctggtgtcgatgttggaccatgcccacgggccgttgatggtcatcgctgtttcgcctttattaaaggcagcttctgcgatggagtaatcggtgtctgcattcatgtgtttgtttttaatcaggtcaaccaggaaggtcagacccgctttcgcgccagcgttatccacgcccacgtctttaatgtcgtacttgccgttttcatacttgaacgcataacccccgtcagcagcaatcagcggccaggtgaagtacggttcttgcaggttgaacatcagcgcgctcttacctttcgctttcagttctttatccagcgccgggatctcttcccaggtttttggcgggttcggcagcagatctttgttataaatcagcgataacgcttcaacagcgatcgggtaagcaatcagcttgccgttgtaacgtacggcatcccaggtaaacggatacagcttgtcctggaacgctttgtccggggtgatttcagccaacaggccagattgagcgtagccaccaaagcggtcgtgtgcccagaagataatgtcagggccatcgccagttgccgcaacctgtgggaatttctcttccagtttatccggatgctcaacggtgactttaattccggtatctttctcgaatttcttaccgacttcagcgagaccgttatagcctttatcgccgttaatccagattaccagtttaccttcttcgattttggcgagagccgaggcggaaaacatcatcgtcgttaatgcggataatgcgaggatgcgtgcacctgtttttattttcataatctatggtccttgttggtgaagtgctcgtgaaaacacctaaacggactctagtttctttatacggcaacctctttccatcctccttgcccctacgccccaccgtcgctttgtgtgatctctgttacagaattggcggtaatgtggagatgcgcacataaaatcgccacgatttttgcaagcaacatcacgaaattccttacatgacctcggtttagttcacagaagccgtgttctcatcctcccgcctcctcccccataaaaaagccagggggtggaggatttaagccatctcctgatgacgcatagtcagcccatcatgaatgttgctgtcgatgacaggttgttacaaagggagaagggcatggcgagcgtacagctgcaaaatgtaacgaaagcctggggcgaggtcgtggtatcgaaagatatcaatctcgatatccatgaaggtgaattcgtggtgtttgtcggaccgtctggctgcggtaaatcgactttactgcgcatgattgccgggcttgagacgatcaccagcggcgacctgttcatcggtgagaaacggatgaatgacactccgccagcagaacgcggcgttggtatggtgtttcagtcttacgcgctctatccccacctgtcagtagcagaaaacatgtcatttggcctgaaactggctggcgcaaaaaaagaggtgattaaccaacgcgttaaccaggtggcggaagtgctacaactggcgcatttgctggatcgcaaaccgaaagcgctctccggtggtcagcgtcagcgtgtggcgattggccgtacgctggtggccgagccaagcgtatttttgctcgatgaaccgctctccaacctcgatgctgcactgcgtgtgcaaatgcgtatcgaaatctcccgtctgcataaacgcctgggccgcacaatgatttacgtcacccacgatcaggtcgaagcgatgacgctggccgacaaaatcgtggtgctggacgccggtcgcgtggcgcaggttgggaaaccgctggagctgtaccactatccggcagaccgttttgtcgccggatttatcggttcgccaaagatgaacttcctgccggtaaaagtgaccgccaccgcaatcgatcaagtgcaggtggagctgccgatgccaaatcgtcagcaagtctggctgccagttgaaagccgtgatgtccaggttggagccaatatgtcgctgggtattcgcccggaacatctactgccgagtgatatcgctgacgtcatccttgagggtgaagttcaggtcgtcgagcaactcggcaacgaaactcaaatccatatccagatcccttccattcgtcaaaacctggtgtaccgccagaacgacgtggtgttggtagaagaaggtgccacattcgctatcggcctgccgccagagcgttgccatctgttccgtgaggatggcactgcatgtcgtcgactgcataaggagccgggcgtttaagcaccccacaaaacacacaaagcctgtcacaggtgatgtgaaaaaagaaaagcaatgactcaggagatagaatgatgattactctgcgcaaacttcctctggcggttgccgtcgcagcgggcgtaatgtctgctcaggcaatggctgttgatttccacggctatgcacgttccggtattggttggacaggtagcggcggtgaacaacagtgtttccagactaccggtgctcaaagtaaataccgtcttggcaacgaatgtgaaacttatgctgaattaaaattgggtcaggaagtgtggaaagagggcgataagagcttctatttcgacactaacgtggcctattccgtcgcacaacagaatgactgggaagctaccgatccggccttccgtgaagcaaacgtgcagggtaaaaacctgatcgaatggctgccaggctccaccatctgggcaggtaagcgcttctaccaacgtcatgacgttcatatgatcgacttctactactgggatatttctggtcctggtgccggtctggaaaacatcgatgttggcttcggtaaactctctctggcagcaacccgctcctctgaagctggtggttcttcctctttcgccagcaacaatatttatgactataccaacgaaaccgcgaacgacgttttcgatgtgcgtttagcgcagatggaaatcaacccgggcggcacattagaactgggtgtcgactacggtcgtgccaacttgcgtgataactatcgtctggttgatggcgcatcgaaagacggctggttattcactgctgaacatactcagagtgtcctgaagggctttaacaagtttgttgttcagtacgctactgactcgatgacctcgcagggtaaagggctgtcgcagggttctggcgttgcatttgataacgaaaaatttgcctacaatatcaacaacaacggtcacatgctgcgtatcctcgaccacggtgcgatctccatgggcgacaactgggacatgatgtacgtgggtatgtaccaggatatcaactgggataacgacaacggcaccaagtggtggaccgtcggtattcgcccgatgtacaagtggacgccaatcatgagcaccgtgatggaaatcggctacgacaacgtcgaatcccagcgcaccggcgacaagaacaatcagtacaaaattaccctcgcacaacaatggcaggctggcgacagcatctggtcacgcccggctattcgtgtcttcgcaacctacgccaagtgggatgagaaatggggttacgactacaccggtaacgctgataacaacgcgaacttcggcaaagccgttcctgctgatttcaacggcggcagcttcggtcgtggcgacagcgacgagtggaccttcggtgcccagatggaaatctggtggtaatagcaaaacctgggccggataaggcgtttacgccgcattcggcaaccaacgcctgatgcgacgcttgcgcgtcttatcaggcctacaacggctgtcaaatgtaggccggataaggcgtttacgccgcatccggcataaaaacaggttgtcattatctgaaaggggcgaaagcccctctgattatcgggtttagcgcgctattgcctggctaccgctgagctccagattttgaggtgaaaacaatgaaaatgaataaaagtctcatcgtcctctgtttatcagcagggttactggcaagcgcgcctggaattagccttgccgatgttaactacgtaccgcaaaacaccagcgacgcgccagccattccatctgctgcgctgcaacaactcacctggacaccggtcgatcaatctaaaacccagaccacccaactggcgaccggcggccaacaactgaacgttcccggcatcagtggtccggttgctgcgtacagcgtcccggcaaacattggcgaactgaccctgacgctgaccagcgaagtgaacaaacaaaccagcgtttttgcgccgaacgtgctgattcttgatcagaacatgaccccatcagccttcttccccagcagttatttcacctaccaggaaccaggcgtgatgagtgcagatcggctggaaggcgttatgcgcctgacaccggcgttggggcagcaaaaactttatgttctggtctttaccacggaaaaagatctccagcagacgacccaactgctcgacccggctaaagcctatgccaagggcgtcggtaactcgatcccggatatccccgatccggttgctcgtcataccaccgatggcttactgaaactgaaagtgaaaacgaactccagctccagcgtgttggtaggacctttatttggttcttccgctccagctccggttacggtaggtaacacggcggcaccagctgtggctgcacccgctccggcaccggtgaagaaaagcgagccgatgctcaacgacacggaaagttattttaataccgcgatcaaaaacgctgtcgcgaaaggtgatgttgataaggcgttaaaactgcttgatgaagctgaacgcctgggatcgacatctgcccgttccacctttatcagcagtgtaaaaggcaaggggtaattacgccccacagtgctgattttgcaacaactggtgcgtctcctggcgcacctttttttatgcttccttcctgggatatgagcgattttttatagtaactcacttcttcttcactaagaatatccattatctcaatgccttatcagagattcttttcctttcgccggtagtgtctggacattcaggctacttttccaggttattttatttctgttatgcagaggttttatgataagtcatatcctaaattctggcggcaataactctttgatgaaacatgatgtggtgcaaggaaataatatagtagatcttgatttactacgtaatttaaatggggtgccaggtttaaacagagataactttatttatatcagcaatattttttcaaatataaaacaacggaacgaaaaaatcatgcaataaatatgtttcgtgaagtctcaatcagtaatgatactataagtgtaaaattctacagaaatgaaaaaaattgaatgcgcttgcaattttctgatggataaagatgcgcaggggtatatcgacctgtctgatttggatttaacaagttgtcattttaaaggtgacgttatatcgaaggtgtcttttttatcatcaaatctacaacatgtaacattcgaatgtaaagaaattggggattgcaattttactactgcaatagttgataatgtcatatttagatgtcgacgtttacacaatgtgatttttatcaaagcgagtggtgaatgtgtcgatttcagcaaaaatattcttgatacagttgacttctcgcagagtcaacttggtcatagtaattttcgcgaatgtcagattagaaattcaaacttcgataattgttatctttacgcttcgcacttcaccagagcagagtttctgtctgccaaagaaatatcatttattaaatcgaatttgacagctgttatgtttgattatgtgcgaatgtcgacagggaattttaaagattgcattacagaacaattggaattaactattgattattcagatatattttggaatgaagatctcgatggttatatcaataacattataaaaatgattgatacattgccagataatgcaatgatattgaaatccgttctggccgtaaaactggtgatgcaattaaaaatacttaatattgttaataaaaactttattgagaatatgaagaaaatatttagccattgtccttatataaaagatcccattatacgcagttatatccattctgatgaagataacaagttcgatgattttatgcgtcaacatcgattcagtgaggtgaatttcgatacccaacagatgatcgattttattaacagatttaatacgaataaatggctaattgataaaaataacaatttttttatccaacttatcgatcaggccttacgatcaacggatgatatgatcaaagcaaatgtttggcatctttataaagagtggattcgtagtgatgatgtttcacctatatttatagaaactgaagataatttaagaacctttaacacgaatgaattaacacgaaacgataatatctttatcctgttctcctcagtcgatgatgggccagttatggtggtaagctcccagcgcttacatgatatgttgaatcctacaaaagataccaattggaattccacgtatatctacaaatccagacatgagatgttgcctgttaatcttactcaggaaacacttttcagctccaaatctcatggtaaatatgcgcttttccccatttttactgcgagttggcgagctcatcgtataatgaataagggtgtttaagtaaaggaaaacatcaccgttcctggcatcctggacggtgatgcccctacggttgccctcgccagcacgggcatcggtaaagcgtaaggttcaacatcgttttaccacttcatgcgattgttgcgtttttgttgcgtattagatcacttaatttgctttacatctcccgtaaacacttttctgcgatacaatgcctttacgttatgtaacggagagttcggcatgtcacaccccgcgttaacgcaactgcgtgcgctgcgctattgtaaagagatccctgccctggatccgcaactgctcgactggctgttgctggaggattccatgacaaaacgttttgaacagcagggaaaaacggtaagcgtgacgatgatccgcgaagggtttgtcgagcagaatgaaatccccgaagaactgccgctgctgccgaaagagtctcgttactggttacgtgaaattttgttatgtgccgatggtgaaccgtggcttgccggtcgtaccgtcgttcctgtgtcaacgttaagcgggccggagctggcgttacaaaaattgggtaaaacgccgttaggacgctatctgttcacatcatcgacattaacccgggactttattgagataggccgtgatgccgggctgtgggggcgacgttcccgcctgcgattaagcggtaaaccgctgttgctaacagaactgtttttaccggcgtcaccgttgtactaagaggaaaaaaatatggagtggagtctgacgcagaataagctgctggcgtttcatcgcttaatgcgtacggataagccaattggcgcgttactgctgctctggccaacattatgggcgttgtgggtggcgacaccgggcgttccccagctctggatcctggcggtgtttgtcgcgggtgtctggctgatgcgcgctgccggatgtgtggtgaatgattatgctgaccgcaagtttgatggtcatgttaagcgcacggcgaaccgaccacttcccagcggcgcggtaacagagaaagaggcgcgcgcgctgtttgtcgtgctggtactgatttcgtttttactggtgctgacgctgaatacgatgaccattctgttgtcgattgccgcgctagcgctggcgtgggtgtacccgtttatgaagcggtatacccatctaccgcaagtggtgctgggcgcggcgtttggctggtcgattccaatggcttttgccgctgtgagtgagtcggtgccattgagttgctggttaatgttcctcgccaatattctctgggcggtggcttacgacacgcagtatgcgatggttgaccgcgatgatgatgtgaagattggcattaaatccacggcaatcctgttcggccaatacgataaattgattattggtattttgcagattggcgtactggcactgatggcgatcatcggtgagttaaatggcttaggctggggatattactggtcaattctggtggctggcgcgctgtttgtttatcaacaaaaactgattgccaaccgcgagcgtgaagcctgctttaaagcatttatgaataataactatgttggtctggtactatttttagggctggcaatgagttactggcatttctgatgatgtaaaaaagccggatgatcatccggctttcttctgggttgcctgatgcgcggcgcttctcaggcctacacaacacatcgcaatttattgaatttgcagattatggaaggccggataaggcgttttcgccgcatccggcaattctctctgattacccttcgccctgcgtcgcactctcaatcgtcaaacgcacgtctgatgtaatcaactccgccagcaactgataaaccttcatcgtttctgccggttcggcatcgccgctatcgctgatatacccttcatcacgcagtgtcagcaccagagaactgaacaccgccttgtcgaagaactccggcgcgttgatgccgtgcagcacggagagacgttgcgcgacggtgcggctctctttctccagcgtaccgcggttgatcgacgggttggcactcaacaaccagaaggtgatggcataacgttgcagcgtttcgcgcgcgcctgcggccagcagctgtagcgtgcgagaatgcgccgggttgatatgcaactcatcatcttgcagggtaatcagcccctgacgttgcatctcatttgccagcgcatcaataacgtccggcaactcgtcgcgatcccagcgcaggaacagctccgctttcagcattgggtaaagcacattgacgtgctccatcaatacgtcgcgggagatgtggcgatgctgggtgacgattgccgccatcagcgaaggcagcaccaacatatgcgcaatgttgttgcgatagtaggtcatcagcaccgcttgctcgcgcggcagaatgatgatgtcgccgattgtgtctttctcgacttcaaacttgttcatttgcagcgcgtgatcgataagctcgctggcgctggctgaaggaacggtagagtccgtggagtagggcacgttgcgcatcagatccaggtagcagttgagttgctcggttaactgctcgcgggtgagtgagcgctgacgtgatgccagtagcgcagtacagcacaggttcatggcgtttgccgcgcctgcgttgttaatgcgtaccatcagatcggcagcaatattattgaccgtcggcgttaaccatgccggacgcaccgcttcgatgggatcgatagattcacgccagtcaggtacatgctggttaaggtaggtcatcaacggcattggttcaccgaagttgacgtaaccctgaccgagattacgcagcttgcttaaaccgcgcagcatctgcggcaggctctctttctctttcgtcgcgccgcgcagttctttggcgtaagtacccacttccatgacgtgctcataaccgatatagatcggaatcagcgtaatcggacgcgtgccgccacgcagcatcgcctgaatggtcatcgacagcgtaccagttttcggatccagcaaacgccccgtacgggaacgaccgccttccacgaagtactcgacggaataaccacggctgaacagttcgccgagatactcccggaaaacggtggaataaagtttattgcctttaaacgtacggcgaataaagaacgcccccagacggcggaaaatcggcccggcaggccagaaattcaggttgatcccggcggcgatatgcggcggcaccagcccctggtgatacagcacgtaagaaagcagcaggtagtccatgtgactgcggtggcaaggcacatataccagctcatgaccgtcgtgggccagctggcgaacgcgctcagcgttatggacgttgatgccctggtaaagtcggttccaggtgaagcccagaatacggtcagtcaggcgaatcatctcgtaagagaaattcgccgcaatctcttccatcagtgcaatcgcgttctgctgcgctttttcatgggagatttttttgctgcgcgcttcatcttctaccgctttggcaatggcgcgggaggcgagcagcttattaaacagatcctgacgagcaggcaaacgtgggcctacggcagccagacgttgacgggcaaagtgcatacgcgccacgcgcgccagtttctgagcgatagttttatccgtgccgtgttcatccgccatacggcgcagcgaaactgacggcgagaaacgcacaaaactgtcgcgaccgagccacagtacagcgaaaaatttctgtacgccgttaagcatacgcagcggcgggttcacttcgcctttttcacgccccggcgcgcgaccaaacatcaccgacactggcaccatctgcacatccagatttgggttgctacggtgcaaatcgagatagtcgtggaacagcttaatagactcttctttcggcgtgtaataggtgaacacacgcggcccgccgtgaatgaacacatagcgcggcagtagcgtgccgtcgatttccagcggctctaacgggtcaggcaagtcatgtgccagacactgggcgcgcaacgtcagcaaatctgctttcgagttgtacggtaaaacgtacataattggacgagaggtatccagccccagttccggggcaggatctgccggaatagacttgctttttaccaggatgcttaatggtaaattcagtaatttgtagtaaattcgtggccagccggacataaacgatgtaaagcctctggttaataatgcaaatgcgcggcaaggatagcagaaagtcatgggaaattctgtggtatccgctcatgtttcgcgcggcgctacgcaaacccgaatcatcggatttaacggtacactgatattgacgctcataatgtaaaaaggttctttcaatggccaataataccactggattcacccgaattatcaaagctgctggctattcctggaaaggtttacgcgctgcatggatcaacgaagcggcattccgtcaggaaggcgtagcggtattgttggcggtggtcatcgcctgctggctggatgtggacgcgattacccgcgtgctgcttatcagctccgtgatgctggtgatgattgtggaaatcctcaatagcgccatcgaagcagtggttgaccgaattggctctgaataccatgagctttccggacgcgcaaaagatatgggatccgctgcggtgctgattgccattatcgtcgccgtgattacctggtgcattctgttatggtcgcattttggataacccttccagaattcgataaatctctggtttattgtgcagtttatggttccaaaatcgccttttgctgtatatactcacagcataactgtatatacacccagggggcggaatgaaagcgttaacggccaggcaacaagaggtgtttgatctcatccgtgatcacatcagccagacaggtatgccgccgacgcgtgcggaaatcgcgcagcgtttggggttccgttccccaaacgcggctgaagaacatctgaaggcgctggcacgcaaaggcgttattgaaattgtttccggcgcatcacgcgggattcgtctgttgcaggaagaggaagaagggttgccgctggtaggtcgtgtggctgccggtgaaccacttctggcgcaacagcatattgaaggtcattatcaggtcgatccttccttattcaagccgaatgctgatttcctgctgcgcgtcagcgggatgtcgatgaaagatatcggcattatggatggtgacttgctggcagtgcataaaactcaggatgtacgtaacggtcaggtcgttgtcgcacgtattgatgacgaagttaccgttaagcgcctgaaaaaacagggcaataaagtcgaactgttgccagaaaatagcgagtttaaaccaattgtcgttgaccttcgtcagcagagcttcaccattgaagggctggcggttggggttattcgcaacggcgactggctgtaacatatctctgagaccgcgatgccgcctggcgtcgcggtttgtttttcatctctcttcatcaggcttgtctgcatggcattcctcacttcatctgataaagcactctggcatctcgccttacccatgattttctccaatatcaccgttccgttgctgggactggtcgatacggcggtaattggtcatcttgatagcccggtttatttgggcggcgtggcggttggtgcaacggcgaccagctttctctttatgctgttgctgtttttacgcatgagcaccaccgggctgactgcgcaggcttatggtgccaaaaatcctcaggcattagcccgtacgctggtgcaaccgttgctgttggcgttgggggctggggcgttaattgcgctgctgcgtacgccgattatcgatctggcgctgcatattgttggcggtagtgaggcagtcctggaacaggcgcggcgctttcttgaaatccgctggttaagcgcaccggcgtcgctggcgaatctggtattactcggttggttactcggcgtgcaatatgcccgtgcgccagtaattttgttagtggtcggcaatatcctcaacattgtgctggatgtctggctggtgatggggctgcatatgaacgtgcagggcgcggcgctggcgacggttattgcggaatatgcaacattgctgattggtctgctaatggtgcgtaaaatcctcaaactacgcggaatttccggcgaaatgctgaaaactgcctggcgaggaaacttccgtcgcttgctggcgcttaaccgcgatatcatgctgcgttcgctgttgttgcaactctgtttcggcgcgatcaccgtacttggcgcgcgactggggagtgacattatcgctgttaacgcggttctgatgacgctactcacctttaccgcctatgcgctggatggttttgcctacgcggttgaagcgcactccggtcaggcatacggtgcgcgcgacggtagccagttgctggatgtctggcgggcagcgtgccgccagtcggggatcgtagcgttactgttttcggtggtttatttgctggctggggaacacatcattgcgttactgacgtcgttaacccagattcagcagctggctgaccgctatcttatctggcaggtgattttgccggtggttggcgtctggtgttatctgctggacggcatgtttataggcgcaacgcgtgccaccgaaatgcgtaacagtatggcggtggccgccgcaggttttgcgctgacgctccttacgctgccgtggctgggtaatcatgctttgtggctggcattaaccgtctttctggcgttgcgcgggctttctctggcggctatctggcggcgtcactggcgcaatggtacctggtttgccgcaacgtgacggttaaaaattctgaataaataatcctaagccaaattgctgactacacttaatctcacgttcagaagaaaagtgaacgtactctcattcacaacctaacgatgaggtcttgattatgaataaagatgaagccggcggtaactggaaacagtttaaaggtaaagtgaaagagcaatggggcaaactgaccgatgatgatatgacgatcattgaaggtaaacgtgatcaactggtcggtaaaatccaggaacgttatggttatcagaaagatcaggcagaaaaagaggtcgtggattgggaaacccgcaatgaatatcgctggtaattaatccctcctgcccgacgtgtacaaggatgtacgccctcttaacgcggtttctttttcacctgcacagagtgatcatgctggcactgttcaggatgacgacacgcttccacttctacacatgccgcacagagcccatgtgcttcaatcacattatgccgcagggcaaaccccatttttgccgccagcgtatgcataatgtcttccacgccttctgcacactcttctttcactgcgccgcagcgatcgcaaataaacatggctgacgtatgggtgggctgatcgaacagatgacagagcacataactgttggtggattccaccttatgcacaaaaccttgctcaagcagaaaatccagcgcgcgataaaccgttggcggcttggcttgcggttcagcttcgcgcagtaaatcaagcagatcataagcgctgatagcgccatcctgcagactcatcaggcgcaacacttccaggcgctgtggggtcaggcgcacattacgctgcgcgcagattttttcagcctgcgctaataactcctgcgttgtggtcttttccatcgggcacctcaaagtgggggttaagaatgtccttactttaccatgttccaggaaaaacaccgagaacccttattgttgccgtaatgttgattttctgttttgtaggtaaggtgttatgttgccttgtcgtaccattatcaacacgataataattaataattcatttttaaataaattgcttcaagttaactcgctatttatttaactgggtttaaacgcatacctgtagttcagaaattatgagcgatttttgatagtgaccagatggcaaaagaattataaggaggacacggtacgacaaaaaaggtagatgaatcatgttgaagataatacccggtgcaactggatactttaataaaacactcaattcaaatcaattcgataatgaagatgcaatcaaagataaattagataatagaggttcaatcaaaggtaaattaaataatatatatggtaaatctattgattatgcagcgctgcgtcatcgggatataattattgcaaaaatagatttgtttattcaacgaatcacgcataatttatggcatgcacgtaaaaaaatgtgtttttaattgtgcaaataaatgatctcaaaatgtgggtcaataagtatattgacgattgcactgatgaggatttaaacgatcgtgactttattgcatcagttgttgaccgggctatttttcatttcgcgattaatagtatatgtaatcctggggataataaagatgcaatgcccattgaacaatgtacttttgatgtagaaactaagaatgaccttccctccacggttcagctattttatgaggaatctaaggataatgaacctttagcgaatatacattttcaagcaataggttctggttttttaacgtttgttaatgcctgccaggaacatgatgacaacagcttaaaattatttgcttcgctgttaatttcactttcatattctagtgcctacgcagatttatcagaaacagtgtatattaatgaaaataatgagagctacctgaaagctcagtttgaaaaattatctcaacgtgatatgaagaagtacctgggagagatgaagcgtctggctgatgggggagaaatgaattttgatggctatctggataagatgtcacatctggtgaatgaaggaacgctcgatcctgatattttaagcaaaatgcgagatgctgcaccacaattaattagcttcgcgaagtcgtttgacccaacctcaaaggaagagattaaaatacttacagacacttctaaattaatttatgatttgttcggggttaaatcggagaaataatatgtgaagttcttcgatagtatggaaggcattatataaaaggacccaatatttattgggttcttttttctctatcaatactattagcagggagatatatcaccagagtttaatgtgtgattttttatttatcgtcgaacctggattgtttatcattggccttaacaaagttaacggctaataagattatttccatcacttcgtgagagcttcatgccttgagaggatctcaattttcttttgcaatgagacaggcgcttcctgttgttatggtatagtaccccgctattgagcctcctgaatagtgatgctgaataacataaccccatgatatatcgataaaataatctctacatttgaaaatgcacggtaattctgaaatgcaaaaaatcaaccaaaccagcgcaatgcctgaaaaaactgacgttcactggagtggtcggtttagcgttgcaccaatgctcgactggacggacagacattgccgctatttcttgcgtctgctttcccgcaatacgttgctgtataccgaaatggtgaccacaggggcgattattcacggtaaaggtgattatctggcgtacagtgaagaagaacatccggtagcgttgcaactgggcggtagcgatccggcggcgctggcgcagtgtgcaaagctggcagaagcgcgcggatatgatgagatcaacctgaatgtcggctgcccgtctgaccgggtgcagaacggcatgtttggtgcgtgtctgatgggtaatgcgcagctggttgccgactgcgtgaaagcgatgcgcgatgtggtgtcgattccggtgacggtgaaaacgcgtattggcatcgacgaccaggacagctatgaatttctctgcgatttcatcaataccgtttccggcaaaggcgagtgtgagatgttcatcatccacgcacgtaaagcctggctttcggggttaagcccgaaagaaaaccgtgaaatcccgccgctcgattatccgcgtgtgtatcaactgaagcgtgactttccgcatctgacaatgtcgattaacggtggtatcaagtcgctggaagaggccaaagcacacctgcaacatatggatggcgtgatggtcgggcgcgaggcgtatcagaatccgggtattctggcggcggtagaccgggagatctttggttcctcggataccgatgccgatccggtggcggtagtgcgcgccatgtatccgtacattgagcgtgaactcagccaggggacgtatctcggccatattacccggcatatgttgggcttgttccagggtattcctggcgcgcggcagtggcggcgttatttaagtgaaaatgcccataaagcgggtgcagacattaatgtgctggaacacgcgctcaaactggtggcggataagcgttaacttttcaccaaaaagtagtcaaattcaccacgccctgcgcaccgtcgcggggcgttttgctgttaaatcaatagattatttttggcatgattcttgtaatgccagcaagagatttcatatttgggagagcatcatgctggaactactttttgtgattggcttttttgtcatgctgatggtcaccggcgtttcgttgctgggcattatcgccgcgctggttgtggcgacggccattatgttcctcggcggtatgctggcattgatgattaagttgctgccgtggttactactggcgattgcggtggtgtgggttattaaggcgattaaagcaccaaaagtgccgaaatatcagcgttatgaccgctggcgttactaagggattgtgcggatgatcacaacctaaggttttatccttagaacaaaataggaattgataatcaaatctgtcactattgcgcctctaacagattcatcgtgctgtaccctacatacagccgaactataaaaagaaagggcttcccaggtggaagccctatttcttttatggaatcagcaggctggaaccttgcgtcgcccggctttccagaatctcatgcgcacgctgcgcatccttcagcggatatttctgctgctcggcgacatcgaccttaatcacaccgctggcaatcaaagagaacagttcattactggcctcggttaattcctcccgcgtggtgatatagccttgcagggaagggcgtgtcacatacaacgagcctttttgattgagaatgcctaagttcacaccggtaaccgcacctgatgagttgccaaaactgaccattaagccgcggcgttgcaggcaatccagcgaccgttcccaggtgtctctgcccacggaatcgtacaccacgcgcactttcttaccgccggtgatctcttttaaccgctcgaccagatcctcttcacgatagttaataacctgccacgcgcccgcttttagcgcgctctgcgctttttgcgcggttcctacggtgccgataagtttcgcgcccagggcttttgcccactggcaggcaattaagccaacgccgccagccgctgcgtggaacaggaactgttcatcgggtttaatttcataggttttgcgcagcagataataaaccgttaagcctttcaggaaggatgccgcagcttgctcaaaagaaattgccgcaggcagaatcgccgctttatccgcaataatgttatgcacagagctgtaagcgcctaacgccgactgcgcatagactacacgatcgcctgccttaatatgctttacaccactgccgactttactcacgatgcctgctgcttcggtgcctaatccgctgggtagcgatggcggcgggtaaaggccgctgcggatatatgtgtcgataaaattgatgccgatggctttattttcgacctggatttcattctccgccggatcggcaggagtgaactctacggcttgaagtacttccgggccaccgtgcttgtgaaattcaattcgtgttgccatgtgtcctccagaacgtatcgtcagggtctgcttcatatgataaagtttcgacccattctttatctcggtaactccattcactatggcaggaaataaacccttcaacaaacagcaggctgaaccccgcgaacgcgatccacaagttgccgggctgaaagtgcctccgcactcgatcgaagcggagcagtcggtgttgggcggtttaatgctagataacgaacgctgggatgatgtagccgagcgtgtggtagcagacgatttttacacccgcccacaccgtcatatctttactgaaatggcgcgtttgcaggaaagcggtagccctatcgatctgattactcttgcggaatcgctggaacgccaggggcaactcgatagcgtcggtggttttgcttatctggcagagctgtcaaaaaatacgccaagtgcggctaacatcagtgcctatgcggacatcgtgcgtgaacgtgccgttgtccgtgagatgatctcggttgcgaatgagattgccgaagctggttttgatccgcaggggcgtaccagcgaagatctgctggatctggctgaatcccgcgtctttaaaattgccgaaagtcgtgcgaacaaagacgaagggccgaagaacatcgccgatgtgctcgacgcaaccgtggcgcgtattgagcagttgtttcagcagccacacgatggcgttaccggggtaaacaccggttatgacgatctcaacaaaaaaaccgctggcttgcagccgtcggatttgatcatcgtcgccgcgcgtccgtcgatgggtaaaacaacatttgcgatgaacctcgtcgaaaacgcggcgatgttgcaggataaaccggtacttatcttctcgctggagatgccatcagaacagatcatgatgcgttctctggcgtcgctgtcgcgcgttgaccagactaaaatccgtaccgggcagctcgatgacgaagactgggcgcgcatttccggcaccatgggtattttgctcgaaaaacgcaatatctatatcgatgactcctccggcctgacgccaacggaagtgcgttcccgcgcacgccgtattgcccgtgaacacggcggcatcgggcttatcatgatcgactacctgcaactgatgcgcgtaccggcgctttccgataaccgtacgctggaaattgcagaaatctctcgctcgctgaaagcactggcgaaagaactgaacgtgccggtggtggcgctgtcccagttgaaccgttctctggaacaacgtgccgacaaacgcccggtcaactccgacctgcgtgaatctggctctatcgagcaggatgcggacttgatcatgtttatctatcgtgatgaggtgtatcacgaaaacagtgatttaaaaggcatcgcggaaattattatcggtaaacaacgtaacggcccaatcgggacggtacgcctgacctttaacggtcaatggtcgcgcttcgacaactatgcggggccgcagtacgacgacgaataataattattttatgaattaggtaattaaagcaaacacttatcaaggaacacaaatgcaagcggcaactgttgtgattaaccgccgcgctctgcgacacaacctgcaacgtcttcgtgaactggcccctgccagtaaaatggttgcggtggtgaaagcgaacgcttatggtcacggtcttcttgagaccgcgcgaacgctccccgatgctgacgcctttggcgtagcccgtctcgaagaagctctgcgactgcgtgcggggggaatcaccaaacctgtactgttactcgaaggcttttttgatgccagagatctgccgacgatttctgcgcaacattttcataccgccgtgcataacgaagaacagctggctgcgctggaagaggctagcctggacgagccggttaccgtctggatgaaactcgataccggtatgcaccgtctgggcgtaaggccggaacaggctgaggcgttttatcatcgcctgacccagtgcaaaaacgttcgtcagccggtgaatatcgtcagccattttgcgcgcgcggatgaaccaaaatgtggcgcaaccgagaaacaactcgctatctttaataccttttgcgaaggcaaacctggtcaacgttccattgccgcgtcgggtggcattctgctgtggccacagtcgcattttgactgggtgcgcccgggcatcattctttatggcgtctcgccgctggaagatcgctccaccggtgccgattttggctgtcagccagtgatgtcactaacctccagcctgattgccgtgcgtgagcataaagccggagagcctgttggttatggtggaacctgggtaagcgaacgtgatacccgtcttggcgtagtcgcgatgggctatggcgatggttatccgcgcgccgcgccgtccggtacgccagtgctggtgaacggtcgcgaagtaccgattgtcgggcgcgtggcgatggatatgatctgcgtagacttaggtccacaggcgcaggacaaagccggggatccggtcattttatggggcgaaggtttgcccgtagaacgtatcgctgaaatgacgaaagtaagcgcttacgaacttattacgcgcctgacttcaagggtcgcgatgaaatacgtggattaatcgttctgtaatatttgattgtctgtgccggatgcggcgtgaatgccttatccggccaataaaatcctaaaaattcaataagttgatgttctttcatgctcttataaaggtcgtgcctctggcggatgtacgtttgtcatgagtctcactctgttgctaattgccgttcgctcctgaacatccactcgatcttcgccttcttccggtttattgtgttttaaccacctgcccgtaaacctggagaaccatcgcgtgtttcaaaaagttgacgcctacgctggcgacccgattcttacgcttatggagcgttttaaagaagaccctcgcagcgacaaagtgaatttaagtatcggtctgtactacaacgaagacggaattattccacaactgcaagccgtggcggaggcggaagcgcgcctgaatgcgcagcctcatggcgcttcgctttatttaccgatggaagggcttaactgctatcgccatgccattgcgccgctgctgtttggtgcggaccatccggtactgaaacaacagcgcgtagcaaccattcaaacccttggcggctccggggcattgaaagtgggcgcggatttcctgaaacgctacttcccggaatcaggcgtctgggtcagcgatcctacctgggaaaaccacgtagcaatattcgccggggctggattcgaagtgagtacttacccctggtatgacgaagcgactaacggcgtgcgctttaatgacctgttggcgacgctgaaaacattacctgcccgcagtattgtgttgctgcatccatgttgccacaacccaacgggtgccgatctcactaatgatcagtgggatgcggtgattgaaattctcaaagcccgcgagcttattccattcctcgatattgcctatcaaggatttggtgccggtatggaagaggatgcctacgctattcgcgccattgccagcgctggattacccgctctggtgagcaattcgttctcgaaaattttctccctttacggcgagcgcgtcggcggactttctgttatgtgtgaagatgccgaagccgctggccgcgtactggggcaattgaaagcaacagttcgccgcaactactccagcccgccgaattttggtgcgcaggtggtggctgcagtgctgaatgacgaggcattgaaagccagctggctggcggaagtagaagagatgcgtactcgcattctggcaatgcgtcaggaattggtgaaggtattaagcacagagatgccagaacgcaatttcgattatctgcttaatcagcgcggcatgttcagttataccggtttaagtgccgctcaggttgaccgactacgtgaagaatttggtgtctatctcatcgccagcggtcgcatgtgtgtcgccgggttaaatacggcaaatgtacaacgtgtggcaaaggcgtttgctgcggtgatgtaatgcaggaaagcaggctggagctacccagcctgcagtgaaattaaactgtcgtcgctttcactctttctttatagatgatttttttgatgccatcgttctacgtgagagataataaacgttgttagttcttttattgttaagcttatcccaattatctggaattccttatcctgtttttttgggtggagtaataatttctgcacatctaaccattattaaatttaataataagtatcgggtttgttacgatagaatatttctatatcctcaagaatatgctttgccttattgcctgtgactttctgagattcaattatagtatcgttaaattctaatgttaaagagaactcttttttccgctttgtgtaagtttaaccttatattgattaccaatatcaaataaaaaggtcctgtaatgagaataatcacctttaacctcctcggcaaaacagcaaagcgtgcaaatatacataaagtctttcttacccctgattttgttaactaaatcaataaatgcgtgaaaaactttacttgcaatagaacttgatacttcttctccaggtctaaaaaatcttttgcaatttttaactgtgtttctatgtataaaaagaaatctttggcataagagatatctttattatttagtgcatctagctcaacaggtaaagatgtcgttttgttgctattcacatatgatatattcatatcatcatctccatcgcgagtaataaaattaatcaccattgtagggtagggggctggtcaatcagaaatcatctttataaacttcgattgtttttgtaatgctgtatcattaagttcattaaatcgtacagcagataaatgttctatcaaatttcgctcatttgccgaggattcatcataataaacgtaaaattaatgtatccttacatcgagtaataaacattttttatacaaaaaaagacaggaacgtatttactgggttaaatataatcatcctgcttttcatcacaaaaaccgcagataatccttcctttccccggcagctggcgttatggtcagatggtttttgcaacaaatctcacaataaaaagtttcaacatactgactatttagggaaaaatatgcgcaagatcacacaggcaatcagtgccgtttgcttattgttcgctctaaacagttccgctgttgccctggcctcatctccttcaccgcttaaccctgggactaacgttgccaggcttgctgaacaggcacccattcattgggtttcggtcgcacaaattgaaaatagcctcgcagggcgtccgccaatggcggtggggtttgatatcgatgacacggtacttttttccagtccgggcttctggcgcggcaaaaaaaccttctcgccagaaagcgaagattatctgaaaaatcctgtgttctgggaaaaaatgaacaatggctgggatgaattcagcattccaaaagaggtcgctcgccagctgattgatatgcatgtacgccgcggtgacgcgatcttctttgtgactggtcgtagcccgacgaaaacagaaacggtttcaaaaacgctggcggataattttcatattcctgccaccaacatgaatccggtgatctttgcgggcgataaaccagggcaaaatacaaaatcgcaatggctgcaggataaaaatatccgaattttttatggcgattctgataatgatattaccgccgcacgcgatgtcggcgctcgtggtatccgcattctgcgcgcctccaactctacctacaaacccttgccacaagcgggtgcgtttggtgaagaggtgatcgtcaattcagaatactgacagagcgggagagcgtgatgctctcccgaatgctgtttttttaatcacacctttatcctttcgctgtcttgctgcaaactgattaagagagttttatcaaggagcagcacatgtggtatcaaaagacgctcacgcttagcgccaaatctcgtgggtttcatctggtaacggatgaaattctgaatcagctggctgatatgccgcgcgttaacatcggcttactgcatctgttgctgcaacatacctccgcctctctgacacttaatgagaactgcgatcccaccgtacgccacgacatggagcgttttttcctccgcaccgttcccgacaacggaaattatgagcatgactatgagggagcagacgatatgccttctcatatcaaatcctcaatgctgggaacatcgcttgtattgccggtgcataaagggcgtattcagaccggcacctggcaaggcatttggctgggggaacatcgcatccacggcggatcgcgtcgcatcatcgcgacactacaaggggagtaaaaaatgaccatttcggagttgctacaatattgcatggcaaaaccaggcgcagaacagagcgtgcataatgactggaaagcgacgcagatcaaagtggaagatgtactgtttgcgatggtgaaagaagtagaaaatcgcccagctgtttcgctgaaaaccagcccggagctggcggagctgctacgtcagcagcacagcgatgtgcgtccaagccgccatctgaataaagcgcactggagcaccgtgtatctcgacggttcgctgccagattcgcaaatctattatctggtggatgcgtcttatcagcaggcggtgaatttactgccggaagaaaaacgtaaattgctggtgcaactctgaaaggaaaaggccgctcagaaagcggccttaacgattacagcatcggcttaaggaagcgtgccgtgtgtgatgcttcgcactccgcgacggtttctggcgtaccggagacgaggatctcgccgccaccactgccgccttctggtcccaggtcgacaatccagtcagcggttttgatcacgtcgagattgtgctcaatcaccacaatggtgttgccctgatcgcgcagtttatgcagtacgtcgagcagttgctgaatatcggcgaagtgcagaccggtggtcggctcgtcgagaatatacagcgtctgcccggtgccgcgttttgacagttcacgcgccagcttcacgcgctgggcttcaccgcctgaaagggtggttgcggactgccccagtcgaatgtacgtcaggccaacgtccatcaacgtttgcagcttacgcgccagtgcaggtacggcatcaaagaactcacgcgcctcttcgatggtcatatccagcacttcgtggatggttttgcctttgtacttaatctccagcgtttcacggttatagcgtttacctttgcactggtcgcacggcacgtagatatccggcaggaagtgcatctccactttgatcacgccatcgccctgacaggcctcgcagcgtccgccacgaacgttaaagctgaaacgtcccggcgtatagccgcgcgcacgggattccggtacgcccgcaaacagttcgcgcacaggcgtaaacacgccggtataggtcgccgggttagaacgtggagtacgaccaattgggctttggtcgatatcgatcactttatcgaaatgctccagcccctgaatatcgcgatacggtgctggttcggcgatggtcgccccattcaactggcgttgggcaatcgggaacagtgtgtcgttaatcagcgtcgatttaccggaacctgaaaccccggtgatgcaggtaaacagacccaccggcagcgtcagcgtcacgtccttcaggttgttgccgcgtgcgcctgtcagcttcagcactttttccggattcgccggaacgcgtttcttcggcacttcaatcttgcgtttgccgctcatgtactgcccggtcaacgactccggcaccgccataatcgcttccagcggaccttctgcgaccacttcaccgccgtgaacacctgcgcccgggccaatgtcgatcacatggtcagcggcgcgaattgcgtcttcgtcgtgctccaccacaatcacggtattaccgagatcgcgcagatggataagcgtacccaacaggcgctcgttatcacgctggtgcaggccgatagacggctcgtccagcacgtacataacgccaaccaggcccgcaccaatctggctcgccagacggatacgctgtgcttcaccgccagaaagcgtttctgccgagcgggaaagcgtcaggtaattcaggccgacgttaacgaggaatttcagacgatcgccgatctctttaaggattttttctgcaatcttcgcccgctgacctgcgagtttgagattgttgaagaattccatcgcatgaccaatgctcatgtcggagatagcaggcagcggcgtattctcgacatacacgtggcgcgcttcccgacgcagacgcgtcccttcgcagctggcgcacggacgattactgataaacttggctaattcttcgcgtaccgcgctggattccgtctctttatagcggcgctccatattatgcagcacgccttcgaacggatgacgacgaatggaggtatcgccacgatcgttcatgtatttgaattcaatgttttctttgccagaaccgtacaacaccactttatgcacgttcgcgctcaggctgccccacggcgcttcgacgtcgaacttatagtgatctgccagcgatttcagcatctggaaataatagaagttgcggcgatcccagccacggatcgcaccaccagccagcgacagttccggattctggatcactcgatcaggatcgaaatattgctgtacgccaaggccgtcgcaggtcgggcaggcccccgccgggttgttaaacgaaaacagtcgcggctccagttcacgcatactgtagccgcaaattgggcaggcgaagttggcggagaacagcagctcttccgctttcgggtcgtccatatccgccactaccgcggtaccaccggaaagctccagcgcggtttcaaatgactcggcaagacgttgggtaagatcgtcacgcaccttgaagcgatcaaccaccacttcaatggtatgtttcttttgcagttccagttttggcggatcggaaagatcgcagacttcgccatcaatacgagcacggatgtagccctggcttgccaggttctccagcgttttggtgtgttcgcctttgcgctctttaatgattggcgcgagtagcatcagacgcttgccttccggctgcgacagcacgttatccaccatctggctgacggtttgcgccgccagcgggacgtcgtggtccggacagcgcggctcgccaacgcgggcgaataacaaacgcaaatagtcgtggatttcggtgattgtccccaccgtagaacgcgggttatgagacgtcgatttctgctcaattgagatggcaggagaaagcccctcaatatgatcgacgtccggcttttccatcagtgacagaaactgccgcgcgtaggcggaaagggattcaacgtaacggcgctgcccttcggcatataaggtgtcgaaagcgagcgaggatttgccagaacccgaaagcccggtcacgacaatgagcttgtcgcgggggataacgaggttgatgtttttgagattatgggtgcgggcgccccgaacttcgatcttatccattcacctttcccggattaaacgcttttttgcccggtggcatggtgctaccggcgatcacaaacggttaattatgacacaaattgacctgaatgaatatacagtattggaatgcattacccggagtgttgtgtaacaatgtctggccaggtttgtttcccggaaccgaggtcacaacatagtaaaagcgctattggtaatggtacaatcgcgcgtttacacttattcagaacgatttttttcaggagacacgaacatggccagcagaggcgtaaacaaggttattctcgttggtaatctgggtcaggacccggaagtacgctacatgccaaatggtggcgcagttgccaacattacgctggctacttccgaatcctggcgtgataaagcgaccggcgagatgaaagaacagactgaatggcaccgcgttgtgctgttcggcaaactggcagaagtggcgagcgaatatctgcgtaaaggttctcaggtttatatcgaaggtcagctgcgtacccgtaaatggaccgatcaatccggtcaggatcgctacaccacagaagtcgtggtgaacgttggcggcaccatgcagatgctgggtggtcgtcagggtggtggcgctccggcaggtggcaatatcggtggtggtcagccgcagggcggttggggtcagcctcagcagccgcagggtggcaatcagttcagcggcggcgcgcagtctcgcccgcagcagtccgctccggcagcgccgtctaacgagccgccgatggactttgatgatgacattccgttctgatttgtcattaaaacaataggttatattgttttaaggtggatgattaaagcatctgccagccataaaaaagaagcctccgttatggaggcttctacgtatcaggtcaaaatcattggccattgtggcggtgtctgattcatctcttctatcatcaccgactcgatgttgtgccagatagcggtgatgtccgccattgtgatgccaagcaaccccattgcgaaccaacaggcggaaacaacgcccagaccgctgctgatcaccgcaagcccgacataatcagaccgacgaaaacggatgttgagtgtgctggccagaaacatcattacggcactaagaagttgccagcgaagaagaaccacgccagtggtgagggtagccatcaaacaattcctctgaaaagagccgatgccctggacagcgcggcgttgttcacgggaggcgtggtacactctggctatcgcggggcttgcagaacacaaaaatgaaacactctgtttgtttcattaattttgtgaactatatcacaattgattgtttgttagccatattaggccgtgacttttattgctgtacagattatgtggtttttcagtggcattaagggcatatcttcccgccgcctctgcattcctgtaggaaattaattttgaatatcaatgaattattttcatccaggtgacgattagaaaggtatcaatttcaaatcaggcaaaagtgctatttataccgtaagatttatctaaagacgtcggtacccagggttttcaccttgcaatggccgggtataaacaggcaggaaattgatagcaatgagtcatcgtgcacgacaccaattactggcgttgccgggcattatctttttagttctctttcccatcattctttcgctatggattgccttcctttgggcaaaatcagaagtgaataatcagctccgaacctttgctcaactggcactggataaatccgagctggtcattcgccaggcagatttagtgagcgatgcagctgaacgctatcaggggcaagtttgcactccagcccatcaaaagcgaatgttgaatattattcgtggctatctttatattaatgaattgatctatgcccgtgataaccattttttatgctcatcgctgatagcgcctgtaaacggctatacgattgcaccggccgattataagcgtgaacctaacgtttctatctattattaccgcgatacgccttttttctctggctataaaatgacctatatgcagcggggaaattatgtggcggttatcaaccctctcttctggagtgaagtgatgtctgatgacccgacattgcaatggggtgtgtatgatacggtgacgaaaacctttttctcgttaagcaaagaggcctcggcagcaacgttttctccgctgattcatttgaaggatttaaccgtacaaagaaatggctatttatatgcgacagtttattcgacaaaacgcccaattgcagccattgttgcgacttcatatcaacgtcttataacccatttttataatcatcttatttttgcgttgcccgccggtattttggggagtcttgttctgctattactctggctacgtattcgacaaaactatttatctcccaaacgtaaattgcaacgcgccctcgaaaaacatcaactttgtctttattaccagccaataatcgatatcaaaacagaaaaatgtatcggcgctgaagcgttgttacgttggcctggtgagcaggggcaaataatgaatccggcagagtttattccgctggcagaaaaggaggggatgatagaacagataactgattatgttattgataatgtcttccgcgatctgggcgattacctggcaacacatgcagatcgctatgtttctattaacctgtcggcctccgattttcatacgtcacggttgatagcgcgaatcaatcagaaaacagagcaatacgcggtgcgtccgcagcaaattaaatttgaagtgactgagcatgcatttcttgatgttgacaaaatgacgccgattattctggctttccgccaggcaggttacgaagtggcaattgatgattttggtattggctactctaacttgcataaccttaaatcattgaatgtcgatattttgaaaatcgacaaatcgtttgttgaaacgctgaccacccacaaaaccagtcatttgattgcggaacacatcatcgagctggcgcacagcctggggttaaaaacgatcgctgaaggcgtcgaaactgaggagcaggttaactggctgcgcaaacgcggcgtgcgctattgccagggatggttctttgcgaaggcgatgccgccgcaggtgtttatgcaatggatggagcaattacccgcgcgggagttaacgcgcgggcaataaaattacaggcggtggcgataatcgctgggagtgcgatcaaactgccgacggaaaacgcgggagaaggtctgctgcgagacataacccaggtccattgcgatatcaaaaatcggacgctcggtggtgcgcaactcaacggcggccagtaacaggcggcgttggcgaatgtaatcgccaagcgtctgatgcgtcaccgtgcggaacattcgttgcaagtaccactttgaatagcctgatttttttgcgactacatcaatgttaagcggctggtcaatatgctcgtcaatccatgcgataagatcctgaataattttctgatgggacataaatctgcctcttttcagtgttcagttcgttaattcatctgttggggagtataattcctcaagttaacttgaggtaaagcgatttatggaaaagaaattaccccgcattaaagcgctgctaacccccggcgaagtggcgaaacgcagcggtgtggcggtatcggcgctgcatttctatgaaagtaaagggttgattaccagtatccgtaacagcggcaatcagcggcgatataaacgtgatgtgttgcgatatgttgcaattatcaaaattgctcagcgtattggcattccgctggcgaccattggtgaagcgtttggcgtgttgcccgaagggcatacgttaagtgcgaaagagtggaaacagctttcgtcccaatggcgagaagagttggatcggcgcattcataccttagtggcgctgcgtgacgaactggacggatgtattggttgtggctgcctttcgcgcagtgattgcccgttgcgtaacccgggcgaccgcttaggagaagaaggtaccggcgcacgcttgctggaagatgaacaaaactaaagcgccacaagggcgctttagtttgttttccggtctttgtctttctctctatcccgctggtacacaggagggtttcccccgacgtcaacacacctcattcgagcacgtggtggaggttccggttggtgttgatgctttaattgtatgtcaccgacgtttcttcgccagtgtaaaagtatactttttaaccgcaatatttttgtcatctcagacgattttttatcgcaatcctgaacggtatacggctcgataacgctgcaatcttgcgcaccgacgataacgtttgcgcatcaattgcctggtttttcatcgtcaagacaataaaagagaaaaaagcagcaaacttcggttgaaaaagccgctatgatcgccggataatcgtttgctttttttaccacccgttttgtatgcgcggagctaaacgtttgcttttttgcgacgcagcaaattgtcgcaaacctggagcaggaagataacgtttcgctggcaggggattgtccgccacgcatcttgacgaaaattaaactctcaggggatgttttcttatgtctacgccatcagcgcgtaccggcggttcactcgacgcctggtttaaaatttcacaacgtggaagcactgtccgtcaggaagtggttgccgggttaacaacgtttctggcgatggtctactcggtcatcgtcgttccaggtatgttgggtaaagcaggcttcccgcctgcggcagttttcgttgcaacctgtctggttgccggactcggttctatcgtgatgggtctgtgggctaatctgccgttggcgattggttgcgccatctccctgacagcgtttaccgcattcagcctggtgctggggcaacatattagcgtacctgtcgcgctgggtgccgtgttcctgatgggtgtgctgtttacggtaatttctgccacgggtatccgtagctggattttgcgcaacttgcctcacggtgtggcgcacggcacggggattggtatcggtctgttcctgctgctcattgccgctaacggtgtcggtctggtgattaaaaacccgcttgatggtctgcccgttgcgctgggtgatttcgcgaccttcccggtgattatgtcactggtaggtctggcggtgatcatcggcctggaaaaactgaaagtccctggtggcattctgctgaccattatcggtatctcaattgtcggtttgatcttcgatcctaacgtccatttctccggcgttttcgccatgccttcattgagcgatgaaaacggcaattcactgattggcagcctggacattatgggcgcgctgaatcctgtagtcctgccaagcgttctggcgctggtgatgacggcagtatttgatgccaccggaactatccgtgccgtcgccggccaggcgaacctgctggataaagatgggcagatcatcgacggtgggaaagcactgaccactgactccatgagcagcgttttctctggcctggtgggtgcggctccggcagcggtatacatcgagtctgcggcgggtacggcggcgggcggtaaaaccggtttgacggctatcaccgttggcgtgctgttcctcctgattctgttcctctctccgctctcttacctcgttccggggtatgcaacggctccggcgctgatgtacgttggcctgctgatgctgagcaacgtggcgaaaatcgactttgctgattttgttgatgcgatggcgggtctggttacggctgtattcatcgtgctgacctgtaacatcgtaacaggcatcatgatcggcttcgcgactctggtgattggtcgtctggtttccggcgaatggcgcaagttgaacatcggtacggtcgttatcgccgtggcgctggtgaccttctatgcgggtggctgggctatctaatctttcatcggattctgaaaacgggtggcaatggctgcccgtttttattttctccgcacattgtgtgagcttttgcgatattctgaaaaaaatgagaattcaggcataacgtctttctcagatcataaaaaacatcgcaaacagggaacgcatggaaatcttcttcaccatactgataatgaccctcgtggtctcgctgtccggggtggtcactcgtgtcatgccctttcagatcccgcttccgcttatgcaaatcgccatcggtgcgctactggcgtggccgacgtttggtttgcatgtggagtttgatcctgaactctttttagtcttgtttatcccgccgttgctgttcgctgatggctggaaaacgccgacccgtgaatttctcgaacatggtcgagagattttcggcctcgcgctggcgctggtggtggtcaccgtggtcggcattggcttccttatttactgggtggtgccgggcattccgctgatccctgcctttgcgctggcggcggtgctttctccgaccgatgctgtggcgctctccgggattgttggcgaagggcgcatcccgaaaaaaatcatgggcattttgcagggcgaagcgttgatgaatgacgcctccggtctggtgtcgttgaagtttgccgtagcagtggcgatggggacgatgatcttcaccgtcggcggtgcgacggtcgaatttatgaaagtagccattggcggtattctcgccggttttgtggtgagctggctgtacggtcgctcgctgcgattcctcagccgctggggcggtgatgaacccgcgacgcagatcgtcctgctgttcctgctgccattcgcttcttatctgattgccgaacatattggcgtttccggcatcctcgctgcggttgccgccgggatgaccatcacccgctccggtgtgatgcgccgtgcgccgctggcaatgcgcctgcgtgcaaacagcacctgggcgatgctggaatttgtctttaacggcatggtgttcctgctgttaggtctgcagctgccgggtattctggagacgtcgctgatggcagcagaaatcgaccctaacgtcgaaatctggatgctgtttaccaatattattctgatatatgcggcgctgatgctggtccgtttcggctggctgtggacgatgaaaaagttcagcaaccgcttcctgaagaagaagccgatggagtttggttcgtggaccacacgagaaatcctgatcgcgtctttcgccggggtgcgtggggcgatcactctggccggtgtgctctctatcccgctgctcttgccggatggtaacgtcttcccggcgcgctatgagctggtgttcctggcggctggcgtcattctcttctcgctgtttgtcggcgtggtgatgttgcctattctgctacaacacattgaagtcgcggatcattcgcaacaattgaaagaggaacgtattgcgcgagcggcaacggcagaagtggcgattgtggcgatccagaaaatggaggagcgtctggcggcggataccgaagagaatatcgataaccagctgcttacggaggtcagttctcgcgtcattggtaacctgcgtcgtcgcgccgatggacgtaacgacgttgaaagttccgtgcaggaagagaaccttgagcgtcgcttccgtctggcggcattgcgttctgaacgtgctgaactttaccacctgcgcgccacacgggagatcagcaacgaaacgctgcaaaaattactgcacgatctcgatttgcttgaagcgttgctaattgaggaaaatcagtaagccgaaagcgacgtaaccaggcccgaggtaatctgaaaaaggtgcaatcttttgcacctttaacaggttagctcgggctaacattcatgattctaaaacaaataaattatctctcttttaaagtcaattcattggctgttcttcgacttaacctcaatctgcatcttgcataatatctgcagtaatcttcatagcgactgcatgaagattatcctcagtttgtgacatgccagtatgagtggcacaatcttcttcaaagaatttctgtagtgttaccaggatatcactattaatggagatattttcctcaccacggagaatggtaatacccattccctggacgctagcctcatcgaaattaacacgatagagacggatattaaacatccaggcttttgttaaaacagaacagttgaaatggcaattgcttaaattggcattattaaaattaacattagccatattagagtcggtacatataaccatttcgaggaacgtatttgttaaccgcgtaaaaaagagtttgctatcaattaagtttatattctggagggttgctttattcaggttgacacgagacagatcagcatgttcaaagttaattaaatcaagtttagagaagctaaggtcggctctaaataaattaatatatggcgctattactttataaagatttacctcagccatgtatgccatataaaaatttgaataatcaaggaaggtatttttaatattggctctattcattgttgcattgtagaattgaacatgcatagcggaacatgaatttagagttccgtcagtcatttttatctgagcgaaatttgagtcatcgagaatacaattatcaaaaagtattttttccattatggcgaaattaaaattcgttttatacatattacagtcctgaaaaatagcgttttgtagtctgcaacctgcaaaattcgaattggataaatcttcatctttaatcacgatacctttcaggctaaggtgtgaaaaatcgtaaccaccatttactgtctgtgggatttcgatagtattattatggacggtgacattatttataaaatataccaccttaattgacacttccttatctttattaaggtaaactcttctcgtaattctatcgtcacatttattatttgcatgtgaagctatatctataaaatatttatgtattttcctgtccgtttctttcgtgatttttcctgatggtaaactatcataaattcttttcattttctgaatcaagcctatcactttttcatgatcatccattttgaaaagagagagggctttattgtcaattaacgtgtttttatgatgtttgctgtaattatctgattttgttttctttgtatgtgatggacttgtgacagagtggttatcgttaatcaggcaaagagggaaaaacatattatttaaaccattatagcgcataaaatatccttataattaacaagaaagaaaaggcatattctctgcattatcattttctacgactgtcaaaaatcgctcattttttaatgagtttatttgtttaatattatgggaaaaggtgatgcatttgggagaggaagagtattccccggtcagacgaccggggaaggggagagattaatgcgcgcggccttgctcaacgccaaagccggtctgggagcggataaactgcgcgcggaacagttcacgctcacgcgcgccttccgctgagttatcggttgccgagaagaaccagatgccgaggaatgccacggtgatagagaacagcgccgggtattcatacgggaagatggctttttcgtgaccaaggatctgtacccaaatcgtcgggccgaggatcatcagtactactgcggtaatcagccccagccagccacccatcatcgcgccacgcgtggtcagtttcgaccagtacatagaaagcagaatgatcgggaagttacagctcgccgcgatggcaaacgccagccccaccataaaggcgatgttctgattctcaaacagcacgccgaggataatcgcaatcacgccgaggatcagtacggtgatttttgatacccgcagctcttcacgttcggtcgcgccttttttgaagacgttagcgtacaagtcatgcgaaaccgcggatgcgcccgccagcgtcagacccgcaaccaccgcgaggatagtggcgaaagcaaccgctgaaataaaaccgaggaacaggttgccgcccactgcattcgccaggtgaacggccgccatgttgttaccaccaatcagatggcccgccgcgtctttatattccggattcgcaccaaccagcatgatcgcgccgaagccgataataaaggtcagaatatagaagtagcccataaacccggtggcgtagaacacgctcttacgtgcttcgcgggcatcgctgactgtaaagaagcgcatcagaatgtgcggcaagcccgccgtaccaaacatcagtcccagacccagagagagcgcggagatcggatctttcaccagcccgcccggcttcatgatgtcgacacctttcgggtgtaccgccatcgcttcactgaacagattgttgaagctaaagccgacgtgtttcatcaccataaaggccataaagctggcaccgaacagcaacagcacggctttgataatttgcacccaggtggtcgccagcatgccgccgaacaggacgtacatcatcatcagcacgccgaccagcaccaccgcaatgtgatagttaaggccaaacagcagctcgatcagtttacctgcgcccaccatctgggcgataaggtaaagcgccaccaccaccagagaaccacaggccgaaagaatacgaatcggcccttgtttcagacggtaagaggccacatcggcaaaggtgtagcgccccaggttacgcagacgttcggcaatcaggaacaaaatgatcggccagcccaccaggaagcccagcgagtaaattaagccgtcatagccggaggtaaacaccagcgcggagatccccaagaatgaggcggcggacatatagtccccggcaatcgccagcccgttctggaagccagtgatattgccgcctgcggtgtagtagtcgctacgagaacgtacgcgttttgatgcccagtaggtaatgccgagcgtaaacacgacgaaaatcaggaacataataatcgcctgccagttcgttggctggcgctctacggccccgctaatagcatccgcggcgttagctgcgaaagggagtgtggcggcaagcgccgtcagaactcttttcatgatgcttgtacctcatgcaggacttcattattaagacggtcgaattcgccgttcgcccgccagatgtagataccggtgagaacaaaggagatcacaatcactccaacaccaattggaataccgcgtgtgacgctggtgttcggattcagcggcgtgcccagccagccgggcgcgaaggcgatcagtaaaataaagccgatataaactgccagcataataatcgacaggatggtggcaaaccgttgccgtttttcgactaactccctgaaatgcgcattgtcttctatccgctgataaatagtgccattcatcacagattctccagaggtaatgtagggattgttttaattcccgctcccttatgggagaaggttaacgctcgggtaacccttgccgaatgtaggccggataaggcgtttacgccgcatccggcaatcaatgcctgatgcgacgctgtcgcgtcttatcaggcctacaaaccgttaccgactcgcatcgggcaattgtgggttacgatggcatcgcgatagcctgcttctcttcaagcagcttctcgactacgccaggatcggcaagcgtcgaggtatcgcccaggttgctggtatcgcccgccgcaattttgcgcagaatacggcgcataattttgccggagcgggttttaggcagggagtcggtccagtgcagcacgtctggcgtcgccagcgggccaatctctttacgcacccagttgcggacttctgcgtacagttctggtgacggttcctccccgtgattaagcgtgacgtaggcgtagatcgcctgacctttaatattgtgcggaatacctactacggcggcttcggcaatcttcggatgcgccaccagcgccgactcaatctctgccgtccccagacggtgaccggagacgttcagcacgtcgtccacacgcccggttatccagtaatagccatcttcatcgcgacgcgcgccgtcgccgctgaaatacatatttttgaaggtggagaagtaggtctgttcaaaacgttcgtgatcgccaaacagcgtacgcgcctgacccggccaggagtcggtgattaccaggctaccttcggtggccccctccagcgggttaccttcgttatcgaccagcgccggttgcacgccgaagaacggacgtgttgccgaaccggctttcagctcggtagcgccaggcagcggggtgatcatgaaaccgccggtttcggtctgccaccaggtatcgaccaccggacatttctcgttgccgatttttttccagtaccactcccacgcttccgggttaattggctcgcccacggaaccgagaatgcgcagcgacgaacggtcggtgccttcgatcgctttatcgccttccgccatcagcgcgcggatcgccgtgggtgcggtatagagaatattgacctgatgcttgtccaccacctgcgccatacgggcaggcgtcggccagttgggtacgccttcaaacatcagcgtggtcgcaccgcaggccagcgggccgtacagcaagtaactgtgtccggtcacccagcccacatcggcggtgcaccagtagatatcacccggatgataatcaaagacatatttaaaggtcagcgccgcgtacaccagataaccgccggtagtatgcagcacaccttttggcttaccggtagaaccggaggtgtagagaataaacagcggatcttcggcgttcatctcttccgcctggtgctgatcgctcgcttgctcaaccaggtcgtgccaccacaggtcgcgcccttcctgccagtcaattttcccgccagtacgcttcagtaccaccacatgctctacgctggtgacgttcgggtttttcagcgcgtcatcaacgtttttcttcagcggaatactgcgcccggcacgcacaccttcgtcggaagtgatcaccagtcgtgagttggaatcaataatgcgcccggcaacggcttccggcgagaagccgccgaaaatcaccgaatgcaccgcgccaatgcgggcgcaggccagcatcgcaaccgcggcttccggcaccatcggcatataaatcgccaccacatcaccttttttaatgcccagctcgagcagggtattggcgaagcggcagacgtcgcggtgcagctctttatagctgatatgtttgctctggctggcgtcgtcgccttcccagatgatggcggtacgatcgccgttttcttgcagatggcggtcaaggcagtttgccgccagattcagcgtgccgtcctcgtaccatttaatggacacattaccgggggcaaaggaggtgtttttcaccttctggtaaggtttgatccagtcaagaatttttccctgttcgccccagaaggtatcaggtacgttaatagattgttgatacatcgcctcgtactgctgagggtttatcaggcaacggtctgcgatgttggcaggaatggtgtgtttgtgaatttggctcatgcttttgttctccttgtaggatgttaataatatgtggcataagcgttaaatgtaggggtattggcagttttgtttagtatttgggcgacagatcacgcaaaagtagaattgtgcaaataaacggcagggtaatttttgaaggtcagcaacaaaagttgattaattctttgaggaacatgcagttatgcatgctgttgaaaaagaggaagatactgactaactctaaagtggtattttacatgcacttacaattgattaaagacaacattcacagtgtggttatttgttacacataggggcgagcaatgtcatgacagtgtaggtgcggttactgtcgtgaaaaacaataaaaaccgccattgcaacaatggcgcaattcggatgaagcccctatgacaaggataaaaataaacgcacgccgtatcttcagcttattgattccttttttctttttcacttctgttcacgctgaacaaacggctgctcccgcaaaacctgtaactgtggaagcgaagaatgaaacctttgccccgcagcatcccgatcaatatctctcctggaaagccacctcggaacagtcagagcgtgttgacgccctggcggaagatccacggctggtgatcctgtgggcggggtatcccttctcgcgcgattacaacaagccgcgtggacatgcttttgctgtgaccgatgtgcgtgaaaccctgcgtaccggtgcgccgaaaaacgctgaagatggtccgctaccgatggcatgctggagttgtaaaagcccggatgtggcgcgtctgatccagaaagacggcgaagatggctacttccacggtaaatgggcgcgcggcggtccggaaatcgtcaacaacttaggttgtgccgattgccataacaccgcctctccagagttcgccaaaggcaaaccggagttaaccctttcccgtccgtatgcggctcgcgcgatggaagccattggtaaaccttttgagaaagccggacgtttcgaccagcaatcgatggtttgcggtcagtgccatgtggagtattacttcgacggcaaaaacaaagcggttaaattcccgtgggatgacggcatgaaagtcgaaaatatggagcagtattacgacaaaattgccttctctgactggactaactccctgtcgaaaacgccaatgctgaaagcgcagcacccggaatatgaaacctggacagcgggcattcacggtaaaaacaacgtgacctgtatcgactgccatatgccaaaagtgcagaacgccgaaggcaaactctacaccgaccataaaattggtaatccgtttgataacttcgcccagacttgtgcgaactgccatacccaggacaaagctgccttgcaaaaagtggtcgcggaacgtaagcagtcgattaacgacctgaaaatcaaggttgaagatcaactggttcacgctcacttcgaagcgaaagcagcgctggatgcaggcgcgacggaagctgaaatgaagccaattcaggacgatatccgtcatgcccagtggcgctgggatctggcgatcgcttcccacggcattcatatgcacgcaccggaagaaggtttacggatgctcggtacggcgatggataaagcggcggatgcacgcaccaaactggcgcgcctgctggcgaccaaaggcatcacccatgaaatccagatcccggatatctcaaccaaagagaaagcccagcaggccattggcctgaacatggaacaaatcaaggccgagaagcaggacttcatcaaaacggtgatcccgcagtgggaagaacaggcacgtaaaaacggtctgttaagccaataaccccgttccgcctcgcaaggggcggaaaacacaatggagtgaatatgagcgtattacgttcgttattaactgccggggtgctggcgtcgggcctgttgtggagcctgaacggaattaccgctacccctgcggcgcaggcatctgatgatcgctacgaagttacccagcagcgtaacccggatgccgcctgtctggactgtcataaaccagataccgaaggtatgcatggaaaacatgcttccgttatcaacccgaataacaaactgccggtcacctgcaccaactgtcacggccagccatcaccgcaacaccgcgaaggggtgaaagatgtgatgcgctttaacgagccgatgtacaaggttggagagcagaacagcgtctgtatgtcctgtcatctgccggaacagttgcaaaaagcgttctggccgcacgatgtccacgtaaccaaagtggcgtgcgccagctgccattccctgcatccacagcaagatacgatgcagacgttaagtgacaaaggacggattaagatttgcgtcgattgccacagcgatcagcgcaccaatccgaactttaacccggcgtctgttccgttgcttaaggagcagccatgacctggtctcgtcgccagtttctcaccggcgtcggcgtgctggcagccgtcagcggcaccgcagggcgcgtggtggcgaaaacgttgaatatcaatggggtgcgttacggcatggtgcatgacgagtcgttatgcatcggctgtaccgcctgtatggatgcttgtcgggaagtgaacaaggtgccggaaggcgtctcgcgcctgacgattattcgtagcgagccgcagggcgaatttcctgatgtgaaatatcgcttcttccgtaagtcttgccagcactgcgatcatgcgccgtgcgttgacgtctgcccgaccggtgcgtcttttcgcgatgctgccagtgggattgtcgatgttaatccggatctctgcgtcggttgtcagtactgcatcgccgcctgtccgtaccgcgtgcgctttatccatccggtcacgaagacggcggacaaatgcgatttctgccgtaagaccaatttgcaggccggtaagttgcccgcgtgcgttgaagcttgcccgaccaaggcgctgacgtttggcaatctggacgatcccaacagtgagatttcgcaactgctgcgccagaagcccacttaccgctacaagctggcgctgggaaccaaaccgaagctgtaccgcgtaccgtttaaatacggggaggtgagccaatgacgcagacttccgcatttcattttgaatcgctggtgtgggactggccgattgccatctacctgtttttgattggtatttctgctggtctggtgacgctggccgtgctgttacgtcgcttctacccgcaggcgggcggtgcagacagtacgttgctgcgcaccacgctgattgtcgggccgggcgcggtgatcctcggtctgttgatcctcgtcttccacctgacaagaccgtggaccttctggaagctgatgttccactacagttttacctcggtgatgtcgatgggggtgatgctgtttcagctctacatggtggtgctggtgctgtggctggcgaaaatctttgaacatgatttgcttgccctgcaacaacgctggttgccgaagctggggatcgtgcaaaaggttctgagcctgctgacgcccgttcatcgcggactggaaacattgatgctggtgctggcggtgttgttgggggcttataccggctttctgctgtcggcgctgaaatcgtatccgttcctcaataacccgatcctgccggtgctgttcctcttctccggcatctcgtccggtgcggcggtggcgctgatcgccatggcgatacgccaacgcagtaacccgcattccacggaagcgcagtttgtacaccgtatggaaatccctgtggtatggggtgaaatcttcctgctggtggcgttttttgtcggtctggcgctgggcgatgacggtaaagttcgtgcgctggtggcggcattaggtggcggtttctggacgtggtggttctggcttggtgtcgccgggctggggctgattgtgccaatgctgctcaaaccgtgggtcaatcgcagttccggcattcctgccgtgctggcggcgtgtggggccagtctggtcggcgtgttgatgctgcgctttttcattctctacgccggacagttgacggtggcgtaagccagaaaagaggtggtttctggacgtattccttcctgaagtcggttttctggcgttgttgttaagtctcggggtcaacgtgttgaccccgttgacggccttcgcgggagtgcggttgcgctggcctgccatgatgcgactcacttgcatcggcattctggcgcagttcgcgctcctgctgctcgcctttggcgtactgacgtattgttttctcatcagcgatttctcggtcatttatgtcgcgcaacatagctatagcctgctgtcgtgggaactcaagctggcagcggtgtggggcggccatgaaggttcgctgctgctttgggtgctgctgctttccgcctggagcgcgctgtttgcctggcattatcggcagcaaaccgatccgctatttccgctgacgttagccgttttatctctcatgctcgccgcactgctactgtttgtggtgctgtggtccgatcccttcgtgcggatatttccaccagcaatcgaaggccgcgatctcaatccgatgctgcaacatcccggtcttatctttcatccaccgctgctttaccttggctatggcggtttgatggtagcggcgagcgtggcgctggcgagtctactgcgcggcgagtttgatggtgcctgcgcccgaatttgctggcgctgggcgttacctggctggagtgcattaacggcggggatcatcctcggttcctggtgggcctactgcgaactcggctggggcggctggtggttctgggatccggtggaaaacgcctctttattaccctggctttctgccactgcgctgctgcacagtttgtccctgacacgccagcgggggattttttgccactggtcgctgttgctggcgatagttactctgatgctgtcgctgctgggcaccttaattgtccgttctggcattctggtttcggttcatgcgttcgcgctggataacgtccgcgccgtgccgttgttcagcctgtttgcactgattagccttgcgtctctggctctgtatggctggcgagcgcgggacggtggcccggcggtgcatttttcggggttatcgcgggaaatgttaatcctcgctacgctgttgctgttttgcgcagtgctactgatcgtgctggtgggaacgctttatccgatgatttacggcctgctgggctggggacgcctctccgttggcgcgccgtattttaaccgcgcgacgttaccgtttggtctgttgatgctggtggtgattgtgctggcgacgtttgtctctggcaaacgcgtgcagcttccggcgctggtagctcatgcgggcgtgctgttatttgccgctggggtcgtggtctccagcgtcagccgtcaggagatcagcctgaatttacagccgggtcagcaggtgacgctggcaggatacaccttccgttttgagtgcctcgatctacaagccaaaggcaattacaccagcgaaaaagcgatagtggcactgtttgaccatcagcaacgcattggtgaactgacgccggagcggcgtttttatgaagcacgccgtcaacaaatgatggaaccgtcaattcgctggaacggcatccatgactggtatgcggtcatgggggagaaaactgggccggatcgttacgcttttcgtttgtatgtacaaagcggtgtgcgctggatctgggggggaggattgttgatgattgcgggcgcattgttaagcggatggcgggggaagaagcgcgatgaataaagggcttctcacgctactgctgttatttacctgttttgcgcacgctcaggtcgtagacacctggcaattcgccaatccgcaacaacagcaacaggcgttaaatattgccagccagttacgttgtccgcagtgccagaatcaaaacttactggaatccaacgcgccggtggctgtcagtatgcgccatcaggtttacagcatggtggcggaggggaagaacgaagtcgaaatcattggctggatgaccgaacgctacggagattttgttcgctataacccaccgttaacgggtcagacgctggtgttatgggcgctgccagtggtgttgttactgctgatggcactgatcctctggcgagtgagggcgaagcgatgaaacagcccaaaataccggtgaaaatgctgacaacactcacgatattgatggtatttctctgtgtcggcagttatctgttaagcccaaaatggcaggcggtacgtgcggagtatcagcgtcagcgcgatccgctacatcagtttgccagccagcaaaccccggaagcgcagcttcaggcattgcaggataaaatccgcgctaatccacaaaacagcgaacagtgggcgttactgggcgagtactatctgtggcaaaacgattacagcaattcgttgctggcgtaccgtcaggcgttgcaactacgtggtgagaacgctgaactgtatgcggcgctggcgacggtgctttattaccaggccagccagcatatgaccgcccagactcgcgcaatgatcgacaaagccctcgcgctggacagtaatgaaatcaccgccctgatgctgctggcttccgatgcgtttatgcaggcgaactacgcgcaagccatcgaactatggcaaaaagtgatggatctcaactcaccgcgagttaaccgaacacagctggttgagtcgattaatatggcgaaattgttgcagcggagattggattaatcatctggtgatgaagattatgtcattgagctgcataaaaaataatcgaatgaacatatgccaaaaataatcactaatcagtattattgcagattaaacaaataaaaatctttccataacaaatggttattcattaatcctgccataaactcgcgttattatgcattaatgcagcgaaaagctctgttgttaaagggttgcgcaacataccgcgcaaatgatactgatcataagcgttaaaaaaatctacaaaccaacgcaacacaattcatgccctggcagtatgtcacgttctcgcgtttctgaacggggaacggcgctccattgaggaagtcattcatatgaaaaatataaaattcagcctggcctggcagattctgtttgctatggtgctgggcattctcctgggaagctacctgcactaccatagcgacagccgcgactggctggtcgtcaatttgctctctccggcgggtgatatcttcatccatctgattaaaatgattgttgtgccgattgtgatctccacgctggtggtgggtatcgcgggtgttggtgatgccaaacagctcgggcgtattggcgcgaaaaccattatctacttcgaggtgatcaccaccgtcgccatcattttggggatcactctggcgaacgtcttccagcccggtgccggggtggatatgtcgcagttggcgaccgtcgatatctcgaaatatcagagcactacggaagcggtacaaagcagttcccacggcattatgggcacgattttgtcgctggtgccgacgaacattgtggcgtcgatggcgaaaggcgaaatgctgccgatcatctttttctcggtgctgtttggtctggggctttcttccctgcccgcgacgcatcgtgaaccgctggtgaccgtgttccgctccatctctgaaaccatgtttaaagtgactcacatggtgatgcgttatgcaccggtgggtgtgtttgcgctgattgcggtgacggtggctaactttggtttctcgtctctgtggccactggcgaaactggtgctgctggtgcatttcgccattctgttcttcgcgctggtagtgctgggaattgtggcgcgcctgtgcgggttaagcgtctggatcctgattcgtattctgaaagatgagctgattctggcgtactccactgccagctctgaaagcgtgctgccgcgaattattgagaagatggaagcctacggagcaccggtgtcgatcaccagtttcgtggtgccgaccggttactcttttaaccttgatggttcgacgctgtatcaaagtattgccgctatcttcatcgcgcagttgtatggcattgacctgtccatctggcaggaaatcattctggtgctgacgctgatggtgacctcgaaagggattgctggcgtgcctggcgtgtcgtttgtggtgttgctggcaacgctgggtagcgtaggtattccgctggaaggtctggcgtttattgctggtgttgaccgtatcctcgacatggcgcgtactgcgctgaacgtggtgggtaatgcgctggcggtgctggtgattgccaagtgggaacacaaatttgaccgtaagaaagcgctggcttatgagcgtgaagtgctgggcaaatttgataaaactgcggatcaataattgaagattgccggggatatccacccggcaatgtgtgaatgcctgatgcgacgcttgccgcgtcttatcaggcctacgccagacagcgcaatagcctgatttagcgtgattttgtaggtcggataaggcgtttatgccgcatccgacatcaacgcctgatgcgacgcttaacgcgtcttatcaggcctacgccagacagcgcaatagcctgatttagcgtgattttgtaggtcggataaggcgtttacgccgcatccgacatcaacgcctgatgcgacgcttgccgcgtcttatcaggcctacgccagacagcgcaatagcctgatttagcgtgattttgtaggtcggataaggcgtttatgccgcatccgacatcaacgcctgatgcgacgcttaacgcgtcttatcaggcctacgccagacagcgcaatagcctgatttagcgtgattttgtaggtcggataaggcgtttatgccgcatccgacatcaacgcctgatgcgacgcttaacgcgtcttatcaggcctacgccagacagcgcaatagcctgatttagcgtgattttgtaggtcggataaggcgtttaccgcatccgacatcaatgcctgatgcgacgcttgccgcgtcttatcaggcctatcttaaccgttggttaatttttcaaactcttcacacccggtatcaaacccttccatacagctcaggttcaaccagtgcagcgccttttgcttgttcttctcgataaaaccttcttcaccgtttaagaacatcattcccgcccagtactcggaataaccggttcgggaaattgcagagctgcgtttgaaataccaggttgccttgtcatcgtcggccttaatgcccacgccgttggcgtaaatcaaaccaagcagcatttgggcatcgacggcagagtcgttctccagatcttccgaggcgttttctaacagcgaaattgcctttggataatccggtttacccgcttgagtatttaccagaatatgcgccagcgttacttcaccttctttactgcccgcttgcgccgctttctctgcaagaacttttgcttgtggatagtccagactgaccggattggtgattttgatctgcgccagcagcgcgcaggcatcagcatcaccgctgtcggcggctttctgtgcccaatattcggctttgctcaaatcgccggagctaaaccagctgtcggcaagaaaatattgtgcgcgtcggtccccggcctctgctgcctttaaatactggctgccaggctcggagtcgttggcgtgggcaaagaatgtcaaaaacaacatcaatgcgataatttttttcattttgataatacgattgggtagggagtaaccagtataaagagttcgaatggataaaaaaacagcctccgaaaggaggctgtagaaaggacggtattacgccagtgccgcttcgcgcaggcgagttttcaacttgttgtactcgtcaatcacgtactgctcggcggcgcgctgatcggcgatcggctcgacgcgaacggcgcagtatttgtactccggcgttttcgtaatcgggcttaagttttcggtaaccagctcgttacaggcaccaatccaccactggtaggtcatgtaaatcgcccctttgttcggacgatcgctgacctgcgcacgggtgataattttgcctttacgcgagtgcacccaaaccaatgcctcatcttcaatacccagacgtttggcgtcttcggtattgatttgtgcgtagccaggttcatcagccagcgccgccagtgccgcacagttaccggtcatcgaacggcaagagtagtgaccaacttcacgcaccgttgacagtaccatcgggtactcgtcggtgagtttgtcgattggcgctacccagtcgcaggtgaagaactgcgccagaccgttcggggtatcaaacttctctttaaacagataagaagtcccctgatcggcatctgaagtatcgcggcaaggccactgaatgaagcccagttcgcccattttctcgtaagtcgcaccgtagaaatccgggcacagatgacgcaactcatcccagatctcctgggtgttgttgtagtgcatcggataacccatacgggtggcgatttcactgatgatttgccagtccgttttcagatcccatttcggttcaaccgccttgaagaaacgctggaagccacggtcagccgcagtaaacacgccttcatgctcgccccacgacgttgacggtaaaataacatccgccgccgacgcggttttggtcataaagatgtcctgaacgataaccagttccagatcttcaaaggctttacgtactgccgacagctccgcgtcagtttgtagcggatcttcgcccataatgtacgcggcacgcacttcgccatgcgctgcgcggtgcggcagctcgctgatgcgatagccggtatgcgctggcaggctttccacgccccaggctttggcgaatttctcgcggttagccggatctttcacgtactggtatcccggatacgtatccggcagcgcgcccatatcgcaggcaccctgaacgttgttctgaccacgaaccgggttaacacccgcatgcggcttaccgaggttaccggtcagcatcgcgaggctggtcagagaacgcacggtttccacgccctggtagaactgggttacacccatgccccacaggatggcggcgcttttcgcctgggcatacatccgtgccgcctgacgaatctcactggcgctgacgccggtgatatcttcaaccgactccggcgtgtagccttcaacgattttacgatactcttcaaagccttctgtacgtgaagcgacgaacgctttgtcgtacagattttcttcaataatgacatggcccatcgcattcaacagcgcgatgttcgagccgtttttcagtgcaatgtgcatgtcagcaatgcgcgcggtttcaattttgcgcggatcgcagacgataattttcgccccgttacgtttagcgttaattacgtgattcgccacgattgggtgggaatccgccgggttgtacccgaaaacgaacactaaatcggtattatcaatttcgttaatagcattgctcattgcgccattaccgaccgattggtgcagacctgcaaccgatgggccgtgtcagacacgagcgcagcagtcaacgttattggtaccaataacggcgcgcgcaaatttttgcattacatagttggtttcgttacccgtaccacgcgaggagccggtcgtctggatggcatccggaccgtacttctctttgatggcgctcaggcgctcggcaacgtaattcagtgcctcatcccaggaaacaggttcgagtttgccgccacgctggcgacggatcatgggggttttcaggcgcggggtcaggatctgggtatcgttaatgaagtcccagccataataacccttcagacacagggtaccctggttggttttcccctgcgctgcctccgcccggacgattttgccgttatcgacgaccaggttgattttgcaacctgatgcgcaataggggcaaaccgtgacgacttttttcatcggtctcgctccagttaatcaaatcacgcatacgcgctctcgactacagtatgcatcttttatgccacattttatgtggggtcattccctgatattacgggcactatttattcaaaactctgacgaaaaacaggctgtcgtcagttttgacgtgacgaaacgaaataccgcgtgacagccatcacgcggcagacattttattttttctcgacgacgggacctgcctgatacccgccgcccagcgatttcatcaactgaatgctttggatcacccggcggctgtccagcatcagtaatgacatctcttcggcaagcactggcaaccgggcttcggtggcctgtaagcggctggttaagccgcgctgataggcggcctcggcagcgcgctgggtaaagcgcgtggcttccacgcgttcagcctgcatttctcgctcgtcgttgagcgtttgcagacgcgtgccgttgacggcaacgtcacgcaccgcgttcagtactgactggttgtaacgttcaatcatcatgttgctggcggcgcgcgtgccttcgagattggcattcaaccgtccaccgtcaaacagcggcaatttcagacccgggatgaagttgaactggcgactggtttttttgaataaggtatgcagatggatggagtccagaccgaaaaacgctttgatatcaaagctcggatagaacaacgcccgcgcggaatccacctgatctaatgacgcctgaacataccagcgcatggcttgcagatccgggcgtctggcgagcaactcataagagagtgtcgccggaatgccggtctggacttgcggtaatgccaccggtctgatctccggcatatcgctggctcccgcgccaatcaatgcacgcagagattctcgcgtttcggtgatttgccctttgacggcaacaatttgtttatcgaccgccagaatctgtgcccgcgcgccgtggaaaggcacttgcgcttccagaccgtgcgccactttactctggtgcgctttcaccgcgtaatcaatcacatcgtgagtttgttctaacagatcgagcatctgatagctggcctgcatactgtaataaagctgcgctacgcccgtggccagcgatagctctactgctgcggtttctgccagcgcggcattatgcgcgccaatggcggcggcaaccgctgagcgatgcacaccccacaaatcaagatccagtccggcaaacaaacctactgtggcttccgtatagtacggcccgtccatacccagtgctggcgcatccattgaataagggcttaaaaagccgttcgccgagacacgttggcggttgagcatccctaacgctgcgacctgtaattgtgaaccggcatctaacaaatcggcctgggactgcgctttttcttcccgcagtttcgcttcggcgagggtgtgtgaaccacttagcgtccgttggatcagcgcatccagctgcgggtcattgagttgtttccaccactgcgcctgcggccagccggagctggcaagatgaatatcgtcggccagtttgatttgttccggtttgagctgttgatgaggtgcagaatccttacgtaccagggcacagccggaaatcagcgtcgtgctgccgagaatgctgcacaacagcagacgtgaaagttgacgattgatcattgcgtggctccttgtgcctgttccgtggcgggcgttaatgccggggctgtccagtctggcaagcgggcgaaaagctggcagacgtgttgctcctgttttaataaggtgggcaggatggcctgagaggcgggtgtctcttcaagcgttatttgaggagaacggctgagtgcggttgccagaccggcagcgtatttctccagggcgtcggcaaactgacctgctctgtccggctgtagtgcgttatccagcgcctgcgccgagttccaggtggcatcccaggcgtgaagaagatcgcggccctgacgaataaccgtttgcgaacgttcaatcagtaatgcgcgttcttcgctgtccagttgacgctccagcgccacgcgttggcacatctcttcacaggcattaaacgccgcatgcagaccgatacgaatttgcagataagtgcgcagagccgtgacttcctgctggcgtgggatccgcattactttacttaacatacccagcgtgccagccagtttttgcggcagtgtgcgcgcttcactttcaggccagacaaaggtgtaaatcaccgcggacaccacggtaccaatgatgatacccagggcgcgatcgcgaatttccaccaggtcgtacactgggccaaaaacgttttcgagcgtggcgagcgcgaaggtgaccaccatctgtgtgccgatataagaagagcgttcagagctggtggcaatccatgcgcccaacaggaaaatcggtgccagcacaaacagcaattcgacaatattgtccagccagggcatgaccagtagcgtgaataacagcgccagaatcgcgccgcaaaaggccccgccaaaacgcagcaccatcttctggtacgacgaaccgacatttgggttagcgacgatcacgcatgtcagcatacaggtgtgaatgccttcccagtccacgccgctgtaaaaggtgtaacagatcaaacaggcgagcagcgtttttaccgcgtagcgcatatagtctggattggtaaaagcatcggcggccattgatggcggtttggctgcgggcgttggcggcgtattcgggtccatctgacccagttgtaacaacgtctggcagatattctccaggttacattcccgtgccgccatcgcttcactttcactgatccgccagtcgctttgccagcactgaccttcagcaacggcatgctgcagcttgttgatttctgaagctaatttttgtcggaattcaataattgcctgagaatcagcaaaagaggtgggatcgtagcgattcagcgtcgagtaaatgtaggttaccgttgccacgcagctttgccaccatgcgttttgagttcgccagttggcatcgtccgcgaggcaaaagacattgagtttttgtagcgccagcgcctctctttcaatccgcgtttcgggtagcggtgcgaggctgtctgtcaggtgactaatggcatcatcaagccgatcattaagcgcctgatgcatttgcgaaatggcacgactgggaaaccacagcacgccgattaacgtcatcagcaaggttggatagaggccaacaacgatacaccacagcgttaagcgcacgaccacttccggatagtcgagcatggcggggaaggtttgcccgtaaatagcgacaatggcgacggcgaaaaagaccagccccaagcgatgggtgcgcatcaaaaacatgcagcccatcaggatcggtccggcgatgatcaatcggatcaacggttcgccgtatgaccatttgtagatcaaaaacaggctgccgatctccagcaccgtggcaaccacaaacaagatcgcgacaaatttggtgtaaaacgcgttcgactgaataccgtaaaacagcactgccagcgataacgccacaaaagggatctcaaaggtcatcgagatcagaatcaccagcaggcagcctacccagagttgcacggtctgcggcacgcgacctggtcgccgctcgcttaactcttcatgaaagaacgccagcagcctgaccaccggtaatggcagggagttgagcgcgctcattattgcggctcaagattagcgactgccgaagcgccgatgcggaacatttccgggtcaggtttatcgaccatgattttgaccggaaaacgctgggcaacgcggacccagttaatagaacgagacactttcggcaggccgcccagcaccaggccgccgtcatccggtagcacgccgtagccaatcgaatccactttaccctcgaaggttttgccgctgtcactcatcaggcgaatcgttgcgggtgtacctgagcgaatatttttcagatcggtttcgcggaagttggcgatcacataccagtgacgagtgtcgattagggtaaaaatagggcgcatggcagaagcaaattgcccgacggaggttttgagggaaatgacccggccatcaaacggcgcgcgaacggtcgccatttccagatgcagtttggtcagggcaatatccgcttcgaccgccgcacgctgggcaactaatgcatccacgccgctgacggcgctggcggctgactgcgcctgtaacaatacggcattaagatccgcttctgcggcgcgctgcgccgttcttgcacggtcaacatcttccgctgagacaaaaccttctttcagtaatggctcggtgcggcgtaatgtatctgtggcctgtttcgcggcggcacgggctttttctaccgtggcattaaccgagtcggcaccaaactgttgcgcgtcaacgctacgctgggtgagcataatttgcttatccagcgccgcgagggaggcttcagctttcgccagattggcttcgtacgggcgcgggtcgatgcggaacagcaaatcgccctgtttgactgcctggttgtcggtgaccgccagttctacaatgcggccgctgacttccggtaccacatcaatggtatctgctgacgcgtaagcgtcattagttgatggcgcactgtctacgcgccagataacgaaaacaagggcaaccagcgccaacgcaaccactaacagagcagggaatttactgcgaggagcttttttcggcgtactttccatgagcgcgtctcaaatagattagaaaaatgccagccagaacagcatggcgtagagagcaaaaagggcggtataaataattccgacaaatgccagattgatatttgcccgctgaataactcgcctcgtgatgagcgtcaaaataaggctggcaatggcgcagaaaaaccagctgggataataagcgccgatcaccgggattgccggagataatgagcatcccgaaaccatgaagacgggaattatccaggctgtttttttgagttgcatcgccatgcgagagagaactgttggcatattaaatacatcctgtctgctgcgaacaatatctgtagtgaatatcaatatccattgaaggcgtcagtatggctattttcttgatgaataaaaatagctttattcagccaccgcattcataacttatatattttatttattaattggctgtatatatttttaaaataaatacttttgggggcttcagcgcccccaaaagcgagtgacattaatttggggttacgatattcacccacaaatcgaaattatccagacaggcgataatttcttccagtttcgcgccattgccaataattttggctttcttcgcttttaccagatccgccattttggcttgtccggtcagcacggcgtgcagatcttcacggctgatgtagaaagaggcgtcggcttgcggttgcagcgttttccggtagttaagcacgctatcgttcagcgtcaggttgaggttatcgccgttgctcatattgaagttcaggctgatatttttacccgcagctttcgcgctatcgaggcgaacggccataaagtcgaacagcatttcgaccgacatcccgcgaatggtgtccggggaaccggtggtgccgtggctgaacttatgcaccccttcgcgcagctctttcgcgccggtcaggtagaaaccgcgccatgtggcggactcggcctgatagcccagctgttcaaagttattcgcttgcagattcttcgcgacctggtcacccgggttggcggcaatcacctgtttcagcagttctgccgaccagcggtaatcaccttgcttgttcgcttcttgcgccaggttgatgacacgggcagaaccgcccagcgcctgcacgtaacgtttacccatctccacctgaccatacggatgcaggttagccgggttaccgtcgtaatagccaagatagaagttatacaccgcgcgggcgttgtggctgacagaaccgtaatagccgcggctggcccagttattggcaagtgcaggcggcagcttaatcatgtcgccgatttcattcatggtgtagccctggttcgccaggtgcagggtctggtcgtgaatgtacttgatggtatcgcggtatttaccaatataatcattgatatgcttattgccccagaccggccaggtgtgcggcataaacagcacttccgcgtcgttaccccacatatccagcgtttcgttcagatactcggtccacttgctggtgtcgcgggttttcgcgccgcgcagagtgtagaagttgtgcagggtatgcgtggcgttctcggcggtacacagggctttcagggccggaatatagaagtgcatttcggctggcgcttcgctacctggggtcatcaggaagtcaaactccaggccgtcgataatcatcttctcgccagttctgacgatagttttcgtcggtgcaataatgctcgggtcgcccgttgccagcgtcacgccaaggccattacccacattgccttgcgcgttgtgcggcagtaacagaccgtaagagtagagcgcacggcggctcatgatgttacccgccagcacgttttcgctgatggcttcgtccataaagcctgcaggggcaatcacctgaactttgccggatttaacatcggcttcagagataatgcctttcacgccaccatagtggtcggtgtggctgtgagtgtagataacggcaacaatcggtttttgcggacgatgctggaagtaaaggtcaagtgcggcttttgcggcaggcggcgtcaccagcgggtcgataacaataatgcctttctcgccctcaacgaacgtaatgttagagatatcctggccgcgcacctgatacattttatcggtgactttgaacaggccagaaataccgttgatttgcgactgacgccacaggctggggtttacggtttccggcgctgcggcattaatatcaaatttgtaatcgtccgcgcggtagtaaactttaccgttcgcatcacgcagaataccttcatccagcagcggggcgataaatccacgctgggcatcgtcaaaatcctgacgatcgctaaacggtaatgatttggcgtaattctgattaacctgttgggtatattgagtggcggctttcgcttcctctttcgcgttagcggtatttaccatcatgccgctggcggcagttaacgcaataacaatcctgctcaaacggaataaccgagagttattcatataaatctccatttatcatttatgtcgtaaatatgtaatccatgcaaaatacgtcatttaaagctggcgttatcataattgggaaattgcgactttaataagtggaagtgtgagcggaacgcgccattttattaggcatttgtgctgaagagggaaaattacagtaaaactatcattgcagaaaataatatgagtcgttttatgtgtttattatatatattgtacctgtcgttggcacagcgggacattgcgctactgtgccaacgttttactcatggggctttagcacagaactgtggcaaaaaacgttgatgcgccaatattgctgcaccctgagcgccattaaagtcagaagatgaggcggcaataaagcgcacgacctgatgcggcagtggacggcgcaggtacttttgggtcatggcaacgagagtctcgcgtgggaaggcgggcatatccatcacgccaccgcccaggatcaccgcatcgggatcgaacagattaatgctggtggcaatggcccgtgccgcgttttcaagcagactctggacgaaaggggcgttttccgcatggacgaaaagatcgcgcaatgggtaatttcggggctgttgttcgtaccagcgtcttagcgccattccagagcaattggtttccaggcacccaggattgccacacgcgcagtgttgggtcatatctcccagggggatatgacccagttcgcctgccacaccgtgtgcacccgtccacggcgcaccgttcatccacactgcgaaccccatccccgtaccgagataggccgccagaaccagttgttgcgtaaggcggttttctactacgtcccaggagagttgcaggttaacgtcgcgggaaaactcaaccggacaattcagcgtattttcgagcttatcggcgagatcatataaatccgccgctgttaacggcaggttaggcgtagaaataatggtgcgtttatctttactgaccagcgccggaaatcccatcaccagaccatgacagcgagcgttaaagcgcctgagttgctcgtcaatcatttcgccgatacccgacaccaggccgggagcaatgacttctgcggtccgctttttttcgcagtgtagcgtttcaccttctgctgtccgcagacaaaagcggatatgcgttgcccccatatccacgcccgctacgacgttatgctgtttttgcatgaggctgtacctcgctttttgcagccagaatctgcgcggtcataattctccatgcttcgtcgatattttccgcatgattaaacaggccggaagtgccgacgataaagacatccgcccctgccgccatcagtttttcgtaagttgcctggttgcaggaaccgtccacctcaatttcgtactccagaccttctcgttcacgccatgccttcagttcggcaagtttatccagcatttcaggaatgaacggttgtccggcaaagccgggatcgacagtcatgaccgtaattttatcggccttatggatatagtatttcatggcctcaactggcgtctccgggttaaggatcagccccactttcatgtcatgacggcggatttcatcaatcaggcggaacgcctggccgttgatggtttccggatgcagagtgatgaaatctgctcccgcacgcgccagttgagcaatgtaatcctgcggccgcgtcaccatcagatgacagtcgagcggtttagttgccagttttttaacctgacttacgaagaacggtgagagtgtcagattggggacaaagtgaccgtccatgatatcgatgtggaagtaatcggcatggctgtcgataaattcgatctgttctttaaatttcagcagatccatacacattaacgagggggagattttcatgttcaattccttacttactgataagacggtcaagggcgacagccgcgataattaatccgcccatcaccaccagttggtaataggtttgtacctgcaaaatattcagaccgttgttgatggtgccgatgatcaacccgccaatcaccacagagaaaatgcgccccttgccgccgaagaaactggtgccgccaatgatggcgctggcaatggcataggtttcaaaacccataccggcaagcggttctgcggcaccgagtcgtgcagttgagacgacgcctgccagacctgcacaaacaccggagatgataaacaccaccaggatgtggaatttcacgtcaatcccggaatagaacgccgaatttttgttgccgcccagtgcgtagatgttgcgcccgagccgcatacgcgttgtcagaaaccaaaggatgagcgcgacaattagtgagaagataacggggacaggtatcccaattacgctggcggcaaagaagttcacgaagtcaaatgagaagccgtataccgagttggcatcggagatcaccagcgtgatcccacggaaaatcgcgttggtgccaagggtgatgatgaacgggtgtagccccgtccagttgaccaggcagccgttgatcgcccccagtgcgccgccaaccagtacaccgccaatcatcgctgcgagaaacgggtcaacacctgccaacatcagtttggcggtcaccataccggaaagcgccagaatcgcgccaaccgagaggtcgataccagcgaccaggatagcgaaaaactcgcccatgccgatcaataccgtcacggagctttgaacaaaaatctgggtaatattattggtggtcagaaaatattctggtgacagcgaaccaaagatggcgacgatgatcgccaggataaaaaaggtgccgtatttatcccagaacagcgcaaagttgaacggtttcttctcgctcgcttcgctttttactcttgtggtaaagcccatgccataatctcctcttcgctcatgtcatcgcgattcgtcaggatttgcgtcagtcgtccttcgcagaacacggcgatgcggtcgcagacggtgataatttcaggtagttcagatgacaccatcaggatgacttttccgtcgtccgccagttggcgcatcactttgtaaatttcggctttcgcgccaacgtcgatgccgcgggtaggttcatcgaaaataatcacttccgggcaacagcacagccatttggagatcaggactttctgctgatttcccccggagagttcggtgatattctggtttaccgaatgacatttcagcgccagcagttcgcgttgattttcagcggtacgttgctcgtcaacttcatgaaacaagcccatcgcgcctttatagccgccgtctttcagactgcggctgatcgccatgttctgagcgatggaaaagttggggaaaaaaccgttatcccggcggctttcagtgatgtaagccatcccttttttcacggcatccaggggtgaacgtggagagatatctttgccattaagacggatttctccgccagcgcgtttatccacgccaaacagacaattcatcagttcagtacgtccggaaccgaccagtccggcaaagcctaatatttctccccggcagacgctaaatgagatatcccggaccttttttctgtcacgactggtgacgttccgcacctcaaaaaccgtttcgtgcgcaaggttgctgacattctccttcatcgcgttaaaacggttttgcagttcgcggcctaccatcagacggacgatatcgtcatttgacacatcgcttactatgccgctgcaaacgctgctgccgtctttcatcaccgtatagcggtcgcaaatacggcgaatttccgccaacttatgcgagatatagacgatggccgtaccctctttacgcaactgattcatgatcagaaacagatagtccacctctttattggtgagtgaggaggtgggttcatccatgatgatgactttggcatcgagcatcagcgttttggcaatttctagcatctgcttgtggctgatagataaattcgccactttctcatctagatcaactttcaagcccacgcgtaataacatcatggcggcgcggacacgcatttctcgccagtcgataatattgacgccacagatttttttcgtcagatgacgaccaatatataaattttccagtacggttaattcatcaataacgctgagttcctgataaataatcccgataccgagttgtgccgctaatttatgatccagcttgttatagctaatgttattaatggtaatggtgcctttggtcggctcatgtattccggataaaactttcattagcgtggatttacccgcgccattttctcctagtaatgcatgtatttcaccaggataaaccgttaaattaaccgactttaatgcgtgaaccggaccaaaggacttgccgatccccgccatcgatatatatggcgtggccataaataacctctctgcacgaaatatcgtattattgcctgatggctacatttatcaggtctacgttcaggttattttgttggccggataagacacttcattagcatcatcatccggcatcattcagttttattgagtgaccaggattgaatcgaccagtttaaattccggtgctttatccagcgggataaccttgccggatttctcagcgtcaaccatcagcttcagacccgttgcgccgatatccgccgggttctgggcaaccgtcgcggtcatttgtccggcttccaccattttgcgggcttccggaatgccatctgtaccgacgaccagcacttttcccgtttttccggcgtttgcgactgcctgagcaacacccattgccatcgtgtcattcgcgcaatagatcgctttaatattcggattacgttgcaacacgttagtggcgacatccagtgctttaatgcggtcccagtcggcaggctggctggcgacaagcttgatctggcttgcttttttgaaggcttcggtggcaccattacgacgcgcttcaccggaggcgttaccggctttaccctcaatgattgcgacttcaccaccttcagcgcccaatttgtcaataatgaacgacgcgcctttcgccccgacagcaacgttatcggtggtgacaaaagcttccacattgccgccagcttttttcagattatccatgtcgattttttcatcgagattaaccagataaatgccttttttccatgcgcgggcgacaggcatgaccagattcactgaggataatggagcgaaggcgatacctttgtaatttttattactgagatcttcaaataactgcaattgagattgaaaatcgccttctgaaggagaggcaaaaatatcaacgctgacgcccagtgtttttgcttcatcttcaatgccttttttcatatctacccaaaatgggttggagagggttttcaatacgacagcatattcggcggcagcaaaagcgctggttgacaacattaagcccacgagtgtgccgctgaaatatttcagatatttattcataataatgttctcacggtaaggggacaggtaactccgcgatggcggaattacctttttcttatttcagcgcgcctggtgagaagaaatcaacaattgcgccggttttttgcatattaatattagcttgttcaatgttgagctgggcgacagagacaaaaaaagcgtccagcaaagttagttgtaatattcttgccgaggcattacgacctaataacggcgtttccggggctggtgagcaaataatataatcggccagtttcgctatcggtgaatggtagctatgggttatacaaataatctttgccccgttcttttttgccagttctacggccgcttttacatcactggttcgcccggaatgggtcactaccagcacaacatctccttcctgtaacaacgaagcggacatcatcatgatgtgagcatcaggataggcctgacagcgtacgccaatgcgcaagaacttgtgctgtacatcagcacagatagcatttgatcctccggcaccgtacaaatcccgctgtctggcctgatagaaaaagcgggcggcacggtggatctcatcaacgttgacgatcgactgaccttccataatggtgcgtaaagtgatgttaaataccttattcaccacatcctgcggcgcttcatcaaaagccaactcggaaggcaatacctgttctgactgagaaaaataatcttccagcgcactgcgtaagttacgaaagccgctaaaccccagcagctttgataccttaactatcatcgcttcagataccgccagagcttctgcgacatctttaattgcgggtgcacaactcaggttaccgggtttgagtaaccactccacgatgcggctttcattttctgtcattccttcctgcttcattcgcaggtaaggcgctaaccctataccgttcggaagcgctgaatcaaactctgactggctcatcacgttctcttgtccttgaattgaagacgccactatatcaccacagcaagaacagaaaagatgctggcgacttcacaaaaaaataaaatttataaagtttattttattgtgaacaatggcgagtggcttaaaattttatttcatttaattagtttaaaaacatgatgttatttgtttttctggttttttagatgatagatgttgctggatggtgagtgtctttaacgctattgcgctgtcagatgtaactctgtaaaacagatcaggaaggcgtaattcatcgattttgggtgtttttaattcattaacatcacaaatgttttttgattgtgaagttttgcacggacggggaagatgaatgaaaaagattgcatttggctgtgatcatgtcggtttcattttaaaacatgaaatagtggcacatttagttgagcgtggcgttgaagtgattgataaaggaacctggtcgtcagagcgtactgattatccacattacgccagtcaagtcgcactggctgttgctggcggagaggttgatggcgggattttgatttgtggtactggcgtcggtatttcgatagcggcgaacaagtttgccggaattcgcgcggtcgtctgtagcgaaccttattccgcgcaactttcgcggcagcataacgacaccaacgtgctggcttttggttcacgagtggttggcctcgaactggcaaaaatgattgtggatgcgtggctgggcgcacagtacgaaggcggtcgtcatcaacaacgcgtggaggcgattacggcaatagagcagcggagaaattgagattcatccactacttgcatggatgagtaatgattaatgtggatagagtttctttttgaggttggctaatgaaacgctttccgctatttcttttattcaccctgctcacgctgtccaccgttccggcccaggccgatattatcgacgacaccattggcaatattcagcaggcgattaatgacgcttataaccctgaccgtgggcgagactatgaagattcgcgcgacgacggctggcagcgtgaagtgagcgacgatcggcgcagacaatatgacgaccgccgccgccagtttgaagatcgccgcaggcagctggacgatcgccagcgccagcttgatcaggagcgtcggcaactggaggatgaagagcggagaatggaagatgagtatgggcgatgaggttgggtatggagcaggcatcgcccctcaccccaatggggagagggagaaaacgagcgcaatattcaatatcgagcacaatcggtcccctcgcccctctggggagagggttagggtgagggggccagcgcgcacattccctctcatcacgccaccccaatctccatcccatcaaaccccacctcaaaccctgacggtagtgcgttttccatcagccacgcatcaaactggtggctgatatgggtcagaatcacccgtggcgagcggataacctgattcagcgcaagcacggtatttaaatcacagtgattacgcggtgcatccgcgcgcggcgggtgactgcaatccatcaccattacctgcggctgattattgcgtaaaaatttcagcgttttttccggcaagcctgcggtgtcagacagccacgccacccggctgtgtgccgtttccagcagataaccgaaggtcagttttgagtggttgagcggcaggggcgtgacctgtaacccctgcaaatcaaacaccacaaacggttccaccgtgtggctgaaatcaagcaggcccggatgtttaaacagatcgtcgcagccctgttcatccggcgggccgtaaaccgggatcggatcgccaacgccccagcgcagcggaaacagcccctggacgtgatccatatgataatgcgtcagcaaaaactgctggaacgatccgggcgaccagcgatcggcgagatcgtgcagcccggcgtcgatcagggtgattgcgtcgttaaacttcactacgccgctgcacggttggcggcgatactgcggcgagcgccgcgctctggcgcaggccgcacactcgcagccccatgccggaacgccctgtgcgccgccggtgccggtgagcgtgagggtcaggctcatgttacagcgccttggtgaagcggaagtggctctgctcgtagccttcgcgcagatagaaacggtgcgcgtcgtggcgcttcacgttggtcgaaagttcggtcatttcggccccggcctggcgggcttcttcttctgcccacgccagtaacttactgccgacgttcagaccgcgcgcctgcggcattaccaccaactcctgaatttcgccgatccagttgacatgatgcagatgaaactgcaaatgcaggccgatcatgccgacaacttcgccatcaagcagcgccagatggtagcgcatgtttgggtcgcgcagattggcgttaaaacccacgcgaaacgcgtggtggtcaaactccgcctgttttagctcacaaatcagcgcgtaaaccgcgtcggtgtcgtactgcgtggccgggcgaagctcacaagcaggcatggtgtttctccttctgatggatcagcgtcagcagcgtgtcgaccgactggcgcaggctgccgtcattgttgagcgtatggcaatcctgtggagtatagcgggcggcgcgcgccaggcgggcgttaatttcactggcgttttcacggccacggttttccaggcgctggcggaggatctccggcgaaacctgtaaacagacgggcagcagcgccgattgatagcgcgcccgcgcctgcggcagatgggcgcgtgagccgttgaccagcacgtcgaatccggcgtgcagccagagatcaatctcgacgccgacgccataatacagaccgttagcgtgccagcttaaggccaacagattttgccccgcgcgggtaaaaaactcctgctcgctcagggcgatatggttttcacttccggcgctggcatcgcgcgtgatgtagcgatgcgccaccagtaactgagtttgttcccgcaggcggagttccgccagcaggctgtctttcccggagccggacggccccattaaccaaatcagttttcccatcatcagaacacccttttaccctgacgccagacgtggtcgatatgaatatgattgtccttgcgatgcgccagcaccaggtcggcgcgtttgccctcgccaatcaccccgcgatcctggagattaagcgcctgcgctggatttttagtcaccagcttcaccgcctgcggcagcgtaaagcggttgctctggtcatcggcgacgcgaaatgccgcatcgagcaggctggcggggtagtagtcggaagagaggatatccagcaggccaagctgcgccagttcactggccgccacgttgccggagtgcgagccgccgcgcacaatattcggcgcgcccatcagcacgttcatgccatgcttgcgcgaggcttccgccgcttcgaacgtggtgggaaattcggcgatcacgctgccaagctggtgagattcagcaacgtgggcgtgggtggcgtcatcgtggctggcaagcgcaatttttcgcgcgcggcacagggcggcgatggattcgcgattcggctgcgaccagcgtgcggcgagcgccagttgctcttcttcgtactgctgcatctgcgcatcagtgagggagtatttgccctgataatattcgcgatacttctcgcggttggcgaactggcgctggcccggcgagtggtccatcagcgacaccagcgtcaccggctcgcgctgcaccagtttttcaaacagcggcagcgtggtgtgatgcggcagttcgcagcgcagatgcagacggtgctcggcgcggttgacgccgcgtttctgcgtctcttcgatggcgttgatcatcttctccagattctccagccgatcgccgccgtcgcgcacgtcgccaattgccacggcatccagtacggtggtgatgccgctcgccaccatcagcgcgtcgtggctgctcatcgccgagtgggcaggccagtcaactttcgggcgcggggtgaagaatttatccagattatcggtatgcagctcaatcagccccggcagcagccagccgccttcgccgtccatcgcctccggcaggcggctctggctttcggcaaaggcgcggatttcgccgttctgcacctccagcgaaccgcttaccacctcgttttccagcaccagcttaacgttattgataatcatgaagaggctcccattgggtgcaggcggtcggcgacgtcattacgtacagcttcgtcatggaagatgcctacgatggctgcgccacgggttttggcttcgcgaatcagttccaccaccgcggcgctgtttttggcgtccagcgaggcggtaggttcgtcaagcagcagaatggggtagtcgacgataaagccgcgggcgatgttgacgcgctgctgttcgccaccggaaaatgtcgatggtgccaggtgccacaggcgttccggcacgttcaggcgggtgagaagacgcgcggctttagcggcgcaggcttcacgcggaacgccggtatcgagcagcggctgcatcaccacttccagtgctgagatacgcgggatgacgcgcagaaactggctcacccagccgacggtggttttgcggatttccaccactttgcgcgctggcgcggtgaccaggtctacccactcgtcaccgtgtttgatctggatttgaccttcgtcgggcagatagttggcgtacagcgagcgtagcagagttgatttgccgctgccggaatggccgtggagcaccacgcattcgcccgcgttgacggtgagcgaggcgcgattgaggacgggcaggcgcacgccgttttgctggtgcaggatgaaggttttactgacgttttgtacgttaatcatttttcgcctcgtggttcgggtgtcggatgcgacgctgacgcgtcttatccgacctacggggagcgcatttgtaggccggataaggcgtttacgccgcatccggcaccggctcaattctgcaaaaccgatgacaccagcagctgtgtatacggatgatgcgggtcgtcgagcacgcggtcggttaacccactctccaccacttgcccctgcttcatcaccagcaaacggtccgccagcaggcgggcgacgcctaaatcatgggtgacaatcaccaccgcgaggttcagctccaccaccaggccgcgcagcaggtcgagcaggcgggcctgcaccgacacatccagcccgccggtcggttcatccataaacaccagcttcggatgcgtcaccaggttgcgggcaatctgcaaacgctgctgcataccgccggaaaaggtggtcggcaggtcgtcgatccggttggcgggaatctccacctcttccagccacttctgcgcggtggcacgaatatcgccgtaatgacgtgccccggtcgccatcagccgctcgccgatattgccgcctgccgacacctggcggcgcaggccgtcgagtggatgctgatgcaccacgccccattcggtacgcagcaggcgacggcggtcggcctcgctcattgcatacagcgaacggttctcgtagtgaatttccccctgctgcggcgtcaggcgcgcggagatcgacttcagcagcgtggtcttcccggagccggattccccgacaatgcccagcacttcccccggccataaatcaaaagagacatcgctaaagcctttgcccggcgcgtaaaggtgggtcaggttattgaccgaaagtaacggttgattcattggttttttgcctcgctctgttggcggcaataatcggtatcggagcagacaaacatgcggtttccggcgtcatccagcaccacttcatcaagatagctgtgggtcgatccgcagatggcgcatggctcatcccactgctgaacggtgaacgggtgatcgtcgaaatcgagactttccacgcgggtaaacggcggcaccgcatagatgcgcttctcgcgccccgcgccgaacagttgcagggcgggcatcatgtccatttttgggttatcgaatttcgggatcggcgacgggtccatcacgtagcgcccatttaccttcaccggataggcgtaggtggtggcgatatgaccgaagcgggcgatatcttcatacagtttcacctgcatcacgccgtactcttccagcgcgtgcatggtgcgggtttccgtttcgcgcggctcgataaagcgcagcggctcggggattggcacctggaagataattatctgatcttcggtcagcggcgtttcggggatgcggtgacgcgtctggataaccgtcgcatcgtccgtacgttccgtggtgtttaccccggtcacgcgcttgaagaagttgcgaatcgacacggcgttggtggtgtcatccgcgccctggtcaatcaccttcagcacgtcgctttcgccaatcacgctggcggtaagctgaatgccgccggttccccagccgtacggcatcggcatctcgcgcccgccaaacggcacctgataaccggggatcgccaccgcttttaagatggcgcggcggatcatgcgtttggtctgctcgtcgaggtaggcaaagttgtagccgctcagattagccatggttctgctcctgttgcagacgtttgagtagctccagttcggcctggaaatcgacgtagtgggggagtttgaggtgtgagacaaagcctgcggcttcgacgttgtcggcatgtgccagcacgaactcttcatcctgcgccgggcctgtcgcgtgctcgccgtactccggggcttgcagagcgcggtcgaccagcgccatcgccatcgctttgcgctcgctcatgccgaacaccagcccgtagccgcgcgtgaagtgcggcggctcacccggcgggtcgataaaaccgttaaccatttcacactcagtcatcagcagttcgccgacgttcaccgcaaatcccagctcttccggcacaatcgacacgtcgatatagccgctgcggatctcgcctgcgaacgggtgattgcgcccgtaaccgcgttgggtggagtaggccagcgccagcaaatagccttcgtcgccgcgcatcaactgctgcaaacgggaggagcgtgagcaggggtaaaccggcggcgtgcgggtgatgtcatccggctgtgcgccgctatcctcttcaaacttcgccagcccctgacgcgccagcaggctgaaaacgtgcggcgacggctgctgttcgctgtcggcggtggtcagcgtcggcgcttcgccgtttgccagcagggtaaaatcgagcaggcgatgggtgtagtcgtaggttgggccaagcagctggccgccgggaatgtctttataaacggcggagatacggcgttcgagacgcatcccggtggtgtcgagcggctcgcttaccgccagcttcgccaacgtggtgcggtaggcgcgcagcaggaaaatcgcttcaacgttatcgccgctggcctgtttcagcgccagcgccgccagttcgcggtcggcaatgccgccttcggtcatcacgcgatctaccgcgaggttaagctgctgttcaatctgggcgacgctcagttcgggcaaatcggtatcgcctcggcgtcggctctcttgcagggcgtgggcggcgtcgatcgccttctcgccccctttcacggcaacgtacatcagcacacctccacatgagtggttcgcggaatagccagcaggcgctcgccacaggtcaggatcaggtcgatgccgagcgggaacggatgcgggcgctcggtgagttcgtgcagaatgcactccggcagctgcggagcgatcattcgttcttcggcaatacccgcaccagtaaggcgcaacatgcgtccgccgctcaggctggcgacctgtaaaatcagcgtcgcacccgcttccggcgcaacggcggtgccggtggaaagggcgttgagctgttcgctggaaatcgcctcatccgtcaccgcgaaggtcgcctgttccggctggctgaccagcggcgcgttggtatgaaaacgcaggctctggttgacgatatcgttatttaatggggtagaaagccacaccggcgtgtcgttatcggccagcgtcagcagcacgctggtggtggcgatattcagcggttgccagccgcgtttgagctgatgcagggcgacaatcacgcccggctcgctcatggcctttaacaggcgacgaaaactgtgctgggcatcctgcacgggaagcataaaagcggtttccagggtcatgcgttgtctccgcgaaccatcgtaaagaagtcgacccggctggcgttcacttcggcctggcgtgcggcaatgcgtgccatacggtcagcgtccagcggggcaataagggtttctgataagttttgaaagtggcgagattgctgcatcagcgcgtcaatcagcgcgcagcgttcggcgtgctgtttatcacgcccctgcacccagctgtagccgagcgtgccgtcagtcaggcgcacggcggcgcgggtcagcgtggcgtcgccggcaaaaaaacgttcgccggtgccgcccatccgcgcctgaatctgtaccaggccagtttcagcggcgcggatcacctcatagtcggcggtgatgtttagcgcgttcaggcgtgctgccagttcagccggttggctgtgcgccagcacggacatccagtgctggcgggtcgcggtatctgcgtgcattcagtgctccatagtgaattcaatcatgtcggcgcgcgtcaggctgacggagtactccgccgggctgctttcaccgtcacggtggttaagggtgcgcacgcacagcagcggcgacatattcgggatttcaagacgctggcactctttggcctgggcgcggcgggcgctgatccgcgtctggctgcggcgcagcgcaattccggtttgctcgcgcagaaaatcgtgcagcgagccgctgtcgaagcgttgcagcgtcggccagagggtgaggtccgcgaagtagtggtcgattaaacagagcgcgacgccgttgacacgacgcagggtgcgcaggtggatgacgttctccccctcggtaatccccagtgcgtcagcgacgtggccggacgcggggcgcaataccgaaagcagtttttcgctggtgggatggctgccctgatccagcagattctggctaaaacgcgcctgggcgttgagcgggtaatcgaacgggcgcatcagcaccagcacgccgacgccctgacggcgctgtacccagcctttttccaccagttggtcgatggcgcggcgcagggtgtggcgattcacctcaaagcgcgctgccagttgctgctcggcgggaagatagtcgccgcagcggtagtgttgacgaagctcctgctcaagttttgcggctatctcttgatagcgtgttgggtagctggtcggatgtgtagacaagtgcatagatatcaatgcctcgcttatcagataaagtgcttacgcaaccgttgagagaggaaatccagcaggctgaccgtgacgatgataagcaccatcagggcgcaggtttgttggaactggaaaccgcgaatcgcttcccacagggtgacgccgatcccgcctgcgccgaccatgccgacgacggtcgccgagcggacgttggattcgaagcgatagagggagtaggagatcagcagtggcatcacctgtggcagcacgccgtagaggatctcttcgagcttgttggcaccggtggcgcgaatgccttccaccgggccgggctcaatcgcttccaccgcttcggaaagcagcttggagagcacgccggtggtgtggataaacagcgccagcacgccagcacgccagcgaacgggccgaggccgacggcgaccacgaacagcatggcgaagaccatttcgttaatggcgcggcaggcgtccatcaggcggcgaacgggctggtaaacccaccacggcaccaggttttcggcgctcatcaggccaaaggggatggagagaaccaccgccagcgcggtgccccagacggcgatttgcagcgtgacggccatttcggtgaggtaatcctgccactggctgaaatcgggcgggaagaagtcggcggcgaacgtcgccatgttgccgccgtctttgatcagcgtaagcggggccatttccgcgccctgccacgagacgaccaacacggcgagtacaacggcccagctcagaagcgagaaccagctgcgcttgggtggggcgatggtgatggtttgcatgtttggctccggtctgtaggccggataaggtgcttgcaccgcatccggcatcaacgcctgcacattgtcggatgcgacgccggggcgtcttatccgacctacgatttactgcaccgctttactcaccgaactcatcgcgcttagcgcgttgttcaggcggtccaggtcatccagctgcgcctgaatctcggtggtttttgccagcttgtcctgctcattcagtcctttattgcttttcacgccctgcatctctttaaacagcgcgagctggcgaatcggcaccagttgcaggtcgctggaagcgcggaatggcgcccagcccaggcgttccagcaccgctttttcttccggcgttttgccgtagttcataaagaagtcgtagatcttgtctttggtggtttcggaaagattcttgcgccagacgatcggatcgcctgggatcagcggcgacttccagatcaccttcagttctttcagcttctctggcgcggaggttttcagcttgtcgaggttttcggtgttgttggtggcaacatccacctgcttgttggcgacggccagcgcgttggtttcatgcccggcgttgacggtgcgcttgaagtcgctggcggagatattgtttttggcgaagacgtagtagccggggacgaggaagccagaggtggagttaggatcgccattgccaaaggtgagatctttccgcttcgccagcagatcgttcaggttgttgatcggactgtctttgttgacgatcaacacgctccagtaacccggcgatccatccgccgcgaccgtctgggcgaagacctggccattggcgcgatccaccgcttccatcgccgacagattgccgtaccaggcgatatccactttattgaagcgcatcccctggataatgcccgcgtagtccggggcaaagaaggcgttgaccttcacgcccagcttcttctccatatcctgcaagaacggcgtccattgcggtttcaggttttgctgtgattccgttgaaataatgccgaaattcaacgccttttcctgctcttcggcgtgcgccgggcttaacagggtgctgaggctgaacatgctggtgaaggccagcgaggcaattatcttagcgttcattcgttttcctcaatgatggggatgtcaggcagctttcgcgttctcttcgacgcggttaatgctgcggtagagatggtcaaaacgttcgttatcaaactgttggctgctgccgtcgtagaagacgtgcccctggcgcagggcgacgatgcgttcgcagtagcgcagggcgtaatccacctgatgcagcgtgacgaccacggtgatgccgtcgttctggttgatgtcgcgcagggtgtccatcacgatgcgcgctgattctgggtccagcgaggcgatgggttcatcggccagaatcactttcgcctgctgcatcagcgcacgggcaatcgccacacgttgctgctggccgccggagagggtggaaacgcgctgatgggcaaaatgcaccatgccaacgcgggtcagcgcctgtaacgcgcgctgtttctgctcgccggtgaaccagctaaaacaggtgcgccagaacggcgtgctgccgagcgcgccaatcagcacgttctccagtacgctcaggcggttcaccaggttgaattgttggaatatgtagccggtatgggcgcggcttttgcggatatcgcgggccaggcggccttcgcgctggactgtgcggcccagcagctcgatatggctaccgacagatttatcgccggtaatcaaaccgcttaagtgacgtaaaagggtggattttccggaacccgacggcccaagcagagccaccatttcaccgtgatgaatgttcagatcaaccgcatgcagcgcctgatgctgattgaaggttttggcgagcttctcgacacggataatcgtttgcatgatgcagcctccctaaaaaagtggctccatcgtggcggattattgtgacgatttggttaattaaaagtgactaacagatgaagagttaacgggaattcgatgacagtgcgggagggcgggcctcccggcgggttattgcgttggttgttgtttgacgacattaatcatccacggtacgccaaatttatcggtgactttgccaaagccatgcgcccagaaagtttcctgccaggccatttcgatttttccgttagcggcaagattgtcaaaccagcgttttccttcttcgacctgttgcgaatcgagcaccagcgtaaagccggagtagctggcttttcctgacggcatggcatcgctcatcatgatgtcgcttccggcaatgcgcacattggcgtgggcgatggcggtatcgggaaattgcattccggaagggcagttctcggcgctgtcctgcgctgattttggcatttcgccgaagctgattttatagagcagttccgcgcccaacgtacgttgataataggcaatcgcgtcggaacagttaccggcaaaagagaggtagggacttaacggcatgatggtgacctcagttaagagaagccagttaagtgtagttcgaaatttatacagatgagaggcggcctgataagacgcgcgagcgtcgcatcaggcagtcggcactgttgccggatgcggcgtaaacgccttatccggcctacggagggtgcgggaatttgtaggcctgataagacgcgcaagcgtcgcatcaggcagtcggcaccattgccggatgcggcgtaaacgccttatccggcctacggagggtgcgggaatttgtaggcctgataagacgcgcaagcgtcgcatcaggcagtcggcaccgttgccggatgcggcgtaaacgccttatccggcctacggatggtgcgggaatttgtaggcctgataagacgcgcaagcgtcgcatcaggcagttggcactgttgccggatgcggcgtaaacgccttatccggcctacggagggtgcgggaatttgtaggcctgataagacgcgcaagcgtcgcatcaggcagtcggcaccgttgccggatgcggcgtaaacgccttatccggcctacggagggtgcgggaatttgtaggcctgataagacgcgcaagcgtcgcatcaggcatctggcaccgttgccggatgcggcgcgagcgccttatccggcttaccgatcacaatacaatcagttctttttcacaaactcagatttcagtttcatcggaccaaaaccgtcgattttgcaatcgatgttatggtcgccttcaaccaggcggatgtttttcactttggtgccaattttcagcatcgaagagctacctttcaccttcagatctttaatgatggtaacgctgtcgccgtcagccagcagattgccgttagcatctttaacgatcagctcgtcgctttcctgtgcaggttctgcgtcgttccattcgtaggcacattccgggcagatgtacatgccgttatcttcgtaggtgtattcggagttgcattttgggcagtgtggtaatgacatgtggatttcctcaaaagtcagcagggcaaaagcgccaaaaaacggcagattgccgaaaaaggccgcaattatacacaaaatccctgagtttgtcgggggtactgctgattttagacgacgatcgttttcatttgaaaggaaacgcaaaaagaaaataatctttttgcctctatttattatttaagataatgttaatgctctacttgttctttttttaattcacatgatatttttatctttctgacgttttaaacgtatcagaagacgttatttattctgataaaaaacaacacactaaatataaaattatttcttgcagtaattataaaagccgaaaacagaactcaaaaacaatctggctaaataaaataacaaaatttgctttaaggaagaattttctatgtacacacagaccctgtatgagttaagtcaggaggctgaacgcctgttacagctttctcgccaacagttgcagttactggaaaaaatgcctctctctgtacccggagacgacgcgccacaactggctttaccctggagtcagcctaatatcgccgaacgtcacgcgatgctgaataatgagttgcgtaaaatttcccgactggaaatggtgcttgcaattgtcggtaccatgaaagcagggaaatcaaccaccattaatgccattgttggtacggaggttctgcctaatcgtaatcgcccaatgactgcgctgccgacgcttattcgccatacgcccgggcaaaaggaaccggtactgcatttttcacatgtcgcgccaatcgattgtttaattcaacaattacaacagcgcctgcgtgattgcgatattaagcatctgaccgatgtgctggaaatagataaagatatgcgtgcgcttatgcagcggatcgaaaatggcgtcgctttcgaaaaatattatctgggtgcccagcctatttttcattgtctgaaaagtttgaatgatttagtgcgactggcgaaggcgctggacgtcgattttcctttttctgcttacgccgccattgagcatattcccgtgattgaagtggagtttgtccatctagcggggctggagagttatcccggtcagttgacgttactggatacccccgggccaaatgaagccgggcaaccgcatctgcaaaaaatgcttaaccagcagctggcacgcgcctcggcggtactggcggtgctggattatacgcaactgaaatcgatctccgatgaagaggtccgtgaggcgattttggcggtggggcaatcggtgccgctgtacgtgctggtcaataagttcgatcaacaggatcgtaacagtgacgacgccgaccaggtgcgggcactgatttccgggacgctgatgaaaggctgtattacgccacagcagatatttccggtgtcgtcgatgtggggctacctggcgaatcgggcgcgctatgagttagccaacaacggtaagttaccaccgccagagcaacaacgctgggtggaagattttgcccatgccgcgcttggcaggcgctggcgtcatgccgatctggcggacctcgaacatattcgtcatgctgccgatcagttgtgggaagattcgctgttcgcccagccaattcaggcgttgcttcatgccgcttacgctaacgcctcgttgtatgctctgcgatctgccgcgcataaactgttgaattacgcgcagcaggcgcgggaatacctggattttcgtgcgcacgggttaaacgtcgcttgtgaacaattgcggcaaaatatccaccagatcgaagaaagtttgcagctattgcaactcaatcaggcgcaggtgagcggcgagattaaacatgaaatcgagctggccctgacctccgccaaccactttctgcgtcaacagcaagatgcgctgaaggtgcagttagccgccttgtttcaggatgattcggagccgttaagcgagattcgtacccgctgtgagacactgttacagacggcgcagaacaccatcagtcgcgactttacgctgcgttttgccgagcttgaatccaccctttgccgggtgttaaccgatgttattcgccccattgagcaacaagtcaaaatggaattgagcgagtcagggtttcgtcctgggtttcattttcctgtttttcacggcgtagttccccacttcaacactcgccagctgttcagtgaagtcatttcgcgccaggaagcaacggacgagcagagcacgcgtttaggcgttgtgcgtgagactttttcgcgctggttgaatcagcccgactggggacggggaaatgagaaatcaccgacagaaacggttgattacagtgtgttgcaacgagcattaagcgcagaagtcgatctctattgccaacaaatggctaaagttctggcagagcaggtcgatgaatctgttacggcaggcatgaatacttttttcgctgagttcgcttcatgtttgacggaattacagacgcgtttacgcgaaagtctggctctgcgtcaacaaaatgaatcggtggtcaggctgatgcagcagcaattgcagcagactgtgatgactcacggctggatttacaccgacgcccagctgttacgcgatgatattcaaacacttttcacggcagaacgatattgaccaagacgttacttgacggccccggtcgcgtgctggagtcggtttatccccgctttttagtggatctggcgcagggtgatgatgcccgccttccacaagcccatcagcagcagtttcgtgaacgactgatgcaggaacttctttcgcgtgtgcagcttcagacatggacgaacggcggcatgttaaatgcgccgcttagcctgcgtctgacattggtggaaaaactggcgtcgatgctggatcccggtcatctggcactgacgcagatcgcgcagcatctggcgctgctgcaaaaaatggatcaccgccagcactctgctttcccggagctcccccagcaaattgccgccttgtatgagtggttttcagcccgttgtcgctggaaggaaaaggcgttaacgcaacgaggcctactggtgcaggcaggtgatcagagcgagcaaatttttacccgctggcgtgctggggcgtataacgcctggtcgttgcctgggcgctgttttatcgttctggaggagttgcgctggggggcatttggcgatgcctgccgtctgggaagcccgcaagcggtggcgttgttgctgggtgatttgctcgagaaagcgacacaacatctggcagagagtatcaatgcggcaccgaccacgcgtcactattaccatcagtggtttgcctcttcgaccgttccgacgggcggggagcatgctgattttttaagttggctgggaaagtggaccacggcagataaacaacccgtttgctggtcagtgacccaacgctggcaaactgtcgcgctggggatgccacgactctgttcagcgcagcgtctggcgggggcaatgctcgaggaaatcttctctgtaaatttggcgtaaataatcagttacatcaatgagtcctaaacgaaatccatgtgtgaagttgatcacaaatttaaacactggtagggtaaaaaggtcattaactgcccaattcaggcgtcaactggtttgattgtacattccttaaccggagggtgtaagcaaacccgctacgcttgttacagagattgcatcctgcaattcccgctccccttttgcggccgtcgcgctgatttttctggcgtttgcggaaatgggccaactctgcgaggaaagctatgctgaaaaggaaaaaagtaaaaccgattacccttcgtgatgtcaccattattgatgacggtaaactgcgtaaagccattaccgcagcatcactgggtaatgcaatggaatggttcgattttggtgtttatggttttgttgcttacgcattaggtaaagtttttttcccgggggctgaccccagcgtgcagatggttgctgcacttgccactttctccgttccctttctgattcgaccgcttggcggactcttctttggtatgttgggcgataaatatggtcgccagaagatcctcgctatcactattgtgattatgtcgatcagtacgttctgtattggcttaataccgtcctacgacacgattggtatttgggcaccgattctgctgttgatctgtaagatggcacaaggtttctcggtcggcggtgaatataccggggcgtcgatatttgttgcggaatactcccctgaccgtaaacgtggctttatgggcagctggctggacttcggttctattgccgggtttgtgctgggtgcgggcgtggtggtgttaatttcgaccattgtcggcgaagcgaacttcctcgattggggctggcgtattccgttctttatcgctctgccgttagggattatcgggctttacctgcgccatgcgctggaagagactccggcgttccagcagcatgtcgataaactggaacagggcgaccgtgaaggtttgcaggatggcccgaaagtctcgtttaaagagattgccactaaatactggcgcagcctgttgacatgtattggtctggtaattgccaccaacgtgacttactacatgttgctgacctatatgccgagttatttgtcgcataacctgcattactccgaagaccacggggtgctgattattatcgccattatgatcggtatgctgtttgtccagccggtgatgggcttgctgagtgaccgttttggccgtcgtccgtttgtgctacttggtagtgttgccctgtttgtgttggcgatcccggcgtttattctgattaacagtaacgtcatcggcctgatttttgccgggttactgatgctggcggtgatccttaactgctttacgggcgttatggcttctaccttgccagcgatgttcccgacgcatatccgttacagcgcgctggcggcggcatttaatatttcggtgctggttgccggtctgacgccaacgctggcggcctggctggtcgaaagctcgcagaatctgatgatgcctgcctattacctgatggtagtggcggtggttggtttaatcaccggcgtaaccatgaaagagacggcaaatcgtccgttgaaaggtgcgacaccggcggcgtcagatatacaggaagcgaaggaaattctcgtcgagcattacgataatatcgagcagaaaatcgatgatattgaccacgagattgccgatttgcaggcgaaacgtacccgcctggtgcagcaacatccgcgaattgatgaataagctgaaacggatggcctgatgtgacgctgtcttatcaggccaattgaactcttaaggttcacttaatctctgacgcgcatactctcctccaggttaacggaggagagtgcaatgaaaaaccgtgtttatgaaagtttaactaccgtgttcagcgtgctggtggtcagcagctttctttatatctggtttgccacgtactgatctttcttcagccgtacccaggcccgcgtgccggaagtctcttgccggttttgcaggaaaaactgcccgtgatgcaactgtgtaatgcggctgacaatacttaaccccagaccaatcccgccataacggctgtccatacgtacaaacgctttactcaactccccgcatttactctcatcaatacctggtccttcatcttcaactgccatgaccgctccgtcatcttcttgcagcttaatcataatgttgctgccttgcgggctgtaacgatgggcgttttctaccaggtttcgcaataacatccgcagcagggttgcatcaccctgaacggtgatgtcggcggcgctctctggcaatagcagggtttgctgtcgctggtcgagcatggtactgagttcgtcatacgaggggagaatgacatcttccagcagttttacatgttgataattaccggaagaaaatgactgtccggcacgcgccagttgcagcagctgggagacgctctccatcatctgatcaagccgtgccactaacggtgctacatcaatgtgatgcgttttcgccagcagttccagatgcaaacgcacccccgccagtggcgttcgcagttcgtgcgcgacgtcagcggtaaacaacctttcgttatccagcgtgctggtcaggcgactgaccagatcgtttaacgccgaaaccaccgcttcgatttcgagggtggcgctgtgaatggcaatgggcgttaagttgtcggcggtgcgcgcttccagctctttttgcagctccgccagcgggcgggtgatgcggcgtaccgcctgatagcagataaatagcgtcaggctgaccataaagacgccggggacaatcaggctggcgaccgcctcgcggatctcacgcatgatgtggcgatcgttgttgcgattgtcgcgtagcgcctgctcaaacagctgaatctgctcggtactttcatgccatagccagaagacgctgatcagctcaaacaccaacaaaatggccccgatggtcaatatcagccgttggcgcagcgatattggtcggcgcagaaaatgcatcagattcaattagttttcctcattcgcgaccagcatatagccaaagccgcgcacggtgcggatacgggctttgcccactttgtcgcgcagattgtggatatgcacttccagggtgttggtcgagggttcattgtcccagttatagatgtcgttgtagagaatttcccgatgcaccggactgcctgctttgagcattaaccgtgacagcagagcatattctttgggcgtcagaatcaactcttcaccgcccatccatacctgacggcgacccatgttcagcgtcagattgccaacaatcagctcactttcgccctgattattatggcgtcgtagcagggcgcggatacgggcatgtaactcttccagcgcaaaaggcttcaccagatagtcgtcggcaccgacatccagcccggcgattttgtcggtcagcgtatcgcgagcggtgaggatcagtaccggcagggtatattttttctgccggatacgggcgagaaaatgcagtccatcttcgtcgggtaaccctaaatccagtaccaccaggctgtaatgacctgcctcaaggctttgttccgccatccgcgcggttgtcacgctatcgcacgcgtagccttcggtttgcgccgccagaatcagtccctgcaataacagcgtatcgtcttcaacaatcagaattttcattcactcactctcctgcaagtttgcagaatatcatccgcagcctggtaatacttcgtctcaacgccagttaatcccaatagcgtggagaataaattgtcttgtgaatagtgttgcgtttgcgcctgtttttgcaggcagttctggtcaacctgataccgtttttgataatcctccgacagccacagcagcatcggcacctgtttttggctatccggggcgatggcataaggcagaccgtgcagatagatgccattttcacctaacgattcaccgtggtcagaaagataaaccaggctggtggtaaatttatcctgatgttctttcagcagattaatcgctttatcaacaatatagtcgacgtaaaccagcgtgttgtcgtaagtgttcaccagttgctctttggtacaggtctggatctcattggtgtcgcaggttggggtaaatttcctgaactgaggcggatagcggttgtaataggtcggaccgtggctgccgatggtgtgtaagacaatcacgccatcaccttgcaggttattgatgtactcttcaagcccgtggaacagcacttcgtcatagcattcgccgttgatgcactgatcaggtagattcagcgcggtgacgttctggtgaggcacgcggtcgcaggcacctttacagccgccatcgttgtcattccacagcacgttgatgcccgctcgctgaatgatatccagcacgccttcctggtgctgtgccagctcttctttgtagtgctcacgcggcatatccgagaacatgcacggtactgaaactgccgttgccgtgccgcaagatgcggtattagggaaatagaccacgttatctttcgccagccgcgggttagtttcacgcgggtagccgttgagggagaagttctccgcccgcgaggtttcgccgacaatcaggatggtcaaatttttacgtttttcgttctgcattaacgggttgcggtgcgcgtcttcaccaattcgcaccagcggcagatttgccagtcgctgatgggagtaccatgaccagctggcaacaatgctgttagaggggcttaaggatttcaccagctctttgttattgcggaacaacgaggcgtagtctttataaaacagtgcggcgaccagcaaaatcagtagtacagaaaccagaatattggctccacggaaaagaacactgcgcagacgcgaggtggcaggtttgatttttatccagcaggcaatcagcgcagcaagcacgccgctgaatcccagcgttaataacatttgcggtgtcatcagcgcataactttctgccggagtggtatcaataatattggcaatcatcgagcggtcgatgacgatgccgtaagtcattatgaaatattgtgcagccgcgccaaccagaataaacaggcaggccagtggtcgattaagccataagaaagagcttagtgtcaggacaatattaatcacgctgaaagcgacgaccggcatcgacaagaaaaccagtacgttatgcagcgaatccagcggcagcgcctgcaacacctgtttaaaaaaggcaatattcaggcagatagagatataaaaagcggccaacaatagccaggcgagtaaattcaaagagggtctttttagtaggcgcttcaacatcacggtgtttccatcgaacaaagtgcgcatatgctcgcaaagcaaaattaagccaaccttaagttcttaaggttggcttttatgtttgctggattaaggggaattaatctttgcttattggtgcatctaagggatacgggtttttatgtagccggttgtaattcagcgcatacatggcggtgatgaccatcagggtgacaaatgaccacataacctctttcgctccggaccccaccacggcccagatgcagtagaggaaggcaatggtagtaactgccagatatgccgggcgtgctttaccaaagtgaccgtgtccgagcagcagtaacgccgcacaggtgtaaagatatggcaccagtgtaaagatgaccgagacggaagaaaccagaccgaactctttggtcgcgtttggtgaaatgctgctgagctggaagatggtcatcaaaataccgacgataatcagccccgccactggcgtacccgctttatttacacgggcaaaaatcggtgggaacagtccgtcatcggcagcggctttcgccgtttgacccgccagcaacgtccagccgcccagtgaacctaagcaacccgcagctgcgcagaaggaaacaatggccccggcggtgtcacccaacgccatccgtgcggcatcaccgaatggcgaagcagaaacgcgcagtgcggcattagggatcatccccataatcgcggtggtagaaagtacatagcaaacggcggcaatcaataccccaccaatggtggcgatagggacattgcgtttcgggtttttcaccacacctgcggcaacggaggcactttccacaccgatgaacgaccacagcgtaacgttaagggtactttgaattgcaccgaaggtgcccaggccgctgacgttccatgccgccatataggtttcaccacggaaccagaaccagccaaatacggcaatcccgacgatggggatcagcgccagcacggtggcaactgcctgcacacgggtgatcattttcggaccgacaatgttcagcaggacgaagatccacagcaccacgacgcaggtgatggttaataccaatggatctttcagaatcgggaagaagtaacttaaatatcctacgccaatgaccaccatggcgatattgccgatccagcaggccagccagtagaggacgttggtttgataaccgagaaacgggccaaagcagcggcgggcgtaagcgtaagaaccaccaggacttgggtcgaggaacgacattttggcgtataccatcgagagccccagtgcaccgataatcgtcaccaaccatccataaatggcaatcccgccagtagaggccaggtttgcaggtaacagaaaaacacctgaccccataatattccccgacaccatcagggtgacggggattaagcccactttgtgagcatcagcatccgaagacataattaaactcctgcgaaggcgagcttcgtgacaataaattacgtcatatcatacgcctgcattcgatagttgaattattatcgaccgggttatcgctgatgccgttattaatatagctcttcgttaaggttaaaaatcaggcgacagtgcgttctctgtgctgactaacataatgcagcggcgtcataccgtagaagtctttaaagacagaaataaagtacgacgtactgttgtagccgcaggactgtgatacctgagagatatttttaccgtccatcattaattcatttacggcataacgcatgcggcaggtggtgattatttggctataactggtgttttcgcttttcaactttttctttaacagacttgggctaagacataaacaactggctaccatactaagattccagtctttgtgaatatcgctttcaataatttgataaacgctgtcacttacacaattacgtaacatatacatcattaatgaaacgaattttttactgtcgagaaaacgggatagcaccgtgaataataatgcgcgtgttcgttccttttctgactcagtttctgcgggcatcatgctgtgttgcgcggcaacgcgaaagacgtctggcgtcaggcatggcagggtgagtatgggcgtagcgctacgttgccatactggtatttgcgagagatctttattcagaaaccggaggtaatctttgatgatgtcgtgactaatatgagcaaccaaagtgttgttaagagaggagacgtcgataatattattttcacaatttaataacgccatatggttagctttaaggctaataggttctttcccattcacccttatccagacatctttttcagtcaataaaacaatacaaggttggtcgctgcaaatcctcatacatgtactcctgagtgcgaataaaagaccagttctcgctaaagcaaagcgataccgggaaatggttatataattgtatgatgaatataaacatgcataaaaataacgagttttactaatagtacaaatttttatagtaatttctcatgtacatatttttttacaggataaataacaggcaaaaaaaagcgcggggtggggccgcgcaaaaagtatgacatttttgtttgcagcaatttttatgaaaacgttgccatactcaaaaggcctaaggccaggcggcgtaatgttatttaaacaattacgccttcagcggaatagtggttacgctttcacgcacataacgtggtaaataccgtcaataatttcagtcccttcagtttcgtgttcaaatccagggaaatggtggtcccaggattgcagcgagcgtaaataacttacttgcggactgtttttatcgccgaagttttcaccagacagcagcatcgggattcctggcggatacgggataactgagtttgccgcgatgcgtcctggcagattttcaatggataccagttcgacattgttgtcgacaatcgcgttgtacgcttcacgcggggtgacttccgccaccggcaggccggaataggcttcgttcaaccgtgcgccagggttgttttctttcagccaggcaaacatggtgtcacccagatcgtgaatccccatgttcgcgtaagtgtcaggatattgttcaacaagttccggcatcacctgcgccagcggtgtgttggcgtcatagtggcgtttgaaggagcaaagggtgttaaccagagttccccatttcccacgggttacgcccatagagaacaggaacataatttggaagtcagtggtgcgggtaggtacaatgccgtggcgaccaagccaggcagtgaccagcgccgccggaacaccggtttcttccagttcaccatcttcacccattcccggagcaaggatgctgactttaatcgggtcgagcatactccagttatccggaatatctttgaagccgtgccagctttcgcccggatgcattacccagcagtcctgaacggtggtcagcagtttggttggtgcgtcagcaaagtcataggttttgccggtttgtgggtcggtgacgacttctttgttccacggtttgaagaaccagctaccgtcagcggtgaactctttatatagccgcgccatcgcctgacggaaatcaaccgcttcgtcaatcacttcctgtgtcagtgacaggccgctgttgccgtccatcatcgacaccgccacgtcgttggatgcgcagatggcatacagcggggaggtggtggcatgcatcatgtaggcctggttgaagcgggagaagttaatcgccccacgaccttcacgtacatgaatataagaagcctgtgacagcgcattcagcagtttgtgggtggagtgggtggcgaaaacggtaggaccgttgtgatcgccaggttcgccgcgcatggcatagtgatcggcatagatcgggttgaaacgtgcatagccgtaccaggcttcgtcaaagtgcagacgatcggaggttttttccagcagatcctgcgcttctttagcgttataacacacgccgtcataggtgcagttggtcaccacgcagtaagacggtttttgcccggctttgtctttggtcagcgggctttcactgattttcttctgcaaggtttcaggttgcatttcctgcggatagattggcccgataatgccgtagcggttgcggcttggcaccatatagaccggtttcgcgcctgtcagcatcaaaccttgttcgatggatttatggcagttacggtcaacgaccacgacatcgttatcggtcatgcaagcctgcatgatggtgcggttagagccggaagtaccgacgactaccgaccaggagcgatcggcaccaaatacgcgtgcggcatatttttcgctttcgccaaatgcgccagtatggtcaagcaaagaaccgagggaagttcgttcgatgcccatgtcggtgcggaacagattttcaccatagtagtcatggtagaaacgtccggcgggtgttttggtaaaaccaacgccgccctggtggcctggcgctgcccaggaatattcatggatgtcactatatttcatcagcgcgctgaacagtggcggcaacagctgctggcggtagcgggtcatcgcggcaacggcgcgtccggcgataaagtcggcggtatcttccagaatccaggcgaattcatcgacaagctccagcaggtcgcgatccattgcggcgagggctttttcccgatcgcccaacaggaagaccggcacgttttgttggcgctcatgaagcttaccgatcaattgtctgacgttttgatgttcgtccggatgttccatttgatagctgaacatcaggcagtcaatggcttcgtttgaagagagaatggcaaaaccatcatcaaaggaggtggatttaatcacggtaacattttgctggcttaaagcatctgccagacgctcaacggcgttaccgacccaggtgtcttgatggagaaactcgctttcaacaattaatactttcatcattgcttacccggttatgaaggaatcttcgttgcgggcaagtatcttccggccttttcgggctgtaaagcgcgtgaaaaacaaacatttttgaaatatttagttttataaacaatacgttatgtgattattttaaattattttcactgcttattatcgacggctaaactatttttttggctgatactgatatcgtctttagccgggaaacgtctggcggcgctgttggctaagtttgcggtattgttgcggcgacatgccgacatatttgccgaacgtgctgtaaaaacgactacttgaacgaaagcctgccgtcagggcaatatcgagaatacttttatcggtatcgctcagtaacgcgcgaacgtggttgatgcgcatcgcggtaatgtactgtttcatcgtcaattgcatgacccgctggaatatccccattgcatagttggcgttaagtttgacgtgctcagccacatcgttgatggtcagcgcctgatcatagttttcggcaataaagcccagcatctggctaacataaaattgcgcatggcgcgagacgctgtttttgtgtgtgcgcgaggttttattgaccagaatcggttcccagccagagaggctaaatcgcttgagcatcaggccaatttcatcaatggcgagctggcgaatttgctcgttcggactgtttaattcctgctgccagcggcgcacttcaaacgggctaagttgctgtgtggccagtgatttgatcaccatgccgtgagtgacgtggttaatcaggtctttatccagcggccaggagagaaacagatgcatcggcagattaaaaatcgccatgctctgacaggttccggtatctgttagttggtgcggtgtacaggcccagaacagcgtgatatgaccctgattgatattcactttttcattgttgatcaggtattccacatcgccatcgaaaggcacattcacttcgacctgaccatgccagtggctggtgggcatgatatgcggtgcgcgaaactcaatctccatccgctggtattccgaatacagcgacagcgggctgcgggtctgtttttcgtcgctgctgcacataaacgtatctgtattcatggatggctctctttcctggaatatcagaattatggcaggagtgagggaggatgactgcgagtgggagcacggttttcaccctcttcccagaggggcgaggggactctccgagtatcatgaggccgaaaactctgcttttcaggtaatttattcccataaactcagatttactgctgcttcacgcaggatctgagtttatgggaatgctcaacctggaagccggaggttttctgcagattcgcctgccatgatgaagttattcaagcaagccaggagatctgcatgatgtctgcacccaaaattacatttatcggcgctggttcgacgattttcgttaaaaatattcttggtgatgtgttccatcgcgaggcgctgaaaacggcgcatattgccctgatggacattgaccccacccgcctggaagagtcgcatattgtggtgcgtaagctgatggattcagcaggggccagcggcaaaatcacctgccacacccaacagaaagaagccttagaggatgccgattttgtcgtggtggcatttcagattggcggttatgaaccttgcacggtgactgatttcgaggtctgtaagcggcatggtctggaacaaaccattgccgatacgttggggccgggcggtattatgcgcgcgctacgtaccattccgcatctgtggcaaatttgcgaggacatgacggaagtctgccccgatgccaccatgctcaactatgttaacccaatggcgatgaatacctgggcgatgtatgcccgctatccgcatatcaaacaggtcgggctgtgccattcggtgcagggaacggcggaagagttggcgcgtgacctcaatatcgacccagctacgctgcgttaccgttgcgcaggtatcaaccatatggcgttttacctggagctggagcgcaaaaccgccgacggcagttatgtgaatctctacccggaactgctggcggcttatgaagcagggcaggcaccgaagccgaatattcatggcaatactcgctgccagaatattgtgcgctacgaaatgttcaaaaagctgggctatttcgtcacggaatcgtcagaacattttgctgagtacacaccgtggtttattaagccaggtcgtgaggatttgattgagcgttataaagtaccgctggatgagtacccgaaacgctgcgtcgagcagctggcgaactggcataaagagctggaggagtataaaaaagcctcccggattgatattaaaccgtcacgggaatatgccagcacaatcatgaacgctatctggactggcgagccgagtgtgatttacggcaacgtccgtaacgatggtttgattgataacctgccacaaggatgttgcgtggaagtagcctgtctggttgatgctaatggcattcagccgaccaaagtcggtacgctaccttcgcatctggccgccctgatgcaaaccaacatcaacgtacagacgctgctgaccgaagctattcttacggaaaatcgcgaccgtgtttaccacgccgcgatgatggacccgcatactgccgccgtgctgggcattgacgaaatatatgctcttgttgacgacctgattgccgcccacggcgactggctgccaggctggttgcaccgttaaaacgcgactaaacgctactgcgccgggggatttattccggcgcacacctctgacgataccaataacagaaggcgggcgttggtaacagcgacccgataccctatgagcatttcaatgactacaaaactcagttatggatttggagcgttcgggaaggattttgcgatcggcattgtgtatatgtacctcatgtattactacaccgatgtcgtcgggctgtctgtgggtttggtcggtactttgtttctggtggcgaggatctgggatgctattaacgatccgattatgggatggattgtaaatgctacgcgatcgcgatggggtaagttcaaaccctggatcctgatcggtacgttggcaaactctgtaatcttatttctcctctttagtgcgcatctgtttgaaggtactactcagattgtctttgtttgcgtgacctacatcctctggggcatgacttacaccattatggatattcccttctggtcgctggttccaaccatcacgctcgataaacgtgagcgcgaacaactggttccttatccgcgtttttttgccagtctggcaggctttgttacggcaggtgtgacgctaccatttgttaattatgtcggcggtggcgatcggggatttggctttcagatgttcactctggtactgatcgccttttttattgtttcaaccatcatcactctgcgcaatgtgcatgaagtcttttcgtcagacaatcaaccgtctgctgaaggaagccatctgacacttaaagccatcgttgcgctaatttataaaaacgatcagctttcatgcctcttgggtatggctcttgcttataatgtagccagcaacattattaccggctttgctatctattatttctcatatgttatcggtgatgcggatttgttcccctattatctgtcgtatgcgggagctgctaacctggtgacgttagtattcttcccacgcttagttaaatcattatcccgacgcattttatgggccggagcatctattcttccggtgttaagctgtggtgttctcctgttaatggcattaatgagctatcacaacgtcgtcctcattgtgattgcgggtattttgctgaatgtgggaacggcgcttttctgggtattacaggtcatcatggtggcagatatcgttgattacggtgaatataaactgcacgtacgctgtgaaagtatcgcttactccgtgcagactatggtggtgaagggcggttcagcctttgcggcttttttcattgcggttgtgttagggatgattggctatgtaccgaatgttgaacagtctacgcaagccctattaggtatgcagtttattatgattgctctaccaactctgtttttcatggtaacgctgattctctacttccgtttctatcgcctcaatggtgacacgctgcgcaggatccagatccatctgctggataaatatcgcaaagtaccgcccgagcctgttcatgctgatattccggtcggtgcagtgagtgatgtgaaagcctgacgtggacaatagctaacgaaaatggcctgatgcgatatgtttatcaggccacgtcttaatgtaatgctttggatttgcaaattttgtagaccggataaggaattcacgccgcatccggcatcaacaaagcgcaagttgttatccggttatcaagccaaagcgccgtagctggcggcaatgaaagcgagcgaggaatatcaccgtcgttaatgcgccaagcagcgcgcagaacatatcggattgcgtgtcccactggtcgccctgggtgccgagaaaatcatccgctccctgacccattgccagcgctgcccaccactcgattaattcatacatcgcgcttatcgccagcgccacgcagcagaccaggaacgccaccattttacgtccgcgcacgtacatcccgcgaacgagaatttctcgtgccaccagtgcaggcaccagcccctggaaaaagtgccccagcttgtcatacggattacgactcaaccccagccattcctgcacctcaaaaccaacggggactttcgcgtaggtgtattgtccgccgaccatcaggatgatggcgtgaaggaaaatgagcgtatagagcagcggcgttaacggataacgtctggcggtggcaagcagtagctgcacgacaataatcaccggtgtcacttccatcagccaggtgagtttgtcatgggccgaaatgccggtataaatcaggattaacgttagcgtcagtgcgctggtgttaagaattaacggcttgagtgtgcgggtcatggtgagttcgcaaatcagggaaaatactgactattcaccagcaagcgtgaaattacaatcgcaaaagaggtggccagggggatcacctggcagcatgctgccaggcgctgggccgaagaggttacttagtgcagttcgcgcactgtttgttgacgatttgctggaagaagtcgttacctttgtcatcgaccaggataaacgccgggaaatcttctacttcgattttccagatagcttccatacccagctccggataagcgacgcactccagatgcttgatgctctgctgcgccagtaccgccgccggaccgccgatgctaccgaggtagaagccgccgtgtttatgacacgcgtcggtaacctgctgactgcggttacctttcgccagcatgatcatgctgccgccgtgggattgcagcagatccacgtaggagtccatacggcctgcggtggttgggccaagtgaacctgatggataaccggcaggggttttcgccggacccgcgtagtagatcgggtgatctttgatgtactgcggaagttctttaccggcgtcaatcagctctttcagcttggcgtgtgcaatatctcggcccacgataatggtgccggtgagcgacaaacgagtggataccgggtattgcgaaagctgggcgaggatctctttcatcgggcggttaaggtcaactttcaccgcttcgccttcaccggcctggcgcagttcttgtggaatgtactggcctgggttgtgttccagtttttcgatccagataccttcgcggttgattttcgctttaatgttacggtcagcggagcaggagacgcccatgccgaccgggcaggatgcgccgtgacgtggcagacggataacgcgaatgtcgtgcgcgaagtatttaccgccaaactgcgcgccaagaccgagtttctgggcctcttccagcagttcctgttccagctggacatcgcggaacgcctgaccatgttcgttcccttccgtcggcagttcatcgtaatagtgagcgcttgctaacttgacggttttcaggttggtttccgcagacgtaccgccaatcacaaacgcgatatggtacggcgggcaggctgcagtaccgagggtacgcattttctcgacgaggaagtttttcagtttgccgggagtcagcagggctttggtttcctggtagagatacgttttgttggcagagccgccgcctttcgcaacgcaaaggaatttgtactcatcgccatctaccgcgtacaggtcgatttgcgcaggcaggttagtgccggtgttgacctctttgtacatgtccagcgccgcattctgtgaatagcgcaggttatcttcgatataggtgttatagacgcctttcgacagcgtttcttcatcaccgccgccggtccacacgcgctggccttttttaccgacgatgatcgcggtgccggtatcctggcaggtcggcagcacgcctttggcggcgatttcggagtttcttaagaattgcagcgccacgtacttgtcgttttcgctggcttctggatcgtgaagaatagccgcaacctgtttctggtgtgccgggcggagcataaaagaagcgtcgtgaaaggcttgctgcgccagcagggtcagggcttctggttccactttcaggatggtttcgccgtcgaagtcggcaacgctaacgtaatcggaagtgagtagatagtattcggtattgtctttccccatcgggaaaggtgcctggtagataaagggtttgtttgacatagcttccagcctgtaactctgtatttgttattcgaaaatggcgtgccgcgtagtcacgggcggcacgcaaagtgcatttataagaacccgtacatcgcggcgaagatccagccgaagacgcacgatacgctcacaccaatcaaccccggcagaataaagctgtggttgatgacgaagcgaccgatgtgggtggtgccggaacggtcaaactgaatcgctgccagatcgctcggataagtcggcaggatgtaataaccgtagcaagccggtgctgaagccacgatgtatgccggatcaacgccgatcgccagcgcgaccggaacaatcgccgccagcgccgcagcctgagagtttacaaacttggaaaccagcagcagaacaatggcataggcccacggatactctttcaccatttcacccagtacgccctgaatttcagacatatgcgcaccgaacatggtttctgccatccatgcgataccgtacaccgccacgatggcgatcataccggaacggaagacttcgttttttgagatagacgcgggattggttttggtcaggataataatcagcgccccggtcagcagcataaacatctgaataaccagtaccatcgacagcggtttgccgccgaaggatggacgcaggtccgaatcagcaccaagaagggcgactacagcgattgccccgaggaaaatccacattgccagccagttgcttttcggcagttttttatccagcagcgtcgcggtatcaccgtaaacatactcacggttttccggtacggagatgaatttctggaactcttcgtctttatccagatctttaccgcggaaccagctgaagataccgatcgccaggataccgattaacgtcgatggaatggtgattgccagcagatcgaggaactcaagatggcgaccatcaaaggtgacattacccagcatcgcaaccagagacacgaccgcaaccgacaccggactggcgataatccccatctgtgcaccgatagaacttgccgccatcggacgttccggacggatgttgttcttaatggcgacgtcgtagatgatcggcagaatggtgtaaaccacatgacccgtaccgcaaagaatggtcagtgtacaggtcacaaacggcgcgacaattgagacatatttcgggttgcggcgcagcagcttctcggcaatttgcagcatgacatcaagaccgcccgaagcttgcaaggtcgccgatgccgccaccaccgcaatgataaccagcatgacatcaactggtggtttacctggctgaaggtggaagacgaagaccagaatgaccagaccgataccgcctaataaacccagcgcgataccaccctttctggcaccataaaacagacatatcagtattatgataagttggatagtaaataacatgtgtgaaccctcgcgataatcctatttaaatttttgctgaatagatcacagtcacgttctgttttgtatgaactgttttcagagcctgactaaatatccgtttggtcgttaccggctttagcaaatacctcacagtgaatattggctgattaaagcagcggcaaatttatgcactgtgataagcggctttttcagagagaaagactctctggcgatgggtttatagtttgtactgcgcagatgttaatgttttgtttgctgttatcttattgatatttatcggtctattttttgttctcagggcagatgtcattaggtttatagattaatctgatctacccatttgtgggtaaaaatacacataatgcgggtgacataatagttaattaacttttgttagcgttttgaaattaaaaacaccgttcacctgaagagatattaatttttagcgatgatggagggataattatatttgatctggcacaagttttactgatgaaggatgtaacttgtgccaggggtattttgcattacggtaataattattacttacagataaccagcgatccgttattggcaatattgtttcagtagtgagtagtgttctgcctgaatacggtaacggtaaactggacgccccgtgacgccataatggatactggtgaacaagatgtggcagttgaccagccagatgaggtatttacggcaggaaacacgcgaaatgttaacctcgttggctagctcgtcggttgaaaattcatagtcctgatgcgcgtcaatccactggcacagtgtgcgtaacgtctgcggcgttaagccttttggcaagcgacgaggatcctgttcgttggagctgctgccgtggattagctgatcaagctcggcctggtcataatactgatgtttttccagcgccattttcttttgccgccagccggtgagcgcctcttcaaagcgggaagcctggaagggtttgatcaggtaatccacgacaccgtaatgcagcgaatctttaatggttgccgcatcggctgcggaggagatgacaatcacatcacttttgcaacgcgcgttatgcaggacaggcagtaaatcgagcccgttctctttttgcatatagatatcgagcaatatcaggtcgataggcgtatcgctattgaagataatctctttggctttctccagcgtcgaggctgttccacagcattgaaagcctgggatttgtgctacgtatcggcgattcagctccgcgaccattgcgtcgtcatcgataattaatacattgatcatctgttcgacctctccccgtcccagggtatctggacaaaaaattgtgtgaaaatcccgggttccgattccacggcgatgctgccgccgagattttctacctgttgtttgacaagtgctaaaccgacgcctcgctcgcttccttttgtcgagacacctttgtcaaaaatgtgatcgattttatcgggtgcgatccccggtccatcatcattaacttcacagtgcagccagccgtgacggtagtgcaatgttacgctaatttcgcctccgggttccggccctaatgcctccagcgcgttttctatcagatttcccaacgtggtaatcagcgtcgcgacctggtcctcactgccgctgtctggcagctggctttcactgtttaaaatcagcgtatggcctaaatcggtcgcgcggttaatcttgctgattaaaaaaccagcgataaccggagatttgatcttacccagcagagagccaatctcttcctgatagttattggctgttttgagaatgtaatcttccaactgcttataactcttcagatgcaataatccgagaatcacatgcaatttattcataaattcgtgggatcgttcacgaagtgcgtcagcatagttgaccagaccgtcgagtcgctgcatcagtttacgtacttcagttttgtccctgaaggttgaaatggcaccgatgataacgccattactgcgcaccggaacggtgttgatcagtaatagccggtctttaatcgtaatctcttcgtcgcggcgcggggtaccgtcgcgtaacacttccgagacatctaccacctgtgaccatgagtggcttagcgtcgacagtttctcatcgtcctgcgacttacggtaattcagcaattcttgtgcggcatcgttgatcagcgtgacctcgccgcgatcgtccacggcaacgacgccttctttgatagactgcaacatggcctggcgttgctcaaacagcgtggagatttcgtagggttccaggccgaaaaggatttttttcagtaccttaaccagaatgcaggtgccaatcagtccgaccagcatgccaaataataccgaccagataatgctccagcgactgtcattgatctgttgggtcacacggcttaactcaaggccgatcgccaccacgccaatttgtttatgattttcatcgtagatgggggtaaatacgcgtaaagcctgcgccagaaaaccgcgattgatagcgacattttcttcgccattcagcgctttaaggatgtcatcacctttaaatggctgaccaatacgctgggcttcaggatgcgagtagcgaagactttgcatatcggtaacgacaataaacagcagatcgttgcgtttgcgtacggcttccgcgatggcctggatgccactctcctgcggttttttctgcaagccctgacggatttccggcgagtcggcgagggtacgcgccactgccagtgccttgttggctagcccatctcgcgtcatatcactgatttgcgagaagtaaatcagatgcaccaccaatagcaccgagaacagtaccgcactgaccattaagatcactgtggtactcaatttcatcggacgtttgcgtaacatgcggtagggcaatgaatgtctcatcagcttccttgtgtgacaaatttcttaagcattatctctgatgaggcgggtaattcaaagggagtaagaatgattggctatataggggaagagactctggcaacggaaactgccagtgctgtatgaagattccggggctatgcttatagcgataatcatactgatgagagagggaaggtcatggatcaggcgctactggacgggggttatcgctgttataccggcgaaaagatcgatgtctatttcaacactgcgatatgtcagcattctggcaattgcgtacgtggcaacggcaagttatttaatctcaaacgaaagccgtggatcatgccggatgaagtcgacgtcgccactgtggttaaagtgattgatacgtgcccgagcggcgcgctgaaataccgtcataaataagcgagggtaaaatggaaatacgcgaaggccacaataaattttacattaatgacaaacaaggcaagcaaatcgctgaaattgtctttgtgccgaccggagagaatttagcgattatcgaacataccgatgtcgatgaaagcctgaaagggcaagggattggtaaacagctggttgcgaaagtcgtggaaaaaatgcgtcgggaaaaacgaaaaattatcccattatgcccatttgcgaaacatgaatttgataaaacgcgggagtatgatgatattcgcagttgatgggagagtacagagtcacgatatttttcattctctccgcgatgtgatgcaggagagcatctgaagggtagggggatgcacaaagaatgggcagagagcgcgtttttttgtcccaagtcatcccctttactgagcaaaaaaaagaatatctcctatatgagaatcatcaatcggggttaataagttttgcgtccccagagcgtttaatattgataggagtcatattatggaaggtaaaaacaagttcaatacttatgttgtttcttttgattatccatcatcttattcctcagtgttcttaagattaagatcattgatgtatgatatgaatttctcctctatcgtggctgatgaatatgggataccacgacaattgaatgaaaactccttcgcaataacgacatcgttagccgcaagtgaaatcgaagatttaatcaggctcaaatgcttagacttaccggatattgattttgacctcaacattatgacagttgatgactatttccgtcagttttacaagtagccaggaaggataagaagaacataaaaaatggcactattctctaaaatattaattttttatgtgattggtgtgaacatatcctttgtcattatctggtttatctcacatgagaaaacacatattcgtttacttagtgcattcctggtcggaataacctggccaatgagtctgcctgtggcattacttttttctctcttttaggagctgtagttgagtggacccgctggttatcgtgaaacgaagcgtctctcctcaaaactggatttgcggaacgatgaacgaagcagtcgcctgactgcttcgttcattaaagtgaaatttatttctgtgggcgcatcgccgggaagagaataacgtcgcgaatagtatggctgttagtaaacagcataatcattcggtcgataccaatacccagaccagcggttggcggcagaccatattccagcgcagtcacgtaatcttcgtcatagaacatggcttcgtcgtcacctgcagctttagcattaacctgttcctggaaacgttcagcctgatcttctgcgtcgtttaattcgctaaaaccattaccgatttcacgaccaccgatgaagaattcaaaacggtcggtgatttccgggttaacatcattacggcgtgccagcggggacacttctgccggatattccgtaataaaggttggctgaatcagatgtgcttctgccacttcatcaaagatctctgtgacaatacgtcccaacccccagcttttctctaccgtaataccgatagattcagctaatgctttagcagcatcaaaattatccaggtcggccatatcggtttctggacgatattttttgattgcttcgcgcatggtgagtttttcaaacggtttgccgaaatcaaacacatgctcgccataagtgactttagtggtacccagaacctcttgtgccagggtgcggaacagtgactctgtcagttcaatcaaatcgtggtaatccgcatacgccatgtagagttccatcattgtgaactcaggattatggcgaacagaaataccttcattacggaagttacggttgatttcgaatacccgttcaaaaccgcctacaaccagacgtttcagatacagctccggcgcgatacgcagatacatatctaaatccagagcattatgatgggtaataaacgggcgagcagatgccccacctggaattacctgcatcatcggggtttctacttccataaagccgcgcgcgaccatgaattgacggatagcggccagaatttttgaacggacaacaaacgtttgacgggatttatcgttagcgatgaggtccagataacgttgacgataacggacttcctgatcctgcagaccatggaatttatctggtaaaggacgtagtgctttagtcagcaggcgcagctcagtacagtgaatggaaagctcacccgtttgcgtcttaaacagcgtaccgcgggcaccgataatgtcacccagatcccattttttaaactgatcgttataaacaccttctggcaggctatctcttgcaacgtacagttgaatacggccaccgacatcctgcaacgttacaaaggaggctttccccatgatacgacgggtcatcattcggccagcaaccgagacttcaatgtttaaggattccagttcctggttatccttcgcatcaaactcttcgtgcaactggtcagaggtatggtcgcggcgaaaatcattgggaaacgccacaccttgctgacgtagtgccgccagtttttcgcggcgatttctcagttcatcgttaaaatcaatagcctcattggctccccgtgtttcttgttcagacattttggttcctctaaatccagctttcaatttagcgtagataaagagacagatcggtacactgtattatctgcctcgactattagtaactcagtttatcttatcgaaactaacgcttacctcaagttgatatcactaataaataaccatcaaaatggtttaaatgacttattaatctcgatttgttagtgttataaactgaaagttaatttattcataaccaattgtttttacgacagttaatcgttgctctcctgtatcatattcgtcggcgtgctaaacagaaaacgggtagcaaaggccaatacgacgatgatcgcgacacaagccaacgtccactctcccatctgagaaaagaatcgctggtaagctgcaattgccataccgctaatttgcgactctgtcgtctgctgtgccacgacgcctgccagccagttggcgaccgcgcctgttgccagcatataaatcccggttaatacgccagacattttcagacgcgtgatttgcgcaatcgccaccgggtcaataaagagttcggcaaagcccattagcgccagcccggatatcatcacgcccattgacgcttgaccgtcagccgctgcatgtcgggcatcaaatgccaacaacataaagccacaagccatcagcagtaagccaaaggcaaacttcagccagacgcgcaatgttgagttgccgcggctttctggcgacgccagccaggccagtacaaccccagcgagcatcaccgcaattgcattcaccgactggaatagtgctgtaggtacttcaatattgaatgcctgacgattcacaaagcgatcgataaacaagctgatggtactgccgccctgttgtgccagtacccagaacaatgtcccgacaaacatcaacaatacaatttgccaaagagcacggcgatgttcggggaatttgatcatcatgcgggcaatgatttgtgcggcaatgaggcaaacgatcgccagcaaatatccggaccagtcgttctccagcagcagagtaaaaaatactggggctaaacagagcatcaccactaaccagctccatactggtaaggcaaatttgacactagtgagcgcttttttatccatactacgtgtggactggaaatgacgatgaccgcttaagaaaatcaacaaaccgataaacatgccgccacccgcaagggcaaagccaacatgccatccataccactgagcagccaggccgcaggcgattggggctgcgatagaaccgatattgcccgcagcatacagcagcgaaaaaccgccatcacgtcgatgatcgttctcgtcgtagagctcgccaagcaaacagctgatgtttgatttgaataaaccgtagccacaaataatgattgccagcgccagatacaggctaaaggttgaatttgtatcaatacccagcaccacatggccaagggtcattaacagcgcgccggcaatcactgcagtgcggttgccgagcaggcggtcggcaagccagccgccgagaataggggtaacgtaaaccagagaagcatatgcgctgaacaggctgatggcatggttatcatcaaaaccaagctgatgggtgagatagagaatgagtaaggcacgcatgccgtaaaaactgaagtactcccagatttggatcgccacgatatagtatatcgcgcgcggctgtgagggtgttttcatgtgttctccttatgagcaaaaaagggaagtggcaagccacttcccttgtacgagctaattattttttgctttcttctttcaataccttaacggtatagcggccatcagcctgacggtatgcaccgtgaatatcggtttcaaagcccggatagtgagcgccgatttcacacagcatctgcaggaactccagaaccggacggctttcttcggtgatcatttcacccggcattaccagaggaactcccggcgggtacggaaggatcatattggcgttaatacgacctaccatttcgtcgaggtaaacttcttcggtcataccgtgcagctctttctggaatgcagcatacggagtcattaccatcgtcggcagcacttcaaatgcgcgatacatcagatccggcagattgtggtgaacaatcagtttgtggatattctgagccagttcctgaatacgcatgttttcatagaattcaggatcttcacgatacagagacggcagcatgtttttcacacgcaggttcaggtcgaacgcacgtttaaagtcagtcagagcacgcagcaggctcagtgctttggtcttatcgataccgatgctgaacaggaacagcaggttatacggaccggttttctcaacaacgatgccatgttcgtcgaggtatttcgccacgatgctggccggaataccaaagtcgctcatggtgccgtctttttccatccccggagtcagcagggtgactttgatcgggtcaagatacatgtgctcgttatcgatgtttttgaagccgtgccaggtgctgtcagaacgcagcggccagcattcagtcgtatcgatatgatccggctgccatacatcaaagaaccagccatcagattccgttctcagacgtttgatctctttacggaatttgatcgcacgttcaatagaaccgttgatcagacgcttacctgcattgcctttcatcatcgccgcagcggtttcagtggacgccacgataccgtagtgcggagaagtggtggtgtgcatcatgtaggcttcgttaaaggtttcttcgtttacgtcacctttaacgtggatcatggaagcctgagagaacgccgccagcagtttgtgagtggactgggtttcgtaaatcactttcccttctacacggccaccgctcataccgcatttaccttcgtaaatcggtgagaagttggtgtaaggcacccacgcggagtcaaagtggatggatttcacatccagtgttttcttgatgaagtcggtgttgtacagcagaccatcataggtagagttggtaattacagcatgtaccggccaggttgcgtttggtgtttctttcacgcgcttagcaatggtagcgtgctggaattcactctgtgggataccaccaagaataccgtaagcgttacgggtcgggcggaaatagattggcgtaacatcgctcatcatcatcaggtgggtcagcgatttgtggcagttacggtcaatcagaatggtgctgcctgctggagcagagtacataccaacaattttgttcgcagtggaagtaccgttggtcaccatgtagctgcggtctgcgttaaagacgcgagcgatatactgttctgcttctttgtgtggaccactgtgatccagcagagaacccagttcagatactgaaatggaaatatcagatttcatggtattcggaccaaagaaatcatagaacaggctacctaccgggcttttctggaatgcagtaccgcccatgtgaccaggagtacagaaagtatatttaccttcacgaacatatttaaacagtgctttagtcagcggaggcagaatagtgttgatatattcgtcagtggtctgcttgatcttattagcaatatcttcagcagcacccagcgcatattcaaagaagctaatctgtaaacgcaggtcattcaggcttacatcgagagtggaatacgtattagcgaacgcgtacaacggcaggttctcgttcattttgctaatttcttcgcacagctcgagattatatttatcccagtcaaaaataacgccgcacagacgcgcattgttttcgatcagttttaataagtcgtcacggtcgttcgggtaaacaatctggaagttcagacgttcaagcgcgcgatgaagttcacggatgggttcttctttaaaataaacccccatgtgattcaatattgcaataacgttcatagtcatatctccaggtaaaaaaggcccctcccaacacatgggacaaaatgaaaggaggagcctcggaaaatacttttaattaatgtgcgttagacgcggtgtggttatccattgagtggctctggcgctcgtgcattttgcgagcgtagaacatcaggataatcaggctgacgatgaaggtacctgccagctcgaaggagcttgcgcccatcagcgcgatgaagcagaacacgcaacccagtacagagcagatcaggctgacaaagttgcggatgttaacgccttcaaaacgaatcaggtcaacgcaagagtagaaatacggcagcatagtcagcagtactgcgataccggtcagttcaccgaacaggtcagatgctttaccaccggcagagttcatcagagtgataaggatcatcagggcagtcattttcactgcagccagcagcagaccttttttcggaataccgttgctgtcgacttcaccataaactttcgggaagttaccgtcgttagcggcacgtacacctgcctggcctaccaacatcatccaggagcccagagaagtcaggcacgcaaaggcggtgaatgcagaaaccagcggcgcagcccagttaccgaggatagttgaagcactgattgcaaacggagcaccggaagccgccattacagaagacggatacataccggaaagcacctgagtcgcagcgatgtaaacaatacctgctaaaccagtacccagcatggttgccagcggaacggtacgtttcgggtttttaaccataccagtacttacagctgcggattcaacacccacgaaggcccacaggcagagcagaatacttttaatgatcgcatgaccatcagtggtatccgcagtattccagttagctgcataagttgccgcatcaaaccaatgccagccaacaatagcagtcatcaccacaggaataagaaccagcaccagaccaatagtggttaaacggcttacccaagtaccgccgagcatatttacaaaggtaaatacccagacgatagcaatacaggcgatacccgccggaacaggatcatttaatactgggaagaaggtggaaagataagatacagcggtaataccaatcgccaggttaccaatccagttagcatggtaataaagaacacctgtctgaaaaccaaatgcaggggaaatttctccggcataagcaattgggccaccttgttgcgggttttttgttgccagtcgggcatatacatacgccagcgacattgcaccaataatagagataatccaaccccagatagcaataccaccgatacttgctaggttcgcaggtaataatgcaataccgctccccatcatattaccggcaacaacaccggtacaggcaaatagcccgatcttcttggcagaactcatgctcttctcctaatttcatttttgaatttggagtccgggtcatgatgtataactatttcctgaccagaccaaactggcgataagattactcacgaaaaaaggattaatcctaaagattaggtgaaataacacaaaagtttctgtaagtgagaacttgaggttttttattaacacatcaggatcgcaagttgatatcatgaaaagataaacatttaatgtttacaatggattgcgtgacattctctggttaaatttatgtaataaaaattatgcggcaaataaattgccgcaacatattataccaacaggaacatacaaaaactcaacaacaaatatttccgagcataaatcaacccggagttacttattctgaagcaagaaatttgtcgagataaggtacaacataaggaacagaagtctggaatataccattttcaatccagtaaagggtgtttgcccctgggcgtaaattaaaggcggtgagatatgcatcagctgcttcccggttcatccccttcatttcataaaccttgccaagcaacacataatttagccaggacatttcaagatcaatgccagtatttatcgcctggtaagactcatctgttttaccttttaccagagcactgaccgcttttatttgatatataatggacaggttgttcaattccggcagtgtaacaatgttatctatttctgtgttcagtgctgctaattgtttttcatctaaaggatgttgagaatggcgcacgatatcaactaatgctttttctgctctcgcgtaggtaaattctggggatgattgaacaatctcacctaataattcactggcacggttcaatgatttatcatcgccatgcagtaaataatcatgtgcctgataaaaattagttaataacgcaccacgatgcggcaaaattttctggagcgtctcctgcattcgttgtggccacggttggtttaacgcttttgataaactctccagtaaatcattttgaatcgccagctgattaccgttagtgatgacataacgtttatccagcatggttgaaccatctgcattgtctaccaattttatcgacataaagcattgttgagcacggtattggcgctgattaacaaacgcaatagataatgttttaccggaactgctcggttcatcaatgttgtagttgattttgtcatgcaccataaaggtggagaaggtgttaagtgatgtcgccaccaaatcacccacgcctatcgcgtaagagagctgatacggggaactccagctgttacaacttttatttaccatattaatgtcaatatcgcgtggattgagcaaaatacgcgatttgctcataggaagacgtgtatcaagacttgaaaacgctaccagtgctacacagatacctaacgacaacaggaaaaaaaaccatacccaaaaggtagtgaatcgtttgcttttaactggggattgttcaggtggcgttgcggtgttttgaatgttaagactgtgggagggagaatctgtggcaggaaccgcctctggtatagggggaggcgaagatagcattatttcctctccctcttcttcgctgtaccagataaccggcaccattaatttatagccgcgctttggtacagtagcgatatagacaggactatcttcatcattatcttttaatgacttacgtagttctgagatactctgcgtcacaacgtgattggtgacaatacttctcttccagacattatcgataagttcatccctgctaagtacttcgccactgtgttgagcaaagaaaaccagaagatcgattaatctcggctcaagggtaagttgacgcccattgcggctaatttggtttatggacggagtaacaagccattcgccaacgcgaactacaggttgttgcataatagaaactcattcgaaaagggaatgatgcaatgataattgccacaacctatttttaccatctatagatgggtttatttacatattattggtgaatgcaagacgttatttttaccagccataaacttcttgattacatagtattacgaaaggattttactgagaaccagaagtaatattccttaccatcaaaattcatcatctttgccaaagaaaaatgttcagaaaataatccatggaaaattgtccggagcacttactattttaatggattgttagtctttgcatgagcaagcgaactgatacatttctctttgttctcattcagaaaatctcatcagtcgccgttcagaccggtgttgtgctttatggatgcgttacgctcctgatgacgtcatttgacgttcaacagcatcacggggccgcacgacatttcacgtcagttagtgctatagctcaggaacaaattttcccgaattgggatatgcccgcaaattgctggtgatgtggggagaatctggttgagttcggtagaattgatttggaggcagaacgcttaaatcgtggcgtcctgaaacgaaaaacggacctccgtggaggtccgtttatatgaatttggtgcccggactcggaatcgaaccaaggacacggggattttcaatcccctgctctaccgactgagctatccgggcaacggggcgcattaaaccgtaatctgcacatctcgtcaacctaatttcagtaaaagcgattcaactgcttaagattgcggcaaatcgcttcttttctgtgtttctgtcaggtcaatgcaccaccctggcggcagcgggcgaagcgcaggatatcttccgccagccgatgtgcagtgtcgacatccgcctggctacgattcaccagcattcggcttaaacagccttccagcaccagttccatctgctttgctaccatcgccggatcgtcaacttccagtgtggttaacagttcgtgggtgaaatcgtaggccgcgcttttttgctgatcggccagttgatgaatagggtggccaggatcgggataaaacgtacaggcagcgataaatagacagcccggatagcggttgtttttaacgcactccgataacgcctgataacgtgccagcagcttttgttcggcggtttgcgtttcgtccagcatcagctgacgacgccagacatctatctgttggctaagataacgcagcgcatcgtagaggattgcctctttgtctggccagaagcggcgtagctcgtccagtggataatccacacgttcagcaaccatctccagcgtggtgttggcaatcccttgtaattctaataatttcagggcttctcccagtacatcttcacgttgcacgctattttcctccgtctttcccactgcaagtgtcgttcacggttggcgatcgcgcaaatgtgcgctgaaggtttcagcatccataaagcccgtgacgcgtgcttgtggatgctcctggccttgtccgtcaaaaaagagaattgtcggtaggccaaggacattaagatgctttaacagcgccacatcttgtgcgtcgttggccgtgacgttggcctgaagtaagaccgtgtctgctaacgctttttgcacctgcgggtcgctgaaggtgtatttctcaaactctttacaggcgacgcaccagtcggcataaagatctaacatcaccggtttgcctttggcttcaacgagcgcctgatttaactcatctaccgttttgatttgtgtaaagttgagatgcgtctgagtttgcgcggtatgcgtcgcaccaaatgcccaatcctgaagtgggcgcacgctaaccaatgccgctgccagcagaataatttgcacaatacgcatccagccgcgtttagcctgtaggctggtgataaaggcccagccaaagaatgcgacacccagcgccgaccacaagcgtaatccccatacatcaccaatcactcgctccagcaggaagaccggcagtgcgaggatcacaaaaccaaacgcggttttgacttgttccatccacgggccgcttttcggcagcaagcggttaccaaagacggtaattagcatcagcggcaggcccatgcccaacgcatagagataaagcgtgccgccgcccagccacatgttcccgctttgggcgatatacagcagaatcgcgctaagcggtgcggtggtgcatggtgaacagatcagtccggcaatcgcccccataacaaacacaccgccaggtgagccgccctgttggcgattgctcatcaacgtgagacgtgtttgcagcgaagaggggagttgcagggtaaacaagccaaacattgacatcgccagcaaggtaaagacgatggcgaggccaatgagcacgtatgggtgctgtagcgccgcctggaactgtaaccctgcggcggcaaccaccagacccagcgccgtgtaggtcagcgccatcccctgcacataaataaaggtcagcaacaatgctctggcagtggagagccgctgtttaccacccagcacgatgccagaaatcagtgggtacattggcagcacgcatggcgtaaaggcgataccaataccgatcaacaacgcccagagcgcggaaaagggcaattgcgcggtgggctgctcttgctgcggaacagacacaggctgtggcgctgcgttgttggcgaccacttcgcttaacggaacggttttggtttctggcggataacagaaaccggcatcagcacagccctggtaggtgacagttaacgtcgctcccgcactcgcctggttgatggtgacgggaagcgtcagccgatcgcggtaaatctcgcttttgccgtaaaactcatcttcatgccagacgccttgcggcagctgcacgtcggcaattttcgcgtgttccggcgtaatgcggatctgtttacggtagaggtagtaaccgtctttgatctgccaggtcagattaaggtcatgttggttttgctgaaaatcaaaagcaaaggcttgatccgcggggacaaattgtgaacgtcccggcgcgtcgaataatccggcaaaaacggaagtgctgcaaagtagcaggatcagcgtaaagatgcgttgagccatgagaggtaatctgtgtctccgtgtgtaacaggtaaaaccagaagttccggggtttgatatggatgatgagacttcaggcattccagcagtgcctgctggtgagatacggtagtttttaaaatcatctgcacttcgtattcttgctccagcttaccttcccagtaatagagagaggtagcgccggggatcaaggtcgcgcaggccgccagtttttccgccagcactttggcggctaaatcctgggctgtcgcttcatctggtgccgtacatagcaccacgacagacgcggtattcgaacttttttcatcaagcataaacacctcgcaagaacagatggaaccgcaagagagaggtcactatacaacggacgggggaaggatgttagtcggcgggaaagaaagcggggcgtgaacgccccgcgattgatcattacagcatgaagctacccagcacgaagccgaagcaaacggccagggcaacacccagagtacccgggatgaagaacggatggttgaagacgaatttaccgatacgggtagtacccgtgtcatccatctgtaccgcagcaaccagcgtcgggtaggtcggcagaatgaacagaccagacaccgcagcgaaagaagcaacagcggtcagcggtgaaacgttcagtgccagagccatcggcatcagtgcttttgcggttgcagcctgagagtacagcagagcagaagcaaagaagaagatgacggccagcagccacggatgaccctgaatcacttcaccagcggtatctttgatccagtcgatgttgttggaaacgaaagtatcgcccagccacgcaacacccaggatacaaatacaggcgctcatacctgctttgaaggtgctggagttgaggatgttgtcggtatcgactttacagataacggtggtcagagttgcaacgctgagcatgatgatcaggattgcgttggtggtgttcatcagcggtttttcaaccagacccatgcttgggctgttgatgattgcatagataaccacgccaactacgcccagcaggaacagccagacggacgtttttgcaccggatttgatttcaatctgcttttcaccgcgcagttcaaccaggccctcttccagacgcttgcgataaatcggatcgtcagagagtttggagttgaacagcatagtgaccaggaaggacatcaccagaaccgccagcagggtggacgggatgaccacggagagcagatggaggtagctgatgccatgaccttccatcacggaagacatgtaaaccactgccgctgagattggcgatgcggtgatcgcaatctgcgcggataccactgcagtagacagcggacggcaaggtttaacgccttgttccttcgcaacttcagcgataactggcagtgtcgccagagagatgttgccagtaccagcaaagatagtcaggaaataggtcacgatcggtgcgaggatcgtgatgtatttcgggttacggcgcagcagcttttctgtctgatgaaccagatagtccagaccgccagcaacctgcatggcagaaatagcggcgataaccgccatgataatggagatgacatcgaacgggatgttaccgggtttaacgccaatagcggcaagaaccagcacccccaatccgcctgcaaaaccaatacctattccccccaatctggcgcccaagaagatcgccagcaaaactatgatgagttctacaactagcatattagccttccttgttttttaacaagttgatattagattgttatttttaagttactgctcacaagaaaaaaggcacgtcatctgacgtgccttttttatttgtactaccctgtacgattactgttcgctttcatcagtatagcgttttgctttgtaagccgggtgcatcagattctgtacggagaaaatatcgtcaagttccgcttcagtcaacagaccgcgttccagaacgacttcacgtacactcttaccggtttcggcacagattttacccacgatgtcaccgttgtggtgaccgatgaacgggttcaggtaagtaacgataccgatagagttgtaaacgtaaccttcgcacacttctttgttagcagtgatgccgttaatgcatttttccagcaggttgtagcaagcgttggtcagaatgtgaacggattcgaacatggcctggccaatgaccggctccataacgttcaactgcagctgacctgcttctgctgccatggtaacagtggtgtcgttaccgatgactttgaagcatacctggttaaccacttccggaacaaccgggtttactttagctggcatgatggaagagcccgcctgcagttccggcaggttgatctcgttcaggccggcacgtgggcctgaagagagcaagcgcaggtcgttacagattttggacatcttcacagccaggcgtttcagcgcgccgtgaaccataacataagcgccgcagtcagaggtcgcttcgatcaggtcttcagccggtacgcatgggaagccagtaacttcagccagttttttcactgccagcggagagtactctttcggcgtgttcagaccagtaccgattgctgttgcaccaaggttaacttccagcagcagttcagcggtacgttggatgtttttcacttcttctttcagcaggatgctgaaagcgcggaattcctgaccgagggtcatcggtactgcgtcctgcagctgggtacgacccattttcaggatgtcctggaattcgacagctttacgttcaaagccttcacgcagttggttaatcgcatctaccagcttaatcagggaagagtaaactgcgatacggaaaccggtcgggtaggcgtcgttagtggactgacatttgttaacatggtcgttcgggttcaggtactgatattcacctttttggtgacccatcagttccagaccgatattggccagcacttcgttggtgttcatgtttacggaagtacctgcgccgccctggtagacgtctaccgggaactgatccatgcattttccgttgttcaggacttcatcacatgcggcaatgatggcattcgctacacttttaggaatggtttgcagctctttgtttgccatagctgcggcttttttaaccattaccataccgcgaacaaattcaggaatatcactgattttgttgttgctgatatagaagttttcaatcgctctcagagtgtgaacaccatagtaggcatcagctggaacttccctggtacccaacagatcttcttcgatacgaatgttgtttgacatgtgaaccttctttttcaagctgccaatgatttgctttaaacacacagaatatatgtggtttcgaatgtttttcgaccgacgattatcccctgcatcgaccgaatacccgagatcatatgctgcttgaggatttctaccgtaatctggatcactttaagtgtcggtttttaccccttaattattaatttgtgaaatagatcaccgctttgggattactaccaaaaatagttgcgcaaacatcttgaaattttgctaatgaccacaatataagctaaacgcgattcgcaacccattcaggtagccggggttaaccggctgctattacaggagaaacctttgcgctggttaccttttattgccattttcctttatgtctatattgagatttcaatctttattcaggttgcccatgtattgggggtattgctgaccctcgtgctggttatattcacgtcagttatcggtatgtcactggtacgtaaccagggctttaagaatttcgtgctgatgcagcaaaaaatggcggcgggtgaaaacccagcggcggagatgattaaaagtgtttcgctgatcattgctggtttgctgcttttattaccgggcttttttaccgacttcctcggtcttctacttttattgccgccggtgcaaaagcatctgacagtgaagttgatgccgcatttgcgcttttctcgcatgcctggcggcggttttagcgccgggaccggtggcggtaatacttttgatggtgagtaccagcgaaaggatgatgagcgcgaccgccttgatcataaagacgatcgccaggattaatgtcgaaacgccggattatgtggttatgccattttccggcgtttttcgttttggcagcaacagccataaccccgccagcatgatcagcgcatagagacttttccagccgaccattgccagtaacagaacgcataacagcccgccaaccaccgccagtagtcgataacgtccttgcaataatttacagcctgccagcatgcataacagataaatcataataaagatgccattggcataaataataagagcgtccagattgatctctaaagcatgaatcaccaaagtgctcaccacacagcagccgagcaccgcattgagggcattattcgggatatggcgagaagagaggcgtgccaggtagtggtcaggattatgttgcgcctgcgaccagaccaggcgggcgaagctctgtatataaatgttgagactggcaaagcaggccagatagccaatcacgcaggcaatccataacgctcctacaccgaacaactgcactacaatttttggaagcgatgctgccgccgccattttttcaccataggcgtcgaagtgtaagacgactaccgtacagccccagtagactaatcctgccagcagcagaccaatcatcaaagcacgaggaaaatcacgctctggatttttaaattccgaggcgagatgggcaaatgcctccagaccgacaaaacaccagaacatcactgataacgcagcaaataacccggtaagttcgatattaccaggtgccggaaaggggatattcgcaggtttgatatcgcccgcccaccagatagcgacaatcagcgcgacgataagtccggcaataacggtttgtagattagcactggaactggcaccgcgagtaccgatataccacaccagcgccagcgtaccgagttctgccaacaacagttgccagctatgccagccaaacatcgcctggccgaacccggcggcaatttgtagtgcggcaggcaaacccacgggaatgaccgataaaaacagccagccggtgactcgctcaagccgcgaaccaaacgccataccgacgaagtgcgcgacgccgcctgcgctgggatagtggcgacccagaatcgcaaacacaatcgcaatcgggaacactaagataatcaaaacgggccacgcccacaggctgttattgcccgctaccagcgcagctaacgcaggaacggcaaacacgccagtgcctaataatgacgtcgatagcaggccaatgccctgggccagccccagttcttgtttgagtccactcatgggttgatgtccgattgcgcccaaattttgggcaactgcgtagattttcgatggtagcacaatcagattcgcttatgacggcgatgaagaaattgcgatgaaatgtgaggtgaatcagggttttcacccgattttgtgctgatcagaattttttttctttttcccccttgaaggggcgaagcctcatccccatttctctggtcaccagccgggaaaccacgtaagctccggcgtcacccataacagatacggactttctcaaaggagagttatcaatgaatattcgtccattgcatgatcgcgtgatcgtcaagcgtaaagaagttgaaactaaatctgctggcggcatcgttctgaccggctctgcagcggctaaatccacccgcggcgaagtgctggctgtcggcaatggccgtatccttgaaaatggcgaagtgaagccgctggatgtgaaagttggcgacatcgttattttcaacgatggctacggtgtgaaatctgagaagatcgacaatgaagaagtgttgatcatgtccgaaagcgacattctggcaattgttgaagcgtaatccgcgcacgacactgaacatacgaatttaaggaataaagataatggcagctaaagacgtaaaattcggtaacgacgctcgtgtgaaaatgctgcgcggcgtaaacgtactggcagatgcagtgaaagttaccctcggtccaaaaggccgtaacgtagttctggataaatctttcggtgcaccgaccatcaccaaagatggtgtttccgttgctcgtgaaatcgaactggaagacaagttcgaaaatatgggtgcgcagatggtgaaagaagttgcctctaaagcaaacgacgctgcaggcgacggtaccaccactgcaaccgtactggctcaggctatcatcactgaaggtctgaaagctgttgctgcgggcatgaacccgatggacctgaaacgtggtatcgacaaagcggttaccgctgcagttgaagaactgaaagcgctgtccgtaccatgctctgactctaaagcgattgctcaggttggtaccatctccgctaactccgacgaaaccgtaggtaaactgatcgctgaagcgatggacaaagtcggtaaagaaggcgttatcaccgttgaagacggtaccggtctgcaggacgaactggacgtggttgaaggtatgcagttcgaccgtggctacctgtctccttacttcatcaacaagccggaaactggcgcagtagaactggaaagcccgttcatcctgctggctgacaagaaaatctccaacatccgcgaaatgctgccggttctggaagctgttgccaaagcaggcaaaccgctgctgatcatcgctgaagatgtagaaggcgaagcgctggcaactctggttgttaacaccatgcgtggcatcgtgaaagtcgctgcggttaaagcaccgggcttcggcgatcgtcgtaaagctatgctgcaggatatcgcaaccctgactggcggtaccgtgatctctgaagagatcggtatggagctggaaaaagcaaccctggaagacctgggtcaggctaaacgtgttgtgatcaacaaagacaccaccactatcatcgatggcgtgggtgaagaagctgcaatccagggccgtgttgctcagatccgtcagcagattgaagaagcaacttctgactacgaccgtgaaaaactgcaggaacgcgtagcgaaactggcaggcggcgttgcagttatcaaagtgggtgctgctaccgaagttgaaatgaaagagaaaaaagcacgcgttgaagatgccctgcacgcgacccgtgctgcggtagaagaaggcgtggttgctggtggtggtgttgcgctgatccgcgtagcgtctaaactggctgacctgcgtggtcagaacgaagaccagaacgtgggtatcaaagttgcactgcgtgcaatggaagctccgctgcgtcagatcgtattgaactgcggcgaagaaccgtctgttgttgctaacaccgttaaaggcggcgacggcaactacggttacaacgcagcaaccgaagaatacggcaacatgatcgacatgggtatcctggatccaaccaaagtaactcgttctgctctgcagtacgcagcttctgtggctggcctgatgatcaccaccgaatgcatggttaccgacctgccgaaaaacgatgcagctgacttaggcgctgctggcggtatgggcggcatgggtggcatgggcggcatgatgtaattgccctgcacctcgcagaaataaacaaacccccgggcagaaatgtctgggggtttttcttttggtcatctttctagtataagattcagacacggacgacgcgagtggcgtccagctcattgattatggggaataacatgcacgtaaaatacttagcagggattgtcggtgccgcgctactgatggcgggttgtagctccagcaacgaattgagtgctgccggtcagagtgtacgcattgtggacgagcagccaggcgcagagtgccagctgattggtactgcgacaggtaagcaaagcaactggctttccgggcaacacggagaagaaggcggttctatgcgcggcgcagcaaacgatctgcgcaaccaggcggctgcaatgggcggtaacgtgatttatggcatcagtagcccgtcgcagggaatgttgtccagttttgtcccgacggatagccagattatcggtcaggtttataagtgcccgaactgatgtgatccagaggctgggtgacaaacgtataattgcctgatgcgcttcgcttatcaggcctacataaggcattgcaactgattgaatgcttgagaatttgtaggccggataaggcgtttacgccgcatccggcatgaccaacgatcacgttatcagtcatttcaggctggatggctccagcctcgcattagcaaagatgagattatttcgcctgtggtgcagttttgctggtggattgaacacgtaagtgatgcagcgcgcgtaagcattgatcctgggttagcggttgggcgttattcgccgctacggtgcgaacatagacctgacatggcacacccgcgagttttttcagtcgtgggctgaaatcaagcattcggcgagtgatcgcttctatttctttacccggcgttgcttcacgcgttttcaccactgcgccgctaaattgttctttgccactttcatctttaaagcggtaaagcaccgccagataatggtcgaacaagttatgtttccattccggttgggaataggtgtcatattccagattgccattgtcctggcagtcaacgtcgtataacggcaggaaatctaacagtgaggtaatacgtaatgccagttcacgcatttccgcattattaattgcatgaatgattgctcgcgccagcatttcaatctgcaactcattgacgactaactcacatttgctaccgtcatgtagcgttaatacgaaggtaagattttcgccttgattatcggtaagttccagcgtgttaacccgacgattaatatcggcatttttaagctcatcaaccagaatttctgggatgttttctgccattttcttaatgactttatcgcgagcttgctcatactgaaggtgtgcagcagcatccagtttatgcttttgatgcagacgactttccagcgcaatcagcaggtcgcgcagttccatgacagacataaagaacaacgattctttattgcgaggttctttaattttcagcgccagtgcaatgaaattattactcttgcgaataacaccggtattaacacccttgatgcttatggccatgtaggttctccctaaccatttctcaattaaataattaattttaatttataagccagataaatgggcttggtagtaatagttgttaaaataacataaatagccgtactcactctatataaacagaaaagaaaggttaattattggtgttagctatataaaaagtaacaacagcaatgcatatgaataattaaaggttatgcaacgggcaaagattaaacttcccagtttaatgacaggttgctgtacttgcgtttgttgctcttgccggatgcagcgtaaacgccttatccggcctacagttcattgcaaatccattcaatttcaatgcacgatgtaggcctgataagcgtagcgaatcaggcaattttaatgtttaacttccctgtttaatcagttactgctggcgtagctggagatccagcggcgttttgctgggttcgccgccaatttctcgcgccagtttcggcaccagatatcccgacaccagtgtcagcaactcacgcataatctgccgtgcttcgtcatcactcaccataaaatgcgccgcgccctgtactttatcgagcacatgcaggtaatacggcattacgccggcatcgaacaacgcattactcaggtttgccagcgtttgtgcgttatcgttcacatcacgtaacagaacgctctggttcagcaaagtaacgcctacccggcgcaacttagccatcgcctgacggaatgtttcatctacctcattggcatggttgatgtgattcaccagcaagatttgcagcgtagaacgggcaaagcattcaaccagcgcctcggtgatacgtgccgggatcacaatcggcagacggctgtgaatccgcagacgttttatatgcgggatggcttccagttgtgtgagcaaccagtccagctcgtgatctttcgccatcagcggatcgccgccggagaaaatcatctcgtccagttccggatgcgcagcaacatactcaagtgcagtttgccagttacgcttgttgccctgattttcggcataggggaagtgacgacggaagcaatagcggcaatttaccgcgcagccgcctttgaccagcaaaagcgcccggttgtggtatttatgcaacaaaccaggcactacgctgtgctgttcttccagtgggtcggtggagaatccgggcgcgatgacaaactcatcttgcgaggtaagtacctgacgcaaaagaggatcgtccggattgcctttctccatgcgatcgataaatgagcggggcacacgcagggcaaaaagctttttggcgctgcgtccggctaacagtttttcctccgcgtctatattcaaaagacgcagaagttcatcaggatcggtcacaacatcggcaagttgcgttaaccaatcttctctggatggggtatttagggttacaatatgcgccattttgtggcttagctaccaattaacaaatttcagagggccttatggcaacgtactatagcaacgattttcgtgctggtcttaaaatcatgttagacggcgaaccttacgcggttgaagcgagtgaattcgtaaaaccgggtaaaggccaggcatttgctcgcgttaaactgcgtcgtctgctgaccggtactcgcgtagaaaaaaccttcaaatctactgattccgctgaaggcgctgatgttgtcgatatgaacctgacttacctgtacaacgacggtgagttctggcacttcatgaacaacgaaactttcgagcagctgtctgctgatgcaaaagcaattggtgacaacgctaaatggctgctggatcaggcagagtgtatcgtaactctgtggaatggtcagccgatctccgttactccgccgaacttcgttgaactggaaatcgttgataccgatccgggcctgaaaggtgataccgcaggtactggtggcaaaccggctaccctgtctactggcgctgtggttaaagttccgctgtttgtacaaatcggcgaagtcatcaaagtggatacccgctctggtgaatacgtctctcgcgtgaagtaatgcggttgtggtgcggcctgcaggctgcaccatcacttattcaggtcagagatgatgaaacgccttatcgttcttgttttgcttgccagcacgctgctcacgggctgtaacaccgctcgcggtttcggcgaagacatcaaacatctcggcaactccatctctcgcgctgccagctaatttttcttctcttccgaaaaatcatcagattcccatcatttttggcgatgttgtctattattaatttgctataggcaaacataaataacattacctaaaaggaagacgttatggtgaagaagacaattgcagcgatcttttctgttctggtgctttcaacagtattaactgcctgcaacaccacgcgtggcgttggtgaagacatttctgatggcggtaacgcgatttctggcgcagcaacgaaagcgcagcaataagcaataacggtacgacagctgtgtcgtgccgtttgttttttctgcgatagtcacaaaggtaatagttgaaattcccctgccacctggcaaaatatccgttcaaccatcagctttgcaggacgacctgcaaacgcctcttttcaccggggacggccccaattctccggagcctgatatgtcctggattatcttagttattgctggtctgctggaagtggtatgggccgttggcctgaaatatacccacggctttagtcgtttgacgccgagtgttattactgtgacggcgatgattgtcagtatggcgctacttgcctgggcgatgaaatcgttaccagtagggacggcttatgccgtgtggacgggtattggcgcagtcggcgcggccataaccggcattgtgctgctcggtgagtccgctaacccgatgcgcctggcgagtctggcgttaatcgtattggggattattggtctgaaactcagcactcactaactaccaggctgctgtacccaaataaatttactgacatcaaacccttcccgggtcgcgactgccagcatctcctgtttcacttcgtcagaaatggttggcgtgcgggagagtatccacaggtagtcgcggtccgggccgcaaaccagcgcatggcggtattcccgatcgagtgcaataacgttataaccgccatagaaaggaccaaagaatgacactttcagcgcagcgcgagttggtgcgccggtaaagtacgctttcccttcactctgctgccacattcctctgtcagggttatagcctttattaatgacattcaggccgccgtcatcacgcaggctgtatgttgcggtgactttttccagtccacgttcaaagcggtgatcaaaacgggcaatctcataccaggtaccgagataacgtttggcgtcgaaattatttactacggtcacgccacgcggcggcgtaggagaactgcaggcaacgaccagaaatgcagctgtcgctgcggcaacgagagggagcaggcgcataaatgtttccttactggtttttttctaagtgtagatgacagcaaggaaaagcggagaaaaggtccgaaaattcggacccgatggaattttactgtagagcgttaagaatctgccaggcggcgtcgactctcgctggattgggatagtttttgtttgccagcatcacgatacccagctctttttctggaataaacgcgacatagctaccaaatccgccggtcgcccctgttttatgtacccatgatgcgcgtactgcaggagttgggggcgtaatcgcttttacggggcgtgctgccagtgcaattttattgtcactgccgttaatgatgctgtcaggatttaccggccagtccagcatttcccagcccaggccctgatacatatcgccggtttgccagtagcgagattgtgccagttgtatcccttgttgaagcgttttctcattgatatcaaggggttttaaattgctttgcacccagcgggccatatcttcaatggtcgacttcacaccataagcttcagcatctaacgccccaggcgaaacatgcactgccttaccttcgcgatatccccaggcgtaattcttttcttctgcgggcggtacattaatccacgtatggttgagtttgagtggctggaagacacgagtttgcatcgcctgctcaaaactcaaaccagacggcttcacagccagtgcgccgaacaaaccgatactggagttggcatacagacgttgtgttcctggagcccatgcaggctgccagttttgatagaagcgcagcaagtcgcttgaggatttcacctcatccggcacctgcaatggcaggccgccagcagtgtaggttgcgagatgtaatagtgtgatcccattccactgtttagcggtaagttcaggccagtattttgttgtgggatcgcttaacttgatttcccctcgagcaatagcgtcgccaccaagcacgccagtaaatgttttgctgaccgaacctaactcaaacaacgtttgctgtgtgacgggctgctttttggcgatgtccgcatagccccaggtaaagtaataaggtttaccctgataaattaccgccaccgccatacccgggatcttttgttgctctataagcggggtaattgtgcgatgcacaatatcgttgatttgttgaggggcagcaaatgtggagcaagaggcggtaattaataaggcgcagagcgtcgttttgaacatagggtctggtttccatacaaaacggcccgccataggcgggccggatttacattggcgatgcgttagattgtaacgacaccaatcagcgtgacaactgtcaggatagcagccagaccgtagaaaacccatttgcccgcaggtacgtggattttcagatcgtgcatcgcgtggtgcatacggtgtaaaccacaccacagcggcagaacgatcatcaggaacaggaatacgcgaccaatgaagctctgcgcgaacgccagaacgcgctcgtagctcagcgcatcacccggaaacaaccccagtggcagcagaatacccaccagcaggatcatcaccggcgcaatgatggcgctccacataccaccggccccgaagaggccccagaataccggttcgtcagaacgctttggatttggattaatcatctcaggctccttaccagtacagggcaacaaacaggattacgatggtggcaaccacagttaccgcccagagacttttgataattggctctggtcccattttttcgtcttttacaatgatattggccgctttcggtgccagttcaaaccaggttttggtgtgcagcagagctgccgccagagtgatcaggttaatgatcacgataaccgggttttgtaaaaagtcgacgaatcccgcccaggcttccgggccatttttcagggcaaacagcccgaaaatcagttcaatgctgaaccacacagccggaaccgccgtgccttcgcgcagcatgtaaaagcgataaaacggcaattttttccaccaggtggacgtcattggccgtacatacggtttacgtttagtcgtcatgttgcactccttagcgtggtttcagggtcgcgataagaaagtctttcgaactttctactttgccctgctgaatggccgcagccggatcgacgtgtttcgggcagacttcggagcagtagcccacgaaagtacagctccatacgccgttctggctgttcaactgcgccatacgctccttcttaccgtggtcgcggctatcttcgttataacgatgcgccagcgtaatggcagccggaccgatgaactctgggttcaggccaaactgcgggcacgcggcgtagcacaaaccacagttgatgcaaccggagaactggtgatacttcgccatctgcgccggggtctggatgttagtaccctgatccgcggtgcgggagttgccgatgatgtacggtttgatcgcttccagactttcgatgaagtgggtcatatcgaccaccagatcgcgttcaatcgggaagttagctaacgcttcaaccttcataccgtcggtgtaatcacgcaggaaggttttacatgccagttttggcacgttgttaaccatcatgccgcaggaaccacaaatcgccatacggcaggaccagcggtagctcaggtccggtgccaggttgtctttgatgtagcccagcgcatccagtaatgaggtagttgcgtcataaggcacttcatagaatgcgctatgcggtgcggtatcgacttccgggttatagcgcaccacctcaattttcaggtttttcatctcagccattcgccttctccttcttattggctgcttccgccttatcggctgcatccgcttcgccaccgtaaacgcgtttagctggcggcagcgtagtaatcttcacgtcgctgtactccaggcgagtcgtgccatcagcatcgcggaaggcgagggtgtgtttgaggaagttgacgtcgtcacgctcggtgcaaccttcgtccagacgctggtgcgcgccgcgggactctttacgtgccattgcggagtgcgccatacattcagcaacgttcagaccgtggcccagttcaatggtgtagagcaggtcggtgttgaacacgctggaagtgtcggtgatgcgcacgcgcttgaagcgttcctgcagctctgccagcttgtcgatggttttctgcatcagttccggcgtacggtagataccgcagccttcttccatagccaggcccatttcgtcgcggatcttcgcccagttttcgccgccatcctggttaaccagatctttcagacgttgttcaacgccagctgcctgcgcttcaattgccgcttcgttgccattaccggcagttgctgcacgctctgtcgcttgttcaccggccagacggccgaagaccaccagttccgccagggagttagaacccagacggtttgcaccgtgcagaccaacagaggaacattcacccacggcgaacagacctttaatgcgggtttcacagttctgatcggtttcgataccgcccatggtgtagtgtgcggtcggacgtaccggaatcggttctttaaccggatcgacgccaacgtacgctttcgccagttcgcagatgaacggcagacgttcatgcagttttttctcgccgaggtgacgcaagtcgagataaaccacatcgccacgcggcgtggagatggtgttgcctttacgccattcgtgccagaaggcctgagagactttgtcgcgtggacccagttccatatatttgtttttcggctcgcccagcggagtttccgggcccatgccgtaatcttgcagataacggtagccatttttgttgaccagaataccgccttcaccgcggcaaccttcggtcatcaggataccggaacctggcagaccggttgggtgatactgaacgaattccatgtcacgcagcggaacgccgtggcttagcgccatacccataccgtcaccggtaacgatgccgccgttggtgttgtaacgataaacgcgacccgcaccgccagtagccataacgaccgcgttagcacggatctgcaccagcgtgccttccatcatgttcattgctaccaggccgcgaacatgaccatcatcaaccagaatatccagcacgaaatgttcgtcaaaacgctggatctgcgggaattgcagagaggtctggaacagcgtgtgcagcatatggaagccggtcttatcggcggcgaaccaggtgcgctcgattttcatgccgccgaagcgacgtacgttgacgctaccatccgggcgacggctccatgggcatccccacagttccagttgggtcatttcggttgggcagtggtggacgaaataatccacgacatcctgctcacacaaccagtcgccacccgctactgtatcgtgaaagtgatattcgaagctgtcatgatcctgcgcgacagcggcggagcccccttctgcagcaacggtatggctacgcatcgggtatacttttgagattagtgcgatttttgcattcggatttgcctgcgcggcagcaattgcagcacgtaatcccgcgccaccggcgcctacaatggcaagatcggcttgaaaggtttgcacgacattcctccagattgtttttatcccacagccacgtacttcagggtaagtacctgaaagttacggtctgcgaacgctattccactgctcctttataggtacaacagtatagtctgatggataagtctgaaatttgacgagatcgatttttttagtgcgcaagagggctaaattatcactgaagatgattaatttaattactaaaccatcagatcgtgctttttttagtcactgcccaccgctgtttgattcctgcgtaaaatttgtctcgccgtcgcgttgcgagtagacttcgtgcccttgtcaaaaactggagatttaactatgagcgaaacggcatcctggcagccgagcgcatccattcctaacttattaaaacgcgcggcgattatggcggagatccgtcgtttctttgccgatcgtggagtgctggaggtggagacgccttgtatgagccaggcgacggtaaccgatattcatttggtcccgtttgagacacgtttcgttggccccgggcattcgcaggggatgaatctctggttaatgaccagcccggaataccatatgaaacgcctgctggttgccggttgtgggccggtattccagctgtgccgcagcttccgtaatgaagagatggggcgttatcacaaccctgagttcactatgctggagtggtatcgaccgcactatgatatgtaccggttgatgaacgaggtggacgatctcttacaacaggtgctggactgcccggcagcagaaagcctttcttatcaacaagctttcttgcgttatctggaaattgacccgctctctgccgacaaaacgcaactgcgggaagtcgcagcgaaactggatttgagcaatgttgctgataccgaagaagaccgcgacacgctgctacaattgctgtttacctttggcgtagagccaaatattggcaaagaaaaaccgacctttgtgtaccactttccagccagccaggcatcactggcgcaaatcagtaccgaagatcatcgggtcgctgaacgctttgaggtttattataaaggtattgagctggcgaatggtttccatgaattgacggatgcccgtgagcagcaacaacgctttgaacaagataaccgtaagcgcgcggcgcgcggtttgccgcagcaccccattgaccagaatctgattgaagccttgaaagtcggtatgcctgactgttccggcgtggcattaggtgttgatcgtctggtgatgttggcgctgggcgcggagacactggctgaagtcatcgcctttagcgttgaccgggcataattctgaaaaattactgaattaacagcgaagaatggcgtgataagcgccattctgtagcatatgttttcatttttccgttaaaggccacaatttaagactggatatttgatatcatccaggtatcaattctgtattggtttttacgctgcctgctcaatgttgcgcagtgcagttcagtgggcacgtgttatacacgcgctgaaatgaaggatggtttcatgcctcacacgataaaaaagatgagtctgataggactcatattgatgatctttacttccgtatttggatttgccaatagcccatcggcttattacttaatgggttatagtgcgattcccttttatatattttctgcattgttattctttattccattcgccttaatgatggctgaaatgggagctgcttatcgcaaagaagaaggcggtatctattcctggatgaataatagtgtcggaccacgttttgccttcattggtacgtttatgtggttttcctcttatatcatctggatggtgagtacctccgcgaaagtttgggtaccgttctcaacattcctctatggtagcgacatgacccagcactggcgtattgccggactggagcctacgcaggtggttggtctgctggctgtggcatggatgattctggtcaccgtcgttgcttctaaggggattaataaaattgcccgcattactgcggtgggcggtattgcagtaatgtgtctgaatttagtattgctgttagtaagcattactattttgttattaaatggtgggcatttcgcgcaggatattaatttccttgcatcaccgaacccgggttatcagtccggtctggcaatgctatcgtttgtggtatttgccatttttgcctatggcggaattgaagcggttggtggtctggtcgataaaacggaaaatccagaaaagaactttgccaaaggtattgtttttgccgctattgttatttcaatcggttattcgctggcaatatttttatggggcgtcagcacaaactggcagcaggtattaagtaatggttccgttaacctcggcaatattacctatgtgctgatgaagagccttgggatgacgctgggtaatgcactgcatttgtcacctgaagcgtcattgtcgctgggcgtatggtttgcgcgtattactggactttcgatgttcctcgcctataccggtgcgttctttacgctttgctattcaccgttgaaagccatcatccaggggacgccgaaagcattgtggccggaaccgatgacgcgcctgaatgcgatggggatgccgtctatcgccatgtggatgcagtgcgggttggttactgtcttcatcctgctggtttcgtttggtggcggtaccgcatcggcgttctttaacaagctgacgctgatggcgaacgtgtctatgacgcttccttacctgttcctcgcgctggctttcccgttctttaaagcacgtcaggatctcgacagaccgtttgtgattttcaaaacgcatttgtcggcaatgattgcgacagtggttgtcgtactggtggtgacatttgcgaacgtcttcaccatcattcaacctgtggttgaagccggagactgggacagcacattgtggatgattggcggccctgtcttcttctcgctgttagcgatggcgatttaccagaactattgcagcagagtggcaaaaaatccgcagtgggcggtggaataacccgatgccctatcgtctacctgacgatagggcgtaaagacaggaaatgttatggatgacaccagccgggacccggcaataaccgaagatgaaatcagggcgctgcaattttctgccggggatgtagcggaaatagagcagacgattctctcttttgtcgatgcctgccacacccgtaaagtggcgatggtggtgggtagcaccattaacaccctcaaagatcgcgatggtaaacggtggggaaacctgccggatatttattgcgcttatcttatccgatgtctggtttttcgcggggaattagtgggatacggcgatttgtttcgtatgcgctatagcgaaattaagcgaccggttaccttatgagtgcgcgcatgtttgtcttatgctgcatctggtttattgtggcgttcctctggataaccatcacttccgcgctggacaaagagtggatgattgatggacgcgggattaacaacgtctgcgatgtgttgatgtatctcgaagaagacgatacccgtgatgttggtgtgataatgacgttaccgctctttttcccttttctctggttcgctttgtggcgaaaaaaacgcggctggtttatgtacgccaccgcgctggctattttcggctactggctgtggcagttttttctgcgctatcagttttgtttgtgagccggattggttcatccggcacacaaacttacaaacttcccgcctgacgacctttgcccgcagacgtcagcgttctccccgtttgtttaccgttgaggctttccagacgcatctggaagggcgggaatggcatatcgataccgtgggcatggaagccagccagaatcagctggtggatctcatggcgtagcggcatacggtgacccatctcagcggcgtaaatacgcagctcgaaaatctgaatcccctgttgcagatccaccaggaagacttccggtgccgggttgtcgatcaccagcgagcagcgacgcgctgcggtgagcaggatttccgtcacttcttcgctattggcatcggcaggggccggtatcgtcaacaccacgcgcgtgaccgagtcagagagcgaccagttgataaactgctcggtaataaacgccttgttcggcacgattatctctttacggtcccagtcgctgatggtggtggcgcgggtgttaattttcgtcacgctaccggtgagatcgcgaattgtcaccgtatcgccaatgcgaatcggtttttcgaacaggataatcagaccagagataaagttggcgaaaatttcctgcaaaccaaaaccgagaccaacaccgagcgcggcaaccagccactgcaatttcgaccactcaataccaatcattgagaagccgaccagcccgccaatcagcatcagcagatatttggtgatggtggtgatggcgtaacccgtacccggcgttaaatccaggtgctgcaaaatcgccagttccagcagcgcgggcaagttgcgcaccagctgcgtggtgatgataaacaccagaatggcaatcagcaccgcaccgagggtaattggctccagactttctacgccctgtaccgtggaggtgacatcccacagcgaaatattttcgaggaagccgaaagcggaatggatttctgaccacagcacaatgacagaaagcagggcgatcaacatcaaaattgagcgcaccagccgcaaggattgcgcactgatggcatcgagatcgacttcgctttcatcgacttcaattgctccttccgggctactgtgatgatgcgcttcctcttcgccacgcgcacgttgcgctaacatctctgcccggcgatgcttcgcccgatcaaacgccagcctgcggcgctggatcagcatccagcggcggataacgtgataaaccaccagtagcaggaaccagatggcaaccgaggtttcaagcctcgctaacagcgcctgtgccgttgccagataacccaccgccgacgccagaatggcaaccaacggcgcgccaatcatcatgttccacagcatatggttggtaatgttgtcgccgctgccctctttgttgagatacagcggaatcccggcctttttcaggctgagggtgaccaccgccagcgcaccgcaaatgaggataaagcaaagccgtcccagcgaaccggagaattcacggtcgtcgaggttatcgaacatcatcagcgccataatcagcggcacaataagcccgatgctcatcaggtagtagcgcatcccacgggaaacacgttcgcgcggccagccaaaatgagcgataaacaagccgttcgggcgggcaaaggtggcgcaaatcatcactacccacagcagcggcacggtggccgttacaccatcgccaatcgcgaccgccagcggataaggccacgcctcgcgcaagccgtaacccagcgtcatccacagcaccggtaacggtgacgcgacgagaatcgaccagaaaagagtgcgcaacgtcagccagaagtgatcctgagtcactttgccaactttcgccgccgaacgttcaagaaaacgggtgaaatagcggcgcgagtaaatactgcaaccgaccagaatcaacgcgccaaacagcggcaaaattgtctctttgctggtcagcatcatcacactggctttgcccaactgactgaaggtgtccagcgaaatgagacgacgcagatcctgggcgatttccagcggccaggcgatggtcatcgggcgcacgtcagaggtccagaacagatagcggtgcgttgcttcgttcacctctttcagcgcatcctccagttgcccgttggagactttcagcttggtcagttccaatagtagcgtgtcgccaccctgcaacaatgagttcagcaactcacgctgagtgcgcagttgtgcttccagaatacggttttgctcggcagtcagcggctgaccgtcggcctgatgaatttgccgtagcagcggctgtttattaagcagatcctcataacgtaaccgttgcacacgcaactgcgccatttcggtatcaagctgttgtggtttcggcatttccggcagccgtgccacctgcgcccgcagcgcttcgccgagcagattggacgatcccagccattgcgactgttcacgcagcgtattcaacgcctgccggacctgtaacgtctggctggcagcctgacgctgttgcgaggcaacgagatccatccgctgcgcctgttgattcaaagccgccgatagttcgcggttaattttgaattgcgcgacgatatctttcggcaaatcggcgctgttttctgccagcaattcggtactttccagcgcccgctccgcctcaagctgacgttggctgtttaattgattacgcaaggcctgcaaatacgcatccagttgctggctctctttttccgccagctctgagcgtaagcgcgctaattcctggcggttattggcagacagctgcgccagctccagttcatcaacgagcgccttaagacgtgcagagtcagactgcaacgcgaaattttgtgcctgattgagcggagtattgccggtaagcgttcccaggcggcgctcgatctcatttaactgacggcgggcgtcggtttgctgttgcggcagttgattcagcgaatcggcaatctcgcgggcgcgctcctgctcttgctgggcctgacggcttttatccagcaactggctgctgacctggagaatttcctgattcagcgcgtcggtagacattcccggcgacacgctgcgcggctcgtcacgcatgttgtttaattgtgcgcgcagagtagcggagagtttcggataattatcgataacttgctgatattgtttgatgcgctcaagggaaccttttcgttcctcaagcgcatttaaggcagactggagcgcctctacgacttccggctgtgcgggtttcgccgcttttgcctgctccagttcctgagtgatttgtttgctatcgggggccgtcgcggcgtacgccccccaactgaggcaccaggccatcagaaaagtgataatcaggcgcacgtcagcgtttcctttgatggattagacctggtcttttttgtcgtcaaccaatgggctggcgtcgtgttctgcttcgatctcttcagcaggaagcggggcaggttcagcgtctggcgtaacaaaggtttcggtagatactgccagcggctggccaattttcgtgacagacaggctttccagttgctcaaccagattcactttacccggtgcaaacaggttgataacggtggaaccgagtttaaagcgacccatttcctggcctttcagcagtgccacagaaccgtcgttttccccggcaggccaggtccagcgcttgatgataccttcgcgcggcggcgtaatggtgcccgcccagaccgtctcaatgctgccaacaatcgtcgctccgaccagaatctgcgccattgggccaaattcggtatcgaaaaggcaaatcacgcgttcgttacgggcaaacagattcggcacgttctgagccgtgagatggttaacggagaagagatcgcccggcacgtagatcatctcacgcagaataccgttgcacggcatgtgtacgcggtggtagtcacgcggggagaggtaagtggtcacaaacgtaccgttgcggaacaggtccgccatcagatagttgcctgccagcagggcttcgaggctgtagttgtggcctttggcttgcaggattttatcttcttcgattttacccaactggctgataacgccatcggcaggcatgaccagtacattcggatcggtatcgattgggcgtacttcgtcacgcagcggacggacaaagaattcgttaaaggtgcggtagctggcggtgtccggcttttgcgcctctttcatgtcgaccttgtagtatttaacgaacagatcgataaccagttttgtcagccatcctgcccgcttgcttgcgccccaacccgccaggcgagtaagccatagtttcggcagaatgtactgtagcgaaagtttaaatgaatttaacaaggtagcctccaggccattgttttgtcgttcctgatccggcctacatgccggatcctgaaaaaaaggggacgattctaacgacggttagcttaattgtcagtcatccgtatcagaaaagtttttacgcgtttttacctgcgccatgctttccagaatacggtgatagttttcgaaacgggtttccgcgattttcccttcctcaaccgcttcccggatagcgcagcccggatcggtatcgtgtttgcaatcgcgatatttacacagacctaaatagtcatggaattcgacaaagccctgagtgatttgttccggctccaggtgccagaggccgaactcacgcactcctggggagtcaatcacatcaccgccgtgcgggaagtgatacagccgagcggcggtcgtggtgtgctgaccgagccccgagttgtcagagatatcgttggtcaggatctctttttgcagccccagcaacgcattcagcaggctggatttgccgacgccagactgcccggcaaaaatgctgatgcgcccggtcaacgcctcttccagcggttttagcccatcctgagtatggctggaaaccatcaatacgcgataaccgatattgcggtagatatccatctgctcgttgacgaacgccatgccttcgtcgtccagcaggtctatcttgttgagcacaataatcggctcaatctgcaaggtttcgcaggccaccaggtaacggtcgataatattgagcgacagctccggcaaaatggcggagacaatgacaatctggtcgatgttggcggcaataggttttacgccgtcgtagaaatccggacgcgtcaacaccgaggtacgctcatgcaccgcttccacgatccctttgacatttacgccttccgccgccggtttacccggacgccagactacgcggtcgccggttaccagcgaacggatggtacggcgaatattgcagcggtgaacgtcgccatcggcggattccacatcagcgtgcataccaaagcggctgatgacgataccttcatcaggctcgccaaacagattgtcgtcgtagtcgggcttctccttagacgttttaagacgacgctggtgattggcgttcacgcggcgctgctggcctttggagagtttatttttactcaatcgtacagactcctggtcgcccctgatgggcaaaacatctatgatacacgcaattgtggatcaatatagtcactgtgaatgggtggaaaatagcatgagtgccaatgaaaacaacctgatttggatcgatcttgagatgaccggtctggatcccgagcgcgatcgcattattgagattgccacgctggtgaccgatgccaacctgaatattctggcagaagggccgaccattgcagtacaccagtctgatgaacagctggcgctgatggatgactggaacgtgcgcacccataccgccagcgggctggtagagcgcgtgaaagcgagcacgatgggcgatcgggaagctgaactggcaacgctcgaatttttaaaacagtgggtgcctgcgggaaaatcgccgatttgcggtaacagcatcggtcaggaccgtcgtttcctgtttaaatacatgccggagctggaagcctacttccactaccgttatctcgatgtcagcaccctgaaagagctggcgcgccgctggaagccggaaattctggatggttttaccaagcaggggacgcatcaggcgatggatgatatccgtgaatcggtggcggagctggcttactaccgcgagcattttatcaagctgtaaaatttttcctggtcacgtaagcgccggaatccacttgcggcggcgtgattttgacgctaaattgaacgtcttgctgataatttcagcacttgagataaaaacgcaaaaaaaacttttttggggggttgcagagggaaagatttctcgtataatgcgcctcccgtaacgacgcagaaatgcgaaaattacgaaagcaaaattaagtagtacgcgggaatagctcagttggtagagcacgaccttgccaaggtcggggtcgcgagttcgagtctcgtttcccgctccaaaatttgaaaagtgctgcaaagcacagaccacccaagcgggaatagctcagttggtagagcacgaccttgccaaggtcggggtcgcgagttcgagtctcgtttcccgctccaaaatttgaaagtgctgtaaggcacagaccacccaagcgggaatagctcagttggtagagcacgaccttgccaaggtcggggtcgcgagttcgagtctcgtttcccgctccaaattcttctctcaataaaatatccacagcgacgcgatgcgttattgctggtttttgttgtctctgacaaactcttgtaaacagagttatccacagcctcaggctgtaatcttaatttcaaagaaacttcgcacggtgaatagtatttttttaacctattgatagataagttaaaaattaagattccgttttgtcgagtcgatcacttgacgattttattcgtcttgaattgcaatgcgtttttatttttattcacaagctgtggatgaatcaggcgtcacgcggtaaccctttttcaatcacccgaaccagacgctgttttttcggcaattgcacttcgactatgcacgcatttcgtctctctatttgctgcgcaatcgcccacgctatgtgctcatcgagaagtgggtgctcacctttacgactttccagcgctgtcaaaatcgtttcatcccaaggggcattgcctaatgctacggcgatattacgcagccaacgcaggtgaccaatacgacgaatcgccgatccttccgtgacttttaaaaacttctcttcgctccaggcgaataactcaatgagttccggtgcgtgtagcggcttacgcgggctgaaatcctcttctgtggtgagttgtgaatagcgattccacgggcagataagctggcagtcatcgcaaccgtaaatacggtttcccattaacggtcgcaactcttccgggatcgccccttcaagttcgatggtgagataagagatacagcggcgagcatcgacggtatatggctcgacgatggcaccggtcgggcaaatcgtcatacaggccacgcatttgccgcatccttcctcgactggttgatccacgggcagcggaatatcgaccagcaattcgcctaaaaagaagaacgaaccggcctcgcgattgaggataagtgagtgcttacctgtccagccgagcccagctttttcagctaacgggcgctcgagaataggcgcagaatcgacaaacggtctaaaattcagcgaaacacaatgttgctgaatcatctcgcccagctttttgagtcggttgcgcagaagtttgtgatagtcacggcccagcgcataacggctaacatagccgagtttggggtttttcagcgtgctggcaaatgcggcgttagcaggaaggtaattcatccgcacgctgatcacgcgcagcgtaccgggcaataactcatgagggcgagcgcgcagcataccgtgacgtgccatccagtccatttcgccgtggtattgtttgtccagccatgcttgcagtttgggctcggactcgctgagatcggtatcggtaatacctacctgctgaaagcccagttccagcccccactgtttaattttttgcgctaactgattgagatcgaggggctctgacatgacggaccatacaatgaagaaaaaccccgtaagtataccacacaccgtctggtacgccgacgatatccgccgcggagaacgcgaggcggcagatgtgctggggctcacactctatgagctgatgcttcgcgctggcgaggccgcattccaggtgtgtcgttcggcgtatcctgacgcccgccactggctggtgctgtgcggtcatggtaataacggcggcgatggctacgtggtcgcgcgactggccaaagcggtcggcattgaggtcacgttgttggcccaggagagcgacaaaccgttgccggaagaggccgcgctggcacgcgaagcatggttaaacgcgggtggcgagatccatgcttcgaatattgtctggcccgaatcggtagatctgattgttgatgcgctgctcggtaccggtttgcggcaagcgccccgcgaatccattagccagttaatcgaccacgctaattcccatcctgcgccgattgtggcggttgatatcccttccggcctgctggctgaaactggcgctacgccaggcgcggtgatcaacgccgatcacaccatcacttttattgcgctgaaaccaggcttgctcactggaaaagcgcgggatgttaccggacaactgcattttgactcactggggctggatagttggctggcaggtcaggagacgaaaattcagcggttttcagcagaacaactttctcactggctaaaaccgcgtcgcccgacttcgcataaaggcgatcacgggcggctggtaattatcggtggcgatcacggcacggcgggggctattcgtatgacgggggaagcggcgctgcgtgctggtgctggtttagtccgagtactgacccgcagtgaaaacattgcgccgctgctgactgcacgaccggaattgatggtgcatgaactgacgatggactctcttaccgaaagcctggaatgggccgatgtggtggtgattggtcccggtctgggccagcaagagtgggggaaaaaagcactgcaaaaagttgagaattttcgcaaaccgatgttgtgggatgccgatgcattgaacctgctggcaatcaatcccgataagcgtcacaatcgcgtgatcacgccgcatcctggcgaggccgcacggttgttaggctgttccgtcgctgaaattgaaagtgaccgcttacattgcgccaaacgtctggtacaacgttatggcggcgtagcggtgctgaaaggtgccggaaccgtggtcgccgcccatcctgacgctttaggcattattgatgccggaaatgcaggcatggcgagcggcggcatgggcgatgtgctctctggtattattggcgcattgcttgggcaaaaactgtcgccgtatgatgcagcctgtgcaggctgtgtcgcgcacggtgcggcagctgacgtactggcggcgcgttttggaacgcgcgggatgctggcaaccgatctcttttccacgctacagcgtattgttaacccggaagtgactgataaaaaccatgatgaatcgagtaattccgctccctgatgagcaggcaacattagacctgggcgagcgggtagcgaaagcctgcgatggcgcaaccgtaatctatctgtatggcgatttaggcgcaggtaaaaccacctttagccggggctttttacaggctctgggtcatcagggtaatgtcaaaagccccacttatacgctggtcgaaccctatacgctcgacaacttaatggtctatcactttgatttgtaccgccttgccgatcccgaggagctggagtttatggggatccgcgattattttgccaacgatgccatctgcctggtggagtggccacaacaaggtacaggtgttcttcctgacccggatgtcgaaatacacattgattatcaggcacaaggccgtgaggcgcgcgtgagtgcggtttcctctgcgggtgaattgttgctggcgcgtttagccggttaacctttgaaaggtggcgggatgatgtatcgcatcagaaattggttggtagcgacgctgctgctgctgtgcacgccggtgggtgccgcgacgctctctgatattcaggtttctaacggtaatcaacaggcgcggataacgttgagttttattggcgatcctgattatgcgtttagccatcaaagcaaacgcaccgtggcgctcgatatcaaacaaacgggcgtgattcagggactgccgttgttgttcagcggcaataatctggtgaaggcgattcgctctggaacgcctaaagatgcacaaacgctacggctggtggtcgatcttaccgaaaacggtaaaaccgaagcggtgaagcggcagaatggcagcaattacactgtcgtctttacgattaacgccgatgtgccgccaccgcctcctccgccgcccgtggttgcgaaacgcgttgaaacgcctgcggttgtcgcaccgcgcgtcagcgaaccggcgcgcaatccgtttaaaacggaaagtaaccgcactacgggtgttatcagcagtaatacggtaacgcgtccggcagcgcgcgcgacggctaacactggcgataaaattatcatcgctattgatgccggacacggcggtcaggaccctggcgctatcggccccggtggtacgcgggagaaaaatgtcaccatcgccatcgcgcgtaaattgcgtactttgctcaatgacgatccgatgtttaaaggcgttttaacccgtgacggggattactttatctcggtgatggggcgcagtgatgtggcacgtaagcaaaacgccaatttcctcgtgtcgattcacgctgatgccgcaccgaaccgcagtgcgactggcgcttccgtatgggtgctctctaaccgtcgcgccaacagtgaaatggccagctggctggagcagcacgagaaacagtcggagctgctgggtggggcgggtgatgtgctggcgaacagtcagtctgacccctatttaagccaggcggtgctggatttacagttcggtcattcccagcgggtagggtatgatgtagcgaccagtatgatcagtcagttgcaacgcattggcgaaatacataaacgtcgaccagaacacgccagccttggcgttctgcgctcgccggatatcccatcagtactggtcgaaaccggttttatcagcaacaacagcgaagaacgtttgctggcgagcgacgattaccaacaacagctggcagaagccatttacaaaggcctgcgcaattacttccttgcgcatccgatgcaatctgcgccgcagggtgcaacggcacaaactgccagtacggtgacgacgccagatcgcacgctgccaaactaaggacgattgatgccaattcaggtcttaccgccacaactggcgaaccagattgccgcaggtgaggtggtcgagcgacctgcgtcggtagtcaaagaactagtggaaaacagcctcgatgcaggtgcgacgcgtatcgatattgatatcgaacgcggtggggcgaaacttatccgcattcgtgataacggctgcggtatcaaaaaagatgagctggcgctggcgctggctcgtcatgccaccagtaaaatcgcctctctggacgatctcgaagccattatcagcctgggctttcgcggtgaggcgctggcgagtatcagttcggtttcccgcctgacgctcacttcacgcaccgcagaacagcaggaagcctggcaggcctatgccgaagggcgcgatatgaacgtgacggtaaaaccggcggcgcatcctgtggggacgacgctggaggtgctggatctgttctacaacaccccggcgcggcgcaaattcctgcgcaccgagaaaaccgaatttaaccacattgatgagatcatccgccgcattgcgctggcgcgtttcgacgtcacgatcaacctgtcgcataacggtaaaattgtgcgtcagtaccgcgcagtgccggaaggcgggcaaaaagaacggcgcttaggcgcgatttgcggcaccgcttttcttgaacaagcgctggcgattgaatggcaacacggcgatctcacgctacgcggctgggtggccgatccaaatcacaccacgcccgcactggcagaaattcagtattgctacgtgaacggtcgcatgatgcgcgatcgcctgatcaatcacgcgatccgccaggcctgcgaagacaaactgggggccgatcagcaaccggcatttgtgttgtatctggagatcgacccacatcaggtggacgtcaacgtgcaccccgccaaacacgaagtgcgtttccatcagtcgcgtctggtgcatgattttatctatcagggcgtgctgagcgtgctacaacagcaactggaaacgccgctaccgctggacgatgaaccccaacctgcaccgcgttccattccggaaaaccgcgtggcggcggggcgcaatcactttgcagaaccggcagctcgtgagccggtagctccgcgctacactcctgcgccagcatcaggcagtcgtccggctgccccctggccgaatgcgcagccaggctaccagaaacagcaaggtgaagtgtatcgccagcttttgcaaacgcccgcgccgatgcaaaaattaaaagcgccggaaccgcaggaacctgcacttgcggcgaacagtcagagttttggtcgggtactgactatcgtccattccgactgtgcgttgctggagcgcgacggcaacatttcacttttatccttgccagtggcagaacgttggctgcgtcaggcacaattgacgccgggtgaagcgcccgtttgcgcccagccgctgctgattccgttgcggctaaaagtttctgccgaagaaaaatcggcattagaaaaagcgcagtctgccctggcggaattgggtattgatttccagtcagatgcacagcatgtgaccatcagggcagtgcctttacccttacgccaacaaaatttacaaatcttgattcctgaactgataggctacctggcgaagcagtccgtattcgaacctggcaatattgcgcagtggattgcacgaaatctgatgagcgaacatgcgcagtggtcaatggcacaggccataaccctgctggcggacgtggaacggttatgtccgcaacttgtgaaaacgccgccgggtggtctgttacaatctgttgatttacatccggcgataaaagccctgaaagatgagtgatatcagtaaggcgagcctgcctaaggcgatttttttgatggggccgacggcctccggtaaaacggcgttagccattgagctgcgtaaaattttaccagtagagttgataagcgttgattctgcccttatttacaaagggatggatatcgggacggcgaagccgaacgctgaagagttactcgccgcgccgcaccgattgctggatattcgcgatccgtcgcaggcttactcggctgctgattttcgccgcgatgcgctggcggaaatggccgatatcaccgcggcggggcggatcccactgttagtgggcggtacgatgttgtatttcaaggcattgctggaagggttgtcgccgctaccgtcggcagacccggaagtacgggccagaattgagcaacaggcggcagagcaaggttgggagtcattgcatcgtcaacttcaggaggtagatccggttgcggcagcaaggattcatccaaatgatccacaaaggctttcccgggcactggaagtttttttcatttcgggtaaaactttaacggaactgacgcaaacgtcaggagacgctctaccgtatcaggtgcatcagttcgccatcgccccggcgagccgtgaactgctccatcaacgcattgagcagcgttttcatcagatgttggcttcaggttttgaagcagaagtccgggcgctttttgcccgaggagatttgcatacggacttgccttccattcgttgcgtgggttatcgccagatgtggtcttaccttgaaggcgaaatctcatacgatgaaatggtttatcgaggtgtttgcgccacgagacagttggcgaagcggcagataacctggctgcgtggttgggaaggggttcactggcttgacagtgaaaaaccagaacaggcgcgtgacgaagtattacaggttgttggtgctatcgcaggctgaatgtgtacaattgagacgtatcgtgcgcaattttttcagaatcgaaaggttcaaagtacaaataagcatataaggaaaagagagaatggctaaggggcaatctttacaagatccgttcctgaacgcactgcgtcgggaacgtgttccagtttctatttatttggtgaatggtattaagctgcaagggcaaatcgagtcttttgatcagttcgtgatcctgttgaaaaacacggtcagccagatggtttacaagcacgcgatttctactgttgtcccgtctcgcccggtttctcatcacagtaacaacgccggtggcggtaccagcagtaactaccatcatggtagcagcgcgcagaatacttccgcgcaacaggacagcgaagaaaccgaataaggtttcgggctgtttttttacacggggagccagcgatcctgcgttccccgctgatctatttagagggttatacgcttgtttgaccgttatgatgctggtgagcaggcggtactggtacacatctattttacgcaagacaaagatatggaagacctccaggagtttgaatctctggtctcttccgccggtgtcgaagcattgcaggtgattaccggtagccgtaaagcgccgcacccaaagtattttgtaggtgaaggtaaagcagttgaaattgcggaagctgtcaaagcgacgggtgcttcggtcgttctttttgaccatgccctgagcccggcgcaagagcgtaacctggagcgtttgtgcgagtgtcgtgttatcgaccgcaccggccttattttagatattttcgcccaacgtgcgcgtacccatgagggtaagttgcaggttgagctggcgcagctgcgccatctggctacgcgcctggtgcgtggctggacccaccttgaaagacagaaaggcgggataggtttgcgtggtccgggtgaaacccagctcgaaaccgaccgtcgtttgttgcgtaatcgcatcgtgcagatacagtcgcgcctggaaagagttgaaaagcagcgtgagcaggggcggcaatcgcgtatcaaagccgacgttcctactgtttcgctggtgggatataccaacgccggtaaatctacccttttcaatcgcatcaccgaagcgcgggtctacgcggcagaccagttgtttgccaccctcgacccgacgttgcggcgtattgacgttgcagatgtcggtgaaaccgtacttgcagataccgtagggtttattcgccacctgccgcacgatctggtggcggcatttaaagccacgttacaagagacgcggcaagccacattactgctgcacgtcattgatgcggcggatgtgcgtgtacaagaaaacatcgaagcggtgaatacggttcttgaagagatcgacgctcacgagatcccaaccctgctggtgatgaacaagatcgatatgctggaagatttcgaaccgcgtattgatcgggacgaagagaacaaaccgaaccgtgtctggctttccgcacagaccggagcggggataccacagctttttcaggctttgacggagcggctttccggcgaggtggcgcagcatacattgcgtctgccaccgcaggaagggcgtctgagaagtcgtttttatcagcttcaggcaatagaaaaagagtggatggaggaggacggcagcgtaagtctgcaagttcgtatgccgatcgttgactggcgtcgcctctgtaaacaagaaccggcgttgatcgattacctgatctaacggcgtagcgtctgaagcgtggagtcatatcctctggcgtcgaaagacaacagggatcaccgcataacaaatatggagcacaaacatggcgtggaatcagcccggtaataacggacaagaccgcgacccgtggggaagcagcaaacctggcggcaactctgagggaaatggaaacaaaggcggtcgcgatcaagggccacctgatttagatgatatcttccgcaaactgagcaaaaagctcggtggtctgggcggcggtaaaggcaccggatctggcggtggcagttcatcgcaaggcccgcgcccgcagcttggcggtcgtgtcgttaccatcgcagcggcagcgattgtcattatctgggcggccagtggtttctataccattaaagaagccgaacgcggcgtggtaacacgctttggtaaattcagccatctggttgagccgggtctgaactggaaaccgacgtttatcgacgaagtcaaaccggtgaacgtggaagccgtgcgtgaactggccgcttctggtgtgatgctgacgtcggacgagaacgtagtgcgcgttgagatgaacgtgcagtaccgcgtcaccaatccggaaaaatatctgtatagcgtgaccagcccggatgacagcctgcgtcaggctaccgacagcgccctgcgtggagttatcggtaaatacaccatggaccgcattctgacggaaggtcgtaccgtgattcgtagcgatactcagcgcgaactggaagagacgattcgtccgtatgacatgggtatcacgctgctggacgtcaacttccaggctgctcgtccgccggaagaagtaaaagcggcgtttgacgatgcgattgccgcgcgtgaaaacgaacagcaatacattcgtgaagcagaagcgtataccaacgaagttcagccgcgtgcgaacggtcaggcgcaacgtatcctcgaagaggcgcgtgcgtacaaggcccagaccatcctggaagctcagggtgaagtggcgcgctttgctaaacttctgccggaatataaagccgcgccggaaattactcgcgagcgtctgtatatcgagacgatggaaaaagtgttgggtaacacccgcaaagtgctggttaacgataaaggtggcaacctgatggttctgccgttagaccagatgctgaaaggtggtaacgcccctgcggcgaagagcgataacggtgccagcaatctgctgcgtctgccgccagcctcttcctccacaaccagtggagcaagcaacacgtcgtccaccagtcagggcgatattatggaccaacgccgcgccaacgcgcagcgtaacgactaccagcgtcagggggaataacgatgcgtaagtcagttatcgcgattatcatcatcgtgctggtagtgctttacatgtctgtctttgtcgtcaaagaaggtgagcgcggtattacgctgcgttttggtaaggtactgcgtgacgatgacaacaaacctctggtttatgagccgggtctgcatttcaagataccgttcattgaaacggtgaaaatgctcgacgcacgtattcagaccatggacaaccaggccgaccgctttgtgaccaaagagaagaaagacctgatcgtcgactcttacatcaaatggcgcatcagcgatttcagccgttactacctggcaacgggtggtggcgacatttcgcaagcggaagtgctgttgaaacgtaagttctctgaccgtctgcgttctgaaattggtcgcctggacgtgaaagatatcgtcaccgattcccgtggtcgtctgaccctcgaagtacgtgacgcgctgaactccggttctgcgggtacagaagatgaagttactaccccggcggcagataacgccattgccgaagcggcagagcgcgtaacggctgagacgaagggcaaagttccggtcatcaacccgaacagtatggcggcgctgggtattgaagttgtcgatgtgcgtatcaagcagatcaacctgccgaccgaagtgtctgaagcgatctacaaccgtatgcgcgccgagcgtgaagcggtagcgcgtcgtcaccgttcacaaggtcaggaagaagcggaaaaactgcgcgcgactgccgactatgaagtgaccagaacgctggcagaagctgagcgtcagggccgcatcatgcgtggtgaaggcgatgccgaagcagccaaactgtttgctgatgcattcagtaaagatccggacttctacgcattcatccgtagcctgcgtgcttatgagaacagcttctctggcaatcaggacgtgatggtcatgagcccggatagcgatttcttccgctacatgaagacgccgacttccgcaacgcgttaatataacgactgcggtacaggtcaataaagccaccgcatcctcagggatgtcggtggttttctttttctataaggataatgaatgaattcgacaatctggctggcgcttgccctggttttggtactggaaggtttagggccgatgctttacccgaaggcatggaagaagatgatctctgcgatgaccaatttgcccgataatattttacgtcgttttggcggtggacttgtggttgcgggcgttgtggtctactacatgttgaggaaaacgattggctgaacaaaaaacagactgatcgaggtcatttttgagtgcaaaaagtgctgtaactctgaaaaagcgatggtagaatccatttttaagcaaacggtgattttgaaaaatgggtaacaacgtcgtcgtactgggcacccaatggggtgacgaaggtaaaggtaagatcgtcgatcttctgactgaacgggctaaatatgttgtacgctaccagggcggtcacaacgcaggccatactctcgtaatcaacggtgaaaaaaccgttctccatcttattccatcaggtattctccgcgagaatgtaaccagcatcatcggtaacggtgttgtgctgtctccggccgcgctgatgaaagagatgaaagaactggaagaccgtggcatccccgttcgtgagcgtctgctgctgtctgaagcatgtccgctgatccttgattatcacgttgcgctggataacgcgcgtgagaaagcgcgtggcgcgaaagcgatcggcaccaccggtcgtggtatcgggcctgcttatgaagataaagtagcacgtcgcggtctgcgtgttggcgaccttttcgacaaagaaaccttcgctgaaaaactgaaagaagtgatggaatatcacaacttccagttggttaactactacaaagctgaagcggttgattaccagaaagttctggatgatacgatggctgttgccgacatcctgacttctatggtggttgacgtttctgacctgctcgaccaggcgcgtcagcgtggcgatttcgtcatgtttgaaggtgcgcagggtacgctgctggatatcgaccacggtacttatccgtacgtaacttcttccaacaccactgctggtggcgtggcgaccggttccggcctgggcccgcgttatgttgattacgttctgggtatcctcaaagcttactccactcgtgtaggtgcaggtccgttcccgaccgaactgtttgatgaaactggcgagttcctctgcaagcagggtaacgaattcggcgcaactacggggcgtcgtcgtcgtaccggctggctggacaccgttgccgttcgtcgtgcggtacagctgaactccctgtctggcttctgcctgactaaactggacgttctggatggcctgaaagaggttaaactctgcgtggcttaccgtatgccggatggtcgcgaagtgactaccactccgctggcagctgacgactggaaaggtgtagagccgatttacgaaaccatgccgggctggtctgaatccaccttcggcgtgaaagatcgtagcggcctgccgcaggcggcgctgaactatatcaagcgtattgaagagctgactggtgtgccgatcgatatcatctctaccggtccggatcgtactgaaaccatgattctgcgcgacccgttcgacgcgtaattctggtacgcctggcagatattttgcctgccgggcgaacagtgtgatacattgctgtgtcgggtaagccattacgctatccgacacagtgttaaatcctcgcttttttccttccccgaactgaaataaattagcgacacagcttgtggctggtttatcatcaatataaatgtattttttcccgatttcccttttgaggttgatgtgcagttaacgagtttcactgattacggattacgtgcgctgatctacatggcgtcattgccagaagggcggatgaccagtatttctgaagtgactgacgtctacggcgtctcccgtaatcatatggtcaaaataatcaatcaacttagtcgtgccggctacgtgactgctgttcgtggaaaaaatggcggcattcgcctgggtaaaccggcgagtgcgatacgtattggtgatgtggtgcgcgagctggagcccttatcgctggtgaattgcagcagtgagttttgccacattacacctgcctgtaggttgaaacaggcactttctaaggccgtgcaaagttttcttacggaactggataactacacgcttgccgatttggttgaagagaatcaaccgctttataaattattgctggtggagtgacgaaaatcttcatcagagatgacaacggaggaaccgagatgtcacaagatcctttccaggaacgcgaagctgaaaaatacgcgaatcccatccctagtcgggaatttatcctcgaacatttaaccaaacgtgaaaaaccggccagccgtgatgagctggcggtagaactgcacattgaaggcgaagagcagcttgaaggcctgcgtcgccgcctgcgcgcgatggagcgcgatggtcaactggtcttcactcgtcgtcagtgctatgcgctgccggaacgcctcgacctggtgaaaggtaccgttattggccaccgtgatggctacggctttctgcgggttgaagggcgtaaagatgatttgtatctctccagcgagcagatgaaaacctgcattcatggcgatcaggtgctggctcagccgctgggtgctgaccgtaaaggtcgtcgtgaagcgcgtattgtccgcgtactggtgccaaaaaccagccagattgttggtcgctactttaccgaagcgggcgtcggctttgtggttcctgacgacagccgtctgagcttcgatatcttaatcccgcccgatcagatcatgggcgcgcggatgggctttgtggtcgtagtcgaactgactcagcgtccgactcgccgcaccaaagcggtgggtaaaatcgtcgaagtgctgggcgacaatatgggcaccggcatggcggttgatatcgctctgcgtacccatgaaattccgtacatctggccgcaggctgttgagcaacaggttgccgggctgaaagaagaagtgccggaagaagcaaaagcgggccgtgttgatctgcgcgatttaccgctggtcaccattgatggcgaagacgcccgtgactttgacgatgcagtttactgcgagaaaaaacgcggcggcggctggcgtttatgggtcgcgattgccgacgtcagctactatgtgcgtccgtcaacgccgctggacagagaagcgcgtaaccgtggcacgtcggtgtacttcccttcgcaggttatcccgatgctgccggaagtgctctctaacggcctgtgttcgctcaacccgcaggtagaccgcctgtgtatggtgtgcgagatgacggtttcgtcgaaaggccgcctgacgggctacaaattctacgaagcggtgatgagctctcacgcgcgtctgacctacaccaaagtctggcatattctgcagggcgatcaggatctgcgcgagcagtacgccccgctggttaagcatctcgaagagttgcataacctctataaagtgctggataaagcccgtgaagaacgcggtgggatctcatttgagagcgaagaagcgaagttcattttcaacgctgaacgccgtattgaacgtatcgaacagacccagcgtaacgacgcgcacaaattaattgaagagtgcatgattctggcgaatatctcggcggcgcgtttcgttgagaaagcgaaagaaccggcactgttccgtattcacgacaagccgagcaccgaagcgattacctctttccgttcagtgctggcggagctggggctggaactgccgggcggtaacaagccggaaccgcgtgactacgcggagctgctggagtcggttgccgatcgtcctgatgcagaaatgctgcaaaccatgctgctgcgctcgatgaaacaggcgatttacgatccagaaaaccgtggtcactttggcctggcattgcagtcctatgcgcactttacttcgccgattcgtcgttatccagacctgacgctgcaccgcgccattaaatatctgctggcgaaagagcaggggcatcagggcaacaccactgaaaccggcggctaccattattcgatggaagagatgctgcaactgggtcagcactgttcgatggcggaacgtcgtgccgacgaagcaacgcgcgatgtggctgactggctgaagtgtgacttcatgctcgaccaggtaggtaacgtctttaaaggcgtaatttccagcgtcactggctttggcttcttcgtccgtctggacgacttgttcattgatggtctggtccatgtctcttcgctggacaatgactactatcgctttgaccaggtagggcaacgcctgatgggggaatccagcggccagacttatcgcctgggcgatcgcgtggaagttcgcgtcgaagcggttaatatggacgagcgcaaaatcgactttagcctgatctccagcgaacgcgcaccgcgcaacgtcggtaaaacggcgcgcgagaaagcgaaaaaaggcgatgcaggtaaaaaaggcggcaagcgtcgtcaggtcggtaaaaaggtaaactttgagccagacagcgccttccgcggtgagaaaaaaacgaagccgaaagcggcgaagaaagacgcgagaaaagcgaaaaagccatcggcgaaaacgcagaaaatagctgcagcgaccaaagcgaagcgtgcggcgaagaaaaaagtggcagagtgatcaataccctctttaaaagaagagggttagattgctgacaaaatgcgctttgttcatgccggatgcggcgtgaacgccttatccggcctacataatcacgcaaattcaatatattgcagagatcatgtaggccggataaacgtagtgcatcaggcaaaacgtaaacaacgagtacattaatgagcgaaatgatttacggcatccacgcagtgcaggccctgctggagcgcgcccctgaacgttttcaggaagtctttattttaaaaggccgtgaagataaacgtctgttaccgctgattcacgcccttgagtctcagggcgtggttatccagttggcaaaccgccaatatctcgacgagaaaagcgacggtgccgtgcatcagggcattatcgcccgcgtgaagccaggacgtcagtatcaggaaaacgatctgccggatctgatcgcttcgctcgatcaaccgttcctgctgatcctcgacggcgtaaccgatccgcacaacctcggcgcgtgcctgcgtagtgcggacgccgcaggcgttcatgcggtgattgtgccgaaagatcgctccgcacagctcaacgctacggcgaaaaaagtagcctgcggcgcggcagaaagcgttccgctgattcgggtgactaaccttgcgcgcaccatgcgtatgttgcaggaagagaatatctggatcgtcggtacggcaggcgaggcggatcatacactctatcagagcaaaatgaccggacgcctggcgctggtgatgggtgcggaaggtgaaggtatgcgtcgcctgactcgtgaacattgcgatgagttgatcagcatcccgatggctggaagcgtttcttccctgaacgtttcggttgcgaccggaatttgcttatttgaagcggtgcgccagcgcagctaatttctcagaattatgaaaagccatccagatttggatggtttttttttgtctatagctggtaagataattacgtattgcaaatattcattttattaatatttaaacttaatctatatggaataatatatgacatggaatccgttggcgctagcgacggcgctgcaaactgtacctgaacaaaatattgatgtaacaaatagcgagaacgcattaattattaaaatgaatgattatggcgatttgcaaatcaatattctttttacttcccgccaaatgattatcgaaacctttatttgtccggtgagtagtatcagcaatccagatgaatttaataccttcttattaagaaatcagaagatgatgccgttgtcatcggtagggatctccagcgtacaacaggaagagtattacattgttttcggggcgttatcgcttaaatcttctcttgaagatatcctgcttgagataacctcgctggtagataacgcattggatctggctgaaattacagaagaatattcacactaattacaaggacgggtatttatgggaattttaaaaagtttatttacgctggggaaatcgtttatctcccaggcggaagaatccattgaagaaacccagggcgtgcgcatgctggaacagcatattcgtgacgctaaagctgaactcgataaagccggaaaatctcgcgttgatctgctggcgcgggtgaaattaagtcacgataagctgaaagatttacgtgagcgcaaagccagtctggaagcccgtgcgctggaagcgttaagcaagaacgttaatccgtcgttgattaacgaagttgctgaagaaatcgcgcgccttgagaatctcattaccgctgaagagcaagtgttgtcgaatctggaagtctcccgtgatggcgtggaaaaagcagttacagcgacagcgcagcgtatcgctcagtttgagcagcaaatggaagtcgttaaagccactgaagccatgcagcgtgcacaacaggctgtaacaacctctaccgttggcgcatcttccagcgtttcgacagcggcagaatccttaaaacgcctgcaaacgcgtcaggccgaacgtcaggctcgcctggatgctgccgcacagttggagaaagtcgcagacggtcgcgaccttgacgaaaagctggcggaagccggaattggcggtagcaataaaagtagcgcccaggatgtattagcaagactgcaacgccaacagggcgagtaatttttttgccagcctcgctaaaaggctggcaactattttaaggataaaatatgtctggttttttccagcgtctgtttggcaaggataataagccagctatcgctcgtggtccgctgggacttcatctcaatagtggctttacgctcgacacgttagcgtttcgtttgctggaagatgaattgctgattgcgctgccgggtgaggaatttacggtagccgccgtcagccacatcgatctgggcggcggtagtcagattttccgctactacacttcaggcgatgagtttctgcaaatcaataccaccggcggcgaagatattgatgacattgatgatatcaagctctttgtctatgaagagagctacggtatcagtaaagagagtcactggcgcgaggcgatcaacgccaaagcgatgggagcaatgaccttaaactggcaggaaaaacgctggcagcgattttttaacagcgaagaaccgggaaatatcgaacccgtctacatgctggaaaaagtagaaaatcaaaaccatgccaaatgggaggtccataattttaccatgggctaccaacggcaagtaaccgaagatacttacgaatatttgctgctaaatggtgaggaatcttttaacgatctcggcgagccagagtggttattttcgcgcgcgttgggtgtcgatatcccgctgacatcacttcatattattggttaattacaaggacgtttacaatgcatatactggattcacttcttgcctttagcgcctatttttttattggcgtggctatggtgattatttttctgtttatctattctaaaattacaccgcacaacgaatggcagttaatcaaaaacaataataccgcggcgtcactggcgttcagcggtacattgttgggttacgttatccccttatccagtgcggcaatcaatgcggtgagtattccagactatttcgcctggggcgggattgcactggtgattcagttactcgtttttgctggtgtcagactttatatgcccgcattaagcgaaaaaattattaatcacaataccgcagcaggaatgtttatgggaaccgccgcgctggctggcggtatttttaacgcagcttgtatgacatggtaatggacgatcatggccagaaaacgcaaatcaagaaataacagtaaaattggtcacggagcgattagtcgcattggtagaccgaataatccttttgaaccgtgccgcaatcgctacgcacaaaaatacttaacgttggcgctaatgggcggtgccgcttttttcgtattgaaaggttgtagcgatagtagcgatgtcgataacgacggcgacggaacgttttacgcgacagtgcaggattgtattgatgacggtaataatgccgacatttgcgcgcgtggctggaacaacgccaaaacggcattttatgccgatgttccgaagaatatgactcagcagaactgtcagtctaagtacgaaaattgctactacgacaatgttgaacagagttggatcccggtcgtttctggatttttgttaagccgggttattcgtaaagatcgcgatgagccgtttgtttataacagcggcggttcctcttttgcttcgcgcccagtctggcgcagcacttctggtgattactcctggcgctccggttctggcaaaaaagagtcttactcttcgggcggctttaccaccaaaaaagcgtctaccgtttctcgcggcggctatggtcgttcttccagcgcccgtgggcattggggaggctaatcatgctgagacacaacgttcctgtgcgacgggatctggaccagatcgccgctgacaacggtttcgactttcatatcatcgacaatgaaatctattgggatgagagtcgggcttaccgttttactctgcgccagattgaagagcagatcgaaaaaccgactgcggaactgcatcagatgtgccttgaggtggtggatcgcgcggtaaaagatgaagagatcctgacgcaactggcgatcccgccgttgtactgggatgtgatcgctgaaagctggcgcgcccgcgatccttcgctgtatggacggatggattttgcctggtgtggcaatgcgccggtgaagctgctggagtacaacgccgatacgccaacttcattgtacgagtcggcttatttccagtggctgtggctggaggatgcccggcgcagcggcattattccgcgtgatgccgatcagtacaatgctattcaggaacgcctgatttcacgctttagcgagctttacagtcgggaaccgttttatttttgctgctgtcaggacaccgatgaagacaggagtaccgtgctgtacttgcaggactgcgcccagcaggcagggcaggagtcgcggtttatctacattgaagatctcggtttgggcgtcggcggcgtactgaccgatcttgatgataatgtcatccagcgtgcatttaagctgtatccgctggagtggatgatgcgtgacgataacggtccgctgctgcgcaagcgtcgcgagcaatgggtggagccgttatggaaaagtatcttgagtaataaagggctaatgccgctgctttggcgcttcttccctggtcatcctaatcttcttgcgtcctggttcgatggcgagaaaccgcagattgccgctggcgaaagctatgtgcgtaaaccaatctattcgcgcgaaggcggcaacgtcaccatttttgacggcaagaataacgttgttgaccacgctgatggtgattacgccgatgaaccgatgatctaccaggcgtttcaacctctgccgcggtttggcgatagctacacactcatcggtagctggattgtcgatgatgaagcgtgcggaatggggatccgtgaagataacacactgatcaccaaagacacctcacgtttcgttccgcattacattgctggataagaatgttttagcaatctctttctgtcatgaatccatggcagtgaccatactaatggtgactgccattgatggagggagacacagtgcactggcaaactcacaccgtttttaatcaacctataccattaaataacagcaacttatacctgtctgatggcgcgctctgcgaagcggtaacgcgtgaaggtgctggctgggatagcgattttctagccagtattggtcagcagttaggaacggctgaatcccttgaactggggcggctggcgaatgtgaatccgcctgaattattgcgctacgatgcgcaaggacgccgtctggacgatgtgcgttttcaccccgcctggcacctgctgatgcaggcgctatgtaccaatcgggtgcacaatcttgcctgggaagaagacgctcgctccggcgcatttgtggcgcgcgcggcgcgttttatgttacatgcgcaggttgaggcagggtcgttatgtccgataaccatgacctttgccgccacgccattgttgttacagatgttacccgcgccgtttcaggactggaccacgccgctattgagcgatcgctacgattctcacttattgccaggtgggcaaaaacgcggtttgttgattggcatgggaatgacggaaaagcagggcggttccgatgttatgagcaacaccacccgtgcagagcgtctggaagatggctcttatcggctggtggggcataaatggtttttctcggttccgcaaagcgatgcgcatctggtgctggcgcagaccgcgggtggtctgtcctgcttttttgtgccgcgctttttgcctgacgggcaacgcaacgcgattcgcctcgagcggctgaaagataagctgggtaatcgctctaacgccagttgcgaagtggagtttcaggatgccattggttggttgttggggctggaaggggaaggaattcgtctgatcctgaaaatgggtgggatgacgcgttttgattgcgccctgggtagccatgccatgatgcgccgtgcattttcgctggcgatttatcatgcacatcaacgccatgtttttggtaatccattgatccaacagccccttatgcgtcatgtcttaagtcgcatggcacttcagcttgaagggcaaacggcgttgctgtttcgtcttgcgcgagcgtgggaccggcgtgccgatgccaaagaagccctgtgggcgcgtttatttacgcctgcggcaaaatttgtgatctgcaaaagaggtatgccgtttgtggccgaagcgatggaggtgctgggcggcattggttattgcgaggagagtgagctgccgcggctttaccgggagatgccggtaaacagtatttgggaaggttccggcaatattatgtgcctggatgtgttgcgcgttctcaataagcaagcgggcgtatacgacttattgtcggaagcatttgtggaagtgaaagggcaggatcgctattttgatcgcgcggttcgtcgtttacagcagcagctgcgtaagccagctgaagaactggggcgagagattactcatcagctattcctgctgggctgcggtgcgcaaatgttgaaatatgcttctccgccaatggcgcaggcgtggtgtcaggtgatgttagatacgcgcggcggcgtacggttgtcagagcagatccagaatgatttattgctgcgggcgacggggggagtgtgtgtgtaagcgtatacgactgatgcgacgctggtttcgattaactaaatgaaatatgtgaaaattgtaggccggacaaggcgctcgcgccgcatccggcattgttcatttgctgtagatgacactcatgcatacagtatcgcctgtacgcgccagttatcaggctgctggtcttcgtacatggtaataatgcggtaccatgacgcaccttgttcatcggcctttaacgccacgatacgttccacgtcctgcggatcccctgaaatattgctaactgagatctgacctatttcattcaggcccgtcacgcagtcagcactggcgaattctgcagactgtgccgtggcgctcgcaggataagtcactaattgcagcgagggtgaggcaagtaattgtttcatcgtcagctccatttttcgtttccccacatgttgcagggcattccatcgcggtaataaacgcccaggcttccagccggtaatttattgtgcacaggtaaacgcatagggacgcaaagcaatgtaaagctgactatgtaagttgtctgatttatttacggtacaaaatggcttgtgaataccactgtcctgtcacgatggtttcgtccaccatgacgacaacgtaataatcagcttttgcagcgacagctttcgctttgatttctgctaatgcgtcatccggagaaccccgaaccatcgtgcttacgctacctattcgctgtaacccttgcgtctggtcgcggcgaatctcttgcggatggtccgttactggcggtgctggctgtggcgtaccttgcagtgcgctacaggcacttaacatcaacaccaataataaactggcaaaccggtaaataacgctattacgtttcctgctaaccatagtgtagtgccttattaatttaactttgggggaatgttcccgaattgttacctggtacgcgattttcgaatgaaaacgtgacgaaagcgtaacccacatctcaacattatgaactaataccgccagcagaaacttgtgctaaggatttcttcatgtcataccagacaaaaaggagagacagatgattgaaatagaatcacgcgagctggcagatattcccgttcttcatgcttatcctgtcgggcaaaaagataccccgttaccgtgcgtaattttttatcacggctttacttcatccagtctggtgtatagctattttgccgttgcgctggcgcaggctggtttgcgggtgatcatgccggatgcgcccgatcacggtagccgttttagtggtgacgcagcgcggcggttaaatcaattctggcaaatcttgctacaaagtatgcaggaattcactactttacgtgcggcaatagccgaagaaaactggctgcttgatgaccgtctggcagtcggtggcgcgtcgatgggcgcgatgacggcactggggattaccgctcgccaccccacggtgagatgtaccgccagcatgatgggatcgggctattttacatcactcgcccgttcactgtttccaccgctgatacctgaaacggcagcacagcagaatgaattcaataacattgtcgcgccactggcagagtgggaagcgacaaaccacctggaacaacttagtgacagacctctactgctgtggcatggcctcgacgatgacgttgtgcctgccgacgaatcactacgtttgcagcaggccttaagcgagacgggacgggataaactgctaacctgttcatggcagccaggcgtgcgtcaccgcattacgcctgaggcgttagatgctgccgtgacatttttccgccagcatctttaaacacgcagaatgctgaccccttgcgcttccagttgttgcaggatttccgggttagcatttttgccggtgataagcatatcgatttgatcggcacggctaaaaagcattcccgcgcgttcgccaatcttactgctatcaaccagtaccaccagtttccctaccacgctcagcatcttctgctctgccattgctgtcagcatatcggttttatacaacccttctgcggtcagcccttttccgctggtaaacatccagtgcccggcatagagactgttttcgctgccctgcgggcttaaagtgatggactgacttttgttgtactgtccgcccataatgatcacgctgtcatgttcttgatcgatcaggtaatttgccagcggtagataattagtgatgatttgcactggcttgccacacatttcccgcccaagcagaaacgcggtggagccgcagttgatgactacgctttcgcccggattaaccagctgcgaggccgctttagcgatacgtactttttcatcgtgattctgcgcctgatgcagattcatcggcgtccagcgcgggcgctgttgggtaatagcttctgcgccattgcgcacttttttcagtttgccgctttcgtcaagtttattgatatcgcgtcgcgcagtggcaggcgaaattcccagacgctcaacgactttctcaacggtcacaaagcccaattgtgcgagcatttccaggaggatttgatgtctttgtgcttcagtcatgagctattccgataaaatttgatttttttagatgatatttgaaatagccaggaaatactacgccggatagcgcgaacttctccacgctacccggtataaacgacagattacaggaatgacttgaacggcagatccggttcaatagtgaagcaatcatcgaaaccgcgcggatagtggtactcgaagttgtctttatccagcggccaggtaaatttgccacccacctgccagataaacggcttgaagccatacttcaggcgatcttttttcatctcccacagcacgcggatctcttgcggatcggcctggaagtttgaccagatatcgtggtggaacgggatcactactttcgcattcagcgcttcacccatacgcagcatatcggcgctggtcattttgtcggtgataccgcgcgggttttcgccgtacgatcctaacgccacgtcgatctgatgttcgttaccgtgcttcgcataatagttagagtagtgggagtcgccgctgtgatacagggagccgccaggcgttttgaacaggtagttcaccgcgcgatcgtccatgccatctggcagtacgccagccgctttttgatcggcaggcagggtgatcagtgcagtacggtcgaaagcatcaagcgcatgaatttcaatgtctttcacttttactacatcgcccggtttgaccacgatgcaacgctctttcggtacgccccagccaatccacaaatccacacaggttttcggtccgataaacggtacgtcatctgcacaattctgcatcacggcagcagcgacgttaacgtcgatatgatcgttgtgatcgtgagtcgccagtaccgcgtcgatctggcgaatcgcaaacggatcaagaacaaacggggtggtacgcaggtttggctgcagttttttcacgccagccatgcgctgcatctggtgaccctgtttcattaacgggttaccgtgactttgtttgccagtgccgcaccagaaatcaacgcaaacgttggtgccaccttccgatttcaaccagatcccggtgcagccaagccaccacatcgcaaatgtgccaggagcgacctgttcttgttcaatttcttcattcaaccagctaccccactccgggaaagtgctcaggatccaggattcacgggtgatacttttcactttactcatcgccatttaccttcatgatagttcaattcgaatcaatatgtgattggttttgattaatcctgacactattttttcaggaaggcaatgaccattttttgactttttgccagggaagttgttgttgattttgagtatggaaagatttaatggaatgtgtaattcaattaactaaatgaatttaaatggataattgtttcgttgtgtgaatcccactctatccatgtggaattatttgcgggtcgcgtcacatttaatcataaataatcttgttgtgattacttttgaaaattagagtgagtgcacaacattccgggtgtgtggaatacccggttacctcttcttcaggagatcgttatggagatcctctacaacatctttaccgtgttttttaaccaggtcatgaccaatgccccgttgttgctgggtattgtgacctgtctgggctacatcctactgcgcaaaagtgtcagcgttattattaaaggcacgattaaaaccataattggtttcatgttgttgcaggcagggtccggcatcctcaccagcaccttcaaaccggtggtggcgaaaatgtccgaagtctacggcattaacggcgcaatttccgatacctacgcttcaatgatggcaaccatcgaccgcatgggcgatgcctatagctgggtgggttacgccgtattgttagcgctggcgctgaacatctgttacgtgctgttgcgtcgcattaccggcattcgcacaatcatgttgaccggccacatcatgttccagcaggccgggttgattgccgttacgctgtttatcttcggctactccatgtggaccaccattatctgtaccgcgattctggtttcgctctactggggcatcacttccaacatgatgtacaagccgactcaggaagtgacggatggctgtggtttctccatcggtcaccagcagcagtttgcatcatggattgcctataaagtcgcgccgttcctcggcaaaaaagaggagagcgttgaagacctcaaattgccgggctggctgaacattttccacgacaacatcgtctccacggcgattgtgatgaccatcttctttggtgccattctgctctccttcggtatcgacaccgtgcaggcgatggcaggcaaagtgcactggacggtgtacatcctgcaaactggtttctcctttgcggtggcgatcttcatcatcacgcagggtgtgcgcatgtttgtggcggaactctctgaagcatttaacggcatttcccagcgcctgatcccaggtgcggttctggcgattgactgtgcagctatctatagcttcgcgccgaacgccgtggtctggggctttatgtggggcaccatcggtcagctgattgcggttggcatcctggtcgcctgcggctcctcgatcctgattattcctggctttatcccgatgttcttctctaacgccaccatcggcgtgttcgctaaccacttcggcggctggcgtgcggcgctgaagatttgtctggtgatggggatgatcgaaatctttggttgcgtctgggcggtgaaactcaccggtatgagtgcctggatgggcatggcggactggtcgattctggcaccgccgatgatgcaaggcttcttctccatcggtatcgcctttatggccgtcatcattgtaattgcactggcttatatgttcttcgctggccgcgcgctgcgcgcagaagaagatgcagaaaaacaactggcagaacagtctgcttaataaggagttttgattatgaccgtacgtattctggctgtgtgtggcaacggacaaggcagttccatgatcatgaagatgaaagtggaccagtttttaacccaatcaaacattgaccatacggtaaacagctgcgcggttggcgagtacaaaagcgagttgagtggcgcggatatcatcatcgcttctacgcacattgcgggcgaaatcaccgtgaccggcaacaaatacgtggttggcgtgcgcaacatgctctctcctgccgactttggcccgaaactgctggaagtgatcaaagagcatttcccgcaggatgtgaagtaaggacgcgccatgaaattacgtgattcgctggcggaaaataaatccatccgcctgcaggctgaagcagagacatggcaggaagcggtgaaaatcggcgttgacctgctggtggcggcagatgtggtagagccgcgttactaccaggcgattctggatggcgttgaacagttcggtccttatttcgttatcgctccgggcctggcaatgccgcacgggcgtccggaagagggcgttaagaaaaccggtttctctctggtaacgctgaaaaagccgctggagttcaaccacgatgacaacgatccggtggatatcctcatcaccatggcggcggtcgatgccaatactcaccaggaagtgggcatcatgcagatcgtcaacctgtttgaagatgaagagaattttgaccgtttacgcgcctgccgtaccgagcaggaagtactggatctcattgaccgcaccaacgcggcagcttaagaaggaattgaacatgtcattaccgatgttgcaagtcgcgctggacaaccagactatggatagcgcctacgaaaccactcgcctgattgccgaagaagtcgacattatcgaagtgggcaccattctgtgcgtgggcgaaggcgtgcgtgcggttcgtgacctgaaagcgctctacccgcacaaaatcgtactggcagacgccaaaattgccgatgcaggcaaaatcctttcgcgtatgtgcttcgaagccaacgctgactgggtgacggtaatttgctgtgcggatatcaacaccgccaaaggcgcgctggacgtggcaaaagagtttaacggcgacgtgcagatcgaactgaccggttactggacctgggaacaggcgcaacagtggcgcgatgcaggcattgggcaggtggtttatcaccgcagccgtgacgcgcaggccgcaggcgtggcgtggggcgaagcggacatcaccgcgatcaaacgtctttccgatatgggcttcaaagtcaccgtcaccggaggcctggcgctggaagatctgccgctgttcaagggtattccgattcacgtctttatcgcgggccgtagtatccgtgatgccgcttctccggtggaagccgcacgtcagttcaaacgttccatcgctgaactgtggggctaaggagcggatatgttgtccaaacaaatcccgcttggcatctatgaaaaagcgctccccgccggggagtgctggctggaacgcctgcaactggcaaaaacgttaggcttcgattttgtcgaaatgtcggtagatgaaactgacgatcgcctgtcgcgcctcaactggagccgcgagcagcgtctggcgctggtcaatgcgattgttgaaaccggcgtgcgcgtgccgtccatgtgcctttctgctcatcgtcgtttcccgctgggcagtgaagatgacgcggtgcgggcgcaggggctggagattatgcgtaaagctatccagttcgcccaggatgtcggtattcgcgtgatccagctggcgggctatgacgtttactatcaggaagccaataacgaaacgcgtcgtcgtttccgtgacggcctgaaagagagcgttgagatggcaagccgcgcgcaggtgacgctggcgatggagatcatggattatccgttgatgagctccatcagcaaggcgctgggatacgcgcactatctcaacaatccgtggttccagctctacccggatatcggcaacctgtcggcgtgggacaacgatgtgcagatggagttgcaggccggaatcgggcatatcgtcgcggtacatgtgaaagacaccaaacctggcgtcttcaaaaacgtgccgtttggcgaaggtgtagtggatttcgaacgttgtttcgaaacgctcaaacagagtggctattgcgggccgtacctgattgagatgtggagcgaaacggcggaagacccggcggcagaagtggcgaaagcgcgtgattgggtgaaagcgcgcatggcgaaagcgggcatggtggaggcggcataatgcaaaagctaaaacagcaggtatttgaagccaacatggagctgccgcgctacgggctggtgacctttacctggggcaacgtcagcgctatcgaccgcgaacgcgggctggtggtgatcaagcccagcggcgttgcctacgaaaccatgaaagcggccgatatggtggtggttgatatgagcggcaaggtggtggaaggggagtatcgcccatcttccgacactgcgacgcatctcgaactctaccgtcgttacccgtcgcttggtggcattgtccatacccactccactcatgccaccgcatgggcgcaggcggggctggcgatcccggcgttaggcaccacgcacgccgactacttctttggcgacattccgtgtacgcgcgggttaagcgaagaagaggtgcagggcgagtatgaactgaacaccggcaaagtgattatcgaaacgctgggcaacgccgagccgctgcatacgccgggaattgtggtgtatcagcacgggccgttcgcctgggggaaagatgctcacgatgcggtgcataacgcggtggtgatggaagaagtggcgaaaatggcgtggattgcccgcggcattaacccacaactcaatcacatcgacagcttcctgatgaataaacacttcatgcgtaaacacggtcctaacgcttattacgggcagaagtagaacacgcgctgcggaaatttccttcctcgggagataactggtctaattccgcagccgtttttcaaaaaaaagccccctgcgaagggggcaaagcaaactatggcaatgtttcgttggttatacctggtgctagcgataaatatccgcgctggcgtgcatattgccgttactccccggttcccgcatcagaattacgtggtagtacgttgcgccttgcgcatctgtttcttcatttaatgcctgacgtgcttcgctttcagtggcgaaattatgattgatataaatcacgcctaagctttgcacatcgtccatatttctggcctggtggttattaatttcaatggctgcccatgtatttgcacttagcaaaagcacagccagaagggctaaaacacgactgaacatagatacctcctcgacggctgactttgtgtgctctcctctgtgatgatcttctgatttaattttaatcaatgataaagaagttgatggtgaccatttctgatgcagttgttcaaaaaaacaccatgatgaagtgtgatgaacttcaaatcagcgtgttagaggttaattgcgaaaggggagatttatttcggctctgcccttgagtttagcgaggcatacaagtactataacgcgtcatttttcagccgacctttaacacgttccttgcctccccgggattcggctgacccagacaggaggctgaataatccgtaaggagcaattcgatgcgtcattacgaaatcgtttttatggtccatcctgaccagagcgaacaggttccgggcatgatcgagcgctacactgctgccatcactggtgcagaaggcaagatccaccgtctggaagactggggccgccgtcagctggcttacccgatcaacaaactgcacaaagcacactacgttctgatgaatgttgaagctccgcaggaagtgatcgatgagctggaaactaccttccgcttcaacgatgccgttatccgcagcatggttatgcgtaccaagcacgctgttaccgaagcatctccgatggttaaagcgaaagacgagcgccgtgagcgtcgcgatgatttcgcaaacgaaaccgctgatgatgctgaagctggggattctgaagagtaatttctgatgaccaaccgtctggtgttgtccggcaccgtgtgcagggctccccttcgaaaggtcagtccatcaggaattcctcactgccagttcgtgcttgagcatcgttctgtgcaggaggaagccggctttcaccggcaggcgtggtgtcaaatgcccgttattgttagcggacacgaaaaccaggccattactcacagtataacggtcggcagtcgcataaccgttcaggggttcatttcatgccacaaggcaaagaacggactgagcaaaatggttttgcatgccgagcagattgaattgatagattctggagactagccatatggcacgttatttccgtcgtcgcaagttctgccgtttcaccgcggaaggcgttcaagagatcgactataaagatatcgctacgctgaaaaactacatcaccgaaagcggtaagattgtcccaagccgtatcaccggtacccgtgcaaaataccagcgtcagctggctcgcgctatcaaacgcgctcgctacctgtccctgctgccgtacactgatcgccatcagtaatcggtcacggtccattaatacgactttgagaggataaggtaatgcaagttattctgcttgataaagtagcaaacctgggtagcctgggtgatcaggtaaacgttaaagcgggctatgctcgtaacttcctggtaccgcagggtaaagctgttccagctaccaagaaaaacattgaattcttcgaagctcgtcgcgctgaactggaagctaaactggctgaagttctggcagctgctaatgctcgcgctgagaaaatcaatgcactggaaactgttaccatcgcgtctaaagctggcgacgaaggtaaactgttcggttccatcggtactcgcgacatcgctgacgctgtaactgcagctggcgttgaagtggctaagagcgaagttcgtctgccgaacggcgttctgcgtaccactggcgaacacgaagtgagcttccaggttcacagcgaagtattcgcgaaagtgatcgtaaacgtagtagctgaataattcgttattcaacgagacgtaaaaacgccgaccattggtcggcgttttgctttctatttttcgtcaggtattagtttcgcaagtagatccattcaccattctcttgtgtccataagtcaggatggtttgctggcgttagatacatacgagcgcaactgatgtctcgctcctgcggcactcgctcgaaacccaaacccgagtagattgcggctgaacttgataaggaacgcagaccaattttcaaatcatggggtaaatcagaatacgcgtttagcaatgcagcaatgatgaatccgagggcattagaaacgcctgtaacagtgcgaagttggtcgatataaagatcgattgttggtagttcagatgaccagcaattaggcatttgggcaggaagggttacaacgtatcctatcgtttggccggtatagtctggagtaccataaccaggtcccaaaaccacttcgtgtattgtgtatttactgttgggttcgaaggattcgacatcttgcaataaatatttcagttctgcggttaacctcgcacccgcgtaagctttattgtatttctgggcgtgaatattatctaatgtagcttcatggttccatccaaaagaattatcaccattcattgtgattccatcgtaagcattacacctcgtcgctaacttattgaatgcttgccagtctgagagatctagtttgtggatctcaacagtacgtctgccatcgcaattatgatctcttccacgatttgaaagtaatgtagcgcgtgcgtattgatgaaattttaattttactggtttgtcggtggacgaaaaacgagataaatatgcaggaaatgaataaatagtcgttggtaatgtcattgtaatgttacctgtttaatgtttttataaatatcgcagctgaatgttcacagaaaaaaatcgatattaataaaaataagtttgttttctgaagtggtgaaaatagcggatggtgaaagatattaatatcaaaaatcgctcattatggatataacgatgcacccggggagaaaatgacttccacgccttacaccgtacattcttgttgtgcggtatgtaattattctacgctgtcggtatcggtgtattcgttaatcagcaggttagccagccacaaaaagccattgagaaaattattgattttacatgggattattatattgctaatccttggtttttaaaaattgtgcatagtgaaaatcaaagtaaaggtgtgcattatgcaaaatcacagcgtctcttagaaattaaccatgcgcacttgcagttaatggaatccttattggatgaagggaagaaacacaatatttttaagccagatatcgacccattgcaggtgaatattaatattgctgcgcttggcggatattatttgatcaaccagcatacgcttggcctggtttatcacatcagtatggtttcaccccaggcactggaagccagacgtaaggtcatcaaagagacaatccttagctggcttttggttgacccttcatctaccgcgcacgaataaaactgccatccggctggcgggtgaacaggacctgttgattattccccgtatcaatggttaagcccgtcaccacgccgctggcgttctggcggattttcaccatctgcccgttttgcaaattactcagcggcttacccgcgccttctacctgcgccattgcatagacatcggtagcgggcagtccgtggtcgcggaacagctgcgccatcgttttaccgggttcgacacggtaagagcgccattgattatcaattccgctatctggctggaatggttgcgtttgggtagtttgcggctgctcttctggctggccttcctgtataggttctggagcgaccggagccacctgatcaggatcattttgtggggtaactaattgcgcccgcagctgttcttctgtcggcggttgtgattgcgactgaatatctaactgcgcttcacgcgtcaccaccggcgcgttgggcgtatcatcagatggaagcagaaatccgaccaccaatacaatggcggcaataatgatcccccgacgatgcatcggcggcagcgggtccatgaagcgaaaattgtccggcgcgtgccagactttctccagggttggttttagttcaaagcgcccgggcatggtttcctcctgctccgcgtcttgttcctcaatcatagcctatgaataagctaacgctatgatgtccgtggtaaacccgcctttattatattcatacgggatattgctattgtttctttttccctgggatttgtcatcattcccgcgacaaagttttacccaaagaagtgtggctgatatgctgcccgctactttataccctaagaaaggaaatacgatgaccaccccaacttttgacaccatcgaagcgcaagcaagctacggcattggtttgcaggtagggcaacaactgagtgaatctggcctggaagggctgctgccagaagcactggttgcaggtattgccgatgcgctggaaggcaaacatccggctgttccggttgatgtggtgcatcgcgcgctgcgtgaaatccacgagcgcgccgatgccgttcgtcgtcagcgtttccaggcgatggctgctgaaggtgtgaaatacctggaagaaaacgccaaaaaagaaggtgtgaatagcaccgaatctggcctgcaattccgcgtgatcaaccagggtgaaggcgcaattccggcacgtaccgaccgcgttcgtgttcattacaccggtaaactgatcgacggcaccgtgtttgacagctccgttgctcgtggtgaacccgctgaattcccggttaatggcgtgatccctggctggattgaagcactgactctgatgccggtaggttctaaatgggaactgactatcccgcaggaactggcatatggcgagcgcggcgcaggcgcatccatccctccgttcagcaccctggtgtttgaagtcgaactgctggaaatcctctaagcagcgcattctgttcccctcgaacgagaggggagcaggcattcagcaataaacccttcagtttgccaaacggcgctattttgtgttgcaaagaccccgtaagcgtgtatttttgtgagctgtttcgcgttatcaccgtgatatgacactcactttaaacataaaattaacattagatctaaatcttagtattcatcccgcgtattgttacctaatatcgatgagtcccgatacagattcgtcgtatcatagactgactaaaggccgtagagcctgaacaacacagacaggtacaggaagaaaaaaacatggtagatcaggtaaaagtcgttgccgatgatcaggctccggctgaacagtcgctacggcgcaatctcacaaaccgacatattcagcttattgccattggcggtgccattggtacggggttgtttatggggtctggcaaaacgattagccttgccgggccgtcgatcattttcgtttatatgatcattggttttatgctctttttcgtgatgcgggcaatgggggaattgctgctttcgaatctggaatacaaatcttttagtgacttcgcttccgatttactcgggccgtgggcaggatatttcaccggctggacttactggttctgctgggttgtaaccggtatggcagacgtggtggcgatcacggcttatgctcagttctggttccccgatctctccgactgggtcgcctcgctggcggtgatagtgctgctgctgacgctcaatctcgccaccgtgaaaatgttcggtgagatggagttctggtttgcgatgatcaaaatcgtcgccattgtgtcgctgattgtcgtcggcctggtcatggtggcgatgcactttcagtcaccgactggtgtggaagcgtcattcgcgcatttgtggaatgacggcggctggttcccgaaaggtttaagtggcttctttgccggattccagatagcggttttcgctttcgtggggattgagctggtaggtacaacagctgcggaaaccaaagatccagagaaatcactgccacgcgcgattaactccattccgatccgtatcattatgttctacgtcttcgcgctgattgtgattatgtccgtgacgccgtggagttcggtagtcccggagaaaagcccgtttgttgaactgttcgtgttggtagggctgcctgctgccgcaagcgtgatcaactttgtggtgctgacctctgcggcgtcttccgctaacagcggcgtcttctctaccagccgtatgctgtttggtctggcgcaggaaggtgtggcaccgaaagcgttcgctaaactttctaagcgcgcagtacccgcgaaagggctgacgttctcgtgtatctgtctgctcggcggcgtggtgatgttgtatgtgaatcctagtgtgattggcgcgttcacgatgattacaaccgtttccgcgattctgtttatgttcgtctggacgattatcctttgctcgtaccttgtgtatcgcaaacagcgtcctcatctacatgagaagtcgatctacaagatgccgctcggcaagctgatgtgctgggtatgtatggcgttctttgtgttcgtggtcgtgttgctgacactggaagatgacactcgccaggcgctgctggttaccccgctgtggtttatcgcgctggggttgggctggctgtttattggtaagaagcgggctgctgaactgcggaaataaccgcattatcatgctggatggcgcaatgccatccagcttttagatcactcacccgccagcgcgcgtgggaacagtacattgttttccagactgatgtgatccatcaggtcatcaatcagttcattaatgccgttatacatcgctttccaggtggtgcaggcttctggcggcggtgtgacgttattggtggtgtgtttaatcacttccagcagttcgcccgcttcatcgtgctcgctttccattacgctgattggccccattgcctggctgcccatgccttgtttgatcatcgggaagaggatctgctcttctttcatcatgtggctggaaagctcttcatgcagcatggtcaggtattttgtcagcccttttggcacgctcggtttgtcggcgtgaacgcgctcgactttagtcgcttgcagaatcagctccggcagttgctcgcggtgacgatcgtggtagcgcacgatgatatggtcgatgatttctgccagcggggcgctacgccagtctttctcaatcggttgttcagcgagctttgccagttcagcttcaatgacctcaacatccagttctttacgtgccgccgcgcgcgccagcgtctgcttaccgccacagcagtaatccatatcatatttacgaaacagagctgaagcgcgaggaatagagagcgccagttcacctaaaggttggtcgcgataagccatagctgatacctcattcttaataagataagatgtattttaaatgcatctttaaggcaaaagctataacccttacgtagcagaggcttatttaactcactgccagcgtgtcaactttctgagacagattcagttaaaggtttttctggttttgctctgaccgcgatgaccacgccaatcactaacagcgcgataccgctcagcgtcattagcggcggcatttgctggcggagtaaaaaggtgtacagcaaacctgccagcgtttcgaaaacaatcagcggcccgagaatcactgtcggtaatagctggctggcgacgttccagcagagtgcgccaacccatgagcaaagcacggctatcgcaaccatcagactaataaacaccagcggacgggggccaaagggtagggagaagtccggcgtttgcgtattcagccagtaacaagcgacgagatagccgataagtgaaaccggcagtgtgaccagcgcctgcgctgttgcccacatcatcggatgtttgtcgggattttcccgcagccagcgggcgttgcgcagggcataccacgcccagcagaccacggaaactaacgccagcacgatgccagaggtataacgtgcccagtcaaaatcggggagtccgtggtttaactcagcaatattcacacacgccaggccgatgccaatacaaatcagtgctggggcgagttttccccacgcgagtttgccgtcgcgctggctataaagcagattggcaaagacaggaatgaccaccggcagggtgccgataatcatcgtggaaacaggcgcgccagtacgttgaatggcactggcaaggcagaagtaatagatgaggttgcccatcatagtgagcatcaaggcggtaagccagtcgcgacgcgccaactgacgcagacgcacgcgtcccagccaggcaatgggcagcgcaattaaccctaacgccagataacgccccatcgactgcaacatcgccgggtattccggcacgatcaacggcccgacaaaaataagcccccacatcaaccctgctaacagggcgtacagcacgccgctaatcattactggcatccattgatctgtcagaagaaagttcaggaagcagacatgattgctcccggcatcccgtcattatcagagaggatgcgggaggatgccactttaattaactagttattaacattaaaaagatggcttacgctttcggctaacgttgtcgttgggtggccaatcaatttgctaagtgttttgctgtcatcaaacagaccgcctttcgatgcgccaacgtcagaatccgccagcatatccgccagtccgtcgggcagtccgacgcttttcagtgccgcggcgaaatcggcttcgctcagattttgataggtaacctgtttgccgctctgtttggtcagctctgccgctaactgtgtcaacgtccaggcactatcgcccgccagttcgtaaaccttgccttcgtgaccggcttcgctaatcacgcgtgccgcagctgccgcataatctgcccgcgttgctgaggcgattttgccatcgcccgccgcaccgataaatacgccgtgttccagtgctgccggggcgctggcgaggtagttttcgctgtaccagccgttgcgcagcagggtgtaaacgatgccagaatcagccagcattttctccgtctcgatgtgctcatcggcgaggccgagcggggaggtatctgcatgtagcaggctggtataagcgataaatttcacgccagccgcctttgcggcattaataacattacgatgctgcggggcacgttgacccacttcgctggaagagatcagcagtagtttttccactccctgaagtgcagatgtcagtgcggcttcatcgccgtagtcagcctgacgcacggtaatgccttgtgctgccagggcttgggcttttgccggattacgaacgatagccactatttggctggcaggaaccgttttcatcaaggattcaataacatagtgaccaagttggccagtggcaccagtaatagcgatcatgggaagtctccatcgttttgtcttgtgtttaaatacgctaacacctaaacttacttttagtaagtacgtacaaaaaggtaagtatgaaatgagtcaggttagcctgtcgcaacaactgaaagagggtaatctctttgcggaacagtgcccgtcgcgcgaggtgttgaaacacgtcaccagccgttggggggtgttgattctggtggcgctacgcgaaggtactcatcgctttagcgacctgcggcgcaaaatcggtggggtgagtgaaaagatgcttgcgcagtcgttacaggcgttagaacaggatggttttcttaaccgtatcgcgtatccggtggtgccgccgcatgtggaatatagcctcacgccgctgggcgagcaggtgagcgaaaaggttgctgcactggcggactggattgagttgaatttgcccgaggtgttggcggtgcgggatgaacgtgcggcataactgccggatgcgctgagcttatctggtctacggtgcatggcttgtagggcggataagatgcgccagcatcgcatccgccaataaatgccggatgcggttgatgatttataggccgaaaaagaagtgttttacttactcaaatccacctgataaatcgcaaacccgatatcatcggtcgcgactttattcatcggatactgccctttctctttaataaacgctgcggctttatctgacggagaggtttcgaaacggatatccagtttcttatcgccagctatcggtgctaaacgccagttgttatctgccgccgggtgaatttcccccgcacgtttcgactcatcagcaatccacgctgccagcaccgagcggttctcatccggtgaagcaaaagcgatatggctgtcgcccgtaccggcaaatttgccgccgtaagcgcgatagttattggtggcaaccaggaacatggcgttcggatcaatcggcttgccattaaaggtcaggttcttaatcctttccgcattggcattaatcatctggcactcgccgtcataacgggcgggctgggtaacatcaatctgataattcacaccatcaataacatcaaagttataagtgcggaaaccatcccagttgatgagtgactgtggtttcgtgctgttgggatcaatctggttaaactgtcccgcggagcactccagccactctttcacctctttaccgctggctttcaccacaatcagcgtattgggatagagataaagatcggcggcattacggaaggtcaactggcctttttccacctccacatagcttgccgggtcatttttgcgaccaccgactttaaacggtgcggcagctgaaagcaccggcagttttgccagatccggatcgccctgaatgtaatgctcgacatacgctttttgcgcgttgttcaccacctgcacggtcggatcgtcctgcaccagcgccagatagctatacatattgtcggcagatttaccgattggcttgctgacgaactggcgtgtggcatcgtgatcggctttgagtgtttctaccagcttgctgtcttccgccgcgagggattttttattagcgatgtcgtaaatcggtcgtgcttccgctttcgcctgcgtcacctgccatttaccgctgtcattactgagttgtaagtcgaccacaccaagatgatcgccccacatgcctggcattaccgccggaacaccattcagcgtgcctttggcgatatcagccccttcgatatcagcaaaatctttacctgggaaaacggcgtgagcatggccaaacataatggcgttaacgcccggaatttcactgaggtaataaactgagttttccgccatcactttatacggatcggcagatagcccggaatgtgccagaacgacaacaacatcggcacctttctcgcgcatttcaggcacgtatttgcgcacggtttcggtaatatcattcaccgtcactttcccggataaattagctttatcccagcccatgatttgtggtggcacgacgccaatatagccaatcttcagcgtctgtttttttccgtctttatcgaccacttcggtgtctttaattaaatacggtgtaaacattggctgtttggttctggcgtcaatgacgttggcatttacataagggaatttcgctcctgccagcgcatttttcaggtaatccagaccgtagttaaactcgtggttgccaagcgttccgacggtatagtccagcgtatttaatgccttatagaccgggtgaatatcacctgcttttaatcctttcgccgacatgtaatcggccagcggactcccctgaatcaaatcgccgttatcaaccagtacgctgtttttcacttcattgcgggcatcgttaatcaggcttgccgtacgtaccagtccgaatttttccgtggcggtgtctttgtaataatcgaaatccatcatgttgctatgcagatcagtggtttccatgatacgcagatcgaccgtcgctgcattcacactggcggcaatcagcgtggccaggagcgttgcgctaaacttaatcatcagggacatccttttatcatcgggaatacgaaagaaaagggagaataaacgtcttacttatagaacagtgaagaatgccacaattttacgctttgaaaatgatgacactatcacagttggcgcattcattaacgatagggtataagtaaaacaataagttaacaccgctcacagagacgaggtggagaaatgttagatcaagtatgccagcttgcacggaatgcaggcgatgccattatgcaggtctacgacgggacgaaaccgatggacgtcgtcagcaaagcggacaattctccggtaacggcagcggatattgccgctcacaccgttatcatggacggtttacgtacgctgacaccggatgttccggtcctttctgaagaagatcctcccggttgggaagtccgtcagcactggcagcgttactggctggtagacccgctggatggtactaaagagtttattaaacgtaatggcgaattcaccgttaacattgcgctcattgaccatggcaaaccgattttaggcgtggtgtatgcgccggtaatgaacgtaatgtacagcgcggcagaaggcaaagcgtggaaagaagagtgcggtgtgcgcaagcagattcaggtccgcgatgcgcgcccgccgctggtggtgatcagccgttcccatgcggatgcggagctgaaagagtatctgcaacagcttggcgaacatcagaccacgtccatcggctcttcgctgaaattctgcctggtggcggaaggacaggcgcagctgtacccgcgcttcggaccaacgaatatttgggacaccgccgctggacatgctgtagctgcagctgccggagcgcacgttcacgactggcagggtaaaccgctggattacactccgcgtgagtcgttcctgaatccggggttcagagtgtctatttactaaattcagatggcagaaacagtgtatttcctgattctgccatcctgatttctcccaacctaaaaagttataaataaaaagagattgtatttaaagtgcaaaaattcaattgctaataagttacattttaataatgagcgttttttgatagtttacttctatagtgagatatttaatggcgacataaagtaaccaaataaaataaggttgtcatatgttacccaggatcagacacaataattttattggtgcggtggagttatttgtaaagtcttcgtatacaaaaacacattcaaacaatttttttaacaacatccatcatgcatttaagaaaaaagattggatttcgaattatgatagcctgttaactttgagggagttctttcgttgcgcaactcagattgataaaagtggttatcaggtgctttcatcaaaaaatgaaactgttcacgccatggataagtttcttatcagtttcagccttaaagataacggtgccgaatatacaatgacattgcgaggtagtggatttgaatacgaagaaatacccataacaataaatgaatataactcattcatggatttcaaaaaccgtgaatttccgttagaacaaaacagacgattgtatgcctgggatattctacagaaaaaacagtctgacataccgaaaaggattaaaggttatattcaccaggcgattggtgacgtgtctttaggttatgccttattggaggatatagtaagcaaattaaaacggggtaaatttgaactccaaataccaggaggtggaattaaagaatgcgatggatggtatatttacgaaaaaataattgatgataattttgccatagtcatagaatctttgggctttgcgcttaaaatctatggaggggatgaacgttttcgtaatggttcctctgttgttttggaggatgaagattactctcttatttataattttctggttaatgcaggttgccaacaagtcgaattagccgaacaagtggatgcgatagtaagtgcgaatctggccgcagatagcgatattaccaaagaaaagatttgcgagaaatataaatcgaccattgaggcgtttaaaaaagagcaactagcgttaccagtattagttcggcgtaagaactcagagacttaattcccctatcccatagataacgataggggaaaattatttttgcagaatttatgttattgccattatttgagcaacttttgcagcaggtccatcacttgctgcacctcttccggtgtgagcgccccgtctttggcccattgcacgcgaccatccttatccagcaccactacagcggaactttcttcatccagctgccaggcaccgagcgcgacgccattgctatcgacaataaactgcgaccagggataaagctttttattactctccagactgctgcgcacaaacatccctgaacccggaatcgcgtcgtcggtgttaacaatggtggtggtctggtaacgatcgtgcggtaacttcgctgatttaatcgcttcaatcagcgtcgcgtttttctcttttgcagaggtgcgaccagcaatatgttgcagtactcgcacttttcccactaactgcgcgctgttccaggttttgtagctaaactgatctttatcaagcaccaactcgccccgatcggtaatgccaatcggcggcactcgctgaccggtttcgaactgatgtgcggaagccatcatcggcaacagcaggcaggtgagtgccagaatcttgcgtagggtcatggtgtttccttcttatgatatgcaggtgatccgaccacttgggtctgagttttaatcatatgtgctatttatcgaatttcccgcaagtgtgatgccagtttgcggtcaagcgcacaaatcatatgaaaaatgaatgcttatactgaagaccgcgcttcggtaaaaagataattctgaataattgtaacctttaggtaaaaaaagttatacgcggtggaaacattgcccggatagtctatagtcactaagcattaaaatttgcgcctcataatagttgggccgattgtggcaccgcacaggcgtaatactcagcaggagataacaatgaaaattttccaacggtacaacccacttcaggtggcgaagtacgtaaagatcctgttccgtggacggttatacatcaaggacgttggcgcttttgaattcgataagggtaagattcttatcccaaaagtgaaggataagctgcatttgtcagtgatgtccgaagttaaccgtcaggttatgcgtctgcaaacagagatggcttaaccaaagtgctatgcagtaaaaagtgctatgcagtaataagacggctcctgattcaggagccgttgatgtttctgggggttacgcgacgctttcttctttatctttagcgtcaggcagttttggcgaaagggcggtggccttgctgtcgatccgggtcaccagcagctggtcgatgcggtagttatcgatatccaccacttcaaatttgtagccggcgaatttcaccgaatcggtgcgtttcgggatcttacgcagcataaacatcataaagccgccgatggtttcgtagttgcccgactgcgggaactcgtcaatatccagcacgcgcatgacgtcgtcaattggggtgccgccgtcaatcagccatgagttctcatcacgggcgacaatctgctcttccagcccctgaccgaccagatcgcccatcagcgtggtcatcacgtcattgagggtgatgatccccaccaccagcgcgtactcgttcatgatcaccgcgaagtcttcacctgcggttttaaaactttccaacgcctctgaaagggttaacgtatccggcacaatcagcgtgttgcgaatttgtacgccgctgttcagtgccaggctttggttagccagcacgcggttcagcaggtctttagaatcgacataaccgatgatgtggtcaatatcttcattacagacgaggaacttagagtgcggatgttccgccaccttattcttcaggctttgctcatcttcgtggagatcaaaccaaatcacgttttcacgcggtgtcattgaagacggaacggtacgggattccagctcaaagacgttttcaatcagctcgtgttcctgtttacgtaacacgcccgccagcgcaccggcttccactaccgcgtagatgtcatcagaagtgatgtcatctttacgtaccattggcagtttgaaaatacggaagattatgttcgccaggccgttgaagaaccacaccagcggggtgcaaacgtacaggcagaagcgcatcgggttgatgatacgcaaagccacagcttctggcgcaatcataccgatgcgtttcggggttaaatccgcaaacaggataaacatgccagtcactaacgagaaagagagaataaagctcagttgctcagagagctctgccgacatatagcgggagaacaggctgtgaaaagctggagaaaatgccgcatcaccgacgataccgccgagaatcgccactgcgttcagaccgatttggaccacggtaaagaacatgccgggattttcctgcatattcagaacgcgttgggcatttatattgccttcatcagccagcagtttaagtttgattttgcgtgaggcggcaagcgagatctcggacatcgagaagaacgcacttacagcgatcaagcagagtatgactaaaatactgtttaacatatcttatccgacctttcaggccagatcctcggaaggggaagttgattaatttgtgtgaaatacacattgaaagccgattcgaagaaagtgaaccggcattttcagtggctagtatagcgtaaggtactgtaaagccgccagagggttaaaattcagacagctgaaaaatgcaaaactgcctgatacgctatgccgatcaggcctacgcagtccttgcaatatattgaatttggacgattttgtaggcctggtaagtcgtttacgccgcatcaggcatagacaaagagcactttatcaacaaactacatttgtacccgtaacgctatgcttccggcggcagacagacgccaattccgccaattccacagtaaccatacgggtttttatgcagatattgctggtggtcatcttcggcataataaaacggtgtggcgttagcgatttccgtggtgatgtgacgatcgtcatcggcggcaagcatcgccgcctgaaaacgttccagactggcgcgagctgcggcatcctgttctggggtcagcggataaatcgctgaacgatactgcgtgccgtggtcattgccctgacgcattccctgggcgggatcgtgattctcccaaaatacctgtagcaactgctcatagctgatgacggaaggatcgtaaacaatgcgtaccgcttcggcatgacccgtatcaccggagcacacttcccgataagtcggatttggcgtatagccgccggtatagcctgcggcggtgctgtaaacgccgggtaactgccagaacagacgctccacaccccagaaacaacccatcgcaaaaatggcaatctccattccgtcaggtacattggtcattgagtgaccgttgaccgcatgcagcgtggctacgggcatcggggtgttacgtccaggcagggcatcggcgggggaaaccagatgctttttatcaaataaactcatggtgtcgctctcccgaaaatcggtcattggggttaaggttgtaacaagaggcgtatttgcacacaataaccaccgtgaataggtctaaagtaaaacataagaaatatttggggtttagtctgctttttaatccatattactggatttttgttaagccgtttaacggcgttccaggggcaggaaaaaaggatattcaggagaaaatgtgcgctatatccgacagttatgctgtgtaagcttactctgcttaagcggatctgccgtcgccgcgaacgtccgtctacaggtcgaggggttatcgggacagctggaaaagaacgttcgtgcgcagctttctacgattgaaagtgatgaagtgacgccagaccgtcgctttcgcgcacgcgtcgatgatgccatccgcgaaggtctgaaagcgctgggttattaccagccgaccattgaatttgatctccgtccaccgccaaagaaagggcggcaggtattgatcgccaaagtcacgccaggcgtgccggtgttaattggcggcaccgatgtggtattgcgcggcggcgcgcggaccgataaagactatttgaaattgctcgatactcgcccggctattggcacggtactgaaccagggcgattatgaaaatttcaaaaagtccttaaccagcattgcgttgcgtaaaggttatttcgatagcgaatttaccaaagcgcagctgggcattgcgctcggcctgcataaagccttctgggatattgattataacagtggcgaacgttaccgctttgggcatgtgacctttgaaggatcacaaatccgcgatgaatacctgcaaaatctggtgccgtttaaagagggcgatgagtacgaatcgaaagatctggcagaactgaaccgccgactttctgctaccggctggtttaactcggtggtggtggctccacaatttgataaagcgcgcgaaacgaaagtattaccattgacgggcgtggtttcgccgcgaacagaaaacaccatcgaaaccggggtcggttactctacggacgtgggaccgcgcgtgaaagcgacgtggaaaaagccgtggatgaactcttatggtcacagtctgaccaccagtactagtatttccgcgccggaacagaccctcgacttcagctataaaatgccgctgctgaagaatccactggaacaatattatttggtgcagggcggttttaagcgcactgacctgaacgataccgaatctgactccactacgctggtggcttctcgctactgggatctctccagcggctggcagcgtgccattaacctgcgctggagtctcgaccactttactcagggtgaaattaccaataccacgatgctgttttatcctggggtgatgattagccgcacgcgttctcgtggtggcctgatgccaacctggggcgactcgcaacgctactctatcgactactccaacacggcctggggttcagatgtcgatttctccgttttccaggcgcagaacgtctggatccgcacactgtacgatcgccatcgttttgttacacgcggcacgctgggctggattgaaaccggtgatttcgacaaagtaccgccggatctgcgtttcttcgccgggggcgaccgcagtattcgtggctacaaatacaaatctatcgctccgaaatacgccaacggtgacctgaaaggggcctcgaagttgataaccggatcgctggaataccagtacaacgtgaccggaaaatggtggggcgcggtgtttgtcgatagtggcgaagcggtaagcgatattcgccgcagcgactttaaaaccggtaccggggtcggcgtgcgctgggaatcgccggtcgggccaatcaaactcgattttgccgtaccggtcgcggataaagacgaacacgggttacagttttacatcggtctggggccagaattatgagtttatggaaaaaaatcagcctcggcgtggttatcgttatcttactgttgctgggatcggtggcgtttctggtgggcaccaccagcggcctgcatctggtatttaaagcggcggatcgctgggtgccaggactggatattggcaaggtcaccggcggctggcgcgatctcaccttgtctgacgttcgttatgagcagccaggcgtggcggtaaaagcgggcaatctgcatctggctgtcgggcttgagtgcctgtggaacagcagtgtttgtattaatgatctggcgctgaaagacattcaggtcaacatcgacagtaaaaaaatgcctccttctgaacaggttgaagaagaggaagatagcggtccgctggatctctccacgccgtatcccatcaccctgacacgggtggcactggacaacgtcaacattaagattgatgacaccacggtatcggtgatggacttcacctccggcctgaactggcaggagaaaaccctgaccctgaaaccgacgtcgctgaaaggcctgctgattgctctgccgaaagtggcggaagtggcgcaggaagaagtggtcgaaccgaaaattgaaaatccgcagccggatgaaaagccgctcggcgaaacgctgaaagatctcttttctcgcccggtattgccggaaatgaccgacgtgcatttgccgcttaacctgaacattgaagagtttaagggcgagcagctgcgcgtgacgggcgacacggacatcaccgtgagcaccatgctgctgaaagtgagcagcattgacggcaatactaaactggacgccctggatatcgattccagtcaagggatcgtcaacgccagcggcacggcgcagctgtcagacaactggccggtggacatcactctcaacagtacactgaacgtggagccgttgaaaggtgaaaaagtgaagctgaaaatgggcggcgcgctgcgcgaacagctggagattggcgttaatctttccggtccggtggatatggatttacgcgcccagacgcgactggcggaagccggattgccgctcaacgtggaagtgaacagcaaacagctttactggccgttcactggtgagaagcagtatcaggcggatgatctgaaactgaaacttaccggcaaaatgaccgattacacgctctctatgcgtacggcagtgaagggacaggagatcccgcccgcgactattaccctcgacgccaaaggtaatgaacagcaggtcaatctcgacaaactcaccgtcgcggcgctggaagggaaaactgaactcaaggcgttgctcgactggcaacaggccattagttggcgcggtgagctaacgcttaacggcattaacaccgccaaagagttcccggactggccgtcgaaactcaatggcttgattaaaacccgcggtagcctgtacggcggcacctggcagatggacgtgccggagttgaagctgaccggtaacgttaaacagaacaaagtgaacgttgacggcacgctgaaaggcaacagttatatgcagtggatgatcccagggcttcatctggaactcgggccaaacagtgccgaagtgaaaggcgagctgggggtaaaagatctcaatcttgatgccaccatcaacgcgccggggctggataacgcgctgccggggcttggcggtacagcgaaagggctggtgaaagtacgcggcacggtggaagcgccacaactactggcagatatcaccgcgcgcggcctgcgctggcaggaactttccgtggcgcaggttcgcgtggaaggcgatatcaaatccaccgatcagatcgccgggaaactcgacgtacgcgttgagcaaatttcgcagccggatgtaaatatcaacctcgtcaccctgaatgccaaaggcagcgaaaagcagcacgagctacagttgcggattcagggggagcctgtctccgggcagcttaatctggcaggaagttttgatcgcaaagaagaacgctggaagggaactcttagcaatacccgcttccagacgccggttggcccgtggtcgctgacccgcgatattgcgctggattaccgcaataaggagcaaaaaatcagcatcgggccacactgctggcttaacccgaatgcggaactgtgcgtgccgcaaactatcgatgcgggggccgaagggcgtgcggtggtgaatctcaaccgcttcgacctcgccatgctgaaaccgtttatgccagaaaccactcaggccagcggtatcttcacgggtaaagcggacgttgcctgggacaccacgaaagaggggctgccgcagggcagtatcaccctttcggggcgtaacgtgcaggtaacgcaaaccgtcaacgatgcggcgctgcccgtggcgtttcagacactgaatctgacggcggaattgcgtaacaaccgtgccgaattgggctggaccatccgcctgaccaataacggccagtttgatggacaggtgcaggtgaccgatccgcaaggccgccgtaatcttggtggcaacgtcaatatccgtaacttcaaccttgcgatgataaaccccatctttacccgtggggaaaaagcagcggggatggtgagtgccaacttgcgtctgggtggtgatgtgcaaagcccgcagttgtttggtcagcttcaggttacgggtgtggatatcgatggcaactttatgccgtttgatatgcaaccgagccagcttgcggtcaactttaacggtatgcgctcgacgcttgccggtacagtacggacccagcagggtgaaatctacctgaacggtgatgccgactggagccaaattgaaaactggcgggcgcgggtaacggcgaaaggcagtaaagtgcggatcaccgtgccgccgatggtacgaatggatgtatcgccagatgttgtattcgaggctacaccaaacctgtttaccctcgatggtcgcgtggatgtcccttgggcgcgcatcgtggtgcacgatctgccggaaagcgcagtaggcgtctccagcgatgtggtgatgcttaacgataacctgcaaccggaagagccgaaaacggcgtcgattccgattaacagtaacctgattgtccacgttggcaacaatgtgcgcattgacgcctttggcctgaaagcgcggctgacgggcgatctcaatgtcgttcaggacaaacaagggctgggtctgaacgggcagatcaacatccctgaagggcgcttccatgcctatggtcaggatctgattgtgcgtaaaggtgagttactgttctctggtccgccagatcaaccgtatcttaatattgaagctattcgtaacccggatgctacagaagacgacgtaatcgccggagttcgcgtcactggtctggcggacgaaccgaaagcggagatcttctctgacccggcgatgtcgcaacaagctgccttgtcttatttgctacgtggacaagggctggagagcgatcagagcgacagtgcggcaatgacctcgatgctgattggtttgggggttgcgcaaagtggccagattgtgggtaaaatcggcgagacgtttggcgtaagcaatttagcgctcgacacccagggagtaggcgactcctcccaggtagtggtcagcggctatgtattgccaggtctgcaagtgaaatacggcgtgggtatatttgactctatagcaacactcacgttacgttatcgcctgatgcctaagctatatctggaagccgtgtctggtgtagaccaggcactggatttgctctatcagttcgagttttagcaatgcgaatatttgtctacggcagtttacgccacaaacaaggcaacagtcactggatgaccaatgcccagttactgggcgatttcagtatcgataactaccagttgtatagcctgggccactatccaggcgcagttccggggaacggaacggtacacggtgaagtttatcgtattgacaacgccacgctggccgaacttgatgccttgcgcaccaggggcggtgaatacgcgcgccagttgattcagacgccgtacgggagtgcatggatgtacgtttatcaacgacccgtcgatggattaaagctaattgaaagcggcgactggttagacagggataagtaaccatatgcatacgccaccttcgggtggcgttgttttttgcgagacgactcgcattctgttttgtaattccctcaccttttgcttttctctccgagccgctttccatatctattaacgcataaaaaactctgctggcattcacaaatgcgcaggggtaaaacgtttcctgtagcaccgtgagttatactttgtataacttaaggaggtgcagatgcgtattaccataaaaagatgggggaacagtgcaggtatggtcattcccaatatcgtaatgaaagaacttaacttacagccggggcagagcgtggaggcgcaagtgagcaacaatcaactgattctgacacccatctccaggcgctactcgcttgatgaactgctggcacagtgtgacatgaacgccgcggaacttagcgagcaggatgtctggggtaaatccacccctgcgggtgacgaaatatggtaaagaaaagtgaatttgaacggggagacattgtgctggttggctttgatccagcaagcggccatgaacagcaaggtgctggtcgacctgcgcttgtgctctccgttcaagcctttaatcaactgggaatgacgctggtggcccccattacgcagggcggaaattttgcccgttatgccggatttagcgttcctttacattgcgaagaaggcgatgtgcacggcgtggtgctggtgaatcaggtgcggatgatggatctacacgcccggctggcaaagcgtattggtctggctgcggatgaggtggtggaagaggcgttattacgcttgcaggcggtggtggaataaggtgtgtttatttatcgcgggcataaaaaaacccttactaaccgaagcccggcgttcagggttattacgccagaagaacttatttattctttgcgcgctcgaaggaggcaacgatttcagctttagcggcttctgcgttttcccaaccttcaactttcacccacttgcctttttcgaggtctttgtagtgctcgaagaagtgagcgatttgcgctttcagcagttcaggcagatcgttaacgtctttaatgtgatcgtattctttgctcagcttgctgtgcggaaccgcaaccagtttcgcatcttcaccggcttcgtcggtcattttcagaacgccaaccggacggcaacggatcacagaacccggctgcagcgggtacggagttgggaccagtacgtcaaccgggtcaccgtccagagacagggtgtggttgatgtaaccgtagttgcatggatagaacatcgcggtggacatgaagcggtcaacgaacagtgcgccgctctctttgtcgatttcgtatttgatcggatctgcgttagccgggatctcaataacaacgtagatgtcttccggcagatctttacccgcagggacgttgagtaagctcatgtctgtttcctttaaaaatatgtggcaaacaagtgccgagtattatagccaactcgcgccgaatgtcttcgcttgttttcgtcttcattttcctttttcaccagttttaagacggtatacagagcaggaaaatccataaccgtagccgcatttttcatagtgagatgaaagcgattacaaacttgtgattaacgttttatttacttttttgaagtgtgatgtaacgcaatctgttacataacgaattgtctatagttttttcgcgaacatcttttaaccaataataactaccccgacgaggacaaccctatgtggaaacgcttacttatagtctctgcagtctcggcagccatgtcgtctatggcgttggccgctccattaaccgttggattttcgcaggtcggatcggaatcaggctggcgtgccgcagaaaccaatgtggcgaaaagtgaagccgaaaagcgcggaatcacgttgaaaattgccgatggtcagcaaaagcaggaaaaccagattaaagcggtacgttccttcgttgcacaaggggtggatgcgatctttatcgctccggtggtcgcgacaggttgggaaccggtattaaaagaggcgaaagatgccgaaatcccggtattcttgctcgatcgttccattgatgtgaaagacaaatctctctatatgaccaccgtcactgccgacaacatcctcgaaggcaagttgattggtgactggctggtaaaagaagtgaatggcaaaccatgcaacgtggtggagctgcagggcaccgttggggccagcgtcgccattgaccgtaagaaaggctttgccgaagccattaagaatgcgccaaatatcaaaatcatccgctcgcagtcaggtgacttcacccgcagtaaaggcaaagaagtcatggagagctttatcaaagcggaaaacaacggcaaaaacatctgcatggtttacgcccataacgacgacatggtgattggtgcaattcaggcaattaaagaagcgggcctgaaaccgggcaaagatatcctcacgggttccattgacggtgtaccggacatctacaaagcgatgatggatggcgaagcgaacgccagtgttgaactgacgccgaatatggcaggtcccgccttcgacgcgctggagaaatacaaaaaagacggcaccatgcctgaaaagctgacgttaaccaaatccaccctttacctgcctgataccgcaaaagaagaattagagaagaagaaaaatatggggtattgagggttgctatgcctgatgccgattcgtaggccggataaggcgctcgcgccgcatccggcgatggtgcactgaagcctgatgcgacgcttaccgcgtcttatcatgcctactgggagcacgctttacaccgggggaaaccatgacgaccgaccaacaccaggagatcctccgcaccgaaggattaagtaaatttttccccggcgtcaaagcgttagacaacgttgatttcagcctgcgccgtggcgaaatcatggcgctgctcggtgaaaacggggcgggaaaatcaacgctaatcaaagcattaactggtgtataccacgccgatcgcggcaccatctggctggaaggccaggctatctcaccgaaaaataccgcccacgcgcaacaactcggcattggcaccgtctatcaggaagtcaacctgctacccaatatgtcggtcgctgataatctatttataggccgcgaacccaaacgcttcggccttctacgccgcaaagagatggaaaagcgcgccaccgaactgatggcatcttacggtttctccctcgacgtgcgcgaaccgctcaaccgcttttcagtcgcgatgcagcaaatcgtcgctatttgtcgggctatcgatctctctgccaaagtgctgatcctcgatgaacccaccgccagtctcgacacccaggaagtggagttactgtttgacctgatgcgtcagttgcgcgatcgcggcgtcagcctgatttttgtcactcactttctcgatcaggtctatcaggtcagcgatcggatcaccgtcttacgcaacggcagtttcgtaggctgtcgggaaacgtgcgagctaccgcagatcgaactggtaaaaatgatgctggggcgcgagctggatacccacgcgctacagcgtgccgggcgaacattgttgagcgacaaacccgttgccgcgttcaaaaattacggcaaaaaaggaacgatcgcaccgtttgatctcgaagtacgccccggcgagatcgtcggtctggctggattgctgggatcaggacgtaccgaaaccgccgaagtgatcttcggtatcaaacctgctgacagcggcacggcgttgatcaaaggcaaaccgcaaaacctgcgatcgccacatcaggcttcggtactgggcattggcttctgcccggaagacaggaaaaccgatggcatcatcgctgccgcctcggtgcgggaaaatatcatcctcgctctccaggcccagcgcggctggctacgtcccatttcccgcaaagaacagcaagagattgccgaacgctttatccgccagcttggcattcgcacaccttcaactgaacaaccgattgaatttctctccggcggcaatcagcaaaaagtgttgctttcacgttggctactgacccgaccgcaatttctgatcctcgatgagccaacccgcggcattgatgttggtgcccacgccgagatcatccgcctgattgaaacgctatgcgccgatggtctggcgctgctggtgatctcctccgaactggaagagctggtgggctatgccgatcgggtgattatcatgcgcgatcgcaaacaggtggcggagatcccgctggcagagctttccgttccggcgatcatgaacgccattgcggcgtaaggagaacagtgtgatgcctcaatctcttccggacaccactacgccaaaaaggcgctttcgctggccgacggggatgccgcagctggtagcactattgctggtgctgctggtcgatagcctggtagccccgcatttctggcaggtggtgcttcaggatgggcgtttgttcggtagccccatagacattcttaaccgtgcagctcccgttgcgttactggcgattggcatgacgctggtgatcgccaccggtgggattgatctctccgtaggggcggtgatggctatcgccggagccacaacggctgcgatgacggtcgcgggattcagcctgccgattgttttgttaagcgccctgggcaccggcatcctggcgggattgtggaacggcatactggtagcgatcctcaaaattcagccgtttgtcgccactctgatcctgatggtcgccgggcgcggcgtggcgcaactgatcaccgccgggcagatcgtcacgtttaactcgccggatctctcatggttcggcagtggatcgctgttgttcctgccaacgccggtcattatcgcggtgctgacgcttatcctgttctggctgttgacccgcaaaacggcgctggggatgtttatcgaagccgttggtatcaacattcgggcggcaaaaaatgccggggtaaacacgcgaatcatcgtcatgctcacttatgtgttgagcgggctgtgtgcggcgattgcgggcattatcgtggcggcggatattcgcggtgccgatgccaacaacgctgggttatggctggagctggacgccattctcgcggtggtgattggcggcggatcgctgatgggcgggcgctttaacctgctactttcggtggtgggggcgctgattattcaggggatgaacaccggaattttgctttcgggctttccgccagagatgaaccaggtggtgaaagcggtggtggtgctttgcgtgctgattgttcagtcgcaacgctttatcagtctgattaaaggagtacgtagccgtgataaaacgtaatttgccactgatgatcaccatcggcgtctttgtgttgggttatctttactgcctgacccagtttcccggttttgcttccacaagagtgatctgcaatatcctgaccgataatgcctttcttgggatcattgccgttggcatgacctttgtgatcctctcaggtgggatcgatctctccgtcggttcggtgatcgcctttactggcgtgtttctggcaaaagtgattggcgatttcggcctctcgccgctgctggcgtttccgctagtgctggtgatgggctgtgccttcggcgcatttatggggcttctgatcgacgccctgaagatcccggcatttatcattacgcttgcggggatgttctttttgcgcggcgtcagctatctcgtttcggaagagtcgattccgataaaccatcccatttatgacacgctctcaagccttgcgtggaaaatccctggcggcggtcgcttaagtgcgatgggactgctgatgttggcggtggtggttatcggcatattcctcgcgcatcgtacccgttttggtaatcaggtatacgccattggcggcaacgcaacgtcggcgaatctgatggggatttccactcgcagcaccactattcgcatttatatgctctccaccggactggcaacgctggcggggattgtcttctcgatttatacccaggccggatatgcgctggcgggcgtaggtgtggaactggatgctatcgcctcagtggtaattggcggtacgcttttgagcggtggcgttggaacggtattagggacgctttttggcgtggcgattcagggactgattcagacttacataaactttgatggcacgctgagttcctggtggacgaaaatcgccatcggtattttgttgtttatttttatagcattacagcgtggattaacggtgctgtgggagaatcgtcagagttcgccagtgacaagagtcaacattgcgcagcaataaaaacgcctctccgtgtggagaggcgcaggagattacgcgtccgggaactcacggataaagcgttcgacatcttcaaccatatggtcgttgccgacaaagaatgaacggcgctggtgcagggtttccgggatgatatccagaatacgctctttgccatcgctcgctttaccgcccgcttgttccgccaggaatgccatcgggttgcactcatacagcaaacgcagtttgccgtccgggtggctggcggtgcttgggtagagataaataccgcctttcagcaggttacggtggaaatccgcgaccagtgaaccgatataacgtgaggtataagggcggttggtggatttatcttcttcctggcagaatttaatgtacttcttcaccccgttcggaaacttaatgtagtttccttcgttgatggagtaggttttgcctttctccgggaagcgcatccgttcctggcacaggcagaaaacgccgagcgaaggatcgtaagtaaaggcgtgaacaccgcatccggtggtgtaaaccagcatggtagaggagccgtataccacgtaacctgccgcaacctgtttgttaccaggctggaggaaatcttcttccgttaccggcgtgccaacaggcgtaacgcggcggtagatggagaaaatggtaccgacagagacgttaacatcgatgttggacgagccatccagggggtccatcagcaccacgtattttgcgtgttcacagccttcaaagacgacaatctcatcttcttcttcagaggcaatgcccgcaacgatatcgcgtgctttcagtgcggctttcagtttttcattagcgaacaagtcgagtttctgctgaacctcgccctgcacgttctcagcaccgctggcacccaggatatcaaccagtcctgctttgttgatatcgcgatggataatcttggcgcccagttttattgccgacagcaaagcagtgagctcaccggtagcatgagaaaactcgtgctgcttttcgacaataaattcacctaacgttttcataaaactttccctgcaatgtttatggagtaaagcgaccgcaacaatcttaacaaataatctcaatgttgcgctcaggtgaatcgcgccagcaaattacggattatcctgaaatgcgtttctcacttgcccgacatatgcgtaaaatgagcggcagattaaaaaaggatagtgacgtatgcgcattcatattttaggaatttgtggcacatttatgggcggtctggcgatgctggcgcgccagttaggccatgaagtaacgggttcggacgccaatgtgtatccgccgatgagcaccttacttgagaagcaaggcattgagctgattcaggggtacgatgccagccagctcgagccgcagccggatctggtgattattggcaacgccatgacccgtggaaatccgtgtgtggaagcggtactggaaaaaaatatcccttatatgtcaggtccacagtggctgcacgattttgtgctgcgcgaccgctgggtgctggccgttgccggtacacacggcaaaaccaccaccgcgggaatggcgacctggattctggaacagtgtggttacaaaccgggctttgtaatcggcggtgtgccggggaactttgaggtttcggctcatctgggcgaaagcgacttctttgttatcgaagcggatgagtatgactgcgccttcttcgacaaacgctctaaatttgttcattactgcccgcgtacgctgatcctcaacaaccttgagttcgatcacgccgatatctttgacgacctgaaagcgatccagaaacagttccaccatctggtgcgtatcgttccggggcagggccgtattatctggccggaaaatgacatcaacctgaaacagaccatggcgatgggctgctggagcgagcaggagctggtgggtgagcagggtcactggcaggcgaaaaagctgaccaccgatgcttccgaatgggaagttttgctggatggcgaaaaagtgggcgaagtgaaatggtcgctggtaggcgaacataatatgcacaatggcctgatggcgattgcagcggctcgccatgttggtgtagcgccggcagatgccgctaacgcgctgggttcgtttattaatgctcgtcgccgtctggagttgcgtggtgaagcgaatggcgtcacggtatatgacgattttgcccatcacccgacggcgattctggcaacgctggcggcgctgcgtggcaaagttggtggtacggcgcgcattattgctgtgctggagccgcgctcgaataccatgaaaatggggatctgcaaagacgatctggcaccttcattaggtcgtgccgatgaagtcttcctgctgcaaccggcgcatattccgtggcaggtggcagaagtggcagaagcctgcgttcagcctgcacactggagtggcgatgtggatacgctggcagatatggtggtgaaaaccgctcagcctggcgaccatattctggtgatgagcaacggcggttttggtgggatccatcagaaactgctggatgggctggcgaagaaggcggaagccgcgcagtaattcggccttagccagatatagtatgcgtaggccggataaggcgttcacgccgcatccggcatttgagcatagtgcctgatgcgacgcttgatgcgtcttatcaggcctacaggtgcaccgtatccggcaaaccatactcacatcaacaacgaaaattacccttcgttctccgctaactcgcgcagatactggaaaatctggcgtgcggatttcggcggcttattcccttctttctctttcttcgcgttgcggatcagagtacgcagttgctgacgatcggcatcgggccacagatttaatacctcagcgatggcgtcatcaccttgatcgatcagacgatcgcgcaggttttccagtttatggaacagcaccacctgctggttgtgacggtttttcagcttatccagcgcctgacgaataggctctacgtcgcgctggcgcagcatcttaccgatgagctgcaactggcggcggcgaccttccatcttaatacgctgggcgagctcaatagccgcgcgcagatccgcatctaacgggatcttatccagcgcgtttttccccagatcaacaatttccgcgccaaggcgttttagctcctcggcatcacgtttaatttcacttttactgacccagataatttcatcgtcttcgtcttcgatgtcatcaccgggaacgtcgtcgagccagtcttcgggctgcttagtcatctcaggctccttaaaaaaagaggctaatgttaccagttaagatgcgcactgaaaaacggttctctgttagacttcagagaaactctctacattatggcacttgcaatgaaagtaatctctcaagttgaagcgcagcgcaagattctggaagaagcagtttccactgcgctggagttggcctcaggcaaatcggacggtgcggaagttgccgtcagcaagaccaccggcattagcgtaagcacgcgttatggtgaagtggagaatgttgaattcaatagcgatggcgcgctggggatcactgtttatcaccagaaccgcaaaggtagcgcatcatccaccgatttaagcccgcaggccattgcccgtactgtacaggcggcgctggatattgcccgttatacctcgccagatccctgtgccggcgtggcagacaaagagctgctggcctttgacgcaccagatctcgacttgttccaccctgcggaagtttccccggatgaagccattgaactggcggcccgcgcagaacaggcggcattgcaggcggacaaacgcatcaccaataccgaaggtggcagctttaacagccactacggtgtcaaagtttttggcaacagccacggcatgttgcagggttactgctcaacgcgtcattcgctctccagctgtgtaattgccgaagaaaatggcgatatggagcgtgattacgcctacaccattggtcgtgcgatgagcgatctgcaaacgccagagtgggttggggccgactgtgctcgccgtactttatcgcgtctgtcaccgcgtaaactctccaccatgaaagcgccagtcatttttgccaatgaagtggcaaccgggctttttgggcatctggtgggggcgatagcgggtggatcggtttatcgtaaatctaccttcctgctggattcgctgggtaaacaaattctgccggactggctgaccattgaagagcatccgcatctgctgaaagggctggcgtcgacgccattcgacagcgaaggtgtgcgcaccgagcgtcgcgatattattaaagatggcatcctgactcagtggctgctgaccagctactcggcgcggaaactggggctgaaaagcaccggacatgcgggcggtattcacaactggcggattgccggacaaggtctaagcttcgagcagatgctcaaagagatgggcaccgggctggtggtgacggaattgatgggccagggcgtgagtgccattaccggtgattattcccgtggtgcagcgggcttctgggtagagaatggcgaaattcagtatccggtgagcgaaatcaccatcgcaggtaatttaaaagatatgtggcgcaatattgtcaccgtcggtaacgatattgaaacacgcagtaatatacagtgtggttctgtgctgttgccggagatgaaaatcgccggacagtaaaaaaactggcgcgacctgccgcgctataaactaaaaaattacacaaaatcattcgcactgcatcgagacggaaagtgaatgagggccggggagcgtactcgcagtacgtgacccggtcgaatgagcgtagtcgtcgatgaggcagtgtgaaggatgaagtgtaaataaaaaaggaactattcttgcagtctcctcgttggtattcagttcggcgtcatttgctgctgatctcgaagacaatatggaaaccctcaacgacaatttaaaagtggtcgaaaaagccgataacgcggcgcaagtcaaagacgcgttaacgaagatgcgcgccgcagcgctggatgcgcaaaaagcaacgccgccgaagctcgaagataaatcaccggacagcccggaaatgaaagatttccgccacggtttcgacattctggtcggtcagattgacgacgcgctgaagctggcaaatgaaggtaaagtaaaagaagcgcaggctgctgcagagcaactgaaaacgacccgcaattcatatcacaagaagtatcgttaattcctcatttccctgttgcctgcactcaggtaacagggaacttatcatcgcaaatgatgcaccacctgattgctgctgccgcgccagatcagggaagggtcttttaaatcctgcacaaatttgccgtcgaccagcacgttaatcaaatcaacaacctgcatttgcgcagcgttgagttcgtcgagtttatagcctgtccacacccagatgtctttacccggacactcggcgcggatgcgttgtaccagtttcagaatatccggcacgttttgcggatgcagcggatcgccgccggagagggaaataccctggcgtttgatacgagtgtcattcagatcgttaatgatctggtcttccattgctttggtaaatggctgaccggaatttacccgccatgtgcttttgttatagcaaccggggcattcatgaacacacccggagacaaacagggtgcaacgagtgccggggccgttgacgatgtcgacaggatagtactgatgataattcattatttcgcctggcttatcagtccgcgtgtaggctgcatccggtaatcaatgcctgatgcgacgctgtcgcgtcttatcagacctggagcaattgccaaatgtaggccggataaggcgtttacgccgcatccggcatttgcttagctcagagtgaagattaacctatctgcccattccccaaatgtttaacgcggcgcttaacttcttcctgcttaccagcgttaaacggacgtgcatccgggctacctaaatatccgcacacgcggcgagttaccgacacacgggaggcgtcatggttaccacatttcgggcaagtgaagcctttgctggtgcactcgaactcaccggtaaagccacactcgtagcactcatcaatcggtgtattggtgccgtaatacggtacatgctgatagctgtaatcccagacatcttccagcgccttcaggttgtgctgaatgtttggatactcgccgtagcaaatgaaaccaccgttcgccagcggcgggtaaggcgcttcaaagtcgatcttgtcgtacgggttcaccttcttctccacatcgaggtggaaactgttggtgtagtaacctttatcggtcacgcccggcaccacgccaaactcagcagtatcgagacggcagaagcgatcgcacaggttttcactcggcgtgctgtagagactgaaaccataacccgtttcttctttccactgatccactgcctgacgcagacgttcaacaatggcgatacctttcgcgcgaagctgctcgttgtcgtaaacatgctcgccgccgaacagcgcgttaatggtttcgtggatgccgatgtaacccagcgaaatagacgcacgaccgtttttgaagatttcagaaacatcatcgtcagcattgagacgcacgccacaagcaccttccatatagaggatcggggccacgcgcgctttcacgccttcgagacgagcgatacgggtcatcagcgccttacgtgccagcaccagacgttcatccagcagcttccagaaggtggcttcatcgccttttgcttccagagcaatacgcggcaggttcaggctgatcacgccgaggttgttacgaccatcgtggatctgctcgccgttttcattttcccacacgccgaggaagctgcggcagcccatcggagttttaaacgaaccggtgactttcactacctgatcgtagttcaggatatccggatacatgcgcttgcttgcgcactccagcgccagctgtttgatgtcgtagttcggatcgccttttttatggttcaggccatcgcgaatcgcaaacaccagtttcgggaacaccgcagttttacggtttttaccgaggcctgcgatacggttacgcaggatcgattcctgaatcaggcgcgattcccagctggtgcccaggccaaaaccaaaggttacaaacggcgtctgaccgttggcggtgtgcagggtgtttacttcgtactccagtgactggaaggcatcgtagcactctttgatggttcgagagttagcgtagccttcggcgtccgggatgttccactcttctgcggtcttgcgatgtttgttgtagctggcagtgacaaacggtgccagcacttcatcgatacggttaatggtggtgccgccataaatatggctggcaacctgagcaataatctgcgcagttaccgcggttgccgtagagatcgacttcggcggttcaatctcggcgttccccattttaaagccctgggtcagcatgcctttcaggtcgatcaacatgcagttgaacatcgggaagaacggtgagtaatcgagatcgtgatagtgaatatcgccacgctcatgtgcctgcaccacgtcacgcggcagcaggtgctgacgtgcatagtgtttagccacgatcccggccagcaggtcgcgctgggttggaatcaccttgctgtctttgttggcgttttcgttgagtaacgaggcgttggtctgctcgaccagaccacggatctcctggttcaggcgaccgcgtttttcacgttcaatgtcgcgatcgtgacggtactcgatgtaagcacgagccagttgtttgtatggacctgacatcagctgattttcaactgcggtctggatctcattgatatccacctggttgcggccctgcatctgctcgctgacaaccgcggcaacagtggcgcaataatcggcatcatcgacttccgctgctttagctgcacgcagaatcgcttctttgatgcgctctgatttaaacggcactttgcagccgtctcgtttcatcacatgcggtgtcatgatcgctccatatttttaagaacaggttatccacagaaattgggaaaggcgttttccggttttttcgtttcgttttccggtgctttccgcaatcgccatccgcttatccacaacgccgcacctttttcgtggggagctgtagtagcaattatagtcgattaatacaacatattgggttgggacgcattttaaagtctatatatagtgctttgcatcaaggatgtttgagctttttttgatgtagctcaaagtaaaaagcagagcgtacggatgacgggcgctacagcgatatgtaaattttttaatgaatttgctggttgaaaaatcaacaaaaacaacatactgacagacaaaaccccggaatgaccggcattaccggggcttagggaagatttacttctgtaaccaccagacagcctcaaaaggccgtaaattcatggcacagggttgtggtgaggcttcttcgtagttatgcatcacaagctgccagttgccgcgcatttgccctgcctgccagggttggatctcacggctaaggttggcaatgaccagcaaggtttgccccttccattcacggcgatagcaccacaatacagggctgtttggcagcagatcctggtaattgccccatgtcaggatggcttcctgcttacgcagtgcgattaacttttggtaggtgtaaaacaccgaggaatcatcggccagcgcggcttctacgttgatttgttgatagttatcgcccaggccaatccacggttcgccagccgtaaacccggcattatcgccgttgctccattgcatgggcgtgcgactgttgtcacgggatttactggcgaggattgccaataactcgtcggcatcacgcccatcgttgcgcagctcggcaaacatattgaggctctctacgtcgcgatagtcagtaatgcgcgtgaaatgcgggttggtcatgccaatctcttcgccctggtagatatacggcgttccctgcatgccatgcagcaccatcgccagcatttttgccgcaggcacgcggtattcaccttcatcaccaaagcgagaaacaatgcgcggctgatcgtggttacaccagaacaaggcattccatgctacgttgtgcattccttgttgccagtggcggaacaatgttttcaacgccacaaagtcaggtttagccagcgtccatttttcaccaccgggataatcgaccttcaggtgatgaaaattaaaggtcatcgacaattcactgcctgtcagagccgcgtatcgctggcaatgctcaaggctggtggaggacatttcacctacggtcattaacccgcgtggcgtaaacacatcgcggttcatctcgtgcaaaaactcgtgtgctcgtggcccgtcggtgtagaagcgacgcccgtcgccgtccaggtcttcagggaaacgcgggtctttggagatcagattcaccacatccaggcgcaacccgtcgaccccacgatcggcccagaactcacagacttttttcagctctgcgcgtaccgctggattctcccagttgagatccgcctgttctggtgcaaagagatgcaaatagtactgttcgctttccgcatgccagcgccacgcactaccgccaaattttgaacgccagttgttcggtggcgtttctggttctccatcgcgccagatataaaactggcggtaagggctttctttgttcagcgcctcgcgaaaccaggcatgttgggtagaggtatggttaaacaccatatcgagaatgatacgaatcccgcgcgattttgcctgcgtcaccagttcgtcaaaatcgtccagcgtgccgtaggtgggatcaatcgccgtatagttcgctacgtcgtaaccgttatcgacctggggagagacataaaagggggttagccagatggcatcaacgcccagtttatgcagatagtccaggtgttggataacgccacgtaaatcgccggtaccgctacccgtggtgtcctgaaaactctttggataaatctggtagataacgccgttttgccaccagtggggaagatgagtcattacgttattcctgcgaatgcgagggggcgcaattgcgccccgaagaaaattaaacaatgtccagcgtgcccaggcggtatttccgctgatagataaacgaggtgagtacaatcgggatgatgatggcgatagccattgccagcgcaaacacctgccagtagctcggttgaatcgagagaattcccggcaggccgcctacgccgatgccattcgccataacgccgttcaggccgcatagcaatcctgccagaccagaaccaatcatcgcgcacagcatcgggaagcgatatttcaggttgatgccgtacattgcaggctcagtgaccccaagccaggcggagatagcggcaggcacggagatctcgcgttcattgtgcttgcggctggaaatgataatgcctatcacggcggagccctgagcgatattcgacagcgcaatcagcggccacactggcgtaccacccatgctttgaatcatctgcaaatcaatagcaagcgtggtctggtgtacaccggtgatcaccagcggggcgtacaggaagccaaacaatgctgcgccaatcggagcaaagctgccggtcatcaggtgacgtaccgcaaaggcaacgccatcgccaatcatgcgaccaaacggaccaatcagcgcatgggcgaggaacaccgcgaggatcagcgaacagacgggtaccaccaccagatagaggtaatccggcacgatgcgtttaaggcgagtttcaataacgcccagcgccagtccggctaacagtgccgggatcacctgcgcctgatagcctactttggcgatgctgaacatgccaaagtcccacacttccggcagctgctgcccgagcagataagcgttcatcagctgtggagaaaccagtgtcacgccaagcacgataccaaggatcggcgtgccgcccatttttttcaccgctgaccagcaaataccgaccggcaggtagaagaagatcgcttcaccgatcaaccacagaaaatcgtagatcgtttgcagggaagggtacatttgcgccagcgtctgaccgttgctcatgggcaaatcgccgatcacattgcgaaaaccgaggatcaaaccgccgctaatcaacgcgggcagcaacgggaagaagatcaccgcgaaatgagagatcaactgctcatgccatttcatattatgccgggcggctttttttacctgctctttatcaacctgcgcctgtccggttgacgcaatcagtgcttgatagtaatcacccacgttggtgccaatcaccacctgaaattgcccggcattggtgaaacagcctttcaccatagggagttgctcaatttctttcggtctggcattggccggttggttgaggacaaagcgtaggcgagtaatacagtggctcaccgtcgcaatattgccgcgcccgccgaccagttcaatcaaccgatcgatatccgtttggtttattttgctcatcataaagccccatggcagatgacatttttggttggctgcagaatatattgcgcggaaaaatttaaaaacgggaacgttcccgaaacgcagcgaagatcacaatttatcgttcaggaaacgatcaggacagggtggcggggatgatgatttgttgcggttcgctgcgcccggttacctgcgcgatcaactggcaagccgcctggcgtccagcttcggcgtaaccgggatctacggttacgatctccggatggaggaatttcattaacggcgtattaccgacgctcgccagttgcaaggtgtcgatgcgttgctcttgcaggtatttacttgcgccaagtgccagcgtgtcggttgcgcacagtaaggcggtagtttcaggcgtaatcacttttgcaacgttctcatagccttgcttcatagcaagccctggcagggcggcaacgggatgcagtttatgcgctttgcagaacgccaggtaggcttcgtgacgtcgcttaccggttgtcacgtcactgtgcggcacgccgagataactgatattacgatgcccctggtcatacagccgttgcatcaggattttgattgccccttcgtcgtcataacagaccgaagcaaagccttttgcgtcacgcgccagcagaaccagcgatgactgccagtgggctaacatttcttctgttatgccagtaaaaccgaacagcactacgccgtcgatattacgccgtttcagcactcccaaatgttcggcaactaattgcggggaaaactgactttccatcatgattgggtcgtaaccttgttcatagaacgctggcagcatggtttgaacggcgagattttctgacaacgaatccagacgggtaacaatgatggcgaccactttatcgctttgcccacgcatagcgcgcgcagagcgggaaggggaaaatccatgctgattcatcactgcttcaacacgctcgcgggtgagctggctcacgccgctttcgttattcagcacccgggaaactgtagatttccccacgccgcttaagcgcgcgatatctttgatggtcagccgattttgcatcctgttgtcctgtaacgtgttgtttaattatttgagcctaacgttacccgtgcattcagcaatgggtaaagtctggtttatcgttggtttagttgtcagcaggtattatatcgccatagatgctacgaatattattggattctccttattatttgcggcgcttttttcacttaccggaggttatatggaacctgatcccacgcctctccctcgacggagattaaaacttttccggtaagcccgtcttttcacggcgttaccggatgcgtaaggccgtgacgttttaacgtccctgctcagctttattaccttcaggtaaggcttcgccacgcctgaagacatttctgtactgtttcagacagtgcggagggactccttatgtttaaagaaatttttacccggctcattcgccatttaccttcccgtctggttcatcgtgatccattgcctggcgcgcagcagacagtgaatacggtggtcccgccgtccttaagtgcgcattgcctgaaaatggcggtgatgcccgaagaagaattgtggaaaacgttcgacacccatccggaagggttaaatcaggcggaagtggaatctgcccgcgaacaacatggtgaaaataaattacccgcacaacaaccgtcgccgtggtgggtacatttatgggtctgctatcgcaacccctttaatattttactcaccattctcggcgctatttcttacgccacggaagatttatttgctgcgggcgttatcgcgctaatggtcgctatttctacgttgctgaactttattcaggaagcacgttccactaaagcggcagatgccctgaaagcgatggtcagcaatactgcgacggtgctgcgcgtaattaacgacaaaggcgaaaatggctggctggagatcccgatcgaccagctggtgcccggcgatattataaaactggcggcgggagatatgatcccggcagatttacgtatcttgcaggcgcgggatctgttcgtcgctcaggcgtcgttaaccggtgagtctctgcccgtagaaaaagccgctaccactcgccagccggagcacagcaatccgctggagtgcgacacgctgtgttttatgggcaccaccgtggtgagcggcacggcacaagcaatggtgattgctacaggtgccaatacctggtttggtcaactggcggggcgtgttagtgagcaggaaagcgagccgaatgcctttcagcaagggatcagccgcgtcagtatgctgctgattcgctttatgctggtgatggcaccggtggtgctgttaatcaatggttacaccaaaggcgactggtgggaagcggcgctgtttgcgctttcggtcgcggtaggcctaacgccggaaatgttgccgatgattgttacctcgacgctggcgcgcggcgcagtaaagctgtcgaaacagaaagtgatcgtcaaacatctggatgctattcagaactttggcgcaatggatattctgtgcactgataaaaccggcaccctgacgcaggataaaattgtgctggagaatcataccgatatctccggtaaaaccagcgaacgcgtgctgcatagcgcgtggttgaacagtcattatcagaccggacttaaaaacctgctcgatacagcggtgctcgaaggtacggatgaagagtcagcgcgctcgctggccagtcgttggcaaaaaattgatgagattccgtttgatttcgagcgtcgccggatgtcggtggtagtggcagaaaataccgagcaccatcagctggtttgcaaaggtgcattgcaggaaatcctcaatgtgtgttcgcaggtgcgtcacaatggcgagattgtgccgctcgatgacatcatgctgcgtaagattaagcgggttactgatacgctgaatcgtcaggggctgcgcgtggttgcggtggcgacgaaatacctgccagcgcgtgaaggagattaccagcgggcggatgaatccgacctgatcctcgaaggatatattgcttttcttgatccgccaaaagagacaaccgctccggcactgaaggcattaaaagcgagtggaattaccgtaaaaatccttactggcgacagtgagttagttgcagcgaaagtgtgccatgaagtggggctggacgcgggagaggtggtcattggtagtgatattgaaacgctatctgacgacgaactggcaaatcttgcacagcgtaccacgctgtttgcccgcctgacgccgatgcataaagaacgcattgtgaccttactgaagcgcgaagggcatgtggttggctttatgggcgatggtattaatgatgcgcccgccttacgcgctgcggatatcggcatttctgtggacggcgcggtagatattgcccgtgaagcggctgatatcatcctgctggaaaaaagcctgatggtgctggaagagggggttattgagggacgtcgcactttcgccaacatgctgaaatacatcaaaatgacggcgagctctaacttcggtaatgtgttcagcgtgctggtagcgagtgctttcttgcccttcctgccgatgttgccgttacacttgcttattcagaacctgctgtacgatgtgtcacaggtggcgatcccgtttgataacgtcgacgacgagcaaattcaaaagccgcagcgttggaatccggcggatctggggcgctttatgatcttcttcggaccgatcagctcgatcttcgatattttgacgttttgcctgatgtggtgggtattccatgccaacacgccggaaacgcaaacgctgttccagtcgggatggtttgtggtgggcttactgtcgcaaacgctgattgtgcatatgatccgcacccgccgtgtgccgtttattcagagctgtgcatcgtggccgttaatgatcatgaccgtgatcgtgatgattgtcgggatcgcattgccgttttcaccgctggccagttatctgcaattacaggcgctgccgttaagctatttcccgtggctggttgcgattctggcagggtatatgacattaacccagttggtgaaagggttctatagccgtcgttacggctggcaataaagaataaactgggcacgatagccccgattcagattgtagacaaagtgagttttgttcatgccggatgcggcgtaaatgccttatccggccaacaaattcaataaattgcaggaatcacgtaggcctgataagcgtagcgcatcaggcgattttgcgtttgtcatcagacttaatccgggcatgatagcccggatttccatcaagattagcgacgaacagcgatcgcttcgatctcaatcttcacgtctttcggcagacgggcaacttcaacgcaagaacgtgccgggaaggtggcgttgtgttcggtgaagaaggcttcgtaagtggcgtttacggttgcgaagtcgttcagatcttttacaaacacggtagttttaacgatgtcgcccactttcaggccagcggcttcgacgatcgcttttacgttatccagcgactgacgtgcctgtgcagcgacgtctgccggtacttcgcccgttttcggatttaccgggatctgaccggaggtgatgatcatattgcccagatcaacgccctgtacgtaaggaccgatagctgccggtgcattttccgtcgcgatagttttgctcatgatttctcctttattacagcggtaaaaagtctggctcattatagggagccagacttttattaccaaccgcaattaattggccagcaccacattatgggaaaactctttttcacagtatttgcatttgagcgcgatatcattggcgcgttttcgcacggcaaagctggatgaaaccggttcggcatggctgatacagttgctgttcgggcagaccagcacattgtcgatgcgctccggcagacttgggcgcgatttacccaccacttcatagttgtcgatacggttaaccgtggcttgcggcgcatacaatgccagttgatctacttgatcttcactcaaaaaggtattttcgattttgatcagatctttgcggcccatctcgccagaaggcaggttcagaccaatggtgatgcgctgatccgtttcggtcagcttgaacagactcaacagcttaaaaccgatctgggcggggatatggtcaattaccgtgccgcgtttaatagcttcaacctgcaatttattatcgtgtgtcatctctatttccccttacagtaccagatcgcgattcagaaccagtgccagtaacgcctggcgagcgaaaatcccgttgcctgcctgctggaagtaccaggcgtgtggcgttttatcaacatccgtcgcaatctcatcaacacgcggcagcggatgcagcactttcatattggctttggcgttgtggagatcgctggcgcgaagaacaaactgcgctttcacgttggcgtactcggacgggtccagacgctctttttgcacgcgggtcatgtacaggatgtctacttccgccatcacttcttcaatagagctgtgcagactccatgcgatccctttttcatcgagcatatccagaatgtattgcggcattgccagcgcgtccggcgcgatgaagtaaaaacggttgccgtcgaacttcgctaacgcctgagtcagggagtgaacggtgcggccatatttcaggtcaccaaccattgcgacgtggagattgtccagacgcccctgggtttcctgaatagtgaataagtccagcaaggtttgcgtcggatgttggttggagccatcaccggcattcagtaccggtacattgccggaaaactcggtggccaggcgcgccgcaccttcctgcggatgacgcatcactatcgcatcgacgtaagtgctgataaccgaaatggtatcggccagcgtttcgccctttttacccagtgatgtattggcgctgtcggagaagcccaccacgctggcccccaggcggtgcatagatgtttcgaaagagaggcgggtacgggtagaggcttcgaagaaacagctggcaatgactttgtgcttcaacagctctggttgcgggtttgctttcagtttcgccgctgtcgccagcaccagattaaggtcatcgcgactaaggtcgtttatggaaatgatatgtttctgatatagcggattagccatcttttatctcctgacgcctgggcaaaaaaaagcccctcgattgaggggctgggaatgggtgatcaacgggaagaaaaacggcaggccagcgtcttttttcagacgcggtaagacaaaatgtcgaacacactgaaccatacatcctcccggcaaattgtccggcattatactcatcgtcagaagcggcgcaagcatttgatgcaatattttgtcagcgcaaacggtttatttgaattaaaagtcaaggtatatgcatttttatttgatgtgattctgcaggggaactgtccttcggtatcaataattgcagacattccctgctttttcctttttcactttcacgcaatcagatatgcattttattccattcatccgacttatagggcggagtgtgaaagcgaacggctaacactattgcttactgctcagggatgcgcgctatcactttaatttcaaaatcaaagcctgccagccatgtaacacccaccgccgtccagtttggataaggtggggcgctaaatatttcatttttcaccgtcatgatgtcttcaaattggttttctggatcggtatggaagctcgtaacatcaatgatatcgtcaaaagtgcatcccgcagctgccagggtcgcatgcaaattatcaaatgccagtctgacttgttgctgaaaatcgggttctggtgttccgtcctctcgacttcctacttgcccggaaacaaacagcaaatcgccggaacgaatagccgcagaataacgatgctcagcatatagtgaatgtcggccagcagggaaaacagcggttctttctaccatttggttatcctcaagatttacgacatgaacagaagatttctctttaccgggagccgcttttagcggacgacgtgagtaaacaaaacccagacatcatggataatggctgggcttaattgagcgtagtcggttatgcgccaaacgcgccatcaatggtatgcatcgcgccggtaacaaaactggcttctggccctgctaaccatgcgaccataccagcgacctcttccggttgcccatgtcttttgatagccatcaaactatgcaacatatcgcgcattggcccgttggcgggattagcgtcggtatcaattggccctggctggacgacgttaatggtgatcccacgcggtccaaaatcacgggccagcccgcgcgccatgccttgcagggcagatttgctggcggcataagcagccatgcctgcaacaggcatacgatcgccattcacggagccgatgattaagatgcgcccgccttcgggcatctgccgggcggcttcaacagaggcatgataaggagcatgaatattgattttgaaaaggcgatcaatatcgtcggcatttaattccagggcctcgccaaagacgccaatacctgcatttaccaccaggatatccaatgcgccgctcttacgaacgacatcaatgacagcgtctctgtcagcactatctgtgaatactgctgtcgctccagtctcttgtgccaggcgtttagcggcatctttcgaccccgcataggtgaatcgtacattggccccatcggtgacgaaacgacgtacgatagcggcaccgataccacgactgccaccgaggatgagaactgtcttacctgtaaaagcgcccataaggactccttgatttattatgtaacatgcattacaaaactgttttaactttctgtcaacaggttttgtaatggtcactaaaaaacaatctcgcgttccaggtcgtcccagacgtttcgctcctgagcaggcaatctctgcggcaaaagtgctttttcaccaaaaaggtttcgatgctgtcagtgttgctgaagttactgattatcttggtattaaccccccgagcctctacgcggcttttggcagtaaagctgggttatttagccgtgtactcaatgaatacgtcggtacggaagctattccgcttgccgatattcttcgtgatgatcgtccggtaggcgagtgcctggttgaggtattaaaagaagcggcgcgcagatatagccaaaacggcggctgcgctggctgtatggttcttgaaggtattcatagtcatgatccacaagcgcgtgatattgccgttcaatattatcacgccgcagaaacgaccatttatgactacatcgccaggcggcatccacaacgcgcacaatgtgtgactgattttatgagtaccgtgatgtctgggctttctgcgaaggcacgagaggggcactctatagaacaactctgtgcaacagctgcaatggcgggggaagcgataaaaactattcttgaggagtgatgcgggccttgacccgaaaggcgggaaagcgcctgccgataagttgtgataagacaataattcacgcgttaaggctagcggaattgattatcttttcgtataacgatagaaatgaaacgttgttttaattaaggagtggaaaagatgatcatcggaaatattcataatcttcagccgtggctaccccaggagttacgccaggcgattgagcatatcaaagcacacgttacggcagaaacgccaaagggcaagcacgatatcgaaggcaatcgactgttttatcttatctcggaagatatgaccgagccgtacgaagctcgccgtgcggagtaccatgcccgctatcttgacattcagattgtgttaaaaggtcaggaaggcatgaccttcagcacgcaacctgcaggcgcgccggataccgactggttagctgataaagacatcgcatttttgccggaaggcgttgatgagaaaacagttattctaaatgaaggtgattttgttgtgttttatccgggggaagtgcataaaccgctgtgcgcagtgggcgcgccagcccaggttcgcaaagcagtagtgaagatgctgatggcgtgatgacttttcgccgtaaataactcaaggtttacggcgagtttgtgaaaagagcgttttttgatatttttttgtgagtaaaatttgtaatgcttagacgttcttattcactcaaggagttcgtcatgagcaaaatatcagatttaaattattctcaacacattacattagccgacaattttaaacaaaaaagtgaagttttaaatacctggcgtgttggaatgaatgattttgcccgtattgccggggggcaggataacagaaggaatattctttctcctggagcatttttagagtttttggcaaagatatttaccctgggttatgtggattttagcaaacgctccaacgaagcgggtagaaatatgatggctcatattaagtcctcatcttattctaaagatactaatggcaatgaaaaaatgaagttttacatgaataatcctgtaggggaacgagcggattcacccaaggtgattatagaaatttcactttccactatcactactatggggactcgtcaaggacatacagccattatatttccacaacctgatggttcgactaaccgttatgaagggaagtcctttgaaagaaaagatgagagttcattacacctgattactaacaaggttctggcgtgttaccaaagtgaagctaacaagaaaatagcgcgtctattaaataataatcaggagttaaataatctacagaaattaaataatctacagaagttaaataatctactgaagttaaataatatacaggggttaaataatcctcaggagttaaataatccgcagaatttaaatgattctcaggagttaaataactcgcaggaattaaatagtccacaggagttaaatgatccgcaggagttaaataattctcaggacttaaataactctaaggtgagttgtacagtttcagttgattctacgattacgggtttattaaaagaaccattgaataatgcattattagcaataaggaacgaacatctgctattaatgcctcatgtatgtgatgaatcgatttcatacttactgggcgaaaaaggtatacttgaagaaatagataagctctacgcattaaatgatcacggaattgataatgacaaagtaggtaacaatgaaattaatgacatcaaagttaacctgtctcatattcttattgattccttagatgatgcaaaggttaaccttacaccggtcatcgattcgattctggagactttttcaaaatccccatatattaatgatgtaagaatactggattggtgttttaataaaagcatgcaatattttgatgatactaaaaagataaagcatgcatgctccgtaataaatcatattaatcttcgcagcgatcagtctaaaatagctgagacattatttttcaatctcgataaagaaccctataaaaatagccctgaattacaggggttgatttggaataagttggttgtatatgtcaatgaatttaacttaagtaatcgagaaaaaacaaatttaatacaaaggctatttgataatgttgagtctatatttaatgaagtacctgtcagcattttagtgaatgatatttttatgaatgatttctttatgaaaaatcctgagatgattaattggtacttccctcagttacttaagagttatgagggtgaaaagatttattttgataatttaaaatatgatttaaatgataatgataaggaatctaataaagaaattttgaagaatcaaccagataatgttatcaaagaaaaactgaataatgaatacaaacttagatttagaatgatgcaaactatcttgcaatcgagagttaatgtattaccatatattaatgaacagcgtttaaataaactaaatccaccggaaaatttacgtatagcaatagaacactttgggtggaagaatagacctatcactgcataaaataatgtgatgccgggatggtttgtatttcccggcatctttatagcgatagcaattatttactgagcgtcgcgaccatcaccgctttgatagtatgcatacggttttccgcctgatcaaaaacaatgctggcggcagattcgaagacctcatcagtgacttccataccgccatgtaggccaaattcttccgccattttcttgccaagcgtcgtttggtcgtcatgaaacgcgggcaggcagtggaggaatttgacctccgggttaccggtcaactgcatcatcttgctgttcacctgatattcacgcagcaatgcaatccgttccgcccatttctcttttgcttcccccatcgacacccacacatcggtatagataaagtcagcaccttcaactcccttcgcgacatcttcagtcagcgtaatattcccaccattttgctgtgccagggcgcggcattccgtaaccagcgcagcttccggccagcacgcttgtggcgcgaccagacgcaaatccagaccggtaagcgccgcagcttcgagcatcgaattgcccatgttgttacgcgcgtcacctgcatagaccagcgtcatttcgttgaacgctttgccgggcaaatgctcctgcatggtgagaagatccgccagcagctgcgtgggatggaactcattggtcaggccattccataccggcacgctagcgtattccgccagtgtttcgacaatctcctgaccatagccgcgatactgaataccgtcatacatgcgaccaagcacgcgggcagtgtctttaatcgactctttatgaccaatctggctgccgcttgggccgagataagtaacgcgagcaccctggtcatatgcggcaacttcgaaagagcatcgggtacgagtcgagtctttttcgaagatgagcgcgatgtttttaccagtgagtttggcttcttctttaccgcttttcttatcggctttcagcttcgcggctaactgcagcaggctgttgagttcagctggcgtgaaatcgagtaatttcaggaaatgcttatgataaaacccggacatagatccctcctgtggctaacgcctcaatgaattaaaattcaatttatatggatgattattcatttgcaagtctaaagcataaatctttgtcacaaaggtggaggcaatgtcagtggtgtgtgacaataagagtatcggcaggacattaagaggaatgagccatggcaaacccggaacaactggaagaacagcgtgaagaaacacgtttgattattgaagaattactggaagatggcagcgatccggacgcgctgtacaccatcgaacaccatctttccgcagacgatctggaaaccctggaaaaagcagcagttgaagcgtttaaactcggttacgaagtgaccgatccagaagagctggaagttgaagatggtgatatcgtgatttgctgcgacatcctcagcgagtgcgcgttgaatgccgatctgatcgatgcccaggttgaacaactgatgacgctggcagagaaatttgacgttgagtacgacggatggggcacttactttgaagatcctaacggcgaagatggcgacgatgaagattttgtcgatgaagacgatgacggagttcgccactaattaagcgtagcgcatcaggcccaggtagttcctgcaacctggtgaatttgtagcccggataaggcattcatgtcacatccggcataaacaaaacgtacgttgttaatgttcgaatgcccgcgagttgaacacgcgggcatttttttagagttcgcgcaacatccgcacttcacaatcgacatggcccgtgcagccaagcgcatagtcgatatgctcaaagcccaaatgctcataaagcgcaatggcttcctttaaaaaagcggtcgtttccagatagcagcgtttgaaacccatctctcgcgcctgctccatcgccattaaggccagtttttttgccagccctttgccgcggatagccggaagaaaatacatcttttgcagttcgcaaatatccgactcactcccggttaatggcgctatcccaccgccgccgaccacttcaccctcgtactcaacgacccaatatgcatggccaggctgactatatacttgatacagctcgtcaagattcggatcggcgacggtgtagcctttatcagcggtaagaccgtattcggcggatacctgacgaatgacgcgggcgatagcaggattatcctgcagcgtcaggcgacgcattacaggtgattgcggcgcaatgttattcatagtttaacccaataaaaataaagtaattatacatttgtttaataccactctcttcttacgtacgcaagcgacttataaagtaataaagtttttgccagcctattactgataagagtattgtaacgtggcagaacattttactgtctgtatatataagttatatcaatggattttttaattcagggaatttttatggctcaagttattaatgaaatggatgttccgtcccattcgtttgtttttcatggtacaggtgagagatattttcttatttgtgtggtgaatgtgttgttaacgattataacgctaggtatctatttaccatgggcattaatgaaatgtaagcgttatctttatgctaatatggaagttaacggacaacgattttcttatggaattaccggtgggaatgtttttgttagttgtcttttttttgtttttttctatttcgcaatcttaatgacagtgtcagcagatatgccgcttgttggttgtgttttgactttgttactgttggttttgcttatatttatggcagcaaaaggactgcgtcatcaggccttaatgaccagtctcaacggcgtaagatttagttttaattgctctatgaaagggttctggtgggtgacctttttcttgccgattttaatggccattgggatggggactgttttctttatctcgacaaagatgctacctgccaatagttcaagtagtgttattatatccatggttctgatggcaatagttggtattgtttccattggtatttttaatggtactttatatagtctggtaatgagttttctctggagtaataccagtttcggtatacatcgtttcaaggtgaaattagatactacgtattgtataaaatatgccattctcgcatttttagctttattgccttttctcgctgttgctggttatattatcttcgatcaaatattaaatgcgtatgatagttctgtatatgcaaatgatgacattgagaatttacagcaatttatggaaatgcaacgtaaaatgataatcgcgcagttaatctattattttgggattgctgttagcacaagttatttaacggtgtctttgcgaaaccattttatgagcaacctgtcactgaatgatgggcgtattcgttttcgcttaactttaacgtaccacggtatgctttatcgcatgtgtgcgttggtggtgatatccgggattacgggcggtctggcttatccactgctgaaaatatggatgattgactggcaggcaaaaaatacgtatttgctgggcgatttggatgaccttcctttaatcaataaagaagaacaaccagataaaggcttcttagccagtatttcacggggagttatgccttctttaccatttctgtaagagataaaaaaggccggagcatgctccggccttcgttttcatcactgtgttttgattacagcgcggcgataacagcctgctgttcaatcagtttcgctttcgcttccgcatagccttccagcttctcacgctctttcgcgatgaccgcttccggtgcgcgggcgacaaagccttcgttcgccagtttgttctcgatacggctgatttcaccttcaatcttcgccacttctttcgccagacgcgccagctcatcttctttgttgatgaggccagccatcgggatcagcagctctgcaccgtcgatgatcttcgtaacggaaaccggacctttgtcatcggcaggcagcacggtgatactttccagacgcgccagggtttgcaggaagccacggttttcatttacgcgacgttctgcatccgcgctgcaaccacgcagcagcagctccagcggtttgcccggcgcgatgttcatttctgcacggatgttacgtaccgcaacgatcgcctgtttcagccattcggtgtcggccagtgcggcttcatcaacctgagatgcatcgtactgcgggaacggctgcagcatgatggtgtcggcagtgataccgcaaagtactttcacacgctgccagatggtttcggtgatgaacggaatgatcggatgcgcgaggcgcagcagaccttccagtacagtcaccagcgtatggcgagtaccgcgcagttctgcttcggtgccaccgttcattaccggcttggtcagctcgagataccagtcacagaactggttccaggtgaactcatacagaatgcctgcggcgatatcgaagcggaagctgtccagcgcttcgcggtacgctttgatggtctggttgaactccgccagaatccagcggtccgccagcgacagcgtcatttcgccgccgttgaagccgcaatcctgaccttctgtgttcatcagcacaaagcggctggcgttccacagcttgttacagaagttacggtaaccttccagacgcttcatatcccagttgatgtcacgaccggtagacgccagcgccgccagggtgaagcgcagcgcgtcagtaccgtgcggctcaataccgttcgggaactgcttctcggtgcgcttacggattttgtccgccagctgcggctgcatcatattgccggtacgtttttccagcagttctggcagcgaaataccgtcaaccatatccagtgggtcgataacgttacccttggatttggacatcttctggccttcgtcatcacgaatcaggccggtcatgtaaacggtgtggaacggcacctgcggtttgccattttcatctttgatgaagtgcatggtcatcatgatcatgcgggcaatccagaagaaaatgatgtcgaaaccagataccatcacgctggttgggtggaactgacgcagggcgtcggtattttccggccagccaagggtagagaaggtccacagcgcagaagagaaccaggtatcgagaacgtcttcgtcctgacgcaggacaacatcagcaccgaggttattttctttacgcacttcgtcttcgttgcggccaacataaacgttacccgcttcgtcataccatgccgggatacggtgaccccaccacaactgacgagagatacaccagtcctgaatatcgcgcatccaggagaagtacatgttttcgtactgcttcggtacgaactgaatgtcgccgttctcaaccgcttcaaccgccggtttcgccaggacatcggcacgcacgtaccactggtcggtcagcattggttcgataactacgccgccacggtcgccgtaaggaacggtcaggtcgtgcggtttaatttcttccagcaggccaagcgcgtcaactgcggcaacgactgctttacgtgcagcaaaacgctccagtttctggaactctgcagggatttcgctggaataaacgtcagattcgttacctttggtatcgaacacctgggcgctttcacggatatcgccgtcaaaggtcaggatgttgatcatcggcagggcgtgacgtttacccacttcatagtcgttaaagtcgtgcgccggagtgattttcacgcagccggtgcctttttccatgtcggcgtgttcgtcgccaacgatcggaatacgacggttaaccagcggcagaatgacatatttgccaatcagatctttgtaacgcggatcttccgggttaacggctacgccagtatcgcccagcagggtttctggacgggtagtcgcgaccaccagataatctttaccgtctgcggttttcgcaccgtcagccagcggatagcggatgtgccacatcgaacctttcgattcgcggttttcgacttccaggtcagagatagcggtgcgcagtttcggatcccagtttaccaggcgtttgccacggtaaatcaggtcttctttatacagacgaacgaaaacttctttcaccgcattggacaggccttcgtccatggtgaagcgttcacgctcccagtcgacggagttgccgagacggcgcatctgacgggtaatggtgccgccagattccgctttccattcccagattttgtcgatgaaagcttcgcggccgtagtcgtgacgggttttaccttcttctgcggcaatcttgcgctcaacgaccatctgggtagcgatcccggcgtggtcagtaccgacctgccacagggtgtttttgccctgcatgcgctgatagcggatcatggtatccatgatggtttgctggaaggcgtgacccatatgcaaactgccggtgacgttcggcggcgggatcatgatgcagaaactttcctggctttcatcgccattaggcttaaagtagccctgcttttcccagtgctcgtaaagcggctgttcgatatcttgtgggttatatgtcttttccattatttccaggttgccgtattcaggttgaaaccagccacgcggtaggctttatagcgttcgcgcgccagttgtttcagagaatcttcataaggaacgaagtctaccacttctgtgaaagcggtggcaaaatctgcaaagcttgttcgcagactaatcaatatatcgcgccggctgctgctacgcttttgcggccaggcgatctccaccggtgcaccgccgcgcggtccttctcccgctaaattatgcggaacaaagctttctgccggacgcgcccacagggcttcatccagccggtaagcctgcttttcatcttcacaggcgatgagcacgcgcttaccgctgcgccaacgttctgcggcaatttcacacaccagttgctcaacggcgcttaagccatcgacggtggtgtcattgtccagaaggtagaacgtcgcgtttttcataaatggggcttcttgtggtggatttaaatacgcatcaggtatacaccgcagcgcctgatgcgacgctgttgtgtcttatcaggcctacgagttcagtgctgtgtaggtcggataaggcgttcacgccgcatccggcaataacagccttgcctgacgcaattactcttcgccgttaaacccagcgcggtttaacaggaactgtgccagcaacgctaccggacgaccggtggcgccttttgctttaccagaacgccaggcggtaccggcgatatccaggtgcgcccagttgtacttacgggtaaagcgtgacaggaagcaacctgcggtaatcgccccaccaggacgaccgccaatgttcgccatatcggcaaaattggactccagttgttcctgatactcgtcacccagcggtaagcgccatgcgcggtcaccggattgttcagacgcggcaatcagttcatgggccagcggattatggttcgccatcagaccagtaatatgatgacccagcgcgatcacgcaggcaccggtcagcgtcgccacgtcaatcaccgcttccggctcaaaacgctcaacgtaagttaacacgtcgcacagtaccaggcggccttcagcgtcggtgttcagcacttcaacggtttgaccggacatggtggttaacacatcgcccggacgataggctcgtccgccaggcatgttttcgcagcctgccaacacgccgataacgttaatcggcagttgtagctccgcgaccatccgcatcacgccgtaaaccgctgccgcaccgcacatatcgtacttcatctcatccatgccttctgaaggcttgatcgagataccgccggagtcgaaggttaaacctttacccaccagcacgattgggcgtgcatcttccgacgcgttgcctttgtactcaatcaccgacatcagcgattcgttttgcgaaccctgaccgaccgccagataggaatgcatccccagctctttcatctgctgttcgccgataacgcgggtgatgacattcttgctgtagctgtcagccagctggcgcgcttgtgaagcgaggtaagcggcgttacagatattcggcggcatattgccgagatcttttgctgctttaatcccggcggcaatcgccagaccgtgctggatcgcgcgctcaccgctggtcagttcacggcgggtcggcacgttgaacaccatcttacgcagcggacgacgcggttcgctcttgttcgttttcagctgatcgaaactgtagagcgtctcttttgccgtctcgacagcctgacgcactttccagtagttgttacggcctttaacgtgcagctcagtcagaaagcagaccgcttccattgagccagtatcattcagcgtattaatggttttctgaataacctgcttgtactgacgctcatccagctcacgttctttgccgcaaccaataaggagaattcgctcggaaagtacattcggaacatggtgcagcaacaatgtctgccccggttttccttccagttcgccccgacgtagcagggcgctgatgtacccatcgctgattttatcgagctgttctgcaatcggagaaaggcgacgtggttcgaagacgcccacgacgatgcaggcactccgctgtttctccgggctaccgctttttacactaaactccatgcactacgctcctgaatcttaaagacaacggcggtggctacagatagaattgcaagctttcgtaactcatgtccgctgttgcgatgacttcgtgttaatcttaacgttattacggcattggcacgtcagaacaaaatctgagaggtgaatccgttgagtataattatcttagcgacgatttcgacgactcaagagaataaatgacgtttaagccatgaaacaagctaaaatcctgcaaaagacgagtttttacgggcgtatttaaagtgataatcataagatatctggtgcgggagacgctcaaaagccagctggcgatactcttcatcttgcttttgatcttcttctgtcaaaagttagtgaggatcctcggcgcagcggttgacggcgatattccggcgaatctggtgctctcccttctcgggttgggcgtgccggaaatggcgcagcttatcctgccattaagcctgttcctcgggctgctgatgacgctgggcaaactgtataccgaaagtgaaattacggtaatgcatgcctgcggcctgagcaaagcggttctggtgaaagcggcaatgatccttgcggtattcacggcaatcgtagcggcggttaacgtgatgtgggcgggaccgtggtcatcgcgtcatcaggatgaagtgttagcagaagcgaaagcgaaccctggcatggcggcgctggcgcaagggcaattccagcaagcgactaatggcagctcggtgctgttcatcgaaagcgttgacggcagcgatttcaaagatgtgttcctcgcgcaaattcgaccaaaaggtaatgcacgtccttctgtggtggtggccgattccggacatttaacccagctgcgcgacggctcccaggtcgtcactctcaaccagggaacgcgcttcgaaggcactgcattgttacgtgatttccgcattacggacttccaggattatcaggcgatcattggtcaccaggcggtggcgctcgacccgaacgataccgaccagatggacatgcgcacattgtggaacactgacaccgatcgtgctcgcgcagaactgaactggcgtatcacgttggtattcaccgtgtttatgatggcacttatggtcgtaccgctgagcgtggttaacccacgtcagggacgcgtactgtcgatgctgccagccatgctgctgtatctacttttcttcctgatccagacctccctgaaatcgaacggcggtaaaggtaagctggacccgacgctgtggatgtggaccgttaacctgatttatctggctttagcgattgttctcaacctttgggacaccgtgccggtccgccgcctgcgcgccagtttttcgcgtaaaggagcggtgtgatgcaaccttttggcgtacttgaccgctatatcggtaaaactattttcaccaccatcatgatgacactgttcatgctggtgtcgctgtcgggcattatcaagtttgtcgatcagctgaaaaaagccgggcaggggagttacgacgcgttaggcgcaggaatgtataccttgctgagcgtgccgaaagatgtgcagatcttcttcccgatggcggctctgcttggggcgttgcttggtcttgggatgctggcgcagcgcagcgaactggtggtgatgcaggcttctggttttacccgtatgcaggtggcgctgtcggtgatgaaaaccgccattccgctggtcttgctgacgatggcgattggcgaatgggtcgcgccgcagggcgagcagatggcgcgtaactaccgtgcgcaggcgatgtacggcggctcgttgctctctacccagcaaggcttatgggcgaaagatggcaacaacttcgtctacattgagcgggttaaaggtgacgaagagttaggtggcatcagcatttatgcctttaacgagaatcgtcgtctgcaatccgtacgctatgccgctactgcgaagtttgacccggaacataaagtctggcgtctgtcgcaggttgatgaatctgatctgaccaatccgaaacagattaccggttcgcagacggtgagcggcacctggaaaaccaacctcacgccggacaaactgggcgtggtggcgctggacccggatgcactctctatcagcggtttgcacaactatgtgaagtatctgaagtcgagcggtcaggatgccggacgttatcagctcaacatgtggagcaaaatcttccagccgctatctgtggcggtgatgatgctgatggcgctgtcgttcatctttggcccactgcgtagcgtaccgatgggcgtgcgtgtggtcaccggtatcagtttcggttttgtcttctacgtactggaccagatcttcggcccgctgacgttggtttatggcatcccgccgatcatcggcgcactgttgccaagcgccagcttcttcttaatcagcctgtggctgttaatgagaaaatcgtaaccgaatgaacgaataaagggagcgaaagctccctttattattgttagcaaagtgtgcttcgttcattcctgaaaaataattaaaattcaatatattgcagtggggtgggcatgataagacgcgccagcgtcgcatcaggcaaagacaaatctcgcctgacttaccttcttctcccccccagcaaactccccaacatcccgcgtacaatctgattcgtcacttggcgagcggcgcttttggccattgtttgcaccacaccatctttcttcccgccgcgtggtccggtagtgccgaacaaaatatccttcaatccaccaagaatgccgtcatccaccgctacctctttccctttcgcgggaggattattttgctgctcggtactggcctgaaagcctttttgcaacatctcataggcggattcccggtccacctcatcctcatatttgccatacaccggagagtgattaatcaagccattacgctcatcttccgtcaccggccccatccgcgaacaaggcgcgatcaccatcgcacgctccaccacagaagggcttcctttcgcatccagaaaagagatcaacgcctcgccggtgcccagttcctgaatcgccttttcggtatcaaacgccggattggcccgcatggtttgcgccgctgccttcactgctttctgatcttttggcgtaaaagcccgcaaagcatgttgaacgcgattaccgagctgcccgagcacattatccggaatatcagacgggttttgcgaaacgaaccagacgcccacgccttttgagcgaataagccttatcacctgctcaatcttatccagcagtacctgcggggcatcgttaaacagcagatgtgcctcgtcgaagaaaaacaccagttttggtttctccagatcgcccgcttccggcaattgttcatacaactctgaaagcatccacagcaggctggcggcgtacagtttcggcatctgataaagtttctcggcgctgaggatattgataacgcctttaccgttggcatcggtgcgcatccagtctttgatatccagcatcggctcaccaaagaagtgtgctgcgccttgctgttccagcgacaacagcccgcgctggatggcaccaaccgatgcgctactgatattaccgtactgattctggaaggatttggcgttatcgccgatgtactgggtaattgcccgcagatctttaaagtcgagcagtaacagcccctgatcgtcagcaatgcggaagatgatattcagcacgccagattgcacatcgttgagattcaacagtcgtgccagcaacagcggccccagatccgaaaccgtcgcccgcaccggatggcctttctcgccaaagatatcccacaccaccaccggattggcatgcggttgccagtcattgacgccgatatttttaagccttgcgagcagtttttccgacaccgttcctgcctgcgcgacgccggtcagatcgcctttcacatcagccataaacaccggcacgccgatttccgacaatgactccgccagtttttgcagcgtaacggttttacccgtccccgttgcgccggtaatcagcccatgacggttagccattcccggcagtaaaaacagttctgtgtccggcgtgcgggcaattaacaggggttcactcatgagatatcctccagtttcctgcctggagtataggcaacgtccggcaaagagaatacgtgtaatgaagagaaaataacctaaagcgtgttgccgtgataaatctgatacccgaggtcaacagtgttgtggttgtgatcgttatttttaattttgctcagcaacatttgggcggccatccgaccaatatcaaaacggggagtaattacgctggcgaggcttgggatcatttgcctgccaatctccagcccatgaaaacccgcaatggaaatttgttctggcacggcgaggtttcgctcgcggcacagcagaagcgcacccatcgcaatatcgtcattggtgcaaaatacaccgtctaaatccgggtttgcgctaagggcatcacgcattaactgcattcctaaatgaatggatgagatggcgcgtggattcatgcgtaatggggaaagattatgcagcatcatcgcatcgcaatacccctgataacgctgttcatcgcgggtgtcatctttggaaccgagatacagaattttgtgcctgactcgcttctccagcatggtacacaccatgtcaaaagcggcctgccgattatcaaaaccgacctccatatccagccgttctccctgtacatccatcaattccacgaccggaatggtggctgaacgcagaaatttcaccgtcctgatggtgtgatatttttccgaaagtataatcccgtcaatgttataagagagcaggttaatcaccgactcttcttcggaatcgcgatcgtaattgtaattagcaataagggtctgataattatgctcagaggtgacggattctattcccgcgagaatgtcagcgaagagttgattttgaaatgacggaatcaagataccgagggtataactttgtgcattcaacaacatgccgggagcgcgattagggatataattgatctcttccataattttggcgatgcgctcgcctgtttcctttgccacctttttcggcgagcggatataacgactcacggtcatttttgttacgccagccagcgtagcgatatcctgtaaagaaattctgtgattgcgcataacttctcccaacgtcgggggaatcttcaatcttcccccgaaactacatcacaatattttattctttcagtgcaatacggcgttaatggctaacacgcccagcaaacccataatagaaataagggtttccatcaccgtccaggtacgcaacgtttcaccaaccgtcagattaaaataccctttaaatagccagaagccagggtcgtttacgtgtgacgcgatcacgctgcccgcaccggttgccagtaccattaaagcgggatcggcatgggtaacgttgataatcggcaacaccacacccgcggtggtaatggccgcgacggtggcagagcccagagcgatacgcaacagcgccgcaacagtccagcacatcaataacggcgaaagtgtagttccggtcattaagtgtgaaatatagtgcccgacaccgctatctactaatacctgcttaaacgcgccgccgccagcgataataaacacaatcatcgcgatagcgcctatagaatccccaatgatatccatgatttgctcgatggtgcgtccattacgtcggcccagtgtgaaaatcgcaataacaatggcaataaacagcgcaacggcagggttaccgacaaattcaaagaagaggcgcacggtgttagttttcggtaacgtaatttcacaaacggcggcgatagccatcaggatgaccgggatcacggcagcgaaaatactgttccagaaggagggcatctcctcttcgctaaacagatgaggattaaataagccttccggtggtgctttctcaaagcgagttagcagtttagaaaacagcggtcctgcgacaataactgtcggaatggtaatgataaatccatacagtaaagtcgttccgagattagcctcaaagatagtcgcgatggcagtaggccctggatgtggcggcagaaaacagtgggttacagagagcgctgctaccattggtacgccaacatacaacaggggtaatcctgatgatgctacgatggtaaataccaacggcaacagcaggacaaaacccacttcaaaaaacatggcgaggcccacaaccagaccggtgatcactagcgcccattgcacgcgttttttaccaaaagtagcaatcagcgtagtggcgatacgttgtgccgcacccgtatcagaaatcagcttgcctaacatggccccgaaaccgaggatcattgccagcccgccgagcgtgctgccgataccattttgtatagagtgcaggacggcctgtgcatccatcccttcggcaaatccgacgacggcagctaccagaacgagggcaataaagccgttaactttaaagccgatcatcaggataagaagcagcgcgacgcctgccgcaataatgattaatggcatagtctttatctcttattagtgccagaaaagcagcgctttcgcgctgcacgtaggggggctgttaaacagccactaacatgccgccatcaacaaacaacaggtggccgtttacgaaatcagaggcttttgaagaaaggaacaccgcagcaccaatcagttcctgcggatctccccagcgtgcggcgggggtccgtttgcacaaccaggcggtgaaggcttcgtcctcaaccagtgctttagtcatttctgttttgaaatagcccggcgcaataccgttgacctgaatattgtggcgcgccagctcgacgcacatgccgcgggtgagcatttttaccgcccctttcgatgcggcataaggggtgatggtgtcacgtcccagttcgctttgcatcgagcaaatattaataactttacctgccttgcgttcaaccatgtgacgagttaccgcttgcgataccaggaacacggcggtctggtttactgcgatcacatcattccactcttgttcagggaactcagtaaaaggatgacggcgctggataccggcgttattcaccagcacatcaatggggccgatgtccttttcgatatgttcaacggcggcatcaatttcatgtttatgagtaacattaaaaggtgcggcaacggcctgaataccctcctggtggagtttttctacagcaagttctgcgcgttcggcagtaatatcattaataattatttgtgcgccatatttacccaggccggttgccagtaaaaagccaatgccctgtgctgaaccggtaatcaagatattttttcctgccagtgaaaatagatcgttcattgtattattcctttatttatctcttagaaaacaagctggacttttgctgcctgggttttatcaccggcgaaacgtagcgcctcttccaggtcagtgaagggatattcagcactcagtaaaggcagtggattgataacgccattcgccagccatgacactgcggtattaaattcgctggtaaaacggaaagagcctctgagtgaaatctccttaccaatcaacgtcatcattgggaattctgccatcgcgcctcccatacctacctgcaccattacgccgcgtgcacgagtgacctccagacaggtattcactgatgaaggatgaccggacacttcaaagctgacatcgaaatagcctttttccgctttccagtgatccatgtcgtcgttttgtgggtttacgagcacatccgcccccatctctttgcccagcgaaagggaacggggactcacatcagcacagacaatttccgcggcccccagtgttttcactgcactgacaatcaggcagccaatgggtccaacaccggaaataaatactcgcttgccctgtaactcgccggcctgatgtgcggcatgaatcgcgacggctaaaggttcggcaaaagccataaccttttcgtcagctttggccggataagggacacattgcgacgtttcgaccattttataacgggtaaaaccaccatcaacatgagggaaatacatggcactgccaaaaaaacgcatatctgtacactgattctcgttatgttcaatgcagtatttgcagtgaccgcacggtttagacggattaatggctaccgtttgcccttcatgtaattctgatgagtcgctatgaataactttaccgataacttcatgacctaacaccatcggtgcctttatcatgaaattacctacttttccttcctgataataatgtaaatcggaaccgcaaattccacctcgggttatttgtactaatgttccattattattccaatctatcgtctgctcggtaacggcaacagttttcttgcccgcaacaacgcaggactgtgttttcacttgcataaattcctcactggtcaggtagacacctcggaagcatttaagcggttttaactgtcattatttgtgatgaagatcacgtcagaaaattgttacattactatgttacgcataacgtgatgtgccttgtaattcttatcagtagaaataaaaaaacgtgaaattattatgccgccaggcgtagtatcgcagcaggtaagatgattcaggagattttaaatggcgggtgaaagctttattttgatgggcgtttcagggagtggtaaaacattaattggtagcaaggttgccgcgttattatctgctaaatttattgatggtgacgatcttcatccagccaaaaatatagataaaatgtcgcagggtattccattatctgatgaagatcgacttccctggctggaacgcttaaatgatgcttcatacagtctttataaaaagaatgaaacaggatttattgtctgttcatcattaaaaaaacagtatcgtgatattttacgcaagggtagcccccatgttcatttcctctggttagatggcgactatgaaactattctcgcgcgaatgcagcgtcgggctgggcattttatgccggtagcgttactaaaaagtcagtttgaggcactggagcgtccacaagcagatgaacaggatattgtgcgcattgatatcaaccatgatattgccaatgtcaccgaacaatgtcggcaggctgtgctggcgatacgacaaaacagaatatgtgcgaaagagggcagcgcctcagatcagcgctgcgaatgattttcaaaaatcggctttcaacaccacgcggtaacgcgccttaccgtcgcgcacatgctggatggcgtcgttaattttcgacatcgggaacagttcggtggtcggcgcaaccttgctgcgggcggcaaaacgcatcagcttacgcagctcataaggcgtgccggtagcagaaccagagacgctgcgatcgcccgcaattaacgtaaaggccggaacagacagcggcgtgagaaccgcaccgaccgtatggaaattaccgccataggtcagcgcctcaaaatagggctgccagtcgaggctgacgttgacggtgttgataatgagatcaaactgccccgccagtgctttcagtgcctgcggatcgcggctattcaccactttatcggcacccatcgccagcacttcctgctctttcgccggattagaactaaaggctgtcacctcgcatcccattgcgtgcagaagttttatagcgatatgccccagcccgccaataccaattaccccaacgcggctggtagcagtgatatggtgcatcaacagtggtttaaagaccgtgataccgccgcacaacagcggcccggcggactcgatatcaatattttctggcagtggaatcacccattgccagtccgcacgcaacttctcggcaaagccaccgcgattcataatcgtcggcaccgcaccttgctcgcagttgatctgattaccgctaatacaggcgtcgcagtgaccacagctacgcgccgtccagccaatcccgacacgctgaccgacctgcaaacctttatcctgcgcggcgctcccgagtgccaccacgcgcccaatcacctcatgcccggcaaccagcggatattgtgaaaatccccattcgttatcgatcatcgacagatcggaatggcagatcccgcagtaatccacctgcacttcaacatcttgtggcctcagctcaccgggatcgtactcataaacttccagttcgccgcccgcttcttttgcggcatagctttttatcatcgacattttttggtccttctctggtgttgtttgggaagtgtagagcatggcagggcggggtgcctggagtgtgacaaaggttacacatcgctgtatgcaatgctgaaaatttcagcacttagcgaggtgcgagcaagctggcgcttgcatggtggcgtgcgacaggtataatccacaacgttttccgcatacctcttcagtgccgaagtggcgaaatcggtagacgcagttgattcaaaatcaaccgtagaaatacgtgccggttcgagtccggccttcggcaccaaaagtatgtaaatagacctcaactgaggtctttttttatgcctgaaatccagtgtttatctatctttcccgctatattaactctctcaaggtcaaccgatatcaacgtacatctaccaacatatgttggtacagatgatggtatttccggttcgataatgcttgtaccaacagggagggaatacgatggcattaacagatatcaaagtcagagcagccaagccaacggataagcaatattagctgactgatggtggcggtatgcatctgcttgtccatccaaatggttctaagtactggcgtttgcagtaccgttatgagggaaagcaaaaaatgctggcacttggggtttatcctgaaatcacactagcggatgccagagtacgtcgtgacgaggcgcgtaagctgcttgcgaatggcgtcgatccgggagacaaaaagaaaaatgataaggttgaacagagtaaagcacgaacctttaaagaagtcgcgattgagtggcatggcaccaataaaaagtggtctgaagatcacgcccatcgtgtgctaaaaagtcttgaagataatctttttgcagcgcttggtgaacgtaatatcgctgagttaaaaactcgagatttattagcacctattaaggccgtagaaatgtctggacgtcttgaagtggccgctcgtcttcagcagcgcactacagccatcatgcgctatgcagtgcaaagtgggttaattgattataacccggcacaagagatggctggggcggttgcttcctgtaatcgacaacatcgtcccgcgcttgaattaaagcgcatccctgagttgcttacaaaaatagatagctatactggtaggccgctaacccgatgggcgatagaactcactttgctgatctttattcggtccagtgagctgcgttttgctcgttggtcagagatcgatttcgaagcgtctatatggactatcccaccggagcgggagcctattcctggagtgaaacattcccatagaggctcaaaaatgcgtacaacgcatctagtgcctctttcaacgcaagctcttgcaattttaaagcagataaaacagttttatggggcccatgacttgatatttattggtgatcacgattcgcacaaacccatgagtgagaatacggtaaatagtgcgttacgggtcatggggtatgatacaaaagtagaggtttgtggtcatggctttcgaacaatggcctgtagttcattggtcgaatcaggtctgtggtctcgtgatgctgttgaacgtcagatgagccacatggcgcgaaattcagtgagggccgcgtatatccataaagcagagcatctggaagaacggcgattgatgctacagtggtgggccgattttctggatgtaaacagagaaaggtttatcagtccatttgaatatgcaaagattaataatccattaaaacagtaatcatcccgggcaaatgcccgggaattattctaggattattttctttgttaaaaaagacaaacggtattaactgatgtatttactatttaccgctccctgcaggggggattatcagaatccgcggttattcattatttatatacattcaataaaaaagtaacctcataaaaaatcctgtactcacagggtgatgcgggataactgacgtaaggagtgctgcagggatttgatggtcccttgtagactggccccctgaatctccagacaaccaatatcacttaaataagtgatagtcttaatactagtttttagactagtcattggagaacagatgattgatgtcttagggccggagaaacgcagacggcgtaccacacaggaaaagatcgcaattgttcagcagagctttgaaccggggatgacggtctccctcgttgcccggcaacatggtgtagcagccagccagttatttctctggcgtaagcaataccaggaaggaagtcttactgctgtcgccgccggagaacaggttgttcctgcctctgaacttgctgccgccatgaagcagattaaagaactccagcgcctgctcggcaagaaaacgatggaaaatgaactcctcaaagaagccgttgaatatggacgggcaaaaaagtggatagcgcacgcgcccttattgcccggggatggggagtaagcttagtcagccgttgtctccgggtgtcgcgtgcgcagttgcacgtcattctcagacgaaccgatgactggatggatggccgccgcagtcgtcacactgatgatacggatgtgcttctccgtatacaccatgttatcggagagctgccaacgtatggttatcgtcgggtatgggcgctgcttcgcagacaggcagaacttgatggtatgcctgcgatcaatgccaaacgtgtttaccggatcatgcgccagaatgcgctgttgcttgagcgaaaacctgctgtaccgccatcgaaacgggcacatacaggcagagtggccgtgaaagaaagcaatcagcgatggtgctctgacgggttcgagttctgctgtgataacggagagagactgcgtgtcacgttcgcgctggactgctgtgatcgtgaggcactgcactgggcggtcactaccggcggcttcaacagtgaaacagtacaggacgtcatgctgggagcggtggaacgccgcttcggcaacgatcttccgtcgtctccagtggagtggctgacggataatggttcatgctaccgggctaatgaaacacgccagttcgcccggatgttgggacttgaaccgaagaacacggcggtgcggagtccggagagtaacggaatagcagagagcttcgtgaaaacgataaagcgtgactacatcagtatcatgcccaaaccagacgggttaacggcagcaaagaaccttgcagaggcgttcgagcattataacgaatggcatccgcatagtgcgctgggttatcgctcgccacgggaatatctgcggcagcgggcttgtaatgggttaagtgataacagatgtctggaaatataggggcaaatccaccttgtgctgatatgaatacggatattttatacagaatacttttcagtacaagcgactgtattacagtctgccatatatgattacctgtgatcaggaagaataagtggctgaggtttcaaactgtctgccggtatattcctctctcccttaaaaaccataacaggttagttatcttcgtctgtcagcggattgaatggcggtatattttcagtacaaataccggtcatccactgaaaaatacctgcgaaatgacgggcactgatttttctactgacgggctgatgagacgttatgtcactggcggtaataatcagtggcacactgtagcctccctgcacatgaccataatgatgaacaggattggcactgtcgctgaccgacagcccaaggccagaaaagtaaagcatggcgaaatgacgtgagtaccggcgaaggataccatcaagctggccaagaaagttatccagtttactgatgctggcgaggtaacaggcaatttttcggggatactgctccaggtaattattcggctaggagttaaggctgtcacacggatttggatgagaacccatcatgtgcaggaaaattatcttcggagaggatgtatccgccagcgcacgttctgtttcctgtaacaacagtttgtcatctgttttacgggaagcgaagctgcctttcttgaggaaagtggcatgctccgcatcagaagcaataacagagatgcgtgtgtcatgctcccccagttttccttgattggatatccaccatgtgctgtatcctgcttttgctgccagcgccaccacattgttgccggaatcagggttctgctcatagtcataaatcagtgtccggctcagggaagacactgtactggaggctgtcgaggtataatcgtcaataaataaaccgggtgccgtattcagccacggtgtggttggtacgggatagtcatacactgacatataatccctgcgcacactctcaccagtgacaataacaatcgtatcatataacggtgctcccggctggattttccagttgtcagccccgtgctactcagttgttcataacgctgcatttcacgtaatgtgtcagttgtccccacaactgttcctttaaccatccgcaatggccaacggtttacagagcataatacgaatagccgtagagccagccagttacggtggtcgcgatggtgtgtccgccagaaaatcaccacgaataccagaatcgcggcactgaccagaaaatgataaacaggaaacacggggcggttcactttgctttctcctgtagtgttttctgtaggttctgaaccggttctagcggggttgtgaggctgatggcaatcgccgggctcttcctgcatgttacactggtactgcaagagggggccttcgctcctctgacattactcagtattttcactactacaccccatctgccatccataacaaccgattcaccccctcgcgaggcgttgttgcccgtcacccggacagacaccgttatggacttctcttgttgcacgatcgatcaattgttatgcatgctgacaccacaaccccggtgggtatgaccgatgcctttctcactctcttcccggtcatcgtcggccttccccgttattgtggcgtgtcagcaccctcgacggcatttcgatggctgctcagtgttcactcacgttacggcccgcataacccgttgacttcctgaagaagtcgtttcagggagagattcagcccttttgttacctcctggaccgcttcttgtccttccagtcggagcgagagttagccggggcggactttcaccgacggaaagatcgtgcatttcaaggcacacacaacaatatctgcgagcgtgctatccgtccggtcgttatgggacgaaaggcctggttgttcgctggttcactggtggccgggaaccgcgcggcacagataatgagccttctgggaaccgcagtctggagccacatgcttggctgacggacgtcctgacgcgtctgccggagtggccggaggagaggttggctgagttactgcctcttgagggctttaccttcttcgggtaagtgatacctgccgtcaggtgtttgtgcaccgggccataacctgcagttgggaattgaacgcctgacaacaggaaatgagctagagcagtaaacacgcgggctgacaatgggtcagaatatgagttagcccggcgttattcctggggtcagtacttcagatctagcctccggtaccagactagctagcccctacgcaaccaaataaatcaaccatcgtcagagtgcaatcgttcatatacactgtcggtgatgcgctaaaaaatgcgttaatgttgagttcctcgaacccttaccaattaagggacatagccagatacgcaactggctgatgcaagcagtctaatgtctttagatccgctggcctgcgggcatgacaatgtcaaacagtcaaagattgtggcgttgacggtcagtcttggggacaaaaaagctcagtattctcgttggcaaccagataatttaacagttgatgctgaaacgaaataggcatcttggttctgtaatgccagtcagttaagcaactgactggctctttttcggggctgtggggtatttccagggcctctcctttaccactctcgggaaggccctttcccttcttgtcggtaatttcacaagttgtcccatacttgcaagatcgcgcatcagctccggtatacgtcccggtgaagcgccctgcaatgtcatcagcattctcatcaccattccgcatgattctgagaaactcagttgattcggccagtaacctttcagatgttccgccattttaatcatctgatatctcaccagattataagccagtaagacaccccacagctcttgctccacaagctccggctttttacttctcagcgtcagcctgctccgttgcatcgtctgttttatctccctgtatcccagttcgatttcccagcgatgactgtacagatcccccatttctcctccggggaagcgcatggcgtccgtcatcgacgtcagcagatggcagacttttcctttgcgcgtcacggtcagcaggcgggcagtcacttcatttcccagtcccggccacttttttcgtgcctgcgggctggttttcagcttcaccagatgatcgcctttacccagttttctgatctcttcatattgcgctccctttctgagaggtatcatccagtggcggtgttctcccgccaggctccaggcatttaacagtcccagtgagtaataacctttatccattaacgtcagagtgttatcgccggtttgttctataagttgctcagcaagctcattttcgctgttcttcatcgtgccgaaggctgcagccgtcagcagatggctggtcagttccatctggcagaccattttgacctgcgggtagagcgccgggttcccggcatgtgtctggcgggggaaggctgcatcgttctctggtgtatccggtgtgcgccagaacacaccatcgatggccagcagggtcaggccgcaccagtgcggatgcggcgtggcgttatgccagagctgcgctgttttcgtgaacacgcggcggacagcctcacttcccaggcgctggcgggcctgaataacggcactgggggcaacgaaggggcgattgcccggcagcatgatgtccaggcgattcacaatctggtgaagaggttctttacgctcaagcgccatgccaacaatacaccagaccatcatttcgaggggaagacggcgcttgcgtagcgttacagtacctgattcggcaaggcaacgagagatgagttcggggtcgaggtaatcccccagagaagtcagtgggttacgcagagaatcgtaacgggataccagatcaagagcctgtccaatgtgcataaaaaaatccggaaacaagtgagcgtttccggattcttacacagccactggatcggtcaactgatccttaactgatcggcattaatcttggttctggtgtttgtaacaaactatcagctacaaaaatatgctcaatttgtgacatcagtaacaaaacgcgttttgttatgtggattgcttgttttttgatctggtataacaggtataaaggtatacagaaaagcaaagaaatactgcaaaggaaaacagctataacgtaagctaaagtaataacctctcagtctttcctcatttgacgaagggagttttattcaacctgaacggactacgaaaatgagcacaatgaataagtcaatttttgaagcagggttgaactgtgccagtggtggaatatctggcgaacattgttttttgttggtgacccaaaactgtaggtgggtatcagttttatctttcatagagtgaaatatgttaagaagaaatggaggaaaagattgtactgattaggtattgataacaatcaatagtactggcgtatttgaagacaatataattatttctggatattgttgaggctccctaatatttactttaagggctatattagaataacacaggaaacaaatatggcaacagcatggtataaacaagttaatccaccacaacggaaagctcttttttccgcatggcttggatatgtatttgatggctttgattttatgatgatattttacattcttcatattataaaagcagatcttggcattacggatattcaggctactttaatagggacagtggccttcatagccagacctattggaggtggtttttttggtgccatggctgataaatatggtcgtaagccaatgatgatgtgggcaattttcatttactcagtcggaacaggccttagcggtattgctacaaacttatatatgctcgcagtttgccgttttattgttggcttagggatgtctggtgaatatgcatgtgcttcaacttatgcggtagaaagttggcctaaaaatcttcaatctaaagctagtgcttttttggtaagtggtttttctgttggaaatattattgcggcacaaataatccctcagtttgctgaagtatatggatggagaaactctttttttataggcctgttaccagttttactagttctttggatcagaaaaagtgctccagaaagtcaggagtggattgaagataaatataaggataaatcaacatttttgtctgtcttcagaaaaccacatctttcaatctctatgatcgttttcctcgtctgtttttgtctatttggtgcaaactggccgataaacggactacttccttcctacctggcagataatggagttaatacagtggtcatttcaactctgatgacaatagcaggtttaggaacactgacaggtacaatattttttggttttgttggtgataagattggtgtaaaaaaagcctttgtagtcggtctaataacttcatttattttcctttgtcctcttttttttatttctgtgaaaaactcttctcttataggattatgtctctttggattaatgtttacaaatttaggtattgcagggttggttccaaaatttatatatgattactttccaacaaaattaagaggattagggaccggtcttatttataacttaggggcaactggaggaatggccgcacctgtattagctacatacatttcaggatattatggcttaggtgtttcattattcattgttacggttgcattctctgccttattaattttgttagttggttttgatattccaggtaaaatttataaactatccgtggctaaatgattggaggctttatgattaattatggcgttgttggtgttggatactttggcgctgaattagctcgttttatgaatatgcatgataatgcaaaaattacatgtgtatacgatcctgaaaatggagaaaatattgcccgtgaattgcagtgtatcaatatgtcaagcttggatgctttagtctcaagtaaattagtcgattgcgtgatcgtagccaccccaaattatctgcataaagaaccagtaattaaagcagcaaagaataagaagcatgttttttgtgaaaaaccaattgcattaagttatgaagattgtgtggatatggtcaaagcgtgtaaagaagctggtgtgacctttatggccgggcatattatgaattttttcaatggggttcaatatgcacggaagttaattaaagaaggtgttatcggcgaaatattatcatgtcatactaagagaaatggctgggaaaacaaacaagagagactttcctggaaaaagatgaaagaacaatctggtggacatctatatcatcatatacatgagttagattgtgttcagcatttacttggagaaataccagagacggttactatgattggtggaaatttggcccattctggtccaggatttggcaatgaagatgatatgttatttatgaccttggaattcccgtcaggaaaactagcaaccttagagtgggggagtgcatttaactggccggaacattatgtcatcatcaatggaactaaaggctctattaaaattgatatgcaagaaacagcagggtcacttaggattggcggtcagacaaagcattttttggtccatgaaacacaagaagaagatgatgatcgtcggaaaggcaatatgacctcagaaatggatggcgctatagcatatggtcatccaggaaaaaaaacaccattatggcttgccagtttaataagaaaggagacgttattcctccataatatcctctgtggtgcaaaacctgaagaagattatattgaccttctcaatggtgaggcggccatgtcggcgattgctactgctgatgctgccactctttcaagatcgcaggacaggaaagtgaaaatcagtgagatcattaaacatacatcagtaatgtaaaaactatacgcctcttgatttaattcaggaggccttttatgtatgatcaagaattttatcttcgataatctcataattttagcagtgccatttatgataaaaacatcccttaaaaccaatctaatctttttcttcctctgtgtatttgttccccatatggcgtcataatttacgctacgtaatacgggatagttacgatacgcagcgatagcgctaagttttagttaaaatcccccatcagcgggatatggggatctctgggaggttcaggttttagcatcgcgactttaatacgacagacgctggtgacgatgatgccaagtagtgactcttccgaataaggttcccactgaccaattggcgcgcgcttcgcaataaaatctcccttcgcccagtattgggaaaagtagatacattcaaactgtgtacgctgtttcgtctcacagttcacgacattgctggccgatgagctgaccattgggcctatccgggctgtcccgatggatattacgccgaagtatgtgggaattgccagcggattgatgaacgccggttccgctgtcgccgacattatttcacctatcgcctttggcattattatcgacaaaacaggcaactggagtttaccattctacggttccgtcgcattgcttgttattggtatattcctgacgttcttcatgcgtccagataagtcattgtaaaagtcgaatcagggctgaagtggcacactgaatttggccacctgaacagaggtgatatgctcacctcagaacaacacaggtgctccaatgaaaaaaagaaatttcagcgcagagtttaaacgcgaatccgctcaactggttgttgaccagaaatacacggtggcagatgccgcgaaagctatggatgttggcctttccacaatgacaagatgggtcaaacaactgcgtgatgagcgtcagggcaaaacaccaaaagcctctccgataacaccagaacaaatcgaaatacgtaagctgaggaaaaagctacaacggattgaaatggagaatgaaatattaaaaaggctactgtagattcaatctgtcaatgcaacacccctttcaattatctctttcggtgttttgaacttcagtgtctttctcggtctgttgtttagctgagcagcaaccagatctagttcatgttgagtatattgggcaagacatgtctttttaggaaagtactgccgaattagcccatttgtgttctcatttgttccccgctgccaaggactctgaggatcgcagaagtaaactttaacgccggtgctgacagtaaattctagatgtctggccagttccattcctctgtcccatgtcagtgattttctgagttctgacggtaaactcaggaatttgtcggtaagagcctgatttactgagacagaatctttgcccctgagtctaaggatgatcgtataacgtgattttcggtctacaagtgtggctatatgagagttttttgtacctgagactaaatcgccctcccaatgccctagagagcgtctgttatcgatatttcgggaacgttcgtgaattggtgttccgttcactatgttaatcgtacctctttcgcctttgcgggtatgacgcctgccatggcgaaggctatgcgaccgtcgcagatgctgtatattcaggtggtgtagcgcttcacggctacgaaagtacagcgttttataaattgtctcaggtgatattcgcagcgttttttgacgtggttttgttcgccttaaccatcctgatatttgctctggagaccatttcatctccagcttttccagaacaagctttcgcaatggtaaattttgatccagtaagcacggttttggccttttcgccattctgttggctcggttattagcatcaacagctttgtaatagcgtctgccccgattacgctgaacttcacgtgagatcgtcgaaggactgcgattcagcgcagtagctatcgcacgaatgctcattttggctgacaaaccagctcgtatctcctcgcgctcagacagtgtcaggtgagctacagcccgcttacgctcatggggttttatgccgccagtatcccttaacatagtgaagatcgttccgggttttgaacccaggatattcgctatttcactgaagcctgttccgttcttccatagttcaaaaacagaggctttttcctctgctgtaaatgttcgtctcattcaaaaaacctccgcaaccccatgttttcacataactgttgcgttgaccaattgaatctacagttgctttttttaatatatctcgctcaaggcgagcttcatttaacgccttacgcagttgcagaatttcagattccagttcagccaccgtgcgggaaccaggagtaccgagcccttttctggcggcggtaacccattgtcctaaagtgccttcaggaagagataatcgggaagcgccttcactgatcgaaagttgattttcaagaaccgttctgacagcttcggctttgaactttttagagtaacgttgggtttttctgctcattattagctccttctgatgccattctatttcaggaaggagtgtccgttaaactcaggctacctcaggaaaaaccgtcctgaaaaaccagacggcagacgggctgtattacgcagtcaggtacttgagctacatggcatcagccacggttcggccggagcaagaagcatcgccacaatggcaacccggagaggctaccagatgggacgctggcttgctggcaggctcatgaaagagctggggctggtcagctgtcagcagccgactcaccggtataaacgtggtggtcatgaacatgttgctatccctaactaccttgaaaggcagttcgccgtgaccgagccaaatcaggtgtggtgcggtgatgtgacctatatctggacgggtaagcgctgggcgtacctcgccgttgttctcgacctgttcgcaagaaaaccagtgggctgggccatgtcgttctcgccggacagcaggcttaccatgaaagcactggaaatggcatgggaaacccgtggtaagcccgtcggggtgatgttccaagcgatcaaggcagtcattatacgagcaggcagttccggcagttactgtggcgataccggatcaggcagagtatgagtcggcgtggaaactgctgggataacagcccaatggagcgcttcttcaggagtctgaagaacgaatgggtgccagcgacgggctatgtaagcttcagcgatgcagctcacgcaataacggactatatcgttggatattacagcgcactaagaccgcacgaatataatggtgggttaccaccaaacgaatcagaaaaccgatactggaaaaactctaacgcggaggccagttttagttgaccacaacagactacctgaagggagccgcggtcgcctggcagttgcagtagcaggagatcatccagccgcagtacaggtcacgatgactctggttaatgataccggctttgaccccgtattttccggctctatcgctgaatcatggcgtcagcagccgtgcacaccatcctattgttgtgactgggaggctgccaccatgcttcgcgctttccctctggcgaaaaagggagaaggacgggcccgtctgccttcactttatgccagcttcggtaagctgggtgagacaccgactcatgaagatatcattgataacaatcgatccatcaactggcctgtataacgtggctgccggtgattaagaaagctgcacctacctaagtagtagcaaacgcacactttttagaaaaatcgatggtcagaaactggattagcaattccgttccatggttgcttttgatttacgttggcgtctgatcattgatttatcctcaaaagcccaacctcattggtaatgaaccagctccgtgaatgtccgctctggcacagagcgaaattttttgatctcccccctgaaatctaaacttagtcatgtcacgtttttgggtttctaaaattttaacttcgcgtttttcgttgccgtaagggttatacagaaatgtccgttaagcagagttcaaaattgattgccgtgatcacgactggtttgaaagccgcgcccaagcctgtacagctctggtttgcgttgattatgaacctgtcagcctaaagcaagcggatggacgatgagtattggtaatctttcagagtccggaaaagttcagccccagtctgaacaggcttgctggcgccagtccagtttcattcagtcgtggtttggttcttacggcctgtgcaatctacctcattaggcacatcggcctgccagataccggctcggggtgtatttccgcttccacgctgaatactgttctcagcaatcctggggtcatcacctcttctggtgtgccttgcgccataacatgtccgtttgccattaccaccagttgatcgcagtaccggctagcctgattaaggtcgtgcagcacagcgaccaccgttttcccctgagtccggagttcgcccatcaaccgcatcaggtccacctggtgattgatatcaagataggtggttggctcatcaagtaatacaacgggcgtattctgggccaggaccattgccagaaatgcgcgctggcgctgaccgccggaaagctcggttaaccgacgaacggcaagatgattgatccgggtctggttcatggcgacattaactcgtgcattgtcttcagcggagagacgcccccagagtgacagccagggattacgaccatacgaaaccagctcctggactgtgatcccctctggcgttaaatggtgctgaggcagcagcgaaagcctgcgggccaactggcgcgatgagagcatatttatgggattatcgccgagaaatacggtgccagactgcggcattaaaagccgcgaaaaacagtttaacagcgtcgatttcccgcaaccgttaggaccgatcagggcggtgatcttccccgttggcagtgagagtgaaacgtcgttaagtaccttgtctgtcccgtaactgaccgtcagattttcagttcgtaaagtcatttatcgcattctcacaagcaaccagacaaaccacggcgcaccgataatggcggtcagcacgccaaccgggagctccagtgggggatgaataattctcgccagcagatcggcaaccaccaacagcaacgcacctgtcagggccgaaacaggcagcagtctgcggtgacgtccaccggtgatgctacgcatcatatgcggcaccacgagaccaataaagctaatcgggccgcaggcggccacgccggtagatgtcatggcgacagctagtaacaaagcccagaatcgggtatggggcaccgacacaccgagcgtggtggcgcgcgcatcgccgagtgcaaggaggtcgagatcgcggcaaaaactcaggctcagcggcagaaataaaatcatcagcgggatggcaatcttcacaaagctccagtcacggccccataagctgccggtcagccacagcagggcgttgttcacatcctgcgggcgcgagagcatcagataatccgtcaggctggcccagcatgcagaaagcgccacgccggtgagcgccagcttcatcggctggtgggtctttgccagcatcttcagcaatatcaaccccgccatgccgcccgcaaaggccagcagcggcagcaccatcacgggcagtgacggcataagaagtagagcccccacagaggccaggctggcggcatggttaacaccgagaatatccggtgatgccagagggttgcgcacaatcccctgtatcagcacgcccgccacggcgagggctgcaccgacaaacagtgccagcagcaagcgcggcagtcggtactccatcaatacataataatgctcgtgtccggcctgccagtcggtcagcagcgcgcgccacggcacggggatcactcccatatggagtgataacagcgcacagcccgccagggcaagggtgatgaaaataaccagcgcaattttcatcctcgcctcctcacaagccagacaaagcaagggctgccaatcagcgccagcactgcgcctgcgggcagatctccggggaaggccagcgcgcgtgcgagtacatctgccagcagcatcagcgtggcccccagcagcatgctcactggcagtacgttgcgctgatcgaagcctgcccagaagcgcgccagatgtggcaccagcagaccgataaacgccaccggacctgctacgctgacgcacgcaccaaccagaagcagcactaacatattgatgaccaaacgtagcctcgtcaggttcactcccagcgtatgggcggtgctgtcgctgaggttgagcaggttcagttgattcgccagcagcaacacgacagggactgcagtgaccaccaccggcaagagctgccagacatcctgccagcgggcgtgggacactccgcctgccagccagtaaaagatgccgtaagcatgatcttcggccagcagcagggtgatgcgggtaaggcccatacaaaaggccgacagcgcgatacccgcgaggatcagtttgtttctgtcatgggtatgacgaaatccgcctcctgcggtcatgaccagcagccagctcacgccgcccccgcatgccgcgatgaatgacagagaatagcctgcaatcggcgtcggactcagcgcgctggtaagcgccatagccagcgccgcgccgctgttaatgccgagcagtgaaggagaggccattgggttgtgggtcagggtttgcagcagcgtgcccgcgagcgccaggcttgcgccgatcagaacggcgaccaggcttcgtggcaaacgaaggttttgcaccagcgcttctggtagcgttggcgtgtgtccaggcagcagggcgcgggttgcatctgctccggaaacaggaatggccgagtagcaaaacagactcagccagaaaataataataagtgctgcaacgggaagcccccacagcagcaccgggtgttttatcgcggtcatttcacaacggtaagcggctgatggtggaagatttttaccgtgtcagcggcaatacgctctgcagcaaaaataccgcgcatccgcgcccaggtgttactgtcgaccgaagcaacctgctgcttctgcgcggcggttaacatctgccagagcggatcttgttgccagcgtttaacaatgctctcttcgcgatagtgggcaaccagcagccaggcaggattgaccgccagcagttgctccaggccgatggacggcatggacgcacccgccatcgcagcgggaacgttcagccccagagaggccagcacgctgccggtccaggtctcctgagtatgcaggttgaattgctgttcgcgtgatgtgccaaaggccacgcgtgtccctttgggaagctggctggcccactgcgccatcctctctttatgttgttccagacgtgcctgcatctctcgctttttacccaccatttcgccgatgatagccgcagattgcaaattttcagcgtaggtttcgttgcgggacttaagcagcagtaccggcgcgatttgctgcaaggcgatgtaaacccccgcatggcgactgctgtcggcaatgatcaggtctggtttcagagcggcaatggcttccaggctcggctgcgcgcgcgttccgacggactgccacggtttcaggtgcgcacgcacttcgggcaggatgcgttttgcatcgttatcgtcggcaataccgatcgggatgacgtccacggcggccagcgcatcggcgaacgagagttccagcaccacaatccgttgtggcgttttttcgagtgtaaacgtgccgtgttcgtcctgaaccgtggcggcaaaggcgtggctgatcaccagcagcaggcctgcaaaaagaaaacggataaatgccaacataatcacattccagctaaaagcccggcaagccgggcgttaacacatcagaacttcaacgacccctgcatatacagcgtgcgcggctggcctgcatagatgcctttgttgttgtcgtcataagagcggatgaagtagtcctggtcgaagatgtttttcacaccgaatgccaggttcagatctgccatctgcgggccaaagtcatacgccacgcgtgcgccccagagcatgaagccgggaatgcggccggtactgccgtcggcgctctctttcaccgtattggcgttatccgcaaactggctggactggaaatcgctgttcagattgaacgtccagtttcctggcttgtagtccacgcccagcgtgcctttatgtttcggggagaatggtaccagattgccgtaggtgtcgcctttctcgcggatttccgcgttcacatacgcatagctggcgtagatggaaacgttatcaagcgttggcgttagcgtacccagatcgtaacgtgcctgcgtttccagcccggtatggcgcgttttgccacgtgcagtgacggtgtcgttggtctggttggagtcgtactgattgttaaagttaatcaggaacagccccatttccgccgtcagcgcgccgtcgtcgtagcgggtaccgagttcccaggttcgcgctttttccggttcaacattgccgctttgcacagccttgccaatctggctgtactgtacggtgccgaacgagccttcagtgtttgcataaagattccagctgtcagtcaggtgatagagcacgttcaacgccggaagcggtgcgttatagctcacttcttcgtgcgtgcctgtgatggcgttgttctggtatgactcgatatgttcgaaacgcatacccggcgtgatggtccagttgccgatgtcgattttgtcatccagataccaggcgtgcgcctcggtgccggaacgcgtatcgcggtcgtaagggcttgagccggacggcaactgcccgctgctggtggcggtgtagtaacgcatttcatgcgttgattcattcaaatagcgatagcccacgcccacttcgtgcgcggaagggccgatcataaagatctggctgtagcgtggctcaataccgcgcacccagtagttacgcggcgagagggtgatgcgtttgccttgctccaggtagccgctgcgcagggtttgggtgtagaacccctgaatgttgaatttatgctggctgtctggctggaactggtagcccaggctcgccagcttgcgacgaccccagaagcggtcatacgggcgggtggattgccagcgatcggcgtcgtaatccgcgcgagacaggccaccgggcatgtcggcttcaccgtcgtaatattgcagcaggctgttgaaggtgtgcacctcatccggcgcatatttgcttttcagcatcaggtcgtcgatgcgggtggcgctgtgctcgcgccagtcactgccgcgcgtgccggagtagagcagcgcggtgccaaaaccgttgtccgctgtgccgcccaccatcaggttgtgcgtctctttcgggttgttttgtgaagaggttgggctgagctgaccttccacgcccgcctcgataccaaagtcctgcggaatggcacgggtaacaaagttcaccacgccgcccacgctctgcggtccgtaacgcaccgcaccaccaccgcgtaccacgtcaatggcatccatgttgccgagcgaaacgggagccagtgaaagctgcggctgaccgtaaggggcgaaggggacggggatgccgtccatcaggacggtcgagcggctggcgaggcgcgggttcaggccccggatgccaaagttcatcgccaggtcgtggctgccggtgccgttgttttccggcgcgctgacgccagggatgcggttaagtacctcacgcatggtggttgcgccggttttggcgaaatcctcacggcggatcacgtcacgcgcgccagcatgttcaaatacgtcgttttcacgcgcatcacccagccagtcgccgaccacggtcagggcatcttcttttggtgcgggcgcgggctccagcgtccagctgttatttcccagcggttttacctgcagtccgctgccgtccagcagttgttgcaggccgctctcgacgtcgtaatcgccgtgcaggccgttgctctgcttgccgcgcgtcaggctggcgtcaaccgagagggtaaatccgctgtgtgcggcatactgattgagcgctttatcgagcgatcccggtgcgatattaacctgtgcagcaaaagcggaaaacgagagaccggccagcggcagcaggctcaggcgaatggtgttaaccaaaggtgttgttttacgaaaaacgcgtaacggcgtcataccttccccatcatcatttttgttgtgttcagctatgagtcgaacgagaagggtaaaaaggacaatcgaaataagaattattttccttacagtggtgaaatgtttatccagtaccgcgtaatagactgaattttaacgggaagcgtttgcgcgataacgttcaggatcgcatcggtatttttcagcgggaacgtcccgctcaggcgcagcccggcaacggcgggatcgcagcgcagcacgccgttgcggtaacgggttagcgtggctatcacctcacccagcggtttatcgctgaagctcaggatgtccttcgtccagcttgtactctcgtcatccagcggtttcactgcgccaaactcagaggcgctgaactgcaggctttcaccagcgttcacgatgcgtttttgcgcgggggcactggcgagaagcacttccacagcgtgctgctgcacgtcaagctgcgtgaaattatcctgctggcggacggtaaattctgtccctaaagcagtgagctggccctgacgggtcaggacacggaaggggcgttgcagggcatctttcgcggtagtaatggcgatttcaccgtaccagagccggacggtgcgctgatgcgcatcaaaacgcacatccgccgcgctttgggtattcagcgtgagcagggagccatcttccagttgctgacggctgactgtgcctttggcggtgcggtaatctgcccgcagaccttcgccggtttccgactgccagagctgccagcctccgccagcgccgagcaacagcagtaatcctttcatcacgtgacggcgggtgaggcgggtatcgtgcaacgcccggctggcaacgtcgccaggcacaccgccaagctggttgcgcaggttttcaacctgctgccaggcccactggttatcctgatcctgttcataccactgttgccagcgcgcttcctgttgtgggctgacgcgctcgccgcttagcacggcataccagtgggaagctgaacgcagcgcctgacggcgggaatcggttaacaaaggattcataacccatactccagacggaacagcaggcagtgctcgacggctttcgccacgtattttttcacggagctgatggaaacaccgagtttgtgcgcaatctcgctgtatgtcagaccatccagttgcgaaagcagaaacgcttcacgtgttttgccgtttagcccgtccagcatgctgtcgaggagttgtagggtctcgagttggctttcgcgttcctcaggtgaaggcgctcccccctccggcataagcgccagcatctccagatacgctttttccagcgcgtttcggcgaaacaggtccaccatcacgcgtttggcgatagtgcagaggaaggagcgaggatcgcggatcgtcgagagcgtttcgctgaccattacccgcaaaaaagtgtcctgggcaatgtcatctgcatcaaaagcagactggagtttgcgcgtcagccagcttttcaaccagccgtgatgtgtgccataaagcgactcgaacgttaaggaagctgtggtagtggcgcggtcagacatgcggagtgcatcaaaagttaattatcacgtagtcatattaatatgagaatggttatcattacaattggaaataaaattgtttccaatagacatttttaacatgttgtttttctaagtgttataaggtaggtataaaatgggatggagcctctgcttctggcatgtgtcggtcagaatgactcatgatgtggtctgctattattgacatcctcactgccctaaaggatggggatttcggtaatgctgccaacttactgatttagtgtatgatggtgattttaaggtgcttgcgtggcttccatttccatcagatgtccttcctgctccgctactgaaggcgtggtgcgtaacggcaaaagcactgccggacatcagcgctatctctgctctccttgccgtaaaacatggcaactacagttcacttacaccgcctctcagcccggtaagcaccagaaaatcattgatatggccatgaatggcgtcggatgtcgcgccagtgcacgcattatgggcgttggcctcaacacggttttacgtcacttaaaaaactcaggccgcagtcggtaacctcgcgcatacaaccgggcagtgatgtgattgtctgcgctgaaatggacgaacagtggggctacgtcggtgctaaatcacgtcagcgctggctgttttacgcgtatgacaggatacggaggacggttgtggcgcacgtcttcggtgaacgcactctggccacactggagcgtcttctgagcctgctgtcggcctttgaggtcgtggtatagatgacggatggctggccgctgtatgaatcacgcctgaagggaaagctgcacgttatcagcaagcgttacactcagcgcattgagcgacataatctgaatctgagacaacatctggcaaggctgggacggaagttactgtcgttctcaaaatcggtggagttgcatgacaaggtcatcgggcattatctgaacataaaacactatcagtaagttggagtcattaccgaccatgtttatttcatacattgtgggtattgttcttattatcgccgctaatcaataaaatcctgccccatatctacatggggcagttgttcattcttttagtgtggtaattcacacgccagcaaaaactctgccgttccttcatcaacaatcaggtccgtgacatatcctcccagcagggcacccaacgttgcgtcatagcctctttccccaccagcaaggaagatcttccgttcaatctgccttagctgagccagactgattcccagaatacgctggtcaacatcagccacgacgggcatcccttccttgtcatagaagcgaccacaaatgacacctactgcgcctaaatcccgatacgtctgcatttccttcttattcagcacgcccacccgaatcaggggattttcatcaagcgcgttacccacgacaaaaaaggctttcgtacagcgagtcagaacgtcaaaattcgatcgaataataggctctgcctgtaactccatggccagtctggcgcttgataccacggcgggcacgtgcagcgaggcgacacggcctgaaagcttgtaggcgatttgcgatgaggattcaatgatcgtcaggtctggctgagatggcatggaaccgagcatctgtataacggtgacatttttacatgacttcggcgtcatggttttgctcatctgatggattgttcttccccaggcaacccccagcacatcaccattctcaatcacctgattcagatacatgccaccggcacgtgaaaggcgagtccgcatcagctttgtatcatcacgttttccggcatgttcgccatccggcacgatgatcactctctggagattgaatttatcgcgaatttgcaaagcagcgtcgatagagccaaagacattcacatccaggttgatatgaaccagtccattttcccgggctgtttgcaggtatttgacaaccgtgacgcgggacacccccatgatagctgcaacttcagtctggcttttgccttcctgatagtacagccatgttgcatgaagtacgggatcatcattgaacaggctgctgtttgtttgatctctatccacttttgtatacctgtattaaaccggggaaatgctcatcttaaccctgtttacccggagagttgatgcagattgccagtggcatgattttatacagatattttattcttttacatgaaataaaccagcataccatttgagcgatcgcccgctgttcccccatactgtaaagccggagacatgctccggctttacagtattactgagaatacacccatcaagcataatcgaaggttcaatatcgcccctttttgatcgccagcgattcgtcaccgtgcagacggttgccgtcactcactaaattatgggggacagtgaacaacaggttggctcactggcaagaacccgattataaaactaagctggcgagcagaataaaaatcagcccactgatggataagagtgtggacatcagcgtccaggataacagcgtttctttggtggtcaggccaaaaaagtctttaatcatccagaaactggcatcgttaacgtgagaacaaatacaggatccggcaccggtagccagcgtaatcaaggccaggttggtattgggatgtactgccaacaatgggatgaccagaccggcggtagagatcgccgcgacggtggctgaacccagacaaatacgcaggaatgcggccacgccccaggccatcaggatcgggttaatatccatacccgaaaccagggtggaaatatactgaccaacgccagagtcgatgagaacttgcttgaatgcaccaccaccaccgataatcagcagcagaccggcaatacccgcgatagcttttccgcaagaatccatcaggtcagggattgttttcccgcgccccaggcccatggtatagatcgcgaatagcagtgaaatcagcatggcgatcgttgaattacctaagaacagtatcacgttgtaaaataagcctgaatccgcggcacttttggcatgagtcatctggatgatggtgacaaccgccatcaggatcaccggcagcattgccgtgagaaaactgatcccaaagcctggcatttcgctttcgctgaatcggcgggtcgcgccgagagaggctatattcccctcttttttaaaggcgtccggaataatgcgctggcagaatttattcaataccgggccgcaaagaataaaggttggaatgccgacaatgataccgtatatcagtaccaatcctacatcagcgccatattccctggcgataacagtcgggccggggtgcggcggcaaaaaaccgtgtgcgaccagcaaaccagaaagcatcggcacacacataaacatcggtgatatttttgcttcacgggcaatagcgaataaaataggtaccagaagaattaaaccgacttcgaaaaaaagtgcgataccgacaataaacgccgaacagaccactgcccagtcaagtttatttttcccgaaataattcagcatggtcagcgctattcgctgcgcaccacccgcatcggccagcaagcgaccgagcataacaccgaagccaaatatcaaaccaatatggcccagcgtaccgccaagtccggattcgactgaggtgacgactttactcaaatccataccactggcgatggcgacagcaatcgagacaataattaacgaaacaaacgtattaagcttaatttttatggttaaaagcaggagtaaagcaatccctgccacaacgataattagtggcataacgtcctctcataacagggtagcgacccatcattatccgactgagcaaataacgaatgatgcagagtcggataattcaggtgtctggatgtttttatttatgctttcagtttttattcataaaatcgcgcaaagccgcgccaattttgtttacatcataaatacaaccggtccatgtcccaccactcacggcctgaagcattgcccatagccgggtatcatctggcaattcaggatcgggaagtaaatcctgatggctgggtctggcatttaatattgcagttgcctcctcctgtgaaggtaattgttcatcgctacgggttccgaggaaattgacttcgccgtgaagctcgcgacaatcaattttaatttcaattaaatccccggtgcgtaatttaccgatggggcctccggccagcgcttctggccccacatggccgatgcacgcgccagtagaaacgcccgagaaacgtgcatcggtgattaacgaaacatgcttaccgtatgacagatgcttcagggcactggtaacctggtaggtttcttccatccctgtacctgaaggtccaacgccaataatgaccagaatatcgcccgccttgatcttgtcatgtttgatatcgtaaatcgcacttttctcggacagataaaccttcgccacacctttatggtaatagataccttgctcatcaatcatcgaggggtcaatggcggtggatttgatcaccgaaccttctggcgcaatattgcccaccgggaaggtgatagttgaggttaatccgcgcgcttttgcttgctgcggagacatgatcacttcgtcagcgttgatttgttcctgatcgagcaggagttgcttgaaccgctgacgccgttcggagtgctcccaccagtcgaggttttctttcagcgtgctgccggtaaccgtcataacgtcttcatgcaacaatccgaggctgcgcagatgcaacatgacttccggcacaccacctgccataaaggcattgaccgttggatgataaaccgggccattaggcagtacgctcaccagtcggggcacgcgcttgttgatgcggatccagtcatcaacggtcgggatatggcaacctgcctggtgagcaattgccgggatgtgtaacagcaggtttgttgaaccaccgaacgcggcatggaccgtcatcgcattctctatcgctttatcggtgagaatttcccgggtggtgatgcctttttgactcaggttcagcgcagctcgcgcggaagctctggcgatctcccgccacacaggctcaccggaaggggccagggctgaatgtgggattgccagtcccaatccttcggccaccacctgagatgtcccggcagtgcccaaaaattgacagccgccgccggaagaggcacaggctttacagcccgcacggcgtgcgtcctgtagagataattcgccattggcgaagcgtgcgccaatggtttgcaccttgccgttgtcttctccatcctttgcgggcagcgtcgcgccgccggggaccagcacggttgcgatgttgtgctgcgcggcgagtgccatcatggtggccggaagccccttatcgcaactcgccacaccaataactgctttcgcgtcgggcagagagcgaataaggcggcgcattaccatcgatgcgtcatttcggtatggtagcgaatcaaacatccccgttgtaccctgagtacgcccgtcacaaggatcggagacgtacacggcatagggcagggcatggttggctttaataacctcggccgccgctttcatctggatgtccagttcgtaatgcccctggtgcaacgccagcgccacgggtttaccgtctgcgccgcgtaagccaccgagtgtactgagcagtaaaataccgtcccgatccagctcgtccggagaccaacccattccggcattcatggtcataccgaacagatccccgctcgggcggttgataagcatctctgcggttaatgggagttcgccgtccgggccatcggcgtgcgttctgacggtgtaaatatcgtggctctcgtcagcaaaaatattgcgaacagacatgagtttctcctcagactggtaaaatgccctgcgcggtaagcagcacgtggactttatcttttgcttcttcagatgcttcaagaatcggtggtaagcaatatgtctctacaggcagcccgacacactgcatgctgtatttgatcagtgagacaaacggtgtttcgagggcgtaaatagcgggcagttgtagtagttttttattcagcgtcgcagcggtcgccagatcgccttcacgccaggcgcggtagatgccgacggagagttccggagcaaagttagcgctggcggttatcgcaccgtcgccgcccagcagcatcgtattcagcaaatgatcatcgtaaccgcagaataccgaaaacgacgggcgtaccgacttaactgtgttgatcatcgtacgcaagtgaccaacgctgtcgatggtgtctttgatgccaacgatattctcgttttgcagagccagacgcgtcacggtttccggggttaagtcctgacccgtcagatccggaaagttgtacaggatcaccggtagggtgacgctacgggcgatctgctggtaatagtcgtcaagatttcgtggtgcgactttccagtagtaggggttgatggcgacgataccatcagcgccgtaggcttgcgcatgctgcgccagtttgaccgcttcgtcagtggaaggggaaccgacgccaatcaataccggcactcgcccgtcgacaatggttacagcttcttcggcgagtgccatgcgctgggctgtattcatttggctaaattcaccaccggtacccagataaaacagcccgtcgacccctttattaatcaggaagtcggcaacttcgcgcattgcctttttatcaagggttccgtcacgatgaaacgtgctggataccggtggaataatgccgctgaattttttcattacctcagtttccttttcgtaagtgctcattttcgtttctgtatcccagcccatatgatatttgctcagcgcatttccggagcaattccagatagctgtctatcttatttcctgaataaactaccggatcgccagaaagtgagattgcatagttaactctgttatacatattgaataccggcatacttaaacataccgccccataggttgattcttcgttgtctatggcccatccccgaaggcgtgttttttgtaattcttccagaaacaattttttatcggtaaatgtattgcgcgtatgtggagttaacgtgagtgcttctaaaaaataatccagttcttctcgtgtcttccaggctaataatgccttacccaacgcggtaatatgcaactcaagttttttgccaatccagcttttgctcgtcggtacagagtccggactttcgatcttgtcgagatagatagccgaaatgctctccatcgccccaagatgacaaaccagtccacttttcagcgacaactcctgcattggccgcttagtcacctcaaatatattttgacggtgtaacgcctgacaacccaattcgtagttttttattcccagtgaatagtagccgtttttgtttttaattaagaaaccacaatccaccattacattcaataaattaagcaggctgcttttggggtactggaatttatttaataactccatataacttgccataccaacccatgcaatgtgggttaatattttttcagcacggactaatgaattacaccctttgcgaaccataatggctcctccttgctcatggaataaatggtatcggcattacatagtggaaaatatgctttgttcagcatgctgaaccgtaatgatgtgattaaatgtgatcttgtacacactttgaataatgaatccagaacagccacatttagtgaatgagaataaaaagtagatggcgtgttgttgcaacatcgtagtgtgtggattgcgcctagagcttctttattcgttcgagcgcatcgccaatattttctattgggtgccattgattatttttgcttgaaatccctctcgaatgaacttacttatcactttattgaatgaggtaaaaacaactgacatccggctcgctgataacgctgtgcaatagtctcaggtaacccgctgtcactgatgatcgttttaatacatgatagtgttgctacagcatgcggctcaacggcatcaaattttgagtgatcggccatgagaataacttcacgcgagcgttgaataatccgtgttttcaccccgacctcaaacatggtggcattggtgatccccgtctccagcgacagcgcatcgcaggagataaacgcacgttctacggaaaaggcattgatcatctccagcgccagactctctcctaccgaaaaataacctgggcgaatcagtcctccgataatgtaactttccacatggggaaaacagcccagttcattggcgattttaatgtcgttgcagatgacctttacccgcgcatcggccaggcatttcgccagttcgaggcaggttgagccggagtcgagaaaaaagcagtcgccatctttgatcattgttcgggcaagggcagctatttctcttttcgccacagattgcaatgtacgtttcacgtcgaagacgtactctttgtcgtctgtactgtcgtcgaagtccaggcaaccgtgaccgcggatcatgcctggatactggttgacaatatactggaaatcacgacggacagtcgcttccgcatagccaaaaagctccatggcctgctgtgtggagaggtgacgatgttgccacaggtagtgcagcatctgtttgatacggtcaggtctctgttggctcatcagaaacaatctcctcttacagggtggcgaattgagctaaggtcgcgcgatagtcagatgaagagaacagggcgcgcccaatcaccatatgttgcgccccagctgctgccagttgctgtgcagctgccagcgtaattccaccgtcggcccagcactcggtctgaggaaaagccgtgcgtactttttggattttctcgcacatggagggaataaaccgctgtccctgcccatcgggctcactggtcatcaccatcactccgtccagctcagacgccagatatcgccaggcgtcgatcggggttgccggattaaataccagtccggctcgtgcgccggtatggcggatctcagttaacgtttccgaaggatagtccagcgtttctgcatgaacgaagatccacgcgggtctgatttcagccagcgcgttaaaccagcgctgtggccgggcaagcatgaaatgaaaggacaagggatgaggcgtctgtctggcgacggcctgcaccgttttcatcccaaacgtaatgttgttaatgaagctgctgtcctcaatatccagatgcaggctcccaaaatccagattgtccaatgccgtcagctcacgaccatagtgcagaggatttgcgctggcgagagaagggtgcaggatcataagcgcctccgttaacctgataccagcgcaaacagtgcatcgtctgtgctggcatttcccactgccgttaagcgttgtggcgaatcaataaactggctgatgcgctgaatggtcaaaatatgtgcgttggcatccgtggcgctgacgcagagaagcagccagacggggtcgcactcctcgttaccaaaggcgaccggggtgcgtagcgtggtgatactgacctgattatagtttgcgccttgctctggtcgggcgtgaggcaaggcgattcctggggctatcagataataaggcccccagttaagggtattttcgatgatcccattaacgtagcatggctgcgcggcaccataggctaccagcgggcgggtggcgatttccacggcctgacgccagtcggtggctttacgttgtgcctgtacccatttaatatcgttaatcatccgtcgttgactccatgccgattcgggttaatctggtagcgatccccgtcgatacttttgacgaaggcggcagggatcgcagaagggttattgctctttgccggggataagcgctctgcttatccccatcttatcggcgtatatgatgcactttctccataaactgactgactcgcgcctggtcaacgaaattggcaaaaacgccgtcctttttaaaggtggttgcggtcacacagccatcggcgatactgagttgttcctccacgttttccaggcagacgcccgtgttggccaacacgacggtgtcaggcaccgtttctttgacccgttttaacagcgcgctgtcggtacgcgtcccggcggtcaggccagaaacacagagcgcatcaggatggttgttaaatactgtcgatttagcaatagaacagatatcgcgattgcccagatacacggcggcctctgggacgatattgaacaaggttttcacttcgcctgcaccaatccggtgttgatgacggatggtctcaccgacgttagtgtcccagacgccaaagtcgctggcataggcaccggtaaatatctcgcggataaacttagcgccggtagccatcgccaggtcgaatgaggcgaccggatcccacagaacattcacgccaaacgggatgcggatatcgctcattaattgcccgatgattcgtgccattgccgcagtggtttccggacgcaccttcgtgagatagggaagactaaactcgttggagaacatgactgcatccaccccaccattttggagcgccatcagatcgtcccaggctttgtcgataacccagttcatccccaactgcgcatcaaaactcgggtcgccgggcaatgcacgtagatggcacatggcgatgaccgctttttccgtcccaataacctctttcagccaactcattgaaagtactccttattccgataattcacgtttacgtaagaacagcacgacgctggcgacaataccgaccgccacgacaacgccaataatcccaagcgacatcaattcagaaatcgaccaaccgaacatattgcccacggacaacgctgagatttgcgcactttcaccggcaaaactgaaaccgcctttgagcgccatttcagtgaagtaaggcgcgaactgggtggcgatcagcaggacggtaatcatcacgatgaccccgcttatcaacgtcctgaccaggtctccgcggtggataaccgtagccatacagataaagaacggtgctaccggcaggtctgcgaggggtaacactttgttgcccggtaaaatgctggccagaattaacataatgggtatcagtagcagaccgacagcaatggtggttggatgccccagcgtcacagcagtatccagaccgatatacacttcacgtcctttgaaatatttctggaagaactttcttgcaccgtcggagatgggcagcaggccctcaacaatcaggcggatcatgcgcgggaacaacaccatgattgccgcaacggtaatcatcagactggcgcaacctttaaagccttcaccagccgccaggccaaaaatcagaccgagcactacgccgataatcaccggatcgccgaccatgccgtagcgtttctggatctcctgagcatcgatattgcgtcccttcatgaaagggattttttcatagatagcatcaagtagaacgaaaagcggtactgaactggaaccgtagccttgcggtatcgaaataccttccagcccgacgatgttctgtacccgttttgccgtccagtcggccatttttaacgatagcgccgcatggcagattgcccccagcacaccataaatcaggctaccggtcataagctggaccaccgtacccgtaatggcgtagtgccagtaattgtaaatatcgacgttcatcgttttggtcagacgggtgaccagcatggcgacattgagaagaaaaataactgggataatcatggcgccaatggctgtcgcataaccaacgccggaggcagggcctgcgccaacgtcaaagacatgcagggctaggccgaaacgctcaatcatcactttgatagggggactgaggctgtcgatcgccatgacgatcaccagtcccataccgacaaaaccaatcccaaccgttacccctgccttaatcgcctgcagccaggggatgcggaagataaggccaatcacgatcatgatgatagggacgaaaacggtaccgccgagagacaggatgtaatcaaacataatgcctccttttattgagttaacagagccttgatttgttgttttaacgcgtcgtcgttgatccctgtgagcagggcggcgccattaagcgtagggatgccgtaatcactgttggttcgcatggaggttacaataaggtccataccgttacagttaagagggatctcattcagacagcattgggcggtagtggctgaaatgccctgttcagtcaggaactcttgcagcttgtgtgcaatcatggttgaagtcgacatgccggtaccgcatgccacaaggatctttttcataatggatgtgcctcttgtgtagtgcctgaatcaggctcaacggggaaatgtgctgctgacatacctgccagagcggtcaataggcggatgcaatcagtcaaatcacgcaggctggcaacctccgccggagaatgggtatagcgacaaggaatagagagactggcgcagggaataccatcctgctcaacctggatataaccggtttctgttatcacgccgggagccacttctcgctgcaccggaatgttgtgttcaagagccgtctgttccaacatccgtatcaggcgaggaggcgtgattaatccggccagcgttccccgaccatggtagttcaggcaggtgatcccaacgccctgattaatcctgacctcggaataatcgtgtaaatcaggggtgtcacacgatggagtgatatcaataccaatcgccaggtcaggttttacacggcgtaatacgggaacaatgccgcggatattaaattcttcctgtaccgaagccaccagataaacggcgatatcaagctccatagtactgatagcatccgctacaccgagcagggcagtacagcctagacgatcgtctagtgctttactgcacaccagatcgtttgccaggagttgcggcgggttatacagagtgacaggcgtaccgacctgaatgcccatccgtatagcgtcgtctttgtctttggcaccaatatcaatccacagtttgtcgacagaaggtgactgcgtgcgctcgtcgcctttggcaaagtggtaggacttaatgccgatacaccccatgactggccctttgtccccggtgagggtgacgatggaaccagccatagtgacctgcgcaggaccgcctacgcgttcaaagcgtaaaaatccagacggctctattttgcgcaccataaaaccgacttcatccatatgcgcaaaaatcatcagtcgcagcgcatcgggtttatcactaccgtagcgcgcgacgacattcccaagcctgtctcgccagacctcttttgcctgacgcctgaattcgcacagcatgacgtcagcgacagcgttttcgtgtcctgaaatcgcattgtgctgcaaaagcgagaacagggtttcctgcacagaaaatgacatagctatctccgtagaccgtaaaacaatcactcgttgagcgttttataggcgcagactggtcgaataattgtgagaacgttcacgtgaaaacgcgcaaagctgaacaaataaaaaattatgtgagccgagtggaataaaagcgctcaacgtttgtgaaagttacgggctggagagaccagtgattatggttgaaataatgaggatgaataaaacgcggtaactgttatagcaccactttgttgcaggacgctccctcttcattacgtcctgcacgtggataccccagcatctccatcagcggatcttagaatgtaatggcgcgtggcaggtcgttggttcccagcataatgtaagaaaacatcggatctcctgaatagattcagagggagtatagataatcagctcaaatcactctccgctttatgagcccaggctggcattgccgtcagataacgttttgcacgcttatgtgcttcctccgggccgactttttgccaggaatcaaggaagctggctaaacctgataccgcttcttcccagggtttgagattgccgttgctgtcgctgcattacgcacaatattgatcactggcactgtgtgcatctggtgccgacatcggcattccgcaagcctgacagaactgttcatgttgtgacatatgatgctccttatggtgacatcttgattaataaacatactgaatatgtattgtgcaggtgatacatcagatcaaagcaaaggtaaagcctcgatatttccagccagaaataccgggaacctgttgttaccgggcgatgagtgcgaacacgccccagccaaagcattcccgcgcgtaggtcacgtagcgtttcggcgcgatgtttagttcggccctgacttcggcggcgaagtcatcgtcaggattcgcttccagccagcggcgcatggtcagccattttgcggcttcataccggtcccagccttcctggtctgccagtaccatttccaccacgtcatagccgagatcgtcgaacgctccgacaagtcctggcagcgtcaggaaatcgcttgtcgagctgacgccgcaggcctgggctatttcttctgttgctggtagctgacgccagtagggttcgccgataagcatgatcccgcccggtttcaggctttgcgctagcagctcctccgccccggcaaacccaccggcaatccatgtcgcgccgacgcaggccgccacgtcacatttttcatttgcgacgtaaccggccgcatcgttatgaataaaatgtacgcgttcgctgacgccgagttcttccgcgcgacgctttgcctgcgcggtgaagagcgaactcatgtcgatgccagtccccgtaatgccatgatccctggcccaggtgcagagcatctcgcccgagccgctgccgaggtcaagaatgcgggtgcccggcttcatgcgcagcacgcgacccagcgtggcgtacttctcttcggtgaacgggttatggatgcggtgttcactttcgctgatggtaaaaatacgtgggatatccattatttaattcctgttattgggttaagccttaaaaaggacacaacaagattgttattcacgtcagtgctccggtttcatcagggtctgcgcaccggatgtggccggtcagggtcatgggctgagcggtgagtgattgcatcatccagcaggctttgtgctcctccgggatgggataaggtgccggatagcctttgtctccggcacagggttcgaacccatgtcgggggtaataggtggcgtggccgagaacaaaaaccgtctggcagcccatcaacctcaggtgctcgatgccagtgcgtatcaaccgtcctcccacgcccatcccttggtattccggtatgaccgccaggggagcgaggatgtgcatcaacggtgaatccatttctcctttgaaggttgcccgggtaaataaaatatgcccgacggctttgccttcataccgggctagcagcgataacgcggggcgcgcgctttcatcctcaagtaaagaggccactaaatcggcttctttgctgaagccaaatgcgcgggtttcgacttcccggatatcactggcatcacttttatctgtgatatgaaaagtgaagtggtgtactgtcatagaaactctccttagcgattatcgagctgagcgcgaactttattcagctcggtggtgttgattcgatagggctggccattgacggacttgataagttttttggttttgagttttttgaagacggcgagcgtgcagtcggtcagcaacagcccttcgcggctgtagcattcaacggaagtgacgcggcctgaagaatcgcggacgtgcgcaatacgtctacctttagcgagaacgtgtaaggtatgttgttcctgacgggataaattcatactgaagaacctatttaatcatcatgtgcaaaacgtgcaaacacaccgcggtgtccgcattcgatttcggcgcattgataatcagtccggcctgaaaaggtcggggaactgattatcggatgattacattctccagcatcaaagcctcgggttgagttgaaaggtatttacggagcgaatattaacacgtagttataggagggatatgtttcagtagaaaaagtgtgatgtactttggaaattgaatgccaacccatttactggaaaaggcagatgacactgacgaatgcatgttgaagtacgcctgaaatggcctcatcggcttttcccttcgggagattattctccttttgttaaatccagaacataaatatgctcacccatcttcgatgcttgaaaaattgaagccaatcctgataagtaatttttttgaaagggtattttccggattcacaccggctttgatgagtgaaaaaccgttctcttttattcagtcaatcgtggcggtaattgcttcaattgcatatccctggcgagcataagcgggactgatggtatagccgagccaaaacacatcgcattgctgacgtaaatagatatcaccaatcaaaacctgcgtcatttgttgacaatggccaattgaatatcgcgagcaagtgtaagaactcccagcaagaccctgtaaataattctgtgtaactgcccacgattaaaggtggccgctcaggcggtcaccgtattcgataataaatgggtctggaaaaagtgcagcatctggcagcgtaatgcaggtagcccagttcaactctcactaccagtatgatcccaagttcgagcgcggaatgtatctgtatgagcatcgtcgctgtttcaataacatcatcgactactgtaactcactttgctatcacggtaagttgcagcctaaaagagggatggaaaaaggacgattttccccgcaatgggatatttacatattgatggtagaggcatgaagccaaatggagggagccgtcataaccctcttgaagctgaaacaatagcagcatggctggtggcacataaggatgatatagagcgccattacggggaaccactgtacaaagttgttggtgttgtgacgccattttcggcgcaggttaatgctatcaaaatgtcattgcgtaagctggaaattaatggcaaagacgagcagggtttactgacagtggggactgtgcactccttgcagggggcggaaagggcgattgttctcttttctcctgtctactcaaaacatgaagatggcaggtttcttgatagcaacagcactatcctcaatgttgctgtctcacgcgctaaagatagttttctggtatttggcgatatggaccttatcgagatgcagcccgcattttcgccgcgagggttattggcaaaatatctcttttcttcagataataatgcgttgcaatttgagtttcagaaacgacaggatttaatttccgcacatacacaaatttcaacgctgcatggtgtggagcagcatgatgaatttttgaacaagactcttgccggagctcaaaagaaaataacgattatttccccttggttatcctggcaaaaagtggagcaaacgggatttctggcatcaatggctttggcccgttcccggggcattgatattaccgtggtgacggataaaaactgcaatatagcgcatgtcgatgatgataagcgtcaggagaaacaacatctgctgaatgatgctgttgaaaagctcaataagatgggtatcgctacgaaattggttaatcgtgttcacagcaaaattgtgattgaggatgaagaactgctgtgtgtcggatcttttaactggttcagtgctacacgggaagataagtatcaacgatacgatacgtctttggtgtaccgtggtgaaggcgtaaaaaatgaaataaaggcaatatatggtagtctggatcaacgtcagctttaaatgtgatgagccgttcatgatacaggagtagtaaagggcatattttaccaatgttaaggcgactttccgttttattgcgagtcgcctttcctgattataaatcttattgtttacctaatcattttcctttgcataatgcgcctgggattaatggcgggtgcttttaggaatgaaagaaaatgcaagcaataatataataatggcctaatttctttgaacatcattaagcatatcatcatcgtctatttgccagaatccgtcgacttataatcgccagaacggcatatcaggacggtgctgcgaacgctgtggcccaaaacgttccagtaaactgtgtagatgttcgtagatttccgagccataatcgaaaaggcgcggatgtctattaaggcatccggctaatctgtaagcaataacaacggtttatgcggtgcgcgtttttcacccttgtgccagattattatattggcaattgcctgctgttcgagcccgcaagtgaagagatattaccttgatctcatttgttttttgttgtctactctgagaacgaacaaggacatcccccatgaataaactccccgctcacctttcgcgccaaaactgcaaaattgcttctacaaatctgtcagaaataatcccccgacgggctgcagtgctgaaatgactgcttcgcagtgccgtcgtccagttctccggtgaccggtacgctgaaccgtaatatcccgtgcttaaatcgtccgggtcttcatcaggcgcgttcgtcagtcctctttcaccttgttgctggaagtcgacgaaaataatattggctaaaacattattttgataattgccataaatagcttcatacgaatgcgggaaattttctttccagtaccaggtggtatcgccgcaaaaccacggcgcgtcagtaatattattaagctgagaatggtattgttttagatccctacgaaaggcttcaaccatatgattaaagtgttgagggtgtgacgcgtagtcactggtcattaagtcaaattcgccttgcatccagcatgcgccgaggaatttgttctgcggattttttgccagtgcggctcgcgttctgctgactaaatcctggtacagcggagtatccgttccccaacgacaagcatcatggctggctccgtgccgttctgaatatgtcccttcgctgcccgcggtaaaagccgatccgccacggcaacacggaacgataagaatccctgcattatcaggaatgaagggcagtaatttccgtgcaatatgcagtgcctggccaacggtgccgtactgtgtttgatgattcgttgccagaggatggtgataaccctgcatatcctgaacatcgtgtgggcagtgagtcagtggaataatgtcgttaaagtgacatggcgggcctccgggatgcgtatgcgcaaatctcgctaattgtttaattctgggatgaggcgcatcttccctgtccggtaatggcagtccttcgccatacgccatggcattagactgaccagcaacggtaagaacatagtaataatcgggcgatattattgcgttcatataaatttcgcgtaattgaaatgacaaattgatagcagggcccctttaccggggccctgaagcgttagttttgtactgtgactttattatccttcacagtgatcaaaactgaatccgtcaccgctttgccgcctgcagtttcaccgccaataatcaatagactattattccagggcaatgatactccgtaggcccgaccttgcgataattcacccgatttatcccatttcccgttatgccaaagatgaatatcagtgctatatgattttttcaggccttcatgcgcatagttcttaccgttctggtaattttctcgtgaacctttgaatccggcccctccggcaaatataagagaatcattgcttatccccgcaaaaccgccagctacgccatctggtgatgagacgggagcaagcttattccattttaaattattaccggtgaaatcaagttcaaatacggcatccgttcgcaatcctggtttggcttcgccattaataagccaggttttatcacctttattcacaaccgccgcaccagccgttccgtaccagggcgattcgccagcgtaactccattgctgtgttgagggatcaaaagacaacagaaacttattgaagaaataatcttctgcttttttgtcaaaatagtgagcattgattttatctatagcggttgaatcttttccagcctcgttgagatcttcaaaatagccattgaagatattctggttaacaccaccagtaacataagccttgccgttgtgtacaaaagtcacatggcccgccatgcccatcggcgcgtgcgacatcaatttaacccaactattggttttggggttgtatttgtgtacgtcattaaatacctgagtcaagccctcgctgtttttgccaatgccgccaaacacatacagattgccatcaataaatgcagaggttgcttgatctcttggtccgccagggaatgcagctaacgctgtccattttttatctttggcctgtgtatccagcttgtaccatgccgtacctgcgctacctaaaccaatgtagacagtgtcgttatcaattgctccggtaccacttttaaatggcacaggagtttccggtaatacagacgcgtttgcggcaaatgaagccatcatgatagcaagcgccgttattgttttattcattgtgactgtctcctgtctactacagtttaaatgacacaccaatgcgataactgttttccgataaattatctctgccgttgtaaacaccctgacggtcaaggtagtcatattctatgtatggcgtaatatcgggcgtcatatggtattgtagaacaaatgcattttccgtcgcccatttcttatggtttgcatagcgataatcgttctgtttgctgtatagcgtcgtttgccatgcgaaggtgaaatcactattaatatggtaagtgacatatccatcccaacgatgaacgttatcacgagacatatcaccggataagtcttgttgtcggtaagctttccagtcgtaacgatagcgaatgccaaaattaagatcttttgtcgcgtcccaggacagttttacgtagggtccgtagcgtgtgccgttgctgctaaaatgcgttaacattcccgggcgcaccgtccattgatcatcaagtttaatcgcgtaattaacttcaacctgaacatcattgagtgcggcattttcctttttattatcatgaatggtattccaggtattactttccatgcttgcccaccatccattttgccatccctcactgactttgagtcgagtctcataggcgtggcttccactacgatatccaccacgtacgtccagtgtcgcagcctgagaaattaatggggacgaaaagcacagtaataatacgccagaaagtattttagcctttttcataaatttcactcatttgtaggatacagaaagcaatacaaagcccgcataaacaattagcatttatgttgtgtaatatttttttgccaggcttatagtgtctttggcaaccggtagctgtattttatatttttttgtataaggtctcctgtgaaaaatctcttttcacattatttaaataaacagagatccagattaaatacctgagtataaaatctcttctgatgtttaattgatttgaatgttcgtaagctatatcacttactcaatccattttacccagagtcataaaatagaatgtctgttgatctcattttcatattcctttcagactgaagtgcgttttcatcacccgatgagaaagaactgaagtgatgtttgccatagattgcgagatgccctgtctcattgactatcttggtgcacctttatacctgttataccagatcaaaaatcacgcaatccatacaacaaaaccagatttgcaattcgtgtcacaaaatatgtcgatctttttctaagaggaagatgccatgtgaagccagacgaacacttgcggtggtcttcaaaaactaaagatcttagtttaactatttgttttataaataatttattaagagtctaaacaaggggagctttgcaagctaactcagtgagcttggtgaaaatcagtgtttacccgccatcaggctgagcataattctcatcatgaaatatgtttcctggtttgtggcttgtaactggtcacttctgaagtcgatctggagaggcttgttgatgttggtgttttcaggatgatgtttcacttagtttgtttgccgtatcgcccggcgaatggctgtgattgaggaaggtttaagtcgtagtgaccaaagctatatttaccaacgaatgtagatgaaaaaatcatctcctgcgttcccccatatctctaggataaaaaggaatgtaacaatctcatggcgtaagctgacgaatcagcaggaataatcgctagggacctaagaattagcatgataatagccactaagaaattactgcgctccatgaaatagccattttgtggcaaatggagttgactaataatgtcatatgtgagacggctagttgaacgaatattaaattttgctgaattttttatgttgattttacttgttacagaacatatcacatgatatatagataagattagttgcattaatgatgagggttattattagattcgtatccgattgataaatatataaaggtacatagcatgcaagagcatggcgtttgtatggcaacgttattataattaacagttgctactccatttaagttcactcagaagaactggtccacttacgttagttattaagcaaacgttcgcttttataaacataatcaggataaaaatgttggattattgctaacccagcacagctagtgcgcgtctgtaattataagggaaaaacgatgaagaataaggctgataacaaaaaaaggaacttcctgacccatagtgaaatcgaatcactccttaaagcagcaaataccgggcctcatgcagcacgtaattattgtctgactttgctttgttttattcatggtttccgggcgagtgaaatttgtcgattgaggatttcggatattgatcttaaggcaaagtgtatatatatccatcgattaaaaaaaggcttttcaacaacgcacccgctattgaataaagaagttcaggctttaaaaaactggttgagtatccgtacttcgtacccgcatgctgagagcgagtgggtatttttatcacgtaaggggaatccgctttctcggcaacagttttaccatattatctcgacttccggtggtaatgccgggttgtcactggagattcatccgcacatgttacgccattcgtgtggttttgctttggcgaatatgggaatagatacgcgacttatccaggattatcttgggcatcgcaatattcgtcatactgtctggtataccgccagcaatgcagggcgtttttacggcatctgggatagagccagaggacgacagcgtcacgctgttttatagagatagttgagataccagggatggtgttaaaaactacattattcttacgatatatcaaaaatgattaaccatttattaattgatgttattgtaagtgtgattcttaattatcataataaacattaagttaaccatatccatacaaaatacaatggtttatgttcttcaaaataaataaacaaaatcattcataaatttacacatcacttaaaatctcctgtttccgcacttttttctttattttttaagcaactggaagttaatccactgcaatctattgttatattgaatcaaatcaatgaaaatagatgttgtcacatcagtgatattttatttttgtatgatatttaatgtaattgactgatagccacatcactccgtgtgtggttatctttttatctattgggctaattttgaccgattgaggtttcctataggtattcattcaaatatatctcagttaggagtactactattgtgagtaaacgtcgttatcttaccggtaaagaagttcaggccatgatgcaggcggtttgttacggggcaacgggagccagagattattgtcttattctgttggcatatcggcatgggatgcgtattagtgaactgcttgatctgcattatcaggaccttgaccttaatgaaggtagaataaatattcgccgactgaagaacggattttctaccgttcacccgttacgttttgatgagcgtgaagccgtggaacgctggacccaggaacgtgctaactggaaaggcgctgaccggactgacgctatatttatttctcgccgcgggagtcggctttctcgccagcaggcctatcgcattattcgcgatgccggtattgaagctggaaccgtaacgcagactcatcctcatatgttaaggcatgcttgcggttatgaattggcggagcgtggtgcagatactcgtttaattcaggattatctcgggcatcgaaatattcgccatactgtgcgttataccgccagtaatgctgctcgttttgccggattatgggaaagaaataatctcataaacgaaaaattaaaaagagaagaggtttgatttaacttattgataataaagttaaaaaaacaaataaatacaagacaattggggccaaactgtccatatcataaataagttacgtattttttctcaagcataaaaatattaaaaaacgacaaaaagcatctaactgtttgatatgtaaattatttctattgtaaattaatttcacatcacctccgctatatgtaaagctaacgtttctgtggctcgacgcatcttcctcattcttctctccaaaaaccacctcatgcaatataaacatctataaataaagataacaatagaatattaagccaacaaataaactgaaaaagtttgtccgcgatgctttcctctatgagtcaaaatggccccaaatgtttcatcttttgggggaaaactgtgcagtgttggcagtcaaactcgtttacaaaacaaagtgtacagaacgactgcccatgtcgatttagaaatagttttttgaaaggaaagcagcatgaaaattaaaactctggcaatcgttgttctgtcggctctgtccctcagttctacagcggctctggccgctgccacgacggttaatggtgggaccgttcactttaaaggggaagttgttaacgccgcttgcgcagttgatgcaggctctgttgatcaaaccgttcagttaggacaggttcgtaccgcatcgctggcacaggaaggagcaaccagttctgctgtcggttttaacattcagctgaatgattgcgataccaatgttgcatctaaagccgctgttgcctttttaggtacggcgattgatgcgggtcataccaacgttctggctctgcagagttcagctgcgggtagcgcaacaaacgttggtgtgcagatcctggacagaacgggtgctgcgctgacgctggatggtgcgacatttagttcagaaacaaccctgaataacggaaccaataccattccgttccaggcgcgttattttgcaaccggggccgcaaccccgggtgctgctaatgcggatgcgaccttcaaggttcagtatcaataacctacccaggttcagggacgtcattacgggcagggatgcccacccttgtgcgataaaaataacgatgaaaaggaagagattatttctattagcgtcgttgctgccaatgtttgctctggccggaaataaatggaataccacgttgcccggcggaaatatgcaatttcagggcgtcattattgcggaaacttgccggattgaagccggtgataaacaaatgacggtcaatatggggcaaatcagcagtaaccggtttcatgcggttggggaagatagcgcaccggtgccttttgttattcatttacgggaatgtagcacggtggtgagtgaacgtgtaggtgtggcgtttcacggtgtcgcggatggtaaaaatccggatgtgctttccgtgggagaggggccagggatagccaccaatattggcgtagcgttgtttgatgatgaaggaaacctcgtaccgattaatcgtcctccagcaaactggaaacggctttattcaggctctacttcgctacatttcatcgccaaatatcgtgctaccgggcgtcgggttactggcggcatcgccaatgcccaggcctggttctctttaacctatcagtaattgttcagcagataatgtgataacaggaacaggacagtgagtaataaaaacgtcaatgtaaggaaatcgcaggaaataacattctgcttgctggcaggtatcctgatgttcatggcaatgatggttgccggacgcgctgaagcgggagtggccttaggtgcgactcgcgtaatttatccggcagggcaaaaacaagagcaacttgccgtgacaaataatgatgaaaatagtacctatttaattcaatcatgggtggaaaatgccgatggtgtaaaggatggtcgttttatcgtgacgcctcctctgtttgcgatgaagggaaaaaaagagaataccttacgtattcttgatgcaacaaataaccaattgccacaggaccgggaaagtttattctggatgaacgttaaagcgattccgtcaatggataaatcaaaattgactgagaatacgctacagctcgcaattatcagccgcattaaactgtactatcgcccggctaaattagcgttgccacccgatcaggccgcagaaaaattaagatttcgtcgtagcgcgaattctctgacgctgattaacccgacaccctattacctgacggtaacagagttgaatgccggaacccgggttcttgaaaatgcattggtgcctccaatgggcgaaagcacggttaaattgccttctgatgcaggaagcaatattacttaccgaacaataaatgattatggcgcacttacccccaaaatgacgggcgtaatggaataacgcagggggaatttttcgcctgaataaaaagaattgactgccgggtgattttaagccggaggaataatgtcatatctgaatttaagactttaccagcgaaacacacaatgcttgcatattcgtaagcatcgtttggctggtttttttgtccgactcgttgtcgcctgtgcttttgccgcacaggcacctttgtcatctgccgacctctattttaatccgcgctttttagcggatgatccccaggctgtggccgatttatcgcgttttgaaaatgggcaagaattaccgccagggacgtatcgcgtcgatatctatttgaataatggttatatggcaacgcgtgatgtcacatttaatacgggcgacagtgaacaagggattgttccctgcctgacacgcgcgcaactcgccagtatggggctgaatacggcttctgtcgccggtatgaatctgctggcggatgatgcctgtgtgccattaaccacaatggtccaggacgctactgcgcatctggatgttggtcagcagcgactgaacctgacgatccctcaggcatttatgagtaatcgcgcgcgtggttatattcctcctgagttatgggatcccggtattaatgccggattgctcaattataatttcagcggaaatagtgtacagaatcggattgggggtaacagccattatgcatatttaaacctacagagtgggttaaatattggtgcgtggcgtttacgcgacaataccacctggagttataacagtagcgacagatcatcaggtagcaaaaataaatggcagcatatcaatacctggcttgagcgagacataataccgttacgttcccggctgacgctgggtgatggttatactcagggcgatattttcgatggtattaactttcgcggcgcacaattggcctcagatgacaatatgttacccgatagtcaaagaggatttgccccggtgatccacggtattgctcgtggtactgcacaggtcactattaaacaaaatgggtatgacatttataatagtacggtgccaccggggccttttaccatcaacgatatctatgccgcaggtaatagtggtgacttgcaggtaacgatcaaagaggctgacggcagcacgcagatttttaccgtaccctattcgtcagtcccgcttttgcaacgtgaagggcatactcgttattccattacggcaggagaataccgtagtggaaatgcgcagcaggaaaaaacccgctttttccagagtacattactccacggccttccggctggctggacaatatatggtggaacgcaactggcggatcgttatcgtgcttttaatttcggtatcgggaaaaacatgggggcactgggcgctctgtctgtggatatgacgcaggctaattccacacttcccgatgacagtcagcatgacggacaatcggtgcgttttctctataacaaatcgctcaatgaatcaggcacgaatattcagttagtgggttaccgttattcgaccagcggatattttaatttcgctgatacaacatacagtcgaatgaatggctacaacatcgaaacacaggacggagttattcaggttaagccgaaattcaccgactattacaacctcgcttataacaaacgcgggaaattacaactcaccgttactcagcaactcgggcgcacatcaacactgtatttgagtggtagccatcaaacttattggggaacgagtaatgtcgatgagcaattccaggctggattaaatactgcgttcgaagatatcaactggacgctcagctatagcctgacgaaaaacgcctggcaaaaaggacgggatcagatgttagcgcttaacgtcaatattcctttcagccactggctgcgttctgacagtaaatctcagtggcgacatgccagtgccagctacagcatgtcacacgatctcaacggtcggatgaccaatctggctggtgtatacggtacgttgctggaagacaacaacctcagctatagcgtgcaaaccggctatgccgggggaggcgatggaaatagcggaagtacaggctacgccacgctgaattatcgcggtggttacggcaatgccaatatcggttacagccatagcgatgatattaagcagctctattacggagtcagcggtggggtactggctcatgccaatggcgtaacgctggggcagccgttaaacgatacggtggtgcttgttaaagcgcctggcgcaaaagatgcaaaagtcgaaaaccagacgggggtgcgtaccgactggcgtggttatgccgtgctgccttatgccactgaatatcgggaaaatagagtggcgctggataccaataccctggctgataacgtcgatttagataacgcggttgctaacgttgttcccactcgtggggcgatcgtgcgagcagagtttaaagcgcgcgttgggataaaactgctcatgacgctgacccacaataataagccgctgccgtttggggcgatggtgacatcagagagtagccagagtagcggcattgttgcggataatggtcaggtttacctcagcggaatgcctttagcgggaaaagttcaggtgaaatggggagaagaggaaaatgctcactgtgtcgccaattatcaactgccaccagagagtcagcagcagttattaacccagctatcagctgaatgtcgttaagggggcgtgatgagaaacaaacctttttatcttctgtgcgcttttttgtggctggcggtgagtcacgctttggctgcggatagcacgattactatccgcggctatgtcagggataacggctgtagtgtggccgctgaatcaaccaattttactgttgatctgatggaaaacgcggcgaagcaatttaacaacattggcgcgacgactcctgttgttccatttcgtattttgctgtcaccctgtggtaatgccgtttctgccgtaaaggttgggtttactggcgttgcagatagccacaatgccaacctgcttgcacttgaaaatacggtgtcagcggcttcgggactgggaatacagcttctgaatgagcagcaaaatcaaataccccttaatgctccatcgtccgcgctttcgtggacgaccctgacgccgggtaaaccaaatacgctgaatttttacgcccggctaatggcgacacaggtgcctgtcactgcggggcatatcaatgccacggctaccttcactcttgaatatcagtaactggagatgctcatgaaatggtgcaaacgtgggtatgtattggcggcaatattggcgctcgcaagtgcgacgatacaggcagccgatgtcaccatcacggtgaacggtaaggtcgtcgccaaaccgtgtacggtttccaccaccaatgccacggttgatctcggcgatctttattctttcagtcttatgtctgccggggcggcatcggcctggcatgatgttgcgcttgagttgactaattgtccggtgggaacgtcgagggtcactgccagcttcagcggggcagccgacagtaccggatattataaaaaccaggggaccgcgcaaaacatccagttagagctacaggatgacagtggcaacacattgaatactggcgcaaccaaaacagttcaggtggatgattcctcacaatcagcgcacttcccgttacaggtcagagcattgacagtaaatggcggagccactcagggaaccattcaggcagtgattagcatcacctatacctacagctgaacccgaagagatgattgtaatgaaacgagttattaccctgtttgctgtactgctgatgggctggtcggtaaatgcctggtcattcgcctgtaaaaccgccaatggtaccgctatccctattggcggtggcagcgccaatgtttatgtaaaccttgcgcccgtcgtgaatgtggggcaaaacctggtcgtggatctttcgacgcaaatcttttgccataacgattatccggaaaccattacagactatgtcacactgcaacgaggctcggcttatggcggcgtgttatctaatttttccgggaccgtaaaatatagtggcagtagctatccatttcctaccaccagcgaaacgccgcgcgttgtttataattcgagaacggataagccgtggccggtggcgctttatttgacgcctgtgagcagtgcgggcggggtggcgattaaagctggctcattaattgccgtgcttattttgcgacagaccaacaactataacagcgatgatttccagtttgtgtggaatatttacgccaataatgatgtggtggtgcctactggcggctgcgatgtttctgctcgtgatgtcaccgttactctgccggactaccctggttcagtgccaattcctcttaccgtttattgtgcgaaaagccaaaacctggggtattacctctccggcacaaccgcagatgcgggcaactcgattttcaccaataccgcgtcgttttcacctgcacagggcgtcggcgtacagttgacgcgcaacggtacgattattccagcgaataacacggtatcgttaggagcagtagggacttcggcggtgagtctgggattaacggcaaattatgcacgtaccggagggcaggtgactgcagggaatgtgcaatcgattattggcgtgacttttgtttatcaataaagaaatcacaggacattgctaatgctggtacgcaatattacctgaagctaaaaacctgcacgttagccctttgtaggccagataagacgcgtcagcgtcgcatctggcataaacaaagcgcactttgctggtctgttcccctcaccctaaccctctccccggaggggcgaggggactgtccgggcacatttttagactttgtcatcagtctgagcctgccattggcaggctctggtgtccttttacgctaccatgctaataatcagcacaataatcagcccaaccacggagttgaccagctccagcagaccccaggttttcaacgtgtcttttactgacaggtcaaagtaacctttgaacaaccagaaagatgcatcgttaatgtgggtgagggtgttggaacccgcagccgtcgccagtaccagcagcgccggattcacgccaaccagctgaccagttgctggatctaggattgcagcactgataatcccggcggcggtcatcgccgaaacgacaccctgacccgtcgccagacgaattagcacagtgatcagccatgccatgatgtagggcgagatattgccgtgggacatcaacatgccgatggtgtcgccaatgccggtgtcgatgatggtctgcttcagcacgccacccgcaccgatgatcagaatcaccattgcaatactcttcaccgcgctttcaaaagcgttcatcacccactgcatgtcatgaccacgtgcggtgccaaagagtacgaatgcaaccaccatcgcaataaacattgcaatcggcgaggaaccgataaagttaaccacttcccaggcaggggtatcttttaccagccagatattggcgatggtggtagagatcataatgatcgccgggatcagcggcaccagaatcgaaacgccgaaagagggcagattattcatatctaccggttgatctgctttcaggaatgatggcgttgggcgctcaagattgccgaggaacttcggcaggatcagacctgcgcagattacacttgggatcgtcaccagtacgccatagatataaaccatccccatatccgcgccataagcattcaccagcgccaccggacccggctgcggtgggaacagtgaatgtgcggtagtggcagctgctactgccgggatcgccagtttcaggaacggaattttagcttcggcggcaataacaataaccagcggcgctaacatgataaaggccacttcatagaacatcgccagaccaaaaatcaggccgatgataatcaccgacagctgtacatagcgcagaccgagacgcgccagcagcgtatgcgctatctggtgagccgcgccggagtcgaccatcaatttaccgatgaccgcaccgaacaccacgatgatagccagttcccccagcgtgttgccgaagcccgctttcatagtgtgcagcagcgacatcaaatccatgcccgccagcatcccgacggacagcgccgccaccaacaaagccaccattgaattgattttgaacttcaaattcagtaccagcatcagaccaatgccgaataccacccagagaatgttaagcacatgcataacgttttaccttacctggttgaaccgttgttattttgggcgatatgttatgtaaattggtcaaccattgttgcgatgaatgtcacatcctctgatcaataaccatcgattaccctttgctgcaatttgcagcaacaaccatgagagtgaaattcttgtgatgtggttaaccaatttcagaattcgggttgacatgtcttaccaaaaggtagaacttatacgccatctcatccgatgcaacgccacggctgcggtctggttgttcatccggatacctaaacaactccagggttccgcgtctctttgctgtggaacccactatgtgaaagaggaaaaatcatggaacagacctggcgctggtacggcccaaacgatccggtttctttagctgatgtccgtcaggcgggcgcaactggcgtggttaccgcgctgcaccatatcccgaacggcgaagtatggtccgttgaagagatcctcaaacgcaaggcgatcattgaagacgcaggcctggtgtggtctgtcgtagaaagcgtgccaattcacgaagatatcaaaacccacactggcaactatgagcagtggatcgctaactatcagcagactctgcgcaacctggcgcagtgtggcattcgcaccgtgtgctacaacttcatgccggtgctcgactggacccgtactgacctcgaatacgtgctgccagacggctccaaagctctgcgcttcgaccagatcgaattcgctgcattcgaaatgcatatcctgaaacgcccaggcgcggaagcggattacaccgaagaagaaattgctcaggcagctgaacgcttcgccactatgagcgatgaagacaaagcgcgtctgacccgtaacatcattgctggtcttccgggcgcggaagaaggctacaccctcgaccagttccgtaaacacctggagctgtacaaagatatcgacaaagcgaagctgcgcgaaaactttgccgtcttcctgaaagcgattattccagttgctgaagaagtcggcgtgcgtatggctgttcacccggacgatccgccgcgcccgatcctcggcctgccgcgcattgtttccaccattgaagatatgcagtggatggttgataccgtaaacagcatggcaaacggttttaccatgtgcaccggttcctacggcgtgcgtgctgacaacgatctggttgatatgatcaagcagttcggtccgcgtatttacttcacccatctgcgctccaccatgcgtgaagataacccgaaaaccttccacgaagcggcgcacctgaacggtgacgttgatatgtacgaagtggtgaaagcgattgttgaagaagaacaccgtcgtaaagcggaaggcaaagaagacctgatcccgatgcgtccggaccacggtcatcagatgctggacgacctgaagaagaaaaccaacccaggttactccgcaattggtcgtctgaaaggcctggccgaagttcgcggtgtcgaactggcgatccagcgcgctttctttagccgttaatatccaccggcatggctgcgcgccgtgccggttccttcttccttgccgtcactctttgaagacggattctggagtttacgatgactactattgttgacagcaatctgccggttgcccgcccgtcatgggatcattctcgtctggaatcacgcattgtgcatctcggttgcggggcgtttcaccgcgcgcaccaggcgctgtatacccatcatctgctggaaagcaccgacagcgactggggcatctgcgaagttaacctgatgccaggcaacgaccgcgtgctgatcgaaaacctgaaaaaacagcaactgctgtacaccgtagcggaaaaaggcgcagagagcaccgagctgaaaattatcggttcgatgaaagaagcgctgcatccggaaatcgatggctgcgaaggtattctcaacgcgatggcgcgtccgcaaacggcgattgtctctctaacggtcacggaaaaaggctactgcgctgatgcggcaagcggtcaactggatctcaataacccgctgatcaagcacgatctggaaaacccgactgcgccgaagtccgcgattggttacatcgtcgaagcgttgcgtctgcgtcgtgaaaaagggttgaaagcgtttacggtgatgtcctgcgataacgtgcgtgaaaacggtcatgtggcgaaggtcgcggtactggggctggctcaggcgcgtgacccgcagctggcggcatggattgaagaaaatgtcaccttcccgtgcaccatggttgaccgcatcgttccggcggcgacgccagaaaccttacaggaaattgctgaccagctgggtgtttacgacccgtgcgccattgcctgcgaaccgttccgtcagtgggtgattgaagataacttcgttaatggtcgcccggattgggataaagtgggcgcacagttcgttgcagacgttgtgccgttcgaaatgatgaagctgcgtatgctgaacggcagccactcttttctggcgtacctcggttacctcggcggctatgaaaccattgccgacaccgtgactaacccggcttatcgcaaagcggcctttgccctgatgatgcaggaacaagcgccaacgctgtcgatgccggaaggtacagacctgaacgcctatgcgacgctgctgatcgagcgtttcagcaacccgtctctgcgtcaccgtacctggcagattgcgatggacggcagccagaagttaccgcagcgtctgctggacccggtgcgtctgcacctgcaaaacggcggcagctggcgtcacctggcgctgggcgtggctggctggatgcgttacacccagggcgtggatgagcagggtaatgccattgacgtggtcgacccgatgctggcggagttccagaagatcaacgcgcagtatcagggcgcagaccgcgtgaaagcgctgctgggcctgagcggtatttttgccgatgatctgccgcagaatgccgactttgttggcgcagtgacggcggcatatcagcagctgtgcgaacgcggtgcgcgcgagtgtgtggctgcgctgtaactaactgattaccctacagacttactggtcaatcaaactgatatttggttgaccagttttcgtttttttgcccacctgtacgtgccaacttccagtgctaatggtatagtttgagattaacgggggccgtaaaattgcccgttgtaggccggataaggcgttcacgccgcatccggcaaaaatttgattaaccgcacctaacggacacaacaccatgaaatctgccacctctgcgcaaagaccttaccaggaagtcggggcgatgatccgcgatctgatcataaagacgccgtacaatcctggcgaacggctgccgccggagcgtgaaattgcagaaatgcttgatgtcacgcggacggtggtacgtgaagcgctgatcatgctggagatcaaagggctggtggaagtacgccggggtgccggtatctatgttcttgataactcaggcagccagaacacagacagtccggatgccaacgtctgcaacgatgccggtccttttgagctgttacaggcgcggcagttattggagagcaacatcgccgagtttgccgctttgcaggctacccgcgaagatatcgtcaaaatgcgtcaggcattgcaactggaagagcgtgaactggcttccagtgcgccgggcagcagcgaaagcggtgacatgcagttccatctcgctattgccgaagcaacgcataacagcatgctggtggagctgttccgtcagtcctggcagtggcgggaaaacaatccaatgtggatccagttgcacagccatctggatgacagcctgtatcgcaaagagtggttgggcgatcacaaacagatcctcgccgcgttaatcaaaaaagatgcccgagcggcgaagctggcaatgtggcagcatctggaaaacgttaagcaacgtctgctggaattctcgaacgttgacgatatttattttgatggctatctgtttgattcatggccgctggataaagtcgacgcctgacttattataataagcgcaagggtaaacgttccttgcgctttcttaaattaagaagtcgcaatgagtattactttgtaaattgcagggtattgtttagctatctgtataacctgaatgttagtactcattcttcctggtagttatttaccaatataattccattcaccattttttaattcaaacagttctggaagagatgacggttgcagagtcatacgtttgagtggtgcattttcatcacccgggataactttatatcccatttttgcatggatctccgcggtaccgggataggcttctataccaattattgggtcattacccaactcaatattagcattaagtaatgcggcaagggcgaatccggaagaatttgctacccctgttaccgtcattatctgatcaatatagatatcaatccttggctgctcattggtccatctttttgcctgagaagctggaagggttgaaatatatcctatcgtggttccggcataaccaggaacattgcaaccagggcctaatgttatttcatgaactgtatagtcctcaacaggatcgaaagggctcttcataaataaatttagccgtaaaccttctgctaactctgtggtagcatgcgcctttttacatatgccaccatatatttcgtctaaagctgaggtgattttcaagttccgatagagcatacgtcctgttgttgtaataccatcggattctctgcatgctcctgtcacataattaaatggccaaggctctttactaatatcaagttttctaatttcgacaacgctttttccatcgtaattatggttattgccacgagtaagaggcggaagatagatgttttccgaatccatgcgtgcatattttaatttacgtgtaaactcactgtcgactattgggtgatgaaggaagtgagcatctgtaataatttgactctgaagggcattgcttaatggcatagacataatagttaccttttatgagtatttcactgatgtttagaaaaatagataaatttttctgtagtaaaaagagaagtaaacaaatgacatgcatgtttctgttgtagtgatatcaactctacacggtgatattaaagggtaggaaacactctaaagtatcaaaaaacgctcatttaaaattatttgcatgcaatttaaaagcatatcttattactaattggaatttgatgttgctatattgaggtctatattaataatgcctgtgaatggtatttttgatgtatttgatatgttatcaatttatattatttacaaactaattgtttcaaataatacatggctgattatgcggaaataaataatttcccaccggaattaagtagcagcggtgacaagtattttcatctacgtaactattcggaatattcagaatatactagcggtttttttttgagtttgatgatttttatcaaatcatgacttttttcctgaaaagtcagtagatattcataggcaagtaaggttttatactttgctgacaggattcaggcctgtctcagactgacatggatgtaatgaacaaaagggaatggctatggaaaatgagcatcaatacagtggtgcccggtgttcagggcaagccgcatatgttgctaaacgtcaggagtgcgcaaaatgatgcgacaatcacttcaggctgttttacctgaaatttcaggcaataaaacgtcatcgctgcgtaaatcggtatgcagcgatctcctcactctttttaattctcctcattcggcattaccgtcattacttgtttcaggcatgcccgagtggcaagtgcataacccgagcgacaaacatctccagagctggtattgccgtcagctgcgttctgcactgttatttcatgagccacggattgcggcgttgcaggttaatttgaaagaagcgtactgccacactctggcgatcagccttgagataatgctgtaccacgacgatgaaccgctaacgtttgatctggtctgggataatggcggttggcgcagtgcgacgctggagaatgtcagctaagcacaatctccagctcgcgcagttcacgccagaagcgttcggcaacgggattcatgcgggtattcatccggtatgcataggcctgaatcgggatcaccagttcgtcccgattcagtacaacgagcttcccgctgcgaatttcttgttggatggcgtactccggcagccaggcaatcccacagccgtcgagggcaacctgctttaaaagctcgctcatcgaagagacaaaaaaggtgctgaaacttaactcactgtggcgcgtcagggtgcgattaatcaatcgccccatgtaggagttgcggctgtaattcagtaacggaaagtgtggctgcgcgaggttaaaaagtgcttctccgtgttcgtcactggcgcagacagggaacaattgagattcaaataagcgaatgtggtcaaacggcgcttccagcaaatcttcgtcgtgaaaggaaaaaatacagtcactttgcccttcacgcagtttatcgaccgcttcatcgacatcaatagcttcaattgcccaggtaaagagcggcggcatctggctgataatggacggtaacagcccgagggaaagagagtgtgcagcggctatcttgatttttcgttgcgcgtaatcgctgccgccacgcagctctgccagattgctctctaactgttgcaacagatggcggatctgcgaatggaagattttcccttgttctgagagttgcagcggcgttacctggcggttaaacaattcaacaccaatcgcctgttccagcgcacggatgcggcggctgaatgccggttgcgagacgttgcgactgactgccgcctgggaaaaattgcggcatttttccagggtcagaaaatcataaagccatttggtttcaatattatgcaaaatcgcaccacagtcatccattacgttttactctgtcagccgcccttgcgggcattctacgtccattcgggcggctgacaaccgtttaagccgtttcaaacgttcctttcacgcaggctttgccgtctttgaccatcagtttgccgcgagcgtatacctgctcaatgcgcagttctggcgtcatgaccagcaagtcagcatcattgcctggcagaatttcgcctttcccggtcaggttaaggaaaccggctacgctactggtgagcgggcgcagggcatcgctgatactgaaatcatagtctttgaccagcacctgcacggtttccagcaacgtttcaaaaccggcaacaccgatatgggttaaattcccttcgtcatcgaagaacggctggctaccgttgccgtcggagctgagggtgacgcgtgccagcggaatacccgcctgaacggcgcgggcaataccttcggcaggggcgaccggttcgtcaatgctgctggtgatatcgatggtgccgcctttgcgcgcgaactccagcgcctgctcaaacaacggtacgttgcggttaacgtgggtcggcagcagcttgctgatcggcacatcgcagttttccagcaggtcataaataggctgtaacgcctttttactgtcgcccatgtggaacacggtgacgccaggtttaccgccgagcaaaccgccaacgcgggattctgccgccatattggccaggtgataaacgtccggtgcggcagaacggtgatcagagatggcgcatttcacgccaatcacacgatcgataatcgccacgtctttttccacggaacccgtaatggtgcgggaagggacatgataagcgccggtcagcatccaggcgctgatgccttcttcattgagcgcacgggtcttggcgagcagggattccgggtggcgagagatagagtcggtgcccagcagaccaaccactgacgtgacgcccgcttccgtcaggcgacttagcgccacttccggcgtgcgcgtcgtgggacctgcttcgccgccaccgccaatcaaatggacgtgttgatcaataaaacctgggcagaggatctgcccactgagatcgacaaccgtgcagttcggtacaatgtcagaagggatattgctggcaacggcgataattttgccgttagcgacgaggacatcgcaaattccccgatcttccggcgcatacaaatgcgctccctgcagcagggtaaaaccggctgcggtataatcaatcatggtaactccttgttaaacaataagctgcataacccagatcgacagcaatgcgttaatcacgcagaccgtaatgatatgcgggtaatatttggcattcacttcggctgtccccaggcagcgaccgacattttgcaccgggttgcccattaaatacatcgcgggcagtaaaacggtgacatcgtgaccggttaatgcgccagcggttgccagactggcggcaacaccgactgcgccacccatactcattaatgcggctaaaaggacggttgccgcttcaccgggtaatccccacagcgccattacgggttcacagatatgccccacccagtcgagcaggccggtaattttcagcgcctgaatgatgacaaacgccatcaccacgtttggcagcaggttggtcgtggcgatagtaaagccacggcgcgcgccatcgataaacatatccatgacgtttttgcggacctgagttgtcatgcttgcgctccttgcgttgggttgcgacgttcttcgaagttaagccagacgcgcaaaatgttggctccgacaaatttaaacaccaggatgacggctaaaggtacgattacggacgtgcccagaaaggcaaacaccgcgacgccggaagagaagtagttggtgatgatggcgctaccgctggtttgatatgcggcgaaaatcactttatcgcgttcggtaatttcaccttcctgcgccagctctttggtcataccggcggcggcatcggtgttttgcaggttagcgatcagcgccagcgagcagatccctggaatgcccaacaacggttttagcacaggtgtcattaactgctgcgcggcgcgtaatccaccaagaccatcggtaattgaaataatccccagagagagaatgactgacggtgccagctccagcgcaaagagaaagccatctttagcccccgcgccacccgcgccgcgaaatgaggtggtggctccgttcgcaccaggcagttgcccaaacgatccgttcagaacggaaaaatcaaaaacgcgccaccagctgtctgttccggaaaaaacaccggaaaaaaagattatggtgagaaaaaaggccagataccctttaatgcccactttttctgtcgccagctccccggctacagcatccccttgttgtgtcataacaatccccattgtttttttgtgtttgtgtgttgcttgagccaggaaaattcctggaactgaaaaaccttatcagccatgtgggtatggggaaaatgcaagtatgtttctggctatgcgttttttgcatagcggaaaaattacgctgtgtggaaaaggctctgcgcaggattgagttgcagaaaattcataaaccaagtgacaatgacatcagtaaataaaaacagaaaatccagggacgaaaacgagatggcaaagtacaacgaaaaagagctggcggatacgagcaagtttttaagttttgtcctccgacacaaaccggaggcgattggtatcgtactggaccgtgaaggatgggcggatatcgataagctcatactttgtgcccaaaaagcgggcaagcggttaacccgtgcattgctggatactgtggttgccaccagcgataaaaagcgttttagttattccagtgatggtaggtgcatccgcgcggttcaggggcattcgacttcgcaggtcgctatttcctttgccgaaaaaacaccgccacagtttctctaccacggtacggcaagccgtttccttgacgagataaaaaaacaggggctgattgcaggtgagcgtcactacgtacatctctctgctgatgaagcaacggcacgcaaagtgggagcaagacacggatcgccggttattttaaccgtcaaagcacaggaaatggcgaaacgaggcctccctttctggcaagcggaaaacggggtctggctgacatcaacggttgcggttgagtttcttgagtggtaagggaaacttccctcatgaagtgaccacttgtagcttaaataattgcactgtgctgataagcgcagcaataaacaacgccgccgcgccgcagagagtggcgctggcaagcgccgatgttccattgctgagcatactggtcagcgccgggccgaggatttgcccaatgccgtaaatgagcgtcacaaagcctaaaagattgagatttcccggtacgctcagttggcgggcgatagtcatcaccagagatgtcgtgcccataaaggtaccgccaaaaccaagactgctgatgataagcaagagaggcgagtcgctggcgagagtaagcagcacacagatagcctgcaccagcaaattcgccgtcaggcagggcaaagccccccaacgttttgctgcccatagccagccaaagcaaccaggcacaattgataagccgactaacgtccagagatgggcggttaacaatggtgagcctgcatctttcgccatgagcggcaggtaagtcgcgacgatgatataaccaaatcccgccaggccgtacagaatagccagtaaccaccagctcattatctgttgctccgtttttgccaatggcattggtgtgatggcgtgttttttcgagggcattaaaagcgtaagtgcaatcagcatcatgccagaaagcgccccggcgccttgccataacgtttgcgaggagaggtcaaaatgcaggcctgccagaacatattcattgcccagtgcgatgccaatgccaacgccagaaaacaaagctgccagcacaaaaggatggcgcgtgtgctgcataatcagcgtcgaaccaaaaatcagcataccggcgctggcgacacccgccaggacgcgaatcaataacaccagaataaatggcggcaaccatgccattgcgaggatcaacaacccgctcgccagggcagaagccaacagaaatgggcgcaggcgcgatggctggtgaaatgcgccaaaagaaaatagcagactgccagccagataccccgcatagttgccgctggcaatccacgagagctggctaaatgaaaacgatccttccgccatcatgacgggcaacataggcgtataaaggaagcggcctaaacccatacctaaggtcagaaccagcatcccgaaaagcgcggtgctgaaagaaaagcgttctacgggatgcgtggacgaaggcatgtttaaccttgtttgtcatttttgttgttaacaagttaataacaaaaaggtgaagcatgccagcctgttaatgcgatgattgaggggtaaagcgataaaaacgatttggttcgctaacgatataaatattaccagaggcatccatcgcaaccccttcggcctgtttgatgttatgcgacaaacctcgactgcctttggttagtgacatttcaccgataacctcgccaaccagggttacttcctggagtgcgcgagattcatgagacagcaccagaagcgtatttttttgctggttaaattctgcgccggacacatcatctaaagtaaattgccgttgtagtgcctcgtctttgctgatgtgtaattcattgctacttaacagcccgttaactttgtagacctcaatcggatttttctctttaaaaaaccagaaagtgtgatcctggcgagaataagccaacccttcaaaaccgcaattggttggggagtcttgcagcgggatttttatttttttgaggatttttacttccgagtttggggtcagtgaaatcacataaatggcgtaatcgcgctcatcgctaatgacaaactgattatcgccaatgtattcgatcgtctcgagatccttaacaaaatccagaggaattgtgcggataaaatcaccattggtggtcatttcaacaatggcggcaggtttgttgatagtgctaaaaagagtattgctttgtgccgaccaggtcagcgaagagatattattcgttatgcctgcaatttctttgccgtcaatggtggcgtggtaattctgaaatgatgctgcatgattgcttttacgggcgcaagattgcacgaagaaagtacacactgccacaatggcaaaaagaatcacaataatggagatgcgtttacttaacgaaatactttttgtcacggtaatccctttaaggcaaatcaataagatatcgagaagtatacgtagcgaccttaatgaatccttaacgcggagaaaccccgtaatgtgcaatgcagcgccagacaccatcctgctggcaataaattgactcagtcagcccagggatcacccattgtatttcctcgccggggggacaggtcagccaaatgcataacccgcagccgccgcgtaaatcacggggaatatcgctgacgcgaaaagtcatgcccgctgcctgcaacgctttgcgggtttgtatgacgccgaccgtggagtgaaataaaaataaaaactctttcatcggcgtgtcctcactcgttgaccaattaccgccgcgccaattgcgccagcaaattgcgcatcaggatgggtatttaccggcattcgcaggtgagattccagcatccgggcaaacttctggcaatgactaacgccaccagtaaacagaatcggcgcttcacaggagagacgagcaatgaaattggcactcctccgcgccatcgcgttaatcactcctgcgagaatcgcttctggcgcgacgcccgctgagcgcaggctgatcgcttctgattcagcaaacactgtgcacatactcgtgatggcgtgcggcgtgacattttcggtaatgctgtcgagttgctcgacgctggtgccaagcgtgcgcgagatcacctccaggaaacgcccggtgcccgccgcgcatttgtcattcatcaggaaatcgcacaggttaccgtcatcatcaagctgaatcactttgctgtcctgaccaccgatgtcgattaccgcgcgcgttgctggcgcaagaaaccgtgcgcccagcccgtgacaggagatttccgttacctgtttatcggcaaaatccaccagttgccgcccgtagccggtgagcgtcagaaacggcgttgtctctaacccttcgcgcagagtttcccaggcttcagtaattgctgttgccgggcgaaagggggttggaacgaggaaacggcgcgtaatcacgccgtctgccagtaagatccctttggtggcggttgagccggaatcaatgccaatcgaatatgccactgccactccttacagcatctcaataaaggccgcgacacgggtactgagctgcccgacatccgaggtggagtagtctgtttcaatagcgatataaggaatgttgtgctgctggcgcacatgacgtttaatcgccagcgattccaccgcgtaggtatggcacgcctgcaaaatcacatcaactacgccatcgacctgatattcctccaccatctggctgagcattttcaggcgctgatcgttcggcgaaacacaggagcagccaatcgccagatatttatccgccagcgcgtcgtagacatcgcccgtttctgccacgcattgctcggtcgctttcgccccggtgcagttttcataaccgacaacccagccgccattctcttcaatcgcgcgcaccactttttctgctgcgccgccaatcgggcagccggtgattaaaatgcgcggacgcgggtccagtcgctggccttcttcccactgctgacgaacgcgggcggtcattgcatccagttcattgatcaacgcctctttatcgaaccggaaggttgcgccgtaaaccactttcagaatgtcgctgccgctaagcgccggaggatttaactgcccaagatgataaaaattagccagtgcgcgacgttcgcggtttttcagcgcaatggcatcgcgcagagcatcttcgctaatctcgtgcccaaaacgttcttctaccgttttttgcaagcgcagcatctcggctttccataacgcacgcgaggcatcgtccttaacgctgttgggcaattgcatcacatgaacaggcttaaactccgccatgtattcatacattttctttttgccgtcgcaggtggtttcaccgaccaccagatccgaaaagtagaagtaggggcatttatcggttttgccgaagccgtagctgcttttaatcagcgggcagaggttgcgcggcagatctttctccgcttcttcaatggtttcatcagaggtggaacagagcgaaaccacaaccgcaccggctgccatcgggatctcttgcggcataaaggtgcagtaagtgccaaccagcggaatgccgcgctccttgagatccatgacggtgagaaagcctgtctggcgagcttcagagaactgatcgaaaatggcgggtagatcggtgacaagtgacatgattttccttccccgtaccacgggagataatgaaaagaggccacattattaccattcttttagtatggtttatttgatctctctcgcggttagccacttagtttttcatggatttctaaaaattgccgagggggaacaaggccgggagctgcgacagcaaatataaaattagcccaatacaaccgccaaccagcgtaccgttgacacgaataaactgcagatctttgccgatatttaactctatttgccgcgacatatcccgcgcatcccagctttttaccgtatcgctgatgtggcgcgtcaggaatgcggaaaactcaggcgcgacgcggtgcgcggcttgttcaagatgaccatttaacgacgcccgcaaggcatcatcggcaattaacgtttcgccaaaccattgacccgctcgtgcgatgcgttctttcacacgagaatcttcactgttgatatccactttcagccattcccgtaaatccccccacaattcactgagatagcgattaaaagcttcatcttctttcagatagctttttacggcatcggctcgcgctgccatttccggatcgtttttcagcttgtcgatcagggcgaaggtggcgcgatcaaacgcatggcggatctgatgcgcacgatcgcgactaatatcatcaagcaaagaattcaccgcgtcagaaaccaactccgcgctatgttcgcccaaccattcggtggggagaattttggctttcagtggatgctcgctctccagccagcgaacaatttgctgggcgataaacttgcgcgatttatcgcgctggagaagggcgatcaactgtgcgatcagcgtatccagcagcacctgatgacgatcgtttttggtcatactctccagcatcaacgcactggtgccggaaagatcgaccttatcaatcgcccgatggaccgcgcgcttaagcaggcgctgaatacgcgcatcatcggtaagttcgagaaaaccgctcatgatctgcaacagatgctgaccaacgcggcgggcgttttctggctggctaaaccagttgccaatcagcaacgccggttcgtggcgtcgaatcaatgccaccagggattgagtatcaagaaatttttcctgcacgaactggccgagattttcgccaatccggtctttattacgcgggataatcgccgtatggcgagaaatgatcggaatcggcacgcggcgaaacagcgccaccaccgcaaaccagtccgccagcgcgccgaccatcgccgcttcagcaatcgccttcacgccgctcacccaaaaattgggcggcaaaaacagcgtaacgacaaaggtagcagcggcgataagcagtaaagagagcgccaaccttttggcgcgtctgagttcgatgagtttattcataacgttaagaatagagcctgacggccggatcgcgcaaaaatcactgctcctccactagctcggctgcctgatgctggcgcacgcgattgagcaatcccgccagggtgaaaacgacgataacgcccgccacaacggctaacagatgaaacggcaagcgaccgccgttaaaccatagccagcggccgatttcgaccgagaccgacatcaccatcaggatcaccatatttagcgatgcggagacggtccctttcggtaacttattggaaaacagcgtaaagcggaataaggtcgggaaaatcaaaccaatcccgaaagcatacagactggtgcccagcaccgaccacagccagacgtgcggcgacagcagattgccgacaatcaacagcgagaggccgaccagttgaatgggtacggcacgccagataaaccgcggttcggtcggatctttaacaaaacgcgccacgatggcattcgcaacaatcaccgcgccgaacaccggaacctgtgtccaggcgaactgcgaagttgttaagctgcctgcatcgataaggatcaccggcgagacagccacccagctcatcatcgggatatagcttaaagagatggttgctgcgccaaagaggaacagccgattgcaaaagacattacgaaaatcgcgcaagacgcttttggcgctaaacggaaccgcgccgcgcttcaccgtctctggcatcgccaacagtaagccaacaaatgagataaaacccataaccgcaatgatggcaaaaaggactttccagtgcataaagtgcatcagagctgcgccggaaagcgggccgataatcggcgcaatcagtacgatggaggtgataatcgccatcaacttgatcccttttgtctgtccgaacgcctcctgcaccgtgacataaccaacggtggcaataaaacagatactggtgccctgaattgcacgcgcgataagaaactgtgtcatagacgttgtgaacattgtcgcggcgcaggcaagggtaaaaattagcgccccggtaatcagcaccggcctgcggccaattctgtcggaaagcggccccagcagccactgtaacgccataccgccagcaagatagagactgacggcagcaggggccagactgacatcggcattaaaatcacgtaccacattaatgatcccaggctggatcagatccgtcgacagatacgcagcaaagtcatacaaaatcaacgccatcgggaaaaacagcgtggcggcatggcgggtaaaaaaacgtggcataacaaacaactccttgtccggagaaccccaacggggaaaacgaaattcaataccgtcggtaatgacgaaaggcaggtgagaagggcaacgagactgcaaatgtactgaatttcatgtaatcaaccacactgcctgtgaacacacagacagagaaatactttctgacttcgggtcagaatgtataacgattacaaatagtcatcagcacattacacctcttgaattgatgggttgcatagaaaatatacaccttaagtgtaattaaaatttgcggttaatcaaaagagcgcggtggaaaggggaatatctgccgggtacaggacatgtaaaacgcgagcttgtttccggaaaaatgtatcgtttgcagaagaataaaaatagcctggaaagcgcctcggggaatgggaaattgccgggtgagaatggttttgttagtcgctaaagtcaggccatctttttcaacaggtgatggatcgccatgacaaacttcacgaccagcacgccgcatgatgcattatttaaaacctttctcacgcaccctgacactgcgcgggattttatggagattcacttacctaaagatttacgtgaactgtgcgatctcgatagcttaaaactggaatccgccagctttgtcgatgaaaaattgcgggcgctacactccgatattttatggtcggtaaagacccgcgaaggcgatggctatatctatgtggtgattgaacatcagagccgcgaggacattcatatggcctttcgcctgatgcgctattccatggcggtgatgtagcgccatatagagcatgataaacgccagccgctaccgttggtcatcccgatgctattttatcacggtagccgtagtccttacccctggtccctgtgctggctggacgaatttgccgacccgactaccgcacggaagctttataacgccgcgttcccgctggtggatgttactgtcgtgccagacgacgagattgtgcagcatcgcagagtcgccctgttggagttgatccaaaagcatattcgccagcgcgatctgatggggcttatcgatcaactggtagtattactggttacagagtgtgctaatgacagccagataactgcgctgttaaattacattttactgactggcgatgaagcgcgttttaatgagtttatcagtgaacttacccgtcgaatgccacaacacagggagcgaataatgacgattgcagagcgaattcataatgatggatatataaaaggggagcagcgcattcttcgattgttgttgcagaatggggcggatcctgaatggatacaaaagattaccggactttcggcagagcaaatgcaggcattaaggcagcccttgcctgagcgtgagcgctattcatggctcaagagctaatcagagacggatgacaaacgcaaagcagcctgatgcgctatgcttatcaggtctacataacccattaaatatattgaactttaaagatttttgtagacctggtcaggcgttcacatggcatccggcatgaacaaagcgtactttgcttaattcaggctggaacgtggcgatgacccagcaaagataaaacgagtcacaggttatgcatgagaggaaatcaggcgcttcgccgctatttcgaatttattccattgcccgatacacggcctcgccaatttgcttcagtgcttcgcgataggtttcgctgagcggcaaagcgcagttgatgcgcagacaattacggtatttgccggaagctgagaaaatcgagcctgccgccacctggattttcatgcggcacagctgccgcgcgacgcagaccatatcgacctgttcaggcaattctatccacagtaaaaatccgcctttcgggcgcgtaatacagatttcgcagggaaaatattcccgtatccagcaggtataaagcgccaaattgcgctgatagatctgccgcatccgccggatatggcgatgatagtgaccttccagcacaaacgttgccgccgccatttgcgtggacggcacattaaagctgctgatggcgtatttcatatgcatcagtttatcgtgataacgccccggtgcgacccaacccacgcgcaggcctggtgcaatacttttactgaacgagctgcacaacagcactcgcccgtcgatatcccaggaatgaatggtccgcgggcgcggatactccgtcgccagttcgccatagacatcatcttcaaaaatcacaatatcatgacgctgagcgagagagagaacggcccgtttgcgcgcgtccggcataataaatcccagcggattattacagtttggcaccagaatgatgcctttaatcggccactgttccagcgccagttccagcgcttcaacgctgatgccagtttctggatcggttgggatttcaatcactttcacgcccatgccgcgcagcatctgcatcgaaccgtaataacagggggattcgaccgcgacaatatcgcccggtttacacactgccattaacgccagcgacatcgagttatggcagccgctggtgatgatgatgtcatcggcggtgaccaccgagccgctgtcgagcatcaggcgggcaatctgctctcgcaatactcgctgaccggctaacaagtcataaccgagaacggtttgcagattatgctgcaccacccggcttagctcccgccacagcggtttcaggctgggcgcttcgacatccggtgtgcttttgcttaacggaacaatggaactgtcgctatgcgcctccagcatatccagcacctgatcccactgggtaatttccaccgggcgctgcaccggacgcgtcatcggcggtactggcggctgggctttacgttgtgcgacaaaataacccgaacgcggctgcggagtgatgagcttcatcgtctccagcgtctgatacgcctgctgcacggtgctgatactgacgccgtgctcctgacttaagctgcgcaccgacggcaatttctccccgtgacgatacagcccttgctcaatccgttcggcaagcagagtcgccagatgttgataacgcgtcatgctgtattccttatgtggaccatacagagagaaaaaccggtacagatgaggctaaaaaaccggatgcagatgctgttttaacctgtctgtatgttaaataaaagtaatatttgaatctgtattgtgaactgccagaaggtggatgatgaagcctctgaaagatgaggaggtagcagatggaatttcacgaaaacagagctaaagcgccgtttatcggcctggtgcaactctggcaggcggtgaggcgttggcggcggcaaatgcagacccgacgcgtgttacagcagatgagtgatgagcggttgaaggatatcgggttacgcagggaggatgtggagtgaggggggatatagatttatatataataaaacgtttttatgtttttaaattaagttataaaaattttcccgagacaattcatcaataggtatggagtgtacaggaatatcttcttcactaacctctttaaactcatgtcgataacggtcaaaaaacgcacagtgattacttgtgttttttgactgactttacaactctcattattcgctattgtgcagtttctctaattgttttataccctggaaagttaaatgtcagctactgaatactttttgattgtttgagatttattttcatttgaaattataaaatcaggtgataaatgagttgtgattaatagatggttgatatcatttttatctaaaattgatttatagtatcgacctgaaaaaatagttgttgccgcctgagtaactatacaatattctgaaaggttttctttcaaattagaaatgttgtggggttttgtttttgtatcttttatctctaaggagcttgctttgggtcaatcagaatacatttcatgggtaaaatgtacttcctggctaagtaactttgtgaatcttagagggttgagacaaccggatggccgtcctctttatgaatatcatgcaaccaatgatgaatatacccaattaacgcagctactccgtgcagtcggtcaatcacaatctaatatatgtaatagggactttgctgcctgttttgttcttttttgctctgagtggtaccgcagggattatgaacggcaatgcggatggacgtgggaccctatatataaaaaaatagggatttcattcaccgccacagagcttggtactatcgtaccgaaagggatggaagattactggctgcgcccaattcgattttatgaatctgaacgacgcaattttctcggaacattattcagtgaaggtggtttacctttccggctactcaaagaatcagacagtcgctttctggctgttttctccaggatccttggacaatatgagcaagcaaagcagtcaggtttttctgccctttcgctggcaagagctgtcatagaaaaatcagcgctgccaactgtttttagcgaagatacctctgtagaacttatcagtcatatggctgataacctcaattccttagtacttactcacaacctaataaatcacaaagaaccagtacaacagcttgagaaggttcaccctacctggcgaagcgagtttccaataccgttagatgatgaaacaggaacgcattttttgaatggactgctatgcgcagcctctgtagaggctaagcctcgactacaaaaaaataagagtacgcgttgccaattctattggtcagaaaagcatccagatgagcttagggtgatagtatctcttccggacgaagtttcctttcctgtaacaagcgagccgtcaactacgcgctttgaacttgccatttgtgaagatggtgaggaagtctctggccttgggccagcctatgcttctctggaaaacagacaggcaacagttcgattacgtaaaagcgaagtgagatttggcaggcaaaatccatcggcaggtttgtcgttagtggctcgtgctggagggatgattgttgggagcattaaacttgatgacagtgaaattgccattggtgaggtgccgttaaccttcatcgttgatgcagatcaatggctgttacagggacaggcttcttgcagtgtgcgaagcagcgatgttctgattgtgctccctcgggataatagcaatgttgctggttttgatggccaatcgagggcagtaaacgtattaggactaaaagcactacctgtgaagggatgtcaggacgttacagttacagcaaatgaaacttatcggattcgcaccggaagagaacaaatcagcatcggaaggtttgctctaaatggaaagcgtgcaagctgggtttgtcatccagatgaaacatttattggtgtaccaaaagtcatttctacactaccggatattcaaagcattgatgtaacgcgttacacgtgctgacaaaacagcattacagccagcaggaagtactgcgttggatcgatgtctgttcagggactcaacctaatgcaaaggatcccgcatttcttaaagtcagggcgcatatcttccagcgtaatacctagggaatatgggcttgtgttgataaagattgcagattaaagcacggtacaccgctcgacaaaggctggccctttggctatgtgtatgtgaaccagcgacaaaattgtgactgtggaagccctgtatacgaagttgcattctgtaatgattgtaatgagcctcatcttctggcacgggacaaaaagggcaaactagtccagtgggaaaataaaggtggcgatgaattctctttgcaggatgaagtacctgttgaacatgacgctacagaagaaaaagtcgaaaaagagaacagttttcagcctccgttgattattgccgcaggagagaccagcgaggcaggttataccctacaacgcctcgaccgtcagacgcgccgtattggcgttattaacaatgacagcattccgctgattattaatgatattgaacaggtttgtagtgccagtggctgtggctacagaggcatgagtgggaaacagcccttccggcgtgcactattaggtgggccattttacgttactaatatcgtgcccaccgttctagagtattgtcaggactttaccagtgatgaaggcaaagagggcgtcggaccagattcgttgccaggacgaggtcgtcgactcatcacctttacagacagtcgacaagggacagcccgaatggcggtgcgtatgcagcaagaagcagaacgcagtcgcttacgcggaagcgtagtcgaaattctcagctggcatcaaaggacgcaaacgtctacagcgccgaatgccaatgccgatctggaaaaattagcggccagggcgaagcaagcccgtgagcaggcagaagaatatcgaagctggggaatgccagaccaggcgaaattgtcacaagcacaggctgaacagcttgaacaggcttatcaggctgcaaccggtgggaaagccgcgactatcctggtatcccgaacctggacggagatggttaacgagcttaaagagagagccgatatccgcgggccggttctgcaatataaccattatcttaagcctgaagtgtttaatgaaaacggcggcccccttaagctttctgaaatgttgttgttccgggaattcatgcgtcgccctaaacggactaacagcctggaaacacaggggctggttcaggttggttaccaggggctggagaaaatacataagagccccttgcactggcaggaaaaaggattaacgctggatgactggcgcgattttctcaaggttacgttggatcattacgttcgcgagagcaacttcacacagctggatgatgagctgaaaaactggattggtagccgtttttcatcaaaattcgtccgtaacccggaatcaaaagatcctgaagataatcagaacagacgctggcctcaaattcgtaatggcaacgtatcccatcgtttagcgaagttgctgatgctgggggctggattcaaaaccgtcaatgcggcaactattgatattatcaatacatggctgaaagaagcatgggcccaacttaccggaccgcttgcagtactgaaacccgatggcaaccgtttttatttaccgaaagagcatatgactttttctttaatcacggatgcctggatttgcccggtaaccaataaaatcctggatacggcttttaaaggcttaaccccttatctgcctacccatatttcgttcgagcatcttaccctggcgcaatatgacacttttgtcgcgcagaaagtcacaatgccggaaatctggaagctggatcgttcacaggaagactacgcagagggtctggcaaaagcacgcgactgggtcagccatgatccgctgatcgcacaattgcggtcggaaaacgtctggacagacattaacgatcgtgtcgtggaaggcggcttctactatcgtactgccgagcactctgcccagcagtcgtcagaacgtctgcaaagctatgaaaagatgttcaagaatgggcaactaaatgttctcaactgttccaccaccatggaaatgggggttgataccgatcgcgtgatgacgctggcctctcgcagccagcaggcaacgattccggggccggagtggcacctgaatgacgaactggtggtgcgtagtctcggttataaaacggtagaactgaacgagtttattctgccggctaaagccaccaacgctgtcgagcgggtcaaagacattcagatccacaaacagttgaatggaccactgtcgcagtttgggcaacgcttctgggacgtgctgtttaacgaccatgaagaagcgcagtcactgatgaataacacgcgaattaccggcgttcactataccgatcgctatctgcaaaacccggttgcgctggcgttgttgggatcaattctgagaccgctaaaaacaaagctgaccgatggcgctgaagtgacgctggatacgctatttaaagataaagatcgccccggtaaccggcctttccatgactggatgagcatagcggattttcaggatttcgctgatcagtggtttgctgctgcgctgggcaggccggtagaactgacggtgttcgactcgccgcgcgatatccctcaccatcgtaaactgacggtgacttttgaggatggtcaggtattgaagatccgcttcgatcaggggatgggctactggcgcatcaacttttcatcgcaatggcattactttgatttccgcgatgacgtttctttccagttagtcaaaatggctcaggcctgcaaggaagggaatgtcgccaacagcgaagagagttgggcaacggatgtgctggtggaggtgatcgcctcctgatgatgagccgctcccgatgtggtgtcgggagcggtattttctataaaacttaccgcttatttgagatattcatcgaaaatgtcgagtaattcttgatgtatacacggccattcctgacctaaattgacggtacacaagccaatatcgaagccattaattttataacgatgtttcactgcggtatctacgtggggatatattaataacccccctatgttttcgccattttcaggctttaacgaccataagtaattcatcagttgataaagattttgcgaatgaaatttttctgttcccattcgtcgtgaaaaaatgctcttatagtatttggcgtcaacgataagtattttttctgatgagcgaatggtgatgtcagtttccattcgaggtaacaaattaagtgactgatccgatatactcgatgcatcccattttaaataagagcgggttgtgtttgcagacgttaattcacgacggcaaaattcataaagaaacttttgataaagtaatgacatctctttttcgtttctttcaaaatcatagaaacggtagtgtcctttgttttgacctggaatagaattattgacgatgaatttgcagacactgataacgaatttataataacgcgtattttttccgccattcagatagctgaaatgctgcggagttaaatgaagagtgctaatgcccggtaattttctataaagtgaacgagcttcatctctgatagttgaatttaacttttcatgcttaattaatatggctaatgtgctttttataattcggttagccagcgtgtcttcattaagcatatcaaaagtactgacggttttcccatgattaagatggaagccgcgtattgttttagcaaactctattcgccctttgatgccaggaatgatctcggtgttaggattgtaatcaagctcaagccctcggcgtgaaagctgtaaaacccctttatttaatacataccccaggatatcaagaagattgttaccgggtatggcttcaaggtttgcctgcttaatttcctgtaaataaccccatgcataggtaagcatgtaatagatattacggacaggtatcacgggctgttccactatgagtcccctaataatttgttggtccatttctgttgtttataggggtcatcaaagaaatattcttcgagtaaaggggcgatatccgtcatcacaatttcattaagccattgcgtatccggagaggtgccatcttccaacccacagcagaagtaactatgcccaatgcggaatcctttcccaaggatagtggcctctttgctgatttcctggttcaactcgttcattttttggcataaagactcaacaaatgaaggttctgcttttttattcagtaaaaaattccggaactgtggtgtatcaaaacctggctcaatatctatgaaagaaaatcgtctgcgtagggcatagtcaacaacggccagagagcgatcggcagtattcattaaaccgatgatataaacattctccgggacatagaatcgttcttcatcgttttcggagtaggttaggggaacagaccagttttcacctcgtttatcatgttccattaacatcatcacttcgccaaatactttactgagattggcacgattgatttcatctataataaaaatatactttttctctggctgctctttagcttgctgacaaaaattgtaaaatatgccgtctttacgtcggaagccgacgccattcggacgatagccctgtataaaatcctcatagctataagattgatggaactgaaccatattgacgcgttgcggagccttttctcctgtcagcaagtaagccagacggcgtgcaacaaaggtttttccaacgccgggcggcccctggaggataatattttttttgatggttaatcgtttgagtatcgtctctattgtggtttcagggataaacaaatcatttaacgcatcttccagacagtatgattcagtttttgacataggtggaataacactcttgccagaattaaatattaatttatagtcgttgattatgttgtccagcatagaggcaaatcgggtgtaatcaataccctgtgagactttttgggaacaggcgtaataggactgtccgtattttttaggatatacacccgaagttgcctgaaaatactctgcgattgttttaggtatgtctgaagagaactgccattgggcatgtggttcattcgtgtcgcttataccataagccaaaaccaactcatcaaaatctttataatagagaataacgggatatataccgttagaagcttcctgaccttctccaagaaatgcaaaccagggaatagacgtaaaattaccataaccgaaactcaattttactcgcaggttacggtaagacgttggataatctttagtggattgcgaacgttgttgctgtgcttgcttaataaatttttcaatccagggttgaatagattccataagatatgccttcctcattgctaagcctctattatcgctttcgcaacgtactgaaacaatagatttttactgcaaaatcagactggtaaatatttactgagggggaaagtttctattgagtcagtggaaggctcccggtggttaaccgggagtaaacgctgttacgcgactttctgtttaccggcaatcactccaataaacgcctgcacctgcttttgtttacgcgccgacagtttgcacacctggcgtagcgactgcatcagttcgctctcctcggcggcgggtggttgggcggtgaggacaatacagccttccatcactttgacatctaccgccgtgccagtggcaaaaccggcggcttccagccactgacctttcagggtgatggcgggaatacggctgtaatccgggtagcgactcgcataaccgacggtgacatgacggttatttgccggggagacttctgcttcgaacggttgtgcaatagaatgcgtgtcagtcataactgctattctccaggaatagtgattgtgattagcgatgcgggtgtgttggcgcacatccgcaccgcgctaaatacctgtatatatcatcagtaaatatggggaaagtccagctaaaaatagaataaaatgggcaatttctggaatgatttaaatatatttatgtgggttatgattggcgtgaaataataaaaagcgcaccggaaaggtgcgccagaaaataatgttcaggattttttacgtgaggcttttttacccccgctagctgcgcgttcagctttgattttttccagcaacgcggcggcgctgttttctccgctgatcaaatccgggttttcggcccgccactgggcggtaagttcaccacggaacgcttttgccaggatggattgcgtcaggttgttgacgcgggctaaggcgttgttgacctgtttttctatggtgtcggcgtaggcgaagagttgctcgacgcggcgaacgatttcggcttgttcttttactggaggtaataaaacaacttgggatttgatatcttttcctgaaatacctttttgaccagaagttgttttcacgcagttcatcattgcatttcgtgctgagggggatgaaaaaaatatttcgatatattctggtaaagcatctttggttaatcgagctcgaataagtttatcaggatatagcaaattttgatgttgtaattttttcaataacccacaaacaccaacaaattctaaacttccgttatagcgagtaaataaaagatctccatcttgtaatttgtggcggtttagttcactttctgaacattctagaaaccgaatatcgttttgatctacatggccagcacgtacagaactaatgcgtagtattggatgaccaacaccactttcatttggctttgatgaaagaccattacgtaattcagttaagatagattcaaaatttaacttcttaaatacagaatgttgcggctcaaaattacgccatttttctgtcaattttccattaactgcgccccccaataccgcttgacgaaaacgtttcaggatttgtgggatttgctcaaaacgtgctttggtgctgtctacctgcgccagcagcgtatcgagtttttcagcgatgattttttgttcggcaagtggtgggattggtatatttatcaaatcaaagcttgccggcttaatattattaatatttgcaccagcagaaagtgatgaaattttgtttcgataaagagaagattttgtgaaatgagcaataaaaccagaaaatataagtttttcaggacgtaatacaccgcaaaatgcgccgaaactacattcaaatggtagatgctgatgtgcggatttaccaactacggatttgctccctgatgacattgcaataacaatatcttcaggagatattttttgactttctttaacaagatttttaggaacaaaaaccaagtccgtagtatcaaacttgccattctgaatattgttcgcacggataagaggcaaataatcatcttttagataatttattgcctgctcttttttatacgttactcctcggattagagttgtgaccgtagatactggggcgataacccacccctccggcaatttccccgcactcattccttcaccccaccaaacgcttcttccagcaactgacgctgcaaatcggcctcatcgctcgcccccagttcacgcatcagcgcatccagttcagacagcgcctgtaccagttcgcccatcgcttctgccgctaatacatccggctccggcaggctgtcggcatcaatactgtctttatctttcagccaggagatatccagcgaatcggattttgcggtgcggatccactcacggctgaacttgcgccagcggctggtagcaagatgctggtcggtgtttttgttctcttcgctgtcggcaacttccgtctcttcggcgttaaaactccattcaccttcagtgcgcgggcttaaaccgtgcgggtcttcgccatacacgcgctcaaacggctgcaaatgctcgtcggtaaacggtgtgcgcttgccgaaactcggcatattggtacgcaggtcatacacccacacatcatcggtacagttcttatcctgattcgggttcgccaccgtccctttggtaaagaacagcacgttggtcttcacgccctgagcgtaaaaaataccggtcggcagacgcagaatggtgtgcagatgacacttatccatcaggtcacgacgaatgtcggtgcctttgccgccttcaaacagcacgttatccggcaccaccaccgccgcacgaccgccgggatgcagcgtttcgataatatgctgcataaagcacaactgtttgttgctggtcgggtgaacaaaggtgcgggtaatgttggtgcctgcggcgctgccaaacggcgggttagtggcgacaatatgcgccttcggcaggttttcaccgtcgctacccagagtgttgcccagacggattgcgccgccgtggtcgaggttgccttcaatatcgtgcagcaggcagttcatcagtgccagacgacgggtgccgggcaccagttcgaggccgataaacgcgcggtggatctggaaatcctgcgtgtcgccatcaaggtcgtccagatcattggtttgcgacttaacatagcggtcggcttcaatcaaaaagcccgccgtacctgccgccgggtcctgcaccacttcacgcggctgcggtttcagcagatgaataatggttttaatcagcggacgcggggtgaagtactggcctgcaccagacttggtttcattcgcgttcttctgcaacagcccttcgtacatatcgccgaagtcatcgcgcgacttaccgtgcgcgccgttgtaccagtccagcgaatccatattgctgaccagtgcggttatttgtttcggctcggtgatggtggtactaacattatgaaaaactgcctgtaccagctttttgtcatcttcgcctaaatgcacgagcatttttcggtagaactgcaactgctcctggccgatgcgggatttcaggtcatcccagcggtaaccttccggcaggtattccgcttcctgaccggtctctttacacattttcaaaaacagcagcgaggcgagttcattgacgtagttttgataggaaacgccgccatcgcgcaggttgtcgcacagcttccacagcttcgcgaccagatcgttattgttcattgtgagttccgtaaattaagcagcggcccaaattcatcgagccgcagaagaagaaattgccgagggtaatatacacaaaatcattcaggttgcatcaaggcggcaagtgagtgaatccccgggagcgtacagaagtacgtgaccggggtgaacgagcgcagccaacgcagaggcagcctgaaggatgaagtgtatacgtgtcaggccagctcgtcccagatataatcgctgaatttgcccagcagggtatcgagattatcgtcaaaggttctttgcagcatcgccttcccgccgcgacggtggaagttgccggttttgaagacatcgtcgtcgagcaccactttctctttcagcgcctgcgctaaacgatcgagccagcttaattgctcgctgctccagtcgttttcgcccttaatgcgcgtcagcgcgtgatcgacacgttcctcaaacggtttcagcgcatcgcccaccgcagcgcggcgaatatgaccaatcagccgggcggcgatatcttcattgcgcgtctctttccatgctttgcgcagggaagattcctcaaagtgctggcggtcaaaccactcctgtagctcgaccagccctttacgggtgagatcgcgcgggcgattaataactgcctgcaatgccggttgcgcgttcggggaacgttgcaccagcgagtcaaaggcttcgaggaaatcctgcggcgtgtcgtaatcaccgtacagcgattttacactcaccacttcatcgtcgatatcgaggaagatcggcgcatcattcaggttgttgatgtccgttttcagcttttccagacgggcgataaagccaggcagtttgttaaagacttcggcgctccagtgcggccctttttcccgcaggcgcgaggcgaagccgttaaagttcacgcccgccgcgtcctggcatagctcatccagacgacgcacctgtttatctatcgtttcgctgcggtcacggttaaacgtggccagaccgatgatacgctggagcttcgccaccagttgttcatggctgtgctcggcaaaactgcggccatccgcttcggtgattttataggtttctgaatcggtaatttcattgaccagcgtttgcagttccaccttcgggcgcaccaccaccggacgcatggtgtcgacgctctccagcgtgctgtagatatcgacacagtcaaaaatcttaaagctggttttattcacctccgggcataagcgcgtggcgcggcctttcatctgttcgtacagaatgcggctgcgtactttacgcaggaacacgatattacagatcgacggaatatcgacgccggtcgtcagcaggtcgacggttaccacgatattgggcagccgctctttattgaagcgggtgatcatggtctgcactttgcgcgcgtctttatcggcatcaccggtgatcttgatgatcgcgtcgtgctccagttgcggatactttttcttgaacgcggcacgcagctcttccaccaccatatcggcatgggcattggtgacgcagaagaccagcgttttttgcgatccggtcgggtcaagataattggtgagttcgttacagacggcgcggttaaacgccgggatcaccaggccacggttaaagtcggcgacttcaaaatcctgatcgtcttccagggtgtcattgatcacttctccctgcgggctgatgcgctctacctgctcgcctttggagagataaaccccctcctgcgcgttgcgggtgatgatctgaataggcggatcctggtcgatcagaaaaccgtcgataaccgcggtacggtaggtataacggtaaaccggctcgccgaaaatctgcacagtatgtagcgccggggtggcggtgagagcgatttttaccgcatcgaagtgatcgagaatgcgacggtaggcagagacgtaatccagctggctgcggaactgcagttcgccttcggtctgctctttatcgagaatatagccgcgatgcgcttcgtcaacgacgatacagtcgtaacgggccaccggcatcggttcatctgattgcagggtgcgtttcaccagcgactgtacggtggcaacgtgaattttggtgctgtcttccgggaatttatccgtcagccctttaatgtcgaaaatgctgttgaaggtgtcgccgttaatacgcgtatcttcaaacgcgcccagcgcctgttcgccaagagaacggcggtcgacaaggaagagaatgcgtttaaaacgctgggactggatcaggcggaacatcatggcgattgccgtacgggttttaccggtaccggtcgccatcgccagcaggatctcttgttgccccttgacgattgccttttcaaccgcgcggacggcatcttcctgataataacgcaggcccagctcgctcatgccagggttatcggcaaaccactgattctgtttttgcggttcgctgccgagcatttccagcagctcttccgggcggtgccactcgggtaaggctttcgacatattgcgggtatcacgcacgtcgcgataccagatgccgcttttggtcttcattgttgcgcggtattcgcgcccgttggtcgagtagcagaaggggattttaaaccgttgtttgccgctggtgtcctgccagctggtttcatactctggcactgcttcatgcacttcatccggtgagtagtgctcaagcaaggtttcccgcaggaagccattatcgaaacatttactgtagcgatacgactcattgagcctggcgggaacgtcgatattgttacgtttcgcctctaccaccgcgatgggtttgaggccgacaaacagcacataatccgcaaagccctgattacccgtttcatcttttccggtcggccattcggcaatggctttattgacgccgggttccggacgtgcgcctttggagaagcgcagggttttgctgtcggcctgccagcctgctttacgcagttgcgcatcaatcaggaagcgactctcttcttcgctaaggttgagtgtgcgcttgatggcctgatcggtaatttctttgtggtaagccttacgttcctgttcggtctgttttgccagttccgcgttcttctcggcgagctgtgcttccagtgccgcaaggcgagcctgggtttgcgcttcggtttcctgctgtttgccttccagaatggcgatatagccgttcagggcaaccagcttctgctgttgcgcttcgacttctgcctgagtctgcgctttttctcgcacctgctgttcaagctgttgttttagcgtcagcacttcctggtgatagaggttttcaccacgttccggcaacacaaacaccggcaccgggaagtcataatctttagtgaccagacggtagtaccagacagccaggcggaacccgagtcgcaggcacatctgggcatcgttgagatcgttatgatattcgtgcaccgcctggttaccaatgcggcgtaatttgtgaaatacagagaggatgttgtcatcaacaaaggcgattttgccgagttcacgcaggagatcgtgttgattctcacaaggggggatgttgagtaacagaccaagatgtttcgctgtggcttcgccaaacatacgcattttaatcagcgtcgtgttgggatcatccgggtagttattttccgccgcacaggcgatggcataagtgaagtcgttgacgcccttcaggaattcaaaattggatttattcatcattgttattaatccattgctgtgcgggcctgtccaaatatttaaggcccataacatctcatcttagctttctgtacctttccgggcaatgaccacggtcacagcaactgactcatttctaacgtgttcgtctatttttgtagtgctatagtagccgaaaaacatctacctgattctgcaaggatgtactatgacggttcctacctatgacaaatttattgaacctgttctgcgttatctggcaacaaaaccggaaggtgcagccgcgcgtgatgttcatgaggctgccgcggatgcattaggactggatgacagccagcgagcgaaagtcattaccagcggacaacttgtttataaaaatcgtgcaggctgggcgcatgaccgtttaaaacgtgccgggttgtcgcaaagtttgtcgcgtggcaaatggtgcctgactcctgcgggttttgactgggttgcgtctcatccccagccaatgacggagcaggagacgaaccatctggccttcgcttttgtgaatgtcaaacttaagtcacggccggatgccgtcgatttagatccgaaagccgactctcccgatcatgaagaacttgcaaagagcagcccggacgatcggttagatcaggcgctaaaagagcttcgtgatgcggtggctgatgaggttctggaaaacttattgcaggtttctccttcgcgctttgaagtcattgttctggatgttttgcatcgcctggggtatggcggccaccgtgatgatttgcagcgtgttggcggtactggagatggtggcatcgatggtgtgatatcgcttgataaacttggcctggagaaagtttatgttcaggcaaaacgttggcagaatactgtaggcaggccagaattacaggcattttacggcgcactggctgggcaaaaagcgaaacgtggggtgtttattaccacttctggatttacttctcaggcgcgtgactttgcccaatccgtcgagggtatggtgttggttgatggggaacgcctggtgcacttaatgatcgaaaacgaagtaggggtttcttcacgtttgttgaaggtgccgaaactggatatggactattttgagtgaaatatcaggccggatgcggctgcgccttatccggcccataaccccttacttcctcaaccccgcaaacgcagcccgaatctcttcctccggcagctggatcccgataaacaccatcgtgctatgcggtttttcatcgccccacggcctgtcccagtcggcgctgtagaggcgctggacgccctggaacagcaggcggttaggttcgccgtcaatccacagcatccctttgtaacgtagcagtttatccgccgactccagcagcaggttttccatcacgcgggaaacttcgctgatatctaccgggtaatccagttccaccacaatcgacgaaatatcgttttgtttatctgcgataaagtggaaacgcggtttggtgctgacgacgttttcttccagcataaaaccgttggtgttgaacagcaggcccagatcgatgtcgccgtgggtgacggtgtagaccggtgcgcgggcgttgatgcgcgccaggcgttcatgcagtttttctgcttcgcctgcgacgtcggttttggtcagcagaatgcggtcggcgtagccaacctgtgactgggcgatggtgaactggttcatctgctcatcggcatgtaccgcatccaccagcgcaatcacgccgtccagcagataacgctggcataaaacttcatgggagaaaaaggtctgaataatcgggccgggatcggccatgccggtgcattcaatgaccagacggtcgaactgaatattgcccttgtcgagattgtccagcaggtcgagtagcgcgtcctccagctcgttggagcgcgaacaacagatgcagccgttggtcagcgttttgatctgcgtggcgcggtcgccaatcagttgatcatcaacagagacttcgccgaattcgttttcaatcacggcaatcttgtagccgtgctgttcgttaagaatatggcgcagcagggtggtttttcctgcgcctaaaaaaccggtgagtagggtaactgcaatcgggttcatgctctctccattaacaacagcgcataccgcctttaccatcgccgccgtagcgcgcgttctggcgttcgcggaagaattcttcatagctcatgtacggcttgtcgggatggttggtcttcatatgctcgacgtagttgtcgtagtctggaatgccaatcaacatcttcgccgcctggccgagatatttttttgcctgtcctaagttaccaaacatagttcactctgataagaacaaagccccgccgaagcggggctaaacacggttagtggtgcgaagagatcttcacgccgccttccgggattggaacgtacggtgtttctttgtcagtacgtttgtcgctgttacgcaccgcaagccaggttttgaaaccgtagaagatgatgctgtacaccacaatcaggaacagaatactcagacctgcgttggtgtagttgttcacaacgatgtggttcatattggcaatctgctgcgccgtcaggtcagtaccgttagcaatcttctctttgtactggcttgccatgtagaagaagccttccatctgcgggttggtgctgaacagtttcaggcccagcgcccaggtggtgcagataagcagccatacagccggaacaacagttacccagatgtattgggtgcgcttcatcttaatcagcacaacggtgcccagtaccagcgctacggctgccagcatctggttggagataccgaacagcggccacaggctcttaacgccgcccagcggatcaaccacgccctgatacagcaggtagccccacagacccacacagcccgcagtaccgatgataccggcaaccagagaatcggtttttttcaggaacgggatgaagttacccagcaggtcttgcagcataaagcggccagaacgggtacccgcatccagcgcggtcaggatgaacagggcttcgaacagaataccgaagtgataccagaagcccatgtcagccatcggcagcactttgtggaacacgtgcgcgatacctaccgccagcgtcggcgcgccacctgcacggttcaggacagaaggctcaccaatgtctttcgcggtttgcaggatctgctctggcgaaatcacgaagccccaggagctgacggtcgctgccgcgtgtgcggtaacgtctttcagctgcgccatgatgatcggcgcgttctcgccacccatttcatgcaggttaggcatggtgatgccaaggccagcaggcggggtgttcatcgcgaagtaaagacccggttcgatgatggacgcagcaaccagcgccataatcgccacgaaggactccatcagcattgcgccgtagccgatgaaacgcgcgtcggtttcattagccagcagttttggcgtcgtaccggaagagatcagcgcgtggaagccagataccgcaccacaggcgatggtgatgaacaggaacgggaacagagcgcctttccacagcgggccagtaccgtcaatgtactgggtcatggcaggcattttcagttccgggttcagcaccacgatacccagcgccaggccgacgataacgccgattttcaggaaggttgccagatagtcgcgcggtgcgaggatcagccacactggcagcagtgcggaaacaaacgcatagccaatcagcgcgaaggtaatggtggtgtctttaaaggtcagtgccggaccccagtacggatcgtgagcaatcacgccaccgaagtagatagaggcaaccagcagcacgataccaatgacagagacttcacccacacgccccggacgaataaagcgcatgtagatacccataaacagcgcaatcggtacggttgagcaaacggtgaagacaccccacggactttcggccagggctttaaccacaatcagcgccaggacggcgaggatgatgatcatgattaagaaacagccaaacagcgcgatagtccccggtactggtcccatctcttctttgatcatctcaccaagagatgcgccattacggcgagaggagataaacagcaccataaagtcctgaaccgcaccggccagcacgacccccgccagcagccacagcgtgccaggcaggtagcccatctgcgcggcgagaaccggacccaccagcggaccagcaccggcgatagcggcgaagtggtgaccaaacaacacgtaacggttggtcggaacgtagttcagaccgtcgttgttaataaccgcaggcgtcgcgcgcgtggggtcgagtttcatcaccttctgggcgatgtacagactgtagtagcgatacgccaccagatacaccgatacagaggcgaccacgatccacagggcgctgatgtgctccccccgacgtaatgcaactaccgcgaggcagaatgcaccgatgattccgagaatcacccagggtatgtgcttgaatatctttttagtatccatagtaaaacctggcatgtattgattaatagttggccgaagccgttctaggtttgcgttgcgtttgaggaggtaaattgaccgctatcctgtagtgatgttgccagagttacgcgcgcgtaaagtaaggtaaataactgagtggttattttagggatgtaagcggtcagttttgcggttgagcggcaaaggcgtcgtttaagtgacgataaatatgtgattcatatcacatatttatattgtgaataatttatgtaaataatggctttttaaattcagagtgtgaataaaattcactcggcgtaatctccgcgggatattcataaagtttttcctttccaggccgaaaatcttgcatcggtccacaggaaagagaaaccatgttaaaacgtatcaaaattgtgaccagcttactgctggttttggccgtttttggccttttacaactgacatcaggcggtctgttctttaatgccttaaagaatgacaaagaaaatttcactgttttacaaaccattcgccagcagcaatccacgctgaatggcagctgggtcgcgttgttgcagacgcgtaacaccctcaaccgcgcgggtatccgctacatgatggatcagaataatattggtagcggttcaaccgttgctgagctgatggagagtgccagtatttcgctgaaacaggcggaaaaaaactgggcggattacgaagcgttgccgcgtgacccgcgtcagagcaccgccgcagcggcagagatcaaacgtaattacgatatttatcacaatgcgctggcggagctgatccaactgttaggtgcaggcaaaatcaacgagttctttgatcagccgacccagggatatcaggacggtttcgagaagcagtatgtggcttacatggagcaaaacgatcggctccatgatatcgccgtcagcgataacaatgcctcctacagccaggcgatgtggattctggtgggcgtgatgatcgtcgtactggcggtcatcttcgccgtctggttcggtattaaagcctcgctggtagcgccaatgaatcgcctgattgacagcattcgtcatattgcaggcggcgatctggtgaaaccgattgaggtggatggctctaatgagatggggcaactggcagagagtttgcgccatatgcagggagagctgatgcgtaccgtcggtgatgtgcgcaacggggccaatgccatctatagcggtgccagcgaaatcgccaccggcaataacgatctctcttcgcgcaccgagcaacaggccgcttcgctggaagagacggcagccagcatggagcaactgaccgcaacggtgaagcagaacgccgaaaatgcgcgccaggccagccatctggcgttaagtgcttctgaaacggcgcaacgcggcggtaaagtggtagataacgtggtgcagactatgcgcgatatctccaccagttcgcagaaaatcgccgatattatcagcgtaattgacggcattgccttccagaccaatattctggctttgaacgcggcggttgaggctgcgcgtgcgggtgagcaagggcgcggttttgcggtggtcgcgggagaagtgcgtaatctggcccagcgcagcgcccaggcggctcgtgaaattaaaagcctgattgaagactcggtggggaaagtggatgttggctctacgctggtcgaaagcgccggggaaacaatggcggagattgtcagcgccgtgacccgcgtgacggacattatgggcgaaattgcttctgcttctgatgagcagagccgtggtatcgatcaggttggcttagcggttgctgagatggaccgggtaactcaacagaacgccgcgctggtggaagagtctgccgctgccgccgccgcgctggaagagcaggccagtcgcctgaccgaagcagtggcagtgttccggattcagcaacagcagcgtgaaacatcggctgtggtaaaaaccgtgacgccagctgcgccgcgtaaaatggccgtggcagatagcgaggagaactgggaaacattttaatcgccatgaaaatgcccgataagcaaaatgttatcgggcataaggagattaatctttacgtgggtcgttgatcggctgacgaaccaggaagatgtacgccagtgcccccgctgcggtgacgcaaccgcagatgattagtgccagacggaatgagtgggtggtatcaacaataaaaccagtaatgatcggcgcaaaagaggcgcagatgaagctggcaaagttctggatactgcccaccgacgcagtcatgcgagaagcaactgcgacgtggatcaagccccagcaggatgttccggcaaagtgaatacagaacagtgccatgccaatcagcagaaccgccgtcatggatgttgtcgcttgtggtactatcagcgtaaaggcggcagaacagaacatcccggcaataatgcagatcttacggcttttaatcggagccattccccctttgaccagccagtcggtaacgtaaccgttgaccagcatcccggcagccccaaacaggaaagggatagccgccatcaaccctgtgctttttaaatccaggttataggctgtttgcaggtaaccaggaagccaggccagatacagccacgcagtgtagttgatgccactgaatccgagcatcattccccacattgtacggttacggaacaggctgcgccattcggcaaaactgagcggatctcggcgggcattgacgctacctgcattgagataagcttgctcaacggcagtcagttctacgtgctcgcggttgcgatagagcatataccagccgatggcgagaaaaatccccagtacaccaatggtaataaacatcccgcgccagcccatcaccagcatcatcgccgccagaatcggtgggcttacggcaacgccaatggtagaagctgcgttgaagaagcccatcgggcgtccgcgctctttgatgttgaaccagtcgttaatgacttttacaccgcatgggttcatcggcgcttcaccaatccccataccgatacgcaccaacacgaactgcgtaaagttgtgcaccatgccagacattgcctggaacagtgaccagaagaacatccccagtcccagcatcaggcgtgggcctttacgatccaatagtgggccgcaaggaagttgcgcaatcccgtaagcgagtgaaaacacggagagcaaagcgccgatttcggtggcacttaatcccaattcttcacgaatcgttaaatttgctaccgacagcgaactgcggtcgagataattgattaccgccgcaaaaaataataacaacatggcggtggtttgaatgcgtttaattcgggtactgcgttgaactaatccatctggtggcacgggaatatctgccgacgaagatggagtaaatgaagaacgcggatcgatggtgatattttctttttccacgccggactcctgtatttataattttaattgtttacgtaattgtgcattacgcaaggttgacattaacggcaggttaaagttttaggactttactaccgctcacaaaaacatttttagtcgactgattgtgagcataggtaagcgggaatttcccggtatttatcttttgataaaaccgtgcacccgctaatagtttgctgtttttaatccgtacttaatgagcataacgcgtgttctcattaatggatcgaatcattgattgtttagctgaattcaaatggttacggagcgcaagggtggcatcaaggtcactgcggcaaatcagagcgctgagaatggtcatatgctcatcgacggcaatgatattgcgctgtttaagatcgctttcgtcccattgatagtgaaaatgaaagatgactgagatgatctcaagcgattgatcaaaaaagatattgtcggcagctgaaagcagtaaggagtgaaaatctctgtcaagttgcgagaacatgcgaaagctattgccgatgttgtcacgcagtagccgatgacgttcgagcatggttttcgcctgcagccagcggggatcatgatcaggcaggttgagaaagtgctgaagtgaatgtgtttcgagcatttcgcgtagctcaaacagctgctcggcgtaggattgatcgaattgcttcatgctccactggccgcgcttttcgctgtgaataagattataacggccgaattttaaaagatattctcttactacaaccgggctgacacccgcggcccgagccagttgcagttcagaaaacgtttcccctgggcgtaactggcgctggtttatcatcgtgaaaaaagcctgctcaaacactttgttttgttcactcattgaagcggtagtacaggcgaaaccgtcatcatggtcaggtttacgcgcaataacatagtcgtttccaacctgcgtcaagacgccgcattcgcgtaagtggctgagaatatgacgcactgtggtgcggctgatgttgtacatttccgccagcgcactttgcgatggaagtggggaagggatatgaccccgcgccatatcatcaatgacctggttaatcacattgtggcgtaaattttgtgaacgactcatattttcctccttgtgagtccattaaaacccgatttaaaacatttttatgcgtgtgttttcacaaaaaagattttccgttccgctgccatttttcattttcattgatatctaaggcaacaaaaagtggagagccgaatcatgtctacgatgaatgttttaatttgccagcagccgaaagaattagtctggaaacaacgcgagatacctattccgggtgacaatgaagcattaataaaaattaagtctgtcgggatttgcggtaccgatattcatgcctggggtggaaatcaaccattttttagttatccacgtgttttaggccatgaaatatgtggggagattgttgggctgggtaaaaatattgctgatcttaaaaatggtcagcaagttgctgtgatcccttatgttgcctgtcagcaatgcccggcgtgtaaaagcgggcgtaccaattgctgtgaaaaaatttcagtcattggcgtgcatcaggatggcggttttagtgagtatttgagcgtgccggtggcgaacattttgcccgcagacggtattgacccgcaggcggcagcattgattgaacctttcgctattagcgctcatgcggtgcgtcgcgcagccattgctcccggcgagcaggtgctggtggtcggggcggggccaatcggtctgggcgcggcggcaatcgctaaagccgatggcgcacaggtggtggtggcggataccagtccggcgcgccgtgaacatgtggcaacgcgtctggaattacctttactggacccgtcagccgaagattttgacgcgcagctacgggcgcagtttggtggttcgctggcgcagaaagtgatcgacgcgacaggtaatcaacatgcgatgaataacaccgtgaatttgattcgtcacggcggcacggtggtatttgtcggcctgtttaaaggtgagttgcagttctccgatccggaattccataaaaaagaaacgacgatgatgggcagccgcaacgccacgccggaagattttgctaaagtcggtcgactgatggcggaaggaaaaatcactgctgacatgatgttaacccatcgctatccgttcgccacgctggcagaaacctacgagcgcgatgtgattaacaatcgtgagttaattaaaggcgtaattactttctgataaggcgagattattaaagttgccatgcagcgtccggggaagtgttgggcgctgttttttttgtttcttaataatgtgttgtaagccgtagaaggcgtgtaggtcgcaccctatgcgacctacacatcagtcaggaattacccttcacgttctaccactttaatttccaccatgccgatcccgagcttacgcggcgagtgtccgaggatattcccttcgttggttgagacaggttccggcggcacaattaccagtgtgtcggcatcggttgggttatcgaaatgcagtgtggtggtggtcacttcattgcccagcacaagagtttgttcttcattgcctacgcgtaccggaataggacggctggcgttattgccgtatgctttggcggtaatcaccaggtcaaatttcttcggcagcggatgcttgtactcgatttttacttcatcgcccagctgcgcgttggaccagcggccccacgactccggacgggaaatcccgctaaactgtttcacctcttctggcgcaccggcgacgttaaagatgaaactgtcggctttgtagcgaatatcgttatcaacaatcttcagcgtatcgacattgcctttgtaacgcgccatgtcgatgaccgtatctttaaatgccgttttgccctgccatgttgttttgtcaacatgctgaacaatttgctgaccgccaagctgcccttgcgagacacaccagtcggtggaaagtgccagttccggagcccagagttgtgccatcttgtagcaacggtcaacccagacgaaattgtcgcgtggagcgaaatcggccagctggaaacgcagcggtgctgagtattcgctttccggcagcggttccacgcgtttgtctgaaacccgcaacagcagcggcaaacggaaatggctacccgagaaggcaatcatgtttttctgctggtcgatggtgaactctttcatctctttagggaatttccacaggcggatgatatctggcttccacgccaatgttttctctttgatattgaggaagatttccgacatcgactgcccggataaactgctacgaccaagtccgagatagttatcgccaccgagaatgtccagcaccgtcgcgccgttatccatcgtgttacgcttcactgccagcgtctcttgctgcggcttgtcgccacgaatgacaaaaaacaggttattgcgatcctgcttattgaggtatttccacgccgtgttgttcatcgctaaatggtcagaagagacgacgatgacggtatctttaaaccacggtgacgctttgattttgttgataaacgtcgcgatgttctcctggctgcaacttaccgcgctgaatgactgattcggtttaccgtcaaaatcatattttttgcggttacaggtacgagagataaaaccatccgggtgatgggtatcgactgtcagggtaaacagtgagaatcgctgacctgagcgggaaagctcttcaaactttttccacgcttcatcgagaacggtatcgtcgtagaatccccagtcgttgcgatagtgcgggtcggctaccacgcttttcagctcttctgagccgtataagtggtcgaagccatgcgacttcaggaacacatctttaccggcaaaacgcagattcgcgccctgcacgaaatagttctgataacccgagtttttcaggatatctcccagacagatgttctgcgggaagaagctggagacagaggcggaggcgttgccttcaaagggggcaaacagcggtatgccgcactgagaagccaccatgcccgcaatcgtgtaatctgttcccggcagctgctgcgtgtggctgaaatccaggccttcatttttcaacgcgcccagttcaggcgtgagatccgggaaagcctcgttatcaaaataggtccgctcgagactttcgccgtagatataaaccaggttgagtttcgggtcagggatagttttcgacggctctttataataagccgcaaagtccgggtcgccgtcgcgtgactgggatttcaccagttccgttatctgacgaaatgccgggctggcgtccaccgaacccagcgccagtaagagcgccagcaggctgtaaccaaaatggtgcggatgatggcgacgacggcgcaggatccagcccagcgcaccgaacaccgctgtcagccccagcacaatgccgatacccggcaaaatgtatttgctgacgccagcaccggtcaggctgttggttaaggtatagagaaccgcgtcgttaataccatcgccagtaaaatagtcgctggcaaacagggtgatatttaaaacgacaaatagccccagcaccgttaacgtggctgcaaaccaccaggtgttacgtcccgctttccatgcgtaaatcagcacagaggcgagaaaaagggcgaaagagagtagttctgacaacgggcgatcctcactaaaccgggccgtttagccaacgtttaagctttttgagaagcacaatgtaatggcgtcgccatattgctgcaattctagtgtcaaaaaaatgcgatgttgttaggaattagtttataaacagacttttttgattacggtcacttcccgtgtaacaggggtaaaaccgtccaggagcagggaaaagggcaggagagagccgcgtcagccgggtaacagctaaaacgcggcgtttcgcggttcaggaaatgaagttcagcccctgttttaacaccagatcgcaggctttggttttcaccttttctgccagcggagttgttccgatgttatccagattgagttgctgaccatctttggttttcagcaaaccctgaatgccgtccagatagttggtgtcttctttttgctcttcactgttcaggcccagcttttccagcacctggttcttgatgttttcggcatcggttaccgacgccagcttttgcttcgcgcagtattgcagaatgcctgcggcattgttcatgttatctgcgcttaaggcctggtttccgctgctaagcaagttagttaatgacgcgagcgaccaaccgccttcctgtgtcgtgctgttttggttgccaagttcgctggcggcgctggagagcgcatctttccaggacgcagcatgcaccccggtggaaattaatgcgctggcggcaatggcacagcacagaagatgtttaacagttttcatcatcattactcaaggtggaattgtgtcgcagtataccgccagaaacggggattaatactctttacctgttacccggctacggtagctatcccagttgaagatcacccacaaactgttacccaggcgcatacggtccatcacgcgttcgcccagcaacttggtcatctcttccatattactgttggtcagcatcccggttgggcgtttggaagaagagcggcgatcgacgatctggttgatgatcactttttcgtatttcgattcggtctgcacgccgatctcatcgatcaccagcagatcaacgttgctcagatcgttaagcagttgttcttcgctggtaccgctattcctgaaggtatctttcatcgccgacataatatcggccacggtgatgatcaatacggatttaccgcgtagcagcagctcgttgcagattgccgccgccagatggtttttgccggttcctggcttaccagaaaagatgaagctggcgatgttgccgtcaaactcttcgacatactggcgcgctttgcttaacgcattcatctgcccttcacactcaacgcgatagttctcaaaggaacagttctgatgcagtggacgaataccggagcggttaaaggtgcgctgcattttcatcgcccgattttcacgttcgagagcggcggagcggatcgctccttgttctttttgccaggccagtagttcttcacccgttttgaatgcgggtttgatatgggcaggcatcattttttgcaggcgttgcatcaggtcgccaacgtttttcatcgttaccctctgaatcctggtggaatttggctgtcaggttcgctgaccgtattcacatctcgtttcggcagtccgccgttgctggcacgaccgatttgcaggctgcgcgccagtttttgttgccactgcacatggtgaaagactttaccttccgcctgccagtaggcaatgaatgaggccagttcttcggtggtcaccggctctcttagcgccacgccccatagcgccgccaggcggataaaatcggcatcgggttgccagtccggatacatggcgaatttccccatgggtacagcaacgggagcggcttgcggttcctgatagagttgatcgtccagagcgacatcgcttcccggacgcgccagcttttcttccagcgccagcagttcagccaggcgtgcaggcgtgacggcataaaacgccggggcattgttagcaaatacggcaaccacaccgccttcagcttttgccagaacggtttggtgatcgtgtaccagggcgtcaataccaacgacgtccggggtcaaaactctggaagacatactgtttctcaaatatggaacgatgaacgagaagggagataacttttatagtaacacacggaggagaggaggctgtctctcatccgtgtgcttaagcgaggcaattttatacgcgagggcgcttgcggtacaaccataatccaggaatggaaagaccgatggataacgcaccaacaatcgatgaagctgtaagaaagttggttaacagggtaatcatcaacggttcgctgtaacctaactggctgatttttaccgccgaaatcattgcggtataagccgatatgcccgggaacatagggataacggccgccacggtaaacactttcggatgcgccagataccagcgcgaccattgaataccaatggtaccgaccagcatagaagccataaaggttgaccactcaatattcaacccgctggtcatcaagatcattcgggaaccatgacctatcgagccaagcagcgcacaccagcgtaacgcccgcacgggaacgttgaacaccatcgcaaagccgaccgcaggaatggcggcgaggatcatatcctgcgccaacgctaacagaaattcgatcacacccatccgcgtagcccccaaatcgtcagtgccatcactacgccgacgcaggtagccagtgtcagcagactggcgatcgcccagcgtgccagtccggtattgatgtggcctttaaacatatcggcgacggcattaatcaacggaaagcccggcactagcagcagaacgctggcggccatcgcaatggtgggggtattgctgaaagtggggagttgcaaaagcaatccggaaatggtggtggcggcgaaagcggtaaggcaaaagttgatctgtggatgaagatgacgttgtgccagcagctggcggatatacatcgcggtcgtactggcaaagaaggtgatgacggcaccatcccagccaccgttattgagtttacagaaacaggcgcaagaaaggccaaccattaaggctaccagccatcttgggtaacgtaatggctgaatttggctaaatcgtttctctacgcctttgtaatccagcagatgatgctccgcaagaatcacaatgtgctggacttcagtcaccacatgcatattaatgccgcgatcgtgatttttacgtgtcgatgtcaggcattgcccatctttaatagttgtcagcactatggcgttcgaagagatagaactttcgacgctgtccattcccagtgcccgacccagtcgtgaggaaagctcatcaaccaacgcgctttccgcaccatgttgcaaaagaaataatccacactggatacaaagccgtgttacggctcgctgttgctcagtttgcataactcgccctttgtcatagacgtgctgcgtattgttcagataatgagaatccatttgtatcatgaagcacggttgttttgcggtaggttaagatcaaaattgcgctgattaatcctggttatcgggagaagctcggtgataaaaagcgaattatctctcgccgcaaacaaactatcacatgaatattatcatcataatgaatttattgtttggcctttacgaatcaggataatagataaccgggcacgttttttaatgttaacaagctaaaaccatcagatttcattgaataaatattggttgtgtgattttgcattctgcgggaagggatatcatttaattataaattaaatgaatgtgatttctgtttttcattaagtattcctaacaacttaatgtagatattttaaatgtctccaggctatttcaccaggttatcatttgatgctaaccttctgacacatgcagtggagttgttgtgcagcaggagtatgctgatatgaaagtgaatgctaaggataatttattcgcttaatctattaatttgctggaaacatttaaggaatgaatatcctgaataaaccatcataatttttagacagtggatgtggaggaaatatgttgccaggatgctgcaaaaatggaattgttatcagtaaaatacctgttatgcaagcagggttaaaagaggtcatgaggactcacttccctgaatatgaaataatatccagcgcctctgcggaggaccttaccttattacaattacgtcgttccggattagtcattgctgatttagccggtgaaagtgaagatccacgttctgtttgtgaacattattattctttaatctcacaatatcgggaaattcactgggttttcatggtgtcacgctcctggtattcccaggcagtagaactgctcatgtgccctacggcgacgttattgtctgatgttgaacccattgagaatctggtcaagaccgtacgttccggcaatacgcacgcagagcgtatcagcgccatgctgacctccccggcaatgactgaaactcatgattttagctatcgctccgtcattctcactctttcagagcgcaaggtactgcggctattaggtaaaggatggggcatcaaccagatagcttcattgcttaagaaaagtaataaaactatcagcgcccaaaaaaacagtgcgatgcgtcgactggcaattcacagcaacgctgaaatgtatgcatggataaatagcgcgcagggtgcaagagaacttaacttgccttctgtttatggagatgccgcagaatggaacacagccgaattaagaagagaaatgtcgcactcatagaaaaatgcgtcatgagtagtatcggtattgagagtttattcagaaagtttgcgggtaacccttataagctccatacctataccagtcaggagtcatttcaggatgccatgtcgcggatctcgtttgcggcggtcattttttctttttctgccatgagaagtgagcgcagagagggattatcttgcctgactgaactggcgattaagtttccgcgtacccggcgtttagttattgcggatgatgatattgaagctcggctgattggttcattgtcgccatcaccgctggacggtgtattaagtaaagcgtcaacgctggagatttttcatcaggaactctttttgtcattaaatggtgtacgtcaggcgaccgaccgactgaacaatcagtggtacattaaccaaagccggacgttaagcccgacggagagagaaatattgcgctttatgtcgcgtggctactcaatgacacaaattgccgagcagcttaaacgcaatatcaaaacgatccgtgcacataaatttaatgtgatgtcgaaactgggcgtcagttctgacgcagggttgttggaggccgcagatattctgttatgtatgcggcattgcgaaacaagtaatgtgttgcatccctattaatccgcatgatgccgggtttacttccccggcagtgctttcatttcagcgtacaatcgccacattgctgcacatccggtaagcgataacgctggcagcaagtgcggcgcaccagcaggccgtcgcgcagtaccacggtacgccagagtggattatcttcaccgttcgtgagcgttttctcaaaaaagagggcatggcgcagcgattcaacagtagcctcgccgagcagttgcttcatctcagtgagataccagttgatcaaataaccggtattactccagataagtttgccgttgatctctccggtcgcttctagtgcttgcacaaccggaaccagcgcctggctgattaacgtttccattcgatgctgcggcgaatgtggtgttgcgtttttatcttcacacacatcgacccagaaacaggcgacgcgtccggtttcgtgaaactcagcatggaaatgttccggcgacacatctaatgccttttcctgcgtcagtagcgccagcattaatggtggcaccatcaggccgatataccattgtgcccatagtgagatcagcggtttgttctcgcggatcatcatcggttggttgcgatagatatgatcggaatagaccgccagcagagaacttagcacattcggtgatgaccattgcgccagcgtcatggcgttaagtggggcaggttcatccaggcggataaactccagcaaatgttcacgatgttttgcgatcgtcgcccgcacggcttgcgcaagcgtgggatcctgcggctggagatgcgttcgccagatgacatcttcatagagcggtgcggaacgataggccataatcgggatagtaatctaaatgataatgattgctaatcatagcgataggtttacccgatagcaagggatttatctggcttgcaaatgataaaaattatcatatgatattggttatcattatcaatgaaagagatgaaatcatgttgcaacgtacgctgggcagtggctggggagtgttgctgccgggattgctgattgcagggctgatgtatgcggatttatcgtcagatcagtggcggattgtcattctgatgggattagtattgacgccgatgatgctgtatcacaaacagttgcggcattacattttgctaccatcgtgcctggcacttattgctggcatcatgctgatgataatgaatttgaatcagggatgaaaaatcaaggaagaaacaagaaaggaagtaaagataattggtgcgaggggggggacttgaacccccacgtccgtaaggacactaacacctgaagctagcgcgtctaccaattccgccaccttcgcacagtcatcttactttttttgatatcgcctcgtttggtgcgaggggggggacttgaacccccacgtccgtaagaacactaacacctgaagctagcgcgtctaccaattccgccaccttcgcccagtgcgagcaatatcaacgtggtttttggtgcgaggggggggacttgaacccccacgtccgtaaggacactaacacctgaagctagcgcgtctaccaattccgccaccttcgcataccatcaattcttaaaaagaattgctaccacggaggcgcattctagtggttttcagcttttcgtcaatagttaattatcgacagaggtgtaattgctggaaaaatgtccatcaggaaactagcgtgcaggtttggtatgcatgcgggggcagatgccagatgcgacgctggcgcgtcttatctggcctacgaagggctaacgtgcaggttttgtaggtcggataaggcgttcacgccgcatccgacacggtattcggcgagataattaacctttcttcgcctggcgggtcataatggcgcgatacaccttgaagcgccctgtttgcgcgatcacttcgtggaagccaaatgtctcatccagcacgtccggataaggcaggaaggcgttcgctacaattcgcagctcgccgccgctattaagatgacgcaccgcaccgcgaatcagcgtttgcgccgcatccaggctggtttgcatcccatcgtggaacggcgggttggagatgatcatatcaaaacgacctttcacctcggaaaagacgttgctggcaaagacttcaccttcaacaccgttggccgcaagtgttgcgcggctggcttctaccgccggggcagagacatcgcacaaggtgagacgaattttcggcgaatggcgcgcaaaggcaactgaaagcacgcccgcgccacagccgacatccagcactttacctttcgtgtgcggagttaacgtcgagagcagcaactggctaccgacatccagaccgtcgcggctaaacacgccaggcagcgttttgaccgtcaggccatcgacgctgtattcgccccagaatttctccgcatcaaataccggctgtttttccagacgaccaaaatagaggccacagcgacgagcgctgtcgactttattcaacggcgcataatctgccagcatctgctcggcgctgcgcacgccgctgcggttctcgccaacgacaaaaatatctgtccccactggcagcagagaaagtaaattcatcaactggaactgggcttccggtttgttcttcggccagtagtaaatcagcgtatcgcaatctgcgacgtcatccgccgtggcgaccagactgaaacgggcgttatcccccatctggcggcttaatacctgccagtggtggaattgctgggtatgagcacggctggccgcggtatctaaacgcgcgggcaggtcatcctgtaagtctccggcaaacagaatacggctttgttcgaaatcatcactgtgacgcagcaagacttcacttgccggggtaaatgcagacatggaatgctcctcaattgatactggcggcgattatagccatatgttggcgcggtatcgacgaatttgctatatttgcgcccctgacaacaggagcgattcgctatgacatcccgacgagactggcagttacagcaactgggcattacccagtggtcgctgcgtcgccctggcgcgttgcagggggagattgccattgcgatcccggcacacgtccgtctggtgatggtggcaaacgatcttcccgccctgactgatcctttagtgagcgatgttctgcgcgcattaaccgtcagccccgaccaggtgctgcaactgacgccagaaaaaatcgcgatgctgccgcaaggcagtcactgcaacagttggcggttgggtactgacgaaccgctatcactggaaggcgctcaggtggcatcaccggcgctcaccgatttacgggcaaacccaacggcacgcgccgcgttatggcaacaaatttgcacatatgaacacgatttcttccctcgaaacgactgatttaccggcggcttaccacattgaacaacgcgcccacgcctttccgtggagtgaaaaaacgtttgccagcaaccagggcgagcgttatctcaactttcagttaacgcaaaacggcaaaatggcggcgtttgcgattacgcaagtggtgctggatgaagctacattgttcaatattgcggtcgatcctgactatcagcgtcagggattgggaagggcgctgctggaacatctgatcgacgaactggaaaaacgcggcgtggcgacactatggctggaagtccgtgcttcaaacgctgccgccattgccctgtacgaaagtttaggctttaacgaggcgacgattcgccgcaattactaccccaccacggacggtcgcgaagacgccatcatcatggcgttgccaatcagtatgtaatacaaggtggaataatgaagtgggactggattttctttgatgccgatgaaacgctgtttacctttgactcattcaccggcctgcagcggatgtttcttgattacagcgtcacctttaccgctgaagattttcaggactatcaggccgttaacaagccactgtgggtggattatcaaaacggcgcgatcacttcattacagcttcagcacgggcggtttgagagctgggccgaacggctgaacgtcgagccaggtaaactcaacgaagcctttattaatgcgatggcggaaatctgcacgccgctgccgggcgcggtttctctgcttaacgccattcgtggcaacgccaaaatcggcatcatcaccaacggctttagtgccttgcaacaggtgcgtctggaacgcacgggcctgcgtgattacttcgatttgctggtgatttccgaagaagttggcgttgccaaaccgaataagaaaattttcgattatgcgctggaacaggcgggcaatcctgaccgttcacgcgtgctgatggttggcgacactgccgagtccgatattctcggtggcatcaacgccgggcttgcgacctgctggctgaatgcacaccatcgcgagcaaccagaaggcatcgcgcccacctggaccgtttcttcgttgcacgaactggagcagctcctgtgtaaacactgattgcctcccccccgttgatgggtaaaatagccgcaatttttcgttttcaacaagcgcggcgcgatgccgcttactcaagaagaaagaattatgacgttgtctccttatttgcaagaggtggcgaagcgccgcacttttgccattatttctcacccggacgccggtaagactaccatcaccgagaaggtgctgctgttcggacaggccattcagaccgccggtacagtaaaaggccgtggttccaaccagcacgctaagtcggactggatggagatggaaaagcagcgtgggatctccattactacgtctgtgatgcagtttccgtatcacgattgcctggttaacctgctcgacaccccggggcacgaagacttctcggaagatacctatcgtaccctgacggcggtggactgctgcctgatggttatcgacgccgcaaaaggtgttgaagatcgtacccgtaagctgatggaagttacccgtctgcgcgacacgccgatcctcacctttatgaacaaacttgaccgtgatatccgcgacccgatggagctgctcgatgaagttgagaacgagctgaaaatcggctgtgcgccgatcacctggccgattggctgcggcaagctgtttaaaggcgtttaccacctttataaagacgaaacctatctctatcagagcggtaaaggccacaccattcaggaagtccgcattgttaaagggctgaataacccggatctcgatgctgcggttggtgaagatctggcacagcagctgcgtgacgaactggaactggtgaaaggcgcgtctaacgagttcgacaaagagctgttccttgcgggcgaaatcactccggtattcttcggtactgcgctgggtaacttcggcgtcgatcatatgttggatggcctggtggagtgggcacctgcgccgatgccgcgtcagactgatacccgtaccgtagaagcgagcgaagataaatttaccggcttcgtatttaaaattcaggccaacatggacccgaaacaccgcgaccgcgtggcgtttatgcgtgtggtgtccggtaaatatgaaaaaggcatgaaactgcgccaggtgcgcactgcgaaagatgtggtgatctccgacgcgctgacctttatggcgggtgaccgttcgcacgttgaagaagcgtatccgggcgatatcctcggcctgcacaaccacggcaccattcagatcggcgacacctttacccagggtgagatgatgaagttcaccggtattccgaacttcgcaccagaactgttccgtcgtatccgcctgaaagatccgctgaagcaaaaacagctgctcaaagggctggtacagctttccgaagagggcgcggtgcaggtgttccgtccaatctccaacaacgatctgatcgttggtgcagttggtgtgctgcagtttgatgtggtggtagcgcgcctgaagagcgaatacaacgttgaagcagtgtatgagtcagtcaacgttgccactgcccgctgggtagaatgtgcagacgcgaagaaattcgaagagttcaagcgtaagaacgaaagccaactggcgcttgatggcggcgataacctcgcttacatcgctaccagcatggtcaacctgcgcctggcacaggaacgttatccggacgttcagttccaccagacccgcgagcattaattcttgcctccagggcgcggtagccgctgcgccctgtcaatttcccttccttattagccgcttacggaatgttcttaaaacattcacttttgcttatgttttcgctgatatcccgagcggtttcaaaattgtgatctatatttaacaaagtgatgacatttctgacggcgttaaataccgttcaatgcgtagatatcagtatctaaagccgtcgattgtcattctaccgatattaataactgattcagaggctgtaatggtcgttattcatcactcatcgcttttgtgatggcgaccattgacttctgtagagggtgaagtctctccctattcagcaatgcaacctcgtgttgccaggctcaaattacgagcaaacatacaggaataaatcgatgactatgacaagactgaagatttcgaaaactctgctggctgtaatgttgacctctgccgtcgcgaccggctctgcctacgcggaaaacaacgcgcagactaccaatgaaagcgcagggcaaaaagtcgatagctctatgaataaagtcggtaatttcatggatgacagcgccatcaccgcgaaagtgaaggcggccctggtggatcatgacaacatcaagagcaccgatatctctgtaaaaaccgatcaaaaagtcgtgaccctgagcggtttcgttgaaagccaggcccaggccgaagaggcagtgaaagtggcgaaaggcgttgaaggggtgacctctgtcagcgacaaactgcacgttcgcgacgctaaagaaggctcggtgaagggctacgcgggtgacaccgccaccaccagtgaaatcaaagccaaactgctggcggacgatatcgtcccttcccgtcatgtgaaagttgaaaccaccgacggcgtggttcagctctccggtaccgtcgattctcaggcacaaagtgaccgtgctgaaagtatcgccaaagcggtagatggtgtgaaaagcgttaaaaatgatctgaaaactaagtaattcgtcgtaattcgtcctcccgaactttgtcgggaggcgcgatgtgcaccacactaaaaatatcgcattgagtgattttcacgctcatatcaagcggtgacattaactatggtaaaggagacgcttatgtttcgttggggcatcatatttctggttatcgcgttaatcgccgccgcacttgggtttggtggtctggccggtaccgctgcaggcgcagctaaaattgtctttgtcgtcgggattattctgttcctggtgagtttgttcatgggccgaaaacgaccctagatttcagaccattaagaaaattttatccaaagccagtccagcggactggcttttgcggttttagcgaataataaattgcgttactttgtcattctttcacaacaaaaacaggaaggcagaggtggggcagcgaatacctgtaacgcttggtaatattgcgccgttgtcgctaaggccgttccagcctggacgaatagctctggtgtgcgaaggcggcggacagcgtggaattttcacggctggcgtgctggatgagtttatgcgcgcgcagtttaatcctttcgatctttatctcggcacatctgccggggcgcagaacctctcggcgtttatctgcaatcagcccggttacgcgcgcaaagtcatcatgcgctataccacaaaacgcgaatttttcgatccattgcgctttgtccgtggaggaaatcttatcgatctcgactggctggtggaggccactgcaagccagatgccgttgcaaatggataccgccgcgcggttgtttgacagcggcaaatcgttttatatgtgcgcctgtcgtcaggatgactacgcgccgaattactttttaccaaccaaacaaaactggctggatgtgattcgcgcctccagtgcgatacctggcttttatcgtagcggagtgtcgctggaaggcattaactacctggatggcgggatcagtgatgcgattccggttaaagaggcggcaaggcagggcgctaaaacgttggtcgtcattcgcactgtgccgtcacaaatgtactacacgccgcagtggttcaaacgcatggaacgctggctgggtgacagtagcctgcagccgctggtcaatctggtgcagcatcatgaaaccagctatcgtgacattcagcaatttattgagaaaccaccgggcaagctgcggatattcgaaatttatccgccgaagccattacatagtatcgcgcttggcagtcggattccggcgctgcgtgaagactataaacttgggcgtttatgcggtcgttatttcctcgccacggttggcaagctattaactgaaaaagcgccgcttacccgccatctggtgccagtggtgacgccggaatcgattgtcattccgcctgcgccagtcgccaacgatacgctggttgccgaagtgagcgacgctccgcaggcgaacgacccgacatttaacaatgaggatctggcttgatttgccgttttatcgacacccactgccattttgatttcccgccgtttagtggcgatgaagaggccagcctgcaacgcgcggcacaagcgggcgtaggcaagatcattgttccggcaacagaggcggaaaattttgcccgtgtgttggcattagcggaaaattatcaaccgctgtatgccgcattgggcttgcatcctggtatgttggaaaaacatagcgatgtgtctcttgagcagctacagcaggcgctggaaaggcgtccggcgaaggtggtggcggtgggggagatcggtctggatctctttggcgacgatccgcaatttgagaggcagcagtggttactcgacgaacaactgaaactggcgaaacgctacgatctgccggtgatcctgcattcacggcgcacgcacgacaaactggcgatgcatcttaaacgccacgatttaccgcgcactggcgtggttcacggtttttccggcagcctgcaacaggccgaacggtttgtacagctgggctacaaaattggcgtaggcggtactatcacctatccacgcgccagtaaaacccgcgatgtcatcgcaaaattaccgctggcatcgttattgctggaaaccgacgcgccggatatgccgctcaacggttttcaggggcagcctaaccgcccggagcaggctgcccgtgtgttcgccgtgctttgcgagttgcgccgggaaccggcggatgagattgcgcaagcgttgcttaataacacgtatacgttgtttaacgtgccgtaggccggataaggcgttcacgccgcatccggcagttggcgcacaatgcctgatgcgacgcttaacgcgtcttatcatgcctacaggtttgtgccgaaccgtaggccggataaggcgttcacgccgcatccggcagttggcgcacaatgcctgatgcgacgcttgtcgcgtcttatcatgcctacaagtctgtgccgaaccgtaggccggataaggcgttcacgccgcatccggcagtcggcgcataatgcctgatgcgacgcttgtcgcgtcttatcatgcctacaggtttgtgccgaaccgtaggccggataaggcgttcgcgccgcatccggcagttggcgcacaatgcctgatgcgacgcttgacgcgtcttatcaggcctacaagtctgtgccgaaccgtaggccgtatccggcatgtcacaaatagagcgccggaaatatcaaccggctcaccccgcgcacctttaacgcatcagccaacggctcaacgtcttccggcgtggcgctcgcccagctttgcgcctcgccatacacgccgtgggcatgaaacgcgttcaggcgtaccggaacatcgccgagtcccttgataaacgccgccagttcttcgatgtgttgcaaataatccacctggccagggatcaccagcaaacgcagttccgccagcttgccgcgctctgccagcaaatagatgctgcgcttaatctgctgattatcgcgtccggtgagttgttgatgacattcgctcccccacgctttgagatcgagcattgcgccgtcgcacaccgggagcaatttttcccagccggtttcgctcaacatgccgttactgtccaccagacaggtgagatggcgcagttgcggatcgtttttgatagcagtaaacagcgccaccacaaacggcagctgggtcgtggcttcaccgccactcaccgttatcccttcgataaacagcactgctttgcggacatggctaagcacttcgtccacgctcatggattgcgccatgggcgtggcatgttgcggacacctcttcaggcaggtatcacactgctcgcaaaccacagcgttccacaccactttgccgtcaacaatctgcaacgcctgatgcggacactgtggcacgcactccccacagtcattgcaacgtcccatcgtccacggattgtgacagtttttgcagcgcagattgcagccctgcaaaaacagagccagacgactgcctggcccgtcaacgcaggagaaggggataatcttactgactaaagcgcatctgctgttcatggcttatcacgcgcggctggcgttccagaatacgagtgttgcgtgcggcttcttcgcccagccaggtggtgttggtgcgtgaaccttcggcgcgatatttttctaaatccgacaaacgcaccatataaccggtaacgcgaaccagatcgttaccgctgacattggcggtaaattcacgcattccggctttaaaggcaccgaggcaaagctgtaccagtgcctgcgggttacgtttgatggtttcgtcgagcgtcagaatgtcgctgatgccggaataataataagcatgatgcggggcgacagtttgcagatgggtgatcggatctggctcatcgccatacggcaaacgcgcgcccggcgtggtgccgatatcggaactgatccccgactgtgcgtgtaacatggcgcgtttttgccagccatatttcacgggggtattggcgacaaactccgccagttgcgcgctgatgcgataacctacttcatttgcggcggcttctttaccgtagcgcgcggcaatcccttctttttcacacagcaagttaaccgcttccgccagcccatacatgccaaacattggcacaaaacgttcagggttaatcagcccttctttcaccaggaagctattctcaaagaagtgtgattgttgatagaggaattcacaccgcgcatcgatgatggcgatctgctgctggcagtagtgcggtagagtgcgcgtaaagaagtcatccagcgattcgctgcgctcggcaatggctttcaggttaaggcgtaccagcgtgctgccaccacccgccagcggcagtgagttgtaacagctcacaatcccgtagcccccttttgtgaaaattttatcatgcaccggaccgttggcgatgtgcggtttgctacattcacagatgttcttcgccacttccagcagcaggtcatcaggggtgatttcaggatcgtagataaaggtcaggttcggtgaaacctgcttcaactctgcatctgcacgtaagatcgcgcgggtaatgggcgaatcagacgggccgatattggcgtgcataaaggcgtctggcagggttctgtcgaggtaacgccagaaacgttttattcgaacatcgatctcgtcttgtgttagaattctaacatacggttgcaacaacgcatccagttgccccaggtagaccggcatcgatgtgaccgacggtacgtggtggtaaagaatggtcagcagagagagtgcgtcatcaagatctttcgcgccttccagctccagccattcggaaccgttcgccagaaaacgggcgtaatcgggtaagacatagcgcggtttgtacggcgcatgaccttcaaacatatcgcagattacaccttcatccagcgcgcggcgggcttcggcaggaagctgtgggtaaggcagattgttttctgcttccagtgccagaaaatggcgcttctgctccgggctaagcactgggctggtgacaatttgctggcaacgttgttgcagtgcattttcatgagaagtgggcatcttcttttccttttatgccgaaggtgatgcgccattgtaagaagtttcgtgatgttcactttgatcctgatgcgtttgccaccactgacgcattcatttgaaagtgaattatttgaaccagatcgcattacagtgatgcaaacttgtaagtagatttccttaattgtgatgtgtatcgaagtgtgttgcggagtagatgttagaatactaacaaactcgcaaggtgaattttattggcgacaagccaggagaatgaaatgactgatctgaaagcaagcagcctgcgtgcactgaaattgatggacctgaccaccctgaatgacgacgacaccgacgagaaagtgatcgccctgtgtcatcaggccaaaactccggtcggcaataccgccgctatctgtatctatcctcgctttatcccgattgctcgcaaaactctgaaagagcagggcaccccggaaatccgtatcgctacggtaaccaacttcccacacggtaacgacgacatcgacatcgcgctggcagaaacccgtgcggcaatcgcctacggtgctgatgaagttgacgttgtgttcccgtaccgcgcgctgatggcgggtaacgagcaggttggttttgacctggtgaaagcctgtaaagaggcttgcgcggcagcgaatgtactgctgaaagtgatcatcgaaaccggcgaactgaaagacgaagcgctgatccgtaaagcgtctgaaatctccatcaaagcgggtgcggacttcatcaaaacctctaccggtaaagtggctgtgaacgcgacgccggaaagcgcgcgcatcatgatggaagtgatccgtgatatgggcgtagaaaaaaccgttggtttcaaaccggcgggcggcgtgcgtactgcggaagatgcgcagaaatatctcgccattgcagatgaactgttcggtgctgactgggcagatgcgcgtcactaccgctttggcgcttccagcctgctggcaagcctgctgaaagcgctgggtcacggcgacggtaagagcgccagcagctactaagtaagatgctttacgcctgatgcgctgcgcttatcaggcctacgagacgtatctacccgtaggccggataaggcgtagacgcatccggcaaaagccgcctcatactcttttcctcgggaggttaccttgtttctcgcacaagaaattattcgtaaaaaacgtgatggtcatgcgctgagcgatgaagaaattcgtttctttatcaacggtattcgcgacaacactatctccgaagggcagattgccgccctcgcgatgaccattttcttccacgatatgacaatgcctgagcgtgtctcgctgaccatggcgatgcgagattcaggaaccgttctcgactggaaaagcctgcatctgaatggcccgattgttgataaacactccaccggtggcgtcggcgatgtgacttcgctgatgttggggccgatggtcgcagcctgcggcggctatattccgatgatctctggtcgcggcctcggtcatactggcggtacgctcgacaaactggaatccatccctggcttcgacattttcccggatgacaaccgtttccgcgaaattattaaagacgtcggcgtggcgattatcggtcagaccagttcactggctccggctgataaacgtttctacgcgacccgtgatattaccgcaaccgtggactccatcccgctgatcaccgcctctattctggcgaagaaacttgcggaaggtctggacgcgctggtgatggacgtgaaagtgggtagcggcgcgtttatgccgacctacgaactctctgaagcccttgccgaagcgattgttggcgtggctaacggcgctggcgtgcgcaccaccgcgctgctcaccgacatgaatcaggtactggcctccagtgcaggtaacgcggttgaagttcgtgaagcggtgcagttcctgacgggtgaatatcgtaacccgcgtctgtttgatgtcacgatggcgctgtgcgtggagatgctgatctccggcaaactggcgaaagatgacgccgaagcgcgcgcgaaattgcaggcggtgctggacaacggtaaagcggcagaagtctttggtcgtatggtagcggcacaaaaaggcccgaccgacttcgttgagaactacgcgaagtatctgccgacagcgatgctgacgaaagcagtctatgctgataccgaaggttttgtcagtgaaatggatacccgcgcgctggggatggcagtggttgcaatgggcggcggacgccgtcaggcatctgacaccatcgattacagcgtcggctttactgatatggcgcgtctgggcgaccaggtagacggtcagcgtccgctggcggttatccacgcgaaagacgaaaacaactggcaggaagcggcgaaagcggtgaaagcggcaattaaacttgccgataaagcaccggaaagcacaccaactgtctatcgccgtatcagcgaataacggtatactgatctgatcatttaaatttgaagcactgagtacggagaacatatgaaacgtgcatttattatggtgctggactcattcggcatcggcgctacagaagatgcagaacgctttggtgacgtcggggctgacaccctgggtcatatcgcagaagcttgtgccaaaggcgaagctgataacggtcgtaaaggcccgctcaatctgccaaatctgacccgtctggggctggcgaaagcacacgaaggttctaccggtttcattccggcgggaatggacggcaacgctgaagttatcggcgcgtacgcatgggcgcacgaaatgtcatccggtaaagataccccgtctggtcactgggaaattgccggtgtcccggttctgtttgagtggggatatttctccgatcacgaaaacagcttcccgcaagagctgctggataaactggtcgaacgcgctaatctgccgggttacctcggtaactgccactcttccggtacggtcattctggatcaactgggcgaagagcacatgaaaaccggcaagccgattttctatacctccgctgactccgtgttccagattgcctgccatgaagaaactttcggtctggataaactctacgaactgtgcgaaatcgcccgtgaagagctgaccaacggcggctacaatatcggtcgtgttatcgctcgtccgtttatcggcgacaaagccggtaacttccagcgtaccggtaaccgtcacgacctggctgttgagccgccagcaccgaccgtgctgcagaaactggttgatgaaaaacacggccaggtggtttctgtcggtaaaattgcggacatctacgccaactgcggtatcaccaaaaaagtgaaagcgactggcctggacgcgctgtttgacgccaccatcaaagagatgaaagaagcgggtgataacaccatcgtcttcaccaacttcgttgacttcgactcttcctggggccaccgtcgcgacgtcgccggttatgccgcgggtctggaactgttcgaccgccgtctgccggagctgatgtctctgctgcgcgatgacgacatcctgatcctcaccgctgaccacggttgcgatccgacctggaccggtactgaccacacgcgtgaacacattccggtactggtatatggcccgaaagtaaaaccgggctcactgggtcatcgtgaaaccttcgcggatatcggccagactctggcaaaatattttggtacttctgatatggaatatggcaaagccatgttctgatggatttgggcggagcgttgactccgcctttgttatgtcacaaaaaggataaaacaatggctaccccacacattaatgcagaaatgggcgatttcgctgacgtagttttgatgccaggcgacccgctgcgtgcgaagtatattgctgaaactttccttgaagatgcccgtgaagtgaacaacgttcgcggtatgctgggcttcaccggtacttacaaaggccgcaaaatttccgtaatgggtcacggtatgggtatcccgtcctgctccatctacaccaaagaactgatcaccgatttcggcgtgaagaaaattatccgcgtgggttcctgtggcgcagttctgccgcacgtaaaactgcgcgacgtcgttatcggtatgggtgcctgcaccgattccaaagttaaccgcatccgttttaaagaccatgactttgccgctatcgctgacttcgacatggtgcgtaacgcagtagatgcagctaaagcactgggtattgatgctcgcgtgggtaacctgttctccgctgacctgttctactctccggacggcgaaatgttcgacgtgatggaaaaatacggcattctcggcgtggaaatggaagcggctggtatctacggcgtcgctgcagaatttggcgcgaaagccctgaccatctgcaccgtatctgaccacatccgcactcacgagcagaccactgccgctgagcgtcagactaccttcaacgacatgatcaaaatcgcactggaatccgttctgctgggcgataaagagtaattgtgtttcgctgcaaggcgattgccttgtgaagccggagcgggagactgctccggctttttagtatctattcatttttctctccagcttgaatattttcgctatacttttcagtgaaatgtgttaataaatctattcaagtatctattcacgaatctattcattaatgagcgagctgactgatcttttactgcaagggccgcgttctgccccggaattgcgccagcgtctggcaatcagtcaggcgacgttctcacgccttgttgccagagaagatcgggtgattcgctttggtaaagcacgggcaacgcgatatgcactgctgcgtccttatcgcggaattgagcgtattcccgtctggcgggtggacgataccggaaaggcgcataaattcgccgacatccggttgtgctggccgcagggaagttgtctggtaacaggcgcagatggcgacgaacagtggtttgatggtttgccctggtatttgaccgatctccgaccgcagggctttttagggcgcgcgtggggcaggaagttagccgcgcaactgaatctgactgatgatatacgtctctggcaggaagaagatgtgctctacgccctgaccgtatttaacggtgaatatactggcggttggttggtcggggaggggaattatcagcgatggattactgcacaacaccctgcggaaattcctctggatcaaaaactcacccattacgaacagctggcaagtgatgcactggcaggagaaattgtgggttcttctgcgggcggcgagcagccaaaatttacctactatgcacaaacgccgtcaggcaataaacatgtgttggtgaaattcaccgtaccacagcaaaccgcggtcagccaacgttggggtgacctgctaattgctgaatctattgccgcgcaaatcctgcgtgacggtgggatccacgccatcgagtcaacggtgcttgtaacaagtaacaggcaggtattcctcgaagcggaacgctttgactgcaaaggtaacgatggtcgcttgcctattgtgtcgctggaggcggtgcagagtgagtttatctcttctccgggatcgtggccgcaggcaatgcgccgtttgtgtgagcaacaacttgtcactcaccagagcgtggcgcaaacagaagtgatctgggcatttgggcgacttatcgccaacagcgatatgcacgcaggtaatttatcgttttatttatctgaaccgccatttgcgctgacgcccgtctacgacatgctgccgatggtctatgcaccaaacagcgctggaatgctgcgtgatgctgccattgaggtgaagtttgatcttaacgtcagtaaaagcgcttggttaacggcgatcccgctggcgcagcagttctggcaaacggtcgccagagatccgcgtatcagcgaggcgtttcgccacattgcgcaagaaatgccggaaaaaatccggcaaatcgaagagaaagttgcccgcatgggcgggtaactaccttacagcccccgccatccatgccgataactcccgtagctctttttcctgttccgggaagtcaaccaacagcgcttcgcactcctgttgcagcatatctgcgcggtacaggcagccttgcagtcgtccggcgagggcttccagcggcgcggggttgaggctgtcggtaaacacctgggcgcgggtgatatggcctttttcaacgtcgaaatgcagttccacgccgccccaggtaaagcgttcatccagcagatgcgagaatgccggagcctgaccgaagttccattcccagctactctggcgggcaaaggtttcggcgaagtttggcaagtctggcgttttgttcggggagatgatttccgcttccacgcgctcgccataatgggcgaaaaaggcctcggttatggcctcgcaaacctgctcatgggtgatccccggcaacagctcggtgaggttggtcacgcgggaacgtaccgacgtaatgcctttcgccgccagtttctttttatccggattgagatagtttgccaggcggctgaggtcggcattgagtagcaaggtgccgtggtggaagccgcgatctttggtttcgcgataggccgagcctgagactttgcggtcgccttcgacggttttcaccaccagatcgttacgtccggacgcttcggcgctgacgccgagcgcgttcagcgcattgagcacaatcgacgtggagatagttttatcgtactccggcttgccagccataaaggtaaagcaggtattgccgagatcgtggaacaccgcgccgccaccgctactgcgccgcgccaggcggacgttatcttcttccatccgccgggtattacactctttccacgggttctgcgcgcgaccaattactaccgtgtcggcattgcgccagagaaacagaacgcgctgcgtggcgggcatttggcgaaaaatacactcttccaccgccaggttaaaccacgggtcgtaagagtcagagatgagcaggcgtaatgtggacataacgatttcctttcttgtagtaatgggtcactcttttttctcgctttcttcctcttccggcaccggtttgctggcggttaacaggaagggcgattgctgccagcgggtgcgtttaccctgtagcagcgtgcgggtcagcactacaccgattgccagtgagagcagcaacatcaggcgtaaaatgttagtggtgttatccacctgttgggcttcggtggcgagcgtatgggtgtcgagtgtcaggcgcagatagccgagcggtccgtttttacccgcaattggctcgacaatctgctggttaaaatagccgcctgcttttttaccgtcgagcgccagccggtcgcgcacttcgacgctttcgccagaacgtgcgataagatcgccttgttcgtcatacacacccgcgtcgaggatacggctttcatccgttaactgatcgaggatcgcctgaatgcgtttttcatccggtgagtcggtacgcatcagcggtgcaacgttcagcgtcacctgacgcgccagggtgcgggccagttcttccagctgtggattacgctgtcgctggtggttttgactaaaccatgacgctccctgcatcagcgccactaacaaggcaagacagaacaggacaatcactgcccgatgcagccggaatttcagttttgtgcgagccatcttccaccctttgaaaatttgagacttaatgttgccagaagcaatggatacaaggtagcctcatgcgttattttccctgcttcgaacgattttacaggagccttaatgcctaacattacctggtgcgacctgcctgaagatgtctctttatggccgggtctgcctctttcattaagtggtgatgaagtgatgccactggattaccacgcaggtcgtagcggctggctgctgtatggtcgtgggctggataaacaacgtctgacccaataccagagcaaactgggtgcggcgatggtgattgttgccgcctggtgcgtggaagattatcaggtgattcgtctggcaggttcactcaccgcacgggctacacgcctggcccacgaagcgcagctggatgtcgccccgctggggaaaatcccgcacctgcgcacgccgggtttgctggtgatggatatggactccaccgccatccagattgaatgtattgatgaaattgccaaactggccggaacgggcgagatggtggcggaagtaaccgaacgggcgatgcgcggcgaactcgattttaccgccagcctgcgcagccgtgtggcgacgctgaaaggcgctgacgccaatattctgcaacaggtgcgtgaaaatctgccgctgatgccaggcttaacgcaactggtgctcaagctggaaacgctgggctggaaagtggcgattgcctccggcggctttactttctttgctgaatacctgcgcgacaagctgcgcctgaccgccgtggtagccaatgaactggagatcatggacggtaaatttaccggcaatgtgatcggcgacatcgtagacgcgcagtacaaagcgaaaactctgactcgcctcgcgcaggagtatgaaatcccgctggcgcagaccgtggcgattggcgatggagccaatgacctgccgatgatcaaagcggcagggctggggattgcctaccatgccaagccaaaagtgaatgaaaaggcggaagtcaccatccgtcacgctgacctgatgggggtattctgcatcctctcaggcagcctgaatcagaagtaattgctcgcccgccatcctgcgggcggcacagcattaacgaggtacaccgtggcaaaagctccaaaacgcgcctttgtttgtaatgaatgcggggccgattatccgcgctggcaggggcagtgcagtgcctgtcatgcctggaacaccatcaccgaggtgcgtcttgctgcgtcgccaatggtggcgcgtaacgagcgtctcagcggctatgccggtagcgccggggtggcaaaagtccagaaactctccgatatcagccttgaagagctgccgcgtttttccaccggatttaaagagttcgaccgcgtactaggcggcggcgtggtgccaggaagtgccattctgattggcggtaaccctggtgcggggaaatccacgctgctactgcaaacgctgtgcaaactggcccagcagatgaaaacgctgtatgtcaccggcgaagagtcgctgcaacaggtggcaatgcgcgctcatcgccttggcctgccgactgacaatctcaatatgttgtcggaaaccagcatcgaacagatctgcctgattgccgaagaagagcaaccgaagctgatggtaattgactcgatccaggtgatgcatatggcggatgtacagtcatcgcctggtagcgtggcgcaggtgcgtgaaacggcggcttatttgacacgcttcgccaaaacgcgcggtgtggcgattgtcatggtggggcacgtaaccaaagatggttcgctggctggcccgaaagtgctggaacactgtatcgactgttcggtgcttttggatggcgatgccgactcccgttttcgcaccttgcgcagccataaaaaccgcttcggcgcggtgaatgagctgggcgtcttcgcgatgaccgaacaggggctgcgtgaagtcagcaacccttcggcaattttcttaagtcgcggcgatgaagtgacctccggtagctcagtgatggtggtatgggaaggaacgcgtccactgctggtggagattcaggcgctggtcgatcactcgatgatggcgaacccacgccgcgtggcagtggggctggaacaaaaccgtctggcaatcctgctggctgtgttgcaccgtcacggtggtctgcaaatggccgatcaggatgtgtttgtgaacgtggtcggcggcgtgaaggtaaccgaaaccagtgccgacttagcgttactgctggcgatggtttccagcctgcgcgacagaccgctgccgcaggatctggtggtgtttggtgaagtcgggctggcaggggagatccgcccggtgcccagcggtcaggaacgaatctctgaagcggcgaaacacggttttcgccgggcgattgttccggcggctaacgtgccgaaaaaagcgccggaagggatgcagatttttggcgttaaaaaactctccgacgcgcttagcgtgttcgacgacttataatgagatatacggagggagatatgtcgtcatttgattacctgaaaactgccatcaagcaacagggctgcacgctacagcaggtagctgatgccagcggtatgaccaaagggtatttaagccagttactgaatgccaaaatcaaaagccccagcgcgcaaaagctggaggcgttgcaccgttttttggggcttgagtttccccggcagaagaaaacgatcggtgtcgtattcggtaagttctacccactgcataccggacatatctaccttatccagcgcgcctgtagccaggttgacgagctgcatatcattatgggttttgacgatacccgtgaccgcgcgttgttcgaagacagtgccatgtcgcagcagccgaccgtgccggatcgtctgcgttggttattgcaaacttttaaatatcagaaaaatattcgcattcatgctttcaacgaagagggcatggagccgtatccgcacggctgggatgtgtggagcaacggcatcaaaaagtttatggctgaaaaagggatccagccggatctgatctacacctcggaagaagccgatgcgccacagtatatggaacatctggggatcgagacggtgctggtcgatccgaaacgtacctttatgagtatcagcggtgcgcagatccgcgaaaacccgttccgctactgggaatatattcctaccgaagtgaagccgttttttgtgcgtaccgtggcgatccttggcggcgagtcgagcggtaaatccaccctggtaaacaaacttgccaatatcttcaacaccaccagtgcgtgggaatatggccgcgattatgtcttttcacacctcggcggtgatgagatcgcattgcagtattctgactacgataaaatcgcgctgggccacgctcaatacattgattttgcggtgaaatatgccaataaagtggcatttatcgataccgattttgtcaccactcaggcgttctgcaaaaagtacgaagggcgggaacatccgttcgtgcaggcgctgattgatgaataccgtttcgatctggtgatcctgctggagaacaacacgccgtgggtggcggatggtttacgcagcctcggcagttcggtggatcgcaaagagttccagaacttgctggtggagatgctcgaagagaacaatatcgaatttgtgcgggttgaagaggaagattacgacagtcgtttcctgcgctgcgtggaactggtgcgggagatgatgggggagcagagataaccgtgatgaaactgctcaaaggcgaggtataaaatgagtttttttgatgagttgaaaacctctctggaagaggctgtcgagattaaacaaggtttgaaaaaacctgcacgggtgacccgccacgaaattgaggatgctaaggctgttgtagaccggaaacggtgttcacgccgcatccggcattcggtgctcaatgcctgatgcgacgcttaccgcgtcttatcaggcctacagttttacaacgtattgaaattgctggttttgtaggccggataaggcgttcgcgccgcatccggcattttacgcattacttcgcaatacgcttgtacttgatacgcttcggctccagcgcgtctgcgcccagcgtgcgtttcttgtactcttcgtactcggtaaagttaccttcgaagaactcaactttaccttcatcctggtaatccagaatgtgcgtggcgatacggtcgaggaaccaacggtcgtgcgagataaccatcgcacagcccgggaactccagcagggcgttttccagcgcgcgcagggtttcgatatccaggtcgttggttggttcgtcgagcagcagcatgttgccgccaacctgcagcagcttcgccagatgcagacgaccgcgctcaccaccggagagttcaccaacgcgtttaccctgatcaacccctttaaagttaaagcggccaacgtaggcgcggcttggcatctcggtgttgccgatcttcatgatatccagcccgccggaaacttcttcccaaacggttttgctgttatccattgagtcacggaactgatcaaccgacgccagtttcaccgtttcacccaaagtgatggtgccgctgtccggctgttcctgaccagagatcatacggaacagggtcgatttacccgcaccgttcggaccgatgatcccgacgatcgctcctttcgggatcgagaagctcaggtcatcaatcagcagacgatcgccataggatttacgcaggttgctgacttccagcactttatcgcccagacgcggtccaggtggaataaacagttcgttggtttcgttacgtttctgatattcggtgctgttcagttcttcaaagcgcgccagacgtgctttacctttcgactgacggcctttagtaccttgacgtacccattccagctctttctcaatcgacttacgacgcgccgcttcttgtgaagcttcctgcgccaggcgctgatctttctgctccagccaggaggagtagttaccttcccacggaataccttcaccgcggtcaagttcgaggatccagcctgcaacgttatcgaggaagtaacggtcgtgggtaatcgccacaacggtgccttcgaagtcgtgcaggaagcgttccagccaggccacggattcggcatccaggtggttggtcggttcgtcgagcagcagcatgtctggtttttccagcagcaggcggcacaacgctacgcgacgacgttcaccaccggagaggttagcgattttcgcgtcccagtccggcagacgtagcgcatccgccgcacgctccagctgtacgttcagattatgaccgtcgtgagcctgaatgatctcttccagacggccttgttcagcggccagcttgtcaaaatcggcatccggatcggcgtacagcgcatacacttcatccaggcgtttcagggcgttaaccacttctgaaaccgcttcttcaatggactcacgcacggtgtgttccgggttcagctgcggttcctgcggcagataaccaatcttgatgtctggctgcggacgcgcttcaccttcgatgtctttatcaatgcccgccataatgcgcagcagggtggacttacccgcgccattcagacccaggacaccaatttttgccccagggaagaaactcagagagatgtttttcaaaatatgacgtttcggcggaacaactttgccgacacgatgcatggtataaacgaattgagccacgttggacttcgcctctatgtttatcgtgataatgagttttcaaaggcgaagtgtagcctttttccccgcctaatcccagccggtcgatcaccctcgcagtaaaagtaaaaaagtgtccgtaacgtggcgtaaacggcaatgactggttagcataaatctattacgcggcatgacgctgcattgatgtatttacacttagaggatgcgcttgtggaaaaagccaaacaagttacctggcggctgttggctgccggtgtctgtctgctgacggtcagcagcgtggcgcgagccgactcactggatgagcagcgtagtcgttacgcgcaaatcaagcaggcctgggataatcgacaaatggatgtggtcgaacaaatgatgcctggactgaaggattatccgctttatccctacctggaataccgccagatcaccgatgatctgatgaatcaaccggcggtgacggtcactaactttgttcgcgctaaccccacgcttcctcccgctcgcacgctgcaatctcgtttcgtcaatgaactggcgcggcgtgaagactggcgtggcttgttagcctttagcccggaaaagcccggaactaccgaagcgcaatgtaattactactatgcgaaatggaacaccgggcagagtgaagaagcctggcaaggggcgaaagagctgtggctaaccggcaagagccagcctaacgcctgtgacaagttatttagcgtctggcgtgcgtcaggtaaacaagatccgctggcgtatttagagcgtatccgtctggcgatgaaagcgggtaacacaggcctggtaacagtgctggcagggcagatgcctgccgattaccagactatcgcctcggcaatcatttcactggcgaacaaccctaatacggtactgaccttcgcgcgtacaactggcgcgaccgattttacccgtcaaatggcggcggtggcgtttgccagtgtggcgcggcaggatgctgagaatgcacggctgatgatcccatcgcttgcccaggcgcagcagcttaatgaagatcagattcaggagctgcgcgatatcgtcgcctggcgtttgatgggcaacgatgtcaccgacgagcaggcgaaatggcgcgatgacgccattatgcgctcgcaatctacttcgcttattgaacgccgtgtacgaatggcgcttggcaccggcgatcgtcgcggcctgaatacctggctggcgcgtctgcctatggaagcgaaagagaaagatgaatggcgttactggcaggcggatttattgctggaacgcggacgtgaagctgaagcaaaagagattttgcatcaactcatgcaacagcgtggtttctacccgatggttgcagcacaacgcatcggcgaagagtatgagctgaagattgataaagcgccgcagaatgttgacagcgccctgactcaggggccggagatggcgcgcgtgcgcgagttgatgtactggaatctcgataataccgcgcgtagcgagtgggccaatctggtgaagagcaagtcaaaaacagagcaggctcaactggcgcggtatgctttcaacaaccaatggtgggatcttagcgttcaggcaacgatcgccgggaagctgtgggatcatctggaagagcgattcccgctggcttacaacgatcttttcaaacgctacaccagcggtaaggagatcccgcaaagctatgcgatggcgattgctcgtcaggagagcgcctggaatccgaaagtgaaatcaccggtaggggccagcggcttgatgcagattatgcctggtacagcgacccatacggtgaagatgttctctattcccggttatagcagtcctgggcaattgctggatccggaaacgaatatcaacattggcaccagttacctgcaatatgtttatcagcagtttggcaataatcgtattttctcctcagcagcttataacgccggaccagggcgggtgcgaacctggcttggcaacagcgccgggcgtatcgacgcagtggcatttgtcgagagtattccattctccgagacgcgcggttatgtgaagaacgtgctggcttatgacgcttactaccgctatttcatgggggataaaccgacgttgatgagcgccacggaatggggacgtcgttactgatccgcacgtttatgatatgctatcgtactctttagcgagtacaaccgggggaggcattttgcttcccccgctaacaatggcgacatattatggcccaacaatcaccctattcagcagcgatggcagaacagcgtcaccaggagtggttacgttttgtcgacctgcttaagaatgcctaccaaaacgatctccatttaccgttgttaaacctgatgctgacgccagatgagcgcgaagcgttggggactcgcgtgcgtattgtcgaagagctgttgcgcggcgaaatgagccagcgtgagttaaaaaatgaactcggcgcaggcatcgcgacgattacgcgtggatctaacagcctgaaagccgcgcccgtcgagctgcgccagtggctggaagaggtgttgctgaaaagcgattgattttgtaggcctgataagacgtggcgcatcaggcatcgtgcaccgaatgccggatgcggcgtgaacgccttatccgtcctacaaatacccgtaatttcaatatgtttggtaggcatgataagacgcggcagcgtcgcatcaggcgcttaatacacggcattatgaaacggactcagcgccaggatcaccgcctggtgatagacgctggcgcgagtgagtttcccggcggtaaacacgccgatcgccccttccttacgaccaatctcatcaataccggtataacgcgacatcacgggaccaagcgcctcaccttcacgcactttttccagaatcaccgcaggcaacggcaaagtagccgaacgcgcctcgccgcgctggctggcgttttcaatcaccacccaactgaaagtgctgtcaccatcgatgccagcttcaatcgccacccaaaaatcagcctctggaagtaaacggcgggcattggctacccgatttcgtgcgccagcgcgcgtttcctcactgccaaagggctgttccggtacaccgctctcgacggcaacggatgcaatatggcaggatccttcgccgaagatctcgtgaaatgcctgcagaatggcctgaattttagcgggattggtggtcgcacagacaacttggtgcataatcagcattactcagaaaattaacgttacagcagtatacggaaaaaaagcatgttacaggtatacctagtccgccacggtgaaacgcagtggaacgccgagcgacgtattcagggccagtctgacagcccgctgaccgccaaaggtgagcaacaggcgatgcaggtggcaacccgtgccaaagagcttggcattacgcatatcatcagtagcgatttaggacgcacccggcgtacggcggaaatcatcgcccaggcctgcggctgtgacatcatctttgattctcgcctgcgtgaattaaacatgggtgtgctggaaaaaagacatatcgattctctgaccgaagaagaagagaactggcgtcggcagctggtcaatggcaccgttgacgggcgtattcctgaaggcgagtcaatgcaggagctcagcgatcgcgtcaatgcggcactggaatcttgccgggacttaccgcagggaagccgaccgctgctggtgagtcatggtattgcactgggatgcctggtgagtacgattctcggattaccagcatgggcagagcgccgcttacgtctgcgtaactgttctatttcgcgcgtggattatcaggaaagcctgtggctggcgtctggctgggtcgttgaaaccgcaggggacatctcgcatctggacgcccctgcattagatgagctgcagcgttaacgacggatcggaatcagcagttcacagcgtagattaattgggcgatctcccgctttggcatcttctgccgggtagtatcgctcaatatcctgacctttacggcgcgtcaggttgagcattggcatgcacgttccgtataccgtcaggataaactcctgcacgccggttcccagaccttcataggtaaacatcacatattcgccgccctgcagcatcaccggatgccccgtcagtacatagccatctgcctgatcctgggctaacgcggtggtatagaatacctcttgctcgtcgtctttatcctgactcggacgcgtttcattcaggccgtagagcaccggcggaatggtcggcgcgttgccgagaaaatcgtgccagaactgataacgcatttcatggcggaaatcagagatttgctccagcgaacaggagtagctctgggtaacaccaatcagcggcgtatcttccagggtgacaaatttgtgctctggcatagtgaattcacccaggcgtagcggcgggcgaataccaaaggcgctccattcaggagaacggcggtaaagtgcaggagtctgggcaaactgcttcttgaatgcgcgggtaaatgtctgttgagagtcgaagcggtattgcagcgcgatgtccagaatcggacgcgcagtcaggcgtagtgcgaccgccgatttcgacaaacgacgagcacgaatatacgcgccaatagcatggccagtgacatctttaaacattctctgtaagtgccacttggaataacctgctttcgccgctacattgtcgagcgacaggggctgatccagatgaccttccagccagattaaaaggtcgcgaataatgccggcctgatccataaaatatcctcatcctttcaacaacgagcacctgacatcaggtaattggataatagcattttttgctgttttagcattcagtgtttttttcttagtagagtatgttttagggcttgacggaaataaaagtattgagattttgttcttaatcaatatgttatttaccgtgacgaactaattgctcgtgtaatagataaaaatggtaacaatatgaaatacaagcatttgatcctgtctttaagcctgataatgctggggccattggctcatgcagaagagattggttcggtcgacaccgtatttaaaatgatcggcccggatcacaaaattgttgtggaagcctttgatgatcccgatgtgaaaaatgtcacctgttatgtgagccgggcgaaaaccggtggtattaaagggggattgggtctggcggaagatacctccgatgcggccatttcttgtcagcaagtcgggccgattgaactgtcggatcgtattaaaaacggcaaagctcagggcgaggtagtattcaaaaaacgcacgtccctggtctttaagtcgttacaggtcgtgcgcttttatgatgccaaacgcaacgcgctcgcttatctggcttactccgacaaagttgtagaaggttcgccgaaaaacgcgattagcgcggttcctgtcatgccgtggcggcaataacagaggcgatttatgcaacgggaaacggtctggttagtggaagatgagcaagggatagccgacacgctggtctacatgttgcagcaggaaggttttgccgtcgaggtctttgagcgaggcttgccggtgctggataaagctcgcaagcaggtacccgacgtcatgattctcgatgttggtctgccggatattagcggctttgaattgtgccgccagttactggcgctccatccggcgttacctgtactgttcctgacggcccgaagtgaagaggtcgatcgcctgcttgggctggaaattggtgctgacgactacgtggctaaaccgttttcaccccgcgaagtgtgcgccagggtgcgcaccttactgcgtcgggtgaagaagttctcgacgccgtctcccgtcatccgtattggacattttgaattgaatgaacccgcggcgcagatcagctggtttgacacgccattagcgctgactcggtatgagtttttattgttgaagacgttactcaagtcaccgggccgcgtctggtcccgccagcaactgatggatagcgtatgggaagatgcgcaggacacctacgatcgcaccgtcgatacccacattaaaacgctgcgtgccaagctgcgcgccatcaaccccgatctttcaccgattaatactcatcgcggcatgggatatagcctgaggggcctgtaatgcgtatcggcatgcggttgttgctgggctattttttactggtggcggtggcagcctggttcgtactggccatttttgtcaaagaagttaaaccgggcgtgcgaagagcaacggaggggacgttgatcgacaccgcaacgttgctggcggagctggcgcgtcccgatttgctctctggggacccaacgcatgggcaactggcgcaggcgtttaatcagctacaacatcgcccgtttcgcgccaatatcggtggcattaacaaagtgcgcaatgaatatcatgtctatatgaccgatgcgcagggcaaagtattgttcgattcggcaaataaagccgttggacaggattattcgcgctggaatgacgtctggctaacgttgcgtggtcagtatggtgcgcgcagcacgttgcaaaatcctgccgatcccgaaagttctgtgatgtatgttgccgcaccgattatggacggctcgcggcttattggcgttttgagcgtaggcaaaccgaacgcggcgatggctccggtcattaagcgtagcgagcggcgaattttatgggccagcgccattttgttggggattgcactggtgattggcgcaggcatggtttggtggatcaaccgctctattgcccggctcactcgctatgctgattccgtcactgacaataagcccgttcctctccccgatctcggtagtagcgagttgcgtaaactcgcgcaggcgctggaaagtatgcgcgtgaagctggaagggaaaaactatattgagcagtatgtttacgcattaactcatgagctaaaaagcccactggcggcgattcgtggagcggcggaaattttacgcgaaggtccgccgccggaagtggtggctcgttttactgacaacattctgacgcaaaatgcgcgtatgcaggcattggtagaaacgttactacgccaggcaagactggagaatcgtcaggaagtcgttctgactgctgttgatgtggcggcattattccgccgcgtcagcgaagcgcgcaccgtgcagttggcagaaaaaaaaatcactctgcatgttacgcccaccgaggttaacgttgctgctgaaccggcgttactggagcaggcgctgggaaatttactggataacgccatcgattttacccccgagagcggttgcatcacgctaagcgccgaagtggatcaggaacacgtcacgcttaaggtgctggataccggtagtggtattcctgactacgcgctttcacgtatttttgaacgcttttactctttgcctcgtgcaaatgggcaaaaaagcagcggtctggggttggcgttcgtcagtgaggtcgcccgtttgtttaacggcgaagtcacgctgcgcaacgtgcaggaaggtggcgtgctggcctcgcttcgacttcaccgtcacttcacatagcttcaaattcttcccacatagtcttcgtatcctgctgccattgcaaaggagaagactatgttgaaatcccccctgttctggaaaatgactagcctgtttggtgcagtattgctgttgttgattccgataatgctgattcggcaggtgattgtcgaacgtgctgattaccgtagcgatgtggaagatgcgattcgccaaagtaccagcgggccgcaaaaactcgttgggccgctcatcgctattcctgtgaccgagctttatacggtgcaggaagaggataaaaccgtggagcggaaacgaagttttatccatttttggttacctgagtcattgatggttgatggcaatcagaacgtggaagaacgcaagatagggatttataccggtcaggtctggcacagtgatttaacgttaaaagccgatttcgatgtttcgcgtcttagcgaactcaacgcgccaaatatcaccttaggcaagccatttattgtgattagcgtcggggatgcgcgtggtattggtgtggtgaaagcgcctgaagttaacggaacggcgctgaccattgaacccggcaccgggttagagcaaggcgggcagggcgtgcatatccctttacctgaaggggactggcggaagcagaacctgaagctgaatatggccctgaatttaagcggtaccggcgatctttctgtggtgcctggcgggcgtaatagcgaaatgaccttaaccagcaactggccgcatcccagttttttaggtgattttctaccagccaaacgggaagttagcgagtcaggttttcaggcgcactggcaaagcagctggtttgctaataatctcggtgagcgttttgcttcaggcaatgataccggctgggaaaacttcccggcgtttagcgtcgcagtaacgacgccagccgatcaataccaattaactgaccgggcgactaagtacgccattctgctgattgcactgacttttatggcgttctttgtttttgaaacgctcaccgcgcaacgtttacacccaatgcaatatttgctggtggggctttcattggtgatgttttatttgctcttgctggcgctttctgaacataccggttttaccgtggcatggataatcgccagtctgattggggcgataatgaacggtatttatttgcaagcggtattgaaaggttggtgcaacagcatgttgtttaccctcgcgctgttgttgctggatggtgtgatgtggggactgctcaactctgccgatagcgcgctgttgttgggaaccagtgtgctggtggtggcgctggccggcatgatgtttgtgacccgtaatatcgactggtatgcgttttcactgccgaaaatgaaagccagtaaagaagttacaacggacgatgagttacgtatctggaaataaggttgaaaaataaaaacggcgctaaaaagcgccgttttttttgacggtggtaaagccgattaatcttccagatcaccgcagaagcgataaccttcaccgtgaatggtggcgatgatttccggcgtatccggcgtagattcgaaatgtttacgaatacggcggatcgtcacgtctacagtacggtcgtgcggtttcagctcacggccggtcattttcttcagcagttcagcacgggactgaattttgcctgggttttcacagaagtgaagcatggcgcggaactcgctgcgcggcagcttgtactgctcgccatcagggccgatcaacgaacggctgttgatgtccagttcccaaccattgaacttgtagctttcaacgctacgacgttcttcgctgacagtacccagattcatggtacgggacagtaggttgcgtgcacgaatcgtcagttcacgcgggttgaacggtttggtgatgtagtcatctgcaccgatttcgaggccgagaattttatcgacttcgttgtcacggccagtcaggaacatcaacgcaacattcgcctgctcgcgcagttcacgcgctaacagaagaccgttcttacccggcagattgatatccatgatcaccaggttgatgtcatattcagagaggatctgatgcatttccgcgccatctgtcgcttcgaaaacatcatagccttccgcttcgaaaatacttttcaacgtgttgcgtgttaccaactcgtcttcaacgataagaatgtgcggggtctgcatgtttgctacctaaattgccaactaaatcgaaacaggaagtacaaaagtccctgacctgcctgatgcatgctgcaaattaacatgatcggcgtaacatgactaaagtacgtaattgcgttcttgatgcactttccatcaacgtcaacaacatcattagcttggtcgtgggtactttccctcaggacccgacagtgtcaaaaacggctgtcatcctaaccattttaacagcaacataacaggctaagaggggccggacacccaataaaactacgcttcgttgacatatatcaagttcaattgtagcacgttaacagtttgatgaaatcatcgtatctaaatgctagctttcgtcacattattttaataatccaactagttgcatcatacaactaataaacgtggtgaatccaattgtcgagatttattttttataaaattatcctaagtaaacagaaggatatgtagcattttttaacaactcaaccgttagtacagtcaggaaatagtttagccttttttaagctaagtaaagggctttttctgcgacttacgttaagaatttgtaaattcgcaccgcgtaataagttgacagtgatcacccggttcgcggttatttgatcaagaagagtggcaatatgcgtataacgattattctggtcgcacccgccagagcagaaaatattggggcagcggcgcgggcaatgaaaacgatggggtttagcgatctgcggattgtcgatagtcaggcacacctggagccagccacccgctgggtcgcacatggatctggtgatattattgataatattaaagttttcccgacattggctgaatcgttacacgatgtcgatttcactgtcgccaccactgcgcgcagtcgggcgaaatatcattactacgccacgccagttgaactggtgccgctgttagaggaaaaatcttcatggatgagccatgccgcgctggtgtttggtcgcgaagattccgggttgactaacgaagagttagcgttggctgacgttcttactggtgtgccgatggtggcggattatccttcgctcaatctggggcaggcggtgatggtctattgctatcaattagcaacattaatacaacaaccggcgaaaagtgatgcaacggcagaccaacatcaactgcaagctttacgcgaacgagccatgacattgctgacgactctggcagtggcagatgacataaaactggtcgactggttacaacaacgcctggggcttttagagcaacgagacacggcaatgttgcaccgtttgctgcatgatattgaaaaaaatatcaccaaataaaaaacgccttagtaagtatttttc

SEQ ID NO: 202 - DNA, 2131 bp, Pseudomonas aeruginosa
  source 1..2131: mol_type = genomic DNA; note = IS21
tgtcagcgccagtgatataagacggtaattcaccatttggattgtccgctccacccaacatgttgtttccttaaggttctcacaccagaaaggacatcaacatgctgagcagagaggacttttacatgataaagcaaatgcgccagcagggcgcgtacattgtcgatattgcgactcagattggttgctctgaacggacggtcagacgctacctcaaataccctgaaccgccagccagaaagacccgccacaaaatggttaagctgaaaccgtttatggattacatcgacatgcgcctggcagagaatgtctggaatagtgaggttatctttgcggagattaaggcaatgggttatacgggcggacgttccatgctgcgttactacatccagcccaaacgtaaaatgcgtccgtcaaaaagaacagttcgcttcgaaactcagcctagataccagctccagcacgactggggcgaagttgaggtggaggttgccgggcaacggtgcaaagttaactttgcggttaatacgctggggttctcccgccgcttccatgtcttcgccgcaccaaaacaggatgctgagcatacctacgaatcactggttcgcgccttccgctacttcggtggttgtgtgaaaacggtgctggttgataaccagaaggctgcggtgctgaagaataacaacgggaaagtcgtgttcaactccggattcctgttgctggccgaccactataacttcctgccacgggcatgccgtccacgcagggccagaacaaaaggtaaggttgagcggatggtgaaatacctcaaggagaacttcttcgttcggtaccgcaggttcgacagcttcactcatgttaatcaacaactggagcaatggatagccgatgtggctgacaaacgggaacttcgccagttcaaagaaacgccggaacagcgcttcgcgcgtgagcaggaacatctgcagccgttaccggatacggacttcgataccagttacttcgacatccgccatgtgtcctgggacagctatatcgaggttggtggtaatcgttacagcgttcccgaagcgctgtgtggtcagccggtatcgatacgaatatcgctggatgacgagttgcggatctacagtaatgagaaactggtggcctcacatcgcctctgttcggcatcgtctggctggcagacagtgccggagcatcacgccccgctctggcagcaggtcagtcaggtggaacatcgaccactgagtgcctatgaggagctgttgtgatgcatgagctggaagtcctgctgagtcgcctgaaaatggagcatctgagttatcacgttgaaagcctgctggaacaggcagctaaaaaagagctgaactaccgggagttcctgtgcatggcgctacagcaggaatggaacggcaggcatcagcgcggtatggagtccaggctgaagcaggctcgtctgccgtgggtcaaaacgctggagcagttcgactttaccttccagccgggcatcgaccgtaaggttgtccgggaactggctggtctggcgttcgtggagcgcagcgaaaacgtgatcctgctgggacctcctggtgtcggaaaaactcatctggccatagctcttggcgtgaaagcggtggatgcgggacatcgggtactgtttatgccactggacagactgatcgcgacactgatgaaagcgaaagaggaaaaccggctggagcgtcagctgcagcaactgagttatgcccgggtgttgatcctggatgaaataggctatctgcccatgaacagagaggaagccagcctgttcttccggctactgaaccgtcgatatgaaaaagcgagcatcatactgacgtcaaacaaagggttcgcagactggggagaaatgttcggagatcacgtgctggcaacagcgatactggatcggttgctacatcactcaaccacgctgaatatcaaaggagagagttaccggttaaaagagaaacgtaaagctggagtgctgaccaaaaacacaacgccaatcagtgatgatgaaatggtgaaaagcggacagcatcagtaacgaaagtatcttagcgggcatgaaaatggcaaataacggtcaaacatcgtggcgttgaca

SEQ ID NO: 203 - DNA, 709 bp, Salmonella enterica
  source 1..709: mol_type = other DNA; note = IS200
tgtctatggaaacccccagctaggctgggggttccggaaagctttcagctttaagccagttattaaaaccccttttgatttgttaaaacatcttgcggtctggcaactgcaaaagttcaacaagaaatcaaaagggggtccaatgggggacgaaaagagcttagcgcacacccgatggaactgtaaatatcacatagttttcgcgcccaaataccgaagacaagcgttctatggagagaagcgtagggcagtaggcagcatattaagaaaattgtgtgaatggaaaaacgtacgaattctggaagcagaatgttgtgcatatcatattcacatgcttctggagatcccgccgaagatgagtgtgtcgagtttcatgggatatctgaagggtaaaagtagtctgatgctttacgagcagtttggggatctaaaattcaaatacaggaacagggagttctggtgcagagggtactatgtcgatacggtgggtaagaacacggcgaagatacaggactacataaagcaccagcttgaagaggataaaatgggtgagcaattatccatcccctatccgggcagcccgatttacgggccgtaagtaacgaagtttgatgcaaatgtcagatcgtatgcgcctgttagggcgcggctggtaagagagccttataggcgcatctgaaaaacctcggctatgccggaggatatttat

SEQ ID NO: 204 - DNA, 1324 bp, Staphylococcus aureus
  source 1..1324: mol_type = genomic DNA; note = IS256
gataaagtccgtataattgtgtaaaagtaaaaaggccatataacagtccttttacggtacaatgtttttaacgacaaaaacatacccaggaggacttttacatgacccaagtacattttacactgaaaagcgaagagattcaaagcattattgaatattctgtaaaggatgacgtttctaaaaatattttaacaacggtatttaatcaactaatggaaaatcaacgaacagaatatattcaagcaaaagaatatgaacgaacagaaaaccgacaaagtcaacgaaatggctattatgagcgcagctttacgacacgtgtaggcacgctagaattaaaagtacccagaacacgtgatggccatttttcacccacagtgtttgaacgttatcaacgaaacgaaaaagccctcatggcttcaatgttggaaatgtatgtatcaggcgtttcaactcgtaaagtatcaaaaattgtggaagaactttgtggtaaatccgtctctaagtccttcgtttctagcttaacagaacagctagaacctatggttaacgagtggcagaatcgtttattatcagaaaaaaattatccttacttaatgaccgatgtactctatataaaagtacgagaagaaaatcgagtactctcaaaaagctgtcatatagcgattggaataaccaaagatggcgaccgtgaaattatcggcttcatgattcaaagtggcgaaagcgaagagacctggacaacattttttgaatacctaaaagaacgcggtttacaaggtacggaactcgttatttctgatgcgcacaaaggattagtctctgccattagaaaatccttcaccaacgtaagttggcaaagatgccaagttcacttcctaagaaatatctttaccaccattcctaaaaaaaattcaaaatctttcagagaagctgttaaaggaatttttaagttcacagatattaacttagcgcgtgaggctaaaaatcgattgattcatgattatatcgatcaaccaaaatattcaaaagcttgcgcatcattggatgatggattcgaagacgcctttcaatataccgtacaaggaaattcccacaatcgactaaagagtaccaatctaattgaacgactgaatcaagaagtacgcagaagagaaaagattattcgcatcttccccaatcaaacatcagccaatcgcttaattggagccgttcttatggacctacatgatgaatggatttattcttcaagaaaatacatcaattttgataagtagaaatggtaaaaacattgtatagcattttacacaggagtctggacttgact

SEQ ID NO: 205 - DNA, 1425 bp, Escherichia coli
  source 1..1425: mol_type = genomic DNA; note = IS621
ctgatgacaaacgcaacattgcctgatgcgctacgcttatcaggccttgtattatccctccagtgcagagaaaatcggccagttttctctgcctgcagtccgcatgccgtatcgggccttgggttctaacctgttgcgtagatttatgcagcggactgcctttctcccaaagtgataaaccggacagtatcatggaccggttttcccggtaatccgtatttgcaaggttggtttcactatggaacatgaacttcattatatcggtatcgacaccgctaaagagaaactggatgtcgatgtgttgcgtcctgatggtcgtcatcgcaccaaaaaattcgctaacaccactaaagggcacgatgagctggtgagctggctgaaaggtcacaagattgaccatgcgcatatctgcatcgaagcgaccggcacctatatggaacctgtcgctgagtgcctttacgatgctggctacatagtgtcagtcattaatcctgcgctgggtaaagctttcgctcagagtgaaggactgcgtaacaagactgataccgtggatgcgcgcatgctggcagagttctgtcgtcagaagcgccctgcagcctgggaagcgcctcacccgcttgaacgcgcgttgcgtgccctggtagtccgccaccaggcgctgacagatatgcacacgcaggaactgaatcgcactgaaacggcgcgggaagtccagagaccgagcattgatgctcaccttctgtggcttgaagcagagctgaagcgtcttgagaagcagataaaagacctgacagacgatgatccggatatgaaacaccgcaggaaactgctggaaagcatcccgggtatcggagagaaaacatctgcggtattgctggcttatatcggtctgaaggaccgcttcgcccatgccagacagttcgccgcttttgcgggtctgacaccacggcgttatgaatcaggtagcagtgtgagaggggcgagccggatgagtaaggccggacatgtgtcgcttcgcagggcgttgtatatgcccgcaatggtagccaccagtaagactgagtggggacgggcgttccgcgaccgtctggcggctaatggcaagaaaggaaaggtgattctcggcgcgatgatgcgcaagctggcacaggtggcgtatggagtgctgaagtcaggcgtgccgttcgatgcgtcacggcataatccggtagcggcgtaaaaatcgcggaagggatgaaaaaaacagcgcctgacggcgctgtgtctggcatgcctgcaatccgggaaaccggaccaggaaaaaacttgcaggccataacagtatctacgcgtcccctgcaatattttgaatttgcacgattttgtaggccggataaggcgctcgtgccgcatccggcataaacaaagcgcactttgccagaaatc

SEQ ID NO: 206 - DNA, 1153 bp, Shigella sonnei
  source 1..1153: mol_type = genomic DNA; note = IS630
aatagctgcgcggaatagtagatcactttgagggaacttagcccggattgtgcgatctgatcaatcgccaaatcaaaacaaatcaccaaccggactgagcaatgccgatcatagcaccaatttcccgtgacgaacgacgcctgatgcagaaagccatccataaaacacacgataaaaattatgcccgcagactgactgccatgctgatgctgcaccggggcgaccgtgtcagcgacgttgccagaacgctctgctgcgcccgttcctctgttggacgctggattaactggttcacgcagtcgggtgttgagggactgaaatcattacctgccgggcgtgcccgtcgctggccgtttgagcatatctgcacactgttacgtgagctggtaaaacattctcccggcgactttggctaccagcgttcacgctggagtacagaactgctggcaataaaaatcaatgagataaccggttgccagttaaatgccggaaccgttcgccgctggttgccgtctgcggggattgtgtggcgaagggctgcgccaactctgcgtatccgtgacccgcataaagatgaaaagatggcagcaatccataaagcactggacgaatgcagcgcagagcatccggtcttttatgaagatgaagtggatatccatcttaatcccaaaatcggtgcggactggcaactgcgcggacagcaaaaacgggtggtcacgccgggacagaatgaaaaatattatctggccggagcgctgcacagcgggacaggtaaagtcagctgtgtgggcggcaacagcaaaagttcggcgctgttcatcagcctgctgaagcggcttaaagcgacataccgtcgggcgaaaaccatcacgctgatcgtggacaactacattatccacaaaagccgggaaacacagagctggctgaaggagaacccgaagttcagggtcatttatcagccggtttactcgccatgggtgaatcatgttgaacggctatggcaggcacttcacgacacaataacgcgtaatcatcagtgcagctcaatgtggcaactgttgaaaaaagttcgccattttatggaaaccgtcagcccattccccggaggcaaacatgggctggcaaaagtgtagcggtattaagcgcagctatt

SEQ ID NO: 207 - skipped

SEQ ID NO: 208 - DNA, 38 bp, Escherichia coli
  source 1..38: mol_type = genomic DNA; note = Region of IS5A that overlaps with ykfC
tcagccgagaagaatttccccgcttattcgcaccttcc

SEQ ID NO: 209 - DNA, 41 bp, Escherichia coli
  source 1..41: mol_type = genomic DNA; note = region of ISX that overlaps with yagB
tgaatcgccacgggtttaacagacacctccgagtcatttaa

SEQ ID NO: 210 - skipped

SEQ ID NO: 211 - DNA, 16 bp, Escherichia coli
  source 1..16: mol_type = genomic DNA; note = region of IS3A that overlaps with eaeH
tcttacccagcaatag

SEQ ID NO: 212 - DNA, 34 bp, Escherichia coli
  source 1..34: mol_type = genomic DNA; note = Region of IS3A that overlaps with ykgA
ttaggcctgtgtccatattacgtgggtaggatca

SEQ ID NO: 213 - skipped

SEQ ID NO: 214 - DNA, 156 bp, Escherichia coli
  source 1..156: mol_type = genomic DNA; note = region of IS2E that overlaps with ydfE
tatgggcgctgcttcgcagacaggcagaacttgatggtatgcctgcgatcaatgccaaacgtgtttaccggatcatgcgccagaatgcgctgttgcttgagcgaaaacctgctgtaccgccatcgaaacgggcacatacaggcagagtggccgtga

SEQ ID NO: 215 - DNA, 37 bp, Escherichia coli
  source 1..37: mol_type = genomic DNA; note = Region of IS2E that overlaps with intQ
gtgataacagatgtctggaaatataggggcaaatcca

SEQ ID NO: 216 - skipped

SEQ ID NO: 217 - DNA, 70 bp, Escherichia coli
  source 1..70: mol_type = genomic DNA; note = Region of IS5LO that overlaps withy yghO
ggaaggtgcgaacaagtccctgatatgagatcatgtttgtcatctggagccatagaacagggttcatcat

SEQ ID NO: 218 - DNA, 1350 bp, Escherichia coli; identical to SEQ ID NO: 74
  source 1..1350: mol_type = genomic DNA; note = insL-2 + 13bp TSD
  misc_feature 1..13: note = TSD
